European Patent Specification EP 3 579 852 B1 - sequence listing, part 2

SEQ ID NO: 2 - DNA, 2500564 bp, Lactobacillus buchneri
aaaagttatccacaggatgtggattctatcaacttttttgtgaataaagccgttgttgtcagctttagttatccacagttgcctgttcattacaccacatttcaaggaccttatccacttatccacaagtgagttatccatttcatccacccctgtgaaacaattatgcacaggctgtttttgcctgtggaaaacttttctggggaatgctaaaattaatttgcatttcgttacacgactaaaaacagagggggaattcgtagtgttagataaggattcattatggcaaaagttaagcgaacaatttcgcagcaacaccactgatcttacatatgacacctggatcaaaccagtcaagccgatcagctttgatggatccacactcactttatctttaccttctgaattgcatcgggattattggaaagaacaattggcaccaaacttgatagagtatgcttttgtgatcactaaaggcaatatcgagccaaagtttattctggattcggacgttaataaagaagcccaagaaaagcctgtggataacaatgtcagccaagatcaggacggcgatgagttttcatttagtaaggaaaatcatcttaatcccaattacacgtttgataactttattatcggcaagggcaatcaaatggcccatgccgctgctttaattgtgtctgaagaacccggcaaactttataatccactgttcttttatggtggcgtcggtttgggtaagacccatttgatgcaggctatcggcaacaagcgccttgaagatcatcctgagaccaacgtcaagtatgtcaccagtgaagccttcaccaacgatttcatcaacgccattcagaccaaccgcaccgaagaatttcgccgcgaataccgggacgtcgacattttaatggttgatgatattcagttctttgcccaaaaagaaggaacccaagaagagttcttccatacttttaacgatctctacaataacgataaacaaatcgtcctcacatccgatcgggttcctcaagagatccccaagctccaagaacgcttggtatcaaggttcgcttggggtctaccagtcgatatcaccccgccggatctagaaaccagaattgccattctcaaaaataaggccaagttggataacctggtcattccaaacgacaccttgtcctatattgccggccaaattgattccaacgtgcgtgaacttgaaggcgctttgtcgcgggttcaagcctattccaaattaaaagatgagccgattacgaccgacctggtttatgaagcgcttcgtggcctcaaattgagccaagataaccgccagctttcaatcgtcgatatccaaaataaagtcgccagctacttccacatttccattaacgatttaaagggcaaaaagcgcatgaagtccattgtgatgcctagacaaatcgccatgtacctttccagggaaatgaccagtaactcgctgccaaaaatcggcaaggaatttggcggcaaggatcacacgaccgttattcacgcttgcgataaaattgccgaaatcatcaaacttgatgccgacttaagaaaagaaatcgcggatatcaaaagtgccctgaactaaaatggtataatcgattgtggataaatcatcgagaagtcaataagttgtgcacagtcttatccacaggttaatcgttagggacaggccacttgtgaaaagttatccacaatatccacatgccctactgttacttctcttttcttttattaattaatatataattacactttccgggaggtcgattaaagtatgaaattttccattggtcgaacagcattcacaaagggattaaacaccgtttcaagagcaatctctaccaaaactaccattcctattctgacaggactcaaaattgtagcaggtcctgacggtctggtactaaccggtagtgacgctgacatttccattgaaaccacgttaaaagccgatgatccagacaatatgttagtcattgaatccgaaggtgccattgtgttgcctgccagattcttcactgaaattgtcaagaaattgcctaaagacaccattactctagaagttggtgaaaacttccagacgatgattacttcaggtcaatcatcatttaccatcaatggtttggatgccaataactatccacaccttcctgaaattcaaactaacgactcaattcctttggctgctgatcttttcaaacagattattagtcaaacggttgtcgcagtttccaatcaggagagtcggccaattttaacaggtgttcactttgtcatttccgataaccacgttatggcggtcgcaactgacagccatcgcttgagtcaacggaaagttactcttgaaaccccgatcaatggttcatatgatttcgtcattcctggaaagagtttgactgaattatccaagatgatcgatgatggacaagatgaagtgtctttatcggttaccgaaaaccaagccctgtttgtcatcggcaacaccctgttttattcacgactgcttgaaggaaactatcctgacaccactcggttaattccagattcacatgacactcggatctcatttgaagcacctgaattactagctgcaattgaacgggcctctctgctttcacatgaatccagaaataacgtggttaaaatcacgattgatcctgacaaaaagacagttactatttacggtaattctcctgatgtcggaaatgttgaagaagaccttgaaccgaagtcattagaaggtaatgaactggagatttcctttaatcctgattacatgaaagacgcattacggtcattcacccaggcaacaattaacattgatttcacgtctgctctgcggccgtttactctcacaccaaccgaggacagtgacagttttgttcagctgattacgccgatcagaacgttctaattcaatatcgattcaccaacaacttccacacgctgggagttgtttttttctgcccaaaatgagttgcttgctatcgatttctttcaaaaatgctgcaatcacatttacataatgtttgaatcctaaaaaatgatcgtcatttcattagaagtccatataggcaccttttagcagtttttgccattttgatgcaaaaatatcaaaaatcttcaaaacggctcataatgcccaagaatcgtcattgacgtgtacttttagtaaacaaagaggtataatagaagaagtaaaaaggtgggtgaaattgtgaaaaaagatgttttcattgatagtccttatatcactcttggacaattactcaaagaagaatcgattattgccagtggcggccaagccaaatggtttttaagagagacaacagttaatgtcaatgacgagcctgacaatcgccgtggtcggaagctgtatgacggtgatcatgtcgaagttccagacgttggcttattttttattcgctcaaagcagggaaatgaatgaagctaaccgaaattgaactgcataattttcgtaattatgttgatcaaacgctcgaattttccgatgggatcaacgtctttcttggtgaaaacgcccaaggtaagactaatttattggaagccatctatgttttggcactcacccgcagtcaccgaaccaataacgaaaaagaattgatcaactggaacagtcagacggcccaaattaaaggtcgcctgcaaaagcggcttggaacggtacccattgaactggatttgggttcaaaagggaagcgggcaaaggttaaccatttggaacaagctaaattgtccacctacatcggtcagttgaacgtcattttattcgcccccgaagacttatccatcgttaaaggagcaccacaagttcgccggcggttcatggacatggaatttgcccagatgagcaatcgctacttgtacaattccactcaatacaaaaagatactgaaacagcgaaatcggtatttgaaagatttgcattataaacgtcaaaaggatcgggtatatctcgatgtgctatccgatcagttatctgcttatggtgcagaaatcatttatcaaagacttcagctacttaaacagctggaaaagtttgcccaaaacgttcattctgaaatttcacaaggtaaagaacagttgacctttgactatcacaccacagtagaggctgaccagttaggatcagtcgagtcgatttatcagagtttactgaagcattttgctgcgattaaagacaaagaaattttgcgtgccaccacgttgattggacctcagcgtgatgatctgcattttgtgattaacggcaaagaagttcagtcatttggatcccaaggtcagcagcggacaaccgcgctttcggtcaaactagccgaaattgacctgatgaaggaacaaacagatgaatatccaattctattattggacgatgtcctttctgaacttgatgatttcaggcaaacgcacttattaactgcaattcaagataaggttcaaacatttttaaccaccaccagtttaagtggcgttcagcaggagttactaaccaatccacgtatttttcggattagtgaaggtaatgttactttggcaaaatagtgaaggagaatcaaaatggccgacgaaaaagaaaccaaaaaagaattagcgcatgaatatgatgccagccaaattcaagttcttgaaggactggaagccgttcgaaaacgtcccgggatgtacattggaacaaccagttcacaaggacttcatcatttggtctgggaaattgttgataatgggattgatgaagcgcttgctggatttgccaccaaaattaccgttaccgttgaaaaagacaacagcatcaccgttactgatgacggtcgtggaattccagttgatattcaaaaaaagacgggcaagcctgctctagaaaccgttttcacgattcttcatgccggtggtaaatttggcggcggcggatacaaagtttctggtggtctgcatggtgtgggtgcttcagttgttaacgccctgtcctctgaactggacgttgaagttacccgtgacggcaaagtttactacatggacttcagtcgtggtcacgtcaagaccaagatgaaagtcgtccgtgaagtttcggatgatctccatggtactaaggttcatttcctgccggatcctgatatcttccgggagaccactacttatgatattaaagtcttaacagcccgactacgcgagttggcatttttgaacaagggattacggattgttgttcgtgacctgcgtccggaaaagccgaccgaacaagactttatgtatgaaggcgggatcaaacattacgttgaatacttggataacagtaaagaaaccttgttggatgaaccaatttacgttgaaggtgtcatgaacggaattaccgttgaagtggcgattcaatatactaacgattatcacaatacattaatgaccttcactaataatattcatacctatgaaggcgggactcacgaagaaggctttaagcgagccttgactcgcgtcattaacgattatgcccgcaagaacaagctgttaaaagacaacgaaccaaacctttccggtgaagatgtccgtgaaggcacgacggctgttgtcagcatcaagcatccagacccacagtttgagggccagacgaagaccaagctggggaattcagatgctcgaacggtgactgaccgcattttcagtgatcatttcaccaagttcttgatggaaaatccaaaaatggccagaaaaattgttgatcgtgggatgctggcctcaaaagctcgttcggcagctaaacgcgcccgtgaagttacccggaaaaagagtggcttggaaatcagcaacctgcctggtaagttagccgataacaccagtaaggatcctaaaatttctgaactgtttatcgtcgagggtgattcagccggcggatcagctaagcagggtcgatcacgtctgacccaggcaattctgccaattcgtggaaaaatattaaacgttgaaaaagcaagtatggaccgaattttagccaacgaagaaattcgttcattatttactgccatgggaaccgggtttggtgaggactttgatttatcaaagattaattaccataagctgatcatcatgaccgatgccgatgttgatggtgcccatattcaaacgctgttgttaacgttgatttaccgttacatgcggccattaattgatgccggttttgtctacgttgcccagccaccgttgtatcaagtccgtcaagggaagatgtcacgttacattgattccgatgatgatttgaatgcattcttaggaaccctgcagccatcaccaaaacccgtgattcaacgatacaaaggtttaggagaaatggacgctgaacaattatgggacaccacaatgaatcccgaaaaccgtcatctgttgagagttgaatcctccgatgcagccgaagcagataaggtcttctcgatgttaatgggcgacaaggtggaaccacgacgcgagtttattgaagacaacgcaacgtttgtggaaaatcttgatgtttaaagttgcttaataactaagcagaaaatgtttcacatgaaacatgccaccgaaacccatgaatggaggtaaataatttggcgaataaagataaccatgatgaaccaattgctggtcgagtgaccaacgttgatctatctaaaaaaatgcgaacgtcatttcttgactacgccatgagtgtcattgttgcccgtgcgctgcccgatgttcgtgatggtttaaagccggttcatcgtcgtattttgtatgatatgcatgaattgggtgtgacacccgataagccttataagaaatcagccagaattgtcggcgatgttttaggtaagtaccatccccatggagataccgccgtgtatgagtcaatggttcgaatggctcaggactttagttaccgttacatgttagttgatggtcacggaaactttggttcagttgatggtgatggcgctgcagcgatgcgttataccgaagcccggttaagcaagattgcgatggaaatgctgcgtgatatcaacaaagataccatcgatttccagcccaactatgatgggactgaacgtgaaccaagcgttttgccgtcacgattcccgaacctgttagtcaacggtgcgtcaggaattgccgtagggatggcaactaatattccacctcacaatttgtccgaagtcatcagtgccattcatgttttgatgaagaaccctgatgccactacagcagatttgatggaggctttgccaggacctgattttccaaccggcggcgttgtcatgggtaaatccggtattcggaaagcctatgaaaccggtaagggaaccattattgtccgcgccaaagttgaaattgaaggggaagccggcggcaaacagcgaatcattgccaccgaattaccttacatggtcaacaaggccaagttaatcgaacggattgctgaattagcccgcgataagcggattgaaggcatcactgatattaacgatgagtctgaccgtgaaggaatgcgggttgtgattgatgttcgtcgggatgcaagtgccgaagtcatcttgaacaatttgtacaaattaaccctgatgcagacttcatttagtttcaacatgttggcaattgtcaaaggcacgccgaagattttgagtttgaaagaaattttgaactattatctcgagcaccaagttgaagttattcaacgacggaccaagtatgagctgaacaaggctcaggccagggctcacattctcgaagggttaaggattgcccttgaccacattgatgaaattatcaaaattatccgtggttcacagacaggtgacgttgccaagaaccaattaatcgaaggctttggtctggatgacaagcaggctcaagcgattttggacatgcgtctggttcggttaaccggtttggaacgcgaaaagattgataaagaatacaatcaattgatgaaggacattgaagaatacaaagcgattcttgccagtcgtgaacgggtcaatgaaatcatttatcaagaattattggagatccaaaacaaatttggcgatccacgacgaactgaactcttggtgggtgaagttctgagtcttgaagatgaagatttaatcgaagaagaagacgtgatcatttctctaacgcataacggatacatcaaacggttaccaacttctgagtttaaagcccaaaatcgtggtggtcgtggtgttcaaggaatgggtgttcataacgatgatttcgtagaacatttagtttcaacttcaacccacgatgtgctgttgttcttcaccgatgccggtaaggtttatcggatgaagggttacgaaattcccgaatatggtcgttctgccaagggaattccagtgattaacctattgaacattggcaataacgaaaaaattcaggcagtgattaacgtttctgataagaacaacgatattgaaaaggatcttttctttgtcactttgatgggaaccgttaagcgcaccccagtgtctgactttgccaacatccgtagtaatggtctgaaagccattaacctcaaggatgatgatcaggttagcaacgttctgattgccagtgaggatcaaaacattatcatcggaactcaccgtggctacgcggtcagctttaatgctgccgacgttcgttcgatgggacgatcagctaccggtgtccggggtgttagattacgtgagaacgattatgtggtcggttctgatatcttgaaacctgacagtgaggtctttatcatttctgaaaatggctatggtaaacgcactccagctgctgaatacccaattaagggccggggcggtaaaggaattaagactgccaacatcactgaaaagaatgggccgcttgccggtttgacaacggttaacggtgaggaagacatcatgctgatcacagaccagggtgtcatgattcgattcagtgttgaggacgtttcgcaaacaggtcgggcaactctcggtgttcacttgatcagaatgaccgatggcgctaaagttgcaaccatggctaaggttgagaagcaggatgattcagaggatgacacaaaagatcagtcatctgattcagaacaagcaagtgatgattccagtaccaatgccgatcaaaactcagattcagataattaatattcagctaattaaaaagtcgatgagatttaattctcaccgacttttttgtttcacgtgaaacataagcatgaattctcctaagaaaatggggtaaaaaagtcgagctaattctttgacttacttttcgtaagtgatatgctttttgtaagaattaaaatacgactacctggaggtaatttattcatgactgttgttaatggttacaaacaaaacgataacgaagaaaaaattaatattttaaacttggaagagttggaagaacgagctaagcaaatcattccaactggcggttttggatacatcgtcggtggttcagaaaacaactggactttaaaagccaaccgtaaagcctttacccacaagcaaattgttccgcgtgctttgagtaatattgaaaatccatcacttgacactaacgtttttggaattccgctaaagacgccaattatgatggcaccaactgccgctcagggattggcccactcacaaggtgaaaaggatactgcaaaaggtgtcgctgccgttggtggtttgatggcccaaagtacctactcatcagtgtctatttcagatactgctgcagcggggaatggtgcaccccaattcttccaactttatatgagtaaagattgggacttcaactactcattgcttgacgaagctaaaaaggctggcgtcaaaggcattatcttgactgttgatgccaccgttgatggttatcgtgaagacgacatcaagaataacttccaattcccaattccaatggcaaacttgactaaatttagtgaaggcgacggtaaaggcaagggaattgctgaaatctatgccgcagctgctcaaaagattgggcccgatgacgttaagaagattgctgactacactgatttgccagtgattgttaaaggaattgaatcaccagaagatgccctttacgcaatcggtgccggggctgccggtgtctatgtatccaaccatggtggccgtcaattaaacggtggaccagcatcattcgatgttttggaagatgttgccaaagctgttaacggccgtgttccgatcatctttgattccggtgttcgccgtggatctgatgcattcaaggcacttgcttcaggtgcagacttggtagccatgggccgaccagttatctatggcttggctttaggtggtgctgaaggtgttcaagctgtctttgaacatcttggtgacgaattgaagaccacgatgcaattggccggaaccaagaccattgccgatgttaagaagacccaacttctaagtatcaactattaatttgtgtgcaacgtcctatcatccgtatcctctaacagaaatgtttaggcatttgcttctgttctcatgatgggaaataatattagaggatacccatgagtgctgcacagtattagaacattccccgtgttcttttccccaaaaatatgtaataaaacagcgttcctcattattgagggacgctgtttttggatcagattttaggttaattaatatttttgcgtggtcggccggttgtttggcctttatccagaatttctgggtgctcgttacgtgcataagcgtatgcatgaggatcctggccgttttgatatcgacttgagcgggtgttggtttgagaacttctgaagtagtaaaatgctgaaaccccaacgatgattaatagtaaaagtgtcattgaattcctcgtttctttatttttgttaaatcatgggacacgtgcgaaaaagcgtttccaaacttcaaattgaatttggaattgatactagtttacttccaaaatcaaaagagtcaagtatctgcttgaccgccgtggatgatttactggttagacccaagtgtagcaaggggttcctaattattaaggaattatttaattcctgatcgtgaattattttctccaaaagaataatccaggtggtttctatcgtatataataagtgtatcgtgaatcacaattaggcaattgatatttaggtccacacgtggtattattttatattgtgagtatctgggtaaaaacagaaactctccttgctctcgggaagagggccataagtccataaggaggtgcaaatcatggaagaaaagaaatacgaaattacttacatcatccgtcctgatattgaagaatctgcaaaatctgcattgatcgaacgattcgacaagatcttgactgacaatggtgctaaggtactaagttcaaaagactggtcaaagcgtcgttttgcttacgaaatcggtggcttcaacgaaggaacctatcacgttgtaactttaacaactgattcagacgcatcactcaacgaatttgatcgtctttcaaaaatcaatggcgatatcttacgtcatatgatcgttgttcgtgacgactaataattgattctaatatgagaggagcaaattcagcatgcttaatcgtgcagttcttacgggtcgcctaacccgcgatgttgatttacgatacactcaaagcggaaccgctgtcggttcgttctcacttgccgttgatcggcaatttaccaatcaacagggggaacgagaggctgatttcattaactgcgtaatctggcgtaaatccgctgaaaactttgccaacttcgttcataaggggtcgcttgttggaattgatggtcgtattcagaccagaaattacgaaaacgcacagggacaacgtgtttatgtgaccgaagttgtagtagagaattttgcgctgcttgagccccgttctgcaaggaacaactcaaatggtcagcaaaatggcaatgctcctcaacaaaataacggtaatgccaatacatttgataatcattcaaatgccggtaccggtaatagtggcaattccaacaataatggcgggaataatcctactaacaatggtggaaataacggtaataacgggaacaataatcccaatgatccgttcgctaactctggggactcgattgacatttccgatgatgatttaccattctaatgaattggtaaagtaaattttcgaggaggaaaaactatggcatatcaaagacgtggcggcggtcgtcgtcgtcgtaaagttgattttattgctgcaaatcacattgaatacatcgactacaaagatatcgatttattgaagcgatttgtttcagaacgtggaaagattcttccacgtcgtgttactggaaccagcgcaaagaaccaacgtgctttaacaattgctattaaacgtgcacgtatcatgggcttgatgcctttcgttgcggccgactaataatgatttatcgaagtcatcctttcggggatggcttttttatttgctcacaagaaaagccttcccagaaactgaaccaggaaggcttgtatcgacatcaattagttttcgttagtaacgggcttggcgttgtcaacttgttgatcaggtcctaatttctttaaaccgaccccggtgaatccactcaatagtgagaagactgggcaaagtaggctgaagaatacaaatggcaggtattggatagttgggacactcaaggtgttggcaatgaagacaccgccaacgccccatggaaccaagtagtttaaaacggtaccgccatcttcaagaacccgcccaagggctcggctggccaggccaccgttattgaacgtctttttgaaggctcgtccaggtaagataatcgaaagaatttgttcaccaacgaagatattcaccccaatgcaggctcccagggccgctgtaactagtttggccggattattcaacctggtagccagtggtgacataatcgcgctgataaggccaaaatggactaatagaccaccaagcgataacgtcagaacaatgagcgcaactgtcggcatcatgctgacgatgccgccccgtgaaagtaataagttgacctcactgttagaagtctttgcgataaagccgttggtgatgatcgtgctggctttggtgacgtttaatccagggttattgacaaacatcatccctgctgaaacaaagatgttcagtagcatggttggaatggccgccattttaaagccggcgcagacaaacaccaagatgatcggaatcaaggcgacaattgaaatgtgaaaatcgttgttcaatgcggcaaccgttgtattgatcttattcatatcagcatggttgtgacccattccaagaagagcaaaggcaatggtggaaatcgtggcagctggaatcgtcgaccaaaggatggttttcatgtgatcaaataagtcggtgtcgaccacggctgctgccaagttgttggtttcggaaagtggtgaacatttatcaccgaagaccccgccggaaataatcgcaccagcgaccagggccggattgaagttcatggtgacaccgatgccgaagaaagcaatcccgacagttgagacaaccgtgaaacaactaccaacggcggcaccaaccagtgaacagaccagaaagacagtcggtaagaaccattgggcactgatggctttaaagccgatgaccatcaacgttggaattgttccagcggcgatccaggtactgatcatcgcaccgattaagataaagatgacaatggggatgatgcctttatcaatcccatccttaatcccggcattgatctcatcccaactaaacccagtcacttttgcccaaaagattgtgacggtaattgctaataatactggaacttgtggagacaatcccaaaccgattaccccggttcccataatggctaatgcaacaactaatactaaaatcgcttcacgcaaactcactctactatttctcatattgccaacctctttttattttcaaatttttgtctactttaaattcagttgactcaaatatcgtggtaaaccgccattcgttgctcttctcatagaaaatcccccttaagtcaataaaaaatcgtccctactgcatataaatgcaatagggacgattttaaccgtggtaccacccaacttgtgtatcaaaaatacaccgctcactagaagataatggattctagttattgaccattgtcgtgatattacggtatttcgccaccttaccctgattggttcgcagcaaccaccaacttcctgacacccagataaggcactacttcatgtaattcgactttaattattaaagagagtataaaacttgatgagaggaattgcaagaaatgtttccatgatcgattgctgggaatgacgaagctcataatcccccaaatgcacattgtcgttaaataatcttagcaattcttccccattcgcctaagattatcgaaaaaattcttattttcacctttttaaataacaaaatgtaaccaaacctaacatcaaatgcctatttatgataatataaatgcattctcattagaactttttaatctaattcttatgttgctcttatttaggaggatgcctatgaagtcaaaaattcaagagaaccaagatggaaccatgcgtgcgttaagtaatcgtcacgttcagatgattgcgattggtggaacgattggtaccgggttgttcctgggatctgggagcaccatcagtaagacgggtccctcagtcatgctgatctatttggtacttggcctgtttttctttttcatgatgcgtggaattggtgaaatgttctattccgatccgtcgcaacatacattcgtttcatttatttcccgttatctgggtccaacagttggtcattttaccggctggacatactggattgggttggtattcgtttgtatgggtgaaatcagtgccactgcaacatatgttaaattctggttccctcaggttccggcttggattattgaagttgttttcttaggagttttagctggaattaatttaattgctgcacggttgtttggagaagctgaattctggtttgcaatgatcaaaatcgttgccattctggcattaatctttactggaatctttatgatgttcagccactcggtgacgccacttggccatgccaccattggtaacattttccacaattttcaactatttccccatggcggtgtgagttttatcgctgcgttcccaatggtcttcttcgcattcatgggaattgaattcgtcagtatcacaattggtgaagctaaaaatccgcaaacggtcatcaaaaaggccgttaatgaaactttgattcggatcttaatcttctatattggggcattgactgtgattatggggatcatcccatggtcatctattacccctgacagcagtccctttgttcaagtattgaaactcgccggattaccagcagcggccgctgtgattaactttgttgttttaacttccgccgcatcatccttaaacagttgtatcttctcagccggccgacatttctatcagttggcaacagaagttcccgaagacagctggatgcgaaaaacgtttgctaaaatttccaacaatggtgttcctgcccgagcaattatcttctcggcagcactggtcttgattacgccactgatcagtttgactaacagtttggcgtcggtatttaccatcgtaactggaatttccagtgatatgtacatcattgtgtacaccttggcaatgctggctcacagaaagtaccgtcaatcagctgacttcctgccaaatggcttcttgatgccggcatacaagattatgagtccgctgacaatcgcatttttcgtggtcatctttggttcattgttctttgttccagaagacattattggtgctgttggtgcaattgtctggacggttgttttcggtgccgcaacttatatccatcaaagacgattggttcccgataccgaccagtaattgtctaacaattcaatgaaatgaatttgcatgtctcttccaataaatatcatatgacgactctgaaaaattcccgacagtgatgctggggatttttctttgcttcatcattgagatgagaacccaccagaaataataaagcaggccgatttatggtaaaataagagcattaagctattatgaagaggaattaacatgaaaaattggttcacaaacaaccgtggtgaactgccatcatttgttcataaccgacgcctcagaagaatcatgatgttcatttcattaatcgtgatctacggcatcgttatttcatttttatataatatcgtggcttccctcattctcattgtgatcagtgttgtcggcctgatttttaccatcgtcatgatgaacgaaatcagttccgataccaaccgctatattaccgacttgtcatacagaattcatcgtggggaacaggaatcgctgctcgaaatgccgatcggcgtcatgatcttaaatgacgacgaacaggtggagtgggcgaacccctatatggtgaagtattttaaggatgagaatttgttgggtcgaaagatcgacgacatcgatcatgacctccagcagttaatcaccaagtacgccgaatcagatgaattccacacgatcacttggcgggaccataagtttaccatgctgatccaaaaggaatataactcggtctatttgatggatattacccggtatgccaacctggaagaacggtacaacgaagagcagatctccgttggtcaaattttcctggataactatgatgaaatcacccaatcaatgaccgaccaggaaatctctaatttaagcaactatgtgactaacgaattggcaacttggtcccaaaaatatgggatgtatctcaagcaaatcgatgatgaccacttcttcctgctggcctactcaaagtcgctaaccgcaattgaaaatgacaagttcaacatcttggacactgtccgagagacgacttccaagcaaaacttcccactgacgttgagtatcgggattgcttacggcgaagatgacctgaataatttggccgaccaagctcaaagcaaccttgatttggcgttaggtcgtggcggtgaccaggtcgttgttaaatcattggatggtaccgcgcggttctatggcggcaagaccaatccaatggagaagcggacccgggttcgggcacggatgatttctcaagctttaaacgaattgatgagtgcctcagatcaggtctttgttcaaggccacaccagaccggacatggactccttgggtgcttgtctggggatcagacgaattgcccaaatgaataataagaaatgctggatcgttcttgataaggagaaggtccactcagatattcaacgattattggaagccaccaagaagtacccggaaattgccgattcaatcatcaccccttcagaggcgattgccaaagcaactgacagcagcatgctgattatggttgatcattccaagccttcaatcagcatttcagaagacttatacaagcgaatgtcagccaaagtggtcattattgaccaccatcgccggggtgaagagttccctgagaacccaatgctggtatacatcgaaccatacgcatcatcaacttgtgagctgatcacggaaatgtttgaatatcagccacatgaagaagaaccaatcaaccggattgaagccaccgcaatgctaaccgggatctttattgatactcagcgcttttcaatgcggactggtaccagaacctttgatgctgccagttacctgcgttctgcgggagccgattctgatgaaatgcagcaatttatgaaggaaaatattgatagttacctgcaacgcaaccatctaatttccaaagttgaattcttccacaagaatatggctttgattgttggcgaagaagaccaggtttatgatccggtcacggcggcccaggcctgtgattcacttttgacaatgtctggggttgacgcatcattcatcatcaccaaacgctccgacggccaaattggcgtttctgctagaagtaccggtgccgttaacgttcaagtcattatggagcaaatgggcggcggtggccacttatccagtggtgccacccaggtttccgacaagtcggttgccgatgtgaaaaaaatgctgcttgaaacgatcaagaatatcgatgataatgaataaaggtatttaaatttttgaggatagtaggagtgatctgttatgaaagttatttttctgcaagacgtccgtggtaaaggtaagcgcggggaagttaaagaagttcctgacggctatgctcaaaactttctgattaagaatggaaaggcaaaggcagccactaaagcggcaatgagccagttaaagggccaacaaaaggccgaagaaaagcgtgaggaagaagagctggaggaatccaagcagttaaaggccaagcttgaagacgacaagacagtcgttgaattgaaggccaaagctggaacggacggccgtctctttggttcaatcccaagcaagcaaattgccacagcactggaaaaacaatacggcgtcaagctcgataaacgcaagattgaattaccggaaccaattaaagttgccggctacaccaacgtgccggttaaattgcatgttgatgtgaccgctaagattcgggtacatgtttccgagaaatagagcgcgaacaacctttatccaggtaaatgtaacagagactcctcacaaaaggaccaccttgtgggtgagtctcttttcttctccaatctgaccagatttaaggggagtgtgctacaatttaactattgtatttaacgtgaacgaatttgaggaataaacatgagcaatgagtttgtaaacgaattaccaccacaaaatatcgatgcggaaaaggccgtccttggatcgatttttctgagtaccgatgctttggttgagtccatggagttcttagagcccgatgacttttataagcacgctcaccaaattatctatcaggatatggtcactttaaacgaccgcgatgaagcaattgatgtggtgacaatcaccaacattttaactgaacaaaataacttggacgacgttggcggcatggaatacatcgccgatctggctggttccgtcccaacggctgccaacgtggcttactacgcaaaaatcgtcaaggataaggctattttgcgccggctgatccagactgccaccaacatcgttactaacagctataataccgatgacgatgtcaccacggtcttggatgatgctgaacgagacattatgaatgtggcagaaaatcggactcagtctggttttaaaccgatcaaagaagtcttaaataacgcctttaacgaaattgaccgcttgtcccaagaaggggatgcggtcaccggcctttcaaccggttatccggaactcgacaagatcacaacaggtttgcacagcgatgagctgatcattttagctgcccgaccggccgttggtaaaacggcctttgccttgaatctggcccaaaatgtcgggaccaaaacagataaaactgttgccatttttagtttggaaatgagtgccgaatcgttggttaaccggatgctgtgtgcggagggtagtattgatgccaaccatttgcggaccggtcaactaactgaagatgagtggcagaatctggtggttgccatgggcagtttgtctcgggccaacatttatatggacgatacggcggggatcaagatgtctgaaatccgcgctaaatgtcgacggctggcgaaggaaaccggtaacttgggcttagtggttgtcgattatctgcagctgattgaaggcagtaacgccgaaaaccggcaacaggaagtttccggcatttcccgtcaattgaagaaattggccaaggaactccatgtcccagtgattgcgctatctcagctttctcgtggggtggagcaacgccaggataagcggcccgtcttatccgatatccgtgaatcaggttcaatcgaacaggatgccgatatcgtcgcctttctttaccgtgatgattattatcgtgatgaagacgatgatagtgatgattccggctctgagggtgaagacgacgaaaataatgtcggagaagttgaggtcattattgaaaagaaccgatccggccctcgtggaaccgtcaaattgttattcgtgaagtcgtataataagttttcgtcgatttcctatgctcagcaacagtaaaatttaccttgatatcattaaagcggcctttggagagttttccattggccgtattttaataccgttatatttgttgaaaatggacttgttaagattaatttgattttataaacaactataataaaaccccttaaattagatttctccaattaaaggggtttagtttagacatttaacttatcctgattacatttgttaaaacttggtcggaataaccgcagccaaaccgcgtcgttctttgccgcgataaccaatccagactgccagtgacccgattaccaggccaccaagtgcaacccaccagagggtctgctggaaggcacctgtgttgccaagattagccatgatgttataactgctgtagatgttttggtacattggcgtcgtttgacttaagaacttgtagaaactggtcatggccgcccgtgggagcgttccgccaccagccatgatttgaaggacgaacagtggtaattgaatcagcaaacttggtaggccgccaaatagaagtgccaagccgctggtaagttcgaaggctgcaaaatcgtacaagacattttgccaaagcaaagcgttgaaaaccccaccgtcaaagctgacgaggcaccgcagcgcaccaacggtcaataatgctaaaacaaccgcggtgataacgccggtgacttgaaggccaaggaaggttttccacttgccggcgatgaagcgaaccgacatgaaggtcatcgtaatgatgattgaagcgatcatcaggcccaaatattggcccatcgagataaacatcggtgccatctggtgctgcatatttacctgcttggtacccatggtatcggtcgatgatttagccgtaatgttaaatggtgctgccatcttagtggcccgagccatgacttgcttttggatcttgggttgtacttttgcttgaacctgtttttggatctgtttttgattaacagcctgaccttttgaggccgtcatggctttttgcatggcggtcttcatcccagtagccattgcggttttcatcatcttaggcgcaagttgtttggcatacatgccgacaagtgactgttgggtcaactgggcgttaactgtactttggatccgggagatcagtccctgattaacattggtttggaccatactgttggcgttgttgacgacaaaattaacggttggtcgtttgccggcacgaacgtccttattaaatccatcgggaatcacaaccgccagagatgctttgcgaagttcgattcggtgtttggttcggcttaggctactcgaagtcgaaatatgcttgaagggcaggttgtccttcaaaccgtcggcaaccttatccgagatctgttggttatcttgattgacaatgacgattggtaagttttgagtattggttggcatgtgcttgaaagccggtagaatgcagaatacaaacgaaactgcaataaaactggcgactaacattcccagccaactaaatttatttgaaaaccattttgacattttagttgttcctccttaaaataacgaatgaatgctcattcatttttgtaacttagcaacaataatctttttctaaacaaatgtcaaacacatttgaaaagtcattccaagtccgctaaactaaaaacgaaatgaggtgcgagctgtggctgatgcagagaatgattttcaacaattatataaagagacgctcaagaaaatggacggcctgacagataagcagaaacggattctccaggcggccctcgaattattttccacccaaggctttagtgaaacctcaagtgcccaaattgctgatcgggcaggcgtggccgtcggttcggtctatcagcgtttccacaataaacaggctttattggtggcggtactggccccactcttaaacgatgtgttgcccaaagccgttgacgagtttggcaatacggctttcagcaagtcttacgatgaggtcgagccctttgtcagagcaatcgttcctgatcggctgagatttatcgatcagaactacgctgccttgaagctacttgccggacaggtgattgttgaagatgaggggattatttcacagcttacagaggcctttagcagtcacatatcatccaacgtgataccgaatatcaaacatctgcaaaagaccggcaagatggctcggttcccggagcgttatgttattcaattcctgttttcgtctgtcatcggctattttggcaaacgaattctcggcattccggtgaacattgaagatgaaattaagtatatgaccgtttttttgacgaatggactaacagatcataacgtcaaatagctgcccatcatcctgtgaagggatgcagtggacagctatttttaggcaaaaaaataacaaccacggctacgagtagctgcgtgatcgttatttaatggtatgtaattgatgggcagtcaggggctcgaaccctggacccacggattaagagtccgttgctctaccaactgagctaactgcccattactaaccgacttaaatataatagcatatgctcaaaatatttgcaacacggaaaagggtatttatttgaccaatatcggtctgtgttataatagcaacatgttggcgtgtgcaaattttagaaaataacaatattaaaatccatgttaggagaaattgttaatggcaaaaaagatactggttgtcgatgacgaaaaaccaatcgtcgacattgaaaaatttaatttaactaaagaaggctacgaagtctcagtagcttatgatggtgaagaagcattgcagcaagtcaaagacgttgatccggatttaattatcttggatttgatgttacccaaagttgatggccttgaagttgccagggaagtccgtaagactaaggacaccccaatcattatggtgactgccaaagattccgagctggataaggttcttggtttggagcttggggctgatgattatgtgaccaagccattctcgaaccgagaattggtcgcccgtgtgaaggctaacttacgtcgtcaggggaccaatagcagttccaataacgaagaagacgaaaataaagacatcaagatcggtgatttggtgattcatccagaggcttactcagtttccaaacggggtgaaaacattgaattgacccaccgtgaatttgaattgttgcattatctggcccaacacattggccaagtcatgacccgggagcatttactgcagaccgtttggggctatgactattttggtgatgtgagaaccgttgatgtaactgtccgccgcctgcgcgaaaaagtcgaggatagtccgagtcatccaacctggctggtaacccgtcgtggggtaggttattacctgcgcaacccagaaagtgatcaagcataatctcaatgaaatcaatgcataaggggtattaactggttgtgaataatcgaattaaattttaccaatcaatcaaatttaagatcgcactggttttcgccctgatcctcctggtaacgctggaaatcgttggtgcggtctttgtcaggcagctggagcatcaaaatttggcaacctttaagaaccaaattcagctgcagacctacgtcaccaattcattgacgactcaattgtcgagtgccgatgaaacaaaagccaacggtcggatcaagactattttgaatgattccgatagtggtaataccgcgcaaattcaagtcattgataataaagggacaattcgcggtaccaatcagattaacaaccaggcgatcgttggccaaaagaccaccgatgacaacgtcaagaacgcaatctacaacgggaaaaaatttgaaaaaacaacctatgattcttcaactggtgcgcgttattacaccatgatttcaccgttgattaagagctccaacaataatagtacggtcgtcggggtggtatacacccgggcgaacctcgacagcgtctatgacagtattaacagcattacgctgatttatctgttcgccgcgtcgattgccattattttggggttattaatctcgattgttatttcgcgagcgattacgcgaccgattgaagaaatgaagaagcagaccatcagaattgcccgtggggactattccggccaagttcacgtttatggaaacgatgagctgggtcaacttgccagtgcggtcaacaacctatctgtcagggttgaagagtcccatgagtcaactgagtctgaacggcgacgcttggattcggtcctggcaaacatgactgatggtgttttggcgaccgatcggcgtgggaacgtgattatcattaatgaaacggccgccagtttcttggatcttgatgaaaatcaagccatgggcaagtcgattttggacgtgttggatattcgcaaagactacagtctgcgggacttgcttgaaaaaccggatgagttaatccttgatttttcaagtgaagatcacagtctggttttgcacgctcatttttcactgattcaacgggaatccggctttattagcgggctggtctgcgtgcttcgtgatatcaccgagcagcagcgaatcgatcaagatcgcaaacagtttgtgtccaacgtttctcatgaattgcgaaccccattgaccagtgtccgttcgtatattgaagcactgtccgatggtgcttggaaggatccgaagctggcaccgaagttcttaaaagtcactcaggatgaaactgatcgaatgattcgtatgattaatgacctgttaacattgtcacggatggattccgggacgcagaagatggaagtggaactggtcaatatcaatgaattgttcaattatgttttgaaccgatttgacatgattcttaaaaaagaagatcatccagaaaagacctatacgatcaaacgctactttaccaagcgggatctgtgggttgacctggacaccgaccgctttacccaagtgttggataatttgatgaataacgctatcaaatattcaccggatggcggcgtgattacttgtcggctctatgaaaccagaaataaggtcattttaagtgtcagcgaccaagggttgggaattccccgaaaggatattccgcatatctttgaccggttctatagagttgataaggcccgttcccgtcagcagggcggtagcggtttgggcttggcgatttccaaggaaactgtcgaggccttgcatggccaaatttgggccgagagtgtggaaggcaagggatcaacgttctatattgctttgccatacgaaccggtagaagaggaggacttgtgggatgaggtttagtaaatacttaataccccttgcgctcaccattgcggtggttgccagtctaacgctctcagtggttctctggaccaatccggctaattatcggaccaataagcaaacggcgcaaagcccgcagacgcagcagatgattaagcccaaacggtacgtctactcaccggttcaggcgattcatacgaatgcggacgggacccaacagattatggtcaacaagttagtgaacaccgtgactgagattaagaaaacgatgcatcattatcaaaatccgcggatgaaaactttaagcaaaaattcgcaagttgactattttcgaatcgctaaccaaacggattcgattatgctgaactattcagacacggtttcgatgcgaacatttaacgcaattgtcagcaatcgattccggaagctgccgaacatcaaaattaaccgagttgttttgccaaccaacaattcaaccaaactgtatcttctctatgataaaaacttcacggtgtatgaagtcgatgttaaaaagcacagtttaaaatctttgaacaaagttctgcagatggacatgcggacacaaccggccagcttcaagttattaaataatcggccaactgtctacgttaccagctctgtgcagatgcagccttataagtatttgattgaccgtcaatctgacgattactatgttagccgactgctgaatactcaggattcaaccagcattaacgttaagcggcgaaagaatatgacgatctacggtgatcaaagttccctgcaattaacgtttaattccaggaatcggatggcagaattttctgactttcggccaaatcataaccgccgcagtttgacgtcaacgattaacgattcctacaagaatatcactaagctagggctgccaatggataatgtccgtttcttcagctatgatccaaagagccggacggtgatgtatcggacctatgttgaaggtttcccaatttttcgagccagtggctttggcactgtctcgacgcggacactgaactccagtgctcagcggatccaattctcattggataatcccgaggtgccgctgccaagtaacaaggggtacgtttcgctgccgtcaactgaaacaatgctgaagcggctggtcaatcgtgggtacaatttaaaggatcttcaaaaagtccgtctgggttatacttggaagaaggattccacgtctccattattgattgacctgaatccagattggtacatctattacaagaatcaatggcgctcttacaccgcacttatgaaccaatactaggaaaggagggagcctggtgaactttcgaagaattgagatcatctttttggtgacctttatcgcaattgacatcttcttgtttgggatgttcaaaaagaacatggacatgcaggccgacaacgtgtcgcaaggcgactcggattcagtgatcgtcaaggaaatgcgtaacgaccagattaaagttggcaacttgtccaagaagaacgaaactgcctattatatttctggtgaacaaagcgacgttttgcgtaaccagatgggacaattggttaaccagactccccaatttgttggtcatgagctggaaagtgaacttaagcagcccatcacggttgataagaataatccacgcaaatcaattgataaattgctgacggattccacgtttgtgttgtttggtgaccagtacgtttacagcaaaaacctttcaaccagtcggaatatcgtttacaatcaaaaggcgatgggaagttcgatttactcctctgaagcccagatcagatttacgctgaattccaattatcagattgtcagttatactcagtcgtatctgcagggaatcaagagcctgcgcgaaagttcggaaaccatttcggaaacccgggcgttaatttggttgtatcagtataatgagattccgaataacactacggttgcatgggccagccttgggtataccaagttattgtcaatcgatggcgatcgagtctttattccaacttggattatcgcgattagaccacaaaattccacccaagttcagttgaaacggatcaacgcgtttacgggtggcattatcaaacaaactgatgagaatttaaagaatagtcaaacatcaatgaattaaagttaggaagaagaacggttatgaataatgatgatatgaaaatcagcgtcctcgccagtggcagtggcggtaacgtgacttacatcgaaacgccggaccacaaagttttgtgtgatgccggattgagcggtaagaagattgaagcgctcatgaattcgattggtcgagacctcagtgacgtcgactcacttttcgtgacccatgagcattccgatcaccgactgggtgccggtgtcttggcacgcaaatatgggattcaagtctatgccaacgaaggcacctggaatgccatggcaccaagaattggcaaggtcgctgacgatcaaaagaacatcattgccccggacagtgtgatggatatgggcgatcttgatgttgaaagcttttcggtgtcccacgacgctgcagagccacaattctatgtttttcatcataataacaagtcgtttgttatcctaactgataccggttatgtttctgatcgcatggaaggcgtcatcaaagatgccgatggttatcttttggaatgtaaccatgatattgaaatgctggaaaatggcgattatccttggatgaccaaaaagcggattttgggtgatcaaggacatttgtccaatgaagatggcgccaacaccatgttggatgtcatcggtcatcggactaaaaaggtcttcctaggtcaccgcagcctgcataataacatgaagacgcttgcccacttgacggtggcttccatcttggaagaccacgatatgggtgtcggtgaggactttaagctgtatgatacatctcaggaccacgcttcacctttaatgattatttaaaaatcctttagatatttctaaacttttaaacacactttcgtcatgaaaaaagtatattataggtaatataaaataataagggggcacactaattggcacaaaataacggatttggaaaattcattgcgaccgttgtgatcgctggcgcacttggcggcgggattacttacggcggagtttcttattttaacaacaataataatggaactggaacagagctggtttctggtacgaacaagaatggcaataccaaggtcagcaacgtaaaagttaatctcaatactcaggcagaaaaagcgtttaacgcaactaagagcactgttgtttccgttattaatttacagaaacaaagttcaagcgacgacaccttatctggaattttgggtcaaattcaaggtggttcttccagcaaaaagaagagcagcggcgaacttgaagcctcaagcgaaggatccggtgtgatctataagaagagcggcaatactgcttacatcgttaccaacaaccacgtggttgccggtgccaatgccctcgagattattctcagcgatggctcgaaggtttccgcttcggttgtcggtaaggatgccgtttctgatttggccgttatcaagattaactctgacaaggtcaagaaagtcgcaacttttggcgactctgataacatcaaggttgccgaaccggttctcgcaatcgggtcaccactgggctcacagtacgcaacttcagtaactcagggaattatttccgctaagaaacgggaagtaccgcaaacttcagagagtggccaacaaattggtaacgcaacggttattcagaccgatgctgcgatcaaccctgggaactctggtgggccactgattaactttgccggccaagtggtcgggatcaattccatgaaattagcttctgatcagcagggtaccagtgttgaaggaatgggctttgcgatcccaagtaatgaagtggttatgattatcaaccagttgatcaagaacggccaagttatccgtccggcactgggaatcggctacaccgatctgtccaacatttccgagcagcagcaacgctctattttgaagctgcctaagagtgttactcaaggggcggttgtccttaacgtgaacgctaattcacctgctaagcgggctggattggccaaatacgatgtgattaccgagctggatggcactaagattactcaacaaagtcaattgcgtgatattctgtataagcacaagattggcgataagatctcagttacctattatcataaaggtgacaagaagactggctcaattactttgaacgaaaaagcaaccagtaaagttttaagcgaagcaagtaaataatccttaattataagtattggtaacctccgttttctcataagcggaggttattttttgccttaaaatgaattgccgatcgttacttacttaacataagtgtaatacttaatattcatgtaatgttaataaattcacatttgagatacaataatgatgtagcacaaattgatcaaaggggatatcgacatgaaaattcatattaagggatcaatcctggtttccatggctgctctgggagtctttgctgcagttgggatatcgcagtcttcaactgtttcagcaaaatctcgggtccgggttacgtcgaacgtaaaattgaagggtaccggagcctcgcgcaacgttacctttaccggtaaagcagcattgtggaccaaggcttcagcactaaaaggagccaagagggtcgcaaccaccattacactgcgggaccttgccaaatctacccgatcaagcaagaatgttcgcgcttatcgggttgccagaaccaaccggggaaaagtgtattataaggtggttacttttgacggtaaggatcgcggttggatctatggcggtaagagtcggtcaagctttgctggcggggtgaaatcttatctgacattccagcagaactcactcactgatgatatgagcaacgggacgttccaattcgcaaacccgggaaccgcaaacaataatcagacagttacatataagcagccagcttggacgcaatataaggttggccgtcaggtaactgattcaagaccttatgcaaatgtcagttaccaaattgaccaaacagggatgagaacccgtgaaggtgaccaatgggttcacatttctgccaccaataacggcaactccggcgcggatggctggattttgtattcaggattgaagaagacaaccaacatcaattcaccaattgctgataacgctattcgaattaagttagttgattcggcgacaggttcgtcattgacctcggttgatttcacaaagactggggtaactaaaggcgctaccatcggcgcaaatgtgaatggcacttggaagctggattcaaatgattccagttcaattcagtcacagattgcctccgcactttcaccacttggctatccaggatttaccttgactcaaggccaaatcgcggccattgcccagggaacctttggatccagcgtgacgatttcagttgtgaaaccaacgattaacaaggcagtccggattgttttgacagatccgagcggaaacgtgattaattatgttgattacacgactgctaacgctgccaatggtcaaccggtgggtgtgcaggatggctcaacttggaaattggcggcaaccgatacggctgctattcaagctaagttagttgatgcgttaaagggtaccggttttgcattaagcgccaacaacacattgaccactgaccaacaagctcaaattgctcaaacgacattcggtaaccaggtttccattaagaccgttgccgttaacccaatcaaagacaatgaagttcaattgtcgtttgttgatcaggccggtaaggctgttggttcaacaaccttgacgaaaggcacaaatgacaaaacggctttggacacgattaagactgttagtgttgctgacccaacatcacctgatgctgctaccttgaagaaggcttatgctgctcttttggccaaggctggtattaagggctacaccactgatggtttgagcaaggatcaacttgctgcgaacttagctgccattaaagcggctgcatatggtcaggatgttaagttggttgtcgctaagctgccagcgaaggcattggtttccagtgcactgttctttgataaatctgataccaaggacgtaactcaggatcttgcatactttgaaaatgcaaacggtaaacgtgatagtgacgcaaactttagcaaagcattggctggagacgcgaatatcaatggttatgccggcgatgtggttacggttgcaaacctcaatgctgctgttaaggatcagggattgaatacaatttactacgcagcaaagaatgacggtttcctctggggagctggaactcatttagcggctagtgactacagtggaacgaatggaacgttatttgcagacggtatgagtggtaagacaatttatgaattcaaattaacctttaccgctaaacctgataatcctgatacgtcgattggtaacagactagattctaataagcctctattcgacaagcaggggaatgcaactattggtgatacaggcaatcaagtggtactgaagtatgatgaagtcaaggctggtaaacagattacccttgatagcaacaatatgaaagccaaaacactcgcagagttgtttggtgaataagcacaaaagttgatcagaggacttcaattctcaagttgggattgaagttcttttgtgtctgtagccacatggcttcttatttaagagccctaagtggaacacagaggataacaccctcctccgtctgaaacacgtgataagactcatatttagggctaatatcctccgggatcggcagcacccattccccgtcgtgattgactagtttgactgtcattggtgattctccaatctttaaagtggatttgtttgggataattcaggtataataattgaattgattcgatttgtccgcaaacattggaccgcatcactgtttacgaacggccttaccaaatatatggaacttgtaccgtacacatggtataaatacgaacgacgaaccaagttttatttaaaaaattcatcggatgtaaagatttgataaactatccacattttggctgtggataactctgtggacaatccacaagattctgttatccactgatagaataacgttgaatagttatcccccaaaaactaaaagttatccacagaaattgtggataactttttttgatataaaaaggagatttgttcgttgagataatgactgatataatagggtttgcggtgacagattgcgaacacacgttgtccacagttctgtggataacatttttgacccttgacaatttttaaaataatgcgggtcactgaaaagttgataaggtgcataaacctgtggataactctgtggacaacttgttaataagcccgcttttttacacaggataactataaatttggaggcaattacatagtgaacatcaaattggtcgttgttggaaaattaaaagagaagtattttaagcaggggattgcggaatacgcgaagcggttatcgcgtttttgcaagtttcagattgtggaagttcccgatgagaaggcgccagagtcactcagccaagcagaaatggatgaagtgatggataaagaaggtgcgcgaattttagataaaataaaggaccgcgagtacgtgtatgcactcgcaatcctaggtaaggagcggacttcagaagcgttcgcgaaggaaattgccgacctgacaacctatggtcattcggacatcacctttgttattggtggatcacttgggttatcgaaacacgttctcgatcgtgccgacacccagatttcctttggccggttcacattgccccaccagttgatgaggttggtgttgactgagcagatttaccgagcatttatgattaatgagggtagtccataccataagtgaccgtcaattaccgagtaaattaaaaccagctggtaaccctatttgggattgtcagctggctttcttcatggtttatgatggtatcagatttagagctgcaataacttttccgcattcccatgcgcaaacaattccttctcctcatccgttagaggactgctctcaatgaaactgccagaattttccggtttgatataaggatagtctatcgagtatagcagatgctcaatcccaacttcgtccttcacgaatttcaattgtggttcggtcaaaataccgcttggggtgacatacacgtggtcgcgataaatctttgaaatgggttcgctcaggttggtttccggatacatgacctgatccattcgctcaagggcaaacgaggcaaactcgccccagtgaccggagatcaatttcagattcgggtacttctcgaaaacaccacttagtaaaagcctgacggtctggatgccgacatcagtatgccaaccatagccggcagttcccaaaataccggaaaccttgtcatcccacggaccgttggagtaatagtagtcgataatctgtgaatctgggaatgatggatgcagatagactggcacattgaggttggctgcggcctcaaaaatgggtaggtagaatggatcatcaaagaatggatgagcctgagaagttggtctcactagcatggctcccttgaagccgagctcttcaacactgcgtttcagttctgccgcagcgtcagtgggatgggaaacagggagcgacgcaaaggcacggaagcgatcgggcgccgcagcaacagcttttgccagctcatcattcgccaactttgtcagttcaaccgcaaacttcggatctgaattttgcgggttctgattgccatatgacagaatttgcattgaaatctggtgttgatccatccattgaatccgactgccggtaacgtcttccaattctgcttctggaggcagtgagcgctgcatataatcgtgcatttccggactgacgtttccgattggtcgttttggtaagacctcggccattttctgacctaacttttgtgatgaaaaatgttcttctaatgtaataactttcatgtgatgtttgcctccttagctaagtagcttgccctttttcaaaaagcggttattcaagaaccagtaatgtttcgggtcccccagcaatgcagtataaggaaccggtgtgccgcctttttcaatgattttctcatccaggtacgctttgagaatccaaggttcctccaaccgggtggggttcaagtccaaaatatcttgaacatgttccggcgtggtatccagatcttgggccacttgttcgattgggacttctgccagtttgaagttggcgttaatttgcttcttggtgtcgatttcttgttgtggtgtgagtgacatgtgattactcctttagttgttggtaaatttgagtgagctggtcataaatcgcatccggtgcaagtaaagctgcatcgactttctcatcgaggacgtcgaacgcacccttgaccgccgtgacggtctcgttgccgtttggagtcagggtcagctgtttttcgcggtcattatccggattgaattttttctcgatcaagtttctggtttccagtccttttaataaattagaaacactggcagcgctgcgtcttaaaataattgtgatcgcccgttgatttgtccctgggtgatcgccaatgtaccgcagcgtgtgggcttgatcgacatttaaattgagttcgtgcaactgctgattaatcaaaccttcttccagcttggcaatttgatgaatgagcgatgatactgaatttcgatctttcaaaacatgacctcctcacttagatttatagtctaccaccaatagttgtaaatgcaactgttttaaccaaaactatgtattaaaaaatcccccctttgattgggaggaattcagattgtttgtttaattaaccgattgaattgatttcccagctaaaaagtccaaaatgttattggcacaaatctcagccattgaatcacgcgcctcaacggttgcgttgccgatatgcggcgtcaagatgacgttattcattgacttcagttcaggggtcacggttggttcgtgctcatagacatccaaagccgcaccggcgatctcatggttctctagtgccgatgccagagccgcttcgtcaacaattgggcctcgggctccgttaattaagaacgcggatgacttcatttgcttgaaggccttggcgtctagttggtgatgattttcttcggtcagtggtgcatgaatcgtgataaagtcactggtttgaagcagatcggtgaattcagcaaaccggatgtttaatcgattttcctcatctcgtggcaatctaaattgttctggctgccagtagtgaacgttcattgaaaaggcttgcgctttcttggcaacatcctggccaatgtggcccattccaatcactcctaatgtttttcccgccagttcatgccctagaaagaatagtggggaccatcccgaaaatccttggttgtgcatcaaacggtcgccctcgacaatccgatggctgatggctagaattaagccgagggtcacttctgcgactgaatttgttgaaacaaccggtgtgttggtcaccaagatgtggtgggtactagcggctttagtgtcgatattattgaaaccagcgccaaaattggcaattaattttaacttggttgcagcgctgatgattgattcgtcgaccttggtggataatgttgtaatcagaaaatcactatcttttacggcattctccaactcttcgtgagtgattaagccctgctcactgtcgtgaatggtaacggatagaccagcactttgtaatttcttaacagctttacttggaatttgatcagcgataaatacttttgtcatgattatcctcctcatatattaatctaactacatcatgtggctaggttgaacaacctgcaataccgcacttttttgtaactgatgaaaggagttggttcaaatgactgatagcgttagagaagcagtccaagaaaaattagcgaatggcattttcaactgtcccaaggaattaactttgtcgatgatcagtggcaaatggaaaattaacatcctgtatcatctcgggacagatggaccctattatttctatgagcttcaaaaattattgcctgcagcatcaagaaaagagattacggcaaagctcaaagaattagtcgaagatggtttggtcaatcgtaagccactgaagactgttccggtcaaggttcaatattcaattaccccgctgggaaaatcattgatgccgattattgacgccatgttgaaatggggccaacagcggctcgacgacttgcagttgggacaagttgaatttggcttgggtaaagtcaaacatgaataattgttaatttttcaaaatgcaaactccaaaatagacctgatcacgagcactcgttatactaatgattgcaattagtaaagcgtaatggtatacgcgaatattttggaggtgtcaattatgaacaataatagtcaaaagccagccaagccatggtataagaaatggtgggtttgggtattggttgtttttggattggtgattgcagtcaatgcagtttccggtgaagaagacgattcagccagtaaccagtcaattaccacagcgactcaggacagttcttccagtaatggcgatgggacgctcaaaagtaattacaatgtcggtgaagtggccaactataaggggtataaattcaagatcaataaagtgaccttctataatggcaatgaatttgatacgcccaaggatggtaatcggtatgtgatctgtaatgtaaccattaagaatgatactgatgagaagcagccatataattcatttgacttcaaattaaatgctaatgggaactccaccaacatgatggaagtcgtgacgaatgaaaaatatactaacaatacgttaaacagtggcgacctggatcccggcgcgagtgtgaccggtaacctgattggtcaggcaaaacaggatgccgacttgaagttggaatatcaaccgtcaatctgggatgataagaccgtcaaagttgatatcaacgaatcagcgtaagttatggggcatttcttttactccatttgctcaatcatatacaataatggtgtaagcgttttatgaataaaagggaggctttttcatgacagatcgtctaaagaataaggtcgcaattgtgaccggtgccggatcaggtatgggcgctgcaatggccaagttgtttactgctgagggcgccagcgttgtcgccgctgatttgaataaagatcgggttgacgaagtggttgcggcgatcgccaaagatggtggcaaagcagtctcaatcaagacagatgtttccaacgaagacgatattcaggcaatgtttaagttggcaaaaagtgaatttggtcaactcgatattgttgtcaataatgccggcatcatggataatatggcgccagttggcaatttgactgatgacatgtggaagaaagtctttgccgttaacactgacagcgtcatgtactcaactcgtgaagcaatcaaggaattcctgccgaagaagcagggagtcattttgaacattgcgtcagttggtggaacgaatggcggccgtgccggagttgcatacacggcctcaaaacacgcggttgttggtttaaccaagaatacggcttacatgtaccaaaatgacggcattcgagtcaatgcgattgcccccggtggcatcaagacaaatattgctgagtcaatgggcaagaatgttgataaatttggttatgagcgtcaatcccaagggatgggtgcatcacctgaacccggaactgcagccgaaatcgcaaacaccgctttgttcctggtttccgatgaggctcgttatgtaaatggtgctgtcttgccggtagatggcggttggactgcctactaaaattaaataagtttgaaccgtggaagtgattccgcggtttttgtttgccatgaagtgcactccagggtatagggtagaaacattatataaatagaaagaggctaccatgacaaaatcattgattatttatttttcactgtcaggcacaaccaaaaccgcagcggaaaccattcaaaaatatacgcattcagacatcatcagactggaacccaagacaccttacccagctggttacgacaagtattccaaagttggtatgcagcaaatgcgagacaaagcagatgttgccatccagactgaaatacccgatctacaccaatacgattatatttttattggttatccgacttgggatgggcaggtgccgcggatttttaatacgttgtttaaggaaaatgatttctcagacaatcgcttggtgccattttcgactagtgtgtcaacgccgtttgaggatacccttggttcgttgaaggcggccgttggggatggggttgcgattgttggtgggtttagatattctggggagacacaagtaagggattatttaaagaataataattttaaataggcttattttttgatactatgaagacattggttagcacactaacactttggaggtatcaaaatggctaaatttgaatcccgcattttgtcgattcctgattatgtacccgcagatatcattcgaattagaaaacttgtttcagctgataagaccaaaatggcattgttcatgaatgtctcattgcggacttacaaaaaatgggaaaccggtcaaagtcatccaagcaaacccgctcgccgtttactgcagatacttgagaagaatccccaattaattgataattggttttaaatcagcatttgatgaccatgtatagaagaataatagctgaaggagtcgcgaaaaaaacgcggctctttttcatattctcacatcgccacgttgcatactgaatattcatgcataatatcaccatatattgacataaagtttaaaaggtttatgattgagtatattaaaattcaatgaggaaacggggaaacattatgagtatttctgttattaaacgatcgttattatcgcttggtattctagcaacaacagttttgctggcggcatgtggctccaagagctccgatcaagggtcgactaagctggcatcaaatcaaaagatcagcttatccacgacagctgaaattaccagcttggatttgtcaaaaatctacgataaaacgtcgtttattcaaattgatgaaacttttgaaggcttgtatcgttatgatgcaaacggaaatgtggaacctgcgctggcaaccaagacaaaaatttctaaagatggaaaaacatacacgattaacattcgtcacaatgccaagtggagtaatggcgatcccgtgaccgcaaaagattttgtctattcttggcaacgggcggtcaatcctaaaacggccagtcaatacacttacctctttgataatgtgaagaatgccgatgcaattgtgaatggtaaactttcaccaaataagttaggtgtgaaagcaaatggaaaatatcaactaaaagttcaacttgctcgtccaacgacctacttcaaaatggtaatggctcgtgagacgctttacccacttgatcaaaaagttgtcaaaaaatacggtaagaagtacggaacatccgctaaatataccgtgtacaacggcccattcaaaaacgttggctggactggaaccaatgattcctggaagctggttaaaaataatcagtattgggataaaaaagcagtcaagctttcccagatcaattacacagttgccaaatcgccaagcacagcatataacctatttcaatctggcaaacttgatttaatcagtcttgttggtgaacaagccaaacaacttgggaagagtaaagatgctgttaaacggccactagccgcaaccgagtatctgcaatacaaccaacgtaaaggcgtcttcaagaatcgcaacttacggttggctttctctttagctttgaatcgaagccaattaattaacaaagtgatgcaaaatggatcaattgtttcgaaaggatttgtgcccgccgatttcgccaagaaccctaaaaccggtgaggattttgccaaggaagcgtatgttcctggaacagttgatcatgatgcgactaaggcaaagcaatactacaaaaaggccttatcacaattgggtaagaagaatttaactatcaagctcttgtccgctgatgacgatcaaaccaaagatgtcattgagtttattcaaagtgaacttcaagaaacgttaccaggtctcaaggttgaatcaagcagtattccatttgcctcgatgcttgcaagagcttcagctggaaactttgaagttaactttacgggttggtctgctgattttgctgacccaatttcatttctttcccaatttacatcaaacaacccagaaaataatggcaagtggagcagccaagcatttgatcaagcgatcaaagattccaataacaaggatgcgaataacgccaccaagagatggcaagatttaatcaatgctgaaaagattttggccactgatcagggaattacgccgatttatcaagcgaatggaattgacctggttaaccctaagttgaagggggttgtctatgatcgaattaatggacattatgactacagaacagcttatttaaccaaataatttgaaaaaggggtaatatcttggataagaagtcagcactaaatttaattgaacatttatccaatgcaaatggaccaagtggctttgaggacgaagtaaaagattatgtcgttcaaacagcctccagctttagctcggttcacgcggatcacatgaacaacgtctatttgaaaaataatcaaaattcaccttccaaaggcaaaactttgatgctagattcacacttggatgccgtcggtttgattgttcaagccgtcaagccaaatggaaccattaaatttgttccgctcggtggttgggtaccggccaatttaactgcagaaaaaatgcgcatccgaaaccaagacggagaatggatcaccggtttggttgccaccaagccaccgcatttcatgacagaagcagaaaagaagaaaccaattgatattgccaacctagtgattgatgttggaacgaacagcgctgaagagaccaaagaggtcttgaagattgatacgggttgtcccattgcgcctgacactgagtgggagtacttcaaaactcaagatgtcatgatgggcaaggcgtttgataatcggattggtactgcatgcttgatgacggcaatgtctgacctggctgaggaaaacttggatgttaacttggtcggtgcgattgcatctcaagaagaagtcggttgtcggggcgcaaaagtgactgttaaaaaggttcatccagacattgcaatctgtcttgagggatgcccagccgatgacacgtttacaccagaatggctgatccaaaccgggttaaaacgtggtccaatgctgcgtgatatggatacatcctttattgctaatccgcattttcaacagttggctgtagatcaagcccaccagaacggtattccatttacccgcgctgttcggactggtggtggaattgatggctctgaattgcttgagttccaaggggcacccaccatttgtattgggattcctgttcgttatgaacatactaactatggatttgtggcatattctgacttcgaaaacaccgttaaattactgaaggcaattattttgagcctcaatgataaggtcattgacggtctataaatcaaggagctggtagatttggataaacaatatgtaattggattgcccgcagagactcgaatcattaataatcttgcaagaaataccgtcaacgatgacgaagtcgctggtgtcatcaaacacggtggagtcccggttctgattcccacccgcaatccagaaatcatggagcactacgttgacctgattgacggcttgctgctgccgggtgggccggatgttgcgccgaagttctatggtgaagagccggttcaaaacctcggcgacaccgatgccttcttggatgccagcgaaatcgcgttagtcaaattagcggttgccaaacgcaaaccaatttttgggatctgccggggcgtccaagtgctaaacgttgcccttggtggtaccctttaccaagatttgtacagccaacggaatcatccaaccctccagcattaccaaaaggcgccgatgccacaggggacgcataccatttccaccactccggattcctatttggccaaaattatcggccagggtgactcgactttggttaacagccaccaccatgaagccgttaaggcggttgctggccaactcaatatttctgcattggcaaaggatggcgtgattgagggcgttgaaagccaagatgacgacttgattattggtgttcaatggcatccagaagcgatgtttaggaccgatgagaagcaggacgcgttgtttgcggatttcatggcgcgagtggaaaaattcgcaaaccagaaagctgtacatgattcggtttccactgagaatgaataacaaactaaaggatctttgataggccagcgccaactggtttaccaaagatcctttgttattcatagtgttcagttgtcgaattgtacgttagcgtaaccggctgattattcaggttaaccgtgatttcccggtaaggttggaaaccatggtgaacaagttcgacgctgacctgaccgtggtcaacgttcacgagataatcgttgaattcgccgtgctgatacttgaagtccaggccgttatcctgatagtgatgatagctgccggaatccccatagacgttgaatgccattgtcgaatcaggggtttcagagatatgatcaacttcggctccccatggcaaaatggttccttgcttgataaacatcggcagcttatctaacggcgcatcaacgacaatgtcttgttggccgtcatattcccggtggttccaaaaatcaatccatttcccagccggaagataaaccagtcgtttggtctgcgatggttggacgatcggtgcgactaagattgcatcgccaaccagatactgatcgttgatgtttcggactcgtgggtcatcttcataattcaaaaccagtggccgcatgagtggcaggccgttcttagattctttggcaaataggtcgtatagataagggatgaatcggtagcgcagctttagaaatttacgataaattgataaggtgggttcaccaaaggcccatggttcctgggcacgggttcccattgcactgtggtttcgcagcaggggactgaagatggctgcctcaatccagcgggtcaaaagttccggcgtcgcgtctgaacccaagccggcaatatcggtgccggcaaaagtgaatccactgattcccagattacacaattggggaatcaggagttgcaagtggggccaaatgctatgattgtcgccggtccagacagttgaatatttttgcgtacccgaataagcggcccgggtaatgacaaatggccgtctaccggttgcacgtttcaccccatcataggtcgccttggccatattgtggccgtagacgttatgcattttcttatgagtcgacggctggtcgtggtcgctgaaaacaatgtcttggggaatttctccttgaaatgaagcgggttcgttcatgtcgttccagatcccagcaacccccatgtcagtcagaaattgatcatttttgccccaccatttttgaacggctcggcggccaaaatccgggaagacggcatcccccggccaaacttggttgacgtagacattgcccgccggatctttgacgaaataatcattcttgatgccttgatcataaatgttgtagccgggatccttcttgacgccaggatcgataatggcaacaatttttgtgccggtggctttcaaatccgtcacaaacttctgagggttgccttgataagcctcgtcattccaagtgaacacccggtagccgcgcatataatcaatgtccaagtgaatcacgtcaaatggtaaatcgtatttgtgcatcgaatccacgatatcttggaccatcttctggctggcagagtagccccagcgtgattgttggtatcccaatgtccatttttgaggcaagggggttcggccggttaagtaggtataattggtaacgatatctttgagagttttaccgccaattaggtagtaattgaggttgccggcttcagctgagtagaaataatagttgggattttctttgccaaaatcaaaatgactccggtagggattgtcgaagaagaggccgtagggatgcccagctttgaggccgattatcactggaatcgatttgtataatctagtgaaattttctagatggggagctggattatcggtattccagtcatcatactcatagccccgtttgttcagataaccggtcttgtctccgagcccgtagatctgttcatcaggtgccaaatccttcacaacttgaaagtagtcgggattattttgatcgtcggcaccgggaacgttgtggccctcttcttggacgaactttttatgttcctcgtcaatcccccgatcaagcggagtccgactgccacggtagtcagtgaccagtggattgctgttggcatcataggcatcaatatgcatggccgcatcgaccttgatggtcaaggcagtggtcgtgatttcataatgatcaggttgttgcttaactgtgtatgtcgttgtggtttccttgtcgccttcaatcgcgtatgaggcaccatgatcaccgcgattttcggagacccgaatgatctctggggtgataatagtcaattgaatttgacgatttgaattgttaaatgtaatggtttgatgatctgtttgataggttggtaacttgggcaagtttgtcagtcctttcgtttagattatcgtagcatacgcggcctaagagatacaatactgttcgaaaagaccagcccgcctgatttggtgagctggtcttggttcttaatgatggtcgtcatcatgatcgtggaggccaatataataaccgtccatataaccggagtcgtagttgtcttcgtcacttcggacatagccgccgccaagcggagtgttccaatgatcaatgatccagacgacaaatataatgaaacccgcgagcattaccagagcagattttacttcttcgaaggtggaatcacgcaagccatatggtgcataataatttttttggatagatttattgaggacgtcaaccgtattcatcacgttggcggcagagacatccatgtaatccagctgcaagcccataaacaaattttgaaagtcataaatgttgtccataaaactttgggatgcaatcggcatcacgtgatacggaaggttcggatcaatgagaatgatattgacatctccttcaatcactatttcatcttgatcgtaggctgtttgagattgataatttaataattttttggcaaagtaatccccaaatggattggcggccatcgcaaatcgggaaactgttgggcccttttttctgatattgacgaggtatcgttcaaattttggatcctgcagctcggcgagggttttattcgttgaaataatccaaatttgctgaccctcgtattttttcatcaggtggcgattgatttgtttaatttggctgatctgcttctgatttaaaatgtgaagttcgtcagaaatgactggtcgagggttgccatccgctgagtttgcatctgctcggacggaggtgttgaacacgaaaatgagcaacagcacgacaggcaaaaggatcgaacgggtaagatagtgcaaccgcgggttcatgattatggtcctccttggattttatgctgagtatagcaccattatttttgtgggcggtcaaggtaactcttttcattttgttgtaataagtactagggttctttcatcttttgccataaaattgaaatgttgattcacgcgtttattcaaattggagggatccgtcatggaactgacaaccgcgaaaaattatttgttattaactgaaagaatcggtaagaagccaatgctgcgaacgcgatttactgcccaggcgtattttgttctggcagcgttatttgacttggtcgaccaaagaattttggacattggggagactatttcaatcaaagatgaccaagagtttgccgaactaccggattatctgagtattttcaaatcagaactgactgatgaaattaagcaagggcatgacctgcagacacaattggcaattatcaccagttgggatattgccaaccagctttatgagggccttggcgccggtctgctggcggatcagttggttgagaagaagtcggtcaagaataatttggacacccacgtcatctatctgccaaaggacgctgctcgaaagcaggttcaggattatctgcgcaatcagattaccggtgcgaaggtcagtcacgacgcagttaatttggtgctgatcctgtcggagttggatgctttgaaatgggtgtttaccgacaaagaggagttggctaacttgacggcggcctttcagcagaaggtcgccggggatgcgttttacatcaaagaaaaagccctggccaaagtagcccaggacgtgattactaagaagaagttttggtatgattcttggctgagttgaagaataatgatattgagtattttacgattaaacattttaagttgactatgatggatcatttcggatagaataacagtaagataacttgagaaggagtaacgctgggttcccgaacgggagtaggctttttagcttagaattcctatgcgcctggagttatctttttttaatctcactctttagtatactgataattctctgagggttgtcctttatttctttttcgattaggttgattgctttttgagagtaggtgtattgattattatttccaagaacatgcttatacgcatagtcaatatttgttttgatttcgtaaaactttatgaacaaatccaaatcacttttattaaaagctacacgaattccgtggctaatcgtaacctgaaaattgattttcttccttgatatccatttgtttatttgatttacaacttcactataactaaaaggatgggtattcttaggatcttgaagtttattaataatagctgctttagtttcgctatctttcgccacggaaacaataaaatctgcatttttcttgtttttggtaatataaatattatggttaataggaattccaaagtgagtgctttcagtatgaattgtttcctcatttaactccatctgatcccttaatatttgttccgctatgctggttggatactttttcttgatggctttggagtcaagcgagtcgatattaactgaaagtgatagaaaatgttggtcaagtcgttcagtaatatcaatatgaaaaaagtcgttaagcttatttacataattgatcacacacgcttggaataacggtgcatacatctgttcatattcttctgttacaaaatggattgaggtgttgcgaagtgacacaattttttcgagatttcttctcagtggttctcttttatcggtgaatacttttttgatacattccgatatagagtacgactgacttctcttggtcgctttagttgaataaaaaattgcctctaatgagtctgccgattttattaaataggacttaagaagaagttcccatgcattacagatataaaaactgaatccttccactctatatttgactgtaggacgattgtagagctctaaaccgagcgtaaatgcttcctgactcttctctagtagggttaaaaaagttttattgtcttttgcgttcaatttgtattcctcacactgtttattgattttttcagatttactattcaaattatacagtattctttccagcaattgccggtaaagttgattggtaaaagtagaatgtccttcttgtgtctgtaggcattcatgacccgaaacacagtactttcagtgcttatattgctagcaaagggttctataaaagagccagattcataatatgaagtgtaatatttctaaaatttaacttgaagtgcccagcgtatagtttgagactaattctcaaactatacgctgggcatttttctcaatggggatttgatgacccatcgttgttatcagactttttgattgtcaatattataaggctctaaataagtttatcttgatgaatcatttccactttactcgttccttaccaacatctgatcccttatcataattcccaacatcctccatattggctcgaaaatcaaagttgccaaattgaccattctcccaagggtcatgatttttgcttttttcgtagatcagttccttgctcgttttgtggaatgcgtattcgcaaatgattctcttctttttcaccatgttaagcattaagcacctcctagatattgtgagtattgagtatatttactttaactaatggtaaaattcattacttagttcttttcctgtcaattcgccgactatgttggtaaatttgataccgaatggacataaaatagatcatcacaagtccgccaactccccagattaggtagttgtggaatgcgataattaagacaatgagtatgacagcaccgatccatgtgctgatgacgtccaaaatttcttgcacgagtaatcccctagcccttgattagcttaattatagccgtttcttgggtgtttgttgaagtataggtatctcagaaatcatactcataaattcaagatgtttgacatgaagtatcaacactatacaactgacacctggcgatatgttagtcataacaggttgtatcatgctgggctattttatagatactaatataatcacttcatttgaattcaaaaacgacggaacccaatttgggattcgtcgttttgttcataatgatattgattaaaattctcgttttccatgcagataaacctgcttatcagtctgctgaaccgccagtacatcttccaacgggttttcagtcaggacttggaaatcggcaaatttaccttcttccaaggtgccatattcatcactaatgttacataaagctgcagaattgattgaggaacactgatatgcctcaaaagggggcattccaagtttggttgtcagcagttccatttccttgggtgtctgatcaaagccattgaagggtgtcccggcatcagtaccacatgtgatcttaacacccagtcgaaaagctcttgagatgttggcataagtatcatccaaagcatcagctgcttttttgacttcccatgcgggcaaagtgtgtttgccgaattctgggattgcccattcagcgatcaatgtgggggttagaaatgtcccttgattaatcatttggttggcttctcgttcggtgacgtaaaaaccgtgttcaatggaatccacgcctgcatctaaggcattttggataccagggtttccttcagcgtgagccgcaactctttgtcctttatggtgggcttcaagcaccgcagtccgcatttctgtgaccgagagttgaggatcagccatgaaatctcctggtgtcataacgccacctgtcgccattaatttgatcaattgggagccattcttgaggccagtgcgaacggccttacgaatctcatccgatgagtcgaccagataagttgagtggggatggtccccgtggccgccggtcattgaaaatgttcttcccgacggcatgatctcgggagtgtgttttagcattcccttgttccgcattctctttaacttaatgtcgatatcataactattgccgcaaccacggataaacgtcacgccggattttagaaatgtctgaaggttctggtatgcatcgacagcagtttctgtttccgagcggtttctgccaccatcaaaagtagccgggttactggtaatgtgggtatgcacgttgatgaatcctggcatgacatatttgtcgcataggtcaatcgaacggtctgcttttggaaaatcagcggttcctcgagcaataattttgccgctttgatcgtcagttatgaaccaggcattggattggatttgatcggttagaccgtcaaatagttgtaaatttttaaataaggtgcttgtcatttgcttgttgcctcctcaaagattagtggttaataacagttaaaattctcgttttccatgaagaaaaatctgtttgtcatcttgttggagggctttaacatcagccaatggatcggcgttgagtacttggaaatcagcatatttatccttttccaaagtgccgtattcatcttggatttggcagagtgttgctgcattgatcgaagaacattgataagcttcaaaaggagttatccctagcttttcagtcatcagctcaagctcttttggcgttgtatcgaacccgttgtatggggttccggcatcggttcccaaagtgaatttaacgcccaatttgaaggccttggataaattccgataggcatcttcgcaggcatcatcagcctttttgacttcccaatccggtaacttacccttgccgtattctggaatcgcccataaagcgataatggttggcgtcaggtactggccgtgatgaatcattttcttggcttcttcctcgttgatataaaagccatgttcaatggaatccacaccggcgtcaatggcgttttgaatcccgggatttccctcagcgtgggcagcaacaatttttcccttatggtgagcctcatcgataccagctttcatttcttccacagaaagttggggatcagccataaaatcaccgggggtcataaccccacctgttgccatcattttgatattttgagccccaatcttcaatccctgccgaaccgcttttctcatctcatctggagaatcaactcggtggccgaagtggggactatccccgtggccgccggtcattgaataggccatcccggatggcatcatctcaggtgttttcttgagcgatccttgttctcgaagccgattcaacttaatgtcaacatcgtagctggttccacattcgcggataaaggtgacgcctgatttcagcatggtctgcaggttttggtaggctgtgacggctgcctcggtttcagaatcacccgggttaccatcaaaggttcgtgggttgctggtaatgtgggtgtggacattgatcaatcctggcatgacgtatttaccatccagatcaattgagttgttgtcctttggggcgcttccagttccttgatcggtaattttcccggtttggtcatcaatcgtgaaccatgcatctgattgaatttgattatttttcccatcgaataaattaaaattaaaaaatgttgtcattaaaaatgcttcctttcagtatttttctacaaaatgtcattatttccagtaagcatacttgtactgggcttcatttaaaatcgagtaggtcagtccgccgaccttactgctgatcaatttgttttcggctggctgatacagcggaattgcgcctttgacactcatgaggtatttatctgcagctgctagtttgtcgtaacgcgcttgtccggtggcagcgttggcttcattgagcatgttgtcataggtcttgttgctccagttggtaaagttaactgaattgccggtctgtagtaagtctaaaaagtcataagcatcaagccagttggtggaccacccggtcaaattgagttggaacttgccgttgaaatctcgatcaacgtgttgggcatgtggcaacgatgttaatgtaattttcagccctttgaagttcttttctgccgctgcttgaatatattggccaacgtgtttgtcttcatcaagatcgtccgtcagtaagttcaacgtgattgatttcttaccggtttctttcagatacttattccagtaggccttggcttttgctttgtctgtcggtagtaaattaccaattgaggtagccatatctttgccggtcgccggatctttttgatcgccaattggaatcatgctcttagcaggcgccgaaccgtcttggagaacatcatctgtaatggtctgattgtcgatgatgtatgaaaatgcctgccgaagattttctgaattggttggtttgtatttattgttgaagtacaaataattcatacgtccagtcagatgtttatgaagatttggattcttggcatttgctttaacatactggccactaacattggtctcttgaatttttccactttgaaataaattgatggctgtattttgatctttggtaaccgtgacgttgattctgttaatcttgacattcttggcgtcccaataatgcggattcttgacataatgccaagatgagttgctgccagtccaaccagtgagtttgtaaggtccattggccattgtttttgaagcgttggttccgtattcttggccatatttcttaacggtcgctgtgtttagtggatagaactttgaggcaactaaatcattgaaccacggcacccgcttcgtgagttgaatctggagtttgtgtttaccgatggcttttgcacccagcttatcggctgacatcttgcctgcttgaattgctgcatagttcttaaaagcgtcgtacagactggcgtattgggcctttgtcttaggatcgacggttcttctaaacgagttaacaaagtcttgggcggtcactgtttgaccatttgcccacttggcgttctttttgagattaaatgtgtaggtggttccattattggttggcttgacaattttggttgccactcctggggtcagtttgtttgccttgttgtacgtataaaggccttcataggtttggaaaatcaattgagcactattggtatcggttgatttattaggatcagcagtcagcggttcgtcaggcaacgtaacgtttaatggcttgttgctcttactcgctgcctgcttattcccacaagctgccaatgatataccggcaattagaattgccccaaaagaaattaatttgtgtttcatagaatccctccaaaatttgttggattagaaatggtgaacgaaaaagcgccccttcagaaattaatctgaaagggcgctttcgcacggtaccaccttagttcgctattaaatagcctcaagtgagcggctggttctcttggaatcagcgattcactgcacgaataacgggtgcatccggtaattgcctactaaacttcagcccacagctcaaaagctacttcccagcgaaatcttctgacctgttttcacttaccaggctcactgcacagaaaattaaagtggtactctctttatcattgccattatattctaatcaatatttaatgtttctaacattaacatgtgaggtgattttagtcaaacataattttcaaaaaggtggtcagatatgctgatgccatggcttgtgcaagtttactttcttgtttttaatatttttaaatgagactttatatgagggaattagattgttgaacatcgttttcgtaagccgacatcagcagcaccagtgaatgccgtcgaccattgacgggatgtcccttgctcagcttgaattcccgaattaccaagcctatttcgttgcatttcacaagcaacctgccataattaaagtgtattcgatgtaaccgtttccattagcataagggggatattatcatggcaatcaaaaaggttactgttgctggtagtggggtcttaggcagtcagattgcgtttcaaagtgcttttaaagggtttgacgtgactgtttatgatattagtcaagaagctgttgataaagctgaggaacgaattaaaggtctgcgccacgcttatcggcacgatattgcggcgaccgatgaagaatttaatgccgggattagtcgattgaaatttacggatgatttagcggcggcagttaaagatgctgatctggtcatcgaagcgattccggaaaatcctgacatcaagcatgaattctatcaaaaattgagcaagttggcaccaagcaatgcgattttcactagtaactcatctacgctggtaccaagcatgtttgccgctgataccggtcggccaaagcagtttttgaacatgcatttttccaaccaggtttggctgaacaacaccgctgaaattatgggatcaccggaaactgatccggcaatctatcaagaaatcgttcagtacgcccgagacattgggatggtaccgattcagctgaaaaaagagcagcccggctacattctgaactcactgttaatgccgttgaacgcggcagcgggggcattgtggctgaaagggatcgctgatccaaagatgattgatcgaacctggatggccgcaaccggcgcaccatggggaccatttggcatcctggacgcggttgggattcgaactgcctacaacatcactttggcagcctccaaaaaggatccagctgtgatgccgcttgctgatgctttcaagaagatgctggatgaaggcaagcttggcgttgagtcaggcgaaggcttctacaagtatcctgatcctgagtataagaccaaggaattccttgaaggttagccttttgttgaatgaacaacaggtctaaatcgttgattaaccagcgatctagacctgttttttgattgccgacaatttttgaaaaaataagtgcagttagttgtaaacgtttacaaacgtgctaaactttgggcgttgagataacttgttggttctactttagaaaggatcgattacaatgaccaaagtgttagcagttctgtatccagatccagtggatggtttcccaccaaaatatgtgcgggatgacattccaaagattacccactatccagatggctcgacggttccgacacctgaggggattgacttcaagccgggtgagttattgggcagtgtgtctggtggcttgggactgaagaaatatttggaatctaaaggtgttgaatttgtggtcacttcagacaaggaaggccccgattcagtatttgaaaaggagcttccaaccgctgacgttgtgatttcccaaccattctggccagcttatctgacggctgatttaattgataaagccaagaacttaaaattagcgatcactgccgggattggttcagatcacgttgatttgaacgctgccaatgagcacaatattaccgttgccgaagtcacttatagcaacagtgtcagtgtggctgaagctgaagtcatgcagttattggcattagttcgaaacttcattccggctcacgacattgttaaagccggtggctggaacatcgctgacgccgtttcacgggcctatgatttggaaggcatgaccgtcggcgtgattggcgctggtcgaattggccgggccgtactggaacgattaaaaccatttggggttaaattagtctacaaccagcgtcatcaattacctgatgaagttgaaaatgagctgggactgacctattttcctgacgttcatgaaatggtcaaagtcgttgatgccgttgtcttagctgcaccactgcacgctcagacctaccacctgtttaacgacgaggtactcgctactatgaaacgtggggcttacatcgttaacaacagtcgtggtgaagaagttgatcgagacgcgattgtgcgggccctgaattctggtcaaattggcggctactctggggatgtttggtacccacagccggcaccaaaggatcacccatggcggactatgccgaacgaagccatgaccccacatatgtccggaacaactttgtctgcccaagcacgatacgcagccggcgctcgggaaattctcgaagacttcttagaggacaaaccgatccgtcctgaatacctgattgcccaaggcggtagtttagctggaacgggtgctaagtcttacactgttaagaaaggtgaggagacgcccggcagcggggaagctgagaagtaggcttgctcatataatgctcaagtaaaataaaaaggttctgcaatatctgtcgttaatagatgtttatctattgctggtggcaggtgttgtagagcctttttgcttgtggtgagcaattagagattgattgttaaccttctgcttcatggatatcatcttggatattgtccagcgaaaagtcatggtccatataatcacgattatcgactggcaggtgttgctccaacgtatcgaacaactggtaagccacgtgacccttatccaggtggaagtccagcagatgaccgccaaatgttttgtcagcggataagaaatggttgtggaatccagcaactgcagcgccgtcaaataaggttggcgaatagtagctgatcagcgtcccttcaacttgatcacgagtaaagatactttggttcttagccgtttgagccaatgtttgaaatggcggcgttgatttcttgactgcccgggtcttgacggctgagaaacttccagtgatcttgatcgagaagaacgtgttgctggcctgggtgagtgagatgagctgttcttccaaatcagcttgagaaagattttccaattccgccaaaggtgagtagttggcgaaatggctgttcgcaaatggcatgttgaaggcatccgagaccacattcacgttgccgtcactatccacttggtagggcgtcccgtctaaaatgatcaattcaccgtcaaggccttcgccggtgccaatcccagtgtcaccatgttgcagtaagtcacccattgtcagggtgcctgctagcaagccggggaccagtaatgccaaagtgccgtgctgatacaaagttgttaattttgtcatcattatcctcctttagtttaagatgtctggtaatagagctgatttgagttcaatgttgtcactgtagtcaactggaatgtcgatgataaccggtccatcagcctgctgtgcctgatcaagggcattggccaattcctcggagttggtagcccgcaatcccttggcaccaaagctttcagcgtatttcacgtaatcaaccggcccgaatttcacgccggcattcttaccatacttggcttcttcttggaatttcaccatgtcatagtaaccgtcattccaaatgagctgaacgatgtttaacttcagtcggactgcggtctcaagttcctgaccggagaacaggaagccgccatcaccggaaacggagatgactttttcggctggtcgcaccaatttggccgcaatggcccacggcagtgacacacccagagtctgcataccgttgctgaacagtaaatgacgcgggcgataaattcggaagtgacgcgccatccaaatataatgactgccgatatccaccgtcaccgtggtctcgtcgtcgactttttcctgcagcgtattgacgatgtccagcggatgcatggtaccgggcttggcagtcgttgcagtggtgctttgaccatcaaattctgatcgcagtttggcgagttgatcgactgccgtttttggaaggtgatagcttgctggcagagcatcggttagggctgacagggtgcccgcaatgtctgattcgatcaccatatctggttggtagtcgacggtcaactctggggccaccgtatcaatgttgataatttggtcgttgtgttctacgttccagttgcgggcctcgtattccaccggatcataaccgattgcgataaccaaatcactttgcttaagcagggtgtcgccaatttgatttctgaacaggccaacccggccaaagtaatccgcttcaaattcgtgagaaatggcgccggcaccttggtaggtttcaactactggtagcgaaacttttgccagcagttggtgcaaggcctctgtgacggctggagaagacgcccgcatgccggccagaatgactgggagtttggcctttttgagtaaatcgataatctggttgagggttttggcggatgtctgagtttgctcgggttctttcaattgttgcatttccagccgggtgacttcgccgcttaacacgtctgctggcagggaaagaaaggaagccccgggcttgcctgaaatggctgtgctgtaggcgttggtgaaggcttcagaaaggttgttggaatcttggacttcaacgctgcttttggaagcgacgctcatcaattctttgctggggatgctttggtgggtgtaacgggcaaggtcgtcgcgggggacctgtccgcccaaagcaaccaccggatcaccttcagcggttgccgtcattaaggctgtcaccaagttggaaaccccggggccggaagtggtggcaaccactcccggtttacctgtcaaacggccgatgccagccgcaatgaaggcggcgttttgttcgtgacgtgtgacgatcaattttggtgcgttgggctggtcgctgtactggagatcttcgaataactgatcgactttggcaccggggatgccgaatacatattgaacctgttgattaatcatggattgaattaaagcttgtgaaccacgttttttatttgccataaggaggacacctcttcatttttatgttgacaattcaacttacatttaaagataaagggcatgtgttgaattgtcaacaagaaaatgataatcttacggtaggatttgacgattggaaaggaaaataattttgaaagatattggctaccttgcacaggatatttcaattttgcaccggcagtattacaaggataccggtaagttgtttaaggagcagcagctgaacccaacggctgcctgtattttactgacgattaatgacaatgccgagattaatcagaaccaggtggccaagtcgttagtgatcgataaaggcctggcgacgcgagagattaaaaagatgcaggccctgggttatttgacgaaaacggccgggagcggcaaatcaattatcttgagtctaacggctgccggccagcaggtgattcccaccattcaggcaatccggaaaaactggtgggaggaacggttcgcagacactgggattcagcccgatagcccgttggtgagtgcgattgagaaggttgttgactcgattgtggatgagagtttggagtaggattgtagcaccaaaaaatggttcattggaaaggtttgaggagatcctcagtagcctttgcaatgaaccattattatgatgaaccgttaatcaatgattgaatttcgaattttgagctcactttcaacaagcactgttttttctacaatcggttggtcggagatgaggtcaatcaatagttcagcagatttttgtcccattttctttggattctgctgaatggtggtgatctccggctgcattaattgcgcccaatcccaatcatcaaatgctgttacaccaatatcttttgggattagaatatggaattttgataacaactttatgacacgcattagaacagttcctttgagggcatagacaaccgctttggtcttcaaggaatcagtttttctcatgatctgattataaatcaaatcatcagaggtattttcagttatttcgatactgtctacgatgacatcggtgcccttggcggcctcttgaacggcgtggtaacgatccatccgcacttcattatcagctagcggttcactgatggtgacaattcgtttatatcccatacgaattatcaagtccgacaatgcctttgaatagccatagttgtcggtagttacttctggccagatttgcggcgttgtttttcgatcaacaataaccgttggtgtatcggtatctttaataaattggtaactggcactgttattatgaatcggttgcaggataatgccatcgacttgaagatccaaaagccgttggagctgatcatgttcccgatcaccagagttgtccgagttcatcaataatatttgatagccatgctgctcgaagattttatcggctcccttaaataaaatcgaggagaaaatattttcaatatcagcgacgaccattccaattaaatgcgtggtttggttctttaatgactgtgcttgacgattgatgtgatagccagtgtcattgattacatgctgaactttaacccgagtttcatcagacattttttcaaagtgaccgttcaagtatcgcgagacggttgcagtggaaactccagccatttttgctatttcactgattgttaaacgctttttcacattaatcacctcacacttccgtcacttaattgtacctgataatttgatgttagggaatagttcatggatcttggatcactggttatcttgggtacagatgatacagacaggttctgcaacattgtgattgactgatagaagtgtcaaatttccgtgcttggggttccgttgaaagatggcgagtgagtcactcttttgattacccacaattacatatttttctgactgatcaagacagaactcacgagggaagttgccttcactggagatgttttgaatcatctccaattgataattagtttcatcaacaccaaagacagacactgaattatgtccacgatttgatacgtacaggtacttttcatctttagaaaggtacattgccccacaaccgttttctccaacccagttatcaggcaacgtcgaaatagactgtatctgatcgaaggtaccggtcttcggatggtatttcaagagaattacctggtttgccaactcacccagtacataggcatatacgccattcctggtaaacgtaatcttttttggtccaaatcccggccgggtatgaaacgttgtggctttttgaaggacatgaccatcagatgaaaggtcaaaagtcaagatttcgtcggtacctaaatcaatcacacagagacgacgcccgtccggcgttatctgtgcatagtgcagatgcgaggtgttttgttgaggtaggaccccgtggcctaagttatgaatttcatcgaccaggctcagatccccgttgctcatgattttaaaaatctggacgaaaccgttattataattgctggcgaaaacaagttttcgcttttcatcgattgtaatgttgacgggagatgaagcattaaataagtgatcagcgagcttgttgaactgaccaccggaaagatcataggcggaaacaccacccttatcgccatcttggttaacggcgtagattacattggtatctgaaagtgccaaatatgtcggggccccaatttctgtagataaatgaactgtccctattttgccagaatctgtatcaaattcagcttggtaaataccctttgaaattcgtgatgaataagtgccaaaaattaattcttctttcaaaatcagttcctcctaagcaaaatgtatcctacttaaacataatggcagccaacaataaattcagaacgctggtaatccagccaaacggaacgccggtcatcaaaaactgcttaacatctagtttctcgtgttcgacaacccataaattccatgattgggtgatgcatgttgagatggcaatagatacgccaggtattaagatggcagcaaaggcaaaatattggttgaagaatccggtggcagcaaggactgcggcggtggccgaaccagcgccccacaccatcaatgggccacggaacaaagccagtggggctaagattccaaaagcaattgccagcacgatgggactgtggggaacaatgctttgcaggatatcgctgaatctgccggtaacctttaccgctgcggcgctgaacatggttaagaatagtaacataataattaatcccgaaatatctgaaatagcctgggaaatagttttgttgatcagctccattgctgatttgtaggttttgagttttccggtaatcaacaggaccaaaaagattgacagcattaatgcagggattggttcccattgaaaggccaagttcataaataccggcataattggcaggatataggcaatttttggtacgttggaaattgcttttttgctgtcatcagcagagacctctttggtgtcatttttgtgaattgattttgcatggatcaagatgaaaataatgacaattactaattgtacagacatcgcactgaaaccataaataaggtatttggcgccgtaaacaaccttagggaagaacaactgtaattgcttgatgataacgatgttgacgtacattggggcgccgatagacatgacaaacgccgtaattgcgacgttctttgatagtcctaatgaccgcaggattggtaggagaatcacctcaatagcgataactgctccgacaccgtaggaactggtaaaaatgaaagcagtaacaaggcaaatcagaattgtcgcgatgattggtcgtttgtagctgactttgacggtctgttcactaatggcactggcaattcctgtatccaccagcacccgtccaaaccaggacccaaaaataatgaccataatggtcgatccatagttaagagcaggctgtgagaaaacgttggtaattgcgtctttataagagataccaccaatgactgtccaaaggattgccatcattaggaatccaatcatgatgtttccgcccttcatgacaaaagcaatgaaaccaacaaatgtcagtaaaagaagaacaccgataataatatttatcattttgatccacactccacacatttatttgtctaggtaaacgattaactgaaatcgattacatattaacccgtaacattgtgaattgtcaaacaaaattttaaattctcgacccctcctttaatgctggttctaaataaatgctataaataaagggattcaaatatattttagttagggttgacttttataattacgtagattagtatgatgttgtcaaagggtaatcgattacatgaaacctacaaacggaggtccaatttgatgaattctaacagattagtattaaacaccttggttgcgcaggcagctcatgatgcgggttcaaatcaggagcagctggtggaagacttgttgagcagcgggattaataatattgagttgagaagagagtatgggaatgccactattaatgagcttgatcaattgtccgaattaggaaaacgtgatcgactgacctacttttattcagttccggataacttatttgttaatcagcagctcaatgtaaagttattgcaatatgttgctgaagcgcagcgcttaggagcgggatatatcaaaatgacattgggagactacaatgacgcaaagcctgattgtattgatgaattgttaactgttattccaaccagtattcagctaaatattgagaatgatcagaccaccagcaacagtgatactggcaagctggtattattcttcaaacaatttgaccggcgtgatcgaaaggtcggatttgttaacgacttgggtaattggatttttacgaaccaggatgctttgactgccacaaatactctattgccatatacccgattcattcacttgaaaggttttgtgttgaatcaggatggaaatcctgagacggtgtcgtttgtccaaggaaaattagattggtgggaaattctcaggatctttccaactgatttaccaattgctcttgaatatccggcagacgcagacatgttgaacagtgatatttcaaagttacttaataactaaggttaatgaaagagggtataaaaatgggtaaagaagttgcattcaatacagataagtttcgtctcgacggcaaggttgccattattaccggtggtgcatcgggattggggtacaactataccaaggcaatgttgatctctggggcaaagattgtgattgccagctatgacgaaaggggctgggaagaaacaactgaattcgccaagagtgttaatggtgaagttaagttcatcaaagttgatgtgactgcggatggagcccctgtaaagattgtcagtgaggcactttcggactttggccaaattgacattcttgtcaataatgctggcatgcagcgccgcgagaattggaaagacttcaaagattcagattggaacgcggtcatcaatctgaatctgaatgctttgtatttcttatcccacgcggttgctaaagttatggcaaatcaaggttctgggaagattatcaacatcggttcgatgcagtcgtttagagctggaaagtttattttcccatacactgccagtaagcatggggtcgttggtttgaccaaggcatatgctgacgcattggctcctgataatattcaggttaatgcgattgcgccgggatacattgacaccccaatgactaaggcccttcaagaagataaaagtcgaaacaccgaaattttggctcatattccggctggacactgggcggatccatctgaactaatgggaaccgttgtctttttggctagtgcggcatccaattatattactggcgttacgatcccggttgacggtggatatttactgagataaatataaggagaatagattatgggaaaaaatgttgcaataccacaaggcttatcgcaagctgggaaagactatttgatcaaccatggaatggatcttgttgagttgccggataccaaagcagaaacaatcatctcacaagcaccaaatgtcgacggaatcgtgctgatgactgaaccatttccgaatgaaactattaagcaaatgcctaatctgaaagtcatcgcccgccatggggtcggctttgataatgttgatcccaacgacatgggagaaaacaatgtctgggtcacgattacacccaacgctaatgcagccacagttgccgagacaaccttggcagagattctggacatctcaaagaacttaacggcgatttctgatagtatgcgaaaaggtgtttttggttataagtcatcccacatggggtttgacctggcagggaaaacactcggaattatgggttatggccggattgggaaaatggttgccaaaaaagtcagatcattggacatggatattttaatctatgatccgttcgtcaaattcgctgaatacggtaagatcgtcgacaaagggacattgattgccaactcggatgtcatcacgctccatatggctgttactccagaaaatgagcaggggattgatagggatgccttcaggaaaatgaagaaatctgcggttctgattaacttgggccgtgggcaattggtgaaccaaaacgatttgttagaagccttgaaaacccatgaaattcgtggtgcggcattggatgtgttcaacgaagaaccacttcccctgacaagtgaattttacaagttggataacgttcttttaactccccatattgcctccaatacaacagagtgtatggcaagaatggccgttgattccgcaagtgaagttgttcgagtactttctggtgaacagccaaagtggccggttaattcagttgagtgatagtccttgataatagccgtggaaattaattgaagttaatagatgatctgaaatggaggaagcgatagttataatgaaaaatagtctgattccccaaatcaccttaaatgatggatacacaatggatgcaatccaatttggcactttcaaaatacgtggtggtgagggtctgcaggagacacttgctgctattaaggatggctatcgcagtttggatactgccacaaattatgataatgaaaggatggtcggtgaagcaattcgtcattcgggcattccccgggccgatttcttcataacttcaaagttacccggaaaatatcatcaatatgatgaagcaaccaaagcaatccaagaatcactgtatcgtctcggactcgattatctgggtttgtatttaattcattggccgctgccaaagcgtgatcactatgtagaagcttttcaagcgatgattgatgctcagaagcgtggcttaattcgttcaatcggcgtttcgaatttcgagccggagcatctggaccgtttggttaacgaaacggggattaccccagctgttaaccaaatcgaggtgcacccttactggaacaatgcgcggatgctgaaagctgaccaggaacgggggattgtcacagaagcatggagcccattgggacgaggaagcgcagctttgcaagaaccaattatccaggacctggcaaagaagtatggtaaaaatagcggtcaaatcattctgaagtggcacactcaaaggggcattatcccagtcccacggtcaagtaatttgattcatcagcacgccaacaaggatctctttgattttgagttaacagaggaagaagttaaggcaatcaatggattaaccaaggcagctggccgtgttgacgggcaggatcctaatgtatatgaagagtttgattagtgattggaactaataccgtttagggtgggaaatgtctccaccataccttggaaagtatctggattattcagtagcttgaattacaaatacaatttgtaaatgcaggagtgatttcaatggagaaggacgttagaacgcacattgatccggaaaagtttgcctatcaagcgctgacgacaattcattttcatgaaacggatgattacgaacggcaaaacaaggagcgattagctgtttttctgatgctaaaatatttggctgatgactttaatgatttggaaagcaaggcctttgatatcagcagtaacaacgacgaacagttgtcgaagctgggatttgacgacttgctgtcacggatcaatcagttgaataagtattgatggatgggcacaaattaataacgggttaatttggatgtaggctgattcctgagacaattgtctttattaattagcgttgtacttgacttgacaatttaagttaaaataaatcaaatcacgcctactgagaagaatagcatttctcagtaggcgtgatttttaatccatataaggacactatttatctttgtcaacggcagtttaaaaatgtaggtttgggggtgacgtttacacccctcttctatattttacgggtgccgtcttaattgtattagtgtttttttacggctattgtggttagcaactgcttaacagcagccttatgattgctcgggttataaagaatatcagaagaatacgttgtatctacatccatatcttcaattggcaagtattgaatcatgggatttacaatttgctcacgtttcataaatggacttggataaaatccaattccaaaattgaaggcaaccagcatgtctcgttgctccagtgtattaactcgtctaattttttcactatcaattttatttggaaacttttctaggaagatagttttaagatatgaggattcaaccggactataatataaaatttccatgttagaaatctggttaaacttgattgctgtctgtctacttagcgggttggatttactgataccaaatactagtttcccactggcgatgctttttgaatgtaaattagagttttctaaaaagagtgttttaccgtagtttggtgtgactgctagatctagtgtcccatcactgatgtgtgtcgctagtcgttggccattttcctctttaaaggcaaatctaacttgaggatgatcttttacaaatggcaaaaacagattttgcagaatcatcccttgattagtagaagaatagccaatctttaacgtacggttacgtttgcttttttctaattggatcttagtaattccactgttgtagctgtttacaatatcttgagcagttactaggaactctttaccagcacttgttagttcagaattgttagtttcccgactaaataatttaatgcctatttctgcttcaatttgattgatttgcttagaaactgcccgtggtgataaatataatttgtccgcagcggctttgaaacttccgtattcaactactttaagaaatgttgttaatttagcaatttccattcatttctcccccagtaaaagaacagttggttcatctcatgtccatttggtcactgttcataagtgtatgttatcgatacaatgtattcgaaaacgttttcgtaatacacatcgatgtattctcacttgctcactgtttaatatgtaatcagcgtttaagcactaatttatatacactggttactttagcacagcttatgacttgttgatagatcaacataaaaaaaggtttaatactgcaattaaaccaagtgcctgataccatccaacttttaagcgctcaactgtgtgaggttggaatagtatatttttttaatgctgattgctcaacaaaacacattcaaataatggaggtacattaaattgggcacttcatatgttgcttttatcggatttgtgatgatgtttatcatcatttatttgctactaaagcaaaaagtaagcaccatgtttgccttttcagttattccaattgttagtgcgttcttagttggtatgacacccactaaccttggtaatgccttggaaaagggattgggaatgacaacacctgtttcacttatcatgttgttctcactgccatatttcatgatgatggctgatacaggtttgttcaacgaactggttagaaagattgtccgtcatgtcaagataacaccacctgtactgacttgtttaacgattgttgttgcaatgattgtcgggatggatgtaagcatcacctcaatatacatcattgcaattccattgttattgccattctatcgaaaattacacatgagcccaatgctgttgatgtttctgacaactttgggagttatcaatacattcgatgttccttggagcgctagaatgttgcgggcagcctcactggtaccaaacgtaaagggtggttcaattgcgttattttcaaagatgctgcctacacagatagttttcacaattgttctgtttgcattagcaatagttcttggcattcgtattcaacataaaaataagaataacggcgagatcaatgacgatgagttggaagatacctcacaatcaacagatagtattcaggatgaccctgaattggctcgtcccaagatgttttggattaatattatctttaccattttcttggttgtttgcttagttatgttcccaacaattccatcgtattacatttttgcgttcggtttagttgttgcgtttgcttacaattacccagacttaaaaatgcagagtaagctattgaagaagtattcccgctcgttgatgcccgttatgccaactatcttactttcaggagttgttgtgggggtaatggaatatagcggcatgatgaaagcaatggtcaatatcttgttgaagattattccatctcaattgggaccgtggctctacattattattgcgttagtcggcgtacctctgatgttcctgtttaccaacgatacttggtactatgtaatgctgccaattgtcatttcaatcatgaaagcatacaacattccaggtgaaatcgttgttgtaacactgtttatgaacatgggagctatgttaacacctattgctcaaccgcagatttacattggtgccaatatgactggtgatgtgattacgattccgcagttcatcaagaagagtttcttgccaatttggggattgagtattgtttggaccctcattggattaatgatgggtgcatttagataaaacctaaaatatgtcttgcgtaagtaactagaagtttaaaaaggagagtattaaaatgagtattccaaaaattgttaaaatggatgtttatccggtggctggctatgacagtatgttattaaacttaagtggggcacacggcccatatttcacacgaaatatcgttgtcttaactactgatgaggatcaagtaggtgttggtgaggtgcctggtggtcaggcaatcacgagtactctagagaaatctaaagaacttatcgttggcaaaagtattggagagtacaaacaaatcctccaaaatatgcggaaaaaattcagctaccttgatgcaggcggccgtggacaacaaacttttgacctacggacgactattcatgcagttactgcgattgagactgcttttcttgatttgttaggcaagcatttccatgtacccgttgctgaattacttggtgatggtcaacaaagggaaaatgttggtgttcttggatacctgtttttcgtgggcgattcaagcaagactgaccttccatatcttaaaaacgatgataactctgatgattggggtaaaattcgtcgtggaccaatcatggatgccgcttcattagttaaatcggctaaagcggcttataaacgttatggatttaagacatttaaacttaagggtggagtttttgatggtgaaactgaagttcaatgcatgaaagctctgcataaagcttttccagaagctaagcttgatcttgatccaaatggtggttggtcccttaaagaagcacttaaatatgcggatgaattaaaggatgttcttcattacatcgaagacccagcaggggctgaagacggattttcaggtcgagaaatcttatctgaattccagaaaaaaactcatatgccaacggctactaacatggtcgataccgactggcggcaaatgtcccatgcgattgcattgaatgcggtatcaattccattggcggatccacatttctggactatggaaggctctgtgagagttgcccaattgtgtgacgaatttggcttaaattggggtatccattcaaataaccactttgatatttcacttgcaatggctgtaaatgctgctgccgccgctcctggttctgtatacgacattgatactcactggatttggcaagatggtcaaaacttaactaagaatccttatcaaattaaagatggccaagttaaggtaccatcttcaaatgaaggtcttggcgttgatattgatttagatgcaatcaaaaaagctaaccaactctatgtagaaaagcatcttggagcccgtgacgattctaaaggaatgcaatatctgattccgggatggaaatttgatcctaaacgtccagcattggtgcgataagataacatgtttttataatacgatttcactaagaaagtaggctgaaataggtatgataagtccaaggattacgtcattagaggtagtgccagttgctggtcatgatagtatgctactcactctgagtggggcccatgcgccattattcacacgaaatatcattattcttcatgatgatgctggtcatgaaggaattggtgaaattcatggtggggatgcaattagtaagatgcttgagagttatcaggacattgttgtggggcaagcacttgttaactaccgaaagatcttaatggatgtaagagaaaacgggtggcgccctaacaacaactccggtcaaggattacaacagttggatctaaagaacctgaagtttgttgtgcatgctgaggccgctttagaatgtgctttgctggatctttacggaaagtttgtaaacctaccaatgtgtgacattattggtcaagggcgacaaagagattctgtggagatgctcggctacttattttacatcgccgactctgcaaaaacgcatttgccatatgtacaaaatgatgatgactcagacgactgggggaaactccgacgtaaaccggctgtgacaccggatgctgttgtgcgagaagcaaaagcagctcagaaacgttatgggttccactcctttaagcttaaaggcggtgtattggatggcgaaactgagatggcaacggttgatgcattacacgacgcctttcctaattgtcgaattaacattgatcctaatggtgcatggtcgttggatgaggcgattaaactgacaaatgatcaccgggattccttaacctacattgaagatcctacgggaccagaaaacggcttttccggtagggaaatcatgagcttttataagaatgcaaccaatatgccagtagcaactaatatgattgcaactgactggaaacagatctatccatccctgatgatgaagtccgtagacattattttggcagatccacacttttggggcattaatggtagcttgcgagttgccagcatcatgaatgattggggcttaacctggggatcacactcaaataatcattttgatattacattggccttatttgcgcaggctagtgcagccgcccctggaaagatcacagccattgatacccattggatttggcaagatgatcagcagttatgtgacgatgctatgaatattcatgacggtaagattacaattcctaataagccgggtttgggaattaatttgaaccatgagaaattagaaatggcgcatcaactgtatctgaccatgcaaaatcatgatcgagatgattctatggctatgcagtatctcattccaaattggcaatatgaccctaatcaacctacattggttagatagattaggaaagggacaaataatgaaaaaagtattaattagtgaaaaaattgacgatgacgctgttcagcttttgcagaaaaatggctttgatgttgaaatatcaccagccgtggacgaagctacgctaacagaacacataaaaggggcctttggcttaataatgcgttcaagtaagcttcctgaaggtgttgttgattcggcagatcagcttaggattatttcgagaactggaacgggcattgataatgtgaatattgatgatgcgacaaaaaatcatgttttagttgcccgggttaatggcgcaaatgcatattctgttgcggaatatgttattactacaatgttagccatgagtcgaagaatctataaatcagatagattattcaaggcaggtcagattgtttcaacgcatggtgaatccttaccagggttagctgtcaaatatgacttgaacggacacgaaattcgtgggaaaaggctgggaatccttggccttgggagaattggtaaaatcattgctaagcttggggatgctttaggtatggacatcattggctacgatccctatgtgaaggccagtgatgtaaagttaacaactgatctcaacgatatttataattcgtgcgactttatctcagtaaatatgccgttaacgaaggaaaccaagaatcttatcgctgctaaagagcttggccaaatgaaagattcagcatttatcgttaatgcaggccgaggcggaatcattaacgaaactgatctggctgatgcattgaataatggtgttgttgctggggcagctcttgatgtatttacagaagagccccctcgtagtgatagtccattattaactgcaaagaacatccttttgacagctcatattggtggaactacttatgaagccagtaaagctgttgcgattggcgctgcgcaagcagtaattgattattctacaggcaaaaagccacagttcacagtaaattataaggatcttaagaattaaacctgttaagtaccaatactcatttttactgtattcgacaaaacatgaggattcaatttatgaatcctcacgtttttttgcattgatttgacttgaaatatattctggtacctttggatgaacacgtcctttatattccgatggtgtggtttttaagtactttttaaacaatcgaaagagggatgaactattttggtatccaaccgtttcactaatttcacttaggtttaggttggtttttagcataaggttttgtgcggcggataggcgtcgcctttcaataagctcattaaaggtttttccagtgttagctttaatcttatttcctaggtaatttgtattgtatcgaaatacagcgctcacattgcttaatgtggttgtggcgaagtttttctcaatgtatttcaatatgggtagcaaatcgtcactcgaagaatctgcaaaattgatcgacttgtaggtgatgagactgggaagtcctaaaattaaggccgagaaaatgaagcgtagtgactccgatctatgtcgtgcatgattgattcccgttgcaatcagtgcatttatcaaattgagggaagtctcggcgttttttaggtcaaacagcataaagttattatgcagcgagtttactcgggttccattatagatgagttgagtaatttcattggttgattgaggaattgaattaaagatttcctcatagggtgaatcagtttttacaataatgttgattaaaatatcgttctcatttgtgtaatcaattctttggacgacatccttgtccatgactaaaagttccttttcatgtaatacagtcttggtgtcattaatgtactgagtacacattccggagtacatataattaaattcgatgaaactatgagtatgagccggtacgtacgaaaaacgattgtttttggtaacatcaatgtcgctgtcccaaaagaaatcccactggggcattcttgggataggatcgtgtatatagtccagatccatatagtttacatttccaccaaaatgattttgtaatttttcaactttagtcattctgaatagttgtgatttaagcgattcaatgggcttcataagtatcttttcccccctgtacaaagtggaatacaatttgtaatctgtgattatgcatgataaatcgagtgattaagatattgtagcataatctggtagcgcttacaattatcactgtaaattgaaggagggaaccaatatgaataataatacagttgattcaagctttaaaaagtatcgaccgctcgcagttgctgctggaattgggtcgatattaggttcggggattatcgttgggttatcggctaccattaccgtttggcaaactggtctaggcttaacgaatacgcaagttggcatcatatctggtgctttaacgtttgcgattgcaattggttcaatgattgctggtcaaattacaaaaacatttggattaattcgttcatttaactggttaaatttattatatgcaattggtgcattggtttgcgttttttcaaacggatacacgatgcttttatttggagtcattataacaggcttagcttctggagcagatttacctattagcttaacagtggtctcgcacgattcaccaaatgaaaagacacagtctcagttagtttcatcaactcagattttttggcaaattggaatatttatgtcatatgtttgtgcatttattgtttcaaaaatggcaggtgcaagtggtgccagagttgttttcactattttagccatttttgcattaattacatggctttggaggactttctcaagtaaattcagggctttccatcaagaaggtgaaaaacgccgaattaaacacgatcaagaagctaaccttactgacaaagtatctgttaagaatgtcttcactggatccaatcgaagtaaatttctgggctttttcttagcaattatgattttctatatttgctggaatttgctagctaacacctttggtcaatttcaaacatttgtgttggttcaggcacatgcaactcaaagctttgcgactgcagcgggattaattcttaacttggtttcactgtgtgcaactattacttttgcatccgtttccggtggtaaatatcgaaacaagttcttcattgttggggctttagttcaggcactagcaatgttgggcttggctttaagtagccacgcactatggccaatcgttatcgccattgggtgctacagtatcggtaataatgttgctggagaggcaatgtacaaggtttggacacaagaatcatttcctgttgagatccgcgcttccgtacaagggtttatcaatggattttcaagattcctatgtggtttatttgcaattgtcaccccagctttagttgttccatctgctatccgaaataccatgtttggttttactgggttagtaattgtatttttcattgccggtttagtaatgatgtatctccaaagaaaacacaatattattccgggtgttgaagagaatgagaggggcgaagacgatggcgttcacatttcaaatcaatgatgaagttcagtttaatcacgatgaacgattacttaataaggcaaagcaatataagcctgttattcatcaggatattgtatttccaaagtccattgttgaattagtacccgactctcaaaaacttgaaggatggggagttcaagatactcaagatattgaaggcctaccaaatattaagctgaaaagaaatcagaagattacgcttgattttggtagtcaccaagttggcaaatttagtatcgatatcaattcagttggctcgccgatggatgcaccactttttatcaaattgaaatttgcggaaatgcctgcagaattgaagcataaaagcgaggactaccacggttggctgagtaagtcttggattcaagaagaatacattcatcttgatgtattaccaacgcatctggaattatctcgtcgttatagctttagatacgttgagatcacagttattgatacttcgccaaagtggcaggctgtcttgtcaaatccacaagtagaaagtgaaacaagtgcctcgaatgaacaattgtccgttccatcgatcaaagatcccgaaatgaaaagtatttatcaagttggattgaaaactttgcaggattgtatgcaagatatttttgaagatggcccaaaacgtgatcggcgcctgtggattggtgatcttagacttcaagcactggcaaattacgcaacgtttaaggatgtggggttggttaagcgatgtctatatctatttggggcaatgacagctaaagatggccggattcccgcaaatgtgtttactcaaccccaagatatacctgatgacacttttctcttcgactatagtttatttttcatttcaattttggatgattttcaacgatttaaacaagatcaagaattactatcggatttatatccatttgcaaaaaagcagatggatgttgctttggagaaagtgcagctcaatggtgagctcattcttgatgacagttaccctgtatttatcgactggtccaacgactttgataaaaatactgccggtcaagcagtgttaatttacactctacggcaatttatccatttagcaaaaatgatgaatgataatgttgatggatactcacaaaagctacatgaacttatttcatatagtcagtttaatttgtttgatgctgagaaagggctctttgtttcaggacctcagcatgaagtaaacattgcttcccaagtttggatggtccttgctcgtgtgttggatgatcgtcagaacaaacaagttatgattcatacaattaatgaattatttccgattacagggattgcaacaccttatatgtaccatcacattactcaagcattatttgaagcaggcatgaacgatgaggctattaagctaatgaaagattattggggacaaatgatctcactaggtgccgatacttattgggaagcatttgagccagctaaacctgaatattcaccttatggaagtccaattttaaatagttattgtcatgcatggagctgtacaccagtttatctgattcagaagtacctgattggggaggaataaccatgggtaatgaaaagatttctttaagtagagataatgtattgctgattatcgtggccggaattgcatcatatctcgacgcggctctacttgtaagtctaggagttgcattaccaatttgggcagactatttgcatttgaatagttggattgttggtttactaagcaccactttaacaattgctgttgctgtcgggtcgtttgctggtggttggctatctgacaagtttggcagggttacggtgtttaattatgacattctgtttgtagcaattggctctgcaattgtggctttttcaagagacgtaccgttactattagttggtgttattgtggctggcctggcttcgggggctgatttgcctacatcattggctgtgatttctgaacgaatggataagcggacgtatggacgtgcaattgcatctacgcagattttttggacggtaggaatcttactttcacaattcattggtatgttgagtgccaatgctggcatgggaagtccgatgaccctgttcggctggattggattggttgcgttcgtaaattggtgtgttcgagtgttttctaaaaatttccgtcagattgaagaagggttggccgaggttgttgaggaaaagatggagtcagttggggaagtaaaaaagcgctacaagctgcgagaattattacggaatagtagttaccttcttccacttattttcctaacaaccttttatctgttctggaatttacccgccaatacttggggatcatttgttaattattttattgtaacggttgataaccgtagccaactatattcaacagtgattgccttagtggctaatgtcttttgcctacttgtgaatgtgatttacctgaagatttctgattccaagtatcgatataaagccatgtatgtcggaattgcgactgccctaattgcatttctttcggcagggatatttagtgaccattggcaggtctttacctttgcatatattttctattcaggaagtacggttctctgtggtgaagctttatacaaaatttggagtcagacattctatcctgtggatgctagagcaaccctgacaggcttctcatatggatttgttaggataattaccgccatgttttctttgattacgccgacgttgatggggtattcacccaaaatcctcttatggatcatggtcggctgcacgctagtttttggaacctgtgcattgatcatcgttcatttggttaagcggtttaaagtgtcagatccaaccaccatcggtcacgctctgtctaatgagagttagcattgttgatcaacttattgaaaggagagatatttatggattcaacagcacactggatttggtatcctggggatttttcgattcaccaaggaatgctacaaaattttgctcgggaagagcggggaatgggttggccggcatattggtatattgatgactgtaatcggaatataaacttttcacgtacctacgatttggataatccaacagactttacagtgtatgctcgcggtataggttatgttgatattaatgggaaaaagtttcggttgggagagactttgaggtgtgaatccggcaaaaatgtaattactatttttgtcggcaatccaactgggcttccctgcgtgtatatcgacggactggtggttaaatcagacaaaggttggcaagcaagtaactttgtttcagaactacctgcaggtaatgatccactgtttacaagcaaagatcagaatcccaatgttatcgaatatcaaaaagctgagttaaatccgactaaagtcaaagaaattgataatggtgttcttttcgattttggtagagctgtgaatggtagcttaaaggtgaaacttcatcaaattgatgaagtaaccatttgctatggggaatcacgcactgaagctttggatgtggatatgtgctactacaagcaggaaagcgttgatgagacaacccatattcgaaaacgtgcgtttcgatttgtgtttatacccaacgcaaagaaagacaacatcaatttaatcgccatccatgaatatattcctaagcagaatatttccgacttccaaactgataaccctctgattaacaagatctggaatgtttcaaccgaaactttaaatttgtgtagtgacctgttctttatcgacggaatcaagcgtgatcggtggatttgggcaggggatgcataccaggctaacttcatcaaccaatactcattttttaacgaggaagttgatcgacggacgttgcttgcgttaagaggccaagataatattaagcaacatataaacacaattgtcgattattccatgctttgggtgattggtgttttgaatcattatgaaatgactggtgatcgtgaattcttaaagattgtttatccaaagatggaaagtatggttcggtattttatcaatcagacgaataaacaaggttttatctatggtcgagaaaacgactggatttttgttgattggtctgaaatcgacaaagatgggactgtagcggctgaacaagcattgttaattgaagtttataaaaccatggttacgtgtggttcggtccttaatcgtccgattgagaactatcaaacattacatgaccaacttttagagaactttcttcaacacttctggaatgaaaagaaaggtgcatttattgatagctacgaatctggtaagaatcacgttactcgtcatgccaatatctttgcgatcttatttgacttagtggatgatgataaaaaagaatcaattctcaaaaatgttttattaaatgataaaatcacccggattactaccccttacttcaaattctttgagcaagacgctctctgcaagatgaaccgtcaagacattgtctatacaaccatcttggattactggggtggcatgcttgccaatgatgcagtcacattttgggaggagtatgatccaacgaaatctggtaaggacatgtactcaatgtatggtgatccatacggtaaaagcttatgtcacgcttggggcgccagtccaatttatcttctaggaagatactttgttggtttgtaccccactcgtcctggatatcgagagttccatgtcgagccagaattggatcagtttaataaatttcatgctattttgcccattaagaatggtaaagttatcgttgataaaaatggagatacgctctctgtgctcgcttcaaagggtggcggaacgttggtcttaggcaagaatgaatatgccttgattcctaataaaaagttaacagtatcattgaatcatgcgaaagtggatgctgggtaattgatgatcatatagtcatttacgcatacgtaaaaggatctactttaatattttcccgagatgaaattgtgagtctggaatatgttggtagacttttttgaataagctgttgttactgaagtaaagctaaatgtagcataatcaccccaccacctacgattcagcgaatgtatggtggattgttagaattagattagcaattactcacgggtatcgtttgcatagttattcgctaaattctgagttctcatgtaaaattatgagcaactgactgtatagtaaatacgattttgaaaggctggttctttaagccattaagcgaatttatagtaataaatatttacaaggagaaattgtgggttgaacttagtgaacatttgaactattttaagataagcatcaataattatattttaggaaggatatgttaacgaatgacgaaacattactcgtttttaaataattttaaatttaaaaatggacttgaaatcaaaaatcgagttgttattccaccgatgaccgaagtctccagttttgaggacggttcaatctctacagatgaattgagatacttgcaaatgcgtgctggaggcgtagggttatttatttctcctgtggccaacgtatcagaaaatggtaagggattcgagggagagttatcgataacaagtgatcgctttatcccgggccttgcaaaagttgcttctgcgatgaaatttaatggatcaaaagctatacttcaaatttttcatgctggtagaatgtctaattctaaagtacttcgtggtgttcagccagtgagtgcaagcgctgttgctgccgaacgccccaatgctgaaactcctagagaattatcaaatgaagaaatcgagggcatcatcaatgattttggtgaagcaacccggcgtgctattgaagctggttttgatggtattgaattgcatggggctaatacgtacttactgcaacagttcttctccccacattctaatcgtcgtacggataattggggtggttccttggagaagcgaatgaactttccacttgcagttatcaaaagggttcatgaagccgtcgttaagtatgccaaccatccatttgttgtgggatatcgaatttccccagaagaaattgaaaatccaggaattcgaatgagtgataccttgaagtttgttaacgttttggcagatcaaccaattgattatcttcatgtttcaatgggttatgcgtggagaacttcattgaataataaggaggacactcaaccactgattttgaaaattaaagaccaactgaatggtcgattaccattaatctgtgttggatcagttgaaacaccagatgaagcagctgaagtgactgataaaggtattgatatggttgccattggaagggaaattttacgtgaaccgaagtgggttcaaaaagttgaaacggatgatgaagatagtattcgttataccatttccgaacaggacttagacgacttaggaattacacctccaatgtggaacttcttaattttcaggcttaaatcagcaatgcacatttctaatcagcctgattatgatccggaacaatttaaaaataaacttgcaccccacgaaggtgcttaaaagttaccaattatcatattaatttttggagtggcctatcgccactctttttttgtgtttatatcaaccttctcacgattgatttattatgagcatatagcgctttcatagtttccagttaaaattatatacaaaattgatggtaaccgatttctcaatcggattggcagctatattcctttggcaccaaccaataattggctttgaaataatgcttgactaagttttggaaaacgtttaccatagatgttggttagaagtgatagattgaacaatgtgaatcattctaaaatcaattctgacgtcaatacatgttggttgttgctattattctattaattcttggaggaatcgattatgactttaattttgaatacatggatttttgaatcagatgtacaaaaaggtgctaaacaagcggacttggttgatcgggtagcaaaacttggtgccaatggtattgaagttcgtcgtgaatatttcaaagatttggatgttgagcttcctgatgttgcaaaacatgctagagaacataatctcattgttaattacagtgtgcccgatgtaatatttgaaccagatgggtctgttaaccctaaactcgccgattattttgaagaaggcgaaacgatggggatttcaaagattaagtttaataccggtaactttgataaattcaccggtgatctcaaaacggaattgggtaagtttccaattgacaagattgagatgaatgtagaaaacgatcaaactccagtttcaggtactgtaaatgcaatcaaaacatttttggatgctgcttatgctgccggattaacgcagttgggatacgtatatgatttgggtaactgggcgtttactcatggtgatgctaccgaagcagcaaagacactggctccatatacacactacattcacttgaagaatgctatcgataacaatggtaagctcaccacttcagatgacttggataaagggatgtttgactggcgacaattattaaccttgttaccttctaacgttcagtttgctttggaatatccaatgacctcagatgctcaaatttccgatcaaattaagttgtttaataaagaagtaggtgaatagcgctatgacatcaacaataatttcaattctacttttagtcacgtttgcagcctttattgtatacattgttaaaggcggtaacttgatgatcgggttcttcgtaatggccatattatggtcagtaattggattagttccattcaatacagctattcaaaaggtttttgctgagcctgcattaaattatgggccgaccattatttacattgtgtttggttcatggtttggtcgtgtgttggtggatagtggaattgcacctgcaatttcagagcaaactaataaagttggtaagaagaaacccttaattgctgcaatcttggttgtttttgtaacatcctttatctttgttagtgcttacggtgttggatcggttattgcaattggtgttattcttcttccaattctgttgtcagtcggattgccacgagatcttgccctatcagcttttgcacttgcaattggggcaccaatgtacattaacgtggttttgtttaaccaaattaaagcctttttcccaaaagcaatttatggtgggaaatacttacaatttgggatggttgctactgcagttcaaattatcgcagttgttattttcttaattattcatcgcaaacggattgacgcttctaaagccgaagaaaaccttcaaatcattggtgctgctggtgccgatgagaaacaaattgaaagtgttccgaagatcgcctatgttgtaccgattattccagttttaatgaatatgctattccactgggacgcaatcccggcattaactttagcaaccttaattgccattgtattgactggtcgagcaaagaactttaagaagtttgttgattttctgaatagcactattaagcaatcaattagtgatattgctggattaattatgtttttaatggctttgattatgttttcaggagccgcatcaattaatgcgccacgttttaagccaatttttgaggcgattttaccgaatagtcatttaactttagctattatgcttggtgtacttgcaccacttgcacttttccgtgggccattgcatgtatggggtgccggagccgcaaccgctgctgttctgtcaggaaccggattgtttagtgatgcattcttgctaccattactgtatgtaccgactctgatggctgtttcaactgatattactcaatcatggaacgtttggggactcgattacatgaaggttgattccaagagcttcttgaagttgggaatacctgtaatgtgggccgtatcaataattaatgagttgttagtttactacttctttggttaagacgttgttgaaacttagtaataaaagaaatgaggaattcaaatgagtgaagttattacagttggagaaccattatgcacatttgcttcaaaggaccctgatgtatcccttgctgatgctatgaattggcataaaatcatgggtggtgcagaattgaacgttgctattggtgttaaacgcttgggacattcggttgaatatatttctcgagtaggagaggatccttttggtgaatttgtcatcaaaacaattaaaagtcacaatgttggaactaagtatgtttctcaagatccggtatattggactggccatcaactgaaacaattggttactaaaggtgatcctgatacctataattatcgtaaggggtcagctgcatctcacttaaccagcgaaatcatggatcaagttgatctgaatggagttaaaattgctcacatgtccggaatttttccggctatctcagatactgctgaaaaatcattccgttcgttactctcaagacttgttgacaacaatattttaactacgtttgatcctaacttgcgtccctcattatggagtagtcaagagaaaatgattagtacaatcaatgaattggctggttcagcgaacattgttttgcctggtttggctgaaggtaagattttgatgggatcagatgatcctgaagaaattgctgatttctatttgaagggcaaacgaacagatactgtgtgtgttaaaattggtcctgctggcgcctatgttaagaccaaagatgggcaaagttacactgtgaatggtttcaaagtcgataatgttgttgacactgttggtgccggcgatggctttgcacttggtgttattacagctttacttgaaggaaaatctttaaagtcagctgtcttgagaggaaatgctgttggcgcattgcaagtgcaaacacctggagataacgacgggtacccaacacctaaagagttaaaagagttttacttacaagaaggagttagcgaagattaatgaaattacaagcagcgattgatagagtgtctcttggggacgcggttaccctagctcatagactggatggtattgccgatgtgatcgagtttggcacttctctggtgaaggattatggtcttgtgatgatcaaagaaaatcctttgcatttgaagaagagtaagcttctgcttgacttgaagactattgatgaaggcccatatgagttcaggagaggtttcgaagcacatggtgatattttaactgtgatggctggttcatcatatgacacgattagtaaaacttacgatatcacccaagatgttcataaggaaatgttaatcgacttgcttgaagtggacactgccaagattaaaactatttctggttttaagaacgcaatttatggattgcatcattcaagagatgcagaaagtaattttgacgcaattagtgctactaagaagtttcatgaagatttcccggatatcaagcgaattgctgttgctggtgggattgatgtggaacaggcaaaaggtttgtctcagcagggcattgctgacactgtgattgttgggagtaagatagttggtgaagaagatcctgtaaaagcagccaaacaatttaaggaggcaatgaagaaataatggcattaattgagcaagttatgcatgaagttgatgaagtcatgtcactggttgatgaaagtcaaattgatgacgccgagaaagtgattcaaaaagaccagagaattttcgtcttaggtgccggtcgttctggattgatggctaaaggatttgcaatgagattgatgcacattggctacaccgtttttgtcattggtgaaactattactccatcaattcaagctggagatgtgctggtttctgtttctggatccggaaagacaggcatggttgttgaacctacagaaaaggcaaagactaatggtgtcaaagttgttgctatcactagtaattcagagtccccattggctaaactgggtgatgcagttatcgtagttccaggagctactaaagccggagacggcgttcaatctattcaactattgagtacgttatttgatcaaagtgttcatattacattagatgttttgtgtttgaaactaagtcggcgtgaccacatttctaatgaaacggctaaagcgacacatagtaatatggaataggaggaagccagatgttacaaaaggttgaagcgattaccaaagttgcaaattcaggggttgtcgcagttgttcgtggacaatccaaagaagaatcgttaaagacggctattgcgtgtatcgagggtggtataagtggtattgagctggcttttacggctccacatgcagacgaaaccattgccgagcttaactcaaggtatactgaggacgaggcatttgtgggtgcggggacagttttagaccccgcaactgcaagagttgctatcattgcgggtgctaaatttattgtgagcccatccttcaataaggacgttgcaatgttatgcaatttgtatgccattccatatatccctggatgcatgactccaacggacattcaagaagcattgtcatatggatcagatattattaagctgttcccaggatcggtagttggtcaaaatatggtctctgaattacacggaccatttccacaagctagtttaatggtaaccggtggggtttctcttgacaatatgcaagagtggtttgataaaggtgcgacagtacttggtgctggaggaaatttggtcggacccgcaaaaacgggtaactttgatcaagttaaaaagaatgcacaagcatatcgtaagcaaattgatataataaagtcttcaaagtagaattgatatcagttgaggccatgacttttatgatgggaatgccattatttagagtctggtctctttttttattatttggtatgctaacaatatgtatttcaaaaataatttacactaatgaaaatgaggaagagagaatgactgataaaggtaagtctaaaacaagtgatacagtaacaatgaaggatgtagcggcacttgcaaatgtctctatagcaactgtgtcaagatttttaaatggcgatttatctcgtatgtctacaaacacggctaaaacggttaagagcgcaattgataaactaaattatgttcctaattctgcagctcgacaaatggttaccaagtcgagtggtttgattgcaataattgtggccaatattgacgactttttttctaccgaattgttcaagggaattagtgccatgttggaaagcaagggatatgtgggagtcctttttgattctaattcggacgttacgcgagaaaaagaactgatgacaattgttagtacccatacttttgatggcctaattattcaaccgtttagttctgtgaaggttatttctgacacgattcgtagaaatatacctattgtcattgttgatcgagaaattgaacaatccccttggacgcaagtcgtaacaaataattatgaagcagcaaggaacgcagctaagtactttcgtaatgaaggatttactcatgcaattgttgtaacatcgaatttgaatcttgccacaaacaggcgagaacgttatcgcggaattctgtcagaaattgataatacgaccctggttgaggtatctgaatcatcctacaaccataaaaaagtttctcaattacttgagaagttgttgaaagattctaaagagaaaacacttatttttgcacttaaggaacggtggataactgaatttgttcctagtctattttataaaggttatattgataataagagagttgccataactggatttgcagacactagtttagctaagtacattgatccgcatacaaaactaatcgctcagaacccgtatcttatgggtgccagcgctgcggaagttatgacagataagctgacgaatatgaatgtaagaattgacaatacaatcgttgttccagcaaaatttgaataggtttaacaacctagagcatgctggaagtactgtagcgcatccaattagtagactgaactaattggatgccgtttttatattcgggggcgattaattataatcttatgtgaacggtcataaatatcaatagaatgcaagattacagcaacagcagttgttaatcatagaaatgaatagaaaattaatgttgacacagaatcatctgaagcatagtatgaaagatacattaaagattaattaaaaaatgctaatgaaaggggatgcgctcgaatgactgttgaatctattattattttaattattagcgtcttagtaatctggatcaaacagtcgtttgatgaatcgtgctaaggctttttggcctttcatgaagagcaaattctcctgcgactgggtaatttaacctagtcgctttttatttatatttttttgttaatcaggagaggatgattttatgagaaaagtatttacatatggattagtggttaccagtgcaattttattgtcagcttgttcatctaaaggatccactagcaataagcaaaaaacactgaatgtaacgatgattcaagaaccttcaacagcagatccaaataaaggaacagatgtttactctgcgagtctggttcatcaaacgctcgagggcctttatgatgtgactaatacagggaaagttgttccgggtgttgctaccaaggtggtcaagcctactaaccatgggaagatgtatacttttacgcttaagaaaaatgcaaagtggcagaatggcaaaccagttactgctgaagattttgtaacatcatttgataggcaagtggatccaaagaccaaatctcagtatgcaagcaggtttcaagctttcaaaaattttgctgatgttcaaaaagggtccaagaagccgacggcactgggagtaaaggctttgggtcaacgcaagctcagagtcactttaaccacaccagatcctgaatttaatttccgggcagctactgagtattatcctttgaatacagcagctgttaaaaaatatggtcaacagtatggcacaagttccgtgaaaacattgtcgaatggcgcgttttcattacaaggatgggacccatcaaaggatgcttggacttacaaaaaaacaagtatttctgggatgcaaagagtgtgaagttacctaaagttcatgtacaagttgtgaaggaaccttcaacagctcaaaatttatttgctagtggaaaaattcaagaaactctaattactggagagtttgtcaaacaagacgccaaacgttatccaaaaaatattgtttacactaaaaaagggcaaatgagatttttgagttttagtgcaaaaaataaaacaacgagtaaccggaattttagacttgctgtaagttacgccttaaaccgaaagcaactgactgataatgttttgcaggatggatctacccccgcaaagtcaatggtgcccgaaggtgatggaactgatccaacaaatggtaaggactttaacaaagaattagcaaccaatttgaagtacgataaacagctggcccagtcatattggaagaaagctcagcaacagttaggaaagaaaacactttctgttcaacttctcacagaagatgatagtgaccagaagaagcttggagaatacgttcaaagtgctgttgaaaagaccttgaaaggcgttacggttgaacttacatcagtgcctcaacaacaacaacttaccagaatgtttggggggaattatcaaattactgcaacaggatggagcaccgactatccagatccttctgattacttaaaccttatgaccaaggcaaatactgttaactttacacattggacaaatgcttcatatgaaaatgtgatggctaaagtaaacgatacttctaagtactcaggtaaagaacgctggaacttgatggtaaaggctggaaacatcgcaatgcagcaacaaccagatgttgcaacatatcaagatacagatgttcatctggtttcgtcaaaagtaggagggctcaaatattcattactaacagactcattgtatcgttacgcttattggaaatagggaggataaaatatgtcacaaatgttgacggaagaagatttctataaattaaaaatgctgagtcagccagttgagactgacaactattactttgtcactcaaacttatatggataagcagtctaacgggtatcgttcaaacatattgggatttgacaaaggaggtaaatttgttggtaactttgataatgataattatgcttcgaagtcaccagttggtgcaaaagactacctgttttttctttcacaaagcaatgctgattcagagtttcaattatttcaagttaaatatacaggtggaacagcccaacaagttacgcatcttgcacattctgttgagcaagtaattgctgtacccggaacaaatacggtattctttaaaacgagggagactaaggaggttccgaagaagccttatgaaaagtatccaagtgttagacatgttttccgggtgaatcacaaggctgacgggttcggattctatccaactgatggtttatacgttttgtactcttataatacggacgaccaacgtcttgaaaaggtgtattctgccaagcaggattttagtttaactgatgttgcatccgacggtgttcgtgtagcagtgataacagataataaacctgataatgatttggattatgggcgtggtgtttatgtgcttgatacatctaaccagcatgttgacaatatcacagcaaataatccagaatgggtgtttacccatgcaaagttctccccggatggatctaaaatgcttctggtgggtcgatctgataagtatgatgcaaatacacaattttctgtttatggttatgactttaacaatcagaaatttctcgattatgttaatgagatggaagaagagaccgctgatttcttgtttacagacttcacacagaatcttagcgacgaagacgctttttgggttaataatggtgcctttgtgtttagaactgcttatcatggcagaacaaagatgtttctttttcaaaatgggaaagtaagctcattctataatgaggctgagagaatcacagactggtcagttttcaataaccatttgattgtaacgtattcaactggaatattaccagtaatgatggcgacattaagcttagatggataccaagctgatgtatttaatcctaatgagcgttttgatcaagagcatgagtatgtgaagccggaaagatttgtctacaaagctagcgatggtcttgcaattgaaggatggttaatggaacctgccaagcctaaagaatccaatcctttggtactttatattcacggcgggccgcactacgcttatggagaaaatttcttcttcgagatgcaggtgcacgcagcgaatggatatggaattctcttattaaatccaaggggtagcaaaacctatgggcaagcgttttgtcaggaaaatgttggtcattatggcgagaaagattttaccgatttaatggaaggaatggactacgtgttagctcatcacccagaatttgataaaaatctacagtattgtgcaggtggctcatatggtggatttatgacaacttgggtggttggacataccaataggtttgctggtgctgttgctcaaaggccggtaactgactggattagcttttctggcacaagcgatattggatttatgtttactcctcaagagcttaaaactgatcgatatgatatagagacactttggaagtattctcccctcgcatatgctaagaaagttaaaacccccacattggtcatgcagggggaatgggatacgagaacacctatcggccaaggcgaggagttcttcagcgccctcgttgagaatggcacggaagcagagatgtcccgatatcctcaatcttggcatggtgtgtcccgaaatggattaccaaatctaagagttgaacgaattaaagaaactagaagctggtgggataagcaccagtaatacattcttcaggtagaagcctttgacttctaccttttttatgaaaagaaaaaaagaccgtcatctttgtgatgacgatccgatggttcttaatttattcgattaaatcaatttcaagaatatcgaagcaatgataacagaagcaactgaaacggttgcaaacccaccaactaacatttttggcatcatgttatgaagtaaatagcgttcctcatccttagttccagcaactgtgtgagcaacttcagacgttagaatgtaatcagctgggaatccaaataacgacgtcagagagcaagcataggccatttgccaggacattccaaatggcttagcaagtacgcgtgaagctaggaacattcctagaagacctaaagcaatcaagacaataatttgaaggataatacttcccatgatctgaggagttgtaacacttaattgtgcaaaaacgtaagcaagtaaaccatacattaaccaattaaatacacctgcttcgttcaaagcattgtcttccaagaaaccgaattggtgagcaataacaccaaagatcagacaaacaacgtttgggttaatagcattgttgattaagcctgcacaccatgtactaaagagcgctaccatggctacacgagccaaagtaaaagctggtgtttcatattctggtttcaaattaaaaacgttttgtgatttgaatgctgaaggctgttcatcttcggcaagttcagtcacctcaggtcctaatttacttccgccggccttaaattctttgattaaccggccaccctcttgacggagcattaatgaagttagaggatatccaaccactgagtgaataacaaacatggaaactggaagagctaccagagctgtaaccccttgagccttcaatccattggtcattagcaatgcagaaaccaaaccaccggtgagtggtggaactgcagcaacaaccgtcttccaattaaagatcaaactcccaattgttaaacataaaagcattgttccacagacacctaataaagcaatacaaacagctttccattgggcaaccaactcttttaagctcatcaaagtaccaagatgaaccaacaacatggcaacacagattgacacaaattcattgccatacgacgcttgagttacaacgtccttgggtaaaatagtccaaaaaccaatcacgaataatacagcggagacaaagactgaaggaataaaagcatgagacattgttgaaacccattcaccaatgaacatgaataccattacaacaagaaatgcgatgataaagttcatatgtataccactcctaacaaatttattgatatatgtatcctattactcattgaattgttagtcaattctaattttaatgaaagctttataaatgccgaaggacaagggctcaattgaatccgctttaaaatgggtggttgactattattcaaatgagaattaatgttatattaattagaaaaaggagtggatatatttgagcaaaactacatatacaaatttcaatttgttcgatgggaaaagtaacgaagttaagaaatccgcatggttggttgttgatgagaccacagggaagattgaccaggttggaacaggtgatgctccttccaccgatcagcaggtagacctaaatgggaaatatgtcatgccaggaatggtcaattgtcatacacatatctgcatggatcccacagcaggagatggtggaacaggtgctaatgtagttgatgcaactgttcatgccgttcaacatttgcatgacctgttgaagtctggtgttacttatattcgtgaatgtggtagtacttttgatattgatattgctttaaacgagttacgtaaaaagggtgttttgaaaaaagtacccgagatcttgccttcgggaagaccatactcaatgactggtggtcatggagactttccaaactttggtcatttagttgattctcctgatgaaatgcgcaaggctgttcggacaggacttaagaaaggcacaatggctgttaaggttatggcaactggtggtgttatgacacctggtgacttcatggcggatccacagctgagtgttgaagaaatgaaagttgctgcagatgaggcccatcacaagggtcggattattgctgcccatgctgaaggaaaccccggcatcatgaatgcaataaaagctggtgttgactcaattgaacatggtttctatgtaaatgatgaagaaattgatttgatgcttaagcaaggtacttatttgaccccaacgtttgtcgccgactgggcaattcctgaatatggtgaaggaaagatgccagattgggaaattaagaaggctgctgatgccttggatgatttgtataagaacatcatgcatgcatggaagcgtggtgttccgattacacttggaacagacgcaggaacgccattcaatgatttcacaatgactccggttgaattccaattaatggttgaacaaggtgctactaattttgattcacttgaaacaagctacacctcagccaaattaatgaagatcgataaagaatatggaacccttgagcctaacaaatatgctgacttcttggtattggataatgatccattagccgatgtgaaggcggttcaacaagaagacaaagctgtttacaagaaaggtgttcaggtttactaatactaaaaagatggctcttgccatctttttgtgattaaggagaataatatgtcgacaatttattacaatgcaagcatctttgatggaaaaaatgaagagataacaagggatgcctggtttgaagtcaccgatggaagaattgctcaaataggtactggaaagccatctaagaaggctgagaagaatattgatttaaaaggtaaatatgtcaccccaggattaatcaatgcccacacgcatatgatgatgaatccagtcactaataagcttgaatacctttcagaaactgaagtcaccgcgacggcaattcaaaatctaagagacttattggaatctggagtcacttatattcgggactgtggctgtgcttttaacaccgatatcaagcttcgtaactttgccaaagaacatgaccttgaagctcccggaattattgcatctggccgaccaatgtcaatgacgggtgggcatggagactttaaagaaggcgctgatggtgaaattgactggtcgtatttgacagactcacctgatgaaatgcgaaagtcagtcagaactgcacttaagattggcgcagacaatattaaagtgatggcaactggaggcgttatgtctgctggagacaacattgacgacactgcgctcactcctgctgaaatgagggttgcggttgaagaagctcatcacaagggtaaaaaagttgctgcacatgctcaggggaatagtggtatccaaaatgcactcgatgcaggtgtggattccattgaacatggtatttatgttgatgaaaagcaagcggattacatggttaaaaacaatgtatatcttgttccaacattgaacgctgctgcaagtatcagcaaatatggacgtgacaaacttccatcgtatatgattcgaaaaaacgatcaggttaaatccgactttttcaagaatgtttccatggcatttaagaaaggtgtcaaagtgatcgtcggaaccgatgcgggaacaccatttaatagtttcaagacaggtacttgggaagaaatgcaattattggtgaacgaaattggtgcaaccccaactcaggctttattaagtgcgactcagtatgcagctgatttgattggaatctcagacaattatggcactttagagccaggaaaatttgcagactttttggttcttgatcaagatccaactcagagcattgatgcaattacacaggataataaattggtatttcagcacggaaagcaaattaaataggcggtgattgaatgcaacaagaagaagttgaacaatatgctttagacaatttagacaatgtaacggactatttacgaatcccaagtatatctgcacaaaacaaggggattaacgaaaccaatgagtggattatgaaacagtttaaggacttgggagctgccaaagttgaaaagtggactgatcaaggtggcaatcctgttgttttcgctgaatttaacgggaaatctgataagactgtcttgttttacaaccattatgatgttcagccacctgagccacttgatgaatggaaaacgaaaccatttgagccgacagttgttggagacaaactagttgcccgtggagtttgtgatgataagggtgaattaatgtcacggttaacggtggttaagtacttcaacgaacatggtggtattccggtgaacttgaagttttttgttgaaggcgaagaagaaattggtagttcagatgttgataaatatgtgcgagcccacgcagaccaacttcaagctgatgtttgtatctgggaaggcgggggaaaagacgaaagtgaaaacttccagattgtctgtggcgcaaaggggattgccagttttaatttacatgttaaaactgctgcagcagaccttcattcatcgttagccagttatgctgataacgcggcttggcgactcgttcaggcattggcctcacttcgaacaccggataatcgggttgctgttgatggattttatgatgatatagaaaaactgaccccatctgaggaaaaggctactcaaagtatggcctttgatgccgataaggtccgtgctaactacgggttaactcgtccctttgtgtataatgatcctcgcgaagagctggttaatggtgctacgatgaccatcaatgggctgaacgctggttatacaggagatggcgtcaaaacgatcattccaaaggaagcctccgcaaaacttgactgtcgacttgctccaaatcaagatccgcaaaagatcgcaggcttaattagtaagcaactggaaaagaatggatatggtgatgttaagcttgactatttattaggtgaagacgcattccgaagcaatttggatcatccatttgttaaactaaataagaaagtcgcagatgaagtttatacttctgaaaaagttcgcttaatccctaatatgcccggtgggggtccaatgaaacaatttgcagacagtgttcatgcaccaattgtgatggtcggcatccactactccggcagtcatccgcactccccaaatgaaaatattcgtttggctgattataagcagggaacttactttttggcacggctgttagaagaatattgatttgaattggcatttgacaaatgtagtttgatgagtaaactagtaagtattctaattgatgtatcatttaaaactcattttacatcagtcggatttaatgtactgttacttgccaaccgttctcagctgggacaaaaaggaatttcaggtacatctaacaagttaattgaaatgtgaaaaatatttttgaaatgatgatgagaagagtaattaacaatttgatttctcagagaacgtcggatgctgaaaagacgtaattggattgctaatgaagatgagctcggagtttaaatacgtgaaagcgatatttacgtttggatgcgttacaatcccagacttaatagcattatttgttattgagttggtaagatgactactgtgaagtagtcataaacgaaggtggcatcacgtattcatacgtccttgtggtatttattactgcaaggacttttattttgcatatttttatatttgaaagagggaaaaattattatgaaaaaatcaattaagtatttaatctgggttgtcgttgttatagcgatcgttgtcattggctacttcagttttggccgtggtaatgcctcacagtctaagaccgttactattggtgtaattacaggaaccaaaaaagatcaagcaatttgggattcggtatctaaaaccgccaaggataagtatcacatcaacatcaaactgaaaaactttacggactattcacagcccaataaagcacttagcagtcataacattgacttgaatgcttttcagagtatgaactttctaattcaatggaatcaagcccataagagtcatttgacttccatcggtaaaacactgattacaccacttcgaatttattccaaaaaatatacgagtgtaaaccaaattaagtcaggatcacaaattgcaattgccaatgatgcagcaaacgaggccagggcactggaacttttgcagtctgctggtttgatcaagcttgattcgtctgccctaccaacggttaattcaattaccagcaatcccaagaagctaagaataaagacggttgatgccaatcaaaccgcccgtgcattaccagatgttggtgcttcagttatcaatggtggcttcgcggtaactgctggtattccagagaaatattcaatcttcaaggaaccattgcagaagcagtatgtcaacgtaatcgttgctaataacaaagataaaaacaaaaagttgtataaagaggttattaaggcctatcaatcggctgcaactaagaaggaaatcacaaaacaatatggcgatttaattttgccagcttgggatttgaaatttagcaagtagtgcaaggagggcaaagatgtcagacagcattattgatattaataaggtgagtgtgagtttcctacagaaaggcaatcgcttagacgccgtgaaagacgtctcattaagcattaaccgtggcgatatatatggaatcgttgggtattctggtgccgggaagtctactttatcaagaacgattaacttacttcagaaaccaaccagtgggacggtcgttgttgataacaaaactttttttgacagcagtaagagtcgcaagccaattattagcgcgaaagaattgcgaattgaacgtcaaaaaattggcatgattttccagcattttaatctgctgaatgaacaaaccgttgttcaaaatgttgaatttgctttaaagcacagtaagttaaaagaaaagcaagttcagcaacgggcacaaaagctactgggattggttggattaagcgaatatgcgaacacctacccagctcagctgtcagggggacaacagcaacgagtggcaattgctcgtgccctggccaatgatccgaaaatcttgatttctgacgaatcaacttccgcccttgatccacaaaatactaatcaaatattagatttgctaaagcatctcaatttacaacttggacttactgttattttgattacgcatgagattgatgctgtcaaacgaatcgcaaataaagcagctgttatggatgctggccaaattattgagtctggtagtattgttgatgtttttgtccatcctcaaaaacaactgaccaaaacactgattggcttcaacgagggtcccaaaaaggcaattagtattctaaacagcaatggtctaaaactcaattctaatgaacagtacatcaaattgacctattttggcaatgaggtaagtgaaccagttgtgattagcctttataaggatctcgatgtcacagcaaatatcatttatagcgacgttgatatcttgggggatacactggttggaacaatgtttatcattattgaaggtaagtcggaaaatgtcgaagaagcaatagactatcttcggcaaagagatattagtatagagaagttggatcgaagcgaggtgaatagctgatgagtacgtggtttgcaaaaacgtttcctaatgttgtttatcaaggctggaatggaagtgatggctggtttaccgctattattcagacgctttatatgacattttggcccgcaatttttggtggcgtcctgggaattatctttggcttaggactcgtcttaacagaagatggcgggattttggaaaataaggtcgcttttaatgtttttgataaggtcgtctcattcctcagggcgttcccatttattattttgctagcatttatcgcgccagtaacccaaaaaattgttggcacccaaattggcacaacagcgtcactggttccgctgtccattggtgtatttccattttatgcccgtcaggttcaggttgccttgaagagtgtggataagggtgtcattgaagctgcagaatctgttggggcaactttgccggatattatctttgacgtgtatttgcgagaagctcgatcagaaatggtacgaatcagtactgtaacgttgattagtttaattggattaactgcaatggccggcgcaatcggagcaggcggcttaggaaatatggctatttcctttgggtataatcgatttgccaatgacacgacttttgttgcgacgctgctagtcatgattttggttcttttagtgcaattcacgggagactttttagcgcgaatcctaaatcataaacagtaagttaaatacaatgcggaggtaaaaaattatcatggaaaaagaagagcagttacagattctcaaagatttgattcaaattaagtcagtcaatagtaatgaggtggaagttgctgagtatattgggaaactatttcagaaacaccatattagttacaagattgacaaatttggagaagatcgtgccaatttggttgcggagattggctctggtaaaatggatgaagtattgggatttaccgggcatcaagatacagtaagtgtggaagaccccagtgcgtggaaacatgatccattcaaggctgagatagatggcgataaactatttggtcgtggtgctgcagacatgaaaagtggcttggctgctcaggtcattacattgatcgatcttgttgacgaaggcatcgaaattgacggcaagattcgatttattgccactgcaggagaagaatatggaacccccggcgctaatcggttaaatgaacagggagtggcaaatgatttgtctgccctagttgttggggagccaactaacggtcaggtgatctatgcacattctggcagtttgaactaccaaattaagagtattggaaaagcagttcacagttcaagacctgctgagggtattaatgcgataacaggtttatctaaatatattgatgccgaggcaacattatttaatgatgctcccaaagacaagatcttgggccaattgcagcatagcattaccctgatcaaaggtggagaacaagttaatatcatccctgactatgctgagttgtatggaaatattcggccaacggaaagctttgataatgaccaggtaattagcacaattaagaatgaagttgctaagattaataaagataccgagtttcacttggaatttcatttggttcacaatttcaggccagttgaaactgaaccagataatccgtttattacccttgttgatcaggccgctaaggataactaccaagatcgtgatgttgaactgcaaacaattaatgccgcaacggacgctagcgtctttatcacaagtaatcctaagttgccggtcgtaattttgggcgcggatgaaagtggtgttgctcatcagaccgatgaatatacaactctgacaagttactacgaaacggttgaaacttatgagtcgatcgcaaaaacatactttaaacagtaatgcagattactataagacaagtaaatgtgtgtagataattttttcaagacaacaagagcagatcaatgtgctgatgaacattgatctgttcttgcttttgtctgttcaccaatggggggattcctcctggtaaagattggattaagtcattcaaaataccccatatacgttgtatgagcctctatcatatctgagttcactaaagttaaaatttattggcataacaatcctttttcccaataaattttccgacatatgtataacctatactcccaagaagataaagattcaatcaaacattatctattaactcacacgaaataaagaaagcgctttcgtataatagatattgaagcttatttcacaatgcattatatgaaggagtgaacataatggacgacaatgtaacgactgttggtgcaaaatcaaaggctaacgatcctgttaatgtctcaaggagatactggtggcgggttgtggcactgtgctttgttggttggattctaatttatgccgacagaacaattcttaatccggttcaggagcaaattggtgctcagttccatatcggtaacacgcaacttggattggttaatagtattttcttcttaacctatgcgatttgccaaattccatttggagttttgggggataagatcggccgccggttagttattatgggtggttttgttctacttggggttatgacatttttcagtgggtttgcattttcttttgggatttttctagtattcagagcccttgcaggtgcaagccaaggaacatattatggaccacaatatgctctgtcaacggaagctatccccaccaaggatttaactttaggaactgcaattattaatagtgggatggcctttggaacctccgggggttatcttctttcgagttatatggtccttcaaaaggggatgtcatggaccagtccgttctgggtaatggcactaccgaccatcattgtcggtattctcttttatgttatcttaaaagaaaaggtaatccggccagaagatcagaaaaatgagcaaaaaactgaagaagcggttgaggctgaaaaagagaaggtaacgctaaaggacttatttaaaaatcgtaacttggtactggcatttattctctgcttctgttcgatttatgctaattttgtaattttgacttggttgccacaattcttgcaggttgaacgaggatttcaaggtagtagtgtaggattcatttcctcacttgttccatgggcctctattcctggtgcccttctctttgccagaatttatgataagttgaagaagaccaaaatgatgattggattcttagttcctatttcattgattgctgtgtttggaattgcgtttgtcaccaataaatcattgctaatcgtgttactaattgtgtatggattaactggtaaactagccattgatccgatcctgatcgcttttgtaactaagaattcaccacgtggttcgctgtcaactgcgcttagcgcctacaactttattggcatgtcaggttcaatccttgcaccttatctaactggttggatttcagaccagtttgggtcgatgcagattggtttctacctagcagctgtccttctgctggttggtgttatcctatttacattcaccagtgacaagaaaaatgcgatccatgcttaactgaatacaaaatgaatcccggtgattgttagatcactgggatttttattttatcttgttagattatttagccattcaattacgcctttataaattgttaaggattcaggtgtgactgttcgatcgaaatcatgatcttttgaagtgacggggatcagcttagcgtctggcagtttagcttttaacataattgagttaatgaaggggacgtcaggatcggaattggattggcacatgtaagtaggcggaaattgtgttttaagtgtgtttggactaatttttagttctgtctcattcctcttaaagatcatttcctgccaatttgcggtttgacgggcgtaaacataaattaaaaagcgctcttcataagaactgtgactgatgggggaattgttcactaattgttttacttcagctttgtttacggttggataacttgaatatagtgcattgggctttagtaaatttgatgctaaaagactttcgaacccataaaaatcgatgaatgcctctggaaattctggcaacccaccagccattagttgcatggaaagataagcaccagcggatctgccaaataaaacataatgattatttggcagattaaggtcgtcaaaatgattgagaaaatacttcacaccagctctcaaagattcaatgattgcagagaatggactttctggtgctaggagataatccaatgtaaataccgagtatccagattttagaaaaagatcaatatatgcttgcggcaggtcatcccggttgccgaaaattaacccgccaccatgaatatatataatcgtgggcttgtctgaattttctggtgttttccaaaaagatccctgaatttgggttctatcggttgtcttatacgttacagtttgcaattttatctatcccttctaattattttcttcatccaaaacattaagcactcggataccaacatttaatctaaaaatttcatcgacatcagagaagttaatgttggttcgttcttgaattttgtttaatcgataactcatcgttttggggtgaatgaataaggcgtcggcacttgccttggcgttttgattatgatccagatacgtttttaaagttgtatatagttctggcttatcttgatagagtttcaataagtcttccgttacaaacgactttaacttggttggatcatcgacttggaataagaagcggtagaaacccaggtcattataattaaagatttgatcggacttgttcaagtggccggcgatttggagtgtctttaaggcttgtgatgcatgacttggaaaatcctttgggtgacaattctcgcttaagccaatttggaagttcattgacgggtgagaggcatccaatgtctgaagaactttcctcaagttagattgcaacttagcggttggctcgtcatcgataattaaaatgattcgattttgtcgaacacggtacacagcatcaggccaaaacgtcttaaattgtgcaacgacgctatttgcatcacggggattatctcgaaaatagtcagtttgaatttcaccatttaccaagacttggattactgtgactcggtaatccttatcttccatgagtttgaaatgtttcaaagtggcttgatattcttcctcacttgtaattttgccattaatcaagtcatcaataatatcattggcgtaagttctaagtccctgctccagggccgcttgcttgataacttccatttgcgtaaagtttacagcgttctcaatagccataaaatcaatgtcttggagtctcttttcctgcagtactcctaaataaagatcatcttgactattggcaattttaaccattaaaaatttatacccctccgggagacttacttcaaaatattgatagttggtatattcagtttttggaagaagcttccgacttgaaaaatcaatggattggataggatattgagcctgcttactatggacgatatcaacaccgttactgtcctcaatcttaaaaatataagtaggattttcaaccaaagttgagagaagggtaacgatcgattgataagaactattttgaatagctaatttgatgaattgttgattaattgttttgtagcggttcaacatccggtttcgttcattgaataatagctgcatggtctccagcataatatcactgtacttaacgtcttgtgggatttcaattaatgggatgtcaaactggttgctatcttcgataatttgttggggaatgtcgttgataaatctcgatgttttgacgatcaagccactacaattgtgcttgtttagagattgcataaaatcatgaattgaatccgttgacaacttatcgaatccatatagagaagaaagtagaacttcatttggtgtgatccagcgttcaacgtcaggagcttcagtgatcatgatattgtcgactgttttattgatacctgcatttccagcgaccaatttggcgctggtaagggaatctatttgttggatatctttcagagtaactgccatatattttcctccttttaaaacgtttaccaacataaacaatactactacatagataaaaatcaattgaaagaaagtgatttctattatctgcgtaggatataataacgcttacaaagttatctttgtgagtaaatgtattatccttctcagaccagtatgataagagcgtaagttaaattgctaagcggcaaaggaggaaaacgatttgctatatacagtaattagaaaaaatagttatcaggattcaattaatctgatgctattaacacaaaatattagttccatgcctggtgttaaagaagtccaggtgatgatgggaacagacgccaataaagatatctttaatgaagctggattgttgacagacgaggctaagcacgcggaaccaaacgatatgatgattgtccttgatgctgacaaaaaagatgttatggatgatgtcttaaaacagattgataaattcttaagtgacctatcagttaaaagtgacgatgaagcaactgattcgaagaccgttacgaactgggatgatgcgatgaaagctgttccagatgccaacttggccgtgatttccgtcccaggtatttatgctgctgacgaaattgataatgctttggaccacaatctgaatgcgtttgttttcagtgataacgtttcgctatcagacgaggcacgcttaaaacagaaggctcataaaaagggactattggtaatgggtcctgactgtggaactggcattgtcagcaatgttcctttggcatttaccaatgttgttcgttccggtaatattggcttggttggtgcatctggaactggtattcaagaagttaccagcatgattgaacgtttgggtggcggagttacccatgcgattggaacaggtggtcgcgacttatccgataaagttggtgccattacgatggaagacgctattgcaggattagctcatcacgatcctacagaagtgattggtattatttctaagccgcctgcaaaagaggttcgtgacgatgttgtcagtttactgcatagtattgacaaaccagttgttgccatcttcttaggtgaaaagcctgatcatcacgaagattcagtttatctggcacacactctggaagaaacctccagaattctgatggatttggcagaagataaaaaagttaaagacaattattatcctgcagagccactggttaaagccgatcctcaactggatggtaagcatatcatcggattgtattctggcggtacgttggcttatgaggccggcatgatggtttctgaagcactcaatcttggtggcattatctctgatgaaggttatgttctccgtgcaaaggggaatgaggtgcttgatctaggtgatgatatctatacccaaggacgtcctcatccaatgattgatccacgaatccgagttgaaaagattaatgaatatgcaaatgattcagacaccggtgttattttactcgacgatgttcttggttacggaactgatgatacaatggcgcgaagtttggctgatgctgtgacaactgcttcaagaaagcatccacgagttaaatttgttgcaacagttgttggtacccgtgaagatcctcaagattatgatgctgctcgaaagacacttcaaagtgccgggattattgttcttgacagtaatgcacaagctgttcgatatgctttgaacctagttggtaaagatgttaatgagccagctaagaaagtaattccatatactggagcaactcatgaagttccaatgccaagtgaatcagtacttgacctgctttacacaaagccacgagttgttaatgttggggttgcagagttcttagacccagtcatcaagtttggtgggactggtgttcaatacaactggaagccgattgctggtggtaaccagaagatgattaagatcatcaagaaagttaaagcacttcaagatcggaatgccgaaaatgcaactattgtagatgcgtataagaaggctgccccattcctagttgatgttgttcctgcaggtactgttatctcagaattgaagggtcacacattgttacacgcaggacctccaattgaatatgatgaaatgaccgaaccaatgcaaggcggttgtatcggagctgttctttttgaaggatgggctgatgacgaaacaggcgctcgtaaattgctggaaagtggcgacgtaaagttcttatgcaaccatgatgtcaacgccgttggtccgatgggcggaattacatcagctcatatggccgttctcgtgattaagaatgccttaaaggacaactatgcatattgcacaatgaatgaaggaattggtaaagtacttcggttcggtgcgtataatgatgaagttattaatagattgaaatggatggcggatgttctggcgcctaccttgagcaaggcactcaagaaaattgatggcggactcaacgttaacgtgatgatggcaaaagctattaccatgggtgatgaattccatcagaggaacattgccgcatcactggtatttttgaaggaagttgctcctttaatcgtttcgctggatattccagaaaaggaaaagcaagatgttatccagttcttggctgacactgatcagttcttcctcagcattatgatggcaactgggaagtccgttgttgatgctgcaaggacctacaaacatggaacagtcgttacaacgatgactcgtaatggaaaagactttggtattcgcatcagtggcttaggcaaccagtggttcacagcacctgttaatacaccaaagggtctattctttactggatttactcaagatgatgccaatccagatattggtgatagtgcaattgctgaaaccgtcggatttggtggtatggctatgattgctgcaccaggtgttacacgatttgttggtgctggtggatttaaggatgctcaacggattagcaacgaaatggctaagattactttggatcgaaaccctaacttcaccattccaacctgggattaccagggaactgcaattggaattgatattgtgaaggttgttgaaacgggtattacaccaattatcaatacagggattgccagcaaggttgccggtgttggtcaagttggtgccgggacagtccatgcaccactagcctgctttgaaaaggcactggttgcgtatgctgatagtatgggactgttggatgacgatgaacaagcagcgattgaaaaagatttagttaaggaataagtgataattatgaaccttaatcataatcaagcaactggagagaagagcaatatgctccctctccatttgtttaataagaatcatggcattgttagtacagtgtttcagcatagttttaatattaagtttcctgaactgttattccacgttggtggcatttcagaatccttatcggccactggaattacaattagtgatgaattagtagatcgattattgaaagatgttgacgttggtaatcgagttctttacaagaatgaacaattattcatatacacaaactcagatattaaaactatttcactctcagacttaacggaagttgatctgcgaattccgcaggtgacttttgatcagactcccttggaacaaattatttctgcatttaaaataatcgactttgctgaggactggggactgagtgataaatattcaccacaaaaagtagttaatatgatccatcaaagccaaacagatactgaacgtgcgaaaacgctgaattttctttatggccgcgggcgaggattaacacccagtggggatgacattatcgttggttgtttgagcatcttagcagcgatgggttacccacaactcacgcaatggcaggaagtcattcataaaagattggaattgggtgggacgactgatgtgtcagaatcgtacattggtgctgcacttgatggatatacttcaaagaagatggttgcgtttttaaaggtcatccaagtgggtgctattgaacaaatagaaccggcaatactaggtatccaagactttggtcatacgtcgggaacagacacattactggggatgtatacagcatttacaatgctctaatatagcatcctggaacaaagacagatattgaataaacacaggaggaatgtaaaatggcaaaaatcgtcgtcgcattgggtggtaacgcaatcctttcaaaggacgcatcggcccaggcacaaatgaaagctgtcaaagaaacggcaaaagaattggttaactttatcaaaaacggtgatcaactcatcattactcatggtaatggaccacaagtaggaaatctgttattgcagcagtcagctgctgatacaccagaaaatcctgcaatgcctctagacacctgtggggcaatgactcaagggagcattgggtactggttccaaaatgcaatgcgtgaggaattactgaatgcagggattgataaggatgtgatggcagtcgtcactcagacgattgttgctgaagatgatcccgcttttcaaaatccttcgaaaccaatcggacctttctacacagaatcagagttagatgacattaaagccattcaccctgaatggcaattaatcgaagatgcaggccgtggatatcgtcgagtggtaccgtcacctaagccattggagattaatgaatatcgtgctatcaaaatgattgttgaagctgggattgtcccgattgtttctggtggtggcggtatcccagttgtcaaaaaaggtaatcagttgattggaactgaagctgtgattgataaagactttagtgcatctaagatcgcacaattgattgatgcagataagctcatcattctcacatctgctggtggagtcttttataactatggtaaacccgacgctgttgagctgaaagaagtaggaattgatgaaattcaaaaacacattgatgccaatgagtttgccaaaggtagtatgatgcctaaagttgaggcggctaccgactttgttcgtaatacaggaaatcatgcagtcattggcgcacttgaagatgttaaacgaattattgccggtgaagaaggaactaccattgttagcgaagatattgctatggttgccaaataatccaaaagataaagatagcgtaaggttcgaatccctcggcaggattcgaaccttttcttgtttacagatttctggataaaaaaatagcccccgaaagaattctcgaggacttcgctgtttatttatatttcactatgttgcttattattgacctgggttgattttgacttagaacgcttttcagggaaccatgcatacatcatctttttgaataaatctgaaccaaagtctaagaagtaaaccccgagtaacatgcatgcagcgagttctactacaaagagtggccaattggtaatagttttgtttaatgaaatttccataaatgttccccaacctaatagccaagctggaattcttgtaaacggtaggattgttccttgaaggatgatggcgataaatgccatgattccgaatactgatgaagtccaaagtaacatgttcatattaggtatttggaagaggttaaaagcaattaggccccatatgatccccattccgaagctaagtgagacgttgattgaggtgtttttctttgatccgtaacctgcatagaatgctgaggtaataaaagcaactggcgccatccaaaattcaagtgaaccggaaagtaacccataaaaaaatgtaaagattccaattccaagtgctgtataaagtgcttctttgctgagtgataagcctgtcttcataacgatagagctcctttcaaaccaacctacataattaagacataacttgctaatctttaagtactttgtgacaagtcaatcatacttgataaagtaaacgtttacattagcccctatggataaaaataaatcgctggattatacctgaagcccaatgtaaccagagaaaaaacgtgtagaatataatttgtaagcgcttaccaataatatgcgcaaataatatggctgctgtgggtaaatgagctgacgaggtgtaattataatggatctattattgaagaatgtgcgtatcaatgatgatgaagagttaatgaatgtcgcaattaagaatggaaagattgaaaagatttcttcctcagcgattgatgaacatgctactaaaacaattgatggtgaaggacatgtgttaattccagggctggttgaatctcatattcatttggacaaagcattgatttctaaccgagttcacaatcagtctggaacgttaaaggaagcaattgctgtcactgcaaaggctaaaccgacgtttacgaaggaagatatttaccagcgtgccaaaaaagccttggagatggaaattgcccatggggtgaccagtatgcgaactcacgcagaattttctccagatactgggtttgatggcttcaagaccattcttcgattaaaagaagaatataaggacatgattgatattcaagttgttgcctttccccaagatggcattttcaagttacccggaatgacagaaatgatggatgaagcaatgcaaatgggtgctgacgttgttggcgggattccttatgttgacccagatcctaaacaacacattgattttatcttccaacttgccaaaaaatacaacaaagatattgattttcatcaagacttctttgatgatgcagataatattaccgttgattatattgcacaaaaaacaattgatgaagggatgcaaggtcgagtttccgttggtcatgaaacagcccttgccgcacttccgcctgatgacttgaaaccaattgttgagttaatgcatgaagctcagattaatgtgatgtctttacctgaaactgatttgcatttagggggcagaactgacacgtacaatgttcgccgatgtgtgacaccgatccgtaagctacgtgatggtggcgtgaacgtttcgctgtccactaataatattaggaaccccttcacacctttcggtaatggggacatcatgcaggttggatttttggcagttcctgtcgctcatcttggtgggttatctgacttgccaaccgtactagacatgttgacttacaatcctgcgaaagcattacggcttagcggatatggactcgctgttggggataatgcagacttggttttacttgatactaagaaaaagaacgatgcggttattgatattcctgaccgactttacgttatcaagaatggtcgggttacggttcaaactgaaaagaaggtttctttgtatcgacgcacagaagatatcctggcaagtcaacgataacatgatattgagtagcagaagagaagttaaacttaaagcaggttctcgtttttatgagattacaaataatttattgacatctcatgtcgcttgggtgtttaatgatgatgttttcaaaactaaatagtggtctggggtgctgatcaaattcggctgagaaatacccatggaacctgaatcagttagtactgacgtaggaagaccgtttagtcaacttgtaatggattttgcctgactaaggaccactcttttttgaggaggtccttttttaatggcttgaattgtcaaattaagtgcaacactacattaaagaatatttcagaaggtgttccccatccaagatatttacgggggcgattattcatttgttcggcgtacgtttgtatttgcttgtcggtaattgaatcaatgtcagttcctttgggtagatactcgcgaagtaggccattggtgttttcattggttccacgttgccaaggagaatgcggatcaggaaagtaaaaggacgtcccgaactcttcagttaggcattgaactttggcaaattccttactcctgtctggggtgatcgtcaacgatctgccaggccataacctcatcaactgacttaaagtattggtaacggcacttgaagttcttttagcagccttgccaatcaggagatagcgagactttcgatcaaccagggttacgacacaggctttaccactctttcccaaaactgtatcgccctcccaatgtccaatctctaagcgattgtcagcttctcgtggtcggtcgtgaatcttgttgggaatgggaattttgccccgcttttcttgataagttttattgtgacgagacttaccatgatgtctcaagtggcgaacggcgctagaactgcccgacttgaatagattatcaaataaacccttcaagatcccacggtagatagttgcggtactgatttgaacggcatgcttttccactgccaagcgattggagatttcttccggcgaccaccggtcctcacaaaaatgttctctgaccacctcaaatacctgcgaaacacttaagagcgatggccttccacaattacgtttgcgttgctggtacttagcttgagcctttgatggtgaataacgaccaccatctgaatttcgcttcaattctcgagaaaccgttgaacaacttttctggatctccttggcgatcgcacacagtgagtttccatggctccgcattaagaatattgtttctcgttcatctatggtaatatgctggtagtggttcatggctagtttcctttcatgattgttctcgcaaacatcattttacaggaatttggccatgagccattctttatttaattagtgttgcacttaaagtgtaaattcaagcttaaaagttaaaagctggactaagtcaaaattgaattaaactttggcttagtccagctttgctatagttattcggccttcgaattcgataggtaatcccttagatgctatacttaaacaagaaaattctttactaaagaggttaagctgaactatttcatcgataatattttgtccaggttaaaggtcattgaaaatgagtgttttgttattttcaaatggctcaacgacggcgtttgtttagtgtattccccacgtacgtaggggtgatcctacatggtaggaaaagtcttagcggcacacgttgtattccccacgtacgtaggggtgatcccagtctggaggactaaacaatgaaaataaccatgtattccccacgtacgtaggggtgatcctagcgataactctgctccaaaccctttggcgttgtattccccacgtacgtaggggtgatcctcaagttctggtttagaactttaggaggtgagcgtattccccacgtacgtaggggtgatccaccagataccggtggcacgatgattcctcacgatggtattccccacgtacgtaggggtgatcccgaacgttttacccgctcggacagctccgtaatgtattccccacgtacgtaggggtgatcctaatctgatttcgctgcccgcctcagtaaccctgtattccccacgtacgtaggggtgatcctaatttccgtgttggacggtatgggataggatggtattccccacgtacgtaggggtgatcctccttcttggtaatctctttgtattgctcaggagtattccccacgtacgtaggggtgatccttcttgaatctgttcatcccgcttggaatctttggtattccccacgtacgtaggggtgatcctcacggtgatagatttaccacgtgattggagctgtaatccccacgcacgtagggatgatccacaattacccccttattacctaccgtacgggggtcaagcatttagtgagcttataaatgaagtccactagtagaaaaggaggcaagtgtactattttacttgtctcctttttgtaaccgcgaaagttcccagggaaagttgatagccaatcctaacaggtggcccatctccggaaaaagctaacaataataatgcctgtgatgtcactcacacactcaaagaaagcgctataatgaaattgaattttatgccataatttgaatcactgtttgcaatcaactcggtagctaagattgtttctcaaagttcaattgaccatccataagtgataataagaaacaatataacccaccactaggaggcccacccaatgccaaccctatcaacaaaagccacaaccctctgggccaaaaagcgcccaaccgaaaacggcaaacaactatggctgccgctcattatccatctaatcgatacccaaaacgtcattaactacctcttcaaccaatggctctccccaaatcaacggagaattctagccggcaatttatccgacgaggatattcataagctgatcaaatttgccggtttcacgcacgatatcggcaaggcgacccctgcttttcaaactaaaccatcgtggggacacgatgatttacttgatgacgagttgatagagaaattaatccggaatggttttccagaactgaacgacattcacctgccatcaagatccgcatcaccccatgcccgggcaggtgaagcaattcttgataaatatgaagtacccgattccattggggccattatcggcggccaccacggtaagcccgaattttctcggcaaaaggatgacattaatgtgcacacatccaactactatcaatgtgaaaaggacccagtcattcaagccaattggatagaagttcaaaaagaattgatggactatgccctagaatcatccggctaccaaactgtcagccagattcccaccatcactcaaccacaagcggtcatcctggaaggcttattaatcatggccgattggttggcttccagtgaatacttgttggatgacgaagagacagttttatttccattaattgaaatcaatcaaacttatgcggacgttgacacaaccaatcggtttcatcaagcaatggccaactggaacttgaacggtgaatggcagccgcaaccagttgacacaaccacggatccgtatgaagcgcggtggggatttcatgcccggccggttcaagcagcgatgacagatgccattgaaaagacaatcgatccggggatggtgattgttgaagccggcatgggtttgggtaaaactgagattgccctgcttgcggcggaacaacttgcttacataaaaggacaggacggcatcttcatgggcttgcctacccaggcgacatctaatgcaatgtttgaccgcgtcagtgattggttgacgacgattgccaaatctcagggagagagctttccaatcaaattaattcatgggaaagcgcaatttaaccgtgattacacaagtttgcccaaggcttccaacgttggcgatccgaatgcggtggtcgttaacagttggttcagtgggaaaaagtcgatcttgacaaaattcaccgtcgggacgattgataacttattatcgatgggattaaagcagaagcatctttttttaaagcatctggggttcagtggtaaagtggtcatcatcgatgaggtgcatgcctatgacgcctacatgaaccagtacctctacaaagcaattacctggttgggcgcctatcacgttcccattgtgattttatcggcaaccttgccaaaagaaaaaagaaatgcgctcttgaaagcgtatttaaagggtaagtacggcattaagtaccagcaaactttccaagcgccagccggttggcaagagcagcaggcttatccgctgctgagcattttagatggcaatcagcttaaacaagttacccattttccgggccagagcagtcagccctcgactaaactccaagtctaccggctgaatttggatgatgctgacctcattcaagccgttctgaaaaagatcagtggtggtgggattgccggtatcgttgtgaacacggtcaaacgagctcaggcactcgccaaacttgttccagaggacgtcaaaatgatgctattccactcggctttcgtcgccactgatcgggaatctcaagaggaagcactccaaaaaacgattggcaagggtgcgacgcggcctgcaaaaatgattgtcattgggactcaagtgttggagcagtcgttggatatcgactttgacgtattgtatacagatattgccccgattgatctgattttacagcgggcagggcggcttcatcggcacaatatccctcggcccaaggcgcttgaatcaccgcaggtttatatcatggggattaatggtccgggcgattatggggatgccaatgagagtatttacccaaagtatttattgatgaaatctgactattttctggaagcaacggtgatgctaccaaatgacatttccaaattagttcagaaagtttatgaccgcacaactgacgctgagattcctcaagagaaaatgccgggaattgcgaacgcccgtgccgagtttgataagcatttggaccaagaaaaaagcaaagccaaggcctttcaaattgcggcgcctcagtatgctggtcatccaacgattcacaagtggctaaagcgcagccagtccggcatcgataccaatgagcagaaggccaatgcggcagtccgtgacatcagagaaacgctggaagtcattttggtacagcacaccagcaaaggtgaccgcttgatagacggtcggcggcttgcggatgttagctcacaaaacattgctcagcaggttattcgcctgccggcagcgactaccttagacattgatgcggcaatcaacactttggagtcactcaccagcacctattatcccgaatggcagcaggatatttggctgaaaggggccttggccctgccattagacacacatttgtccgccaagcttggcgattggaatctgagttactcatcaaagtttggattaagttattcaaaggaggacgatcatggctgataaacggtttaacttaacgaccgatccatggatcaaagtacttgataaaacaactaatcgggagcgaaccgtttctttgattgaattgttcaaaaatgcacaagacttttctcaactatctggagagatgcgctcgcaggatttggcgattttgcgcttcctgctggcaattttaacgaccgtttattctcggtatgatgccaatggtcgtgggtatgactggttagatgttaatcctgacacgatgcaggccgagatgaatgatgatctggaagacagtgaaatcaacgtttacctttatgaaacgtgggctcacttataccggtcaaatcatttcaccaatattgtgactaagtatctgaaacgttacgcggacaagtttgatatgtttggcgaccagccattttaccaagtaactgaaactcagtacaaccgactcgtgcccaagaagaaacaaatttctggcagcgaggggccggggacggttgctgtcaaacagatcaaccggttaatttcagaaagtggcaatacacccagcattttcacaccaaagtccgatgagtttaaaaatgacattcaagtggatgaactggttcgctggttgattatgtatcaaaacttcaccggcgtcactgacaagaccaagattgaaacggccgataagttctcggcgtccgctggctggctgtataagctgaatccggtgtttgccgacggagagacgctttttcaaacgttgatgttgaatctggtattgcgaagtgatgagcatgcatcagtgattcaacaaccagtctgggaatatgacacgattgatgcttatgtaaacgagcgaaaaaagcaggtgcaaccaactaatattgctgccttatacacaacctggtcgcgactgctacacattgactggagtgagcggggccaaccgactattttcagcgccgaactgccaatgtttgacagcgacgaggctttcattgaaccaatgaccacctggcgggaagacaagaagaccggccgctatcgtccagcagttaaaacccttagatctttgggaacggcgatgtggcgcaactttggcgaatatgtgaaggttgatccaagcgattcaggtcatgaggccgggattgttgactggttaagtgatttgagaaatcaagatgacagtgacgaccaaattatcaggggatccttgctaaccttagcatcggttggcttggtcagtgatggcaatgcgacttcgcaagcgccggtggctgaagtctatgacgatatgcatatcaatgccgatgttttgtttgatcccgatgaagaccaagcgctgcactggccgcatcgaattgaagaaatgattcagttgactcaaattattggatcggattattggcactttgcggcggatgttgcgcgaattcgtaacttggaagttcgaccgtttgccaatcaactgagtgctcaattttatgaaggtctcaataagccgtttaaagactggttggcagatttaaccaaccaagacgatcgagatgaaaagagcgaggagtggcggaagttcctgcgcaaatatgtccttgatgcagctggcaatgtcatgcaaaccagttcgtccagagatattggcggctttatggatgtcagcggcattattgacaagaacaagggcctcgtgaatattttcaccgtcaataatcgactgaaatatcgagttcaggttcatatgaatcagaattaaacaatggaaggtggtcattaatcaatggaacgcacaatcaaccagattacgtatgaaattattcaagagctgtacgggcacggcaatcctaataaagccgtccttgccagcatcagaagtgctgcttcaatgacgagcccgcgggcgcaaaaagtgtggccaatcatgatggataagttggaaaaatcaatgctgagtaaaaatgggcagccgacccatgcggaaaccgcaatttatgcggccttgcggctctatgcgattcatcagcaaagcagtcgggatgcatttgtctacggatcgtctggtagagatgcctcggcagatggcctgacatttttccaggcgctggcgaatttgcgaagaaatagtgacactcgcgaagcattggatcggcgggtgcaggcgctttttggaacgacgaatgttaatagtgtcatcaattcaatgactcatttgattgatattttgaaggccactaatccgactcaaaaaattgattatcccaagttggctaatgacctgtattggttccagaaaagctatcaggacgccacccagacccgtttgaaatggggacaacagtattatcaattcatcaaaccaacaactgaaggagagaaaaaataatgactaatcaaaacttatacgttgacatcaatgtgctgcagacggttccctcatcaaatatcaaccgtgatgataccggtgcccccaagaccgcgatttatggtggcgtcagtcgtgcccgagtatcctctcaaagctggaagcacgccattcgggaatcatttaaagccaatgatataaccaccggaattagaaccaaagaagctgttcaactgctggcggacaaactcaatgaaattgataccagcttagatgaagacgcagccttggttaaagcggcagatatcttcaaggctgccggcattaaagtcagcaaagacaatgaaactggcgcgctattattaatcagtccaggtcagattgaaaaattggctcaatacgccactgaccacgatgagttggataagaaagaggttaaaaccctgctaaagagtgataattcattagatttggcgctctttggtcgaatggttgccgataatccggaattaaacgttgaaggctctgcccaggttgctcatgccatttcaacccatgaagttgtgccggagtttgactactataccgcattggatgacctgcaatcagatgatacctctggtgccgcaatgcttgggacgattgaatataattcctcgacgctttatcgatatgccaacttaaacgtcaatgaattggctcacaacttgggcgagtctagtgcggttcagggagcagcggattttattaaatcatttctgctatcgatgccaaccggtaaacagaatacatttgctaataagaccttacccaattacgttatgatcaccgttcggacggatacgccagttaacttggtcaccgcatttgaagacgcggttgcttccaagcatggctatgtggcagagtcggtcaagaagttggaagatgaatatcaatcgaccttgagattcgttgatcaaccagtttcaacaattgttctcagtgacagtaaatatcactcaaagcttgatgatcaggctgccaatttgtctgaattgttgaaacgggtcaccgaggttttaacgaaggcggtgcaggatgaagacactactaattagattaacgtcacctttgcagtcgtatggaaatgaggccactttttccagaagaaccagtggcgactatccgtcgaagagtgctgtaattggtatgattgccgctgcctttggctatcatcgagacgattctcgaattactcatctgaataacttgagttttgccgttcgggttgaccagccggggacgacactgacggatttccaaacggtggagtggaagaagaataccagaaagattacttatcggaattaccttcaggacgccgttttcgtcgttggcgtgggtagtaacaacgatcaacagattgataacatcaaagaggcattaagacggccgcagtttcagctgtttttagggcgcagatcgaacgtccctgcaggggtgctcaaaatgacggttgtcccgaatgctgatccggtaaaagcactgcaacggttggagtggcaagcttcacgctggcaccagagaagatatttgcggcgtgagcagaaacagtatgccgaaaatgttgaattgatcgcagatgctaatttattgcctgaacaaagaagcgcgatggtcaaggaccgggtcgtctcgtttgaccaacggcaccggcaacatggctaccgggcatttgccactaagacgcttaaccgtgttaagctgaatgattcatacatccaaagacctgacactgatgtcgctcacaaccaggtggaaaccagccacgacgcattcgatgcggtctagaaaggagctcatatgtacttatcaagagttgaaattgacttaaataaccgccaaaagatcaaagaactgacccaccttggcgcctatcacaactgggttgaacagagctttccggatgagattgctgaacacacacgactgcggcatttatggcgaattgatcgactggccggtaaaagctacttattggttttgagccaagaggcccctgatttagaattgctgggggcttatggtgtcgagaacactgcgatgaccaaaccctatgatccatttctggaccggattaaggaaggcgagatcatgcagtttagattgaccgccaaccccgtccgtgccattagccagcccggaaggaagcaaccaagaatggttccccacattaccgtcgagcagcaacgaaaatggttgacggaccgggctgaaggccttggctttgaaattgttaagacggtttcagccgattcaatggattcagagggaaccgaaaactttgacatcgtgagccgagactggccaattttgagaaggggtcaccgaaccctccggcttagtcgagtgacttatgagggcttgctacgggtgaatgatttggatcaatttaaacagacgttgatgaatggggttggccgcgagaaggcctttggtatggggttgatgacggtgattccgagaggctagcggatgaagaggaaatttggcgcaaaaaagcccgagctgacagaattaagccgggtacgtgatcggattacgtttttgtatttggaacatgccaagcttaatcgccaagatagtgcaattattgtgactgatagtcgaggaacagtttttgttcccgcggcaattgtcagtgtcctgatgctcggacctggtgtggacgtcagtcatcgggcgatggaactaattggcgacgcgggtttgggagtggcttgggttggcgaacaaggtgtccgcgaatatgcacatggccgaccgttgaaccactcatcaaagttgctggaagctcaagccagactggtttccaatccgaaaactcgggttgcggttgcccgaaagatgtatcaaaagagattcccaaatgacgacgtgtccggtctgtcaatgcaggcattaagaggcaaggaaggcagccgggttcgtcaggtgtatcgcacgcagtcgcagaaaaccaacgtgccatggtctcgccgagagtataatcccgataattttgaggccggtaccccgattaataaagcgttaaccgccgcccatcaagcgttatatgggttgagctacagtgtgattgtcgccatgggggcatccgctggattggggtttgttcataccggtcacgatttgtcgtttgtttatgactttgcggatttgtataaagctgaaatttcaatcccggtggcatttcaggttgctgctgaatttggcgatgataaagacatcggtgctcgaacccggttggccatgcgggatgccttcgctgatgggaaattgcttgtgcgcatggtcgacgatttaacgagtttactgggggttactgaaaccagtattggtgcaggcgtcatcaatctctgggacgacaagctgggcttgcagaagtttggcgttcaataccatgaattcaaaggagatggcgactcatgatcgtcattactttgactaaagtgcctcagtcgttacgaggtgatttgaccaagtggtatcaagaagtccagaccggggtttatgttggtaacgttagtgctcgaatccgggatttgctgtgggagcgggtcatcaaagggattggtaccggtgaagccaccatggtttatagcaccaataatgaactgggttatcaaattaaaactaccaggagacagtatcaagttgttgattttgatgggattccgttgatgatgcgcttgaatgcggagacaactcccgtgaaacacgggtttagcaatgcatcgaagtttcacaaagcgaaagtgatggcccacaaagtcgcgaacaaggaccaccattctgccgttcacccattggtcgccattgatattgaaaccaccggattggatgttaccaaggatcgtattatttctattgcggctgtcaaacacagcggagatggggatcctatcagcttccagcaactgattcaaattgatcagccggttccccatcagataaccgagttgacggggattttgtcagaaatgctgactgaacaaggcgttagcttggagtcggcactggcatcgctacgtgattttattcaacaatttccggttgttgggtataatttgcattttgatgcatcatttctttctatggctttcaggaagcttgaccagcctgatttaagcaatcagatggttgatttgatgccggtggttaaaaaggttaaccaatttctggataattatcgcctggaaaccgtgcttgcagaatatcacatcaaaaattctgacccccatcgtgcgttagccgatgcgaaggcaactttgtccttagcgttgaagttgattgaaaatggcgatttgacgatttgagaatggctttaggacgcggtttgtttagtgtattccccacgtgtgtaggggtaatccgactataccgaatcgttcatgaaaaatcaacaagtattccccacgtgtgtaggggtaatcctatccacgccttacacctctacttctttggtttgtattccccacgtgtgtaggggtaatccttacgaacccaaatcgtcaaagcatctggcatggtattccccacgtgtgtaggggtaatccccaaacgcggaagtcttcaacgctagtgaatcggtattccccacgtgtgtaggggtaatcccatgtatcagcacattgatgggttaagtggttagtattccccacgtgtgtaggggtaatcctagtgagcgcgattgtagacttcatccaatcttgtagtccccacgtgtataggggtaatccttagtcatcgtttgcgtgtaagttgatgtcgccgtagtccccacgtgtataggggtaatcccatacctgcccgccgtttcctggaacggaccaagtagtccccacgtgtgtaggggtaatcctcggattgagcttgtcaaagaacaacaggtcaagtagtccccacgtgtgtaggggtaatcctgtggtcttcactgatgccaatgatatttacctgtattccccacgtatgtaggggtaatcctccttacgagaccccgctcgctgctcagtatgtgtattccccacgtatgtaggggggacctccaatccaaaccaaacaaaaaacgacttcaccaaccaaaggcaaagccgtttttcaacatcctcaaagatccttatttcaaatacatcgcccgcaacttagcaatatcggtattcgaaaccctgaggcccttattcaagaaattatccatcgtgccataatgcttcttcaccgccgagtaagtggcgttgatgtaagcaggtttgacatcttctagtgccttcactgtctggagttccttttgagaggcgccactcttcttcaactgagcataatgtttttcataaacccccttggttgccaaatagtcgtcgacaatcgtcagcttcttgacgccgagtgctgacaagatgaaaatcgttccggcacctgcccggtccttgccggctgaacaatgatacaagactgcggagttccctttattattcaaaagagtggtgaataggttgtgataagcggttcgagcttgtttggtagtgacaaaatttgtatagccctgttccattgttttgtccgtaatcgtctgatttgacgaagtattcacatttttaaagactggatccttgatgaagtcgacccctgccatggtgggatctggcgcggctttcatttccatgggagttcttaggtcgacgtcgtacttgagattgcaagttctggtaagtttctgctggtcggcctttgtcaaattggctaaactagctgaccgaatgatgcggccacttttgatcgtttttccatcagtggttcgatacccgcccaagtctcggacgttcatggcgcctttcaaatcaatttcatgcactttgactccctgggttgccacgacctgggcatttgctggagcaaccgattggatggctgcgcccgtagcggagaagacggccagtgccagggatgcaatcagaacagattttttcaatgtgatttcctccaaacttttttgattcagtgtttagtttacgggaggcgtgtaatgattttgtttgcataaggtaatgatttggtaaatgatgcttagcagattttttgctggataccagaggatcgtgaaataaaatggttgatggagctgtacactattgggataattaaaacggcagaatcggctgatttgtttcatgcgactaaataattaaggtcagatgctttcgtatttgcaagtcattgaaaatgagtgttttgtcattttcaaatggcttaatggcggcgtttctttagtgtattccccacgtacgtaggggtgatcccttgccgatccacaaccgatgtaaattcatcaagtattccccacgtacgtaggggtgatcctagacaggtgcaactagagccgccgcaaaaatagtattccccacgtacgtaggggtgatcctgttcaccccgaagtgtttcaaggcactggcaagtattccccacgtacgtaggggtgatcccaagcgactgaaaaagctaagagtaccagtaaagtattccccacgtacgtaggggtgatccttgcattctcagggaatagtgttcaagccgctagtattccccacgtacgtaagggtgatcccaagcgactgaaaaagctaagagtaccagtaaagtattccccacgtacgtaggggtgatcccgactccaaagtcggacctcaccaagaagcaatgtattccccacgtacgtaggggtgatccctccaggcagggatttgcaccctacaagcctctgtattccccacgtacgtaggggtgatccccatcagctgattatttcagggtttgagactctggtattccccacgtacgtaggggtgatcccttgatcccgacgtttccacctttatcaaaagcgtattccccacgtacgtaggggtgatcccccaggtgtcaccatgaagtgaatcgatgtactgtattccccacgtacgtaggggtgatcccaattgagaactggaacacaaccacgatcagtagtattccccacgtacgtaggggtgatcctaggaatggcatatcgcgtcgcatcaattgaatgtattccccacgtacgtaggggtgatcctaaggctgaaacttacctgaagcgattgattgagtattccccacgtacgtaggggtgatccctggcgctcgtgttggcgaggttgccaatctcagtattccccacgtacgtaggggtgatcctatgctgccgggcaccgggtcgatgtaatgggcgtattccccacgtacgtaggggtgatcccatgaaactagcaggccaaacagacccagccaggtattccccacgtacgtaggggtgatcccaagcccggtcggcattgtacgagtcagatcctgtattccccacgtacgtaggggtgatcctgatgatagccacgatgagggcgacaacaatgcgtattccccacgtacgtaggggtgatcctcgcgttcacagcgtcctgccaatggtcaatcagtattccccacgtacgtaggggtgatcctataagagttgggggacagcagccttgctctcagtattccccacgtacgtaggggtgatcctcttccaagtgaggcggtaaggagcattttatggtattcctcacgtacgtaggggtgatccttacggtggcgatcacattgacccatacggctagtattccccacatgcgtaggggtgaaccttcacggtgtccagatttttgccggaactcccagtattccccacatgcgtagggggggtgatcctgctcgcgcgggacccggcttccctggacccttgtattccctacgtatgtgggggtgatcctgcgactaacgaacttcaaatgatggattcttagtattccccacatgtgtgggggctcctttcttgcaaaaaactattttcacaaacgcgttgggttggctccaaaaaggtggaacacattcagaaaagttcaagacaaaaattagcctctgatggcgcaacagttgtaacccgccgctcaagtccggcaataattctgccgaaactcaaaaatagcacctaaccagttggctttcaccaactagtcaggtgctattagtattttgcgtaaccatcaaccaatttcaaaacagatacaataatttgaaaatgccatatagatttcgtttctaacgataattgtctaacatcttaaacttatggttgtcttggaaatatgctccaacctttagcaacaatttatcattacccttagccgcctcaaattgaattcccagcggcattttctgcttgctaacatatgttggtaaactgattgccggctctcctgaaaggttggcaagctgagtgaatggtgtcttggtcaatccatgaagccaagcatcataaattgtttgaatttgctggttgtgatcaagattaccaatgtctctcagtttatcaacgtattgaggaagataagcaggatcagtattctttggagctgtaacggctgtggtaggtgttaaataaagtggatattttttgtgaaacgcagtcatttgccggttgaccagattcaattcattttgaacagttgtatcggcattagcaggttgcttctggtcagcttgataaagtgcccaagtcattggcgaaacgtcatcaaaagtcatgttcttgcctgtgacgctcttaatgagattattggcactggttcccgttccggtggattcgagatagtagatgtgcatcaatttaacgccatcaacgggagaattggcttttacaactttaaagccttttgatcttaagaatgaaacggcttgttttactgcgttgacagcatctttgctgacgggtgtgttaaccggcgatttagttgaataagcaattggaattttcttgatattctttggaacggatttcagcatcgcatcccctgagtgatcagacgttgctaacatgccattaaatagcgtttgcatatcctgaatgtttttggcatcggcaaaattaactgaagatggtgttgtatcgtcaccttcgatcacaccttgagttggtttcaaaccaatcacgccggtccatgatgcgggaattcgaagtgatccaccagcatcatttccggtagcgacaggaacaatgtcgtctgcaacgctggcaacagccccaccagatgatccaccagtattatcagcgtggttccacggattgtgagcaaccccattcagagctgagttggtaatgttaattaagccaagctccgggaagttggtctggccaatcacgataaagcccatcgattgcaaacgctgaacaaatgaactagtggtggttgccttttgatctgctagaggaactaatcctcgcgtatttgatgaaccaacgatcggctgtcctaaccctttaatcaacaatggaacgccataaaatggctgacccgtatccttcaagttggcagcttctttcattgcttgatcttctcgcaaggaaatcactgcatttaactgtggattgtcagctttaatctttgcgacagcgtgttcaatcaattgctgtggtgtaactttaccactgcgaaccatttttgccagctgagtcgcggatgaatggtaatatgtctgatccgaaatgttaggcgcagatatagtggttgaagtgattgacgagtcggctttcacgctaactgtgttagttgatgcaagcccaaacaagatcaaagacgttcctaacaagatcgttcgtcgtaaatacttcataaaattaacccgagtttccatggttgcctccctcaaacaaatttgttgtaccaaagaatatgctaagcgctttcaatgggatgtcaatgctatttaggggtcagcttctgattcaggttattgacttcaagtcaaccaatcattaggctaattaaggaatcacttgtttggagagttaaatttaagtaattttgcaaatacgatgctttaagccggttcagttggattggggggagtgtgtaaggatgcgttccaaaattggcatggtgatttatgattggcttattgtaattttggctttgttctcaatacttttggtggttttggattttacaaaaacgattaatttggatgctagcccatggttctttattgataatggcattctgttgatttttacgtttgactacttttcgcgtttgttcgccagcaaaaacaagtgggaatttttcaaacacaatatttttgatttgttggccattttgccgttttattcggtgtttagtttcttccgatttgcgcgagtgttccgtataatgagattagtcagagcgtttaggtttgtgcgattgattggttttgttggtaaagttcaaaagtattcgtccaaatttctaaaaaccaatggcttcatttatctgctttgggttagtttggcagtgttaatcatttcagcaacattgtattctcttgcggagaacgtttcgtggggtgaatcgttgtggtgggcagtcgcaaccgcaacgactgtcggttatggtgatatttcgccacatacccttgtgggaaagattgctgcggtgatgctgatgatggtgggaattgggattattggctcgcttacgagtgcgatgacaacgttctttaccaatcgagacaacgtggataattcgtccaagatttatcggaagcttgagatgattgagtcggagaatagggatttgaagaagcaattggataagcttgagaggaaattggataagtgattgaatcgcaactcaaagtgatgggaaatgagtgatttttcattttaaaacggcttggttgcggcgtttgtttagtgtattccccacgtgtgtaggggtgatcctacttcgagttaccagccttacggataccgtcagtattccccacgtgtgtaggggtgatcccaagcatatcaagtcttctcgcgggaacgcggggtattctccacatgtgtaggggtgatcctgatttgattcaatcatttcgttatcagatttggtattccccacacgtgtagggggtgatccttctccgcagggtgtgctttgcttcatcagtatcacagtaagtgtggattgattctaagtatctagaaatgtcgaggttcagtacgactaaataaatagtattgcactgactcattaacttgggtcatacctaatgctataaatattgataggagaactagcatgacaacaccaaaagagattttagttgacggtttacaagaatttgccaagaaagttggcgggaagagtcgcaatggtaaagagctttttattaccagaactgctgttacggatcagctcacaccagacggtaagcagtatacatttatttctttaattcgaaatgatcaacaagctagtggtccgtattctgggatttccttaaaagtaaatccgggtattaatcattatcgaatttctttagatatcggtagtgagggttttggagatgactaccaacttgtggctacccctggtacaagaagaaggtttgttgaactccaatctgtgatcaacgaatattctaaggagaataggaagcaaatttcgtgcttctgtgctctcaattttacagataatagcaataagcaacagttaaaaaatcttgaaaagcaattttctgatgataatatcaattctcatccacaagacttatttgttgtctatgttgataaaccaacgattgacaatggcattcatgaagatgaagatttttggaaaatatataaggctatggtcggcacgtattcagaaattcgaaattggccaaataaaggtgaacggtcaacaatcaataaatttaagaatgcgtttaacttacaggcttcttattccaatgaggatctcgcccaagtaaagaacttgctatcgcgtgaacactacgtcgttattcagggagcaccaggagtagggaagacttatctgacatctcaacttgcacaggagtacaacccccagaatataatttttactcaatttcacgctgaaacaacatattctgactttataggtgggtacaaaccagtgcagcttaatacgggattatcataccaataccaagaaggaccactacttaaggcaattcgacaatccattgcccatcctgaaaacaatgtcttattaattattgatgaaattaatcgggctaatttgagtaatgtgttgggggagtcattctacctcttcgaaaaatctgaattaaagaataggtcggttattcatctaggagaaccagcgaatgatgtggacacggctcgaaagccattatctgtaaagcagttaccaaaaaacttgtatgtagttgctacgatgaatactgcggatcggtctcttgctgttatcgactttgccctgagacgacgttttgcctggtacaccatcattccacataaattggttaaatcagaactgcgaaacaatgaggactttcattctgacgagttcgatcgtattcatgatatttttcaagaatatgcgacatctcaggaactgatgatggaaccggggcaatcgtatttcattactgaaaaaggccagtccatcaaagaacgtattcagtatgaactattgcccttaattcgtgagtacctggataacggctacttagctaatgccgctgatgaatttaatcaattttttattgatacaattagtacatcgatttatttataggaggtggctcatgggcttagatacaaatgttccgattattgagctcaagactttttccgatacggaatatacgttacccaaaagtatgcgtggagatccacgttatcctaatgagagcaatgataagtttcttcagttgaaccaacatgcttttgaatttctaaatattgaagcgcatggaaagaacgggaagattcattttagaacaaatgaactggtaggtgccatccctataagaatgccaaataacggttcaggaactcctcagactgatttagttgtgaaaccacgctaccaatcgaatcaatctggtagttggtacgaatggatgtctgggttggcagaattttctaatcatacgttgattacagaacagaactcattattcccgctaactcgacttgaaggtagtccctcacccaaatatctgttagcaaaagaaatcattttaaagatcttaccagttctaagagaaaattcttggcggaaatttgatagtttgcaaaaagttgctaatcgacctgttggaaatgttgattgggaccaatacgctattaattcggtggatcctcaaaaacgattgatatttgaaacaagaataaattcaatatctgaagataatcgagaatttaggaatgcactggcttatttcaatgctgcagttcaagatttgcgttcatttgagacaccattgtctgtaaaagttcctttacaaagtttcatcgatcaaattcaaaaccggataatttctttaggaatcagaccgtcctgttctttatgtaatcagaaatttgctatacttcatcaagatccaacgtcgatacagaaactgaaacgagcaattaataattatattgacaacgagtcgaaacaagtgtttgcttggagaattgatttctccaaaatatatgaggattatgttcaaaaaattgtccagcttggcttggaatcagtaaagaataatgatcgaatttcaagattggcaattcctggctattcacaccaggtgacaaggctcatgccaggatatttggaacctgatataattgctgaatttggtggcagtaaaattgttattgatgcaaagtacaaatcctacttttttgatcgccaattgaaagtcaaagaatcacaacgagaacgaatgcgttcagatgtccaccagattgttgcatatacgagtctattcaactcaaagatagcgatgttggttgcacccgtgatcgatcaggatattcggtttgatttaattcagtatggtgacgtttatgttgccgttattggattgccgctggaatggagacgtagtggagagtatgcaagacaaattcgaaaatttgttaggggtattcttgaacaaatgtaactgacggatacgtgtggtttctattggaacaatgtgtgttgactgttttacttgaaatatcatcttctaagtattttcaacatttctgaccaatatgtgctttttagagaactttgcgtttgagcctattccaaatatcgttgtgagaggttagattttttaccttttttgtaatttaatgggtaactagctcaactagacatggtatacttagttataaaattatgcattcttaatcaagtgagaatgcttttttgttggattaactggaagactatctaaaataaatggttctcaaactttgctatgggccatgacgtgaacgttttttgcccatttagaagttttactttgaagtctcacgatcttatgatattctattttaggtaataatttggtactctttttatataatgggatgttctgcgtgacgatttatagattaattttgaaattaccttgaggggaggtgattcacatggagagtaacagtcaaagtcactcaaatggtcatgctgcatttttatctattggttgggtatcggctgttgttagcctatttatcccatttattggtgttttagcaattatttttggtattttagatattgttaaaagtaaatcaaagactgctgggattgtgctattagtatttgccattatcttcttataccttggtttaacagggtttggatacggcttttcatcatcgtacggttcataattatagaatctcagtctagttatgttacaagtgcattcctcaccggtgttcaagataggttcaactcctatcggggaagttatcaataatttattggagggaaacatagtgaaaagtaaaggaattaaaaaggcgggaattgcactaattattggattgtcattggggatcggtggagctacagctccttgtgtggttggcaatacaacaaatatcattgttgctagtgcgtcatcttcccggagtgctgcattgtctagcgcttatttttatgcacgatctgagcatatgtccaaacgggcaatttatcaccaattaatttcaaaatatggtgatggattttctaaacatgcagcaagttatgctgttcgtcatcttcatggaattagttggaaccataatgcactaaaatctgcacgcttttatcgacacaatgaacatatgtcaaataatgcaatttatcatcaactgatatcatcatatggggatatgttcacgcgatctcaagcacgctatgccgtacgccatctataaatattttatagatgaaaatcacgactccaaaacatgaaatctaacagttatttcttttttgattttctacgtagttttatgctatataattaagttaatttaaaatgattttagcatgaaacaacaaggggatttcaatatggaatataatcagttgattaaggagttaactgccttcagagatagtcgtggctggaaccagtatcatacactaccggcattggcgcgagctgtcggaatcgaatctggtgagctaaacgaactattcttatgggatatggaaaatgataacaaattctctgagaaacaaaaacatgacatggaacttgagctagccgacatactgacatattgctactatatgtgtgataagttgggtgttcagccgaatgacattgttcaggaaaagttagatataaacaagaagcgtcattggaaatttgatgagtaacattgaaggtgtttgtgatgagtgatattggctatccgataatcgaaaaaatcaaatatgattcccaagctgcaactaatctggaagacgccatcgatggagataagctcaagcgtaaattacttattgagtatccaacggtctatgtaatctgctcacccataaagtccggcggatttaaagtttatgttggggaaactaacgatatcgagcgaaggacagaacagcatttaaatgaagatcccaaagttagggatgattggcgagagctttcacacgctaaagatgcagaaatgtttgttatcggacatgatcacttcaataaatcgttaacactagatattgaaaatcaaatgatgctttttatgcttggtgttccaaacgttaagcacctgaataaccggcgtgaaaatgagcaaaacgaatactacacgtctgacgaaaaggacaaaattttctcccgaatttggcgtaaactccgtggattcaatcaagatctatttccagttgaaaggattattcgtgactctgccatttttaaggcatcaccatttcataatttaacaactgaacaaaaaaacgcccgggatctgatcattgatcgtgtaattgacgctttgctatcaaagaaaacgggtcagctgatcttagttgaaggtgaagcgggatctggaaagacagttctgttaagcaccatcttttatctgatcagtacgttaaaggatgacggtagtccacttcgccaaggattcgacaatctgaagaactatgttctggtcaatcacgatgagcaattgaaggtatacgaagacatcatcaataagctgaatttaaattataaaaatgatgatgttgtcagtaaaccgactcactttattaatacccatgacgaaagtgatcctgctgatgttgtgctggttgatgaagctcatttattatggactcagggaaagcaggcttatcgaggtaaaaatcagcttgatgatattcttaagcgagccagaattacagttgctatatttgaccgcaaccagattttgaaaaccgaggaatatttggaaccgcaacaaattcagactatagaagaaaaagcaatggaacaaaacaatttgattatgttgagtaatcaattgcggatccatgctaacaagcaaacgattgaatggatcagagacattactgataaaaaaatcatcaaaaaaatccccagggatagtacatatgacctgaggatgtttgacgatgcaaaagaaatgtatgatgcgatccgagagaaagctttgggagaccaaaaatccgggttgtctcgaatcttagccacctttgattggaaatacaacagtaagagaaaacctgaggatggcgattactggatggtgactgctggggatttgtcgttgccgtggaatttgcagcttaagcaaaagggacgctcactgaaaaagctggcgtgggctgagcagccacaaaccattgatgaagtcggttcaacgtatactattcagggcttcgatttaaattattgtggtgtcatcattggaccatccgttaagtatcggaatgggcatgttgtttttgacccagatgccagtgagaatactaatgccattcgaaaccgcacattgcaagatggtaagaaacgtaaagttgccagtcagctgttgcctaatgagttgaatgttttgttgactcgtggagttaatgggctttatatttatgctgtggatgatgagttgagaaatatattgttgagatcacaataatagtgtacttcgggtgatgatcgagtagacgctaaagggaggggaaccttttgcttggcattaataacaattttgtaataactggagattggggaagttcatctgacaatcttaatgtttcgggaacattaacctttaaaagtggaaaagtcacattggtaacagtacaacgactatcccttaataaagattcaacaccaagtattttcggtattggacatataaaagttgagggaataaatactgatgatattgtgatgatctctttgctgggagttgtagagtctaagaattatagtaaaactaagttctttcctcataatacggcaatacagtcttctaattatgaatacaccgcactcagtatgtttacaggcgatgtgtttgtttcaaaggatatagtcatcagaaccgtcaaagagtacccaactaatttttctgcgtggatgcacagcttacaagactttgaacaaagtaaagaagactcaggggttctacaagtctcggctaaggagaatcagggctatgttatcaagtctaaagatggcaaaaaaacttattcttttcgccgttcactagttccaacacaacagaatcaggtgaaccagattaatcggactattcaaataacagatttttttcaagtagatgatagtagtggaatgtcgttagaggaatcaatgacgataggacccatggtatccagttggtatcagttaattacaaataaagatgaaaacatttattgtaactgctttactactgtgactggtgaaaacatcactttctttaatctttccaagagcgtatcaattcaacaaagagattactctcgagaaacgaccgttttgagaagaacaaggcagtggaaggaaaatatgctttgctcactagttaattggattcgcagttatgaggtattagccccaatagcaatggctatttacccacctcaaactctgtctgttgattttcgaattcaaacagagtgtgtggcgatcgaaacaattgttgataattattataaggagataaagaaagcatattataagaaaaaagtgtcttactttatggaacaggtggatgattttgttactgtcgatgcatttaaaacttttccagtagcagagaatgtggattctttggcagacaaaataaagcagtatcgaaatccactatcccataattatttgcaggccggaataaaaccattggaagaaaaggtgttattattcaacgttttaaaagctatgataagggactggacgttgaatataatccaaattgaccaaaaaagtattaaaacggattttcaaatattttcttccatcccaggacgcgttattaaagccctttaggggattgatgatacatgtaacttctatttgatctcagaaggatttcatataatcactctaagtcattcctaatgcagtcaatgatcatttacccaacatttaccccaaataaacaaaaatttaccctcccaatgtatcctaaccatgtaggaaccccgcgttccgcacaccacatacattgggagggtaatctcatgctcacaaaacactcgttgttaatgaaactcatgctcggctcagtcaccgtcatcttgtccagtaccgcgatactgaccactcacaagcctgttcaggcgaagtcgcaatcgtctgccaaaattgaaaaactgctcgcacctcacaaagccgactacggttactacgttgaccaatacctactaaatcgcaaagaaaacgataccccagacaccaatccatccacggcgctattcaccaacaccttcgccaagttctacaagggggacggcaccaaactcaacccccagattctccaagaaaacatcgacaaatcaatcaaaatttctgaaaatgttaccccagcagaagaacttcgctcctacatcaccgatcgccaggacagcccctacgatgtaatccgcggtctgggaccatacgctgaggcgttcatcgaaaattccaacgccaagacattattctacaatctaccaaccagcgaactgccggctgacaccaaagacgatccgggatccggcattacttgggctgatgacagttccaagctgggctcgatggtcaacttagtggacaccaccgcgctttggtactactcctcatccgggaacgccaagcagttctacaaatacatccggccattccggcaggatccgcgggtgcaggtcaatccctatttgaaagcggcctttgatgccaccccgcaaaacgattacgatttcccaagtggccacaccacccaggcctgggaaaccggcttatcgatggcctacgcctttcccgagcgcttccagcaactggttacccgctcgtctgaagtcggctacgatcgcatcctagtgggccgacactcgccgctggcagtcatgggcggccgcattctcggtaccgcggtggcggcagccgttttgaataatccgcagaataaacagattgctgacaaggcgtaccaaaacgctcaaagtgtcctgctgaaatcaaacgtcaccaagtccaaggatgactataagaactaccaaaccaatttgaagaacttcgagtaccggatgacctatggctacaagccgatttcttcgatgaaggaaaagatgcgggtgcctaagggtgctgaagtcctgatccaaacccgtttcccatacctcaacgcaacccaacgccgtgaagtgctctatacgaccggattcaaatccggctacccgatgggccaggatactgaaggctggggtcgtttggatctgtttaaggccggcgccggatttggcagtctgcttggcaacactgtggttaacatgaatgcgaaacgagggggattcaatgttagtgatacttggcgcaatcatatttctggtcgtggtgcactgattaagaaaggcactgggagcctgactttggagggcgcgaacagctatcaaggtgggacgtttatcaagggtggcacaatgtcgctgccaatcagcgggcacttggttctggcagttttaaattatccaatggcactctgcggctgtccgccaaaacggttaatgtgaagggcaattacacccagcgtaagcgtggcgcacttcagcttgctggcaatcaggcattgaacgtcaaaggcaacggccatctttccggaaaattagtcattaacttgaagtcccggctgactaagaatcatgttttgatgaagttccatacccgttccggcaagtataagcatgttaccatcactggtcagtacagtcactatcatgttaagtacacatcaaacagtattgtgcttgttaagtaattttcacaactgatagattggcacattagtcgataggatgtgtctaattgcaacccacatcaccctttaaagttgacaaaactgagaacaaatagctgattccaaaatgtggcgtttcaggccacgtccagatactgccagtgtttcttttgatcgaatggaacaaccacgccgactaaccaaaataagacggtgattaaacaaacagatatcaatgagtaacaggcaaggactcgcggcagccgaacgattggcgtgcaggtccttgtttttgcaatttatgctatttggggaacatgtcggtaagataaatcatccgtctcattttaggagttcctcaatgacaaacctttctcggtggattaatagtagccgataataaatactcattttcaataatgaatttcagtgtacagttgcagcacgtggcacaagacttatgtaagacaatgcggtgatgagagataaattctcaccaccgcattgttttaaaaaatgaaatcaatcacgattgaatcttgctgatgtttcatttagctgcggaattttcttaactttccgatcccaagtaatcctaacagcgagagcccaagaagcgctaaccagttggcactgtgtgtgtcaccagtttgtggtagcattgcggctcccttaacgtttaaatcttgttgaacggctggcttaactgtggcatcagtcgtactgttagcgtacttgaatgttttaccacgctcacctgatagtgcctgcaagctggtcatgccacgtgacgctgagttagggttgaccttgaggtaaagtagcccttcctttttaccagactgagttttcttgtctgatgagctggtggcttccttctcgtcgtccttggcaggtaatccttgtggttgctccacaatgtcgtcaggacttggaatttcggtaactggtggttgtggggtgggggtttccggcgtaggtgttggtgtcggagttggtgtttctggcgtttctggagtcacaccaggagttccgccaccgttgttaccaccgccaccaccacctggaggagtaaccgttttttctaccttaacaccgtagcgttcgttgactgcgtatgtgtaaaggggcgcttcagatttggcgtagctttcattcatcccgtaaatgtatgaggttttggcaggggtgatcttgacaccatattgggtgttttcagcgtaatagcgtgtacttccgccaccttgtggcttataaaaaactgtatctggatggaaattttgattgtcatgagccgattttacaatataaggcgtgttgttaaatgtcatgaagtcggagccatctttaacggcggatttgatagcagcctcttctaacttacttccaccttttttcaataatgctttggtttcagcaacggcggccgcagcattatattcattttgttcttccggtgataattcgactagatcacctgattcagaatcgtatttatagacatatccatcgctgccaatgaacactgtgtgaatctcagttgcattcgcatcacttggcttcacgtaatccttttgttctgccgtttcatgggtaaaggatgaagcaccatttggaatcctatcttcatcatcttctgtgatcactttatacttattccaagtggtgagttgggatccttcagcaatggatgcttcatagtccctttggaaatctgttaaatcttcatcagttgtgtatccaacctgaagtgcgccagcgcggatggcttcatcgatatcgcttgaatcgacggggatgtcaaatgcatcactatctggattatacgaaaagtaagacggttcaccagttccattatcaaattgggcgacataaactggaacagcttggttaggcttgttgccatcattcttgaagtaatactgtacaatcattgccacgccgttgtccttaataacttctggtatgttccgtggatcatttgtatcgtttcggacaatcttatatgagagaacgttgtcatccccatcttcgacggccttcaagaaggcagcagtgctatcttcaccaagcagagttgtttgtacgactccggcatcatctgctttattaatttcatcaattaggggatcattgttctcaagtaatctatatttacccgttccttcgggatcatttgcgttgtccggttcgaataaataatgttcgatcgttgtttcccgcgtttgtgggttaatggtaacctgacgataaatgatgttccggcgatcatcttgaccagttgcgtttttccataaaacaaatgtttctttgacttcttcagccttattttgcttggttgagttggtatcagcctttgcggtctttacggccttcttatcttgcttaggtgtttgagaagttgttctttgtttatgctttgatgtggcggttgtccctttagaacttgaatgattagttgtttgggtatctgtctgggttgcttgcgctgtttgtgcagcagtctgttgagttgccgccgatgtctgttccgtcacaccctggttagtcgtttgttgtgcctgaggggcctgttgggtttgagcagtgacagtcggttgctgagtcgttgtctgtgttgtctggtcagtggttgcttgcggtgtctgagtcacagttgctgattcagtggccgatgttgtcggcgttaccgtttcttccgtggcttgtgtgtccattttcccagtgccataggcttgtggtgtcgatggatccgttgctgtctgctcagcctgagttggggcttggaacgtaacttggcctgaatcggtgttagccgaagttgttgctggttgttgagtcgtgggggttgttgcagtggttggtacctggtcgtcagcgtgaaccttcgactggtcgaggccggtagtggttgaaacacccaccagcacacctgcagctaataaaagctggcgcttcaattgcttgtttgaatgtttaatcataaatgaatcctccaaaatatatataagatttaggtacggggatcatattagcaaatagttatgaataaagtttgaataaagatagaattaaaatctgatttgtaaatgtgcaagcaccacgtagtccaaattcttgagcaataaagccggcatggctgccaatccacgggcaacatgaagcttcacatccggttcaggaagcttgaatatgttaccatcaccggtaagtacggccaatatcatattaagtacacgcaaaatggtgttgaactagttaaatcctggctataaattaagctggtacatctggggggattcaggtgtaccagctttttggttgggtcacacagaatggccatttccgattccccacttatagattgaatgattgttgactttctcacaaaaaaatctaccaaatgtttggatgaacccacaaacatctcatagtgattatgtcataggattgttggtgaaagatagttgaggagtaatgacagtatgttcaatgtttgaaggggagttgatcatatgaatcggatgacgaaaacactattgtctgttggcgcgattttatttggtgtgacctgtttggccggcttttcaaccactacgcaagctgcgacagttagtccaccgacgacctcactggcccagccacaagctctggctgatgaaaatggcggccagctcggcgatgtgacttggaagattgaaggggacacgctgacactgagcggcggcaccctgcccaatttgggtaattctgattatgattacccgtggtcgcattccggtaccccgtcatcggtcaccaaagtggtgattgaaggtggcttgaccttggaaggggactccgggcagggtctcttcaaggatctgacccacgtcacctcaattgagggcttggacaagttggtgacaaccaacaccaccagcatgcagaacatgtttcttcgtgactatgccttaaccagcattgatctatccgcttttcacactgaaaatgtgactaacatgagcgacatgtttggcgaggatcatgccttgaccagtttggacgtttctcaatttgaaacgggtaaagttgagtcgatggacggcatgttcgatggcgataacaatttaacatccttggacgtttccaactttgataccagccaagtaacagatatgggctatatgtttgatgaggactatgaactaaccacgcttgacttgtcgaactttgatactcgtaaggttgaccagatggacttcatgtttgcccaagaccacaagctgaccagcatttgttttggtaaattatttgataccgccaacgttgtggggatgacttctatgtttgaggaagaccgtgctctaaaagccgttgacgtttctcattttgacaccgcaaaagtcgaaaatatggatagtatgtttctcgacgacgcgtccctgtcatcactcgacctatccagctttgacacagatcaagtcgaagaatacggcttagatgatatgctgaccggcgccaccaacctgactcgattggttctcggaccccaagttgaattacgagacggtgttggtctcgaagctgccaaagatgacagtgattggcaagccgtcgctaaaggcaccattgagcaaccgtctggtcaaacctttgatcctgacagtctggtagaaaaatatgcagccgccggggttcccaaagaactgtatgttcccgaagatggtttcaaagatcaatccaaggtgaccgtcacaccaagtatcaccttgtcactcggggacaaatttgatgcgaccgagcacttcatctctgccattacacctgaaggccgttcggttacgaaatactgtgatgcggctgctgaagggctggtcattgatggcggtaacatcgacacctcaaagctgggcacttacacggttacctaccacttctatgggagtgatcaaaaggcaacgatgaccgtcacgatccctgccgctggtggtggcggtggcggcagcgtcactccaccagcaccgatcaccccggcaccacaaccgacgccaacaccgagtccagcgccgacgccgactgaacccactaagccgacaacaccgaatatcccgaactatgcggcaaccaagaaggcggcagtctatgccctcaagaccatttacctctaccaaaatccaactttcaagaaggcgcagcgaatggcccgttatccaaagcagaagcggattaatcgcccaatgtttgtcgtgatcgattacgcacggtcaaatggtggcgcacttcgctacaaagttcgtgacgtcaaccaccacagcaagaccgatggcaaaatcggctacatcacagccaagtggtcccatgttcgtccggtatactaccgttcaatgccaaagggcaacgtgattaccgttatttccaagaagggtgttcacgcctacaagaacaagaatttaactggacgggttaagtcatacaagaaaggcacgcacctgaaagttaagagcttagttaagcacaatttgaccacccgttatgtattgagtaatgggtaccatgtcaccgccaataagaaattggtgattcaggggaagtattaattaatatatgttaaatagacagatccaatgcggatctgcctattttgggactaattttaggaataccagcttattgactgtcgatttactaaatccatttgtctttgaaccgccaactcgatacaatatctgtaacaggtgatcgcacaatttaccacagttcatgactctcactacgcgaagggacattcagtaatgaataaagatgatcaaaaggaactgattacaaagattaataaaatgcaaccggaggaaatcaagaacttcgttttgcgactagcttctctggatgataatttggccggggttattttgaccgtattaaacgatgaaccaattgaggcttctcatccagatcgagaagcaccgcttgccaatggcagtagctttaccgaagtggaccaagaggccgtcgaaagagatattcgccgtatccgcggattagtttccaattcaattcgggaaactgttggcaacacggattatctaacaccaaagaagactgaagagttgactgagttttttaatcacttggttaagagatttcaggatgggtataagtctggtgagatgccgattgaacttacggtaccgttattgctaatgctctaccaaaatcagattcagttattacctaaagtggttggtcgcagggatacctttgaggatggttgcaatggtgtgctctctgctctggaggaagtgattggtaacggcaactcactgagcgcgaataagaaaaatcggttgatgcagcaagtcatcaagctgtttaagaaaaatatctttcaaggttttccacaagaaagatatgatttgttctacgcgactttgccattggtaaccgaggagaccgcaccaaagatgcttacggtttccaataagcttaaaaagcaagccagcatattggatatgatatatcttgagtcaaatcagattattctgaaactccgaattgcgctcatattggggcacaaagacgaggcccagcaaattattgacgacaacattaccaatgacaatgtgcgattagaatatgtctcaatccttgaagcacagaaaaaatatgccaaggcagaagaagtcattcaagatgcgttgacgaacaatgtgggtgatcgcagaatgtggcgatttcaacttggccaaatctatgaactgacaaatcaaattaacaagttaaagcaattgttgaaggatgacttgatgtcaggaaatatccaggtatataaagaatataaggacttgctggttaagaacaatgaatggaaacatgagtatccacagttattaaccgagctagaggacaatcttggtcgatacgattattgcgaaatccttcttcaagaaaaagagtacactaaactgattgatcaacttaaaaaatacaatagcatggtcatgatcaggaagtatgctccagagatttatcaatctgccaagattcccgtgaccgacttatatttaaaatcagtcgtcattcctcagtctaataagaagacggtaaccgggccagcccaactggcaagtgatattagcaagttcctaaactttagcggcgaccttaagacaactaagaaatgggttcaccaacttagagcccgacttggtgataacgagaaattccgggatgcatttgacaagatggacgattcaattagtagatattccccacattcggggcgatcattatcagactaaaataccactcacccgtaagttaagcatactttgatcacccgttatgtattgagtaatgggtaccatgtcaccgctaataagaaattggtgattcaggggaagtattaatcgtatgtcaaaaaggcagatcctagtcgggtctgcctttttgtgtgttcattgaactggtttaaagatcagtctgcggctaacagttatgtctaatttggtatgacagcccctcatcaaaattcaagtgttccgttatacggccaacgttgtgaagaatgacgacgataatccggtggagattaattcaatttccaaccagtatcagaaaatcagcgattatgacaaagcgtactaacaatattcaagaagaggcatacccccaaggtaatcacataaaccttggaggtatgccttttctcgaatttcaaatgtgaacaaactaagctttcacgaaatcaaggttctggtattccggatttggataatgatagaagccttcgccggtggcaacccccagcttgttggctttgaccagttcattgagtttatcggcaatcttttgataagtctcgtccttggtattctcatagaatcccatttcgatgttgacggccgtgttgagccccatgatatcaagaaatccaaacggaccgcggtcgactcccatgctgaccatccagttcttatcgattgaaattgggtctgagaacccatttgcccacagagatagtgcggcattaatcattggcaggaaaattgaattcatgatgtacccagagatttcttttctgatcaaaatcgggatcatgtgaatttgtttggcaaaattttcggcatcatcaatggtcgactgaggggtgtcaggggcccacattatttcagcaacattgtgaatccaaattaaattagcaaagtgcattgccataaatcgttgcttgtttggcacaaaatcaatcaattgacttggaactagtgtcgatgaattcgtcaacaatagcgcatcgtcggcgataaacggtgccagattcttgtaggtcgattccttaatatcgagtcgttccgggacggcttcgataatgacgctggcaccagtgacggcagactttaaatcagtggtgagtgatagattactgttggcggtgtcaatttgggcatcggtggcgttgatgtcctgttgatactgttttggataactggcaactttttgcttggcactatcgacggcttcatctgaaatgtcatagatgacggttgggaaccctgaaaaagcggattgataagcaatctgacttccgagaaccccgccgcccagaatgacgactttattaacgttcataatatccatcctttcttaatgcacacatattgtatgccggaatggaagcggttacaataatatatttttaaatttttgagtgggactagtcagaaacgacaaaaaataaccaacggcatgatcccgatagaatatcaaaatcatgccgttgaagaaactgcagaacagttttaaatatttaattgtctactcgaccgggagtatttctgctccaaattaattggtttcatcggcaaatttatcataaagttgagtgaagttaatggtacctaatccacttgcctggttgtaaatcttgccgggttgaccggtgtagtacaaattattgttgttatcagcgtcatcgaggacgttaaacgggctgtcggattcctgagcaaatttgtaaatttgcggattccagaaaccgattggggtttggcggccgctgttcatcacagcgttggcaccagccatctgtggtgaggtgtaactggttccgccgccaatcagccattttgtgcttgggatgcgaagaacctttttaccctttagcactggattttttccggtgacgtaggtcgcatacccggtttgcaaatcagcgttgccggcaacgtcaggaatgttgcgtgagttgccggttccaaaaatgatgtggggatgtttggtgagagtgaacttgccgtttttatacgttagaaggttttccgctctaaacgtattcacaccggaaaccccttgttgataacgaggggtcgggttcaaggctgagaagccgccgccaccgccgccaaatatacccatttgcttttcctgggcggtttgggcgtaggtgtctccccaagctcgttccttggaaacggtaatgaccttattattcagaatcttctggtatggcaaggtggttccgcccactaagacctgataaggggaagttgacaaaccgtggttttccttggcactcggttgactaaccgggccatagtcaccactggcctgaaagacggtaatgccttgcgctgcggcctgttcatacattaagttaaacgcgtccgaagtttgtttgaccgttgcacttggatcgccccagtcggcggtcacttcaggagcagccgagaagcttgatgaaagctgcttgtcctggttgtcggaaatggccgacatcgtaccggtgtagatcgctgaagggtcagatgtatttggattggtgtcatcgccaatgtagagatcaatatctgcctttggggcaaccgatgaggctgattccacatcgaccgtcgtttcggtctgcgggctgccgaggagatagttgacgctcttttggacctcggcctttggattgacgaggtagtggtggtgaatttgactcacattagcgtcaatgccggattgcttccagtaagttgccacgtcaccgtcatgaatgtcgctaacagtgataatgccgatccgctgaccttgaccctgaaggcccttttgatacaggggatttagttggtaggctttggcaaactttccggcaccgtacttcagtgaaaaggtgtttgctgaaacgttggtgttcggctgctgactggaaatcggcaaatcggccattaatgcatgggaagcagctgcttttttggttgttttcttagcagtcgtctttttagtcggcttttgcgcatagagcccaattacggcaaccaccttactcgacaaattgccaggcagcttatagctggtagtggcttcgtaacccttcttggccggtttgacatactttgcgttaaaagccttttgcatgtttttcggcgtggcagtcagcttcattgccaagttgccgggatacgcgtaactgcgaatatgatatttgttgagatagtctttaaatgactgtatatagctggtggattggccaaatttgtcggcaaattcactcggcgttaagtaatgatgatggttgggacttgttggatcgaccgtgtcgtaaacgtagttgctcaaatcagcctcgctggtactgggcttgaacgtcacgttgacgacggtccgtttaacggttgccgcctgactcgcagatccgatggccgcactagctcccaaaaccatcaggccgcttaaagcggtaatgacaaaactttttcccctcaatataatcactcttttcttgtgttatctggcttcaattataccaatctaattgtgagattacttgaatttaggctggtttcaggggttagttaaccacttttgccagccagtacccaaaacgtgcgatgatggtaaaacatattaatatcataaacagcgcaaatcaaaaggcttggcgagtcaacacactcaccaagccttgatttgccccttaagactcactaaatttaaacttcgcaggatcccacatccgcgaatgcccaacccgatcatacccatagtgaaaattgatgtaagggtaggggtcatccggctggacgtccttgccgatcatcagcagctgggattggatgaagctttgcacactgtggccaatgatcgtcttgtttgcattgctgagttgctggaaattgtcattgactttaacaataaagccgcgccgcttatcataaacaattccgccaacaaatagtgaccaagcataggcatcctcgccattttcggcctccttttggtcttgaatcaactcatcatccagactttggttaaattcatcccgttcttttgcggacaaagcggcgtacggatcttcgtcgtcatctgattccgatgacgcgggttcctcggcttccgtcgattcatccaacgactcctctgacgcactggattcagtcgctgagtcggcttgctgactggtttgagtcgaactggaattatctgactgggttccgcccgtggccatcccaatcacaaataacacacagaaagcaatccccaggtgcttccagccaaacggtgcaggctcttgcttctgccgtttttggtataaataaattgctgcaatgataaggccgatgtagcccaatcctaatagtacttgaagaaattccataaaatacctccgaataaagtgacgaataattgcaaatttaattgctgccagctaggccataccatatagatacggcacaaagctcgtttatcgtcattatctctaagaatttcttaaaattacagtttaaactctggatctgggcaaaaatccgcccccggcgacgacccgattcattaacagtgttacaatttctttggcgaaccaatcaatttgaacaaggaagatgaaaatatgaataccaaaaataaattaaaggcaaccttactaatcgctgccggagcgctcttgctgggcatttcgacgacccagccgaccagcgccagtgccacagcatcatccactaccagcaccactaaatcaacgtccacccgttacgatgcccaaattatcacaccaaagtcacttgcaagcggctaccaaatttattccaacgtccctggggtcaagaacaccaccggaacgccaacgactacaacagacagcagcaagtacaacaaccaatacgtccgcgtgatgcagacgcaaaaggccaagtcggttacatatgcacaaatccgcctcaatggtaaaatcttgggttggatcaacgccaatgcacttaagcagacttcgtttaaggcaatcgcccaagccaccatgcaaaagtacaacgccgtcggcagcgtcctggtttctcacaacaagagcctgcaacccactttggttaacaacggctatgccaatatgctccacagcaccaagaataccagcgatgggtcggttctctatccactggcctcgcttcaaaacaccatgactgcagcaatgatccaacaattgatcaacaccaagaagttgactgccaccacgactttgagcaagtacttcccacaagtcgcccacagcaagacgatcactatccagcaactgctgacgatgacttccggcatcaaagggacgatcaaggcgcctgatgatcaggtcaccgaagatcaagcctacaccaacgccattaaggctttgaagtccaccaacaaacacagtttcagctacagtgacatcaactacgttctgttagctggcgtcatcgccaaagtcaccggcaagtcgtacaccaagaatctccaatcacggattttgaacaagctgggcatgaagaatacctatgcgattaacgaaacccaaccggatttgacggcgattaaggcggtcagctacagcagttctaacggcaatgactaccagaactcccagtcggtttcctacccggctctttcagcgctgcccggcgccggcaacgttttgacgacgccaaatgactactacaagtttgttattggcctgcaaaacggcaaagtgctgactgccaaggggtatcagcagctaaccagttacagcaccaagtattccggtgggatgtacgttgatcaaaaagggatgaagtccaataacggaacttatcccggcagcggatttaacaccggctacactgcctcagacggcaaccagcacgtcgcagtggtcttcttgaaccagtcaccactgaagaacaacatgacggcttcggcatttcttgccaagatgaacattgtcgctacttattactaaaatgttaatcattaacgcccttgattgagagcatccaaatgcttggaactcccgatcaggggcgttttgttatccattcgtttccggaattgttatgcggaggcgataacttaattattaagatttaagaagaaaaaccatgccaaaaccatcaccgaaaattaaagaaattctcaagaaactaaaacttagctaaagggcggctgaatttcctgcgaaatcgttgccatttatttcggtttgttcataatggacttaattaaatgttactggaatattacaaacggtttacagccgtgtttccggtttttaaaggggggtgagcccatgaaacgggggcgcacgtacttatacataacactgattatcctggcggttgttggtactgtgggcggggccatgtactggcgggctaacaaccaggagcttcgaacgcaacaagcggccaaacgtgccaatcgccgcaggcaggagcagcagctcagctcaacggctaagaagcgggaggcaagcacacaaaagtcggcgccaagacagattcagcacaaaacgacccagcagaccaagcagattaccagttacctgaagcggaatcactttgtcggctcggcgattattgtcaaaaataaccacattctctaccagcagggcttcggttatgccaattacaaatcagacatcccaaatacacccagctcggaatttcaaattctatccattcaaaaatcactgacagcggtaatggcaatgaagctgatcactcagggcaagttgtcattgaacaccaagctgtcgaagtactatccaaagattgccaattcccggaacatcaccatccgcaatctaatggatatggattccggtttgacgatgagtgaggccggttcggtccgcacactgaatgaagaaaacgtcattaagtacgcggttaaccacatcgtcactcgatcaccaaagtataaggactggtaccaaccggtcaacttcgtcgtattagcggggattatttccaaaattacccacaagtcatacggcaaatatttcgatcaattgtttaccaaaccgctgaacctcaagggaaccggcttcgttcagcattggggcactcgaccgaaccggacgcttgggtaccactggttggcggctaaccaactgaagcaaaattacagcaggcagtatcacgaagccaaagcatcgatgcaaaatgaattgggcaccggccaggttttcatgaccccatttgacctcttcaaggttgagcaggcgatcctcaaaggaaagattattccgaaagccagtgtggccattttgcatcagccgggtctcaatgccccgtatggcggcggtatttataaccagcaaaacgggattcgctcccatggcattggctacggatatgaatcgtcattgttcatcactcgcaatggcaaatccggtgtcgttttactcagcaacgactaccggccggccaatcagattcaaaacttagccgccaggttatttgacgacctggcaacgtaaaaattgaaaggtcactttgattgaaagcgctgtaaaacaagatattatatgggtgacgaaacgttacccatttaacaagggggatgatcatatgccagtacgacaatggttgcaaaagccgtgggtgcgctttacgatcacgacgctcatctacttttcgatcatgttggttcttttttacctctacgactatagcggcattaatcaagcgaaatttatctataacgacttctaagggggaacaaccagatgattgaaacgctcatttcaacaatcgattcacatgcacaaaaccagggggataaggttgcttacgcctacgatggcgagaaacacacgtatcaagaactcaaagattactcggatgctttagccgagcggattgactcgatggcactaccgctgaaccagccaatcatcgtctttggcggcaaggcctttacgatgatcgtgtcatttttggcggcggttaaatccggtcacccatacattccggtggacattaattcacctaaggaacgtttggaaatgattaatcaaattgccaaaccggtagcagtcatcgcgactgagccactgccggagaaactgccggatattccagaaattgatcaggaacagctcgaccacatttgcctggaaaaagttgattatcgactgacccatccggttcatggggatcaaacctactacatcattttcacctcaggaactactggtgttccaaagggtgtcgaaatcagttacaacaacctggccggctttgtcgactggatggtgagtgatgctttcgacttgccaaaggatctgcagatgcttcagcagccggcctactcatttgatttgtcggtcatgagcctgtatccaacacttttccaaggcggtacgcttcacgtcttatccaagaagaccaccgacaattttatcgtcttattcacggccctgcggacgatgccgattaatacctgggtttcaaccccatcattcgtcgacatttgcctgttggaatcaacttttgatcaggcccattatccgaagctacatgattttctcttctgcggcgaggaattaacccacaagaccgcggccgcccttaacaaacggttcccggatgctcatattttcaatacatatgggccaaccgaatcaacggtggcaattaccgaaattgaaattaccaatgacattttgaaccactatgagcggctgccaatcggctaccttaaacctggtatgaatgcccaggtggtcaacgaaaatggtgcacaggtaaccgatggccagaaaggtgagttggtcatttacgggcagaacgtttccaagggctacatcaacaaccctgagaaaaatgctcaggccttctttaaaatcggcgaccagcaggcttatcgaaccggcgatattgtcaccatggctgcagatggcttactgcgctactttggccggaaagacttccagattaagctcaatggcttccggattgaactggaggacgtttccgcactggttagcaaagaagaacacgtcaagcaggcagtggtggtgcccaagtacaactcacagcacactgtgtcgatgctgattgcctacgttgtaccgcaggaaaatgatttcaagaataacttggaacttaccgcggcgattaagaaaaacttggggcaggatatgatggcctacatgattccacaaaagattgtttatcaaaaatcactgccgttgagctctaacgggaaggtcgacattaaagcagtgattgccgaggtcaacagtcaatgagatggtacattccatacggcaacccaacctacttcatctggctggcgctggcgattatcccgttaatgattgggttgttgtatgggcaccggttccgcggctaccagacgattatctcgctgttcttcctgattttgacttttggtgggcccaactggaaaaccgggatttcactgattggttacctgatttatcagctgatcctcgtgtggctgtactcaacgtaccggcagaaaaaggacacgcccaataagggatggatctttgtcaccgcagtggtcctggcgatcgtgcctttggtgatcgttaagctcacgccgctgtttacgcctggtcgccaatcgattatcggctttatgggaatttcttacattacctttaaagtcgtgcagaccatcatggaaacccgtgatgggatgattaaggaattccatccggtgttgtttggccagtttctattgttcttcccgaccatttcgtcaggaccaatcgaccgttaccgccgatttgaagctgattatgccaaggtgccggagcagagtgcctacctggatatgattcaaaagggtgtccgctacgttttccaaggctttgtctacaaattcgtcctggcctactactttggctcggtcctaatgccccaaattcaaatgcgggcgttgatggctcacggcttttcctggaacatcgtcgcttacatgtatgcttacagtatggatttattctttgatttcgctggttacagtttgttcgccgtcggcatcagttatctgatgggtatcaagacgccgatgaacttcaatcagccgtttaaatcaaagaatatcaaggacttctggaatcgttggcacatgactctgtcgttttggttccgtgattacattttcatgcggttggtcttcttctgcatgaagcatcacatctttaagagtcgaaccaccactgccaacgtgtgctacgtgattaacatgctgatcatggggttctggcacggcgagacctggtactacatcacttatggtctctaccatgggtttgcgatggtgattaacgacacttggctgcggttcaagaagaagcatcaggaccacattccacataacaagttcacagaagcctttgcgatttttctgacatttaacgttgtttgtttcagtttcctgattttctcaggattcttgaacacattgttctttgcaccgaaaccattttaattaagaggagttgttcataatggatgataaacaaacggtacttgatattttaaaagacttaactggtgaagatttttctgacaatttggatgaagatttatactcaagtgcgttgctggactcaatggggacggtgcagttactgctggatctccaagataaattgggcgttcaagcccccgtttcagaatttgatcgaaacgagtggaacacgcctgctaaaattattgcgaaagttgaagcagccaaatgagtgttaaaaagcggctcttcatgatatttgggccgatttttgctgcagcactgttgatgctggccgtgtttttatcgccgctgtggtcggggttcagctatgtgaatcccacagtcgtcgacaacgccgccgcatcgctttcgccgcaggttttaaaaggccagctgattaaacgtaacgcacttgaacatgattatgtcccattctttggttcatcagagtggtcgcggtttgacccgtttcatccttctgttctggcggccaagtacaaacgaagttatcggccgttcttgcttggtgcccggggcagtcagtcactgacgcatttctttgtcatgcagtcggtcaatccccagttaaaaaataaaaaggccgtcgttttcgtatccccccagtggttcacgcccaagggagaagaccccaatgccttttcgttctattactcaactttgcaaacgaccaattggattaagcagcagaacggatccaaaatggatcgctatgccgcttatcggctcttgcagatgccttccggtaattccgacaaggtgattgccggcgcgttggcccggatcgctgccggtctaaaaccgacaacttctcaaatgttgtatgtcaatttgcgcaaccgcattttgctgaatgaagatcaaatcttctcgcgatatcggattccgctgaacaacgaggaaaccatcgataagaacgaggagctgcttccagctcaatacaactatcaaaagttggatcagctggccggcaaaattggtgccgaaaaaaacgtcttcaaatgatttccaaatttccaacagcttttggaatcgccgattgaagacccacgtgaagaaactcaagggattccagtccaatatgagcttcttaaagtcgcctgaatatggtgatttccaattgatgctcaaccaatttgccaacgaccataccaaggtgttattcatcattccgccgattaacgcgaaatggcagaagtacaccggtttgtcggcaaaaatgctggatcagttcagcaataaaattacttatcagctgcggtcacaaggatttacccacattgacaatctcagccatgacggcaacgttccttactttatgaccgacacaatccaccctggctggcggggctggctgaaaatggatcaggcaattcggccgtttttgacgaagaaggtcaaaacgccgcattaccgaattgacaactactattactctaaagattggcaaaacgaaagtggaagtgacaacgattttgatgaataagtttaaaagcaggaccgtcatgttattcttggcgggcctgttgtctgttgggggcttgatggccggaaacaaggcttttgctgcctataatgcggtgatggcaaccagcaataagcattacgatgcccaaattgtgaatcaaacgactgttaagcgcggctataatttatacaccgacggcccttacaataccaacgccacgaccaagacggccgatggcaatggttataaatataacaatgcctatgtccgggtcctgcagaccaagaccaccaagactggtacttacgtgttattgaggtactacaaccagaagctgggctggatgaatattcacgggatcaagtcggtgagtttcaatacgattgccagtaacatgatgaagcaatataacgtggttggaacagctgtcttggcttctgccggcagcaacaataccgccgttgtcagcaatggctatgccaatgcgttgagaaacgtggttaacaccagcaacggaacggttgtctatccgctggcttcgctgcaaaaggcgatgactggcgccattattcagcagttgatcagtgccggccagctgacgccgacaacgccgttaagtaagtactatccgaccgtgccatatagcagtcagattacaattgccgaaatgctgtcgatgacgtctggcattgataacactgatgtgacgccaagcagccaattgacggaaaatcaggcgtacgccagcatgattcagcgcctgaagtcgaccggtcagaatacttataattacagtgatgccaatttcgtgctgttggccggtattatttccaaggtgaccggcaaaagctatgcccagaatctacagagccggatttttaacgcggttgggatgaagaataccatcatcgtgggcagtaagcagcccagcaccaaatcaacggtggcggtcggctacaccaatcaaggtaaatacaattaccaggatgccgacgcggtttcttatgcccgactctcggcaattcccggtgccggcaacctgttaagtaccccgagtgatttttataaatttgtccagggcctgcaaaacgggcagatcttgtcagccagtcagttccagcaattgaccagctacggcaactactattccggcggcctgtacgtcaacaaggacggcctgaaatataataatggctcctttggcggctcaagtttccacaccagctactacgcgcgagatgacaactaccacatggcactggtgtttatgaaccagtatccgctggtggggggcattagtgcgaaggcctttacgcagaagatgtatgatgtggcgacttattattaaacaatttcataataaaagaatcggtgatgatttggtcaccgattcttttttttaatgagtaattaaaatgttaagcgagtcctgacgaatgacttggaaatgatataatcaagaaaaaatggagatgtcaaaatgcctattgtagttctcaaagacttttatcaaccgaacgatttaattcaaattgtgaccgccgcaattcatgccaacaacgctgactgccatgccatcattgagccaaacatcatcgtttcgtcttcaaatgttgtcagtaatccaaggcgatatgaagatctcatgcactttaccgtcagaccctttaaccagaaattaaaagggatttatagtttttataaagagcggggtaatgtttatctagaaaaactacccgacaattctgtcatgggactgtctccaatttacttaggagaaggtaaagaaagcacagttcccaagcaattaatggcggctctcgaaaaaaagattgaatcattctgttatgagaacggcgtggccaatgtcgatcgttatccttttgatcagttaaaattggcagaagtgactttgcgaattgtatcggaagatacttatcaagttcccggttttactttcgatattcaagcattgcctgaggttgaggttgaataatccgactaccactcaatctcctcaaccggttccggcgaatcattcaactcatcattcttaacctggccatcaccaatttcgatgatgtggtcggccattggtttaatcatgccattgtgggtaacgatgatgacattcttgtccgttttgtggctgaaatcttggagtaacttgaggatgcttttaccagttttataatccagtgccccagttggctcgtcacagaggagcagctcggggttcttggcgatcgcccgggcaatggcaactcgctgctgctcgccgccggatagttgggccgggaaattgttggttcgtttggccaggccaacgtctttcatgacctcgggtacgtccagtgagtctggtgaaatttgggatgccaactcgacgttttccaaagcggtgaggttggggattaggttgtagaactggaagacaaatccgactgatagccgtcgataggttgttagctgttttggcgaataggtcgcgatattgcgatcgttgacgattacgtctcctttagtgggcgtatccattccgcctaaaatgttgagcagcgtggatttccccgctcccgaggcgccgacaataattgtgagttcgccctttttaatttcaaaattaatgtcgtcgttggcgcggacttcctgctcgccgctgccgtaaattttggatacgtgtttgacgtcgatatatgccatgattgcctcccgaattgtttctttatcgattatgatacttgtggtttgcagggaaagcaaccatgattgagattgaaaaaatcctctcgtgaaggaacattgcgagaggattttgcttacttcttcaatttatcaatgacttccttaagtgattcctcaaaagtcggtagcggatgtcccaaagcttctgggaggtcgttggaagtttcttccaggtcaccatttcgaatcaagcgctgcatgccaacgattgaagcggcagctgctggactgtatcctgtggccacaaggcgcttacggtattcatcatcggaaactgacatcacttcgaagtcgttatcggtgactaattgtagggcgcgggccaaatcggcatagtcgtgttgcggtccggaaaattcatacaccgttttcggctcatcggtcattagaactttggcagctgcttcggcgtactcccgttccagtgcccagccaacccggccgtttccggcagaatagacgaagggtcggttgttaatggctgcgggaatctgcaggcgctcattttccagataccagttgtttcgtaagaacgagtaaccaattcccgattgacggatagcctgttcagtattcttgtggtcaacggcaagtggcgatttggccgtgtctgcatgtgggaagctggtgtaggcgatgaaccggacaccggctttttttggcggcattaatcacattttggtgttgttgaatacggctgactgcctgacctggaattgaggaaattaacagcagtttatcgataccggccagtgatttttccagcacctcctgcgaatcataggaccctggtcgagcttcaatacccggcaacagtttctcagccttctcagtgttccgtgccagtgcgatgatgtctcggttatcaacgttttcagctaacactttaatgacagtttgaccaaatttccccgtggcccctgtaacggcgtatttcatattggcgatcccctttcaaatcataatctgaacgactaaattatcctgtttaattgatgttaccaaggattggaggggcttacaagaatttgaacttggagaaattttcaataaaatccgattattcatgaaaattttcatgatgttcgatatactaaaatgaggtttttaactggaggacatgatgaaaaataatggctggtatcgattagggcaggttagtgcggtattctgcggtggcgcgctgggtgggatttcccgatatgaaattggaaactggatccatagtgccaatgggttgcttggaaccagcgttgtaaatttgctggggtgctttttactgacatttacaatctatggcctagatttgcggttcgatttacctgagtggcagattcttgggctcggaacgggattcgttggagctttcaccactttttcaacgtttactctgcagtttgtgcaggggatttccaataatcccttgggctcactgatcttcttactggtcaatctcattggtggcatgctttgtgtcccccttggctacttagcggctaccagagttgggaggcgtcagcgatgacaacgatgatctgggtaggactcggcgccggattgggggctgcttgccgctatgggataaccgttctgggcaaattagtatcgccgacgattccctacgcaacaattttaattaatgtgattggctcgtttctggctggatggttgactggaagtcagctaccgggaacttgggcgctatttttactgactggggtttgcggtggcttcaccacattttcaacgttttccgtcgatacgtttgtgcttgttcgcaatcgtcggtatctgcttgccggttggtattggtgcgggaccgttgtcttaggcgtgttggccgtggtttccggtttgtggttgagtatgcattcttagtgaacgtattttataatgagttgtacataaaagaggtgttttccattaataaacaaattttgcgcaacgacttacaaattatcgtaggggcgttggtctacgcaattgccattaatgattttctgattccacatcagatcggtgagggtggcgtcactggtttgacgaccattggctattacgcgttgaacattcccccggcggtgacgaattttgtcttgaacggaatcttaatgctggttggtttccgatttttggacaaaaagaccatctggtattccttgtgggccgtggcttggatatccatctttttgaaattacccagattgctgaattatcacacctcacaaactattattccagcaattgccggtggtgtcctaatggggatttcgatgtggattatattccgtggtgaaggcacgattgccggcagcaccattttggccaagatcatgaatcgttattttggcatgaaaaatgggtcggcaatgttgatgtttgatttatgcgttgcaattccatcggtgttggtgattggttttcaaaatatgattttgacggtgattgaactgtatatctctgcggtggttctcaatggtttgctgtcccgatttggggctcgaaaagccgtgaccattctttccaatcaaacggatgaaattacctcagagctctccagccagctccatcagggaattactctcattagtgccaagggatattatcaccaggaaatccggccgatgatttacgtgatttgtactgataagcaagtcgcccagattgtcccgctggtttccagtgttgatccagacgcgtttgtggtggttgagaatgtccatagcgtcaagggcgaggctttggagaaaatattataggagaagttccagattttgatcacaaatcgggaacttttttaatactcagtaaaatttaatttgaaaaatttgtgcaaacatgctgtgttgtcaaacgctttcatattcgttacactattatttgttgagctatatccgattaatccaataattttcgtggtgggggattattgattaataatcatattactaggcaggaccagtgaaaaatctgatctattttgtgttgtacttctcagaagggggaaaattatggacgcacaagtcgaaaaaccaaagaagcatttcaagctgaaaatgcccggtgcctttgtcattctgttcattttgacaatcgttgccgtggctgccacctggatggttcctgccggtagttattcaaaattatcgtacacgaattcatctttgcaggtaactgacccacacggtaaagtcaccacggttcccagcacccaaaaagaattagacaagctgggcgtcaaaattaacattaagcaatttacagatggcggcatcactgcgccggtatcaattccaaatacttaccagcgactcaaacagcggccggcaagcattgcggctgtcccgaccagcatggtcaaagggaccattgaagccgtcgatattatggtcttcatcctggttctgggaggcttgatcggagtcgtcaaagccagtggcgcctttgaatccggtctgctggccctgaccaagaagaccaaagggcatgagttcttgttgatcttcttcgttgccatcctgatggttctgggtggaaccctttgtgggatcgaagaagaagcggttgccttttatccaattctggtaccgattttcattgccatggggtacgattcgatcgtgtctgttggcgcaatcttcctagcgagttcgattggaacctgtttttcaaccatcaacccgttttccgtggtgattgcgtctaacgctgccggcatcgactttacccaaggtctgccggagcgggtcattggtttggtgattgctgccagttttgtcgtgacttatctgcactggtacagcaagaaggtcaaagctgatccaaagttttcctattcatatgatgaccgtgatgaatttaatgcaatgtgggaaattgccccaactggggaagatgccaaatccaaatttacaatgcgcaaaaaactgatcttgatattattcgttgttactttcccactgatggtttggggcgtgatgtctcaaggctggtggttcccaaccatggcggcttcgttcctgtcatttgcaattatcatcatgttcctaacggcaaccggtaaaaatgggcttggagaaacgggtgtcgttgatgctttcgtgaaaggtgcttccagcttggttggcgtttcgctgattattggcttggcacggggaatcaatcttgtgctgaataacgggaagatttctgacaccatgctccagtattcatcaaccttggttgcccatatgaacggcccaatgtttattgttgtgatgctgatcatcttcttcctgttaggattcatcgtcccatcttcatcaggcttggccgtgctgtcgatgccgattctggcaccgttggccgatacggttcacattccacgttacgtcgtggtaaccgcctatcagttcgggcagtatgcaatgctgttcctggccccaaccgggttggtgatggcaaccttgcaaatgctgaacatgaagtattcacactggctgcgtttcgtgtggccggtggttgtcttcgtcctcgtgtttggtggtgcattgctggtgactgaagttttgattaattaatatttaatacgtgaattcaaagtgcctccccgtcaggattgatggagaggcatttgcgctaattattaaacaacttccaacaaatccagtgacaaaccagctataataattaataatctgcacagtcacaaatcatgaggaggttcatcatgggaaaatatattatcagttcaaagcttagaaaagttggtgctcaagtcgacacaaaaacaggcattcatcaatttatcgttgatgaaccaattgccggtcacggaacagatgccggtcccaacccggtccaatatctgttatcggcggtcggcagctgtttagccattactgccaacgatatcgcccgaaagcacccggaaattcaaattaagaagtttgaaaccaagacgactggcgagaccactcagtatcaagatgggcgatccgcggtcactaaaattgtcgttcagattcatgccgaaacgaatttggacgaggctggacataaggcgtttatgcattcagtcgtcaaggactgtacggttcatgaaacgttaaagcacgcggttccgattgagttgcaattcatctaggaggggtactatgggaaagatccgaaaggtgtcgttaagtattggaattgtcatggttgcggtatttttggcggcttgtggcaagcagtcttcccaaaataatgcgcagaacaagtcgattaccttaatgcagacatctgatttaacgtcgttggacaataccaatcaggccatgctgccggagtttaacaccctaaccaacatttctgaggggctctaccggcttaacagcaaggatcaaccagtcccagcgatggccaccaagattgttaaaccaactgataacggtaaaaagtatgtctttcatatccgttcgaatgccaagtggagtaatggtgatcctgtaaaggcggaagattttgaatattcatggaaacggtctttgaaccctgcgaataacccggtttacacttatgtctttagtggaatcaaaaatgctgatgcgattatcaatcataagaagtcgtacaaaacgcttggaattaaggcaaccggcgacaaaactcttgaaattactttggatcatccgatggcctatttcaacaagttagtcgcaatgccggtcttcatgccgcaggataaatcgtttgtccaaaaggtcggtgttaaaaagtacgggactaacgccaaaaatacgatttccaacggcgccttcaagattaccaactggaccggcaccaacgatgcttatcgattggtaaagaacccgtattactgggataagtcggcgattaagttagaccaaatcaactataagaccgttaaggattccaatacggcccacaatttatttgaggatgggaagttggacgatgccaccatttccggggttaccgccaagtccctgcagaagaataaggacttgaagcgggtacctaaggcctggacttattatctgcaggttaaccaacggaaagggcgaccacttgctaaccaaaagttacgacaagccatttcattggcgatcaaccgaaaagaactgaccaataaggtcttggcggatgggtcactgccagccagcagttttgtcagcccaggaacagccgttgacccaacgactggtaaggatttcagtcaagagactagttttagtgtcgcgcccaacatcaagcaagccagaagtttgctggcagccggtaagaaggaagccgggattactggtgatttgaagctttccattgttggtgatggtcaagatgtaaccaagaatgttgctcagtatatccagggacagttagattctaagctccctggtgtcaaggttagtatcgccaaccttcctgacaaagctcagcaggcccgccgaagtgaaggcaagtttgaccttgctcagtggtactggttagccgattttggtgatccgatcaattacttgggaatcttgacttctaataatacgatgaatccgggcaagtttagcgatgccacgtacgattcactgattgaaaaagccaagacagccgctaatcagactgattactggaaatatctcagacaagctgagaagcgattgatgaaccaaaacggcatcattccgctgtattatgtaagagaaagccatttggtcaacccgaaactcagcggggttgagtatcatgtcgctgggttcccagattatacgcgggcaacgattacgaagtaagttgctgaaaaattgataatcgattttaaaagtaggagtgctagctcgattcagacacaatctgcattgagacaacatttctgaacagaaccccttgaattggatttttccagttcaaggggttctatttatcaaatatattttaaattcatgcgtaattccggtcagagaaccattgccagaaggctctctttgccgaatatatggtgattctagttaaatacatagaccttactttcataaggacgtaattccgtaccttgatcattatcgtaattgctgatgacgagtttgtcggctttaccctgaccataatctcgcgtcaccgtgtcggcagtgaagttactgattactagcaacgtcttgccttgataatgacgccggtaagcaaagacctctgcgtcatcaggatcaatctcatcatagcttccgaacttaaccaagtcggaatcatgacggagctgaatcagcttttgatagtggtaaaagacggaatctttatcgtccaccacagctttagcattgatttctttataggttgggttcaaagcaaaccatggttttgcatctgagaagccggcatttttgccatcgtcccacggcattggcgtacgagcattatctcgagaaatgttagctaaatatttcagcatggttggcccatcgactagattcttttcttcaaccaactcgtgataggcattgattgattcgagatcttcgtactgatcaatgctggtgtagtgtacattggccataccgagttcttcaccttcaaagacaaatggtgttccttgcatcatgtgaagggtcgtgcccagcattttggcggcgcgaacccggtactttggatcatcgttggcgaagcgcgaaaccgctcgcggttgatcatggttgttccagtagagactattccaaccctttccatctaaggctttttgccaacgggatagggcattcttcaactctggtagcttgaccggctgatcgttccatttacccaagcgtttgtctggattgggttccaaggcaacgtgctggaattgaaagaccatgttcagttcatggctatcgaggccagtgtagttgatggcatcttcgggctttgaactcggcatttcaccaaccgtcatgacatcgtagtgggaaagtaccttttggttcatttcgtggagatagtcgtttaacttaggaccatcggcaaccagaccttccgtgagcgggtaggtgccgggctcaggtgcgtccggcaggccttcaggtttggaaatcaggttgatgacgtccattctgaagccatcaattcctttatccaaccaaaatcgcatgatgttccaaacggattcccgaacggctgggttttcccaattcaaatcaggttggccaggggcaaacaagtgcaggtagtactggccacgttctggaacgtatgtccaagcactgccaccaaaggctgcgtgccagttgtttggctcatgaccgtcaactggatcgtgccacatatagtagtcagcgtacttgttatccttggattgtttgctttcttggaaccagcggtgttgatcggaagtgtggttaaccacgaggtccatcagtaacttcaatccgtgggcatgaacttctttcaacagttcatcgaaatcagccatcgtgccatattccggtaagattttctcgtaatcggcaatgtcgtagccgttatctttgagaggtgattgataaattgggttcaaccaaaggacgtcaacgccaagcttctttaaatagggcaggcgtttgatgatcccatgaagatcaccaatcccatcattgttgctgtcttgaaaactttgtggataaatctggtaaattacgtcgttttgccaccattttttggtcatattgcattctcttctttctcgtgattatagtttaaccggtttacttagttttgagtggataaagccaactgaaaatgcagcgattactaatgaaaccccgccaaccaagaacattgctggcattgagtgcccaaccattgggaagatgaagaagctgcaaagagatgctgcaatttgtggtaagcagattgaacaattgaagagtcccaggtaagctccttcattttcaccgttcaaagcctctgttaagagtgagaatggttgggtgttcatggtgatataagtgatcccaatcagacagaacggcaaaatgagcagccatttgatgtggatgaagaagatcatgatgaagccaagggcaccagcaagtaggccaaagacataccatgcttttcgatgttctggctttgtccgtgcttgaaccagcaaaccaaagataaccgaagcaacggcctggatgcaggtaaggacgccataccaattaccagcggcttgataaccggctgatgaagggttggatgtgtgccaaacattgagggaaatggcaccagcagcgtaggtccaagaatagagaatggcaaaccaggtaaaaaattggacaattgagatttcccagaagactcggggggcttttttagttaattcccaaagactaggctgcttcttttgcttggttaagtcaatattgtgatataaagcatattcttcaggattgtattcgtgaactttggcaatcgtgtaaaacgaggtcaataacagaacggctgcggccaggtagtaggctaatttaacggtaattggcacttcacctttttgagcgacgtttgaaaggccaatgaatgcaaggaaaaatggaaccaagctggcaagaactccaccaagattggagaaggactgctgccaagaccaagccatatctttttggtcttcgttgaccatgtcaccgatgatcatcttgaagggctgcatacaaacgttggatgaaaggtccataaatagtgtggcaatagcggcaaaccacagtgcggccgccgaaccgtaaccgaatccgaatgaaccggcgttaggaagtaataccaaaacaattgctgcgacgggtgcgccaataaataaatacggcatgcgtcttccaaaacgggtccaagtgcggtcagagtatttaccgattaagggttgaataaccattccggctaacggtggcaagataaagaaaaatcctaagttattcgggttagcgccaatagtttgaaaaattcgccccatttgtgattgttgaagcgagaatgccatgttaaccccgaaaaaaccaaatgtcattgcaaaaatcgtacttactttcaaacttggcaaatgggatgcaaaacttttaggttcagttttaacgtcaccatttccagcttttacttttgcgtccatagtaattcctcctaaaaagtgagcggatccaggcggttagggatcggagtgtaagtctcttcggcagaaagctcagttctggaattttttgtcgaaaacacttatatgtagatcgctgcttggataagctatctccgtgaacgcttttgcaacttggccaatagatatatattgcaagaaaacgtttacagcgattataatagcacccaaagaaaacgtttgcaaaccctttatatcaataacacaaacgattgtgttttactaaaaattaaagtgacgtttactgtgctaaaatggggtgagcattgtaaaacgcttaacgttaatgatcccagtaaagctttacaacgtacataatagagaggtggcgtaatcatggcagtcacaattaaagatattgccaaacaggcaggtgtctctactgccactgtttcaagggtgttgtctgaccagacagcattttactcagaaaagacagcaaaaaaggtaaaaaaacagccaaaaaacttggctatcaaaaaaatacggctgccgttgaactggttacccgtcgcagcaaggtgatcgcagtcattctcagctcaaccaaatcaaacttttctgatcagattatcaatggtattcagcaagaggcccgccggcatgatttgaacgtgattatcgtatttgccggcgaaaatgattcccagatggagcgaaaagcattggaaaccgtgatcgagcggtcagtaatggggattttgctggtcgccgttaaccttaatccggctaacgaggacttgttactgaatgccaatattccgtttctgttcctgtcaatcaccattaaaaatcggggattgccgttcattacctccgacgattttcagatcggctatcaagccaccaagtatttgattgataaggatcattccaagattggatttgccgctgcagatttagactctgtgaccggtcagttgaggttggatggttatcgtcatgccttggcagacaatgggttacctttgaattcaggttgggttttgggcggtgactttgcctatgaagatggcgttaatgccatgaaacaatatggccgtgagccggaagtgaccgcggtgatcgcatcgagtgacttggccgcaatcggcgtgatgaatcaggcgcgggattatggattaaaaataccggctgacctagctgtgatgagcattgatggtacgaaactttgtggcatcgtgcggccacaattaaccagtgtcactcaggagttcttggagatgggagttcgggggatgcagcagattatcagtccgctagcaaaagctgccaagtcatcctttaccccatttaaaattattccaaggcagagtgtctaggaccgccatacaaagaagcaacccgaaactcagcggggttgattatcatgtcgttgggttcccagattatacgcgggcaacgattgcgaagtaaattattttaaaagtttgtaacaaaataagaagcctcagttcaatgcggacgtgtgtctgaatcgaactggggcttcttattttgtccataaaggcttgaatgctggatttcaattttatgcgaatagaaattcttagcattaccgattaggcgatattctttgaacctcgccgtcgaatgaggatccagccacctgccaagatgatcagtgaaataacgacggccacgacaaacaaatgttggtaagcttgctgggcaatttggtaaaaggtggctaatttgtcggagtgcgatccggctgcttttgctaataaaatccgatagtattcctcaagcggtgtgctcagcgacagacgactaaatccgctttggatgatggtcgcataaatggttggcgcaattgtcaggcccacttgacggctgacagacaacgttccaaacgcaatcccattatcggcttggtcggcgaattgggccatcaaaacggaaagctgggcgcccatcagcatgccgaatccaaagccagccaacgttgaggtagctaagaaccaaccggctgctgaaagaccaccggaaacgatgactgtttttgttgctccgagtcgggatactaaagtcccaccaatgcctgcgcctaagatggaccccaaaccaataccactcatccaaataccactgttattggccgaaatgccgtaaacttgttcgacaaagctgggaatgaagacgaaaattgcaatcaacatgccagatagcagtcccatcaacagggttagtaaaaatcctttattggccaaaagatggtagggcaagaaagggtcaaatcgtggcgcaatccgtttttcgaccaacacaaatcccacaaacaagccaatcccaaccaatcctgcaccccaaacctgaggggttaacaaacttacgagaaggtggccgctttgtaagttagtaatggctaacatgatgctaaagatacctaaactcaggatcgtcaggccctttaagtctagtgatttcacatgggatccaatggtttctggaatcaccagccagccggcgacgatcacaaagatggcgatctgcagattaatcagaaacaaccaattccagcgcccagtcaaatttaaaatcaaactacccaaattaggaccaacaaccgatgctatgccgttaactgcacccaaggctcctaacagtccgccctgggctttcttggggtaagttgataggacatgacttgaagcaatcacgaagattcccccgccaccgacagattgaatcatccgcgccactaaaaacgtcatgttggactcaaagcaaccaataatgatcctagttcaaaaatagcaatttcaattaaaaacaattttcgtctgccaaatttatcagctaattttccaataatcggggtcgcaattgccattccaagcgtataaagcgtgatcccccatgttccttgtacttcgctaatatgaagtgaataattaatacttgataatgcactggcaataatcccattatccaaggcagacatgaagacccctaagattaaaatgcccattgcaaactttgagtgttgctttcctgttcccatttttctgatcctccacattaggtcctattccattaattatcgtaagtgacattgtgtcacttaactattgatgaaattataacacactaatgacaccgtgtcattagtgtgagttgggaactatttcaagcagcggatggcattcatattgaatgaattgatgaagtatgaacaaaatattttagaagtgaggtaaggtgattatgtcagactggttgtgtgacggaagaatccccaagtgacaatgtttctctatattcctcggcatctggattttcatgaaaatcgacagtgacatcttgatattgttttaattctttttcaatttcttcaattggtattttaaagtattcctttcgattattaaccttatttactcgattgttagcaaattgattgtgcaatttggactctaaggcataggcgttttcactaaaaattaaagcatgtacatcaaatttgaacggtactgaggcactactaagttcattaattcggtctaatggctcgagacgccgtgttacacctattttaacaatatcctttccaaatgaaccaatgttggaaatgatatagacgtatccggcagtggcatttgattcccgataatctatgccactctttttctcgcggaggccatctagcttttgctgaagattttgtatttctgcccttaacccttcctcatcagtattttctaggggcattctgttttctaattcttgaattgcttgactatagtgttgaatttctttatcaaccttttttcgttcctgtttaatttcttgttggagttttttctcttcacgttctttttctctttgttcacggagtaagtctttttcctcctgctttttttgagcatactcgaatgccaaatttaattcctcatatttcagttttaggtaactaggttgcatttgtacattaacaacttcatacatcttattgtgttgcaagaatgatttttcgattctttttgctaccctttcataatttgaataagtgactttattaattgcatctgtgcattcattattaaaacttctaaaaatagctttaatattattctttgtcattttctttccttgggataatttgccatttactgtccacatggtatcaaaacttaccgcagttcgattcttaatggcttgcttttgctgatctcgtattgcattgagtgcctctttgtatcccaacgatgttgcaaattcatagtggggtgtatacaacccaaaactactcatttctttgctagcctctagttctccaacttcagcctgtaagttttccacctcttgctgtaactgtgcaacccgatttttcagatcttctgcctgtggggtaaggctttgtattatgccagatttttcatcaattaacgattcgagctcaacaggtttcatctgctgaactgaaagtttaattttgagtgacttctgtaagccctcgttttgtgaagttaagttatcattggttatcttaagttcgttaatttgttgtttgaattccttaattttaaacaagtcagaaattgccatgtatttatcctccagtaatgtgagattatttattcaaagttaattttagtgtatcaggtggataaggagacagctaggataaactctgtgtattcgcctgagtaagcacttccattcgattgttaaaccggatatactacagatatagtgagtatttgagcaaacagaaggaggtcatcttatgaaaattgcaacagcagttgcccagcaacagggcacaaaattgacagttgaatcggcagagttggatgaacctaaggcaaatgaagtgttagtcgaaatcaaagcatccggaatttgtcataccgatgctgctggcagggactttgccaccaccccgtatccagttgcattgggacatgaaggagcagggatcgtcaaagaagttggcagcagtgttaccactgtcaaacctggagatcacgttgtcttgtcattttcttattgcggtcattgcgaaaactgtttaactgggcatccagctaactgcatccacttgaatgaacttaattttggcggtcacaattttgatggcacccaccgtattcatagtgaagatggcaagaatatttctacattttttggccaatcctcattctccacgtactcagttgtcgacgagcatggtgtgaccaaggtaccaagtgatgtcgatattaatttgcttggcccattgggatgtggatttcaaactggagctgggacggttttaaattatttgaagcccgaattcggcagctctattgctatttttgggactggagcagttggattgtctgcaatgatggccgctaaaattattggaatggatcatattattgcgattgatattcacgataatcggttggaactggcgaagaagcttggggcaactgaaaccattaatagtcagaaacataatccggaagaggttattaaaacactcttgcaagctggcattgagtacagcattgatacaaccggtgttcctgctgttattaagcaggccgttcatgtattaaagccatccggaacttgtgctttactgggtatggctggtgatgtcactttcaatatccaagaagaagtaatgggtgaatcgaaacgagtcgttggggttatcgaaggcgacgccatcccacaattatttattcccaaactggtcaactactacaaaaagggcttattcccatttgacagactggtaaaatattataagtttgccgatatcaatcaagccttcgaggactcagccgacggcagtgtcatcaaacctatcgtaaaaattagcaactaaaaaagtagaaacgctggctcaatgtggattgaaatccatatcgaaccagcgtttctatttttgcagaagattatctttcccaaccacacaaccgatagccatggctgcgggcccaatgcttggtcacgtggcgcttgtaaccggcgttactcaggccacggcaagtctttgagtagtgatatcgtttgccgtggtttggcgcgatccaaacataggtggttctggccgaaacttcttggggcggaattgacattaatccgccgcccatcgtgaatgctgcaacaactgtcaaagttgctttcttaagctttaacatgatgtttcccccgaaatataaaatatgtgaataatagcacaaaaatagtttaccataaattatcaggtattaatatcacaatattaatatttctataaggaaaatcgctaattatcctggataattttgccaattcgttcctgcaagtccggcacgacgtccgtcaaaaaccagggatgctgcttcatccagccatagtttaatggtgagggatggaccaaaggaaaatagtccggcaaatagtcttcgaagtggcaaactgtttcagttaagtttctttggcgccgatttcctaaataatatttttgagcatattggccaattaataatttcagtttgatattcggcatctctgccaatagcggttggtgccacttttcggcgaagccttttcgcggtggcaaatccccgtgggcgcctttcccgggatagtaaaagtccagcggcatgacggcaattttgcctgaatgataaaattctgtcttgcttaatcccatccagtcccgcagccggtcgccactcgggtcatcccaaaagaccatcgatgcttgggccttgcgactgggtgcctgactgataatcaagatttctgcttggggatcaacgtggaacaacggctgaatgccttgttcggtgaacgactgattttgtgggtcgtcttgaatctgcttaaatagttccgcaactgtggccatgagatcacctcgttctgacttttaccttcattttccaccaaataattatcctgtcaaagcaaattcaccattaacaaggaccaatggcgtaaaataaccttagctaaaagaatccgaagggggaaagggcaaatgggccaaaagacaatctattttctctgcactggtaattcctgcagaagccaaatggcggaaggttttggcaaacaatatttgggtgaccactatcgggtattgtcagctggaatggaaaagcacggcgtcaatccactggccgttcaagtcatggccgaagtgggcgttgatatttctgggcaaacctccaagctgattgacccgacaattttaaaccacgctgacttggtggtcacgctgtgcagtgatgccgagaaacgttgtccgataacgccaccgcaagtcgctcgtcaacattggccattccctgatccggccgtggcaactggcagttccagtgaacgattacaggccttccgagaagttcgcgatgggatcaaggcgcggattattgcctttgacaatcttgaggccggccaaaaaaatcattagtttaggcactgttatatcagccgttcacgccaccgaccccaaaaatgtccttgcaatctgcataatcgatgctaatattagtattaaattaaaacattaagcgatgatgagaagagtagcaagtatcctttggtaaagagagccgcgttaggtgagaggcggtcaaagtcaatcttgtgaagatgagctcagagcattaggcacgtgcaagcgatgcctacgttaagacacgttacgatctcagacttaattaaccaatttggttaacgagttgtgaaggtggccgattgtgaaatcgaccataaaactgggtggcaccacgtgtttacgtccctgcagtatttaactgcaggggcgtttttttgttgggataaatgaaatccagttatttgtctccggagtgctcttacgtcatccaaggaggacgaacaatgttagcagcagaaaaaattgaggttaataaagacggcactagacgaggattatccaacctggccgtacaaatgattgcttttggcggttcaattggtaccggcctgtttcttggcgccggtagtacgattcatcgaaccggtccatcgatcatcctggtctatctggtcattggcatctttttctttttgatgatgagggcgattggtgagatgatgtattctgatcctgagcagcatacctttgtgtcgtttattggcaaatacgtcaacgaacgcttgggcaaatttgcggcatggagctactggctggaactcatcctagccggaatggccgaacttacagccatttcaacctatgtcaaatattggttccccgatgtcccggcaccgttaatccaagtcgcattcctggtgatcttgagtggggtcaatttggcgatggtcagttcctttggcaggtctgaaacctttctatcaggaatcaaagtcattgcgatcttagccctgattgtcatcggcgtctatctggtctttacccatcatcaaaatcccgccggcacccacgcctcttggggcaacctgaccgatggtttcacgatgtttccaaacgggattcatcaatttatcatggcttttccaatggtcttcttcgcctttcagggaatggagtttgtcggcatcacgaccgcagaaactaagaatcctcggcgggtattgcccaaagcagttaaccaaatcatcgctagaattttactcttctacattggttcattaatcattatcatggcgatcaccccatggaagacgttgaatcccaatcaaagtccgttcgtccaaatctttaatttagccgggatccccggtgcctcggcagtaatcaacctggtagtaatcgctgcggcaatgtcgactttaaacagtgccattttttccaccggccgacatttgtatcagctggctcaggagtcccactctaaggaaatgaagccgttccaaaaggtttccaagagcggcatcccaattgtcagcgtcctcttttcggcggggatgatgcttttggcacccgtaattagttcctttaactcgcttggtgcagccttttcattcattgcctcagtttccagcgatatttatattctggtgtgcatgctgacaatggtggcccactggaagtatcgtcattccaaggactttcggccggatggctttaagatgcccaaatatcgttggtctaatcccttaacaattgcctttttcattgccattttcgccagcctgttcttcagtcatgattcactgttgccggcagtcggcgctgtgatctgggccttggtattctatgcggtcttgcggcggcggaataccgagaatttgggcgttgaagacagtagtgactgattttgaatagaccggcgattcagcttcctgtatgatggacttaacatacaaggaggatgaaatcgtgaaaaatgtttactttgaccatgacggtaacgtcgatgatttggtgtcgttattactcttattgcaaatgcccgaagttaatttgattggcgtgggggtgattgatgctgacggctacattgaaggatcggttccagcttcacgaaaaattatcacccgattcggcaacggcgctcaggtgtcagttgcggcttccaactctcgcgctgttcatcaatttcctaaagaatggcggctcagctcgttttccttcgatgctttcccgctgctcaacgaacacggcggaccaaccacgccgttggctgagaaaccagctcacttggatatgattgacaagcttaagcaggctgacggcaaaactgacttggtgatgaccgggccattgactgatttggcaagggcgcttgaagtcgaccctacgattgttgataacatccagcggctatacaggatgggtggcacgatgcggacagagggcaatgttttggagcccaaacatgacgggaccgctgaatggaacgcttattgggatcctgaagccgttaagacagtctttgatgccgacatcgatatccaaatggtcggactggaaagcaccaaccaagtgccattaaaagccgacgtccagcagcattgggccagcttacggcgttacccaatgatggacctgatcggtcaaggctatgcgttggtatcatcttatgaagctaactcaacctactacctgtgggatgtgttgacgacggtggccagccaataccctgacttgattcagtcaaaggacattcatggtgatgtcttgaccacgggtgccggagcgggtcgcacgtttgagactgataacggccggctgattaacctcgtcactgaagttgacggccaggccttttatgacaaatttgatgaattactgactcagggtcattaaaaattgaaaatgtgaatcgatgaacaatcgcctccaatatggtagactcagcgtagagaacgttgacttatcaatttggaggcgattttatgtcgacacttaaaatgaaggacattaaggtaattgccaatattggcgcgggaaccatggggcatgctacggcattacagtttgcgatgaacggttatccagttaatctcctggatatgaatcaagcggctttaaaacatgggatggaattgattgaacacgatctagccacttttgaagaaaacgggctgattaaaggcaaccagaaggcggatattttggcgcggattgtgccgaccaccgattattctgacgccttggcagatgcagatttcgtgattgaatcagttgtggaaaagttagccgtgaaaaagaccgtttggcagaaagttgaacactatgtttccgaagatgccagtatggcgaccaacacttcgggacttagtccaactgccattcaagctgatctaaagcggccggagaacttggtggtgactcatttctggaacccggcacagttaatgccgttggtcgaagttgttccaggtgagcagacgtcagaagcgaccgtcaagaccgcaacggccttaatgaaccacatcggtaaacacgctgtcgctctgaagaaggaatcgctggggtttgttggcaatcgaattcagatggcggttttgcgggaagccttcaagattgtcgacgatggcattgccagtccggaagcggttgatgacatcatcaaatacagtttgggccgtcgttggagtctggtcgggccaatcgccagtgcagacttgggcggtttggatatctttgaaaatatcagcagttacctctacgatgatttagccaataataccggcaccgacccagtcttgaagaaactggtggacgccgggaacctgggattgaagtctggccagggattctacaattgggaaggcgatatgggtaaggaagccattgcccatcgagatcaggccttattgcaattattggtggaggatcaaaagaagcgctaagagatgttacacgtgaaacaaccaagtgacaggggaaatggttgaaccctgccatgcttgaatcttcaaaatacctaagaaccaaaaatggcatctatttctatgatttagaaataggtgcctacttaatgctatctaacttgactttcattttcattgtcctttagtaactgagttccaaaagagtcggttgctttcactggtttgcagattgccggcatcttgaaccttcttggcaaatacacgttccaacatcttcttcaaagttttcttcatattacatgccctccctgtgttcaatctaagagtcattaatggtgtgatatcaaggattcaattcagttgattgagacacttttctttgactccacctttagtatagggcataaaatattacatttgaaatgttttgctcatgaatttgtaaaataattcatgaaagtgcaatgtatgcgtttacattagcccaagcgattcattgaaaaattttacgattcaggacaggggaatccttttaacatccttgtcagtttgtgggcagcctgcgatcggcaaagaaaaaagcacaacgccatcagcgctgtgccaagtgcccccacacttgtgatgaactaaatgctctaaacttgattcgatacatatctcttggatgatccccaataacgtttgagcgatactccccggctgatagctgttaagccatcgcttgtgatccgtgggacgagtgatgattactgaatacctgccctgttcacagggttattgtacgataatgtgaagaaatatacaagaagaatttgaattgacagcccatggttagcaaaagtaacgctcaatccctactggtgactaaatgcccagtttccaagaagtgataatttccataatcgccatcacgaccatggttgcgccaaagatctgcagtaataccagaattgtgccaaacggattaaatgccagcaggatgccaactaggatcagtaacacaccatacaacacaaatggcattggcgaaacattgacgtattgacgatgattgagcgccgtgaagacgttggaaatgcccgtgacgatcaggacaatccccaagataaatggcaaaaatgacaagagtggttctgccaataagaagacgatcacggcaacgattaactgagtaatgccgaccgccagactatagtcgaccacttcgttatttcgccgctgccgccaagcagagattaaattgatcaccccaaagacaatgaagaaagccgcaattaaattaatggcgatattcaacgtgtcgtgtgggtcaaacaggaacagcaggccgaagactatgtaagcgatacttttcagccaaatataatttctaatctgattaatgaatgaatacatctgaattccccctcaagactcatattacctatataatactagtaataagtttaaaacgacagtctcgaggtgcgtgatgcaatatcctaatgttcatttggccaaattcattgatcgacccaaccgattcatttctcattgtcggctgatcgaaactggtgaagtcgtgaccgttcacgtgaaaaataccggccggacaacgattctccaacctggggtgacgacggcgctggtgcataatgacaatcccaaccgcaagacagcctacgatctggtggccgccaagaagtacgatcgccaatggatcaacattgattctcaggcgccgaataaagtggttaaatcagggttaatcagcaactacattcaactgccgggaatcgaatcgattgcgaccgttaacccggagacgacctatttggactcccggttggatttttccggaaccggcgatttgggccaacgattcttcctggaagtcaaaggggtgaccttggccaatcaagggattgctgcattcccggatgcgcccaccacccgtggattaaagcacgtgttgaccctggaaagggcggctcaggctggatatttcgcttatttattatttgtcatccaaatgaaaaatattcataaaatgactattgaccgcgatatttttaatgacttagcgttggcaattgcaaaggcccaaaacaatggcgttcacgtcctggcctatgactgtcaggtcgaaccgggatccttaacgttggaccagccaattctatttgatttggatcagccatttgtcagtgatgggctgccgtcatcaattggtcatatttgaaagattgacagttcttggttcaaattcccttgaatgtctccacagtcgtgttattatgataggcgcattagtgcgagtgctgcattgttgatcgcacatacttgatttatttggaaggaagcaattttacacacaatggtaagtaaaacattgatcttcggccaccgaggctatccccatatgttccccgagaattctttgaagggctttgcgtacgcgattgatcacggcatcgatggtttggaatttgatgtccatttaactaaggataacgttccagtgattatgcatgatgaaaaaatcgatcgaaccacggatggaaccggcgagattcgctcatataccttaaagcagcttcgtgagttccatttgagtgatggtgagacggttccaatgctcaaagagttattgacgctggcaaatggccaaccggttcatttgaacttggagttcaagaccaacgaaatccactatgacaatattgaacagatcgtgctggacatggtgaagcaatacgacttggtctatccggtcatctactcatcatttaacctcgactccctcaaaattgcttacaaacttgatccgactcagcaatattgctacctgtcggaagaagatattaaaaatccccgtgagttgatggcaaaggaacacttggtgggcttgcacttgagccactatgtcccaatgcgtcacgtgaaggaacgaatctggactgttgatgaccccaaagtgcaaaagcatttgtttgggctcaacgttgccggtattttcaccaataactttgaaggtgctgaaaaaattaaagcaaacgtcactgcttaatctgatcatttcaactgcatttccatgacactgagtgttgtggggatgcttttttattgtcttggatccgtgagccaactgttcagaaaatcactgttttcgtgctaaaatcgattcatagagcaccatgaggacactgagggggatggatgagatgagtaaatggattcgtagatttttagttggttttgtggccttattttcactggctttgtttaattcagcagccgcttcgaccgtcgatgccttcgggacgatttttgaaaatatgattatggcgaaccgaatgaaaccgacggccctgaaagccaattcgaccgcgagcttcgatattgtcatgaagccacaggactcgaccgcttattatcaaaaggcgttggatgtcaatgatccaaccaaggctgattttaaggattatctcagcacttcggatattcgccagcagtttggccagcctgatgccgtcatcaatgggtgggttgccttgtttaaaaagaatcatctgaccactcacgtttaccaggacggattggtgttgaatgtgcaggggaagaccaaggatgtgaatcgcctgttcaaaacgaatttgagcgatgccacctatcactcggacccactacagtttggcaaatccaaacccagcattcccgccaacctgcaagactccgttctggcagtgatgggaatggccgatcataacaagaaattctggttcccggattctgacgttacctttaagagtacccctaaagcgactaaagcactggctgataaaaatgccggctataccagtcattttacgaaaacctatggcgttgatcagctttacgaccaaggcctaacaggcaagggccagacgattggcctggtttcttttggcaatgtccaaaccggtgacctcacgcacttttggcggcatgaacatgtaaatgcatccaagtcccggttccaaatggtgaaagttcttggtgataattatcggaaagatattaaatcgaccagcgacggagaagccacgatggatgctgaatatgccggatctgtggcgcctgaagccaacattaaaatgtttaatagtggctcagtaattccaacgttaatcaatctcatcaatacttacttaacggcctatgacgatggcagtgtcgaccagatttccagcagttgggggatggggcccaacaactacttccagattttggagaaaatgaatttattgccatcccaatacgttgaggtgttgaatctggtgcttgctcaatcggcactgcaggggatttccaattttgtcgcttccggtgacagcggtgccttgaactacaccgtggtcggcattcatggaaatgatgttttgttggatcggaaaattagtgacgctgatccgtataccactagtccttggatcacctcggccggcggaaccagcttaccgtttaagcagtccgttgctccaaacggcaaatcaattggcacaatctccaaccaaaagcaacgagcttggggcagcgattattggtggccgttccttcaggttaacgatgattacctgctgacaatgcctgaattcttcaacgacattagtgatggcggtggcggcgggttcagtcacgtctaccagacgccggcctatcaagaaggcgttcccggtgtgaatacctttaatgcccgcgagtatctgtcgcaattaagtggcccagtctataacgcaccactagtttccggaactgatgatggtcgaaactacccagatatctcagcgaatgcagatgcgactaccggttacttcacgtatcaaaagacgagcacctctaatggctgggagataagcgggggaaccagcattgtttcaccacagtttgcgggggtggcagcgttgattaacagtcaaactgaccatgcgcgaatgggattctggaatccacagctgtatcaactggcaaccaaatcggattcaccactgcaaccactgaacgacactgagaataattcaaatctgtattatactggccaacccaataccgtctataatcaggcaagcgggttgggaaccgttgattttgcaaagttgatggatgtttacaagtgatgtaattgatagtgatataaaaagtgcaaaccgaaaacgcggtttgcacttttttgtgctctaagacggtgacggatgaagctctattcttcgtcagggctatatttcaaaatatctccaggttggcagtccaacgctttacagagtttctcaagggtactgaatcggattgctttagccttacccgtttttaagatggaaacattggtgggagtaatgcccactttcttggctagttcaccagtcgaaatatttctttcggccatgacaacattaagggtaattttgatcaattagatttcccccttccttaaacggtgaggtcgttttcttgcttaatattcattgccattctaaacaacgtgtagattaatgcgacaaacaccaacataaccgcatcatccagcaaattttcccaggtactattgaatataccattgttgactcggcccaagaatgactgggtcatttgatttccgatggcaagaaacacatctgagcagattgccataatttgggaatgaacgattctgcgcagcattgccaaattatcagccacaaagtattgttttttccccaagttgtgactgattcgaataaatgctgaaagggcaaacagggcagagaggatggctaagaagatcccaatcgccattaagatcgagtatggaagaattggaaaatgggcgacagcgctgtgagctacttgggtgtgtccaggaacaatcaagaaatcgccgttgtcggcaatcattttcataatattggcatgggtgaagccgttatacaagtaaacaaacggcgtaatgaaactgaagcagacaacaacgaaggcgatctgcatcaggacggaaacggcaccaatactgcgatctaataattttgacatggatatcagcctctctcttttaatctggattaattaactgtatcgaatatatcatatcgataaacgaatatcaatatctatttttcgataaaatatatttgaaattcatttgaatttattcgatggtcaatatatgaatgtcaaaaaattggctggcaggttggactttgagtggctaatatatggttataccacaatcaatttggtcttatacaaaagcaaaatgaaatttttacattcattatcatttttttactttcaatttacattaacgaaactggcaatttacattgaaccctcacaataaatcttgtaacgaaataaatgattttgaggtgagataattgtcaattactttaagaaatgtccgcaaagattatgatgcgcagacagaagtcctaaaagatatttcggtgaaagtcgaaactggcgagttcttcgtcatcgttggcccatccggatgtggtaaaagtacactacttagaatgatcgccggattaacaccgattaccgccggcgaagtcagtatcaatgacaaggtcgttaatgacttgccgccaaaggctcggaaattaacgatggtctttcaaaattatgccctgttcccatttatgaatgtccgagataacgttgcttttggtttgaaggcccgcaagatggaccaagcagatattaagcagcgggtcgacgaagccttaaaaatggttaacttaactgaactcgcgaaccgcaaaccccgtgagctatccggtggtcaacgacagcgagtggcattagcccgggcggttgccagtgatgccaagatttgtctgatggatgaaccactatccaacttggatgcccaactaagaattaagatgcgccaagaaatttatgccctgcaacgcaaactgggtctgacactgatttatgtcacccatgatcaagttgaagcaatgaccatggccgaccacatcatggtcctgaatgacaaacacgttcaacagattggaacgccaagtgagatttatcaaaacccggcaaatgattttgttgccaagttcttcggtaccccacagattaacattctgaatgcccagcgttcgcaaaacgataaccatgttttgaatgtttcttctgatttggaaattgctttggatgaagaagttcccgctgaaaatgtgaagattgggattcgtcctgacgatatgaaggctgaagcggctgaaagcgttgaagccaacgccaccgttaagaacaccgaattcttaggggacgaaactattatctacgccaccttgaatagtggcgaagacattcacgtcgttgtccctggccaggtcaattaccgtattttccagccaatcaaagtttccgcagattccaacctgatgttttttgatacagaaggcaagcggatgaacctttcaaaggaggcctatgttcatgcttaaatctccagcacaaagcacaccgacaagcccggtttcggttgagaaaaccaaaagcaagcttgccgaacaggaagccaagttcacattaaatgccaaggataagtattttgcctgggcatttctgggaccgtcacttttgatcttgggcgttttcattttctacccaatggttaagacactttatctgagtttgttcctcaccaacacggttggtaagccaacggttttcgttgggatttccaattacatcaacttattgacttcagctgattatctatccagccttggggtcacgttattctacgttttcgcggtgaccattatcacgatcgctttgggattggttctcgcaaacctggctagcaaacggctgccgggaattggcctttttcgaacactattttcggcaactatgggagtttccgtttccgttgccgccatcttctggctatttatttttaacccatcaactggattcctttctctgattagcacctggatgcatctaccacaaattccttggctgactgatccaactgctgcaatgtgggcggtcatcatcaccaccgtttggatgaacctgggctttaccttcttgattttgctaggtgccatgtcatctgtaccaacgactttgtacgaagccgccaacattgaaggcgcctcatcaagatttcagttcttccacatcacaatcccatccatttcgccaaccctgttctttgtttccatcattactttgatcgaatcatttaagagctttgggttgattgacctgatgactaaaggtgggccgaccaacgctactaacatgttggtttatcgaatttacaaggatgcgttctacagcggtaactacgcgcaagccagcgccgaatcgatcatcttaacgatcatcattgcgctgttcacgctcctgcaatttaaagttttggaaaagcgggtgaattactaatggatcttgtgaccaagccaaaattgtcccggcgaatttgggactacgctttattaacgattctcgcagtgattgttctggcaccgtttctgattggtttgtggaccagttttctgccaaccatgcagatcgcgcagggaaacttcttaagcaccaaggtttccttccagaattacattgatgcctttacccagacgccaattctcagatacctgggaaatagtttggtaatttccacggcaaccatgattgcccaactgatcttttgttcgatgagtgcctacgcctttgtgttcctgaaattcaaagggcgcaaattcctctttggcctgttcttggcaaccatgatgctgccatttgaagccgaaattattcccaacttccagaccgttaaggccatgggactgctcaacagctactccgttatggtgattccatttctgacatcggcattcggagtctttatgctccgtcaatcatttatgcagatgccgattgaacttaaagaagccgccgatattgaaggcttgggccacttccagttctattggaaaatggtcctgccttataaccgaattccactgatgactttaggtgcctacagtttcctgggcgcttggaaccaatatctgtggccaatgttgacaactttcagcaatgatttccgaccagtccagaacggattgcgccaacttcagtcagaagaaacctttaacgactggggcatgattcaagccacagctgcaatcgttgtgattcccacgctgattgtgctgttcatcggtcagcattacttcaaatctggtgtgaatgaaggtgcggttaaataatgaaaagagtaacagcatttctcaaaacatacgcactgccaatctttgcgatcttcgcaattgtcttggggatcgcctttgtgaatggctccaagaatgccagcagtgccaaagccggacgaattccagtcgtcttctggcacgaaatgggcggtccagctgagcaagctttggataagatggttgatgatttcaacaagtctcaagacaaatacgaagtcattcctcaataccaaggtgcttacgatgaggccgttcaaaagattattcaaagtcatggaaccagcgcctcgcctgccttgttccagtcctttgatatttcaactgcccagatgatgcacagtaagtacaccaccccggttcagaaattcatcgatgaagacaactatgacgccagcgacatttcaccggttgcccgttcgttctattctaataagggtactcagctggcgatgccgtttaacacttctcaaccagtgttgtactataacgcttcgttgttcaagaagtatggcgttactccgccatccaagtcaccaagctatagtgacgtgacccgggcagccaaggaactttatgccaaatcccatcacaaggtgaagggcatgaccatggaaatctatggttggttaatggaagaagcccttgccaatgcccacacatcattgattaacaatggtgatggtcacactggcaatccaaccaagattgatttgaataaccccacaactaagaagttcctgacctggatcagaaccaacatcaagtccggtgacttcgtcaattacggctccggagccagtgctgaaaccaatgaaattgccgccttcctggcaaacaaattagggatcttcgttcaatcatctgcctatatcggccagttgaccaccggtaccaagaacaagctgggaatttcctacttcccacatccggatggtgtgaaggccaatggtgttggaattggtggggctgcgctttggatctcgaatgataaacccgctaagacccaacgcggtgcctgggaattcattaaattcgctgaaacagctaagaatcaagccaactggcaaaaggcaaccggctacttggcattaaacaagaattctcaaaagaccaagactttacaagatttgtacaaaaagattccggctgcccgagttcctggtgaacagttagccagtgccaaacccaacaataccaactccggtattttgatggaaggcatgcagctgacccgtgaattggaagaaactgcgatggaaggcgtttacaatggtcagaatatcaacagtgcgctaaacactgccaacaaggccatgaatgccaacttgaagacgactaacaaagcagatggcaggtagtttggatttactttccattaaggttcacaactgaatcttaaagggaaagtcgttaagagagttgaagaattgaaaggaagttacccattttgagtactaaaacattaatttttgggcatcgcggttacccgttcaaatttccagagaattcactaaaaggatttcagtacgccattgatcatggcattgacggcttagagtttgatgttcacctgacaaaggacaatgtgccggtcatcatgcatgacgaaaaaattaatcgaacaactgatggtaaaggtttaatcaactcatacaccctcaaggagctccaacagttccacatgccagacggcgaaaccatcccaactttgaaaaatcttttggcgttggcggttcatcgtccggttcacctgaatttggaatttaagaccaacaagatccactacccgaagattgaacagattgtccttgatttggtcaagcaatacgacctgatgtatccagttatctactcctcatttaacctggactcactcaaaattgcttaccaaatcgaccccaaccagcagtattgcctgttatcggatcacgtcattaagaaccctaagtcattaatcgttaaggagcatttggctggactgcatctcagtcattaccaaccattagccaacgttgacgaacggatttggactgtcgacgatccgcgaacgcaagaaaaattattggcggatcatgtcgccggcattatcactgataattttgaacaggcggtcagaattaagaatcgcgctgtcgcaatctagcattaatgtcgacaaaaagagcattcggattaggtttccgaatgctctttttgtgttatttggtgacatacaaacctttgtatccattactcataccggctggattccacacaaatccgtggatgttggttcgccagagctgagtggtggctggctgatacagtggaatgacgccttggtctttcatcaagactttttcggcgtttaccaaatccgcatatcgcttggtgcggttatttgcatcagtggttttggatgcttcaatgtagcgatcatattgtgaattagcccagtgaccattattggttgggttattcttagtcattaagtccaagaagttgattggatcagcgaaatcggcaccccaagaggaaaccaccagatcaaaatcaccgctggttgaccgtgacagcttgctcttagttggcacattgtggatggtgatactcaatcccggtaacttgttgaactggctttgcaggtactgggtggtcttcttagattgatcagtatcatcacttagtagtgagaggtgcagtttcttcactccagtctgcttgaggccggctgcccagagtttcttggcttggctttggttgtaggcaacccctgatttttcataggcatcactggcaaaatcggcaccagttttaggattctggaagaagttagtggagacgaatccctttggtgcggttgacccatcacggagaacttgggtagccagggattgtttattgataatttgggataaggcttggcgaattttgacgttctttaaggccttgacccgcttttgattcatttcaaggtagatcgttgagccgccgacaaactttttgaactctggccggttcttgtaggacggcacttcttcaccggacagtgtcacaacatccagcttgttttgctggtaaagcgaaagtccggtgcttggcgttttgacaacttggaacttaagcttgtcgagtttaacggcctgcttgtcccaataattaggattgcgcttcatcgtccaggtatcactggttccattccagtcggcaagctcaaacggtccgttgtatgccgttgtggtgctgctggtaccgtaactgctgccgaacttcttcaccgcggattcctgttgtgggaagaaggttggaaaggcgagcagtaatttgaaatatggaactggatggctcaggtgaaccactaaagtcgatttgttgggggctgatacgcccaacttatttggcgatagcttatttttttgaatggcactgtagttcttgaccccttcaaacaagtaagaatacccggaagcagtctttgggttgaccactcgacgccagccatacacgaagtcatgagcgaccactggttgaccgttattccatttatcattggttcgcagcttgaaagtatatttcagaccatcttttgaaaccttggtgctggtggccagggcgttttcaactttggattttggaccaagccgatagattccctcgccaatttggtaaagtggtgtcaaactaccgctgtcagaagctttggcagtgtccagtgtcgaaatctccgaatcggtactgatattgacagtttggtccttggccatctggttgctggactttttggcactttggttgccgcatcctgccagcaccaaaatgagtgccagtgcgccggtaattgttagtaaatgttgattgattttcacgttttacccctcttttttgacatgaaaactgccagcacattgatacttgctggtcagttgatgatgcatgaattgagttacttggaatttgttagtgccaaggttgactatattaacatggaatgtggtggggtggcaaatgtggtgtgggaaaattttacctagcggaaacgtgttttcaacaactgaggctaacttctaagggtactttggctaaaaccccaagaccagggactttaatcagagtacccttagaaaacgcctcacccgttgctcaaaacactctgagtgaaaacgtgttccgacacccctgacccctaccacataaggcaaagctaccaacaatgaacacaatccgttcattattgatagctttaccttatgctccggggccacccggggtttgtcacactctaatcaaattcctcatacacattcggatcctgcccatccactctgccatccggcttagtgagagcgttgatttttttcatttcatcctcagtcagttggaaatcaaagaggtctttgttcgccctctgatggattaagctgcttgaacggggcactgggatgatgcctctttgggtatgccactttaagataatttggccggtattcttatcgtactttttggctaactcttgaattaatggttctttcaaagcggcacttcctctgcccaatgggctccaggcttcggttacgatgccgcgttgttggtcctcttttaacatgcgttcgttattccaatagggatggacttcaatctggttcaccgctggggtgacgccagtttcgttaatcaatctgtccagatgttccggttcaaagttggaaacaccgattgaacggatcagaccacgttttttagcatcaatcattgcttgaaatgcttctacgtagtgattacgcttcggcagcggccagtggatcaaatataagtcgaggtaatccaaccccaaacggtagagagattcctggattgccttggttgcttcgtcatattgatgatactttcccggcagcttggaagtcacaaagaactctgaacgggggatcccggaacggcgaatcgcctcgccgaccatgccctcgttatcataattggtggcggtatctaaaccgcgataaccgtcctggatggcagcgagtgtctgctggagaccttcgccaccgcgaatttgaaaagttccaaactgaatcgtggccatcttgtagccgtcgtttaaagtgatttctggaattgcgttatttgtcaatattcgtacctccatgtttaatccttgcgcgacaatttatagttacgaaaaaaggagaactatttttttgtttgctgatcattatttttgggttgagtttttggatgcggcttggttggctgttggtcgacttttttgatcgtgatgtaccagccgacctgcatcgatttgttggggttaatgtattccacgctaaagtcataaaatttggcgtggggacttttttcgatgagcatattttttacctgcagggcatctgcccgactttcaaaccgcagattgctattggtgctgtacccactgtgcttattagggtcattataggtctggttaaaaaagtccaggtattctttggagtcgttcaaggtatcacgtccttccttcttccattgtacccaacatgctgctcaatttcattgtccgtggctaattaagtggaaaacctaaaacttttcagttgatatggggaattttgatcaggattgaattgtgtttcacataggaaacctctaaaatatacatatatggcgaggaggggatcgtcttggtgaaaaatggtttgttattggtgaatttgggctcaccagtgtcgcccagtaatgcagatgtgaaagcttatttgaaagaatttttgagtgatcaaaatgttgtaacgctgccgaagtggttttggcagcctattttgcgtggcatgattctaccgatgcgcacttggcggtcggcaaccttttatcagcacatgtggaccaaagccggttcaccgctgacggcttacacagaaatcatgaagcaaaaggttcaacaggacttgcctgattgggacgttcagtatgctatgaattatgggcaacccaggattgtcgatgttttgcacgagatgaaagatcgcggtgatcgtgacatcgttgtcttgccgctgtttccggattacacacaaagcacccacgatactattattgaaaaagttcagtcgtcgggagtcgcgactcatattattaagaacttttatgatgagccggtgtatcagcaaattttagcccggcaaattgacgaggcctacccaaagaaacagtatgatgcggtgattttcagctaccatggcattccaatgtcgatggtcaaaaaaggtgacccatacgaaggtgagtgtctcgccacgactcaaggtgtgatgaaatacgttaaacaggttccgagtgacaaagtcaaaacggtttttcaatctaaatttggaccgatgccgtggctcaaaccttatttgaaaaattatttgatggagttggccgcaatgggtaaacgcaatgtgttactggtgacgccatcatttgttgaagactgtttggaaaccatcgaagaaaataatgttcaaaactatcagaccttcaaggcaagcggcggcaacgtctttgactcagtcaaaccgatgaatggcagtgatgatttttgccaattcttagccgacctcagtgttaaacaacttcggggaggcggggccgatgagccaagagcaaacgcataaaagccttgatgaaattaatcaaagtgttgaagttcccagcgtttatgaaacttcatttgtgcaaaagtttctcgcatacagtggccctggagcgttagtcgccgtcggatacatggatcccggaaattggctgacgtcactttctgggggcagccaatatcggtattcacttctgtcagtattattgatgtcgattttggtggcaatgttcatgcagacattgtcgatcaaattgggcgtcgttgcccggctggatctcgctcaggcaattgcccaaaaggtgcctaaagccggtcgctacacgttgtggatcatcaatgagttggcgatgatggcaactgacatgactggcgtcgtcggcacggccatcgcattaaaattattatttggtttaccattgttatatgggattttgttcacgatattcgatgtattgttagtgctattatttttaagatttggaatcagaagaatcgaatttattgtgttaacggccattttgattgttggggtcatttttggcgttgaggtgtcacgggcaacgcccaatctggcacaaattgctggtggcctgctgccgacacccaagattttgactaatcatgaaatgctgattatgagcttggggattgttggggcgacgatcatgccgcataacgtttatctgcactcttcactcgctcagagtcgccggtatgattaccataatcccgcccaggttaatgaagccttgagatttgccaaatgggattccaatgttcatttggtggccgcctttttgattaatgccttgttgttagtccttggcggaacgctatttttccacacgaacgggcatttgtcggcctttcaggatgtttacaacggattgaagaattcggcaatcgttggcaacctggccagcccgttgatgagtaccttgtttgcgtttgcgttattgatcactgggatgatttcttcaatcaccagtacgttatccgggcaaattgtgatggaaggctatcttcatattcgtctgccactttgggagcgtcggttactgacccggtttgttaccctgattccgattttagccatcgggtttctggttggctttaacgatcacgactttgaacagattattgtctatgcacaaattgcgttatcgattgccttgccattcacactgttcccgatggtggccttgaccagtaaccatgatttgatggggattcacaccaaccagcggtatgtgacgatgattggctacctgctgacgacgatcattactgttttgaatttgcagtttgtgattgcggctttttaatcaatgtatttagaatatttaagagataagggggagttggattgaaaatacttggcattttggggtctcatagaaatgacggtgcgacagacatgatgctggaaaccgtgctgtctgcggttaaagcgcctaataccactgacatgatctatttggaagactatccatttaagccggatcagggagatcacaaagatccggtgctggatgaacttgaagcaaagatgctggaaagcgatgtttgggtgattgcagccccgacttattggggtggcttggcagggaagatgaaagacttctttgactgcatgcgccaacgcctggtccgctttgatcatgagggtggcactcatccggaccgtttcaagaataagcactacttaagcatcaccgattgttataccggaaccttcgagaactgggtaaccggcgtcaccgaccaaagttttcgaaccattgacaaagtgatgtcggcagccggtgtgattaaaattcacgaactagtgttgaccaacacttggggaatgaaggcattacccgagaacaaaaaacaggcctgcctcaaatggggtgcccgcctgaatactgaacaaaagagagatgatagtacattgaaacgatatattgagttattctttatggttgctgtgatggcgttattgacgatgggaattcaagttggtttgcgtttggtttccactgctgatttctggtggcgctacgcttcgtttgtcgtcattttctatgtgttgttgggatgcattcttcatttctttacggttgtgaaacatcgccgacgataatctaacttgatactaacatgagagtccgacgcacgcgttttgatctcatagtttaacgtaaacaggccatcattcctagttttggaatgatggcctgattgtgtttcagccgatcgtttcacgtttattctcgataacagtcggattcaacaagtctaagattagatagcagcttcagcaattattgtaactttttcttcactttattcagttcctcagcaagcgcaggcctggatggatactcatcgattaagccatcgatccatttgatagcggtttgcacgctgccgaatgcggtatagttcttgattcttcggcccattcgtcgataggcttgtctgccgggatgcttttcgttaagaacaacgttttggtaatacagcttgttgacgacatctgggtagttggagtacaggtccttgctgtaggtttcagtgagctcgggatgctgcatgactagttgcatgagcttatcgaattcacgttccttgtctaaaatgaaggcatagttttccggtgtcagtttcttcgccgctttagccaggaaagtcggatattgggcatcccaactcttatcctgttgtcgcaatttcttgagtggttcgtatgcatcagggtagtttgcgaacagacggttctcgagaaccgcttcttgtttttgctgctgatcggtagcgtcataaattttgatgagatattgctcccaaattcgccgccacccctggtcctgttttgaagcctcaaggcacagttcttccgctcgaacatagtttttgttttgaatcgcattttggatttccacttcgcgaatttgcggaatggttttatgctcgtccataaacttctcggcatcggactgctctccaagttgaatcaggatccgagcatgaagcactttatcgtaaatttcagactgagtcgtttcaaatccttcgtcggctgctttgataactgcccgagatgcggattgagcaagcttggcagactttggcgtgatcagcgggagggcattatacaatacctgatagcgttgttcgggccagccggcaaatatttttcgcttaaaaacgcgaaccacgtccttaatgacgatttctttttgtgattccaaaatctcaggggcgatattggtgctcaaatttttcattgatccaaagactcgatcgaacgtgtcggttagggcgccggaactgctgtcggcatcactgagcattttcgcagccgtttccacaaccaacagcaagccattcattgcatgatgataatggccttgtctgaaccggagcatgtacttattgatcacatcatccaagacattgcaaacaacaatgcagccttggtaatcaataaagccgtaagatttgtttttacggactgtactttgaatcagtttcttggtttgcaccaactcagcatccgtgtcgagatcgccaaattgggcggtcacgtctctgaaaaatgtgggatcgaactgcgcctgattaattatgaattgccgaagcccctcaggagaggcttcgttgacggctttgattaaggattgtttttctccggaattcataattgtttcacgctcctctgacgatatcggaataattcaaatcgatattaccatagattatgagcgactgctaccgctttcagtaactaagtactaaatcttaatggacaaggtttgcaggctgaaagattacttcagtccacgggtgtttaaaaggtaccattgtgtggtattatctatatgggagctaaatcccaaattaatgaaaaacattttgcaatcactaggatctggtcggggagaaatctctggccttttttgtttggtttccggtttgcgtgttgcaataccttccattcaagatatataattaaaataatattagaactatctcattttcatataatattcacgagggagatattgccatgaaaaatgttaagaagtggttggtgatcgggacgattagtctgtcgacattggcattcgcagcctgttcgaacaacaaatcatccgagtctcaatccaagcctatttccatgccgacaacctatagtgcgactggaaaggcaaccaaaacaggcaatgatagtacgctgaacgctgctgaagtcgttgacgcaccgtttaccgggattacgcttgccgtgctccaggataacgttgaggattctgatgtctattcgccaggtggtggcgatcagttgtttaagagcaacaaagattttaagattgtgaagggcggcctcgcgaacttgaagctggaccgatcaaataacacggctacgattaccattcggaaaaatgccaagtggtcaaacggcagcccagtaattgccaaagatgttgagtacgcttatgaaatcatcggcaatcaaaatactggcgctgaacagtactcgtctgacatggcaaccattaaaggcatggctgcttatcacactggtaaggcgaaacagatttcagggattacctatcctgatggacaaaacggcaagcaagtggtgatccactacacccatttatcccctgcgatgcaatacgctggtaattcattcttatgggggactgtggttccttatcaacatatcaagaacgtcaagatttccaagttatcgtcctcaccggcagtccgcaagcacccaattttcgttggcccttacaaactgcaaaaccaggttcaaggtgagtcgactgcttgggtacccaataaatattactggggaccgcagccaaagattaagcacgtcaatatccaagttgtttcctcaagcaatgctgcagcggcgtttaaggcgaaaaagttcgactttgctttgggcggcctgcctgccagtcaatataaatcagttaagaatatcaaaggctacaccctggcaggggcacctggtttaagttatggttactttggcttcaacgttggccactttgacaccaaaaccaacaagaatgtcatggataagcacagcaaaatgggtaacaagaacctgcgaaaggcgatgctgtatgcagttgacctggacaaggttaacaagaaattgttgagtggggttcaatggcggccaaataccttgattccaccaattttcaagaaatatcatgataataaagcagccgggttcccatatgatatggcaaaggctaaaaaactattgaaagacgccggttacaagaagaagggcaagtggtacgtacagcccaacggcaagaaattgaccattcacttcggcgcgatgcaggggtccgctgccagcaacgaaatttctcgatatgaagttcaacagtggcggaaattaggtctgaacgttcaaatgaccaacggccgaccacttgagattaacagcttctattcaattctgggcaagccaaagcaaaagcagatcgacgtgttcgttggcggttggcagttaacctatgagccgacaccaacccagttctatggcgaagatgccacttataacatgggacactttgtgaccaagaagaacaccaagctgctcaacagcttgaatagtaataaagcttggaatcagaagtatcggatcaagcaatttaagaagtggcaggtttatatgaacaaagaagccgcttatgcccctcaaagcaccttgctgagtttcacgccggttaaccaccgactaaagaactttaagcaggccgcctacaataactacctcttcccaactttctgggatcaattggaattgacttcgaagactcctaaatagttctgtataaaagtagcgtcatgggatttagcttccatggcgctacttttatgtgctggataaatcaaatgcaaaattcactcacaaaaagagaaaccggaaaccaataacgcaaacctaatgtgaaattaggggggcgcaacaaatgcttgctggtaaagatagtaaagttttgtatattggatgtagaatcaaaatactttccaagcgaggtgccgcatgataacacaaaataaacctaattgggtcaacaatcccagaaagtggatttggatgctagtgggatttattattatcgagaaatttttggagaatggcatattagttccagtactcctaaaactgccctttggagatcttaccagcaatattttgtacaaagggatcgaagtgttgctagttttggggttaaatatctggctaatcaaacagaagttgtatttctccgttaatgttaccttaaagacaactctctttttcctttttggtattgtctacattagcctgtttatctcatcaggaccggtgaaacttttgcctccaattatactgtggacgttgttgacggcgatttctgaagaactgctctttagggggagtgatttttggggatttattcaaacgcctcactcagcgtcatctgacgaagtggaacgttgcaattgcaattggtttatcaagcctgctgttcagtttgcaacatttgagcaatttggcaaatcagtcattgatggatacagtttgtcagatggttgaaacgtttgggatggggattttgctggcagcgatttatgtgagaaccggatcattgatcacgacgatttttgcccattttctaattgactttccgattttgtatttaagtcagatcagcactggttttgcttctactgcaaatatgtctgggaatgtttcagtggtcggatcgattattgtcgcaattgtttatgccctggttggaatagttgtcatccgatcaaaaatagccgataacaaattaccggcaattacacatactatagaaaatctaccaaattaaaagtcgcgatcccgatagtcgtcccaatccggcatctttgaatggttctccttggcggttcgaatgtcatgataaaatctgaccttgcgcttgatgtgacgttcgttctttttcaaaagtgccagttgttcaaggacgcgttgatagtggttatccaaaatctcacaggttttgtccaagtccgcatcgtcgtcttgggcggcaaacagttcctgcaattctttgagggtcatcccagtatccttaaagcagcaaatcgcccccaggcggttgagatgctcctgcgtgtatgcccgtcgccctttgatccgaggaatgtcataaagcagccccaagtcttcgtagtagcgcagggtggtcgtcggcaagtgatacattttagatacttcggtgatcgaataagttttcacggttgcggttttcaaattgttgacctcccaagtcgaaataagtttacttcaagtatactcgaagtgttacatttaagctaaacaatttaggagatggcgaaatgtatcaagcatccaaagatcgttacgataaaatggtttataaccgggttggcaaaagtggcctcaagattcctgccttgagccttggactctggcataacttcggtagtgtcgattcctttgaaaatcaaaaggcgattatccatcaagcatttgacctggggattacttattttgatttggccaacaattatggcccggaacctgggagtgccgaagagaacttcggtcggattatggcagaagatatgaagccttatcgagatgaaatgatcattgccagcaaggccggctattacatgtggccgggtccttacggtgaatggggatcacggaagaatattattgccagtgccaatcagagtttgaagcggatgggattggattatgtggatatcttctattctcaccgatttgacccggacacgccactggaagaaaccgcccttgccttagatgagttggttcatgaaggtaaagcgctctatattgggatttccaattatgacggcaaacaaactgcagagattaccaagatctttaatgatttgaacacgccgtttgtgattcatcaaccccgctataacatgtttgaccggcacatcgaaaatgatctcttcccggtattgaagaaggaacataaggccgcggtcagctttagttcgctggcccaaggtttactgacggacaaatatttgaatgggattccagctgattcacgggctcacaaatctaccagtccatttcttcatgaagaacaggttgaagagacgattaagacggttaagaaattgaatcaagttgcagctgatcgtggccaaactttggctgagatggctttggcttggaatctgcgtgagccggaaattgccagtgtattgattggagccagtcgaccggaacaattacttgataacgtgaaggcactggacaatcttgaattttctagtgaagagcttaagaaaattgatgatattttggcgacccaaaagccgattaaataaataagagtggaacgcgaggcgttttgcttaaatggccgggatcagccgatcgttgcacgtttaaacttcataccattggaactcaagagaggccgagatataactgacaatcagttgtatcccggcctcattttgatatacaaattaacttcccattgatggttgacttgaagtgtaaactgctcgatacttcagaacaatattggctttcttttgggtgccaaccgatgaccacttacccttggtcttttggtagacaaattttggtgaagtgccattcagttgaacaaagaactgaccgtcacctgatttgcgtacccggtagacttttgttttgctggttggtgaaagggtcgtttctggatcggtcttgttataagcgacaatactttgtcgaatcatatctttatattgattggtttgatggcttttcatgataatcccgacgatgccggcaatcacaatcagcaccatcagtgacagcatgatccacatgatgttggctcgtttggcgttttgagctttttccttctcattcattctatatcaccccatctatttccattggaatcgaaaaaccttacatgttaaatgtatcacacaaatggcctcttgagaaaaatgtggggggatttcttcaacagaacgtcgaaaagtatttccaactttgtgttaaataaaaatcatttcaaattgtgatcagttggatgattggcaggttgatgtcaaggtgtacaataatcacattattgtaattggaaggaatgacttgatgaacattctgttactgattatcgttggctttatcatcggcactgttgtgattacccttggcggtggtggggccgccttttaccttggaattctcacgacggtctttggcctggggccagcgagtgcggccgccacttcattggtgacctcgtttccatcattgttaatcggctcgtactcttattttcgactacacaaaattaaattacggattgcctggaggatgatcatttttgccgtcccggctgtggttgtgggatccttgatctcgccatatatcccggtcaaaatttattcgtatattatcggcggcattttggcgattttagggcttcagacgttgtttagcagacaaaaggatcaccaaaatcctaataaatggttggcaccagtctatggtgtcatcagtggtctaatggttggtgtcggcggactcagtggtggtgggccggtggttgccggactgctcgtgatgggatcggacatggtcaccgcagccgccacttcttcattagtcctggtcgtgatgaccgcaactgggttaatctttcacctttctgctggtaacgttgactggtcggtgggcctcggactgatgtttggggcaattctgggatcgtttttagctccggtactgttgggcaggctcgatcctcagaagttcaccagatatgtgaaaccgattctgggagttctgttggttgtgatgggtgtctttacggcattaaaatgaagtccataaagctcctgaattaaatcgtggtggatgaaaattgtgaatacaagcaaacacaaacctggtttgcaattggtttgcgaacaaaagccaattcaattacattcagatttcccttgatcatcaccttacgtcatcagctataacagaatcaggaggtgaaaccgatgtcgaaatatacaacaggagagcttgccaggttgggtggtgtttcgatcagaaccatccaatattatgatcaaaaaggaatcttgaatccgacaaccatttcagatggcggccgtcgcttatacacggacaaagagttgaaaaccttgcgattgattttattgttgaaatcaatgggcctctctctgacgacgattaaagacctgttatcagaagataattcaactcaagtcctgtcgttgatgcttaaggaacaggaaaagaaaattcagcatgagatgacaatgaccgcggatcagctggaaatgattcgcaaggttcaagacagcctggctgattatgcgctaatttcccaacctgaccttgacggcatcgaaaatatgatggaaagtaaaccaaaattaaccaagtttcgctggtggatgttaacttggggactgatgatggacgcactggaaatcttagcaattgccgtttggatcatcactggtaattgggtaccagccgcaatcatcttcccagtcgtgattgtaatggctatttggattatccgggagtattacaacaaagttgagtatatctgcccaaattgtcaccagcatttcaaaccgagctggcgtgactttacattttccaagcatactgccaagacgcggaaactgacgtgtcccaattgcggttaccgtggcttttgcgtcgaggtttacgatgtgaagcaaacgagtagatagtaaaaacacctgaccagaaatcggtcgggtgctttttggattattcatgttccaaaatctgattcatcgcgctgtcggcactactcttatacattgtgccgaatttattggtgtgaaccatcaagtaatacagccgatagaagttcagccgttcattggcgcccggatccaaagggtagactgcgttataagcggcgtagaagtccgcgtcaaagccaccaaagacggtggtaatccccaggtcaaattcccgatcaccatagaaagaagcgggatcaatcaatgccggacgaccgtccgccaagaacatgtagttgccgccccacaaatcgccgtgaagcagggatggctcgctttcatgtttcgacaactgatcgagaatcacttcgcgaacccgtttgtacttttcatcgtcacttggattccataaatgctttttcatcaaagcatcgcggagccggtccaatcggtggttgacgaacaattcactccaagagtcggtccaactgttatcgaagctttcatcgttgctgacatagggcaggtcaaagccaaattttccattcttgctataatgctgatgcaagttggcaaccagttcacctaagtcactctgactgccggaacctgattccaaaaagttcagcagcaaataagcatcgccgttaatttgaccattgcccaacactcggggagccaagacgttggcttcctcgaaagctttgagcccagcaatctcgccagcgtaaaagtcggcagtcgtctggggctgaaccagtaggaaatatgtgtcatcttttgtttctaatcgaaatgcctgattaacatcgccaccaccaaccgggactgctttggtaatccctttgatgggcagttgcgatagccattgatcatccattgaatcatcacctctgggttcattgtaactgaaaattgaattttatgtaggctggaattgcgatgggggtcaaatcgggttaccattaaatcaaatcatatcgtcgattaagcaaatttgctggaaaggagccgcaaatgaattacttacaagttgccaagccgttggtgttacccaacggtcagcaggtcaaaaatcgattctttaaatcggccatgagtgaaacgatggctaaccaagatcatcagccagatgatcgttatgcaaccttgtatcgagcatgggcaatgggtggttctggaattgtggtaactggtaacgtcatggtcgattcaaccgccttggcagaacccggcaacgtggtcgttgaggatgagcggagcttggcaacccttcaaaagtgggctcaagcgggaacgacaaaccacacccagttgtggatgcagctcaatcatcccggtaaacagtcacccaagtttttgtcggctcaaccggctggacccagtgccattccggtgcatggccctaatcagaaatattttaatccgccacgtgaattgaggaattctgaagtacatgagattattgccaaatacattcgaaccgcagagattgcccaagaagccggcttctccggtgtccaaattcatggcgcatacggttatttggttaatcagttcttgtctcgcaaaggcaaccagcggacagatgaatttggcggctcactggagaaccgaatgcgatttctcgcagatatctataaagggattcgcgaatcatgtgggccccagttttcgattgggctaaagctcagcgtgcttgaccttgatttggaaggattcaccgaacacgactcaattgccgtgatccaaaaaatggccacccttggcatcgacctgattgaaatctctggtgatgattacgaagattcggcggttggtttttccggctatgcccatatgatccatcaacttacagatgtccccattgtgctcagtggtgggtttagaagaatttccacgatggaagaggcgctgggaacccacgacgccgacatgatcggaatgtgtacaccaatggcggtaatgccggacctgcctaatcaaattttagctggcagctaccaaccagttccactgccactaacgatggggagtcgaaagttggatgagaagtattcgccaacattcattaccgcatattgtgaacaacaggcgcgtcggctggcagaggggaaacgaccacagctatacacgagtgcctggcgcgccttggcggcaagtattcaaatgcacgggccaaatgggctaacacctcgccgggctcaataaataattgaagattggaagaaattcatgtcacaaccatttgaaccaaattcattagatgaactaaaagatcagtatgacgttgttgtcatcggctcgggtagtgctgggcttaccagcgctattcgggcaaccgaactcggattgaaaccagtgatttttgaaaaaatgccgaatgttggcggtgatactaaacgggcctcgtcggggatgaacgctgcggcaacctttgttcagacggagcatgggattgaagatagcgttggcgccttttattacgagacgttgcgtggcggtcatggccaaaacgatccagcgttattgaagtattttaccgagcatggtgcccgggcaatcgagtggctttataaacagggtgtacagttggatgatctgacaattaccggcggcatgagtgtaccacgggcgcatcgaccaagctcaactcaaccaattggtggttacctgattaatggtctgctaagccaagttcaggcaaaacgaattccactgttcaccaacgctaaagtgattgaaatcctgcacaacgaccgagtttccggtgtgcaaatttcaacaccagacggtccgcaaaccgttcacgccaaagcggtgattattgccgctggcgggtttggtgccaacaagtcactcattgcaaagtatcgccccgatctgactaaatacaagacaaccaaccagcctggaaataccggtgatggcatgttgctggcagagcatttgggtgcccagctggttgatatggatcgaattcaaattcaccccaccgttcaacaggatacggaccacgtctatttaatcggtgaaacggtccggggcgaaggcgcaatcctagtcgatcaaaacggaaagcggtttgtgaatgaaatggaaacccgcgacaaagtcaccaacgcaatcgagaagttaggcggcactggtgcatacctcatctttgatgccaaggttcgcaaacgtgccaaggcaattgacttctatgatcatgttggcctggttaagacaggcgatgatttagccaaacttggtaaactgattggtgttgatggtgagatattatcgcaaaccgtagcgaagtggaacgaagcggtttccgatcgaatggacattaactttggcagaacgaccggccgccacatccttgaaactcccccatattatgcgattcacattgccccggcgattcattatacaatgggcggattgaagactaacgatcaaactcaagtgcttaaggcggacggccaaccgattccaggattatatgcggccggagaggtggttggtggcctacatggtgataatcgaattggtggcaactccattgcggaaaccgtcgtatttggtttgcaggcagctcagcaggtacgcgattatatctttgagatgtgataggcgggtgcagcaggaaacacgactaatggtaaagtgtttacagcaagacattggactagtatttcaatccataatcaatagtattattcatacggaggcatgttgctgatgagccaaggtaaaagagaatcaggctattcaaaatggtttaggatgttgaatcatttgattggaccagttatcacaattgggattatttctggaataatcattattatttctgacaatgcttatgcatatgttgttgatgtcattgtgtcagtgtttacatttatctggttatcaacgttcatagttgaatcggtaattaaaatatttggaaagaaataagtaagttaaaattgaaaatgagctgcactcaaagaaattatcgctttaactttggggcagctcattttgacatatgcggacttggcatccatgaaagaaagtatttctgatcatgctggctgattaattaaaataatccattaatctcatcaaattctgctgagctcagttgtacatccaacgctttggcattactgtcgacttgctctggcaatcttgcgccgggaatcaccacgctaatatctggattagcaatgtaccaagccaaaatcgtttgagcaatcgttgcctgatgattttcggcgatggttttgatttgatctaaactatccatgatctgattgaattttgatggagagaacctgctgaacttgtctgcatcgtttcgactgtatttgccagttagtaaacctgaagccagtggaaaataggggacaaaggaaatttggtgtgcctttagatacgggaagatttctgattctgcatcccggtgaaccaggctgtaattgttctccacgacatcgacttgattgtcttgattggcctccttgatctggtccagattaaaattagaaatcccgattgcccgaatcttaccggccttttttgcctgggccagcgcgtcaactgcttcggcctttggggtcttgtcatccggaaaatgaatgtaaaagatgtcgatgtaatcggtttgcagccgttccaacgattcatcaatcgatttggtcaagaacttaggatcgttattaggcttcaagtcgttattgggatcctgcgctgccttcgatgcgatgacaaattttgaacgatcgaaatcttgaatgacattgccaataatgtcttcagacttgcccaatccatacataaatgcggtatccaataaggtaatcccatcgttcagggccgctttaataaccgcctcgccatccgaatccttcaggccgtcaaataaattatggccgccgaccttgttggttcccagacctaaggggccgctgacaacttcgctcttaccaattttaactgagttattcaaagtcaattcctccttacatatcaataatgctctgccataaaaatagggctgaaattaaaatatttcaacccaagtgtctatttacgataattgattattcgtcgtaaggccctttgccaaggtaggcgttaatcatccaaatattcttgtcaatgtcttctttaaagccattcagcatatcttgagttggaaaatctttttcctcgtcagtgacctcaatgcccttttgatattgatcacgcaaatacctgaattgatcaaccagccgctgcatgaagtcacgcatggttaattggtcccaggtcaccttttcgtctggtaagccggtgttatcaatgaattcatgagtggttgcgaacggcgaaccgttgattgcgatcagtcgctcggcaacgttgtccagttgatcagctaattgatcattataatcatccatcagcgggtgcaggcgaaagaagttttcaccccgcatgtaccagtgggtttgttggatgttggtctgcagctggctgagatctgcgactaattgattcaattgtgcgcgtgtctttggaaaatcatacttgtctgccatcagattacctcccagaataattttgaattcgcttacacagtcagtgtactcgattccgggagacggtcgcaaggaagttgccttttagttttcgaaaggcttagtggtcttttggtccactaacagtcggggcctgtggttggtcaggctccgtcgtttccggtgattcttccagtttggaatgcttggaggtttccagcatccggacgtagaccaggaagctgataaatgccgctgctgatacataatagaagaaccagtcttcatgaccgatgtgcttgagccacagggcaatgtattcaacacttccaccaaagatcgcaacggtcagcccataaggaaaaccaaccccgagtgcccgaatttcagtcgggaataattccgctttgacgatggcattaattgaagtgtagccactgacgatcagaaggccaccaagcatcagtaaaaacgatgccactgggctatcgaaggatttgagtccgagaaagatcggcacggtcaaaattgtcccaccaatcccgaaccagtagagtaacggctttcggccaattttatctgaaaggtggccaaacaatggttgggcagccataaaaatcaacagggcaacaaagttgatcatcgtgaccagttttggtgccagccccaatgaattgatcatgtatttctgcatataggtcgtgtaggtgtagaaagcaattgtcccaccaaaggttaatccaacgacggtcaacacttgattgggatattttgccaactcacgcaaggatcctctggtggcctttgttttctcagtctgtttaaattgatttgtttcgtccattgaaagtcgcaggtataaaacgataacggcaccaaccgcaccaacggcgaagggaatccgccagccaaatgcccgcagttgtgcatccgaaagcattgactgcagaatgatttgaacgattaaggcgatcagttgaccgctgattaaagttacatactgaaacgatgcgtaatagccacgccgtccagaggttgccatttctgacagataagtggcagaaatgccgtactcgccgccaagtgataatccttggaccaaacgaatgcagaccaacagcaacggcgcaaaaacgccgattgaactgtaggtcgggataatggcaatcaacagcgatccggtggccatgatgctgacggagagcgttaaggcggcccggcggccttttttatcggcatatttgcccatgataaagctgccgaacggtcgcatcaggaagccaaccgcaaaaatagcagctgcactcagcagttcgacggtttgatcaccgtctggaaaaaatgatccggcaaaataaatggcaaaggatgcataaatataccaatcgaaccattcaatcatattgcctaaagaacctttaatgatattgcttgtaacccgtttttggctgtatcgttgcatgttgggacctcctttaattcagaaccgaattagaaattaattagatatattctaattaattacctagtataggttaataattaatgggatgcaagatatcatgttaggttatataacatgttaccaaaacaaaaatgactgtcacctgtgaaccaattgtgggttcaattccatggggcagtcatttgagcttgattcaattagacaattgcttccagccgcaggagatgatcaatctcataagttggcttcaatcggatggtattgggctgatgggttgggttgaaccagactgaatcgaggccatataaattggcccctttaatatcggaggtcagcgaatcaccaatcaccagtgactggtcttttgaaaagccctgaatgttgtgtgcaacatagtcaaaaaagccaggattaggtttttggacgccgacagtttcggacgcgaaaacattagtaaagtagggtgccagaccagactcgttgagccgccgatgttgagttttggcgatcccattggtcacgacataaatatcgtgacttgcactgaggtcggccagcaattgcttggcttgcggcatcgggctgtgaccttcggctagaaaactgcgataccgttgttcataggcttttccgtcaacaacttggccgtaatggtcgaagaaacgacggaatcgagtatccagcagcgtttggcgactgatttcgcctaattcatattgctgccaaagctgctcattaaattgatggtagtcggcatagacctcagtcgtcagtggctggccgatggtttggaataactttttgagggcgtcgtgctcagctgcctggaaattcagcaacgtgtcatcaacgtcaaagagtaatgtcgaatatttcatgaaaggagacctcacgtcatttttgttaaattctatcacaatcagacggtaattttgctgatattcacaaacttgtcagaattgttggcttactcttcctgcgaagtgctaccattaaaggaaaggtcttttacattacacacaggggagtcttaacatggcaaatcatatcacgctatatcagcacggaacgctggcattacttgttcccgggcttttaaagggaaccattacaatgggggaactgttaaaacatggcgataccggcattgggaccggtgaaggcttggatggggaactgattattcttgacggcaagccatatcacgtccacgccaccggggatgtcacactagcccccaagtcgtttaccatgccgtttgccaatgcccattttgcccgctacacgccactggccgaactggaaaacgttgatcaggctgatttgaacaaacaattggtctcgttaagtcgagctgccaacacttttttctccattaaaataaccggcacttttgccaacatccaaaccagagcggcggttaaatctcagccgccgtacaatactttggctgaaaccgctgaaaatcagagcgtctttacccgggatcagattaatggaacgttgattggctattacgcgccgcaactgttcgagggcgcagcagtgggcggctttcatcaccacttcatttccgatgaccgcaagtttggtggccacgtcttgaatttccaccttgtaaagggtgatgtcagctaccagttatttgatacctttgaacaacacctgcccgtcagtgacaaggactacatgcagcacgatttttcaaaggacgacatcgccggcagcattcaaaagtctgaatagtgggactgttaattacaattattccgattatcgttatcataatttaacactttataaccttttagtaaacgtaatactaatattagtaaaacttttgcattcgccgtaaacactggggtgagtgcatttttgtttggcctaaattacaaatttatatgataaccagttttagtacttgatttatacggatgaatccgttaacataacaaactatggacgctggttattttttgatagcggtccatatgtaatactgtaaatgaatgtaagcgttacgactgtacgtataagagagaatgtcacacaacaaagaatgtgttggatttgtctgatttgttatgtaaccccttccattcttttgggttggggaatcacgactaatcaagcgttggcttaaagtgtaaaggagaatgatgatggaaaaggctgttgcaacagaaaagaaaatctcaagcggatttatttatttctttggttcattcggtgggattctgtttggatatgatattggggttatgacgggggcactcccatttttacaaactgattggggactgcaaaataatgcgacgatcactggctggattacgtcagctgtaatgttgggtgccatctttggtggtgcgattgccgggcagctgtccgataagatgggtcgaagaaagatgatcctgctttcagctctgattttcatggccggatcattgttatctgccatctcaccgcatgacggtcaattctacctgattgctgttcgcgtcttcttaggccttgccgttggggcatcttcagctctggtgccggcctatatgtcagaaatggcgccggccaaaatgcgggggcgtttgaccgggattaaccagacgatgattgtgtctgggatgttgctatcttacgtgatggatttcgtattgaaagacttgcctgagaactgggcatggcgttcaatgcttggcctggctgccttgcctgccttgatcttgttctttggcgtattgaagctgcctgaatcaccacgtttcttagttaaaaacggtcgccctgacgatgctcgcagagtgttgagctacatccgggaaaacgataccgaaattgatgacgaattagagcaaattcaagatactgcttcacaagaaaagaaaatttcaaaatcaaccagctgggcaactgtcttcagttcaaaataccgttacctggcaatcgctggtatcggcgtggctgccttccaacagttccaaggagccaatgcaatcttctattacattccattgattgttgaaaaggcgacaggaactgcagctaactcagctttgatgtggccaattattcaaggaattatcctggtaatcggatcactggtattcttgggaatcgctgacaaatttaagcgtcggaccttactaattcttggtggaacggtcatgggattatcattcctcctgccaactgccattaagttcctggtaccaaacgccagtccattactgattgtcttcttcctgagtatttacgttgccgcatattcatttacttgggcacccttaacttgggttctgattggtgaagtcttcccactggcaattcgtggccgggcatcaggagccgcttcatctgccaactgggttggttcattcgctgttggactgctcttcccgatcatgaccgccagcatgccacaggacgccgtattcgctatttttggtgtcatctgtctgttgggtgtctggttcatccattcacgggtaccggaaaccaagggccgcagtttggaagatattgaagaagaaaacattaataaataatctgatgatcgattccggacaaattctgggatagcaccctataaaaattaaaagcgtctgacacgaatttttctacttgtgtcagacgtttttgattttgatagttacttctatatgatagggcaacaaaactctttacgaacccttattgcagcagctctttaataatcgcttcaccaacaccagtcgctgagttgggattttggccggtaatcagccggtcgtcgaccaccacattcggctcaaaagcggtccccttcacgaagttggcacctgctttgtccaattcatcttccaacaggaactcaacgtcattcgtgagaccgtttaaggcttcttcatcattggtgaaggcagtcagcttgcgaccatgcacaaagcgtttgccatcttctgtccgcatgggcagcaggccacacacgccgacgcaattggctgagataattccgccgttggcataaattgtttcggccagccccgccaattcggtgttctgtgggaaatcggtcatcgttccgtggccgccaacaaaataaattacttggtagtccttgggattgacgtcggccggggtgagtgactgggctaaatgctgatttcggaaggtgtcgtccagataatattcccaatccgtggcgtccatgtcatcggttcccaagctcagaggatcgagcgggacataaccgcccttgggactgacataatcgacatcgatgccgttatcggccatcactttgttgaaatgggtcgcttccttcagccagattccggtggcccgttgaatcttcttgaatttggggttgtttgtcacaaccattaaagctttcgtcataagcagcgttacctcgatttttcgttctgattagacttgtcgatttcatttcctcacccccatcataacagataattcatgaggatgatgagaaatggggtgttgtataagttttaacacatatgttatccttaaggccaaccattcatgaaaatgagtggccctttacttgtagaattgtgtttgagtataaatactaggaggaacacatggcagactcaatattaaatgtcgagcatcttaacaagaactttggccgtaagcaggttctcaaagatgtgtcgttttcagtacaaaccggacatattgtgggcttggttggtcccaacggtgccggtaaatcaaccattatgaaagccgtcttaggactctttaattactcaagcggcaagatcaccattgatggcgatccggtttcacccaccagtcatcgagcgatggataaggttggcgccttaattgaataccccgggatttacccattcctgacaggttatcagcacctgcagttattttcaaaggaatcgacttcaaaagatcagattatggacatcgttgacaagatgaagatggattcatacataaaccgcaaggccaagacctactctttaggtatgaaacaaaagcttgggattgctttggcattagtcgaccgccccaaactggttattttggatgagccgatgaatggtctggatccccaagccaacaaagacttgcggaccattattttggatttggccaaacaaggaaccacattcctgatctccagtcatatcttaagtgagttggaaaaattggtcgatgacctggttgtcattgataagggacagatcgtttacactgagagcatggccaacctggaaaatggcggtaagaagttattggttcttaagacctcagatgacgcccatgctaaaactattttgagccaaaacggctaccagcttgatgacggcgataagctcagcattgtcgaaactgactcaaccaagatggctgacgtgatcaaattactgtccgataacgatatcgacattgaagatgtccaacacgttcacagtgatttggaaacatcactcttaaatctgctcaaaaacgacaaagtaaaggagtcatagcatgataacgttagtcaaacaagaaatctttaaactgcttcataagaaaagcacctacgcggtctcagctacattattgattctgatgactgtttttggtgtattgacccgaaactatcccaagtactggggcgatcccaaaggattatttgtcgaaatgtttaccgggatcaactggatcgtcttattcatgattgcggcctgcagttcaatcattgcgatggaatttcagtacggcacgattaaagaattgttgtatcgcaagtattatcgtgggcaaatcctggtcagcaagtggattaccatgttgctgtactcgatttatttctacgctttgagctttgtctggtcgatgcttttgaaagttgttttgtttaacgataaattcaaactttcagatacctatcaatcaggtcactccgttatcgaagcgcaatggctcggcattatcggctcctttctaacgatctggctggttcttagtctagtgcttttattagcgaacgtcttcaagagtaccgcagcagcgatttcaatcgggattatcggttactttgctttgagcatggtttccggggtcatgttcttattgatgcacaaatgggaatggcttaaatggaacccattgaacatgatgaacctgccacaacagcttttgtccagttcggtgcataaaatgaccttgttgtcgacaccggaaatggtggttggcagtctggtatacacggcaattttcatggcaatcagctacgttgtcttcaagcgccggagtgtctaaattaaaattgaacgtttcaaagatggaatcggctaacagctggttccatttttttgtgcaaagattcatgtttccaaaaaggtgtcattttaataacaatctcattatttgttaagagtgtctaacgtttgctcagaatgaaagcctgtgaatagcaaaatctgtgatgtttggtactatgtatctgattaaatgttacagatatatttcaagattgcatgacggggggattgcatatggtacataagagttggctgctattgccactgacggtattgttgatgggatgcagcgcgcacaagacgaccaccgctcagacgacttcgagcacggcgagtgaacaggatggcaaatataacggagtgaccttagacgttgcccgacgccactaccaagttgggacgttgcaaaagttcattcaattagtgggggatcataacggtcggtttattcagctgcacttaagcgatgaccggaattttgcgattgaaaatgactacgttggtcagtccttgaagaatgcccagaaggttgatggggtttggcataacaaaaagacccaccagttcttttacagcaaggccgaaatcaagtatttggtcaacgacgccgaacagcaccacgtgacgctgatcccggaaatcgacaccccagcgcatgtgactgccttggtgaagctcatgaaggccaatggcaaggcacaactggccaagcaagtcagttggtactccaagagttaccgcgacgagattcacctcaatcaaaccggcattgatttcaccaaaaagctggacgacgaggttggcgccttgtttgccgggcaggccaatccccgctttcatttaggcggcgatgaattttccgataagctaaccagcaacgcggcttacgtcaaatatctaaacgccaccagcgccaatgtggaaaaaatgggcttcacaccggaagcttggaacgacggctttttaaacagcagtttgagcaaactcaataaaaatatccaagtaacttactggaactggaccgcagatcaaaccggcaagttagctgctgagcgccacaaatactgggcctcgatgccaaaattgatcagccgcggtttcaaagttttcaactataacgactactatctgtatttcaatttatccaaaaccaacatgtccaagaaaaacgtcgcttatatgattaaggatatgaagcaatactggaaaccgacgttatggcacaacgatgttgataccaagttgaagtccaaacgggggattgtcggcagcagcgtatcactatgggcagactcagcgggatcggtcaatgatcagcaggtatatgccgctagtgagcagttcatcaaaacctttttggccttggccgaaagtagatagaatggggggatattatgagtaccttgagtgattttgtcattttatatccagtaattgtgtcgacaatttggatcgtggggtcaatttttttctccattcaagaacggcgggtgccactgaataacgaccatcaaggacaaccagctgacctggtttcaattttgattccagcccacaatgagcaggacaccctggctcaagtggtcgagtcggtctcaaagatcacttaccaacggattgagctgattttaatgaacgatggcagtcaagacaataccctggcggtgatgactcagcttcaggaacggtatggtcatcagtttccggtcaaaattgtcgatatcaaggtcaataagggtaaagccaacgccctcaatgaaggggccaaggtggctcaaggggaattcttgttgtgcctggatgcggattgctacgtcgatcaaaatgttctcgaaccgatgctggcgcgattctatgatgacccgaaagtcggcgcagtcgccggcaagccaatcgtccgcaatcggaccagtattctaggtcggctgcagttgctggaatatgtgggcgtgatcgatattatcaaacgcggccaggctttcgttattggtcacatcacaacggtttccggtgtggtggtggcttatcgaaaacaggcgattattgatgccggctggtggaatatcgatgccattactgaggatattgatattacttggcgcctttatcaccatggctggcaggtccgttactgcccggagtcggtcgcatggatcttggttccggaacgaataatcgatttgattcaccaacgaaggcgctgggcccgcggaggcttcgaagtgctgtttcgcaaccgggggatgtttatcaccggtcgcttgagtgaacagtggctgctgatggacatggtgctcagtgatttgtgggccatcagctgctcatttgtgacgctgttttaccttttcacgattatgttcacaggtgacatcatcatggacggcgtgattttatttctcctattgctcattagtttgattcaattcttgattggttatgccgattccagagagtccgatttcatcaaatggcaggacctgtcactattgccgctgtatgtgattttttattggttcatcaacttggtcagttgcctaactgccctgggatcgttcttcctggatccgagtcatgttggcagttggcgtagtccggatcgggggctttaatcatgaaaaagaagactaacaacctgattattcggaaacgatcctcaattcttaaattgttggaacggttcatctttttggtggctttgtgggccatgacagtttacgtgatctacgtcaacgtttgcttcctattgaacgcatactcggacacgctggtttctgattacctctttttgaacctgtcctactttgcctatgcccgatttgccatcctggtcgtggtgatggtcatcttgatgacaatttttggttggctgcgaattaagaaacttgagcggagggcgaaaaatcatgagcaaaacaagtcgtaagtggattttaagcgggtttattctggtctttttggtacttttggcagtcagtgttcgacacaatattgcctatcagctgggcaatcggcctgattttgcgatttccaaacgtgaccagcgaatcaaaaatggcatcatggtgttctcctaccaccggattttggcaccgaatgacattgtccggttcgatgaaaaagtgtcgccgaacacacagtttcacgattttaacgtcaacctgccttcctttaaaaagcagatgtattatttgaaatcccatcacatcaaagtcatttcaatcaaacaaatgattgctatggctcacagcaagcgacccattcgcggtaagtacgtggtaattacctttgatgatgttgaccgaacgtcgatcgacaatgcgtttccgatcctcgaaaaattacattacccgtttacccagtcgattattaccggcaacaccggttggtacaagcagggaactaaattggcaacttggccggcaattcaaaggctgcaaaaacaggccggtagtttagtgacctttggtgttcacaccaatcggatgcattatttggttgaccacgggatcccggtgttcaacattccggcgaactacactcgctttaagcgtgattatgcggtcagccaggatgtcttgaaggaaaaggtcggctataagtcaccaatttttacttatccatacggtagtggcgactctcagattcaaaagtttctcgctaaccgccccggcctaaaagtcattttgaccttgaacgatggcttggtgaccaaccatagtaacttaaaactcaccccaagaattattgtgaataattacagttggccgagcatcaccaaatggattaacaattgaacgaaactttgagataaaatgaagataacgataaagggggatgcacaatgacgttttacacgtacgactatcttcaaggttctcaaagtagctggcagtacgccagaatcattattttaagcgtgctggcagtcatttttattggctttttggtccattaccttcgtaatcgaatggacagcaaatacaaagatttaaccattatcgtcgggacgctgctgctgcttattttagcgatccaatacgacgactttagtgcgattcagtccgcttctgcgcagacaggccagattacgcagacggttaagcagattgccaagcggcttcatgtgggaaccaaaagcgtcagtatcaattcgaccacccaaaatgccaacctgatggctaaaacccccagcggttattaccgggtcgactataacgctgacgggagtcagtttgtgttggaaaaggttgagttagatggttcgagccacatcaaagttcaggaggcaaactaatatgtttacatattcagacgttgcacttaaattaatcgtcggtttcttatttatcaccatcttgattaacctgaccggcaagggaaatctggcaccgacatcagcaatggatcagctgcaaaactacgtccttggtggcattatcggcggtgtgatttataatccggccatcacgatggcgcaatttttagtgattctgttgctgtgggcactgttaatcatggtgactagatacttgaaaacccatattcactggtttggtaaatttatcgagggtgagccaatcacactggtgcgtaatggtcagctcttggtcgagaattgtattagagccaatctctccggtaaagatgttgacttcaagctgcgaactgccggcgtttacgatattcaagacgtgaaacgggccattttggaacaaaacggtcagctgacggttttgaataaaggggagggtagtattcgctacccggtaatcgtggacggccaggtggatccggacgtcttagatcttatgggtcgagaccagcagtggcttgaagatgagctggccaagcaaggtttcgacaatatccgcgatgtgtactgggcaacttatcgtgaaaatgtgttgaaagtcgcggctttccctgaaaaatgataatggtggaactaacacggccgtgtaagaataaacgcgattttaccatacgattattgaaatacacggcaatcaagaatcaaaggcataattatacaatcgattgatctttcattgacttctcagagaattgttatattattaacaataacttttaccgaatcattggcaggttttaaatctgaattttccggaggtcaccattatggaattagacagtatcaacccttatgtgttaaaagtcatgccgtccgcaatgcggaaatttgatcatgacattagttccgatccaaagattatcaaattaactttgggcgagcccaacttcaacgttcccgaccatattaagcaggccgcgatcgacgcgattaaccacaacgaatctcattatccttactattggggttaccaaccgcttcgtgaagcagcatcaacttattatcaagctaagttcggctatcactattccgctgatcaaattttggtgacggttggggcgactgaggccgttgcttctgcagtgaagaccttatttaagcctggtgatgccgtgattattcctacgccggcctatccgctgtataacgctttgacgaccttaaacgagttgaatacgattctagtggacaccagcgatgatgactttattttgacaccgactaaagtcgagcaggcaattgccgaccaccctgactgggatgttaaaggcctgatcttaaacgacccgaataatccgactggagttgcatacaccgaagaacaaattaacgcgttggcgcctgttttaaagaaaaatggcatttgggtcatcagtgatgaaatctatggcgagctgacatacgggcagaagcattattccatttcaaaagttctgccggatcaaacggtcgtgattaacgggttatccaagtcgcatgccatgaccggttatcgattgggattggtatttggccccagcggtttcatcgatgaaattgccaaagttcaccagtacaccgtgaccgcggctgcgtcaatcgttcaatacgcagcgattgaggcgttgacacacggtcaggatgattccaaaccaatgctcaaggaataccagaagcgtcgagattttgtcgccaaggagatggctgaagccggttttggcgtcgttcatcctggcggggcgttctatgttttcgctaagattccagcagatctgcagatgaacagttgggactttgttaatacactggcaaaggaataccacattggcttgatgccaggagatccgtttggcgataacgaatacgttcggattagttacgccgccagtgatgaggccttggctgctgctatgaaggctgttaagcagttggtggcggatgattcagcgcaaacaactgaataaaatttgctggccgacggtttaataataatttagatttaaatggtactcaaaaaggtcgcaacgtaatttttgctaattatgttgcgacctttttgatttttattcaagattcaattatgcgcgcttacgatccttaatggtaaatgaaagcaggaaagccactgcagccacgatcaacgtaaaccacagaccaacgtggaccccattggtaaaggcaacttgatggctgacatgaccagcagccgtgtttccaaatgccaacaaactggtagcgatggcggttgccatggccccgataatttgctggaaggtgttcatgatggtgctgccgtccccggaagtttgttcatccaaggcgcccaggccaaatgtttgggcgggagacatggcgagcggcacacctaacataatgatgatgtgagctaagatgacgtaccacattggcgaagttgagctggctagcagtaatagtaccaggccgacgatggtcacgccaaagcccagcgttgtcagcagtttggtgctaaccgtatctgagaagcgcccagcgatcgcggagacaatcgcgttgacgattccccctggtagcatcacaattccggtcatagcgacgggaattgccaaaccattttgccagaacattggcagtaagtacattgatgaaagaataatggcgaagtccaacatcactaaaacagatccaaccgtaaattgatgcttttggaacacgcggaaattcagaattggggtttcagattttaattggcgacggatgtaccatgccaagagaaggattgaaacaatcaaggttccaatgacttggggtgatccccaaccggaatcactcgccaagctgacaccggcgacaagaccaccaaaaccgatcgctgacaaaacgattgagaaccagtcgattttgggcttggtgatgtcacccacgtttggcaggtacttgaaggccaaaataaaggcgatcaccagaaatggtacaaacaaccaaaaaatccagtgccatgaaagcaggccgaggatcattccggccaaagttgggccgacagcgggcgcaaacatgatgacaagtccaatcatccccatggccgaacccagcttatagggtggaaagattaaagtcgctaccgtgaacatcaagggcagaattaaaccggtggcaatcccctgaatcattcggccgaccagtaaaatggcaaaattcggtgccagtgctgaaatgaccgcaccgacgataaaatcacatagggcgaataagattaatgagcgggtcgaaaaaatccgctgaagcaatgaagacatcggcaagacaatcccgattaccagcatgtagccggtcaccagccactgcatggtgccgatgctgacatgaagttcggcaatcaaacttggtaacgcgatgttgagggaagtttcactcaacatccccacaaagccgccaatcagcatgcccaacattgctaagaatggccgggcaaccggtttggctgcgtgtttttgttttggttcgacagacgcttggtctgcatttaacgatttttccataatgtttctcctaattcttaaaacttttatatcacgacaattgattacactaccataaataaaagctgctcgtaagttttattttcaaaaaatttcataaaacatgaaaacttggtttaacagtggttactgggaacgcttacgaaaaaagtgaaaatatgtagataacggtcacacatttatgccggttttctactacaatataggcagatgcgtagacggatttggcaaacgcatttcgctgaaattattaacggggagcgattgaatatgaaacatacagtgttaatcctgaccggaatcggtgtcgtggttgccggtgcctgccttttgaagtcgatggggtggtttgaagatgactctcacctgtacgatgagtacgaagcgaaataatttgtttggaggaattcttaatgacaaaaaataaagcaattatgatcggtgccggcttggctaacatggcggctgcggtatatttgattcaagagggtaactggaagggcgaccagattactttttactcgattgacgaccatggttcaaatgacggttcacctgccagcgaggctgccggagaatattggaacaaagttcacccaatggaaaacaccaaaggcttcattgcccgtggtgggcggatgctcaactatcgaacatacgttgatctgatggacttattaagccgagtgccttccgcaactgaaccggggatgaccgctgccgaagatacccgtgattttgatgccaagcatcgcacgtttgacaaagcgcgtctgatggaaggcggcaagggcattatcaatggtggcaagatgggcttcaataataaggaccgactgaaattaaccgaattgatcatgatgccggattctaaagaagaacaacttgataacgtcacgatcgctgattacttcaaggatgatccacacatgtttaccaccaacttctggtacatgtgggagacgacctttgcctttcgggtacaaagctcagcgcaggaactacggcgttatatgcaccaaatgatttacgagtttactcaaatcgagcacttggtcggcgtcaaccgaactcggtacaatcaatacgagagtattatgctgccgctgatcaattacttgaaagatcaaggcgtcaacattattttgaatcgaagagtaacgaattttgaatttaaggatacgccaatgcaagacgagattacggtaactgccttgcggatgacgaatacggaaaccggcgaggaagaagacgtgccggttgatgatgacactgccgtgatcttcaccaacggttcaattaccgattcagctacccttggtgatttcaatacaccagctgaagaaaatatggattatggtgctgcggccagcctttggaagaaggccaccaaccggttctataatttggggaatccggacaaattctttaacgatcgtaatgccagtgagtgggtcagcttcactttgacgacaaaagatcatgttttgttgaatgaaattactcggattaccactcaagttccaggcaatgctctgaattcattcatttccacttcaccaattaccccaatgggcaataaggatgtcaacatgtcgattgtcgtgcaccaccagccgcatttcaccacccaaaaggccaatgaatcggttatttggggctacttcctgtatccacgacggaaaggtgagtttgtggacaaacagtacatcaagatgactggtaaggaaatggttgaagagctgctgggtcaattatccaaggttgatccgggacccggtaacattatggataagaagcaggaaatcatggacagcgtgattaactgcatcccagcatatatgccgtatgcatccgctttgttcaacaaccgtgccaagacggatcgaccaaaggtgattccagaacactcaaccaatttagctttcactggtgaatttgtggagcagccgtatcaaatggtcttcaccgagcagagtgctgtccgatcgggagaaatcgcggcttaccactttgccggagtgccaatggctaagctggtgaagaaccctcgttatgacaaggatattaagactttggccaaggctacgcggaagatgttcgagtaatctggcctatacgtcggttgaatgagtcttaaaagcaacgtttaagccacatacttaaacgttgcttttttgtctttgaaaactatcccagtaaatgaggataaccatgatgagttgtacaccttcgacgcaccaaaaactgctgagaagagtcacctgacattgattccatattatgcttgggcaaatcgtgacgaaaagcaaatgaacgtctggatccaacaagcaagaatctaattgccaggattatatgagtggagttgaattaaccacgttagatatttgaacaaaacaaagaatcctcctgtaaattgttctcattggtttacaggaggattcttcattacataaattgactaccggcgccgtcatccggtgtgtttggttttagactgatgtatttcttacggtattcggatggcgacatgccatagccttttttgaaggccattgagaagtaatagacgttctggtagccgaccttcgtggcaatcgtactaatttggtcagaagtcaatagcagatacttggttgcttcttccaaacgatattttgtcagtagattattgggggtgatgccgaatgttttcttcatatataaagaaacagaattcggatggatatgaaattccttgcccaactcttcataggtaatcttttcgtcaaaatgatcttcgatgtagcgctggatcttgttggcaatcatcgtggttggcgattcttgcggtgtttgaacctgaatctgctggagcaggtccaaaaataattgctgggccttccagaactcaattgaattttgggtggtgtcagagtggttttcattggacttacggctgttggcaaagatctttttgatcattgagatcaccgtatcttcattcggaatcggctgttgcttctccaaaaataaggtaatcgctgaggtatagtaatgaattgccggcacggggatgactggtcgcatctgctttggttccggggcttggacgtaattgccggctgtcgcaaagtgaatccagtagtattcggtggtttcatccatcggtttccatgaatagtgatggtgctgtggttggagaatgaacatctcaccggcactcacggtgtattcggtattatcttctgcgataaataattttccgcgcttcatgaacatcatgacaaagaattggaaattcttccggttgggatgccgctcaccagggctaaaaaccacgtggccgctttgaatataggtcggtgtcgggatacatgaaatcgataggaattgcttaaccatagaataacctccagtgcaaaatcgaattgtttgctgatcacaatttggattttataaatctttcttttgttattataaaaatagttcagaaagcataaaaagtcaattggaaatcagctttttatttcacaaagaaatcggctaatgactacttttacgcgaattcttgcttgttcagcaaattataaaagcgcttttataaatatgttttattttataaacacttgatagatttttagattcaattgatgccgtttacacggtattctatacatcgtaagcggttacagaatcagatgatttgctgatcacattaaataaatttgttttcagaaaggacaattcaaaatgaaaccggtatcatattacgacattaaatatttgccagattcgactttgaaagaaacgttcgaaagaaacattaactggatgctttccctcaccccagaccaattgctatacaactacttgctgttgctactttcttagccttcaccgcaccaaacctgcatagtaccgctaagctctggtatgccgggttcacttatatcttggccgctggtgttatttacactggtattcaaacaccaattactgctattcttcctagtttgaccactaatggccaggaacgtatcaatgccaacacattccgtatgtgtggtggtgccattggtattcgataaggtggtgatgcattcattcagaaaattgcagtatttcacaattcggacattatttctgacataatgctttcacgaaccccattcgtgttccgagttatccactaataaatcaagaggctcaaatcgttgaataaacggtttgggcctcttttgttgaatatatatttgataaatataataaaatgtgaagacttctaataaaatttctgctaagatattacctaatgatgtaaatgacggttgtgagtctacaaccggtttacaggatgtatttgtcacacaagctaatatagaaagtgggaataattttgaccaacgttaagtcatatattgaatcaatcaaagatcaaattgatcgtcgagatccgaaccaaaccgaatttcaggaagctgtatttactgtcctggatagcctggcgccaattttagaggcccatccagaatatgtgaagagcaatctgctcgcgcaattagtcgagccggaacgggcaattcaattccgggttccttggcagtcagacgatggccaattcaatgtcaatcgtgggtttcgggttcaatttaactccgccattggtccttacaaaggcggtttgaggttacatcccagtgttaacttgagcgtggtcaaatttcttggcttcgaacaaattttgaaaaatagtttaactggtttgcccatcggtggtgccaagggtggcagtgattttgaccccaaaggcaaatctgattctgagatcatgcgcttctgtcaaagctttatgactgaattacaacgccacattgggcctgacctggatgttcctgcaggcgatattggtgttggcggccgtgaaatcggctacttatttggtacttataaacggctgaatggttaccaaaatggtgtgttgactggtaaaggattgacgtttggtggcagtctcgcccgtactgaggcgaccggctttggcctgctgtattacactaacgcgatgctaaaggcacagggcgacactttaaccggcaagaagatcaagatttcaggggccggcaatgttgccacctatgcgattcaaaaagccacggaactcggggctaaagtcatcaccgtttctgattccaacggctacatctatgaccccaaaggaattgactacaaagttgttcagcagattaaagaagttgaacgcggccggatccgtgaatatgccgaccgggtggcatccgctgaataccacggtggatctgtctgggactttgacgttgactatgatattgccttaccatgcgcaactcaaaatgaaatcaacaaggatcaggcaaaattgatcgtcaaagatggtgtcaaatacgtctgtgagggtgccaacatgccgagttacccggatgcgattgccatttatcgggacggcgatattctgtatggcccggccaaagcagccaatgccggcggcgtggcggtatccgctttggaaatgagccaaaacagtgaacggctggcttggagctttgaaacggtcgataaccggcttcaagacatcatggaagatatttttgccaagtccgaagctgctgacaaaaaatatcatttggataaggactatcaagctggcgccaatattgctggatttgagaaggtcgctgaagccatgatggcacaaggattagtataaacacttaacaagatggaactgaatttttggtggaaatacctttgatgagcacttattgaaagcatcaaagatccatcaatctctcagttccaactttttgtataaaatatacaaaatatgaataatatctatttgaataattagacaaatactcatcattcccttaaaatcaacccgcaagcggctttaagcttaatgatatgtgaggtattgcgacatctaaattgagccaacctcttcccatagtgctgataaaatgctatattttataaaagccatttttgaggagtgagtattttgaaaaagattagaagattattaattatatttgtgtcggcgttctcgtttttattcctaatgaataatgttgcatccgcacaatcgaaagaacactacacaattggtgttggaccgacctttgtgccgtttgaaattcaagccaagaatggatcctacaatacggctcaccccgggctcgatattgaaatccttcgggcagccgccaagaaggagaacttcacctatacgttgaaagtcatgaactttgcggcagccattcaagccttggaaggcaatcaagttgacggcgtgattgccgctatgatggcgacgccggaacgagctgagaagattgatttttcaaaaccatattataacgtcgggctcgcattggcagtgccaaaggggagttcgattaaaggatataatgatttgaaaggcaagaccgttgctgttaagacaggatcaacctctgagcagtatgccgaaagtattcaaaagaaatatggttttcacattacccggttcaacgatagtaacaccgagttgagtaacgtcttggttggaaactcggctgcggcgattgattccacggccacgttgttatactcaatcaaaaacaagatgaagctccagttagttgggaaggctgccaataaaaatccggttgccttcggggttaagaagggtcacaatcaggaattactgaaacgctttaatgccggtttggcagctatcaaaaaggatggcacctacgacaagatcgtcaaattctacaccggtgagcacagtaaatctgcgattccagtgcaatccagttctgatcggacgtactttggcttgttgaaaagtaacgccacctcgtttggcaacgggattaagatgaccctggagatcacgattgttgccattttcttcgcgacgatcattgggatcatcctcggtatcttgggcgccacgccaaacaagttcctccgaggattgtcttccacttacgcctttgtcttcaagagtattccagtcatggttttggcattcttcgtgtacatcgggattcccaacctgacaggtgagaaaattccactgtttattgccggggttatcaccatcgttatggaaaacagtgcctatacggcttcctttgtccggggcggaattgaggcagtcgaaggcggtcagatggaagcggcccgctccaacgggatgtcctatttccaagccatgagatacattgtcctcccgcaagccttgcgaattatggccccatcatttatcaatcaattcatcatcgcgttaaaagggacctcggttctgtcggcgatcggggtggctgaactcactcagcaaggaaccatcattatttccagaaacatggaaggtttcaaagtttggttgctggtatcgttgatgtacctggcaatgattgggttgttgagttacctgtccaatctcgtgaagaaacattatcaattggcaagttaaagcgaatctaacttaatagcagcaagaaatgagcaggaccaccggcaaatctggtgatcctgctcattttgtttcttttagttcaagtattgttggccaatttctttgtatgtgtcaatcatattgtagtaagtatccagatcaatatattcatcgtgctggtggctggtcgtattccccggcccaagaaccaccacatccatcttttggttcactcgagtgtattcagaggcatccgttcccagtgacaccccgatcgttggcaggtccagagattcatgcaagtggtgggcgccggctttttgggcgatgtcgataatcgctgatccgggatgattgatcaccggccgtttactggtaatatcgattgtcaggttataccctggctgttgatttaaatgatcaatcagctgatggagcttcttgatgatcgtttgattatcgaactcagggatcgtccgaattttaacttttaagctggcaatgtcaggaatactgttgatttgtttaccaccggcaataattgtcggagcgtacacggtatcgcccagaattggatcagtggcttgaatgctttgatagaactgcttttccttgaggtagtaattcaccagcatatcgatggcgttgattcccatctttggcattgatgagtgggccgccttaccatgggcaacgacctcatacatcagccagcctttatgggcaaagaagataaaatgctgttcaggcgccttttggtcatgactgacctgatggagcttggctgccaattctggcgtgaatttagcaccaccgctatcgacataggcatcgaggcgttctttagagactccactgggctcaccgatcactacggcgtcgagatcatctacgtagcctttatcagccaataattttgacccgagctcaccgacttcctcacccatggtgacataaagcctcaagatgccattgtggacgctttttgactccaccaggctgatgaaggcgattgtcaggccagctagaccgcctttcatatcggcagctccacggccatataaccggttatcacggacattgggttcaaaaggtggcgttgtccaagttgataaggccccttcatggacaacgtcggcatggccggagaagcccagaaccgggccaggattacccgtgtcaaattcggcaatcaagttatctcgatcttcggcgtatttgataaaagttgagcttatcccgtgtttggccagtaggtcgtgaatataggcggttaccagatgctcattgccattgacggtgcgaaaggaaatcagatcttttaaaatcctcagcttttcattattatccatattgtattattccaccttatctttctgattaaaatgagctaacagtgccaatgcagcctgctcgtggaacttcgctgcgtacttgaggccctcggggttggcaataaagtccgggtgatgtaagttagcctggcccttgctacccatgaatgcgtaacagccgggaattaattgctcatactcggcaaaatcatcatcggcgttggaagggatggcatcggtgactttcatgaattggcttgcctggtttgcgatgaggtttgtgattgcttcactgttgtccaccggagcgggtccctgatcccatgtaatggttgctgtttggccataagcgctggcggtggcattcacaatctcgtaaaagcgccgtttggcaagtttgcggtcggcttcggaaaaggtccggatggttcctttaaagccggcactttccggaatgacattgttgacatggccgccggaaatcgcaccgactgtcaggactagccgatcagaaggcgagatgttccggctgacaatcgtctgcagggtcataatcgtgtttgcgacagcgacgattgggtcacggccggtttgcggcattgcggcatgggagccaactccggtgatggtcacgtcaaaattgtcgttggaggccatcaacttgccgattttcatgccaacggtccccactggaatggttggcatgttgtggattccagagattgccaggacatctttaaggatccccgcatgaatcatttcccgtgcgccaacgtggcgttcttcgccgggttcaaagattaagcggacattgccggataactgcgattctcgttcttttagtaacttcgctgcccctaagagtgccgcaatatgaaaatcatgtccgcaagcatgcgctgcgccggagatttctgatttataaggtaaatcagtttcttcttggagcggtagggcatcaatatctgcacgcaacgcaattgttggaccatcacctggaccaatttgggcgacaaggccgctttgaatagggaagtccagaatggaaatcgccattttatggagttcagcagtaatcttggccgtcgtccatttctcttgatcacaaagttcggggtggcgatgaaattgtttaaattgctcgatcatatagcgatcgagttcgtctgtaacgggcgctgtttcaaccatcctaatcactcctaatcattctttaatatatatttaataatactttaagagtttaagaaaagatagtcaagcaaggcttaaaatgtttcgtgaaacgacttaggcagattaagcttattcaataaatgggccggagaccttttgtattggcggctgatatgatacatttaagtgaaacaatgcaaggaggaacacacaatgggactattaattacaggaattatcatcatcgttctaatcgtgatcgttgtcgccttatacaacggcctggttagccaacggaacctggttgacgaagctgccagccagattgacgttcagcttcagcgacggggagacttgctgcccaacttgctggaaaccgttaaaggttatgccaagcacgaacaggaaaccttcgaaaaagtgaccgcaatgagatcacaaattcaagaccccaacgccagtctgggcgataaggttaaagccgataatgaattaaccggggcgttgaaccatttgtttgcggtttccgaaaactatccggaattaaaagcaaaccaaaatttcttggcattgcaggaagaactgaccaataccgagaataagattgccttttcacggcagaactacaatagcaacgtcatggcatataacaacaaactgcaaaccttcccaagtaatttggttgccaaattcggaaccttcccggctcgttcttatctggaagttcctgaacaatccaaagaagtaccacaaatgaaattttaaaggggcctgactgataatggataccataaatcagcaagttcagcagaatcgacgacgaacctggtcagtcatggctttctttgttgttttaattgccgttattggctttctaattgggttggtgtttgcggttgccacccaagatgaaagtattgattggctgattccgacttacacgatggtcggctttctcattggggcgaccatctattcgttctttgtctacatgagtgtgaccaacattttgatgaaatctgccaatgcgcatcaactccaagaatcagacgacccggaattgtttaacattgtcagtgacttggtgatggttgcccatatcccaatgccggcaatctatttgacggatgatccttctccaaatgcctttgcaaccggaagagatccgcaacacgctgcggttgcggttactaaaggtttgcgggaaatgatgaaccgtgaagagttggaaggggttttggcgcacgaaatctcgcatatcaaaaactacgatatccgagtatcatcgattaccgttgccttaaccacgtttattgccggggccgggacagttctgattgtttccggaatcagcttaatcagaggtggccgttggttcagctggttcggcagtgacagcgacgatgatgccaaatccagttgggcaattgcggttggaattttagtttttggactcatcatgtggctcggcggctggatcatccgcgcagtcggagtgccagttgcccaaatcctccaattctccgtatcacgtgaacgggaatcattggccgatgtttccggggttaatttgacccgggatccgcaaggcttaattaatgcattaaccttgttaaaaaatgacaccacaccaaccaacaatccgactgccaagagtgccgcgctttacattaatgagccggtcaccagacaagggaagacaccctttttggccaagatgtttgatacccatccaccgttggatgagcggattgctagacttaaacggctgctgggtgaacaataactaattcaaattatgtatgcaaatgggcaaccgactcgtgttttgacacgtctcggttgcccattttatattttagattatgccacttgtgcactaggcgtaattttggttcgattgagcaatactgaactggtaacgactgacagggaactcaaggccattgccaaaccagccaattcgggactcaaggtcattccgataaagtagaatactccagcagcaactggaattcccaatacgttatagacaaaggcccagaataggttcaacttgatccggttaaatgtcttcttgctgagttccaatgccttgtaaacatcgcggagatcatttttgactaagacaattccgccggactcaatggcaatgtcggttcctgatcccatggcaatgccgacatcagcggtactcaaggctggagcatcgttaataccgtcaccgacaaacgccactttgccggtgctttgaaattgcttgacctggtcggccttgtcggctggcagcacgtcggcaacgacttgatcgatgccaacttggctggcgattgcctgtgaaactgcctgattgtcaccggtcagcatgactgtctttagtccttgtgatttaagcgctgagatggcatcctttgaagttggcttgggagcatcttgaatggcgataaggccaacaatttggtgattttggccaacaaagacgacagttttggcttgtgcctgtaaagttgccatttgttgtttaaatgtgtcactgacttcaacgtcattcaacaacttggcattgccgacaaaggcactttttccatccaccacggctcggacgcccttgccttcaatggccgagaagttttcagcaggtgagtaatcaatgccgctatccttggcattcttgagaattgcggttgccaatggatgttcggatgaagcttccaaacttgccgcaatctttaagacttgggtggtgtcaccaacaatgtctgtgacctggggcttaccaaccgtaatcgttccggtcttatcaaaaatgaccgttttaacatcgttgacagcctctaaaacttcaccatttttaatcaggattcccattcgcgcactgcggccggtgccgaccattaaggcggtcggggtggccaaaccaagtgcacatgggcaggcaatgacgaccactgagactgcaaagatcagggcgttggcaacgctggcaccaatgaaaacgtaccagattaagaaggttgaaatggcgattatcaataccagtggaacaaagatttccgagactttatcggttaatccttgaattggcgcatggctattctgagcttttttgaccaattcgacgatctgagccagcatggtgtttttgcccactttggctgctttaaaagtgaacgttccggttccattgaccgtggcgccaacaactgaatcaccggcctttttttcaaccggcatactttcgccagtaatcattgattcgtcaatcgtcgatgatccactgacgatttggccgtcaacagcaatcttttcacctggtcgaactttgatgagatcgccgacgacaatctctgagattgggactctgacgatcttgccatcgcggataacttcggcatccttcgcctgcaaattgaccaatttttcaaccgcattggaggcgttgttgcgcatccgctcttcaaagacctgtccaagcagaacaaaggtggtcacgaatgctgcgctttcaaagaacaccggctgatgagttgccatggcgtaaatgctgtaaacgtatgccgtggtcgttccgatcgctaccaaggtgtccatattggagtgatgctttttaaacgatgcccaggcactattgatgaatgggccggctgcgacgatcattacgattgtggtcaggacaagcattgtccattcaccacccgggatcatccagccgaagggcttgagaatcatctcggccaacattggcagcgaaaaaattagcgcaatccaaaatcgttttgtgatagtcattagataacctcaactttccctttgaacatgtccatgccacagctaaaaccaaattcgccagcctggtccgttggcacttgaaccgtcttggtgacgttgactgggagttcttcagaaaagccaagttcattggaatggacaacatccaagcacccctggtcattaatccgtttgaaattgatttcggctggcacaccctgcttcaatttgatgacagatggctgatagcccccggcgacggttacgttaactgtttgtttattttcattcatgattgattcctccatttacttaatcactaatttaccgtgaaacatatccattccgcaggcccattggaactctccggattggctggtatcgatttcaaccgattctttttggttctgcggcaacgcttggttgattccaaaatccgaaaagacgactcgatccaaacaggatgacgaatccgttcgggtaaagttcagagtcgcgggaacgccttgcttcaacacaaccacttccggtgaatagccacctttgacctcaacatcgacgacttgctgatcatcgttaaccttggcgttggcttgagcaacttggtgcttgccgaagaaccaccagccgataaaaccaatcaaggctaatccagcaattaaaacaactattttcaaaaacccatctcctattcgtctaaaatctacatgtgtaaactttaattgtctatatcttatcgtcaaaggttacacttgtcaacgtgaaaaatggaaattctttcaaaccttgactgcaagtggattctccaaggccgtgtcaggcattccaaaaaaagtttccaaattttggttgacaattaaaattacgtgagttagattataggcacattaaaatttggttgaaaaaatgcagcgatgaggagagtagattcgtctaaccatttcagggagtcccgttaactgagaagggatgatggttatcgaattgaaagtagcctctaagcagtagatgcgaagcgatgagtatcttcggtgtgcaccccttaaagtgccagtgtatcgtcagcaatggccgtacatgatgagacgatttgtgtgagcagatcgtgaatttaggtggtaacacgcgaaagcgcccttaatcttagagataagattaggggtgcttttttcagtcaaaaataaaataaaaaattggagtgtggtttttatgaagtttgcaatgattggtgcaggagcaatgggattacgatatggtattttactgcaagaggctggcaacgatgtcacatttatcgatacatggcagccacatatcgacaagattcgtgaacagggtggcgtatatgtgatgcgtgatcataaggaccgccacttgactaagattaagttagaaaccccagagacctttgatggccatccggacatgtttatcttctttaccaaacaaatgcagctgcaagattatcttgatcgctgttcacatttcttccacgaagatcaatacgccttcactgcgatgaatgggatgggccacattgaaaaactacagaagtacttcgctgatgacaaaatcattggcggaaccgcattaattgcgaccgtgcttcccggtcccggcgaagttgacttcatgggtaagcggggtgccggcaagatgaacatgtgcccactcaacgaaaagccggacgcaatgtgccaggcactcttcgacgagcttcaaaaagccaagatgaatccaaccttaacggatgacttcaccggaactttgatgaccaaggttatctttaactcagttattaacaccatttgtacgatgtttgaattgccaatgggtgaatttggcaacttcaaaggagcttatcaaatgggccggcaattgattgatgaagcctatgacatttgtgcccgagccgatatcaaattagtttccagccgtgacgaagaaatggctgcccttgaccataacacccgaatcgatatgccgcttcattacccatcaatgtatcaggatatgattaaggaccggccaactgaagttgattacattaacggctacattgccgaacttggccgtaagtaccattatgaagccagcacccatttgtttgttacccaagctgttcacctggcagaatttcatcgtcagaatttggccaagcaacgtgccatcaaggctaagcaggaggccccagcagctcagacagcatagtagccgaggggatgaacctgataattggcagccatccgctcaagcgtcttaaagagatcagcttgttgatcacgggttccagagacttcgagataaaatgaatagacgcctaactgcgttttggtcggcaaggacattaatgccaccagatttaattggctggccgcaaagtagccgagaatgtcgtagagggttcccgggtgatcgttgaaagccggcgtgacaaatagtggtgccttgaactggtcagtcactaatgtttgctgggcaagcctatccaggtgcgcccgtcttgatttgaacacaatgaaccgcgtgctgttatcgtcttggtcggcgacattatccatcattaacggtacggataaatcggccatctgcgattgggggatgatcgccgcgtcacccggctggccggactggaacttctccagtgaaatcatgtttgatgatgtggtgataatttgcacgttggggatggttgacaataatttctggcactgaccttctgtcttgaattgaacataaagtcgtttaatttgctgtaaatcagcaacgtttgccaccagtccaaaatcaaccggaatggtgacttcgccgatttccgtgacgtcggcggtctgcaggcgttgaagggttgcggacacataaccgtcaagctggttttctaatggcaataaaccaatgttgtcgccggaaacggcttggtagacttgatcgaaagtgggatgatagtcaaaagtcacgttggttaatggctgggttttaagataagctttcgcggctgcgtcggcaaaggtgccggctggcccgaggactgaaaatttcatgatataaccaccttgtcgttggaattgagataatgctgttattatctcacactggatttcgaaataatgataaaaatgaaagaaaactcttttgatatctgtggaagcggaaaatttcctgatattggaagagtttttgtttttgttaaacaaaagtaaagttgtttgacttcattccaacgagtaactactattaatattaacgtttaagggggattaacaaaaatcaatgaaattagcaaacatcaaaccatcaaaatttaaaacactgattttaccgctgacggctattactgccggcagtttttgggttagtctcaaactctttgacatcgcgtttaagcgggtcgattatgttcctgaaacttcgaaagaaaaacagcagtacgccgatctctactatcaatatgtggattggttccatcaaatgccctctgaagaatggtatttgaaccgcaatgatcccgacaagcggatggtggcgacttacattcctgctgaaggtatttccaagaagacagttattatcgcccatgggtataaggggaaccgggaaacaatggccaattacgccaaaatgtttcacgaaatgggctttaatgtcctgacgcccgatgaccgtgggcatggtgagagtgccggaaaatacatcagttttggctggctggatcgtctggattacctgaagtggatcgatcaagtgattgaccacgtcggcgaagacggtaaaatcttactcttcggcgtcagcatgggcggagccacggtggaaatgctgtcgggtgaacgcttgcccactcaagtcaaagccatcattgccgattgcggctactcaagcattaaggaagaactcacttatctgttgaagaaacagtatcatctcccggaatatccggttgaaccaatggtcagtgagatcaacaaacgggctgccggatttggtctcgatagtgcttcatcggtcaaacagctggccaagaacaaacggccaattctatttatccatggtggcaaagacacttatgtgccagcccacatggcctacgagaactaccaagccacccacgcacccaagcaaatctggattgtcccgaatgctacgcatgccgagagtttctggtatgatccggtggcttataagcggcgggttcaggaatttctgagaacttatttttaatcattgaaacaaactgaaaaagtgttggacatctgaaaatgcccaacactttttctatttataatgacgtcatttatcgttttcaagtttacattaaaccaactggttatacttacgaaaagtaagtctaaatgctggcattccattttcagcatgcctatacttaataattgaaccaaagatatattggtgtttcaccattacatgatatctaaatgaaggagattttgttgatgactaagatgattgcaggacaagctttagttaaagtacttgaagactggggcgtggaccacgtctatggaattcccggcggctcaattaatcatactgtcgaaggactctaccttgaaaaagataaaatgaagtatattcaagtccgtcatgaagaggttggcgccattgctgcttctgctgatgccaaattcaccggaaaaatcggtgtcgcatttggttcagccggccctggtgcaacacacttgttcaacggattatatgatgccaaaatggaccatgttccggtgttggcgttagttggccaagtaccacagccaacaatgaataccaattacttccaggaaatggatgaaaccccgatgttcagcgacgtctccgtttataacaaacaagtcacaaccgctgatcagattccttacgttgttaaccaagcgatcaaggaagcttatcgccaaaagggtgttgccgtggttatcttgccagaagacttaacctctcaagaaattgattacacaccaactcgcacgccattaacggttgctgacgatttcaaacagagcgtggatccgaaagctgtcgacgacactttgaagatgattaaagaagccaagcacccattgatttatgcaggccgtggcttgttgggtgctcgtgataccttaaccaagttctctgagcagtttaacattccggtgatgaacagtgtgccagctaccggtgttattagcactgaccatcctaactttgtcggaacgactggccgtctgggcaccaagtcaggatttgaggcgattcaaaacgccgatttgatcttattcttagcttcagagtatccatttgccaactattggccacaagataccaagatgatccaggtcaataataacccttacgatattggtaaacgaatcgacgttgattacgccgttatcgctgacgccaagagttacttacaagcaatgattgatactggtgagagtcggccaaaagatgcttggctcgaagccaaccaagagaataagcagaactgggacaaatggctcgagcaattggctgatgatgacagcgatggtttgaacgccgaatcagttaccaagaagattgccgagttggctggtcctaacgatacctatgccgtcgatactggaaatgtttcagagtggggtgtccgtggcctgccaatgaacaagaaccaacgcttcgcaatttccggattgtttgcaaccatgggctttggccttcctggcggtcttgctggtgctttgagcgttccagatgcacaagcttggtcactctctggtgatggtggttttgccatggtcgccccagatattttgactgaagttcgctacaagctgccagtgatcaacgtggtcttctcaaatgaccgcttcggcttcatctggtacgaacaaatgcagaccaagcagcacttctacggtgttgacttgaacgatgctgactgggccaaagttgctgaaggcttgggtgcaattggcttcactgtcaagagcattaaggatctcgatgaggtctttgccaagattaaggatctgcaggcttctggcaatcaaaagccaatcgttatcgatgccaagatcaagcaggacgatccggtcgcaactgcctttatgccgttggatgctcaaaagtacggtgaagagaccgctgaaggatttgcaaagcaatatcacattgatcgcaagcaacaaccatcattggaagaattactgcgttcaaaggaaaagtagtcgatatatgagttcgtatgaaagtggtcaaatctttacaatgatttggccgcttttttacgtttgcttcgagacaatcagaattaaaagaaactgaaccgttgccggacctgttgatgagttcataatgttacaaaatgattacaaagactaggcagagattgatatacgagtttgtgaattttacattaatgaaacattgttatatcagcctattcatgactaataagattgtgcataatcaaatggtaaccgctaacttaatatttggtaaaggtgaaaatgttacatcaacatttcattgacatcatcctgtaacgtggcataatgagtttaatcttttagggaggtagcatgattatgaaaaaatttgcaacaatcattaccgtagcttcactggcattaccacttgcttttgcagccccattggccgtatcagccgcaacaacaccaaccacgactgcagccaagaccaaaggtaccacttacactattgctaagaacggtgttaagaacttcaaggcgcgggcatatcacattaagaagaacattaccttatataagggcttcttctatgccgatgctggcaaggtaaccttcacacctaaaggtaaattgaccaaaccaatgacatatagtgtcacccgttcggtcacagtcgctgcaactaagacatccaaggctaagacattcttatatgttaagggctatggttacgttctttcatcacaaattaccaaaggacgttacatgtcagctgactaattgaatttgaataaatgattaagcttcatccttctataatctggtcaagagcaattgtgttcttggcctttttatatggggtataattgagaaaattgatattgaagaggcgattgcaatgactgcaactttaactttaattaccggtgctgataaggggatcggctttgaaacggcgatggcgttagctaaactcggccaacatgtcttattgggatcccgccatcaggatcaagggcaacaagccgttgataaaatccggcaggcaggttatgatgccgaactggtgattttggatgttaccaaacaaagtgatattgaccgagcaaaggcaacaattgatgaaaaatacggctacctggatgttttgattaataacgctgggattgcattggataatcacgaaaacgccgaaactttgtccacgaatgtgatccggactgagtttgatgttaatttctttggcaccgtcagcatgatccaggcgtttattccgctgttaaagaaatccaagtctgccaagattatcaacgtttctagcaatatgggctcgctggggctggcgtcagatccgaattcgcgcttctataacgttagttccctgggctatcagtcatccaaagctgcggtgaacttcgccacgattacatttgccaaagagctcaaggatacccacatcaccgttaattctgttaatccgggatggactgcaacttcttttggcggccgtgatgtcagccagccggtgccacaagggatgcagtcggtccaccagggcgcccagcagattattaagctcgccagtgatcctgccaatgaactgaatgggacgtttactgagaatgaggggacgcttccctggtaagttgattctattcaaaaaacaacaacggcaccaactcgatctgctcgggctggtgccgttgtgcgatggtcattcattattcactttggctaataattttttaataaaggcaatgtagattaaaaatttgtcattggtcagtcggtaatccagaccagttcgtttgtagatcatctccagccgataacgaacggtgttgggatgcgtaatcagagcttgactggtctttttgacggattcgttttgtctgaaaaattcccggatggtttcaaacatctcgtggttctccaataactggtccatctcttccgggtacagacggctgtcttgaactctcgagagctttttcaccaagtcccacaggctgacgtcccggtaaaagatgggtcgtcgtgaccagtccaaggtcttagcgatgttgatgccgaagctggcctcaatataggagcgatgaattttttggccgggtgggcattggagacgccttcgtagacggtaaaacgaggaatgcggacattactaatcagccgtttaaaaggaatgcggtcatcgggcggcaattccatttgttcgtggtcaaagaaggaaatcgcggtcgcaccatcagctgattcaacgataaagtaggttttgattcgtttttcctgttggactcggtcaaaaaacgcccggatttgattcatcaggttaaactggacagcgattcgttcacttggtttgggtatttccgataacgagattctggcgactctcactttgagactgtataggtcaacgttcttcaaactggagatgaagtcgaagtctttatccgaagcggaattggtttttaataaatagtccagatccaaatcggccatcttattgatccggcggccctcaaatagaatggcgttaatgtcattcatgatttgaatgtaggtggtattttcccgaatttgaaatagcgggaagtctaagtgcgtacagtaatcgattaacgtctgggggatgtctgattcctcattgtctgcgtaaggtttaatcatcaagcagctggcttgtttttccactaactggtgaatcaacgttttggctgtctcaatcttttcgggcatcatccgagaactggtaatcacgatttggccggcctgtgcccagccgtcagccgtgccgctgtccataatggtaatcgcgttgaccttgcgattggccaacggtacctggttgacttgaacaatgtacttttgctctttattggcgattttctgcaaatcaatcacaaagctcacctccaaaatccgacggtttcattaccattatagtaacgcttttttaaatcttagtacatatgaattgccaaaatgatagctgttttgttattgaatggtttgtcgagagcagttttggacatttgtgctaaaaaaccgctaattttttggaggatggcacaaaccttttaggctgtcgggatgatacactcatccttgaaagatgacatccttcaacatccttcaaaatggaaagaacgagtgtttattagaaggtgtacgccatgtatttacttgatgtgattcaatattgtcgatgtcccccaattggggaatcacccttccattgccatcatgacgcttggagttaagatccccttcagagtgttactagacttacgagtggcagaagctgttagatgatgcagtaatatcaactgagagtgatatttaaccactaacatcggcagattagtggttcatcattgacggcaacatgcaccttgatggcagcaaaaagcacgttggtaaccagcattcagtgttggtcatcagcgtgcttttgtttattataaattaaagttcaacgccgttaacaatgtaatccggcttatcacccttgtccattgcgacggtattcttagcaacaatctcagccatcgcgtcacgtgcttctacggttgcgttaccaatatgtggtgttaagatgacgttcttcaatgctttaaagccatcgtcaacttttggttcggcttcataaacatccagaccggcaccggcaatttcaccgttttgcaaagcggttaataatgcggcttcgtcaattagcggtccacgggcggcattgatcagcattgcgctgtccttcatttccttgaactgctcggcacctagaagatggtgggtttctggagttgccggggcgtgcagggtaatgacgtcggcgttcttgacgatttcatcaacggtggcaaatttagcacctaatttttcttcggttgctgaatcaagttgatgacgttggttgtagaggatcttcatatcaaatgcgtgcattcgtttggcaaccgcctgaccaatttggcccatgccgataattcccaaagtcttgcctgagagttcgtggcccaagaagaacagtggtgcccagccagtgaagcccttggtccgcatgagttggtcaccttcaacgactcggtgggccaaactaatcatcaaagcacaagtgacttccgccgttgaagtggtcgaaacctttggtgtgttggtcactggaatgccctttgatttggcataatcagtgtcgatgttattaaatccggcaccatagttggcaatcagcttgaggtttggggcggcgtcgattacatcagaatcaactttcgtggaaagtggtgtgatcaagaagtccttgtcagcaactcgcttgctgagctcatccttggtaatcagattttgactgtcatcaaatacatcaatgtctaatccggcatccttgagaatattcaaggcgtgctctggaattcgacctgcaattaatactttcgacataaactcactccctaacaaatatttcatacaactccattatagggcatatcagggctgtatgaaaccgcttttatgagtaatgctatcaactgattaactgaatgacagtgacaatttggtagggaaaacccatgttgttttaagctaaaatagatcttagaacgactattcgttaaaccattgttatatgcattaatcctttgatcggtttcgctgaaaaaaccaggtaacaattgaaccaattaggataacgacgcctataactaagaaaataaggttcataaccttatcaactatatcagcagtccccttataaagggtgtatccgctatctgcgacgatccaaatgccgattaatacgctaagtaatagcccaaccaccggaacaactccagctttcattttctttttcatacgtaactcctttcaagttgtctcaggaatcagcctacatccataatgctgtccatattttttattaacgtgggcaataaagtggatcggaatatctggtatatttccttttaaaaatgatatgttcgtttttattgcctttggggctaaattaaaatgtgttgctgcgtgaattagacccagtgcagtggtaccatttttgtctgtttgtgcatatttacgaattgttgatattgatactcgtgacccataatacttcaatatcatcgccagagctgcagccccacagtcggtttcatctaattgactgacataataatgattccacatcatatttttcctccatgaatgccatgctcaaatttttaatcgacaattaaaaattaagtaagatattttctaatagacatattgtaacattattttggtgattttatataaaatattgtacctaataaataatattatacctaaaaatattaatgtggtatataatgtttatgattagacaatggactctggaggactagttatgaatgtttcacagaaaatacaatattgcagaacactaagaaatcttacacaagatgaagtcggaaatttgttgcacgtatcgagaaagacaatttcaggctgggaaacaggaaggagttctccagatattctcagcttagtcaaactttgcaatctttttgacatttctcttgatgatttgctatgtgacgaacatatgattgatcgtgattaccatggatagggttatagttaatggccaacaacaagaaagcttcaccaacgagatagaaatgtcattcttgctatgtattttaaaaatttgtagattgctcctaggttgcacagaaactcgttaaatatcatctttacaaattactattgacattgtactaatggatgtctacaatatttattaaacaattagaaaacgctgtgagaaagttgagtagcgtcaagacaacctgaagcgagcttcgtttggtgagaggaagcaggaggattgacgcgaaaatcccttttgagcgatgtaccgaagaacaagagtaacgtgcattggtgacacccattatcgtgttagcgtatcgcttttttggccgtacgtgaaaggcagttgtagcgatataactgcaaatataaggtggtacagtgcagtaggcgcccttaattcagcattagctggataaggggcgcctttttagttgctcaaaattcggaccgttttctagtgaatcttgataggaaaagagttggtgaaaatgaaatctcagattgatattagtcagattaggaatcaaattcaggacttaaataatttattcactaaaggagatcttcatttatgcaggaattacatgacttaaatccaagcccattacggaaacgcgattatttcgtcgtcagctcaatgttatttggcctcttttttggagccggaaatttaattttcccaattcatttgggccagttggccgggggggcactggttactcgccgcgggcggctttttggtgactgcggtcttgctgccgctgttgtcggtactggcaatcagtgtgactcactctgaaggggtctatgacgttggaaaaccccttgggcccgtatttgccttgacattcatggtattgattcatgcaaccatcggcccattatttggaaccccacggacagccacggtgccatttaccgtcggggtgcagccactcttgccgtcgtcgatggcccatgttggcctgttagtctttttcgccgtcttctttggcttagcttttctggtttcttataaggaatctaacgtcatgacgtcagttggaaaagtgctcaatccagtctttttattgctattattcagtgtttttgcattaggatttgccaatccgatgggcgttgccggcaaacaagccgtcaccgctgcttacaagggcgattccttcttcaatggtttcctgcaagggtataacaccatggatgccttggccggtttggcatttggggttaccgtcgttacggctgttcgccagttgggaaagaccaagcccagcagtaatgccaaagtgactgctaaagccggtgtcttcgcaacgggggccattggcttgatctacctcgggttgatctggttgggtgccacgacactttccacgtataaggcatctgccgacggtggtgtggccttcaaccaattggtaacttattacctgggtggtctgggtcatgctctgctggccactttgttaaccgtcacttgtttgacgactgccgttggactggtggctgcctttgcacaagattttcataatcatttctctaaggtcagctatcgtggctggttaggctttatgtgtgttgcatcatttgccaccgccaactttggccttgatacgattatccagtggtcgacaccaatgctgatgttcttgtacccattcgcaatggttttgatcttgctgtccgtcttctcaccgttgttcaaccgtgatccactggtttatgcgctggtcgttggcttcaccacggtcccagccttgctggacatggttgccgctttccccccagttgtcagccaaagtgcctttggccaagccttgggtgctttccagcagcacgtattgccatttgccaatttggggatggactgggtcgttccggctgctgccggtgccgtcttgggacttggcctgcattttctccggccggttctgggcagagccaaagcaccttcatctgaagaaaataatgattaatacagtcgataatgttttagccgataaaaaaatcgttgaaccagcaaccagtaatagccagttcaacgatttttgtgatttaacagctgattattgtaaattagtaaatgcgccattttcctgaagtaatttcacaaatccaggaacagtatcttgacggttccaatcacgctgcagttcgcagactaattgcgggatcgtaatcaggtgagcgccggcttgttcaactcggcgcagggcagtttcgtgcgcgatcgttgacgtgccgccgactgcgtcgacaactgggtagacatcaaagccttcagcgatggcatcgatggttggaaacgtcagacaagcttcggtccataaggctaaaataataatctttttccggccggttgccttgattgcatcattgtaatccttgtcttcccaagcattgatggaagaacggtcgtaggaagggatgtcgcccactaaatctttcaatggtttaacggtatctgaattgcgttgattatgggcatttacggtcgaaagcacaattggcagtttaaatagtttggctgcttccacaaccatttctgcgtttttcagtaagtccgcatggcgcattgaaccaattgaaccaatttgcactggttggtaatcaatgattgttaaaacggcattgtcaggtgatagcaagcggtcgtctgcgcctcgtttgtcaaaacttgtcatagtatcttcctcctcaaaattaaatccataagtcctctagaattcgctttcatgatacaacgatcagggagtcgatactactaattacaccttgaccccaaagccttgggaaaggattcaattgttgaaaaatttacattgaagactaacatggaaattggaagaaaaacgtagtaaataatttcaaagcggcgacaaatgaaatggttaaaaaagtctttttagcaatggtgacaatcttagtttcagttctaatgcttgggtcggtcaattctcaggccagttccaaagtgaataactacatagcaagtcacaatatttcgcacaatcaggtctccagtaagatttggggcggctttccacactataaataccgccatggtaaaaataagcctgagggcgtggtcgttcatgaaaccgggaactcccactccacgatttttggcgaaattgcgtatatgaagaagaattaccgaaacgcctttgtccacacttttgtcgatgacgaccacattattaacattgccagcaccaagtatctctgttggggcgtcggctatcccggcaatgcccgctttgttcaatttgaacaggtcgaaatgcacagtaagaaatcatttgccggtgaggtggaaaacgctgcttactatacggcctatattttgcacaaatatcaccttaagcccaatgacgcggtatacgacggccacggcaccgtctggtctcatggtgcggttgcccattatcttggcgggtctgaccatactgatccgaagggttattatgccaatcgcggcaaaaaatacttccaccaatcttataccatggcacaattttatcagctggtgttgaccaactatcacaacctttaatttggtgaaatatcaaaaaaacctttacaggtggaatcttttagattattatcaaaagagtaatcgttactatttgcaagggagaggatatctcatgttacataaattttcgggcttcaaggcctggctgttagtcgtagtagcagttgctttaggcattggcctaaccggttgtgcaagcaactcagccagcaatggcaaaatcaagattaccgctacgactgatttctatggcgaggtcgcaaaggcagttgtcggcagtaagggggacgtgacttccatcattaccaaccccaacgtggatcctcacgattatcaggcatcgacaaaggtggccaaggaaacggttggctcaaagattgttattgccaacgggattgggtacgatggctggatgaataatttggttaaggacagtagcaaggttgactatatcaaagtcggtgaagacttgatgggtaagcagaacggcgacaatccacatttgtggtataatccggcaaccatgcctaagttagccaacacgattgcgacaaagcttggtaaactgcagcccaagaacaaggcctactttaagaagaatgctcagaagtacatcgcttcattgaagccggtcaatgataaaattgcccagttgaagcaactcgccgcaacaaagaagaacaaagaagtctacgtcagtgagccggtatttgactacgcccttgaagcaaccggctttaaggttggcgacacccagttcgaaaatgacactgaaaaaggcgtcgatccatcaccgcagacaattcgcacgatgcaaaacggcatcaagaaccacaagatcgccttcttcgttttcaacaaacaggttgacagcaagactgtcaataatctggtggccttagctaagcagaacaaggtgccggtattaccggtcactgaaacattgccagctaataagacttacgtcagttggatggattcacaatatacccagttaattaatattttgaaatagttcgtatcaaaaaagccgagaagtcagaattgatttctcggcttttttgtatttaattttaaatttttcgatcggcgattaattcaaataaccgcgccaaatccagccaccgtgattgccgacggtactgcgaacgtgatagtaaattgcatagttgccggtgttcttcttgtacaacttttcatgcgcatcggttacccaagtcacgttggggagttctgaattgtagccataccgggtgccaaggtgcttggagtatctggcacccttagtggttgtgtagtagtgcttgcccatattggcgcgccaaactaatttgacggatgccgaacgagctgccgaatactgcttaccggatgggccaggaatcttgacgatttccccatcatttttagaactggaaccagagttgcttggttttgtcgcactgctggaactggatgcactggaagcactcgaggcactacttgagttcgcgttggtgttggttgaagcagccgctgaaccggagttcaagtagaagctgttgtttaattggctaacatccaaattctggttgatatttgggaaccggtagtcggaagcccattgccaggcattggctgaagggtacttcgacccggttggtgttgccggatagtcggcaatccagccctggttggaggcgttggtgtcaacctttacgcccaaccaacttgccatggtatataaatcggtcttgttatagccgccctgattcaaagctgaatcaaaagctgccaaattggcatcgttattcgctttggaaattccacctaattctgaagattcaaagtcagctaccatcacgacatctttcgaactggtaactgattgaacggcattcatgaagttttgggcttcctgagcggcttgatcagtcgtcgtaaagtgaacaaaatgatagaaattaatacttaaccctgcctgctgggcatactggacctgttgagaaagatacggattgatatatccggttccctcagatgctttaattgtgaccgctttaaccccattttgagctaatgtttgataatcggcggcagttaaatttccctgccaactggaaacatcaaccatgttagcgccaggttgggtactggacggcgtcaaagccgcgtgggcagtggcgttcgtcccaaataaaattcccccggcgaagagccctaagataacggctcctcttttgaaacttttcctcataatcactcaactcccatctatgtatatacacatcactgtgatactaacatgaatgagggcctttcggaagaatgtttacttattgtttccacttcgtcgatcaagtgaaaagctccagtaaattgcgagtaacaaaacggctgcgattgaaatagttgtaatattattggccatcgcatgggtgctgacctgccaggcaacgtaaattaacgcgagttggaaaacccacgataggatggactggccggcaaattttttggtaaaaaatttcatgagataattcctcctattattctggaatgtcaccattctcagggatgtaatcaattgaatcggcaattcgcttgggaattggaatctgtggatcaacgtggggattgttaagatgaatcaggttgtaggacttgcgatactctgtcggcgataagccggttgcgctcttgaaacgccgcatgaagacctttggatcgttgaagtaagagttgtcggcgatttgtttaatcgacatatcggttcgaatgagcagtagagtcgccacttcgattttgacgtgattcaagtactgcagggttgtcataccggtgcagtgcttgaacagcctggttaaataatctggattgaggtgactgcggtcggcaatctctgcgacggttaaatcactggacatgttagcccgaatccattctttgagactgttaatccgcgagctgtcttcattggcatcgggacgattgaagtatgacttgtacagctgaattaaaagtgcagaaaccagatagtcccgttcttcaatgaatgatagttcattgtggattgatagaatctgatgaatcagaatagttgcctcttcataatcggctaatttgaaatactgcggtagaaaaatttgccgcttcttgctggtactggctttaactttttcagtcatgtcgtcttcatcggcagtgagcgtatcttctttgtgctgggagaaaaagtgaacccagtagaagtcgacgtcacctggggaatcttgataaccataaaaagtggtaaacggcgggacaatcaagacttcgtgggtgttgagggtataccgccgatcgccaatctgtagataaatcggtcccttaatacagaggattaattcataatcacccttatgatacatgcgtcgatggtgccagcctttatgagctaaaaattcaccacctttataatagagcagcgttttttccattgtgaacgttgagaataacatttcaagccaacctcctaacggtgtcggaaatcgtcaccaaatgtacgcaaaaatagttttacggcaatgtcggaaacggtcaccaaatgtacaaaacagtgtcactattggcctcgtgacgctatcacggaacccaatattttctcaactggtcggatatcatcacttcttttgccattatagacctttttttattatttggaaacgcttactataagacttgtaaaaacaagttatgttttgaacattgatttttcagaaaggaagttgaggccaatggttcaaattgacgatcgactaagaagctcaccagtttcttaattgggttagtttcagtgtttcagcaatcatttttatccgcccaacaatgagcgggttaccaaaattaatttatttggaggaattatcatgagctcaaatgcaaacgtagattcaaatacggcaagtgctcaagcattgcttaacgacacgttaccttggcacagaaagattacctatggttttactgatatgtctggtaacttactgtactgtattatcagttcttacatgctttacttcttcaccaacgtcttcggtctctctgttggaacggccggtgttttacttctgatcggccgtgtctttgatgccattggtgctcctgtcatgggtatcttggttgaccacacccacagtaaatatggtaagagtcgtccttggttcttgtggatgtcattgccatttgccatctttgtctggttactgtttaccaccccggcattgagcggcactttaaaagttgtttacgccggtgttatgtacatcttagccgacttatcatacaccgcaatgtcgacaccaatcacttcggttttgcctaacttaacttcaagtaccgacggccggatgcaagccaactcaattcgtttggttcttggtaacgttggtaacttcttcgctgttactttcatcattccattcgctggtttactcggcggtgggaacgagcaaaaaggttggtcattagctgttggtgtttactcaatcgttgccttccttctcttaatcatcgccttcttcgatatgcgtgaaaagaatatcgaaaacgaaaaagtgattaccattaaagaaagtttgaaagccactaaaggcaactggccttgggtcttgattgttgttgccaacttggcttactggactgcatttatcgttcgtaacgcttcaatgccttactacttccagtacaacatgggcagcaagggtctgatttcattcttcaacggtttcacaattatccaagttatcggaatggcttcagttccattcttcgttaaatttatgcacaagtggggcaccacaatcttcttcctgttgatgaccatggttggtcaagcatgggttggtttagctggatcaaacgtcacttccgctctgatcggctggtgtgtcgcatgtatcggttcaggtagtgcctgcacaatgttcttcgccatggtcggtgataccgttgactttggtgaatggaagactggtatccgtgctaacggattcttaactgccatcggtgcttcattctgtatccaaatgggttcaggatttggttcattcattgcttcaatgcttctcaaaggtttcggtttcaacgctgccaatgcaactcaatcaagctcaagtcttggtggaatcagctttaccttcgtctgggttccaattatcatttacgcaatcagtgttatcttgatgattatgtatcgtaaatgggaaaaccacgaaccagttgttaaggctgaccttgcaaagcggaacgccgaagctgaaaagaacgctgaagctgcacaagcttaattgtgagattgattttaaactttaggaggaacgcatagtatgcaagtttataccacaccaaaattaaataaggtcaaggttacttcggatttctggaaacgctaccgtgaactcgtcgttaaagaagtcttaccatatcaatggaaggttatgaacgacgaagccgacatttccatttctgaagatccccaaaacaatggccaagacaagaacagtcatgcgattgccaacttgaagatcgctgccggtcaaatgaaaggccaccactatggttttccattccaagacaccgatgtctacaagtggttggaagcggccgcatactcattcgggtatcatccaaatccagacctcaagaagattaccgataatctgattgatttgatcgctgacgcccaagatgacgacggctatctgtcaacctacttccaaatcgacgccccagaacgtaaattcaagcgactccaacagtcacacgaactttacacaatgggtcactacatcgaagcaggagttgcctatcatcatgagactggcaacgaaaaagctttggacattgctaaacggatggctgactgcatcgaccgcaactttggccttgaagaaggcaagattcccggctacgatggtcaccctgaaatcgaattagcgctgtcacgtttatatgaagaaaccggtgagaaacgttaccttgacttggcccactatttcttgaaccaacggggacaagatccggcattctttgaaaagcagattcaagctgatggcgacagtcctgaccgtgacctcatcccagggatgcgtgatttcacgcgtgagtactatttggccgcagaaccgatcaaggatcaaaaagttcctcatggccacgctgttcgagttgtctacctgtgcaccggaatggcttacgttgcccgttacactggcgacaaagatttgttagctgcctgtgatcgcttctggaacgacattgttaaacgccagatgtatatcactggtaatattggtcaaaccacgactggtgaagcctttacctacgactatgacctgcccaatgatactgattacggcgagacttgtgcttcagttgggatgtccttctttgcccgtcaaatgctgaacatccacgccaaaggtgaatacgccgacgtgctggaaaaggaattgttcaacggtgcattaagcggcatggcacttgatggcaagcacttcttctatgtcaacccattggaagcagatccagttgcttcaaagggtaatcctgggaagtcccatgttttgactcaccgggctgattggttcggttgcgcctgctgtcctgccaatcttgcacgtttgatcgcctcagttgatgagtatctctacactgtgaatggtgatacgatcttgtcacatcagtttatctctaacgatgctgaatttgatgacggtctgaagatttcgcaaacgaaccacttcccatggagcggcgacattcattatgaaatcgccaaccccgacgccaaatcattcaagctgggcattcggattcctagctggtccgctaacttcgacttgactgttgacggtaagtcaaccaccttgcctgttgaagatggcttcatctacatcgatgttgatgccaagtcgttaaccattgatttgaagctcgatatggacgtcaagatcatgcgcgccagcaacagagtcagtgatgactttggcaaggttgccgttcaacgtggaccaatcgtttacgcagctgaagaagccgacaaccaagcaccactggcttcatatgaagttgcaacagacgctaagaccgactaccacttcgatgagaaattgttagatggtgtcggagttgtcaaggttgctgctcaacgacaaaagttggattccaaggatgcacctttgtatgttgacgccagtcagccggttgagtcagaatcagttgacctgaagatggtgccatactacgcatgggctaaccgtgagaatggtcaaatgcgagtttggttaaataaataaatcatttaaagttagcgttttcaacctctttcataattggttaaaatgctgtatagtatgacgagatcctgatgttatttctgacatgacatcacaacgaaccccattcgtataaggatcgagcccctccaagcaatcctgcttggaggggctttttgtgtattggcaggtaaaacagctggcattttggggttgaataatgaccttttttggctggaatccggggcattttcaaaagattttcattcttaacgcttacatcatgaaaatgtttcaaaaatctatatactgaattttcataatggcctataataaattcgaaagcagcaaggttggcttgctgccgggggttcgagtgcttaggaggctattaaaacatgaacaaaaagtctggaatgatgtcgttttcgattctgatgctgtcattattaccaatgtcaacgggggcgacggcttccacaattcccggattaatgaaacaatttccagcggtttcatcggaaacggccgagctgactgtcaccatcccatcattcacgatggccgtggtgattatcctcagcagcttgattgtcaaacgaattggcaccaaaaaattagttctggcaggaactgcattaaccgcatttggagcaggcctttcaatgttttcaccaagcgtttcagtcttgttgattgccagagcgattatgggagctggaattggagcttttaacaccctttgtatcagtttgattgatcgcctgtacagcggtcagcagcgtgaacggatgctgggttttcagaacacttttcaaggtttgggggctgccggcggtgcactgggagttggtctgatattgatgtactgatgtacagtaactggcggatggcgtttggaatttatttgatcagcgtcgtcttgtttatcctgtatcttttctacgtacctgaagttcgttatgataacgatgatccccaaactgtcggtcaagctgacgagaaagtctcttggatgtccaagttgcagtttggttattattggatcgtcatgttcatcctgatggtattctacatgaccgttaatgtgaaaatgccaacctacattttaaacaatcatttcggcgccttatctgttggctccacggcggttgttgtgatgtcgatcggcacgattattggcggcctgatttatggctttattgaatcgattgccaaaaacgccactttggtcatggcgattgccattgaagccgtgggtgtcttcatgatcagtacggccggctcagcgttggactgcttcatcggtgcttttgccgttggttttagctttggcctgtttattccattcatcttttccaaaggattgtcgtttgttcccaaaaaatatggcaatgacgcgacgactattttgatgatcagtaccaatggtgccaacttcctctgcccatatgtcagcaagttcatcaacatcggcggtactgaccgcagtttgtttatgatggcgggcgtgattgcctcaattctgggaatcatcgagttggtcaaattattagccaatcggccgcgaagaactgttcccgaagcttaatgtttttgtgaattttactaatctaaatgtatttctgaacctctgtatgatattattcatacagaggttctttctatattatgagccatgctgagtgttacacttgagatggctttaatacaaggatcgagtgttaaaaaatcaattcggaatatgagtgtaatgggtgataagatgacaacaattaaagatgtcgctaacgaagcgggtgtttcgatatcgacagtttcacgaattttgaacttcgacgatacgctttctgtgggggaagacacgcgtagaagagtgttggaagttgctgaaaagctgcagtacaagaagcggaatcggcatgtacccaaaggcggtaaaaagattggtattattcaatggcattctgataaagaagagctgactgatctttactacctgcaaattcaatacggcattgagaataaggcggccagcttaggtgccggtgttgagaagctgacgtttgattcaattgataagagtcgggtgaagggcctcagcgggatgattgccgttggtaagtttgataagaccgaagtcatgagtttgaaatcatacgatatcccactggtctttatcggtgagaactatttagcttacgattgtgacagtatccgtagtgatttcgagtcaccggtccgtaagatcattgaccggtttattgagcacggtatcaaggatatcgggatgattgccggtaaggaaacgaccgtgactgaaaagcagggcgttcgcgatcctcgagtgtcgacatttgattcgtatttgtcagaaaagggtttgttcaatgatgccttcgttttccaaggaccatttggcccggattcagggtttgagctgatgaacactgcaatcaaacagttgggcgacaagctgccccatggattcttgattggcagtgattcaatggccgttggtgtcttgcgagccctccagcagcagaatatcagcgtcccagatcgggtcagcttaatcagctttaacgatgttgcaattgccaagtataccagcccggcattgacgacggtccatgttcacaccgaattgatgggtgagcgggcaattgaaatgctgacggaccggattaaagaaccaaagaaggtcccagagctgacggtgattgcgacggaattgatggagagggagagcagtttatagaagagagtggagcaagaggcgcattgatcccagaatgtaagaccgttaagcgattattcccggttttggaatgattgcttaacggccttacatggccgggatcagccgattgttgcacgtttcggcaaggtaaaagtggtgctgatgcaagagtggagcaagaggcgttttgatcccagaatgtaaggtaattaagtgattattcccggttttggaatgattgcttaacggtcttacatggccgggatcagccgattgctacacgttttagcaaaataacagtggagcacaaacaggtagggtcaaaagcgaataacttttgcccagcctgttttttagtaaatttaaagattaatatctatgataacgtagaatccaagtcatcaaaggaaaaagcaagcctcattctctaggatgattttctcaatagcgacggggattctcgtccccctcagaatagttttactaaaatctattgactatacccgataatatagtaaaattaaagcaacagcacaaaagaaagcgcttgcgaaagtgataaacaattaccacttttaaaccctaggaggatgaaacgatggaaaaaggtttactttatccagttaccaatcaatttagacaagatcaaaagttagacggcttatgggattttaagtttgacccacaagctcaaggtgaggccaagggatggacaaccggttttgatgatccaattaagatgccggtcccagccagctttaatgatttctttaccgacaaagattcccgtgagtataccggggatttctggtacgccaagaagttcttcgtaccaacctatatggacggccagaccattcagttgcggtttggagcagcaacccaccgagcaactgtttatgtaaatggccaagaaattcgctcacacgaaggtggctttctgcctttcactgcagatattaccgatgcagtgaaattaggtcaagaaaatattgtgactttgaagatgaacaatgaacttcatcgagatgcattgccagccggtgatacagccactttgaagaacggcaagaagatggctaagcctttctttgatttctataactattcgggcttaaaccggagtgttcatttattagccgttccgaagaaccatatttatgattactcaacaacctatgatgtcagtgaggatcaggcaaccgttcattatagtgtccaagcaactgacggcagcaatttcaaagtcagcctgagcgatggggatggcaaggtggtcgcaaccgctgaaggacagactggtgatttggtggttaagaatccgacattatggcaggttcgcgacgcctatttgtacaccatcaaatttgagttattggatgctggcaaggctgttgatgaatacagtgatgaaattggtttgcgaaccatcgaaatcaagggtcacgaaatcttagtcaaccacaaatctgtctacttgcgcggctttggtcgtcacgaagacagcatttacgccggtcgggcatttgatttgaatgttgaacgacgtgatatgaatctgatgaaatggattggagccaactcatttagaagttcgcactatccatacgatgaacaagtctataaattcgccgatcgtgaagggattttgattaccgatgaagtgcctgctgttgggttcaagatggctgcagccagtttcctcggcggtttaaaccaatcattctttgacggtgactggattgatgaattgtacaagaagcatattgatcaggtcaaggacatgatcaagcgtgataagaaccatccaagtgtcctggcatggagcttatgcaacgaaccggatacttcaactgactcggcggtgccatactttaccaagttgtttaatgattcaaaggatttggatcctgaacaacgaccaagaacctttacccttaacgaggacgacacctttgaaaaatccaagtgtttgaaattccctgacttctacctcctgaaccgttatccaggctggtaccacaagtggggatacgaaatctcagatggtgaagctggtttgcgggctgaattggatgaatggaagaattctgacatcgataagccgattgtcttctcagaatatggtgccgatactgaaccaggactgcacaagttgccatcgattatgtggagcgaggagtatcaaatcgaattgctggatatgttcgatcgggtatttgactcctacgactttatccggggtgaacaaccttggaacctggccgacttccagaccgtggaaggcaacatgcgggttaacggtaacaagaaggggatctttacccgggatcgtcaaccaaaagccgcagccttttatttgaagaagcgttggacttcattaccactggattataaagcaggtaaatagcattgcaggagaggtcggaacaatacttaacgagtactggtgttccggcctcgttgtttaaaagcaaatagggtgactgaaaaggagtgttaacatgaaccagacaagttttgtcattgacggggagcaactggatctaaatgccaaagatgccaatacatttaaaggctttggctacttgagctgtaacaattcttcccgactgctgctggattataaatgggaacatcgagacagttatgatcagattttgcagattctctttggtggtaagcatccattaatgcggatgttgaaagttgaaatgggcgatgatgccaacacgtcttctggaactgaaccggcaacgatgcgctcggcttcggaaaccgcaaacgttaaccgtggggctggtttccagttgatcgccgatgccaagaaaatccaaccaaccttgaaaacagccattttgcgctggggtgagcctggttggctgagaaaagattggttcgacgccaagtcggctgatccggatggtgatgtcccggaaactgcctatgagccgatgtatcggtggtataagcagacaatcatttcggcctatcagacatatggttacctgatcgattatattgatcccgaccggaacgaaaccaagcatccgatggtcaaatggatcaagtggtttgcggatcgattggcaaacgatcagtccgggtttccgaatgactttccgattagtcggtatcagcaaatcaaaattattgctgccgatcagaactatgaacgtgattttggcgatatgatgattgctgatgcggacttgcgtgaacgagtcgaagcacttggctttcactacaacactgatgatggcgaaaaacagccgtttacaaagttagcagacgattaccatcatgaagtttggtacagtgaaggaattgcgccgatgacgatgggtaagtaccgagttcgcgccagcaatggtgacggaatcggcggacgtcaaagcggcttggatgttgctaaccgactgattaagagctacgtgaaatctcgtcgaagtttgtatattttccaaccggcagtttccgcttattataccggggtcaattacagtcacaaagagctgatcaatgcctgccgaccgtggtcaggttactacgaagtcgataatgtcgggctgcagtgcatgaagcactttactgattttgccaaagcaggttgggaagacgaaggtgcttggcgatatttaaccagtgcttgtgacagtcaagtcggtggaaccgaaaacctggatcataatcggcaggcccccagctacatgaccttgatggcgccagacaaagccaactactctgttatttttgataatgatagtcctgaagcgcgcacctaccagattcagctgaaaaatcttccggcttgtgaagacaaaccggttgccgtttggcaaagcgttggtcccgagcatactggagatgcatatgacagtcggatgaaacagttacgccaaaccgtttcgccaacggacggtttgctcaaaattattgttgcaccccattcgattgcaaccgccaccacattggatttggctgacgatccggaagtggtctatcatcgcttggaaagcccccatgaagaccacacccttggtatcaaatctgacgatggcgttttgtatgaagacgattttagttactcgggctacccagaaaattatttatcttctcgagggaatacgccgcggttcactgctgatcaaggcggcgcctttgaagtggtccggaccgacgaagacaacgtcatgcagcagatgatcaccgagaagcagcgggcccttgactgggaatattcatttgctcccaacttaacatttggcgacgatcattggacggattacgaggttgccgtgtcaatgaaatttgacgatcaaactcaacaaaattcgccaaccggaaactactttgggatcggtttgcgggaaatgaccgacgtcaagggtcgccttgaaagtgccccgtatgtctttaaagtagccattgatggtggatgtgagttggttaaggatgaccgaattgttgctttggaacacgttgacggcttggatgtttcggcaactcatcaagtcacgtttgcagcggaaggtaatcatttaacggcgacatttgatgggcagctggttttcgattataccgataccgacaatccacattacagtggccgcgtcaaaattgggagcgggtattatcatacccagattaagcaactaacagttacccagggcaaacagccacatttgattgaacacagggtggatgatcttgattcagctgttcaatatacaggcaaatgggatcatgtttgcggtttgggcaacaccaaatggaatcgaacactgtcgacagcaagtgccgaccaagataatgtgccaggctttaaatttgacttcaacggatccggattctcactcattggggtccaagacgttgccagtcatctgaaggtgacggtggatggagccgttcgcaattggaatctggcaccacaagttggtgctgatcggacagagaatatcgttgttcatgggttgtctgccggtaaacatcatgtctccatcgaagttgttggtggtcgttacacactagatgcggtggatttcttaaaataatccagaaaaaagcgaactgaaatttcagttcgctttttgtatcccttaatattgacgaattttaggtggcgtgtaggtggtcatgaacgtataaatttcatccagtgaatcggagaacagcaccttcttgcggtcagctgccgataagaaaccttcgctggtcatcttatcaaacattttggccaacaggtcatagtaaccattcacgttataaaacacgcaggggttgggattatcccccagccgagcccacgagaaggcctgggtgatttcttcaagcgttccgatgcccccaggaagggcgatacagccattggagatgttcatcatctcagctttgcgggcagacatgttgtcggtgaccgtcaaatctgataattctcttaaacgcggtgactcagctcctcgagcaaccaactgcttggtggtgacaccgtgaactttcccgccttcagccaatacttgatcggacaacacgcccatcaacccgacgccaccgccgccgtaaatcaattcaagatcgtggctgaccaaccaagatgccagttttttagcggcggtgacgtatacgggattcgtgccggttgcggccccgcagtacacagctatccttttcatatccagtctcctttgaaaatagtctagtcttattctaccagtttttctgaaaacaatttttgaaaatcgacataggggactataattaaattaccatttcacgaaataatttaaggaggttaccatggaaacctatattttagatgattcagacgacatgtggcagcattttgccaaactgattggcgacgtctcatggcctgcaggtaaatatttagccaatgaaatgctcggcggacgggtgtctgattgggaacgggttatcgttctaatggatgacgaccagttggtgggcttttgtgcggtcgttcgggaagatatcgttaaaggaaccggctattcaccattcattggctttgtctttgtcagcgaggattatcgcggcagacacctcagccaacagttagtcaaattggccgagaaccaaatcaaacaaattgggtttcataaggcatacattgtcaccaaacacgttggactgtacgaaaaattggggtacgaacaaatcgatacttccgtcgaccaattgggaagaaagatgaggattctagcaaagcaattataatttgattgaggagagaaagaactaatgagagaagagaccacagtaccaaaccgccagaaagtcattttgggtgctcttctgatatttttagtgggtgcaaatatgcggacggcgattacgattgtgccaccaattttgaccaatattcaaaattcgtttaagatgccggaatggtttctggggagcttaaccacaattcctttgatctgctttggattattatcaccgacggttacatattttattaagcgcttcgggattctgccggtaacgatggtggatctgggcttgctgacaatcggcaacttcatccgggtttattcctttaccagcttactgtttgggacaatcttgattggttgtgggattgcgatgttgaatgtcctcgcaccaaccctggtttcctatttgtttccgatgcagattgggacttataccgggatgtatgttttcgcactgtcactatcgagttcgatttctgccggctttagcgccgtggtcagtcacttgattacttggcaggtgatgattcaattcatttcgattattccagtgatcacaattatcgtggcgatcatgttgagaacttcaggcaaacgcaagacatcggccaaaaagccatcaacaccacttaatccagaagtcaaagtgagcgtttggaaacggccgcttgcctgggcattgggtggcttcatgggtttgcagtcacttcttttttactcaattctaacctggctgccaccaatcctgatggcatcagggattaatcagaatacggcgggatacttgttggggctgctccagttggttgcactgccgatttcctttgtcgttccaagaattatcagctcggttgccaaacagtcaacgatgattgggacgatttctggtttgtttatcgtcgggttgggatcattgatgatggctgaaaccagtttctggtttgcggtccttgcctgtgtccttctgggattgtcaaccaatatggcgttcagcgaggcaatgaccttgttctcgctgaagacaagaaccccgaacgaaacagcctcagtctctggaatgggtcaatcatttggttacctattggcagcgacgggtccaatgatttgcggctggatgcatggcctgactacaaactggtttgcggttttgattttcctactggctgtgaccgttgtcatgacttttgtgggattgttggttgaccgtgaggagtatgtgttttaaaaatcagtgtgggcaaataagcgcctagcttccagagtgtaagggggagtcgtcaaatatccagactctggatgtttgacgactcccccttacacggccggaagctgcttatttgcccacgattccactaggtaatagttggagaccagggcttggatgtttggtgaacgcctttatacggccagaagctgcttatcgtcccactattccactaggcaatagtagggaccagaccttggatgtttgacgactcccccttatacggccggaagctgcttatttgcccactattccactaggtaatagtaaaaaagcacaaagtaaacaccaaaataacattccacaatcaccatcattaaaaataaattaaaaaatgagttgactctcagaaataatctgttacgataatcactaatatatttaacgaagatcgaatgagtaatcagtggagttagcccagagagctgtcgcgtcggtgaaagatagcctaacgagattgatgaatatggttcgtgagttgcagtagccgagcacttgtaaggctacgatgttgggcacattatcgtctacagtttgaaaactgactgagaaagcatgcgtgagtgtgctttgaaatagggtggtaccgcgatacgttcgcccctatggcagctttaacaattgaccggtttgttaacgcaaaccggttttatttttcgaaattttgaggaggcggatgctgatgaagaagatagtcgtttcagtagtgggattggtgagtgttttggtgttaagtgcctgtggcaagtcgacgtccagtaaggatgcgaccagccggacctttcgaacgacagcccagacaaatgtcatcacggtcgatcctaatcgggcaactgatgttgggagttatttggcaatttcgcaagttgtcgagggcttgtataaacaaaataatcaaggaaagattgttccgtcggtggcaaccaaaattgttcagccaactaatggcgggaaaacctacaccttcaacttgcggcatgatgccaaatggaacgatggcagtcgggtcactgccggcgactttgtggcctcgttcagacgacaagttgaccccaagaccaagtctcaacgtgccggtcatttgagcgacattcagaattatgaagcggttaattccggcaaagcggcgccatctaaattaggcgtcaaggccattagtaagtataaactgcagctcaagttgagccacccggttccgtactacaactacgtgatcgccacccaactttatccgattaatcagcgggcgctcgccaaatggggcagtaaatacggtcaggattcaaagcacgcggcttccgacggtgcttatgaaatcaagaactggaattcttccaaagatacctggaacttggtcaagaacaaagactactacgatgcgaacaaagtcgacttaaccagaattcatttccaggttgtgaaaacaccacaaaccagcatgcggttgttccaggcaaaggatattgatgaaactcagatttccggcagtttggttgctgatgccaagaaacaatttaagaatgaaacggtggtttcaaaatatggtcagttagcctttatcccttggaacaattaccgtaagacgacgcggaatctcaatttgcggcgggcactaagctacgctattaatcgacaatccttggcaaagaacgtcttaaaggacggatcactgccggcccaatcagtggttccggagggtgaagttaaagatgccagtggcaaagatttcaatgccggcgttaccccaaagttgacgtataatctcactaaagcccgccactattttaaattggctcaagaagagttgggaaaagaaaccatcaatgttcaattgttaaccgcggacaccgatgcctataaagccgtcgcagaatatattcaatcacaggccaaaaaagtatcgcccaactttaatttgacggtgcgctcaattccactgcagcaagagatttccgatttcagtaatcacaagtttgacgccggcacgctcgggtggtcgacagacttcccagatccaattgattatctgaacttggctgccaaagccggggtaatcaactttaccaagtggaccaacgataagtatcaaaaactgattgatcagattaatgacacgacgcaccaaactgcagcacaacgagtaaaactgcagcagcaggctgcctcgttgttaaacgaacttcagggcgtcacaccgctgtaccagtatgcttcggttcatttgagaaccaagaatatcaaaggcttggattatccattaattggttatcagaagtatgagtatgcaagctggaagaagtagtagaggagatctgattttatgacgattaaaattggcattgccagtaatcatttgattcatccaactgaacgattcggaacaaattttgtcgattatattcaacgagactatgtcactgggctgagacatgccggcacgttgccattggtcctgcccttgggtgatccgaaagatgctgaagattatattgccggagtcgacgggttgctgttgtcaggcggccaaggggtgacgccgattctgtacggcgaagagccgctggctgaagttgctgaaacggatatttaccgggatcaatttgaaattgcattgattaaagctgctcagaaagctgacaaaccggtgctggggatctgccgtggcatgcaggtgattaacgtcgcgttaggcggcaatctgtaccaggacatctataaacaagccggggcaacggagaaacacaatcagtatccaacgtcttgggagattcccactcaccacgtgacaaccactgacgactcgtggcttcaccaaatcttgggtgagcggtttgcggttaattcctttcaccatcaaggcattcatgaaccgggtgacaatttgaaagtcgttgccaaaagtgatgatcaggttgttgaagggatcgaatcaaacgatggtcgaattatcggtgttgaatttcacccggagatgatgcgggtagtgcatccggaattccagcggatttttgattattttgctaaattggcaacagagaatcagtagagatagcaaaggctgaagcccagtgattgtactggtgcttcagcctttttttcgcctacttaacaatgatagagttgatgatgttacggcaactttgagccccacttctatctagaccaaacgtgcagcaatcggctgatcccggccatttaagccaacaaaccaatcattccaagtcccggaataattggtttgttggcttaaattctgggatcaaatcgccttttgctccactctactcttaaatttccgccgccggattggtcgtatacgttgcccatgcctgaacagcgaccgtgcccaggattaggacggcgccgatggtttccggcacgccaaagctgacgccaagaaaaatgatcgaaagtgtggtagccgatagcggttcgaatgaccccaatacactggcagtcgtcggttgaatgtatcgcaggctttgaaggtaaaataggtatgcaaacatcgtgccgaagatcaccacaaaggagacgctgccgtacgttgtccaagaaaaggccggcatgtcgtcccagatccggtaataaaggctaaaagcggttcccccgattagcattgaccaaccaacgatgggaatcgagccgtattctttcaggaggtttcgcggtaataaggtatagagggtagaactaaccgctgcccccacaccccacacaaagccgcctaaaggcattgccaaggtggttagctgtccgtgggttaccagaagaactgtcccacacagcgccataatgaccgagaagacgtcgattcgccgcggaaaacgccgggtccagagagccaaataaataataatcattgctggtgccaaaaattgaaggatggtggcagtggcggcattaccggcctcaatcgccatgaaatatgtatattgtgaagcagccattccaataaagctaaagaagattaagcttagtgaatcccttttgtggtgccaaacccgcatttcttgtcgatgattgccaatcaaaccatacaggaccaatagaatacctgaaatcagcattcggacagaaaccaaccagtgtgagcttacatggatatcgtcaaataaaaattgggcaagtgttcccgagattccccacagtaaaggtcccaacattgccagtacaatgccgcggatacttccatttttcacctgattcacctcccatacataatgaaccaattatattacaaagataaccgatttagaataaccctttgtaaaataaagtgaattgcgttagagtatcattaatatttaatgatagaacaatacataagaggaggcctgcgcatgtttgataaaattggccagattattttcaacaacgaaattgtcgcaaatgccagcgactttaatatgggcattgaagtcgaaacgattcggattgattcggctggaagattgacgaaggaaccgtaccccaaagcgcttggcaatcaacgaaagaaccatttcatcaaaacagacgtttaccagattcaaagtgagattatcacgccgactgcccgcaagtccctggatgcgatgcattatttgatggcacttaatgatacgctgcgaaatgctttggagcctaacgaattattatggccgttgagcatgccgcccgtgttgccccaagataagagcaccattccaatcgctgatgttgaccccgaacagaaggcctattacgaaaaatggatcaaaacccgtagcgatacccaggggattcctgtcggggtccatttgaacgtcagcattaatgacgacgtgctcaaaacggtttggcaggcagttgacgatcagtatgattcatacgccgattttgtaaattatatttatatcaagatcgcccaaggctttgattactaccggtggttaatcacttatttgtttggcaatagtccaattgctgaaaagaatttctttaaaccggacgaggatcagccgcagcatgaagtgcgtagtattcgttcatcgaactatggattgacgtctgatgtgacccacaattatcgcagtgtgccggattacgtcaagaatatcgagtcaaatattgccagcggcgccttgttcagtgaagcggaataccattcaagcgttcgtctgaaaaccatgcatggcgacctaactgatatgattaagaacgggaccgaatacattgagttacgaatgctggatcttgacccgacgaccgccttgggtgtgcggacatccgccatccgctttttcagaatcctgctaagttatttcatgatgatgccgactcttgaaagcgatgagaagatcaacctcaagttggaacaggggcgggcaatgaacgaagtggttgcccttgaaagcccatcccaacagacaatttatcatcatgaggcgcaaactttcttggatcaactccaattgtttggcgcccagattcagtggggccctgaataccaggaagtcttggatacgatgcaggatcgactcgacaacccgaacctgaccccggctgcaacgctgtgcgatcatgaggttgacggctcactgatgtcatacggtctggcaatggccaaccgttatcaaaatcgcgcccatgagaatcctaatccatttaccggctttgaggaacagcccgatatgacggccaacgaactcaggcagcgtctgtttggtgtcatggggaaaccggaaaattataagaacggctgattcgttgacatgcggctgacgaatcactaaaatacttgataattaattgaagcctctaccaggtttagacgaagcgaagctgtgatgtcctacaagttttttcttgtaggatatttttgaaaataaaggatggtgggcaaatgaaacaagcaaaagaagtttctgatttcattaattcgacggttgggttggaggtggaaacccaccggataaataaaagcggtcagttgagtcacaagtcatatcctaaaggcctgctaaacgagcgtcagcaccattttatcaagaatgactttttggaaacgcagtctgaattgattaccccgccaaccaaaaccaccttgaaggggttgaaatacctgggcgtgtatcatcaggcactgcgaagtgagttggctggtaaagagtacctctggccatacagcatgccgccgaaattaaaagcggaccattctgatattgtgatcgcccaaaccgaccccaagagctatgagtaccgccagcaggtggccaagatccgaaaaattgaacgaactgccgagaccggagttcacgtcaatatcgggttgacgaagaaggccatcaaggacttaactgctcaggatgccaatgtgagcaccgatgatctgtatctccaggcagcggttggctttatgcgctaccgctggctgttgacgtacctgtttggcgcaacaccggtggcctttaccaattattttgctccagataccgatgcgcctaccagtccggtcagatcactgcgcaactctcattttggctttggaaatgggtttatttccagttatcaaagtgtccagcagtacgttgacggcatcttgaaggccgtggatgatcaaaagctgattgcccagcgtgagtattatgggacggtgcggttaaagcgcagcgataatgtttctgccctcctaaccaagggaattgcctacctggagctgagaatttacgatttagatccttttgaaccgttgggggtgtctgaagatgccgttgacttggtccgtttgatgtttgcttattttgtcagtcatcgtccatttgatttgcggacggcggacgaagatattgccaaggcagaccagaagaatgatgtcgttgctttggaaaatccattgaagattagtcaatatcatgatgaggcggcggaatttatcggtaaactggaaaagttcagcgctcaagctgttatcccattcaatgctcaacatctgtgtttcaaattaatggaaatgattgacgacccggtgttgacgccgagtgggcgaatggttaattggctcggtgaagactcgaaaaaggtgtttgatgaactgttaaaatttgccaagggctaccaggatgatttgattcataacccggcaatcggcttcgaatcattgagtgccgcggaccagaaggaaattttggcgaccttgaagcagggaattccagtgagaattaaataagagtggagcaagaggcgttttgatcccagaatgtaaggagattaagcgattattccgggacttggaataattgcttaattggcttacatggccgggatcagccgattgctgcacgtttcggcaaggtagaagtggtgtacaaaggttgcgggctaagcggaggaagcagcctgaaagcccattccatccaaacagaaattgcccacacaaaaaggtcggaacaataggctaaaccacctacgttccgacctttcaatatgcattgatcaattaataaaaactaggtttgctccactcagttcccggctcacccaagcctaagctttctcgatggtaatccgcttttccggttaacaggtcggtgacaaactgagcaacggcttgtcgggtgacttgcgcttccttgaagggttcaccctttttagtaacgtgaacctgcgtattgccggcttgattatacagccaggtgatccgcaaaatcacatagtccaaatcactggcttcgacaatgtcggccgacttctttcgatcagatttccaaataattccggtgtgttttcgataccaggcttgaaacttgccggtaacttcctggtataagtcaggaatgttggcggaaatgaaccgagtgaccttggcttcgtcgagaaccttcacaatgccgccggtgatttccggtccggcaacaaagctcagatacactgcatcaacgccacttaagttggctttgattttatcaaactcggtgaagtcgccatcgacaaacgtcacgcggggactctttttggctgccaagcgagatgagacgttatgaccatacaagaccaaatcaaaatcggtttgagttaacaggtcatcggtcaccatttgaccaatctggccggctgctcctaaaatcattactttcaaaattttacctccattgggttacttatcgtcgttgttccagcgaccgccgccacccagacgttcaaccatctttggatcacggtgatcaaagaatgccgattccttcatatccaggttttggatgagctgcatttcttcatcggtcaattcgaagtcaaagatgttgatattttcaatcatccgctctttgtgaactgacttggccagtgtgacaacgccacgttggtacagccagcgcagaacaacttggccaacccctttatgatgattttgggcaatttctgataagacatcgttggtaaataagccgtgcttgccttctgcaaacggtgcccaggcctctggctggatgcctaatttcttcatccagtcgagttcatcctgctgctggaaccagggatttaattcaacttggttgacctgcggggtgacctcgttatgctgggcaaggtcgacaaatcggtcggcattaaaattggagatcccaatggctcgaatcttgccttctttttgcagctcttccatggctcgccatgagccgtaaacgtctccgtatggttggtggatcaagtaaaggtccaaataatccagcttcaatttggttaacgcctgctcaaactctttcttagtcgcgtcatagccggtatcactgacccaaactttggtggtcacaaacagctggtcacgagggatgccggattctttgatggcgtcgccgacttcggcctcgttgccataagcctgagcagtatcaatgagtcgatacccagccgagagagcatcggcaacagcttgtttagttccaccgttttcgatttggaaaacgccgaatccggctgctgggatttcaatgccgttatttaatttaaatgttggtgtattcatgatgattattctcctttatgattgtctttcaaatatggcttctgccagagtttctccgcgttgtcggcggtcatttcaccggcatcgaatttggctaaatgctcatcgaaggtgtcaattttatatttcaacagggcttgcgtgtcctgcatttctttgagcttttcgtttaaaatcgtcaactgttcatgcagaatatccttttgagcttgccggacggccccacctttgcgggccagggtagcaaactcaatcaaagattcaattgacaggccggcgcttcttaaacttttcgccaggaaaatccaattcaagtcattggtttggtagacacgataaccgttgtgatcgcgtttaaccggggaatgacgccaatccgctcgtaatagcgaagcgtatcggtagaaaccccaagtagttccgagactttcttactgttcatgatctcaatacctccgttcctcaactgacaaatacaatataaaccgtggagtggactccatagcaagcaaaaaaactttaaatatcaatttaatttatttcagatctggttatttgatttttgaaagactaaactgagtttcaaaggagtgatgaatgaatgtgtacaagtgtgacttttctatctgaaacgggcgacaactttttagctcgaaccatggattttgcttttgaattagatggccgaccaatcgtgatcccccgaaagcagcattttgacagtgatgccgcagaggctggatacgatacgacctatggttttgtcggtgccggcagaaacttgggccattatattttggttgacggtgtcaatgagaagggcttaagcgcagctgcactgtatttcagtggcgaagcaacctacgccaaaacggctaagactaaccgggtcaacctggctccccacgaagttttgaattggctgttgggcaatgccagtgactgtgaagatctgggccgcaaagtcgaccagctgaacatcatcgatgcaccagtcaagattcttggcaaggccaccccgcttcactggatcatttctgatcgctcgggtgcctgctatgttttggaaatgctggcagatggcgttcattatcaaaagaaccccgttggcgtcatgaccaacagtccagactttggctggcatctaaaaaacctcagcaactacaccgagttgaaaccatcaccacatcctgcccgctcgtataacgggtatgaaattacgtcatttggccccggaagtggggcgctggggatgcctggtgactatacttctgtttcgagatttattcgcaccgtatttatgcgggaatatgccgatcaggtaccaactgatcaaactgtcaacgaactcagccacattttgaactcggttgaaattcccaagggtgttaagttgaagcaggatggcagcgaagactacacccagtatcgcggctatatggatatgaaaaattgtgcttactatatgcagccttacgataatcaaacgatctacaaggtgtccttgtcggaggaacttctgaacaagaaggcaccgagtgaatttccaattaagcaccaacaagtatacgaaacgcttcggtgaggtatcctcactgaaagcggcttgtggacacatgagttgttaaaatccaagaaaaaaacgctcgatcatccctttactggaatggtcgagcgtttttgaatgccaaggaaacctattttcgggtcttgtcagcaaccttttgactgcggttaatgaagtccttgaacagcttccgcgagtcttcataatgcttgtaaatgttttctggatgccactggactgctaatatctgatcattatctactgattcaatcgcttcaatcacttggtcatcggctctggcggtcaccttcaaatacggagcgacgtctttaacggcctggtgatgacgtgaattgacatatgggcgctggccaataatgtcattcaagcggctgtgtggatcaactgtgacgtgatgagatggcatgttgcctggggcttcctgggaatgtttcaaagtcgcgtgtaagtcctgggacaaatcttgataaagggttccgcccaggccaacgttaatcagctgcatccctcggcaaattcccatgatggctttgccggcagtcacggactgtttcaataattcaatttcaaataagtcgcgtttgagataagtcatgcccagcttctggaatggttcttcaccatagaaagtcggatcaacatcagcgccgccaaggaaacagacgccgtcaaacagtgtcatataatcgcgcacgtcttcgggattgacacttgggaaaatgacaggtacgccaccggatttaacgatggcttcgattgctggccggggcgcgaacgcggcgtttcgttcattaatgacgttggttgcctcggcgagcgtgtcagcaggtaatgcgattcttgggcgcaataaaatccctcctcaataattagtttcagtctatttgtgttattgtactccaaactaataaatttacgtgatattttgattgttgtcaatgtaatttgagcttatttgtctacttttgatttgtcgggttcccaactgcccttgaataattcctgctttaattcattggctgacagcttggctttattttcaaatcctttaaatgggcgaatcgactggagtgccgattgttggtagcgcttggcccgtttaatcgcatattcttccaaagaaccatttttcaaatgagtgattaatttcgcgcttggcgtggtgagtggattttcgacgcggtcttggaggtcttcaagttcttcttggtattcaggtccaagctggattctatccgcgtacatttccaaactttggagaaacgctctggcattggcttgatatttggaaacatcattgggatgttcttcggagacttcttcgttcatcttatccgaacgggcgatgaccttctcaacttcctcaggattcattgccggcgacatgatgaaatagctggccagtaaacggataaaccgtaacgtattggtccgaatccccacagaactgctggggtcaaggtcgagcattctcaattcaaggtagctaaccccggtcttcggtaactcccgtaaatgggtattgcccttaaagcggacggcaccatggaattcgtaatctgaaatcagcttgccgtcagcgacgcctttttcaattcggtcaacataacgctgaacgttcgtatagtcgccgctaaatggattgccaaagccgtgtgaactctggcggatactacgaatcggtgcttttggtcctttacccggatcaaaatagttggcttcagcgacagggctggcaccaaatagatatgtaatgacccaacgataccgcagaaagccttgggcaatcttggcgtataagtagttttgcagctcaactttggaattgaaacgatcgctcatgttagccagaactaaatcaaacacatggggatcgatactcaagttgatgtgcgcgccacaaggcgttccttgagaaaatccgtgacgtttcagccattcttttaagtaggcttccttcttgggtcccattttagcaaggggaatcttgctcttgtcttttggcagccgcggcggcatcgataacggccacaacagctcacctggcgacagggccgaccgcaaggcgttgttaatgctgaacaagtagtgcatggcgtccagggcgtgagcggcaggtggggtcacgacctcagacatggtttccagaaaatcattggtaatccaggggttggtttgttcgtcaccggccccggctgggtagggttcttggcttaaattgccattttcatcaactcgctgcatctcaatttcaattcccatggtaaagtctgaagttttcgcaacggcttcgttatcaaatattaactgaccaatttcactgaacatggcatacctcctagttgaattaaaatttgatgataattgatgacaaaatactaacactatcgcggactataagcaatgctaatggtgttatgtcacggagatttgtgctaaaattattttatttaattaatttctaatttagaggtggaatcatgagtatctttgtcaaactgggctggtatttcaaaagggaatggaaaatctacctggttggtttatttggcctgctgctgacggcgttggtcggaattattccgccacggattatcggtaatctggtcgattcgattcataacggtaaattaacagctaaatatctcatgtttttgctgattgttttgacgattgtctcctttgcccaatacggagcccgttatatgtggcggaccgcgatttggggtgaagctgcgaaattggaaaaagtgctccggaatcggttgtttttccactacaccagtatggatcatgaattcttccaacgctatcgaaccggtgacctcatggcgcacgctaccaacgacctgtccgcgattcaacgggtggccggtggtggaattttgcagttcgccgattccatgattaccggcggcacgaccttgatcgcaatggtcacgttgattgattggcgattaaccctgatcgccattttgccgtttccgctattggcggtgatggcgcgatatttggggactaagattcacattgcttttcgagattctcaagctgccttttcacggctgaataataaggccgaggaaagtattaccggcatcaaggtcattaagggccttggccagcaaaaagaagacatgcaggattttgacaaccaggttgccaggacgattaatatcaaccggcgggtcaattttctggattctttgtttgacccgatgaccaccatgatcatcgcgctgtcctatgtgattacgattgtttacggtggctatttggtcaccaatgggacaattacaattgggtcgttggtttcgtttgtttcctatctggccatgatgatctggccgatgtttgccgtcggtatgctgtttaacacgttggaacgtgggaatgccagttatgatcgggtcatggacctgattaaccagcaaagcaaggtaattgacgatcccaatggtgtgacgactacaccgaagggcgaaatcgattatgacgttaagcgtttctcatatcccggtgataaacgactggccctgcaaaatattgattttaaagtgccggctggcaaaacggtcggtttggtcggcaaggttggttccgggaagagtacgattttacggctgattttgcgtcaatttgataattatgaagggtcgattaagtttggtggcattgacatcaagcaatataagatggacgctttaattcctgcaatcggctacgtgcctcaagatacattcctgttctcacagagtattcgggaaaacatccgctttgcccgtcctgacgctacccaagctgaagtggaacaagctgccaagaaaagtgatttgtatgaccagattcaagcgatgccagatggttatgacacggctgttggtgaggaaggcatttcactttcaggtggtcaacgccagcggctttcaattgcccgcgcgctgttaatcaacccggaactattaatcttggatgatgcgttatctgcagttgatgcggaaacggaaacccaaattctcgaaaatctgcacgctgaacgttctgataagacgacgatcatttctgcccaccggttgagttcagtgatgaatgccgatgagattttggtgatcgatgacggcaaaattgttgagcgcggcacgcacgatcaattaatgacccgcggtggttggtaccacgaaatgtttgagcgtcaggaactggaaaccaaagtgaagggaggcaacagctgatggctgattcatcaaagcatcaatctgcctggtcgaaatccattccagttaagcagcagatgcacattattgggcggctgttcaagtacgctgccccctataaatggtatttctacttttcagtcctgtttgcgattgcggttgccgttgtcaatattctcttgccaagaatcattcaaacctttatggacagccacttggtcgttggtcatcctgattttgcgatgatgtggttctttgccggtttgtacttctttggcatgttggcaaaggctgtgatgcaatttacccagacctatctgtatgaaatgggtgctgagtatatgctcgaaaataccagacggaaactgtttgcgaaactgcacaccttggggatgcggtactttgaccagacccccagcggttccattctttcaaggttaaccaacgataccatggcctttgcaaacttctgggccctgttcagtagtttggtggtcaccatttcggccatggtttcctcatttgtcgcgatgtatttggcagacgccaaaattgccatgtggctgttggtgttcatgccgttcttgttcgtgacagtctggtactatcagcgatacagtacccgggtctaccgtcggatgcgtgaacggttgagccttttgaacgctaaattagctgaaggcattaccgggatcagtgtggttcagcaatttcgtcaggaaaagcggatcaatcacgaatttagtgacaccaatgaccagtattacaatacgcgccgagcgatgattcgcatcaactcgttgttgttaaacccaatcatcaacttgttctatgctttgggtaccgtgctggtattagggatgtttggtatccgtgggctgcatggctatgtgcctgccggaataatttatgcgtttgtgacttatctttccaacttctataatccaatgtccgaaatgatggatcgcctaagtgacttccaagatggggtcgttgccgggtccagagtcctgcggattatggatgatcagacgtacgaaccgcagcagcacgcggatcccgatgccacaattacccgaggaaaaatcgaattcaaacacgtcaccttttcttatgatggcgaaaatgatgtcctacatgatatttcctttgtggccgagccggggcaaaccattgccctagtgggtgaaaccgggagtgggaagacgtcaatgattaacatcttgatgcgcttctatgaatttggtgaaggggaaattctgattgatgaccgtgatattcgtgattacaccattcaagaactccgcaagaaaatggggttggtgctccaggaacctttcatgttttacggaaccgttgcttctaacattcgaatgttcaaccaagaagtcaccgatgaagaagttcatgaagcggcacgatttgttcaagccgatcaatttattgaagacttgcctgatcaatatgactcacgggtgatcgagcggggggccagttattccagtgggcaacggcagttgatttcctttgcccggactttggtgactgatccgaagattttgattctggatgaggcaaccgccaatatcgataccgagaccgaacagattattcaaaccgggttggccaagctccaagaagggcggacgaccattgcgattgcccatcgcctttcgaccatccaaaacgctgacttaatcttagttctggaggccggccggattgttgaacggggaacgaatgacgagctgttggagaaacatggtttctattacgatatgattcaacttcagaattccgcccatttggattagggtggtttgcgaattttgactgaaaaaatggttgatagcaaattttactttgctatcaaccatttttatattacggtattaaattattgaatctcaatattgccactgtcttcatgactatcagcagcctttggcaatgtgatggtcaagacaccatcattgacttgagctgagatgttgtcacgatcgacaccaggcaattcgtaagttctggacatgacaccatgactacgttcgctggcaacgacccggccttgttcgtccttcttctcagaatcacgttcttggtcgatgctcaatgccaagtcaccatgttgatatgccagatggatgttcttcttatcaatacctgggacatcaaccttcatgatgtagttcttatcattttcggtgatgtcagtctttaaatcaccatttaccatgtagtcgttgtctgcatcagttggactgaagaaacgacgtgccaaagtatcaaagaaaggatccattgcgaaacggttcattaattcatttgccataataccaatctcctttgttgattattaataagattaattaataagcgtcaaaggtggtgaaacggggtctcggaatcacgttcccccaaaagaagctttactgaagtttcaaaagctgactacctgaatccctaaccaaccactccaaaatattcgtcaaaattactgaatatcaatgttgccggtttgatcttcgctttcagtgacttttggtaatgtcacatttaaaacaccattgtcaatgtgggctgaaatgttgtcgcggtcaacaccaggtaattgataactacgtgacataacgccgtgactgcgttcgctggcaattaccttgccgttttcatctttttgctcagatgaatgttcctggttaatattaattgagagaacgccatcttgatagttcaagtgaatgttgttcttatcgatgccgggaacatcaatctttaatgaatagtctttatcggtttcgttaatatcggtcttcaagttgccgaagttctcataatccttgtcgaaatcagaagggctgaagaagtggtgagccattcgatcaaagaacggatccaaatcgaaacgattcattaattcatttgccataatatctatctccttaatttcaaaatgattattcaagataacggggaacaacacgtcacttttttgttcctcctttacctttcaactactatgataatcagttttaaaatgaataccagtatttagcactctaatgttgagagtgctaaaattttctcttgaatggacaatatttgcatctaacaaagctcgcctatgcgcgttatcattgggatgtgctatgctgaagtgagaaatcaatgaagctgggtgaatggtcatgatcgatcgttttttcaacaaaaagtttatttggaagatgatttgggtgggcattgggacaattctggcctgcctgttatttctgtcggtcggattttctacccaactctcaccagcattagtcgatcaaaatgacacccccacccagcaggtcgatacaacgactacgccggcgtacagtccggaaacgaatttccactggtcaaccaagacagttgcctactttattactaagcagacgaacggccattaccgagatgtttggatgcgggcagtcaaagcctggaatgcggtcggggtcgttgatctgataccagcagacgatgcggatcgtgctgacgtcatccttagtgtcaaacaatcctatcatgaaggcggcggtacggttgagaatatcactggtggggtggttggctacaccagtgaggaatttggtcacgtggacgggatcccgctattcgtccatcaaaataaaagttatctgattattgattccctgaagcaagcccactacgattctgtcaatgaacaggcaagcgtggcaatgcatgagctggggcatgacttggggttggagcacagcgacagtccccattcgattatgcagcaggcggcaccgacttatttggatagtattccagaagttgatgccaagcatttggcacagttgtatgctggggtgccgcgggggtgaaagtagccgtattacctattatggtgatgtttaccatgcaaaaaaagagcggctcagaaagtcgctccaattaatagaactctaagtattgaactcaccaaacttacactgccagcaataccccgacagagtagtgaatgatcatggtgatgatcccaacaataatatttcgaataatagctgttttaaccaaaccattccccaatcgggcacttagataacctgtgagtccaaccgagaggcagacggccagaatagttgccggccactggaaggcaactggtgtcagcgtcatggcacacaaggggaagataccaccggcagaggcggaaaagagtgatgagaacgctgcgtcccaaggattcatgtagtgtcccaacttgagaccgtatttgacattgacaatggtttccaaaggatttttgctcattaagtctttggcgatcttatcggcagtttctttggtgacaccctgatcaacgtaataatcggataccacgttgagctggtcttgataattggtcttcaataatgctttttctttcgtcaccacagattgttcagtatctttttgggtactaacggacgcatattcgcctgatgccatcgagaaggcacaagccaacaggtcggataatccagcaatgaagatcgtaaactgattggttgtcgcaacggcaacactgaacagcaccccaacaacggttaagatcccgtcgttggagcccaacacaccggcgcgtagggtattgagcttttcgtccattgtctgcccatcttttttctttttggaacgaacacttaccatgttcttcgcctcatttctctaaaatgtgatgttcaagatccaattaaagtcccaattgtgtaggtgactaacatggtcaaaatcccggaaataatgtttcgaatcatgccccgacctttgttggcgttgcctaattgagcggcagtgtaaccagtgatcgccaatgcaattacgacggcaatgaaggttgccggaatgcgaatggtctttgggaacaaagtaatcgctaaaagtggtaaaattgaccctgtcggaaatgaaatcattgaagcgattgctgctgataatgggttggtgtattcaccaacgttgaagccatatttttggcgaaccgttgtcttaaccgggtctttcgccatcatttcagaagtcgcttgggccgctaaattggcagagatgccgtcacccatcagtttgtgcttgacggtgttgaattcattatcgtaagcggaacttaaggccgctttttggagactgatggcgtgtcgttgagaatctttttgggtattaacagatacccactcgcccatggccattgagacggtcccggctagcatcccggaaataccggaaataaaaatagcaaaattatttgatgtcgccccggcaacaccgataacgattccggcaaccgaaacgatgccgtcattggcccccatcaccgaagcccgcagaacattaatcttttgtgaaagcgatcttttcttcgccatatgctcacctacttcatagtttataatcattattatctaacaaaaattattctagtcctttattgtttaaaagtaaattaaaagtattgtgttagctaacgacgttatcatgtcacttgacacatatgctgtgaagaaccaatttagaatcactatcaaatagttagccattaatcttaagaaggagatgccactcgtgaccaacccgattcttgaacaattaactcagcaccgtagtattcgtgaatttgaagatcgaccgctgagcccgcaccaagtcactgaattagtgaatgcggcccaacatgcttcaaccagcaccttttctcaacagtattcgatcgtcagtgtaactgatccagccaagctccacgcgattgctgacgtcactggccatcgttggatggtaaatggcggtcactatttcgtgatggttgcagatcagtatcgaaatctaaagattgccaaagcacatggtatcgatccatacatgttgcattcaacagataaatttctggcaagtgtctttgacacggcaattgccacggaaaacatcatggtggctgcagaaagcatgggcctcggcgggaccattatgggcagcgtcttgaacaatcccagaaaaatgattgaattattaaatttacctgagatgacatttccattattggggattgcactggggtatccaaaagacaaaccagaattgaaacccaggttgccaaaagcatcaatgcatttcgaaaaccaatatgatctggatgcaaactttgaccaggaactcaccgattatgatcagctaattcgcgagtattatcagtctcgcagcaccaatggtcgatcggaaaccttcagtcatcacattgtttctgaactcagcgggaatcggaatctgcggtcggatttgtttgcgatgatccaagcccaagggctgatgacccactaaacaattattagtaaaaatagttgacttttgagatgtttaacattacattattaggtaattgattgacagtcatttgaatttcacaatgttgaagagaagagtacgttgttgggctgcacaaagcgaccgctgatagtgaaagagcgggcagacattgaccgaaagtgcgctcggagttgtggcatttaattaaagatgcattcgaaatgaggcgttttgtttttgacaagacgcaaaaaagggtggaaccacggtaattcgtccctgatgatcagctgatgctggttgtcagggacgtttttgtgttcaaatgactgcaaaataacttgtgaggagatgattgacaatgagcagctgggccgttatccaacagagcttaccgatgtttgagaaggggtttcaactcaccctgtggctttctttcgtcgggattattggatccattattgttggcataattgtgagcctgcttcaatatttcaaagtacccgttttgcaccaagtggcatcgatttacgttgaagtttcgagaaacacaccgttattgattcagctatttttcctgtattacgcgtttccagtgatcggcattaagtttggtgccgagttgtgtggcattatcggattgatatttctcggcggcagttatatggccgaaggctttaccggtggcttcaacggcgtttccaaaggccagctggagtctggtaaggcaatcgggttgagtcgttggcagcttgccagatacattgtcttcccgcaaggattctcactgagtgttccggcgatggcagctaatgtcatctttttgatcaaggaaacttcgatctttacggtgattgccattccggaattgactaacactgcgttggatttgattgggatgtattaccggtccaacgaatatttattcgttttggttgtcggctatgcgatcattttaattccactatcaatcattttgactttactagaaaagagggttcgctatggatcattcgggaattagtgttttattcgaaggaaccaattttgagcggttactcggcggcctctgggtaacggttaaaattgcggcagtggctttgattgtcggcctcatcttgggaattatcctgggtgttttgaggacctttaagaatcggccattgcgagtggttttgagactgtatcttgaattcttcaggattgtcccaaccgtcgtgctgctatttttgttctattacatcttgccacgccaattgaattttaatctccctggcgatcaattggccaccttggtatttgccttgtgggtggctgctgaaatgagcgatattgttcgcggcgccttaatctcagtgccacagcaccaacgcgaatccggtaaagcaattgggctcaatcgttatcagctctatcgttacgtattgattccccaagcaatcagtttggaaatcccggcgaccatcaatttggccacccgggtaatcaagacgacttctcttttgatgctgatttctgtgatggatgtgattaatattggccaacaaattattgaagccaataatcacactcatccaaccggcgttttctgggtttacggattgatatttctattctatttcctgatcgattatccactatcctggtgggccaagcgattagagaagaagagattggagcgggcaaatggctgagcagattttacaagttgaacatttagaaaagtattatcaaaagaaacacgtcttacacgatattaattttcatgtcgataagggcgaggtcgtcacgttattaggaccgtcaggatctgggaagagtaccttgattcgctgcctcaatggcctggaggaataccagcaggggacaatcacttttgaggggaagcagattaatccgaccgagaaaaattggcagcagatccgccaaaagatcgggatggtctttcagagttatgacctatttccaaatttgaccgtcatggacaacatcctacttggacctaccaaggtgcaaaaacaggacaagttcgctgctaaaaaggaaggtctggagttgttggaacgagtcggtctcgaggattatgccaacgcatatccccggcaactgtccggcggccaaaagcagcgggtcgcgattgttcgcgcccttgccttgcatccggattttatgttatttgatgaagtgactgcttcactggatcccgagatggtccgaggaattctcaacatcatccaagacttggctgatgttgatcacatgaccatgatcgtggtgactcatgagatgaactttgcccagcagattgctgacagagtgattttcctggaagatggccatattttggaacaaacaccttcaaaacagtttttcagcgcaccacaaaccaaacgcgcacaagcatttttggatagtatggatttctaatattgaggaggaacaatttcatgaagaaaagatcatttaccagaattatcgctatcgtcagtgtcttcgctgctttattactggtcttaaccggctgcggtaacagcaagaagtcaagttcgcaaagcaataacccaagttccgttcagcaaattaagaaaaacggtacgattagaattgcggtcttcggtgacttacctccttacggttgggtcaacaaagacggcaagcgcgttggttacgacgtaacattagcccaccaggttgctaaagacctcggagttaaagttaagtttgtccaagtcaatgccaacaaccgagttgatgctttgaactccaacaaagttgatctggttctggccaacttcacggtcaccccagaacggaaacaggttatcgattttaccaaaccatacatgaaagtttccgttggtgtggtttcacctaagaacaaggcgatcaccaaggccagccagttgaagggtaagaatgtgattgtgaccaagggaacgactgccgaaaactatttcacgtccaagcagcctgatgttaaactgttaaaatttgattctaagacgcagcagtttaacgccttgaagaacggccgtggggttgcccttgccgatgacaactcatacctgtacgcctggtccaaggataacccaaactacacggttggcatcaagagtatcgggcctaagtcctacattgctccggctgtgaagaagggcaacaaatcacttcttgattggaccaataaggaaattaataagttgaccaaggagagtttctttgtgaaagattacaatacccaattgaagccttacttcggtaaagaagtgaaaccttcagatattgttctgccagttaaataatcattgattaggcagccaaaaaagcttttggctgctttttctaacattaaaaaataattagagttgacgaactgattctaatatgttttaataagttcaacatttcaagaaaggaattatctctatgaatactcaacttcaacaattgaatgcctattattacggctatgcatggtttaagtagcgctcgtcagatgcgggcgcacaacgcgttcgcgtctaacctgggcaaagtcgtaactttgttgctgccagctagacgctagagtctagctggatgggtataatttcttaagcgagtgaataagaaatcagccagctggattctaatatccagctggctttttgtttacttacatacttgggagagtgatatcatgacagaattaatgacaaaatctaataaacgcagattatcaatggccttatacctcaactacctggttcacggcattgggttgattattttaacccagaatatgcaggctttgggtggcttttggaacgtgccgattgcgacggtttcctacgttatttcagggattggaatcgggaaattaattgcttacttcatcttcggttacctctcagaccgttttggccgggaaaagttggtcttaaccgggactctgagctacatggtattctttatcgggattccgtttacccacaatatcgcgattgcctacctgtttgcaattattgccggagtagccaattcggcgctggattcgggaacttacccgacatttgtggaaatgggcggtaattcaagtgcctcgaatgttttcattaaagcatttatgagtgtaggtgaattcatcctaccgctgtttattgctactttggaagctcatcaattatggtttggttggtcattcattggcgccttgctggtgttagtcgtcaacttattcattcttcgcggcgcacacttcccagatcggaaccaggttgacgaagaattcagcgaggagcaccaatcactttccaaagttcggcgagtgattgcgacgattgcccttgcgttgtacggttacacaaccatggcaatcatgattttatttacccaatggattagtctattcgcaaccaacgaccttggttacagttcattgatttcccacggtctgttgtcgctgtacagtatcggttcaatcagtggtgtggtcgtgatgtttatcctgttaaaattgaatttcaccgaaacgaaactgttagtggtgaccaatacaatttcgttaatcgcaattctcacggtgacccacgcctcaacggtcattgtcaccgccgttgcctgcttcgtattcggcttcactgcagcaggtggggtgatgcaaattgccctgaacgttttgttgaaaatgtttccgaagcataagggtgtgattaccggaacttactttacgtttggcagtatcgcaacctttacgattccgattgtgaccggaattttgtcgaaaaccagtcttcaatctgtgatgaattttgatgtgatgattggcttggttggaacggttttagtggtcgtgacggccttggccatcagtactgggaacgtcttcgcccatgccggccagtcgatgatgacccttcttcatatgggaccggcaccagttagtcagggacgctcaaaagacgaatagtatgttaatcaaaaaggaaaccgcaactttgcggtttccttttattgtgtttcaaatcgtttcatttctgttcgcagatcgtcaatcgcaatctgtccgggggctgatgcatcaccaaccgtcgcaaagctcataactgatccaaacaatggcgcggtgattcgagagattcttcccagactgcccatggaaattgcaatgattggaatttccaacttgtctgattcggttgcagtggcccgcatcattgtgaggacgtccttgaatttattgggcatggcagcaatcttggcaatatcagcgttttggttctgcatctgctccaggagattgataatctccagttccggcggggtgccttggaattcatgggcactcaagattaccttgatgttgtgttggtgcgctaagtaaatcaggttactaattgcctcttcgctgaaatgcagctcgacatccaacatgtccgtcaattcattggcaatcaaccgtttatatagggtcacataagctgcttcatcaaggtcggcttcaccgccttcgccagcagttcgaaaggtggttaagagaattgtgtcgcccaaaatttgccgtaatttggcataagtggcttgataaatggcgggatccaaaccagcttgatcatagtcgatgcgccattcaatgacgtccgggtgagcagatactgctgcttgggcctgcgcaagaatatcatcgacggtccgaccggtgatcggcaccgctattttggtggtcccggttacaaatgacgttcggcgaactgttagctttccactcatctcatcaacctctcttttctgtattaaaatcttgtcccaattctaacaagcggtgaccgcaacttcaatctaaaaaagcctcccaaatatcgggaagcttctaatttcagttaaaatccgcggaaatctcctctgccaaagtactgcaggttagccaacaatggtttttgcatcagcgtcggcaaggtcacaaatgtgtagccccgtttcttcagcgatcgaataatctggggaacagcggcaactgacgtcgggtgaatatcatgcattaaaataattgagccaggatgagtcgttgccagaacatgactgacagttttcggtgtatttagatatgcccagtctctggagtcaacgttccaacggacaattggccggtcaaacaagttcccaatccgactgttaacggcgccgtatggtggccggatataggtgggaattgttcccgtggccttataaatcgctgcatcggtcaaggcaatctggtgaattgctttggcactggagagagtggttaaatcaggatggttccaagagtggttaccgatttggttgccatatttgagaaccagccggctgatacttggatagcggataacactgctgccaacctcaaagaaggttgcgtggacgttatagtgctttaaagttttgagtaatttcggcgttagggtcggatccggaccgtcatcaaaggttaaagcaacgactttcttgggtgtttttggtttgacaaagtcatattgcgatggcatgtagcaattgagaataatgccggttaacttactcaatggaatggcgacgtctttgacaccatatgaatttttaaccagatgaatggttaaagccgttttgctcaaggtaaagttatgggctgttaatcgcttgggtaacggcaggtaaatcaagttttgaacctgcttgccggacagcttgtgatcttcagccagttgggcgcgcgtcaattggcggatggtgcccagacggtggagactgttattggtgattttgccataggttaatgtagtcgctgcatgtgcttgtgggactgaatgattgctgatgctgaatgtcaataacgatgcagctgcgatactgaacgttaataatgcgcgtttgttgatcatgatgatcaccccaaattactttcaaattttatttcaatttcattttcacattgcctttgtgggaagtcaatcaaacttatttttgaaattttttcgatgcgattaatccttgatgacacggtgatgtgacaatcaaaacgatcaattcaccagtgttgattttaagaataggtgttgacaatttttccagaattcgttattgtacatgatattagatatcgatgagaaagtgcttagagaaattgaaaagtcggtattaagaaattccaagagagcgtcgttatctgtgaaggcgtaatttcttaatcacttaaagtcaattttgagcacggtggttcgtcaagagtcactagggtgcgcccaatacagcgccaacgtataccgagtcgaccggtcgtacgtgagaggtggaatgattttccacaatgaaggtggtaccgcgcaaaagcgtccttttagaagtttaacttctgattggacgctttttgtgtttcatggacacaagcgcggctgtatggtcatcgatatcaatacaaaattattggaggaattgcgatgtttaaggatattagatttacagccattatcagtgttgtcattgggttcatggctgtcttattaagcggctgtgcgtcgacagcagtcggcggcggtgcaggaagtgccgaaaaagccttaaaaataacaatcccaggggagccattgacgattgacccaaccaagtcgattgaaactaatggcggtgcggttatcgatcaggtcagcgaaggcatttatcgcagggatgcgaataacaaaattgctgccggagtggttgataaagttgtcaaaccaactgataacggcacaaagtacacgtttaatatcaagaaggatgctaaatggcaagatggttcaccaatcaagtcggaagattttgtcaattcgattgaccggcaggctgatccgaaaaccaagtcccagcagacgacatccattcaatacatcgaaaactttgctgctgttaacagcggtaaggccgatccaagtaagctggggattcatgcagttaacgaccgaacatttacggttaaattgaccaagccggtgccattcatgaattatgaatttacgaacttctatccgattcaaacggcggccattaaaaaatatggcagtcattacggcactaattcagagacgactgtggccaatggtgcctacaccatcactggctggaacggtagcaatgattcctggaaatatgaaaagaataagaactattgggatgccaaaaacgtcaaaattccagaagttgatgtgacagttgttaaagacaataacaccgcgcaaaacatgtttaacggcggacaaattgatttgaccagcttgactggacaatacgttaaacaaaataagaacaacaaaaatttggtggtaactgaaacaggccgaaacaattacatttacttcaatgataagaagaaagccacttccaatgaaaacttgagaaaggccatcagcatggtcatcgatcaggatcaattggcaaaggatgtcctccaagatggctcgattggcgcaaacaacatcgtcccaaagaattacgccaaggatccgaaaaccggtgaggatttcacctcggaaatgggcgatcaagcaccaactgataccactaaggccaagcaatattgggcaaaggctcaaaaagaaattggcaaagacaagatttcccttgatttcctggtggatgatactgacacagaaaagaaactcgcagaatatgttcaaggagccgtttcagacaatctgaagggcctgaccatcaatattgaatccgttccgcatgccacccatgtaacgcgtgatttctcaactgatttcgatatttgtacggttggctggggacctgactatccggatgcccaaaacttcttggacggtatgcgcagcaataacaccattaacttctcgaaattcaaagatcaacagtatgatgacttgatgaataaagtggatgacacaactaagtacgatgccaaccagcgttgggactttgaaaagcaggcagataagcgcttgatgtcaatcgccgcggtagcgccaacgtatcaagcatcgcaggcccatttgatcagcagcaaggtcggcggtttgaagtgggatgcaatgtcgggccagtccgggaagttgcagtatgcgtattggaagtagagagagcgcgacgagacccgggtggtcccggagtgtaagacgaaaattttaatgatgaacggtctttgttcatcgttgaaatttttgacttacacggtagggaccagggtcgtcggagcgtattttcaaagccgaagggagcacacaagaagctaacaaacgtgcatttcgcctgaaatctgggcgactaactgacaaatggaagttagcgcttgggtcgtcggagcgtattttcaaagccgaagggagcacgcaagaagctaacaaacgtgcttttgccccaaaactcacagcttggctaatctaaccccatctccacaaaagtaaaaagaaatctccaaccaaaaaatcccacttaaggaggcggttgccatggcatatcagttaacgaaatctaaagatgtcccatctcagttagtctgcaaccaagcattttacatcgaaaggaagatttattatgacaaaaatcaattatacgaatgttgcaatttacaaccatgagaagcagaactttatcgctaaccaacacatggtcgtcgatacggataccggcaagattgttgaagttggcaatggcagttccacaaaccaagttgtcgatgaagtttccgatatgcacggcaggtacgtgatgccgggaatcatgaacgctcatacccatatcaccagtattccaacctattggtggaacgatggcaaagagcagcgccattccgattcacgggaatttaataccatgtttgccgtgagaaatatggcggatgcaatcgatcacgggattacttacattagaaatgttggtgcggcttttgacattgatatcgaagtcaaaaaaatgcaggaaaaaggctggatcagagggccgaaggtgatgacttccggcaaggcattttcaattaccggcggtcatggatccggtggcggttatgaagttgacggcgttgacgaggttcgtaaaggcgttcgccaagctatgaagaatggtgtcgacaacattaaaatgatggtgactggtggcgtccttaaaaatggggaaacgcctgatgatatccagttcacgcctgaagaggccagaacagcagtcgtcgaagcccaccacaaggggaagactgctgcagctcatgcccaagggaacgctggtgttaaagaggcagttgcagccgggtttgataccgtcgagcacgcatttgatatcgatgatgagacgatcgcaatgatgaaagaacacggcacggtggtggttccaaccatgaacgcgatgtacgccatctacaaatatggaaaagacacggttcctgattgggctcgcaaaaaggtgattgtcaacatcaagaagcattttgccagcatcaccaaagctgttcagtccgggattccgatcgcaatgggtactgatgccgggacgccatataatggcttcagaaacgaaagtgcctacgagatggaattatatgttgagaaggcgggcatgacccctgctcaagcgatcgattcggccactatcaattgtgccagagccatgcacgttgatgatgagtacggccaaattgttgccggcaactacgccgattttatttctatggcagaaaatcccattaatgatattagtgtcattcagcacgacaaagacgtctatcaaaacggcacccgcgtccacaaacaggctgtcctcactgccactgagcggcaatcagccccaagtaaagtcagtgctgctatctaaaagtggcatcatctgctggaattaaaatccaatgagtgaatgattagggttgacgaataatttctaatatgttttaattaatacaacttttacgagaggaattgataaccatgacaaagcaattcactgaaacttcagcctattattttgactatgcctactttaagtagtgtccgcttcggggcggacgcaaatttgagcgttcgcgtccaagtggtgcagagtcaatgctttgttgagcccactagacgtaatagtctggctgggtgagttatcattctttacgaatttagtaaaccagctggataccatatctagctggtttttttaatggcaattaggggtgttaatcatgacaaataaaattgaaacagcaactgagagtgataatcaggcaattcgggcggcccgtgaacagatcaaccaactggatcaagggattgttgacctgctgaagcagcgatttcagacgtcggcactgatcggtatgattaaggaaaatgctcaacttccggtgcttgacggggatcgcgaaaaacaggttttggatcaggttgctcaactggactcggatcctggtacccgcaagtatctgcaaaagatattccaagaaattttgaagaactcacgtgattaccaacatgaattaatgcaaaaggagactaaatgatgaattacttaacagctggagaatctcacggcccacaattgaccggtatcattgaaggcattccttcggggctgcatttggatgttgatgcgattaacgaccaactcaagaaacggcaaggcggctacggtcggggcaatcgccaaaaaattgaacatgatgaagtcaccattaccggcggggttcgccacggaattaccctcggttcgccgattgccctagtggtgaataatcgtgatcatgcccattggagtcaaatcatggatccggttagccccgaaacgccggagaacacattgagaaaagttgaacgtcctcgtcccggccacgctgatttggtcggcgggataaaatatcgtcacggggatctgcgaaacgtcttggagcgctcgtcagctcgggaaacggcaatccgggtggcaatcggtgccgtctgcaagcaatttttacaacagttgggaattgatattgttggttatgttgaacagattggccaaatttccaccgatgaaaatcctgaacttaatgtggctaaaattgaagcagaaattagtcaaaacgacttgcgaatcattgatcagaccaaggttagcccgattcatgatctgattgatcaaactaaacgtgacggtgacaccctgggtgggattatccgcgtggttgccaccaacgtgccggctggactggggagttacatcagctgggataccaaattagatggcaagttggctgctgccgtgatgggcgtcaatgccatgaaaggcgttgaaatcggcgatggcttcaaggctgcgaccagcttcggcagtcaagtgatggatgaaattgattggaatcaggaccagggattcttcaggaataccgatcatctcggtggctttgaaggcgggatgactaacggaatgccaatcatcgttaaagcggcaatgaagccaatcccaaccttgtacaaaccactgcaaagcgttgacatccagaccaaagaggttaagaaagccaatgtggagcgatcggacacaacggcaattgttccagcatcaatcgtcatcgaaagtgtggttgccattgaattggctaaggctctcaccgataaatttgatggtgacaatttacaacgactacaagaacagcttgaccaatatcgcgatgaactgaaaaaattctaggaggtttctatggaaaaagttaaaacgcaatcaactaaacagctccaaggaagtctccaaaacggccttcaaggtgaattggccgtccccggcgacaagagtatttcccatcgaggcattatgtttggcgccattagtgaagggacaacgattttgcaccattttctaactgcagaagattgcctttccacgcttaaggcgtttcaacaacttggtgtgccgatcacccgagatggggacacagtcacgattcaaggcgttggtctccacggactccaccaggcggaacaaccgcttgatatgggcaattccggtacgaccacacggttgatcatggggctgcttgccggccaaaactttccaagtgaattaaccggtgacgcttcgttatccaggcggccaatgcgacgggtgagtgaacccttggcagagatgggggctaacattgaggtgaccgatggccatcttcctgctgtgattaacggggaacaattacacggagtcgactatcacctgaaagtggccagtgcccaagtcaaaagtgccctcattttggcggctctgcaagccgatgggatctcgatcctagttgagaagcagccgaccagaaatcacacggaaaagatgctgcgggcatttggggctgagattgaaactgaatcggatgacgtgacgattaccgtctatcctgaaccccacatgaaagggattaccctgaatgttcctggtgacatgtcgtcggcagcgtttttcatggttgccgccagcttagtgccaggttccaaagttaccttgagaaatgttggcatgaacgacaccagaaccggtctatattcaattttgaaacgaatgggcggcaggatcagcctatcaaacgaacaaagtacgggcgaaccgacagcggatttgacggtggaagctgccgagttaaaaccaatcgaaattggggcggatgaaattccagcagtgattgatgagttgccattagtcgcgttactggcagccaaggccaacgggatcagtaaaattactggtgccggggagctgcgggtcaaagaaaccgaccggatttcagccatcgtcactgaattccggaagctgggaattgatattcaagaactcgatgacggcttcatcattgacggcagaaaaccatggcaggttttggattcgaaattagacagtcatggggatcaccggattggcatggtgatggcagtggcagcgctgctggttgatcagccgttaactctcaccggtgcagacagtattaacatttcttatccggagttctttgatgatttggcaactttgattgagaggtgaccgttgatgacaaccgttttgattagtgggctggggctgattggcagttcaattgcccgaattatcaagaatggggatacaactgttgagatcatcggcagtgatcccgatgatgattccgcccagtttttgttggatcatcaaataatcgatcagcgagctgacttcgcccaggcagccacacaagcagacttgattattctggcgggtccggtatcggttattttgaggcagattgatgagttggcccaattaaaattaaaggagcaggtcttggtgacagatgtcggcagtaccaagcaatcgattatgacagaagccaagcgcctgacgcataagggagttgcttttctcggtggccatcccatggctggttcacatttgaccggtagccggaacggctcaattgatttatttaacggttcaaaatacttcctggtaaccagttcacaaaccaaacagcaacttcgcgactttgaacagctgctggattcggcaaatgttgattggacggagataacagcggaaacccatgacaaactggttagcgaactgagccatctgcctcatgtggttgcggcaaccctggttaacagcgtcgcggacggcttggcccatgatccagtgggcttaaaagcggctgccggcggcttcaagagtatgactcgaattgctgcgtcggatccaaaaatgtggacggcgattatgatgagcaattcccaagcgattgcgcaggaattggccacttttcaaaccgcgttaagtcattttgaagaagcgattcaagaccaagacgaagctgcgatttatgccgctttcgccaaagcagaacaaatcagaaagtccttggacgattaaggagaaagcctatgaaactcatattggttggatttatgggaagcggcaaaaccaccgtcggcaacttattggcacagaaactcggcttgccatatcacgatctggatgatgtcatcgtggaaacggccggcaagtcaattaaacaaatatttgccgatgacggagagccggcgtttcggcagctggaacatgatgctttgaaagcgtctttggcagatgatgggatcttgggaaccggtggcggcacgccgattcaagctgccaattttgagctgttaaaggccagtgacgtcccagtcgtgcttctagacgtgatgccggaaacaatcattgcccgattgaagaatgataccgaccggccgctagctcaacagcttggcctgcatgggttggtggatttgaaaggtcaacgggacactttataccaacaggtgagtgattttcgaatcgccaccgatgatttgacgccccttgaagtcgttgacgccattagccaagaggggtttttgaagatgtcgtttgggaggaattaaaatgatcgatggacacacaaaattatttggcttattagcccatccggctgctcacagcttgtcaccgttgattcacaataccagtttccaagtgacagggatcaacgggatctatttggcctttgacgtgacgtctgccgggctcgccgacagcttggcggcgatgcgggcgatgcacattggcggttttaatttatcaatgccgctcaagaccgacgttctgccgttacttgacgaaattaccccgcgagctgagcgcctatctgccgttaatacggtcattaaccgcgatggtcgattgattggtgacagtacggatggtcagggatgggtagatgctctcaagcaggatgatattaccatcgatgaaaaggtcgtgaccgttttaggtgccggtggtgccgggcgggcgattatttccgctgccgttgatgctggtgcaaagcaagtatacgtttttaagcggactaacgatctgtttgatgccagaaaagaacagctggaaggctggtcggatgtcgtcactgtcctgccttatgaggatgaaggtctaattgccgaagcgtttgatgaaagccaaattattgccaatgcgaccaacgttgggatggccggcgatcaatcgctgccagttagtcagtccgtgatgaaccatttgacaccacgacatattgtgtccgacgccatttactttccactcgaaacaccgttcattcatgcagctaagcaacgcgggagtcgtacatataatgggattgggatgctggtgaatcaagcggccggttcttttttggagtggacaggacagcgaatgccgattattccagtgattgaagccgttcatcaggccgtcttacaacggtcgaagaattaaggggctaaatgaccgacaagcattctgttttcggttatacttaatgaagtgtcaaaattaaatattagataacattaggggagccaatcggctgagacggaacatcttcggacccttcgaacctgatctggtttgcgccagcgtagggaagtgttaaaagaagccaaaagcctccttttgttatctaacgaaaggaggctttttatgcaaagaaatacgacttataaaatggtgctaacggcgattctatctgcgatcggcgtggtcggcggcagtatgtttgagttcactgtcggcgttgccaaagtggccccgatgcagcatttgatcaacttgatttccggtgtcctggttggtccatggtgggcagtcacccaggcatttatcacttcattaattcgtaatttattgggaaccggaactatcctggcatttccaggcagtatgatcggtgcgttctgtgtcggctggcttttccagaaaaccaatcgactgattattgcggcatttggtgaattgatcggtactggcatcattggtgcaatcgttgcttatccgattgccagttggatgatgggaaccaccggtgcgatttacctgttcattcccagtttcttcttgagtgccttggtcggtgttatctttggctatatcattctcaagagtatttggaaacggatcattgtaccgcaacaggacaaattggggattggccgcaagactaatcgggattaaacgtttcccggtagtggaatttgccagggatgatatttctgacgtgccaatcccgtgggaacttgacgagggtctcggcgtgcaggactgctgcgtaccccaattcaactttgggcagccaaatgctggtgagcgatggtgtcaggtatgaagcaaattccaggtcatcaaaactgataattttgacgttttttccaggaaccacgtggtgtttggctaagcccttcatcaccccaattgagagtgggtcggaggcgaccagcaggccgtcgagctgattgccatattcattcagcaggtcatcagtggcatccattgattgcttggtagtccagtccgtcaatttcacgattggctgatgatggttgatcgaacaccatgttttataggtgagggtccgtgcgtcatcaatgatacgaccctggctgccgtccaaattcacttcatgacgggaaccgccgataaaaccaattgtttgggcatgcggtgtcatttcgttcaaggctttatccgttagctgagctaaattcgtatcaaccgtatcgacaacgtcatcgacatcactgccgccatcaaccagaacgacgttgggattaaatgatttaatggcgttgatggcggatttggaaagactgccaacaatgatgacggcatcgtaagccgcaaaatcgtttggctcaacgccttcatccaacctgaccacccgcttgatactgatattctgagatttagcagcttcatagacccctctacggacaaaccgccagtactcatcacgcgtttcttctttcagactgagggtagtgatcagcgcaaagttcaactgatttttgtccggtttgggggctagggagtatttataacccagcttatcagcaacttctctcactttgtcgcgcgtttcttttgccacatattcgcttttatccggactcagcgcgcgcgagacggtcccgggtgagacctgcgccagtcgggaaatgtctttgattgtcgccatccatcttcactcctcaattgaattgtattacctctagttaaacacaattaaatgttttaataaatctttggtttgttttaataaaatttattgacaatttaactgtaaacgtttacattctagatagcaattattttttaaaatttatttttatgggggattaatttatggcaagtaataccaacattactactggtcgtagaatcacatctcgattatcgtactcatttggtgcgttcggtcatgatatgttctacgcaacgctgtcgacctactttattatgtttgtcacctctcacttgtttgataaaagtgccggtggacaaaatgatcgaatgatcttttggatcaccacgattatttcactgttacgatttgttgaattagccattgatccatttattggaaacacgattgataataccgaaaccaagtggggccattttaaaccttggatcctcgctggtgggacggttggttccattacattagctattttattcactaacatgggtggtttgaaccaatccaacccattgttgtacctgttaatctttggtgttttgtacatcaccatggatatcttctattcatttaaagacgttggtttctggtcaatgattccagcgatctcatttgattctgcagaacgtgaaaaaacggcgacgtttgcccgggttggttccaacattggtgccaacattgttggggttatcgtaatgccgctggttgtgttcttctcaatcaatgccaaccatggtcaaggtgacctgcgaggctggttcatgtttggtgccatcattggtttgatttcctggctgtcagctgttgttgttgccatgggaaccaaggaaaacgattcattattgcgtaagaatgctgaaaagacccggatgcgtgatgtgttcaaagtgttagcccgtaacgaccagttaatgtggttatcattgacttatggtctgtacacctcaggaattgccattaccaactcacttgaactttactacttcacttatatcatgggtaaaccaggcgaattctctgtgttggcttcattgaacatggtaatcggaattatttcagtgttactgttcccaccgttggcacagaaatacagccgtcggaacgttttcttcctatctattagcattatgatcgtttcaatcatcttattcacatttgccggcacatcattaccactggttctgctcgccgcaattctcttctatattccacaaccactgattttcttggttgttttgatgatcttgagtgattcagttgaatatggccagttaaaatttgggcaccgtgatgaatcattaaccttagctgttcgtccactgcttgataaactaggtggggcactttccaactgggttgttgggattgctgccgttcttgcaggaatgactgctggtgcgactgccagcgacattacaactcatggacaaattattttcaagctgttcatgttcggtattcctgccttactgattttgagtggaaccttcatcttctttaagaaagtaaccttggatgaaaaagaacatgccaagattgttgatgaacttgaaaagacttggaacgagcatttggaaactaacggagaggaatcaatggccgacatcgttaaagaagttgccaaagatacgacctataaagcgccgattagtggaacaatgattgccctttcagatgtgtccgatcaaaactttgcctctgggaacatgggtaaaggatttgccatcaaaccatctgatggtaaggtctttgcaccatttgacggaacggttgaagcaaccttcccaacccgtcatgccatcggacttcgttcagataacggtatcctgacactgattcatattggaatcggcaccgttgaaatgcgtggaaccggatttgttcaatacgttcaaaagggtcagcacgttactgaaggccaagaattgcttgaattctgggacccagcaattaagaaggccggctatgatgacacagttatggtggttatcaataactggaaagatatcaaagacttcaactacacagttgagtccggggatgttaaccacggtgatgatttactgacattgtccaaacctgaagaatcatcagacgatagtgatcagaagtaacgcttaacaaaaactgaaaagggattgataaacgtggcaattagaattgaagatcagaatctgctgtttcatttacagacggaccataccagctatatttttcacgtgatggaaaatggtgaactcggccagatctattatggcaaacgggttcactcaaagccttcatacgataatttggcaactagagagtggcataatgccgccgctgtttggcgacttgaccataaggatgtccagccgcaggttcttaaacaagagtatgccagcttggggaagggtgatttccgttacccagcctaccaagtcgcgcaagcaaatggcagccgcattactgaatttaagtatgagagttacgagttggtggacggtaaacaacgcttggccgggctgccatcggcatttgatgatacggatgacgacgcccagacgttgacgattgcactacgggataaattgttgggattagtgatgcatttgaactacacgatttttccccatcaagatgtcattatccgcagtgcagagttccagaatcagggcaatgaaaagctcaggttaaattcggcagccagcgctcagcttgatttaccagacgccgactacgatttcatccaattctctggtgcctgggcccgcgaacgccatatgattcgaacacatttacgttccggtgttcaaagtgttggcagcctccgcggtacttccagtcatcaacaaaatccctttgtgatgctggcacgtccgaatactgatgatgcacagggttcagtctttggttttaatctgatttattctgggaacttttccgaccaggttcaagttgatcagtatgatgccagccgggttcttgtggggatcaacccagaagaattcgcttggaatctgaagccgggcgacaaattccagactcccgaagccgttctcagttatacggatgccgggatgaaccagttaagccagcaaatgggcgccttctaccaagatcacctggttaacccacgatttgcccacgagcagcggccaacgttgattaataattgggaagctaccttcatggactttgatgaagacaagttattaagcttcgcaaccaccgccaagaagctgggactggaaatgtttgtcctggatgacggctggtttggtcaccgaaacaatgacgacagctcattaggtgattggtttgtcaacgagccgaagttcccgagtgggtttggcacgtttacccaaaagattcatgacttgggattgaagtttggcctgtggtttgagccggaaatgatttcaatcgatagtgaattgtataagcaacatcccgattggttaatcaatgcacccggacgccacgcatctccagagcgccagcagttcgtgctcgatatgactcggtccgaagtcgtcgactatctcttcgatgccatgagcaagatcattgagatgaccaagctggattatatcaaatgggatatgaaccgcaatattaccgagacttacagcagtcagctcagtgctgacgaccaattagaagtgccgcaccgatacattctcggcgtgtaccagctctatgatcgtttggtcaaagcttatccggatgtcctgtttgaatcatgctcgtctggtggcggtcgcttcgacttggggatgatgtactatgctcctcaagcttggaccagtgatgacaccgatgcagttgagcggatgctgattcaatttggcacatcttatggttacccgcaaacgatgatgggcgcccatgtctcagccgtgccaaatgatcaagtcggccggatcacttctttgaagacccgtgccaatgtggcctacttcggtgattttggctatgagctggatatcaccaagatgtctccagaagaacagcagcaggtcaaagaacagactgccttctacaaggaacaccgccaactcttccagtttggaaaattctatcgaatcgataacccatttgccaatggcggtaatgtcatgagctgggaagtcgtcagcgatgatcaacagcacgcaatcgctgcgcgttaccaaattttgaatcgaccaaacaccggttacatccgcttgtatctcaaaggactcgaccctgacaccaagtacacggttaatggtggcagcgaacagttctacggcgatgagttgatgaacgctggattgtttgtaagtgacattctccatgaaacgcacggaactgatcagtcagcggactttaattcaaagctgtttgtgattgatgccgtcaaataatcaattgaataaccaaaaagtgccagctggaaaactgatgatcatcagtttctaactggcacttttatgtttttaaagttattcccaaacatccaacttatgcgacttgaagtaatattccttatcatgatcgttaatcggccgggcgacccgacatggattaccataggcgacgacattatccgggatatctttggtcaccacgctgccggcaccgatgacggtattgctgccaatggtgactcctggtaagatttggacaccggagccgatccagacgttatcttttaaagtgattgggaaattatattggtaactattttgcctcagaatcggcaagaccggatgcccagcagtggtcatcaccacgttggggccgatcatacaatgattgccaatggtgatatcatcatcgtccaccaaggttaagttgaaattgatgtacacatcgctgcctaaatgaaggtggtgagcgccccagttagcgtgcatgggcggttcaatgtagcagttttcgccaacttccgcgcacatttcagccagtaactgactgcgtttgtcagtttctcttggggatgtcatgttaaatgaatacaatttctccaggtattcctgttgtcggtccatcaattccggaacgtccgggtgatacagcagatgtttggcttttcgctcgagattattcatggtggaatccctcctttaatgattcaagcttatcatttttggccatatgacaggggagatgtgtcgaagatatttttgtacagttcggcggttttgaaattcttactttcttattctggtataaaagttgtagtatagaaagagtgacttttataagaaagaggagaatatcttgtctaaacgcgatatcatgattgtgacttgtgcactattgctgtcaaacgcaatgagtggactggacaacacaaccatcaatactgctttaccagcaattatatccgatctccacggaattgaattaatggggtggatcgtcgccgttttcctgttgggaaccgcggtcagtacacctttatggagtaaattgggggaacacattggcaacaagcgcagctaccagttagcagccaccttatttgtggttggctcatttctacaagggatggcgccaaatattgtcttcttgattctcgcccgaaccttgatggggattggcaatgggggaacggtttcgctgccatacattatctatgccagaatgtacaagaatccccgcaaacgaatgcaggtgttgggatttgtttctgctagttatagcatggccacgattatcggcccactagtgggtggttatatcgttgatacatttagttggcactgggtcttttatctgaacgtgccgattggcctgatctcaattgtcttggtccaaatctattataaagtcagtcatgaaacccggcagacccaagcagttgactatcggggagccatcatgatgaccattggattggtcggtttgcttgccggaattgaaatgatcggtaatgccaacttaattttggtactggccgtgattggattttccattattgtcctgattgtcatggggattttggaagaaaacgttgatgatccgattattccaagtcgattgttcaaaaacctgccgttgatgattgactttgttctgttcacattaatctggggagcgtttattgcctttctgatttatagtccaatgtgggcgcaagggttattggcaacctcggccctgattggtggtgccacgcaaattcccggtgcctttaccgattttatcgggtcggaagtcgttgcccccatccggaactttttgtctccgcaacgggtgatcgccatggggatcgttatgttaatgatttcctttatcatcatggtgatctccggggttcaaacgccttactgggtactgttgatcgccggtgcctttgaaggattcggcaacggtgcctgctttaatgaactccaggttaaagtccagcaggatgccaacccgacggatatcccaattgcgacttcgtttagtttcttgattcggatgctcagtcagacattcacggcttcaatctttggaatcattatgaacaatgctttacgtgacggtgtcagtaaggctggcggttcgatttccatgaaaatgatgaacgaattaagcgatgcctccagtagcggttccttgccgctgcacttactgccgcaaatgagattgattttgtataatggtcttcacaacattatgtggctgtcgttgattttgatgattgtttccctgcttattaacatttgggcacagaaattggaacatgataaatttgttaaacgggctgccaaagcatcataaaaagtctccatcaaaaaccaatttgaaaactggttttcgatgaagactttttttattgtgactatttcttagcagtcaatgacgtatctttaaaggttgatagtgaaacatttgcggttgccaagctattgccggtaaccgtttcggccttgaagctgacccgatcgccttcagcgatgaactgcagcaatgggttgaagttcttggcgctggtatcaatcttataaacttgattgttgttcttcaaaatgaacagtaaactgttatccgttcgaacaactcggttgatggttccgctcacggtcttaccggctggaaccgatgctgcaaccccggtctttgcttcgactcgttgttcgaagattgccaaggtgctttgggcatcgtcgccaattgcgtaagtgccgctttggttattaccatcggccaggagataaacgtatttcataaatgagttattatcccgatcaagcatggagacaacccaagtgggatccccattgattcggtacagtaacggtaatgttccgcgataattctggggattgatatcctgttgcgcgtaagagattgcccgctcaggtgtcataacgttaccatgctcacggtagtaatgcagggtgttggtccgtgcatcaacgaaagtatatccaagaatggaactctgatgttcgttgacactggtcataccggtgaagtaatagacacgacctttgtaagcgtaaggcgtcaacttgtcgccgccttcagttccggcggtagttggcttcataacgccactgtggccaccaaagctggtagcgttccagaagccgtgccgataacggccaaacattgagacttcctgactgacaaattcaggggtgaccgcaatatcaacgaacttcggcacctgcttaggtgagtagactttcactttaccggtaatcgtgttcagaacggcgactttatagtgtttaaagtcataattccggttcaagtatgaaattggtttggcaagtgttcgaacatagtaaggcgtgccgttatcgtcaatttccaattgagccgttgcgccaaccattgagtagcccaaactgtgggcactgatccgccggtcggcatcgttattgaaataggcacttggggtgtatttcatcggcttggcgacaaattttggatcggcattcttgtcggtagcgttggttctaaagtaaccaggcacttttaagtaatgaagataacgccagaaaccaccggagaattcgacaggggcaacataaatcatcttgcccttatacatctgaacccgcatgtgattcaaatcataaacgttggagttcttaaaactattcaatgagttattcatatcggtcgaaatcgtttgtggtgcgtttaccacaggcgtttcggcactgttcttgatcacgggcattggcgcgttcttggtatcatcgttcatatccgtttggattgattgaacggctggtcgtggattcatcttggtgaccagggatgtaatgctacctaggatgatgaagacgatcaccgcaagaacggcgaccatggcaattttacccaaccagccaaatgcgccggtgaatcgctgaacaatttggccaacaatcccgtcgccggcttccgttgttcgagcaacagcagcgtgtggtgaatacaggaagcggcggagcgcagcgaccacaatcattccgaagatgaaccacatcaaccatccatcgatcaaagacggatacgcaagatccggcaggttgaagtaggtgttaatgtaactgacgatgaacaatagcacaatggctagcgttccgtacgttcgaccccggcggtctgcgataaccagcagccagataaatggaattaacaaacctgacagcttaaccagggtgatgagtgcaaaataactaagcatgaaatttctcccttcaatactgttaacgagtttgagtattaagactattataccttactcaagaggcaacacctaaccgctttcaaacggttaattcaggtacccgcttgcaccacaggatcacaaatgcgttcgagccgatgtgagttccaaccaccggtccgatctggccaacttgaaaactggctttgggatatttgggcttcagggatgcacaccatttttgaacagctggcaggttattggtgccggtgaccatcacgtgaagcggataagcgacttgctgatactgggtgttgaattcttcatccaagtgcttcagggccttcttcatcgtccgaatctttccaattgcttcgatttgatgctggtcgttcaaagttaatagcggtttaactctcagtaagccacctgcaaatgcggcggcgttggtgagccgcccgccggtaactaagttcttgaggtcatcgacgacaaaatattcatcgatagttgcccggacatcatccagattttggagaattgtgctcattgattcgccttgattggccatcattgaagcgtatttcacaagatatcccaacggttcaatcgtgatgtgtgaatcatagacttcaacctgggcgttggtatagccccggactacagtgcgcagattgttgacaaagcccgtgatgccagcagtcaaatgaatacttagaatttggtcatagccttgattggccagctgatcatacacttttaacatttccatcggtgtcggcggtgcagttgtgggcaactttttggccttcgccagtgcggaatagaattcatcattggtaatatcaattccctcacgataggtggtaccgttcatgttaacgacgatcggaacgacagtcacgttgccaagccgttggacttcttcatcagaaaggctggccgtgctgtcggttacgattgcgattttactcattgtttcatctcccgatcttagtgatgttaaattgattatagcatacactccagcatgccatgccgcatctgagggtacggtaagccaggaaccgtaaagtttgatgaattatgaaaggattctcatcaaaatagcaaatcaatatgagaagattacccagccaccaaaatttcaattgccgatcgttcatcattttactgatcatattgtctatcgctcattaagcaatgcccttaaggattgcgaccgcttacttcaaaagcggtctatgtacacaaatggcgcccaacaatttcttttctaaaatgggtgttgacatctccacgtaatgatgtttaaatgatagcaatttcatttttatcattattttctcacgcaattataattatagaaaaaagcgaggtaatgccaatggatacagaagcaaataagccagttgataaactgacagtcaaagattacgtatacttagtttcagcaggggtttcaaacgccgtcctagtgatgttaggggtcggattattaacccagaccattgccaacttcgtgaattggccacaattacatcaagtcggggcaattgcccaatggttactggcacctgcatttggtgccgctgttgcatctcaattaaaaaccaacacactggtcctgtttagttccatgattgcctcaactgttggtgccaacgccgtttatttcatttcatccggcgttcacgcagcaaccgccactggtaaccagatggcacaagcagccggaaccggtgtcttcacaactggtcaacctattagtgccgttgccgccgggttaatcgctgccttagttggtaagtatttaaccggtaaaacgccacttgatatgatgttagtaccacttgcctcaaccttagttggttcaatcgccggcttgggacttgcaagtgtcaccacgccagcccttaactggttgagtgcttttatcgctcaatcaatgcaggttaacccaatcctcggttcaatggccgttgctttggcatggtcactcttcttgatgacaccggcatcctcagctgcccttgcagttgccgttatgcttgatccactttcatcaggtgccgcactcattggaacgaccgctcaattcgttggcttcacggtcatctcatggcgtcaaaacaaccttggtgccaacattgcccaaggcttcatcacaccaaaggttcagttcccgaacttgttggccaacccacggctcgcaattccttcaatgactgccgctgtggtggccgctccgattgcgacaatgttcttcggcttcaaggtgccttacacattaggcggcctgggattaaactcatttatcgccccacttaacctggcatcaaccaacatgaacatgttcgttgcatacctggcaatgggaatcgttgttccagccgtgatctcaatcgtgctttacagagttcttctcggcatgcactgggttaaggatcaacaactgcatcttgaaattgtttaagctattactacctatattactaatataaaatcaataacaaatagaagccccggagctggattgctctggggcttctattttgttgatcatactgattatgtttagtgaacgattgctgttactttggaaactgaggtagctgtgtaatgctggtaatgagcagcgggatactttggctccccatttatacctgtgattttataaccaatcttgacagtcttccaattcttttcaggtgtaatgaagacccaaatagcttttgacaggtcattgttttccgattttttaacaaatttgtgaaggaaggtatttaaaatatttttttgatttcgctgttatatcgcatatatagaagaaaaaatctaacaaaattcaacatgccgttacccattgaacaaagctattgtaatatattcgtaaagtgctataaccagaaatgggtacgagaaatgttacccaggtaaaacaaattatttggggggattaagaatgaaagccaataagtttgcaaaaacaatgttgttagcgttttccataacgggagttttgctggggggagcggttggtgcacatgcggccactgccggcacaaatagtcaaccgattgctcaaacctcagttgtgtcggctgcacagggggcatggaaaccagtatactcaagtatgcttggtaaaccttataagcataaggtaatcaaatatagtcccactggatggggagatttcgaaggtggagatcgaaaagcttactttagttcagataagcatattcagtatcggtacattaaaaagtcgcgaactatgatttatcggtataacaatcatgataaagcgcttaggtctaagtacaattatcaaaagattgtgctgcgtcatggccataagacacctgaatattcgtactactataagttgggtaagcagaaatgggtttacacagtgacatataagttctggttggtcaaaccggttaaatactaatcaggttagtcgcattcgagattgttggattgtggatgagtattattcacaatcatccattaaatgaaaggtcgatgatgaacttgttaggtaccagacaacatcagattactttaaagcggttgttaatgttagcattcttttctctattggttttagtccctacctcagcgtctgccagtaccaactggaaacacttggatatgaattcattaggaactgccacaaagatgaaagttcttaaatacaattcacttaattggggtgagtattatgatgatcagagtgatttgtttaaagatactaagcatgtgcagtataagtacgccaaacgcacccgaacgctcatcatgcggtatcggaatccccagcagtttcttttaaaaactaagtataattatcggaagctgatttatcgacatggtcataaaaatccaattgtgacccattactttaaagtgggacacgaaaagtggaaatttgcaacgaccattcattattggctaaagaagccaatccgatattagttatcaacggaacctcgaagctgatacttcagggctttcgttgctatgttttacctttcagtatcgttttaattatgtccccaaattgcttaattttaaacaatttggggacataattaaaatagcttgtctttaagaatcggtggcgtagctatttaaatctaacctgacgtgtgaatatccactgatttttaggaaattgggtgataatacaaaagcaccaactatattgaaatagttagcgctcgcctgtgatttaattcaactcagtgagatgcattggcttaagacattaatcaaaaaagccaaaaatatctttaacggcagtcatagcttgtgctaattctgccgcattgacatgatcaacaatcttgccggatccggcgatgtagtcataacccaaaagaccggttaaaataacatggccttctatcttatgagaagaaagtgtaatctgaaaaggtgccttaattttagttgcatgggtaattggaaagccgataatcatacctgtccgttgattatatgctttatcactgacaaccagtaacggtctaaaagtattactgggatctggattatggccaccatattcaaggcctgcatgtggttcactatcaatccagatgagatctccttgctgcgggatgtctttagtcattccaaatatcctctcgtccaaccggcgtgccattgtccccaatgttttcttcttccattgcttttcgaagatcgtagttcgagtctgcactataaatgttgtgtcgaactggtaacaaactgatcacgccgttttcatccttgattggttcaaactcaacgttttcccctatgttaaacgaagcaggaattgtcaccataattgaattgccttgacgccgcgtttttacagtcattattatcaccctttctacacgtaattatatatgtaattacatttaagctcaagcaatttgtattgattaaaattagaacgatctatttgttttgtacgttgaaaacatagactgggaggcttacacttataagcatgcgaagtacatataataggaagaaaagatgaaagtaatcaagagcatcttcagctggatcctgccaatcgcaattggattggcactggcgttactactcaaagcctatattatttcaccagtcagagtggatggtgattcgatgatgcccaacctgcagaacaacgagcacgtggtcattttaaaagccaagcccatcaaacgcttgtcagtggtggtgtttaatgcttacaaattggcaccggatacgcaaccgaacactgaatttgtcaaacgggtcattggcattccgggtgacaggattacctatactaagacggggcatttatatgtgaatggtaagtacatcaagcagccgttcatctcccgtcagcagcagaccactggtactttgagcaacgtcgacgataatggttttaatttatcgattctttccaagaagtggcgcagaggtggacagactgccgtggttcccaggggtcagtattttgtgatgggtgataatcggaatatttcctatgacagccgttactggggatttgtgccaaagtcgcatatggaaggggttgtttatacgttcccgtgggatgccaatcgtcaggaaattaataactatggataaaacaatgtccttcaccagttttagatctggtgaaggacatttttaggttctacaatacctgttcgcaattaaattgtaaccgtaacgttttcagtgatctggcgaatagatggcgttctaaaaaaattctttgagaacgcctgaaatagtttggattggattgaagtcaatatttgaaatatattttaagatccttgaccaagaacccatttgaattacttaccatttaattcacgaacctgatcaattaagccaagaaactcattagctgcctggcggtaatcctcaatcttatccccgtatttctcattaaagccttccaaaccaccggcaacaaatgcatattcataatcatatactttgtcataggctgccgtgaattttgtcagcaggtcgtgatgcttgccatctagttgcaaggccatttgaacgacccgaacatcggtgtagccaagttcaaactgaattgcccacgcccgaatgaagtcgtgctgcgcctcaatgtgggcaaagtggtgctgggtgttccaagttaatctgtctaatgatttaataacgtctaacatgtctgtacctcccctaaagttaacaacatgattcacgttaattgaaccgcgtttggtggggaagggcaagtgatttgactttatcattttaacgataagaattttaaattcaagggcaaaaaaatcctccaaaaataagcccttttcacactttattataaaatatattccgataaaaacattgaaatataatgaaagagtgatattacagatatgtaatctagattacgtatcttatgaaacagggggaattattatgttgttgaagcgttggattaggtttgtatatgtaacggttgcagtaatgggattcgtatttgttgcaggtactatttgtgtaaatgctagcgataatgttaaccagggtacaaatgatgaacaagttggcgcagttgcaactaaagtaggaaatactcaaaaagtaggcattacttctggtacaacgagcgataattctgtggatgaaaataggcagaacagtgccttagcacagcgccctaaggcaactgcaagcaatccttctaataaaaagattgtaacgaaccgtttacagatgactaagcctaagaaagcaaaattacaaaagaataaggcttcaaaaaagtcagttactgtcacaactgcaattccatggtcaaaagctaagaagcttgataaagctgaagcaaggagggaagcaaaagtagcagaaattgataagttgaaggcggaacttaataagctaaaaaaagaacaggccgcgaataataaagtgccagctacaaatcagactactggccaggaaacaaatggaaatgttacaagtaataattcatcgaattctacaagcacacaaagtacacaggacaccagtggatctggtcagtcagcggcaacctcacagcagacagatcagttaacgccgtctcagcaagctgatcaagacgcccaggatgcgaatacgcagttacagccatcgttgacaagagcccagattacctattatcaaaccgcgtccgtatctaatgttgttggtcagggtgtatcaattgtgaatgcaattgcagaagtaatatctgcattacgtagtttaatataataaacaagatttagggggatatcgatgacattatgaacaaggtaaaatttaacaatacacgctgcttaagaatgttgttgatggtactattggtaccgacattgggtatgctagttactgagagcggggtacatgctgatcaaagcatgtctgattctcaaacagcaagttctaatgagaataataataataacaataataacagcaacaataataatggaggaataattatccctggcgggggctcaattaataatggaaggaatagtggaggaatcgtaaatactggatctacgattggatctggaacagtaagtaataatccttctaccttaaatacaccaagtagtcagcaagttgttaattcgaactcgaaccgtagcaacgttaattctggattaacgaatggaaacggttctagtattgcttctcaaaattctaatcagcctcttaacggatctggaatgagtggatagccaggggagggtggattaacacctaatgaccatgtccctcctgtagctcatttaagcaagcctaaagttattagagatgggcatgccaagtatcaatggaggcgtgtatactcaacgactaaaaaagaaaaaggcacgattgatgtatcgagaaaagtgtctaatggtatgactggatcagtcggaatgagtaaaaaggccattggcatgaagttaggatttaatgtgtcaaagtcaacgacagtcaccgtccatattccctataagacaagtggaaaaggtcgagaagtcgttgaatatacagtcaggaaaattcgatacaaaataactaggactaagactataaccactgggataaatggctatgtaacttcacggaagaagttagtcgcttatgtttataaatacgatggtattattggacgagttgtaaaggattaaaggagctaagcgaaatgaaatatcttcaaacttctgcagtgtttctcagttttggactgctaacagttttcttcatgcaaattattcaagaaatttcagatacattcacgataggtggcgggcccactgatgcgccaatcaactactgggcaagcagcatgatccttgttccattagcctttggagctttgttcattatcacgttcgcattgggcatgtaccaaatttatcaagagaaaaaacaaagtaaaaagtgaagaaacacaaacaagcacccttggagaattgagtctccgagggtgcttgtcattttttaagcgattatttaatcaattgtggttgaaacacacccattactgtatcctgagcagtaaataccggaacttggtgactgagggcattggcgaccaattgtttttgatcgacggtttcgtcctctgaactcagagcaaaggcgaggttgcttggccattccattccttcgtggtaggtttgaatgccaaagccgctgccctttagttgctcgactaagctggcgttgttggcatcaaatgctgacaggagcacatcaccagtcaggtgattggtatcaatgtggtagctgtcaaacagcgcattgtgtaaggcttcctgcaggttgtggccggcgccgatatcttcgccggttgacttcatttctggactcaacgcggttggggcacctggcagtttggcaaatgagaagactggcgccttcacataaaccttggctggttctgggtgtaagcccggcttcaaaccaatttcagctagtgatttgcccaaaatgagctgagttgccaattgtgccaaatgtagtttgacaatcttactcatgaacggcacggttctggatgcccgtgggttgacttcgatgacgtacacttcgtcagcgacgatgaattgaatgttcatcatgccaaccgcatgaacctgcttaccaatcttggtagcgatagcaacgatcttttctttctggtcgtcagtcaacgtctgtggtggatacatggcaatcgagtcgcctgaatgaatgccggcaccttcgagatgctccatgattccaggaacaaagacgtcattgccgtcgctcaggatatcaacttcacactcagttccagggatgtactgatcgattaagattggttcaccatgactgttcttgagcgccgggatgaggtattcgtttagctcgtcatcattatggacaacggccatccctttaccaccaagaacgaagcttggacgtaccaataccgggtaacccaggtggttggcaatttctaatgcttcaggggcatcggtagcggtagcaccctttggatgagcaatgttttggtcaattaagaggtcttcaaattgatgacgatcttcagtttgctcaatgccgtggagggaagtgccaaggatggaaacgccatgcttagtcaagccttcggtcaagttgatggcggtttgaccaccaaattcaacgatgaccccaatcggctgttccaaattgatgatgttcatgacgctgtcaatggtgagcggttcaaagtaaagcttgtcggaaatggagaaatcagttgaaaccgtttctggattattgttaataataatggcattgtaacccgctgcttgaatcgctttgacacagtggacagtggcgtagtcaaattcaactccttggccaattcggattgggccggcaccgataacgacgatactattccccagtggcttgctttcgttttcgttaccaactgtactatagtagtaaggcgttgtgctttcgaattctgcggcacaggtatcgaccatcttataaaccagatgttgatctgacattttgtctaatttggtcaactcatcatcggttgcgtgatgaatggcttggatcatggtgttgttgaagcctaatttacgggcttttaagacttcatcagcgcttaagaggccatcggtcatctgctgttgcatcttgatgatgttttccagtttcgataagaagtacatatcgatttgagttgaacgattaatctgttgaatggtagcacccttaccaatggcggcaaagatttcaaataatcgataatcagttggtgtcttaatcttttccagcaggtcgcccattgacatgtttcgagtataagccggaatcaggtcagtttgcgcttgttggtcgagttccaatgattgaacggcctttaacagtgattcttcaatggtactgccgattgccatgacttctccggtggctttcatttgggttcccagtttgcggtctgcgtttgtgaatttgtcaaacgcaaagcgtgggatcttagcaacgacgtaatcgagagccggttcgaacatcgcaaacgtggtttgcgttattgggttcatgatttcgtccaggttcaaaccaatggcgattttggctgcaattttggcgattgggtagccagttgcttttgaggccaaagcggatgaacggctgacccgtgggttgacttcgatgacgtagtaagcttcactgtttggatcttgggccaattgaacgttgcacccgccttcgattttgagggcgttcacgatggtcaacgacgcgtcacgcagacgttgatattctttgtcggtcagtgtctgcgttggtgcaaagacaattgaatcaccagtgtggataccgactggatcgaagttttccattccagtcacgatgattgaactgccgtggtgatcccgcatcacttcaaattcgatttctttgaagccagcgatactcttttcaactaaacattcagttgagggtgacatggtgaggccacggttcaaaatggtggtcatttcatcatcgttatgggcaattccgccgcctgttccacccaaagtataggcaggacgaataatgacaggatagtcgatcttgtgagcgaagtccaatccatcttggaggtcgtaaaccgttttggaatcaggaattggctggtgaagctcttccatcaagtctttgaatttctcacgatcttcagcttcgttgatggtttgcaaactggttcctaacaattcgattcccagttcatccaggataccgtccttgctaagttcaactgcgaggttcagaccggtttggccgcccaaagttggcaagatagcgtctggatgttctttgttgataatcttcttcaggcttggaacggttaatggctccaagtagaccttgtcagcaatttcatcatcagtcatgattgtggcagggttggagttgaccaagattactgagtaaccttcttcacggaggctgaggcaggcttggctgccggcatagtcaaattctgcggcttggccaatcacgattggacctgagccgataatcaatacttttttaatatcttctctttttggcattaatgaacccctccgtttacgtgcatcatttcgataaagtcgtcaaataatttggtggcatcgtgtggacctggtgcggcttctgggtggtattgaactgagaataccgggcggccgggatagcgcaggccctcacacgttttgtcgttgacttcaagcgcagttacttccagtggggtgtctttaacggagtcgacgtccactgcgtaaccatggttttgtgaggtgatgcaaatgtcaccagtgatcaggttcttaaccggatgattaatcccacgatgaccaaacgtcattttgtaagtggtggcgccgttggccagtgccagaagttgatggccgagacagattccaaacagcgggaagttgtcctggagcttttgaatcaccggcacaaagtctgagtaatcggttggatctccaggaccattggataacaagatgccggttggatgtaagttggcaatatcttcaaacgttgattcaggtgtaacgacggtcacatcaacgcctgggcgctggagtgacttgacgatgttatctttgacaccaaagtcaacaacgacaacatgttcaacatctttggcgtcgcctgcggacaatgtggctgatttgataatggatgccgagcggtcagcttttggttgatcaacgattgggtgattggtaaggctggccttcattgtgccatagcggcgaataatcttggttaactgtcgggtatcaatcccgctgattgctggaaccttcgactgctttaggaaagcatcgaggctgataacgctttggtaatgaaatacttgatcggtcatttctttgacaacgactgctgctgcttgaacggtgtccgattggttggtgcccagtgagatgccatagttaccaatcaacggataggtgaaactgatgatttgatgtttgtacgatggatcggtcaatgtttcctggtagccggtcatgctggtggtaaagacgagttcaccatcaatttcggcgcccaagtcaccacacgcttccccgacgaagacatcgccgttttctagagttagatactttttcatgtccgaacctcctcaatttgttcctaacaatgctgcggtatttacagttaacgcttttgaatatttaagatagaagtatttagggcaaatgtcaagggaaaatatgcaatatttgccgatattcggataaatatgtacaaataaaatacaatatgtatatttattaaatatgtcccaatgtcttgaaatcgcgtccttatagataagttagtcgtcactttttaatatattcgatttgttggataaataaacattttcaaaattaatttaacaactagacttgttttttctctcaaaatagaatatgattctaagtaatcaaacagaacctttaacattaaccccgtgaggttaagaaggtatggcgaatcttgaggagactcagggctaactcaaacctctttaccgaacgcggtaaagaggttttttgttacatatctactaattcttattgacgatttaactgttcccgtgagagcaaaacgtcctggaatgtggttcccgacacataaggagcgctttgcgaacacggcaaggcgcttttaattttaggaggaaatcacaatgatgcagattactaaaccggtaagttttgaaaatgttgtaagtatggaagacctttcagccgaagatgttttatcatttatccatgaagcacaggatttcaaagccggcaagcagattgagctaaagcggccggtatacgccgctaaccttttctttgaaagcagcacaagaacccacaccagttttgaaatggcagaacgcaaattaggccttcaagttgtcaactttgatccttcaaacagttctttgagcaagggtgaatcaatgagtgacactgttaagaccttccaagcaattggcgttgacttggttgccatccgtgataagaagaatgaatactacaaagatttaattgctgatccaaacgtccatgtcggtattgccaacggtggtgacggctcaggtcaacatccatcacaatcattgcttgacatgatgactatatatgaagagtttggtcacttcgaaggtttgaaagttgccattgttggtgacttaacccactcgcgagttgcccgttccaacatggaagtcttaaccatgcttggcgcccacgtctactttggcggaccaaagaagtggtacaccgaagaatttgccaagtatggcgaatggatgccaatcgatgatttggttgaagaaatggacgttatgatgttcctccgtgttcaacacgaacgaattgctgacgacgaaaatggcgccttctccgctgaaaagtaccatgctcaatatggtttaactgcagaacgtgaatcaagaatgccacaacattcaatcatcatgcatccagctcccgttaaccgcggtgttgaaattgccgacgaattggttgaatgcgacaaatcccgcatctttgaacaaatgcacaatggtgtgtttgtcagaatggcaatcatgaccagcatgcttcgcaaccgtgacctcattaaggaagaatattaatagcgaggagaatttcgactgatgaaacgcatcattgcaaacggacaaatactggatcgtggccaattagttaaacgcgatattttaattgagaatggtagggtagctaagattgctgaagacatttcaactgatggagtggatgaagtaatcgatgccaaagggaactttgtctcggccggcctaatcgacgtccacgtccattatcgccagccgggtcaggaacaaaaagagaccgttaagactggcagtctggcagctgctcatggtggcttcaccactgtttgtgcgatgcccaatgtcaccccggcacctgactcagttaataatatggaagctttaattaaattgaaccacactgacggtgctgttcacattaagcaatatgcggcaattaccaccaaccgtggtggtgatgagttagttgatttcaaggcgttaaaggatgccggtgcctttgcttttagcaacgacggcaatggcattcaaaagagcagtaccatgtatgaagcgatgcagcaggctgccaagctggacatggccattgttgaacacgttcaagacgacgctttgacatatggcggtgttttgaacggcggggctgctaaacgtctgggaatgaaagaaatgccctgggtcagtgaaacagcccaagttgcccgagatgtcattcttgccgaagcaaccggcgttcattatcatgtctgccacgcatcatccaaacataccgtcaacgttatccgggctgccaaacaagctgggattaacgttaccgcggaagtttcaccgcaccatctgcttttgtcggacgccaacattaaagaagacaacgcgatgtacaaaatgaatccacctttgcgcggagaggatgatcgccaagcattgatcgaaggcttgcttgatggcaccattgatatgattgccaccgatcacgcccctcataccaaggcggataaggatcaatcaatcgccacagctgcctttggtattaccggcagtgagacagcattcagtatgctatacaccagatttgtgaagaccggtcggttcacgttagcccagttggttaattggctgaccaagcagccggcatccgtcttcaaaatgagaggcgctggctcactggcagtcggccagcctgctgacattgccatctttgatttgaaacacgaacatgaaatcaaagaaagcgactatttgtcaaaaggcaagaattcaccatttactggcgaagctgtctatggcgatacggtcatgaccttggttgatggcgacattgcctacaagagatcgtaaattaatcacataaaaacatattggtatcaataagaataaaaagctgcagttcaccgagactcctaactcgatggactgcagcttttgtattatttgagaaacatcgtgtaatagccgattgctgaaaccgcttgggcggtgttgactttaccttcgcggatccaatcgacgatttgttgaagtggcactaattcactgttgacgaactcgtcttgatcaaagtggcgttccacgcgttcgctgggatcaaatttaatcaacatcaggtcggcaaattggtccatgaagccttccgaagaggtgattcgggtcatcttagtgactgactgggccacgtagccggtttcttcccgtaattcgcgggcagccgcctgttcgctggtttcgcctgggttcacaatgccagctggcaaggaaaccgaatcactgttaacgccagcccggtattcactgctcatcacgacttgatcagccggtgaaattgccaggatggtgatggtcgggtcggttttaatcagatcgcgctcaattttgagaccgtccggtgtctggatgtgtagttgatcgacggcaaagacgcgaccagtgtagatgtttttctggtcgaggatcttgccggggtggtgccatgttttaaacaaacaattatctccttttgatgacttttctttcatatcggtcaggaaggctgatgtgaaaagccgattcattacagcaattattttatcatcatttagacgcccatcaaggctgaaggagcactcaactggtcatcttaatcccaacaatgcttaccagcagcagaatcacaaaaccccaagtaatcggggaaatcttgtcgccaaacaggataatgccggcgatcactgttccgacggcaccaatccccgtccataccggatacgcaatgctcagcggtaatgttttggtggcatgtgctaacaggaagaaactgatcagcatgccgacaatggtgacaatcgatggcatcaagttggtaaacccgtggctatatttcatcgccgttgcccaaactacctcaaagatgcctgcaataatcaaaaatacccaattcataaaaatcctcctaaagaaaaagggtacccctcacaattccttctatgacctaacggaattgtaaaaagtacctaaagttgctgcccggtggcagtcgaatatcaagttgttattagtgtagcacatttgaaatcgaaagggaatttacttctttatgccaaacttctcttccaatgctttcgttagtaactgggaaaagtttaggtttgattcaattcctttttcattcaaataatttggaatgttgacggttttcttgacaggatgggaatcatgttggcgacgataagcactgatattcacatctaccaaagtggccaattcatttggcttagtgtctggaagactataaactgattttggcacagaacctccgtcttcaatcagatctaatacttttagaccaataaaatctcggcccatttcaatggagttttcaatggatgtaccttgtgtatatccgcctaaatttggaatactaacaatatacggaaccgatttatcgttgggatcttttataataatgattggatagactactttgacatctttcataatgacctccaaatattgatttaacgtaattgatgtttccttattagatctcgagcaagccattcattaatatttggatgccgtggaataacttccttttctttaccgtttgtccaaatatcatgatttccaccatggcgatataaataccaaccatgccgttcgaagagctgcaacaaacgcttccgcttcatcgaagataatcctcaactttctgtatattttatacgtgcattgtacgtagatcaagtaatttgtatttcctcaaagcacttttttgaaggtgacaaatttgatgacttacataattaattacgtataaatgcaagaaaggattttaaaacaaaaaatggatgacatccgccatccacaaaatgcaacgattcaactacttctgcagcactcgtaccctaaacaccgcgtcaatctttgaaagacggtcaaccaattggtgttcttcctcgttgttcaagttatccaaatcaacgattgtgtaggcaacgtcttttctggccgcgttactcatactttcaatgttaattcccgcgtctgccaacaaggtcgcaatttggccgaccatgttcgggatgtttttatggatcaacgttaagcgataaggggtgttaaacggcacttggaggttgggcaggttcaccgaattttcaatgtttccagtctccaaatacgtcatgattgtgttggcgccttgagtggcgccgttggcttcagcttcgagtgtcgatccgccgatatgtggagtgaccaccacatcgtctcggttcaacaggatattttcaccaaagtcggtatagtatgtccgaattttgcgggcgtccagatagtccacggccgcctcgttgtcgacgattccgtcgcgggaatagttaaataatttgacgccatccttcataatggccatttgttcagcgccgatcagtccggtcgtctcctcattcttaggaacgtgaacggtgacgtaatcagcttgctggagcgcttctcccaacgtggttgcccgggtgatggttgtcgaaatgtgccaagcggcatcggctgatagatatgggtcatagccaattaccttcatgcctaaggcgctggcggcattggcaaccaaggagccgacgtggccaaccccgatcactgccaaggttcggccggtcaattcggttcctttgaacttggtcttgtctttttcagttcgcagcgaaatgtccgcgccactattgtgggcagcgtaatcggctgcagcaaataagtttcgcgatgaggccaccaataacgcgataatcagttctttaacggcgttggcattgctgccgggggtgttgaagactgcggttccgttggcagtggccttgtctaacgggatgttattaaacccggcaccggctctggcaatgaccttcaatttcttgggaaattcctgatcatgaaggttaaccgatcgaatcagataggcatcggcgtcatcggttttgttaatttggtagttgtcggagaagcggtctaatccagcctgtgcaattgcattgtaagtttttacttgatacatatgagttctccctaatgttgtttttcaaagttgtgtaagaaatcaaccagtgcctggacgcctgccagcggcatcgcgttatacagacttgctcgcagaccaccaacacttcggtgacccttgagattcatcaaaccggcttccgtggctgctgtaatcgcctgggtatctagatcggcatcaccagtggtaaatggaatgttggtcaacgaacggtcagaggccttgatgtggttggcaaataattttgagtcgtctaagaagtcgtaaagcagggatgctttttgccggtttaccttctcaattcctgcaattccgccctgatccttcagccatttcaataccaatccggtggcataaatgttgaaaacgggtggggtgttatacatcgagttctttttgacgaataaattgtaattgagaatgcttggaatatggtcgactggctgaaccaaatcatctcggacgatgaccagggtaacgcctgcggggccgaggttcttttggacgccaccgaagattaagccaaagtcattgacgttgtactgttctgccatgaaattggaagataaatcaccaaccaaggtgacatcgccgtgttcaggcagctgatgataagccgttccctcaatggtgttgttcgttgtgatgtgtaaataatcatagtcattggcggagattcgctggttcagttgtggcagtgcttgataatgctgatttttggttgaagccaacacatcaacttggtagccgaggttggctgcttcatcaccagcccgggtagcccaatggccactatccagtaaggcaatcttcttatgcttggttgccagattcattggaacggcggcaaattgacccgtgccacccccttgaaagaagaggatgtgatagttatcaggaacgtccatcaagtctctgacatcctgttctgctgcattgataatgtcgtcaaacattttggaacgatgggaaatttccataatactcattccactgccgttgattgaaggcagttcagcttgaatctgtttgataaccggatcaggaagcgttgccggacccgccgcaaaattgtataccgtcatgaccaaaaactcctttatataaaattaaaaagctcccacaggtttgctgtgagagcttctaactgacgtttttagcggtctcacagtgatgaaaaagatttcatctatgcaaggccctttgttgaatcgcacgtatcaaaagatggcctacatagatgtgactgtagaccaggaggatgatgtagttgtcgttaaatcagctaattgcatgttcatgtgaacaacctccatttcttataactaaaatctaacagaactcacagataaaagcaacacccattttgaagaaagtgtcacggaactgtttgcatgtgcttgaagatcatggtaaattcaatggataattaatttattgggaggaacgcgcatgactgatttttactttgttcgccatggccagacggctgccaacgccgccggattaaagcagggcaccattaactcggaaattacctacctatcggaaaccggaaagcaacaggtggaaagtttgcggaaaggtttcgatatttcgtttgcggatagaatcattgccagcccactgcagcgggcaaaagacacggcggccatcttaaatcagagcgcgaacttaccggtaacctatgacaaccgactcctcgaaatttcatacggcgactgggatggtgagaagaacactgatttgatgagcaaatatcccgaattttttgacttcaccctaaacgacgttcttcctgcgtatgccgatgtggcacatggtgaaactttcgatcacgtcatcgatcgcgtcgctgaattgatgcaggaaactgcaactaattatcctaatgacaagattatcctggtcactcacgggtttacgattaaagcggctgtgttggcagccatcggtcgtcccaaggacatgatggtgattgaggagccggataacaccagtgtgacccggatcactttgcagaccacaactcactcgtattatctgcggtattacaaccgggttgtcaattctcagttttaaagtgattgacaaatgaaagtcaattggttatattaaatggcatcaagtaacgaaagaggaggaagccattcatgcaaatgtcagctgctaatatgatgtgttgttcaatgtgtcaagctcaacttagcgctgatcgtggcttctttggtaaacgattggatttttgggacaagctgtgagctgatagttgacggcccattttctcaagaattaccaatgccaagagtgtctcatttcagcgtcaaagctggagtggggcattctttttgtataccagaggatctcttttgttgaataaataatcttaaaggtggcggttgcagtgtgtagtcagatgttgattgaagtgaaaaggacaaactaaattctttggaggaatcattcatgcgaaaactcagatcacttttattattagccttgagcgccattctggtagtgactttggcggcttgtggcaaaaccgcaaccaaatccaacagccaaaaacagacactgaatctcagcacgacggccccgttggatacgatcgacatttcaaaatccaccgggtatggccagaccgggaacgtgtttgaaagcttttatcgcttggggaaagacggcaaaccaactgctggcttggctaagagcggtaaggtttccaaagatggtaagacgtggacctttaccttgcgcaacgctaaatggagcaatggcgacccaatcactgcccaggattttgtctactcgtggcgccgaaccctgaaaccaagcaccaaatcgacttacgcctatttattcagcggaattaaaaacgccgatcaggttaacgccggcaagctctcaccaaataaaatcggtatcaaagcactgaataacaagacggttcaaattcaacttgagaagccaatcgcctactttaaggtcctgatggcctatccattatttggaccgcaaaaccagaaaattgttgataaatacggcaaaaaatatggtaccaactccaagtacatggtgtactccggaccattcaaaattcaaaactggaacggcaccggcaataagtggcagtttgttaagaataaccgttactgggataaacaggccgttaagcttcacaagattaactataccgtggtcagcagcccgacgactggccttgagttgtatcagcaaaacaagctggatttgacgccgctttctaatgaacaagtcaaacattacaaaggcaacaaggaatttcagcagtatccatattcattcatcggttacttgaagtacaacttcaaagacgctaaccaaaccaaacgcaaagccatgagcaacaaggacattcgtctcgcaatttcactggccattgatcgccaacagctgaccaaaaaggttcttggtgatgggtcagacacaccaactggctttgtggcctctggattggctaagaatccgaagactggcgaagactttgccaaagaacagactgttccaaatacggtggattacaacgtcaagttagccaagcagcattggcaaaaaggtttgaaagcccttggtaccaagaaggttaccctgacaatcactgcttccaacgatgatccaaccagcaacccgattacacagtacatgaagtctgaattgcaacgggacttgcctggatttaagctcgatattcgaaatgtgccgagccaagttgccaatcaagaagtcttaaagggtgactttgacctgtcattatccggttggggtgcagatttcaacgatccaatttccttcctgcagatcccggaaaccggcaccgcatacaacagcggcaagtacagcaacccggcatatgataagctgattaaacaagctcaaaatcaggatgccaataacgctgataaacgctggaatgatttggttaaggcagctaaattgtttaatgctgatcaggggatgacgccactgtaccagcaagtcacctcgtatctgcaaaagcccgacttaaagggtgttattcataacactgccggtactcaatggagttacaagtacgcttatatgaagtaaatgaccgagactcaactgccttgcgtcgaacgattgtcatctcattaacttaaattaaaatgagaatccattgaccattgagagcgatatcatggtacacttttctcaactaaaacttttgaggtgattaaggatgacaagaaaaattggtgttatcggaatgggccacgttggctcaacagcagcgcattacattgtcgcaaacggcttcgcggatgatttggtattgatcgatatcaatgaagataaagtgaaggctgacgcaattgattttgaagatgcaatgtccaacctgcccgtccacaccaacattactgtgaatgattattctgcactgcaggatgccgatgtcattatttctgcattgggaaatatcaaacttcaggacaatccgaatgacgatcggtttgccgagctgccattcaccagcaaggcagtcaaatcggtggcacaaaagattaaagactccggcttcaatgggatcattgtcgccattaccaatccggtagatgtcatcacttcgatttaccagcaaattaccggtctaccgaagaaacacgtgattggcactgggactttgctggattcctcacgaatgaagcgggcggtggctgacgaacttaatttagatccacggtcagttaccggatttaatttgggcgaacatgggaactcccaattcactgcttggtcaacagttcgggtactgagtcatccaattactgagattgctaaagaacgcggtctggaccttgatgcgctggacaaagctgccagagaaggtgggttcaacgtcttccacggtaaaaagtacaccaactatggtgtcgccaccgcggctgttcgtttagccaacacggtgatgagcgatgcccatactgaactggcagtttccaactaccgtgaagagctcggcacctacttgtcatatccagcggttgttggtcgtgatggaattattgaacaggttcaactgcagttgactgacgatgaaaagaagaagctgcagatttcagcttattatattaagacgaagtttaaggaatctatggaaaactagaacagattgggactaaaggcgctttgatcccagaatataacgcaatcgggccgtcattccggaatttggaatgatggcccgattgcgttatatggccgggatcagccgtttgtaccaagttttatcaatataaaattggtgattgcagttgcaataaaaatcaccgtaacaactagtggtccaatctctgtttcgggacaaaaaaataacctccagcaattaagaactgaaggcttgaagcaatttatctaactcgaattgttaatatacttacattataacgcgacgaattcgacttgtcaacgttgcctgcaaaagatattcgagtttgactgggtggcagattcagcctaaaattgagccaataaatcacgattggagcaatcaattttggcaaactacgaaacagtgtttcatccagacggttacaattctcctgagtaccgcagcttaaattattcctatcagaataaaatggctgaattattctcccaccgacggattgattatccggccaaagaacttcaatttgaaattgaaaccgtcaaaatctccagcaccatgactcagcagcaatacctcaaacttcagagcttggtggaatcatttcccgaaactcaacgcagtggggatgcccccgtcattggcaaggacgattaccagagtattattttgtatcatgactaccgattatttgattcgacccagtatgttgtccgcagtccgctgggatttggctataccgtcagcaagttgatcacgattacgagtgagccggcgggaggtcctcatcaccaggtgaaggtgactttggcaattaacccgaatcgcttcgttggtgttcccgaagaacctttgcttcgtctggtcatcgaagaggtgttgccgctgatggtgatcccacagatttctgaaatggatttaacattggatatgccgctaatcatgaacaactttcatgttcagatgggtggccaagctgggacaaaacagcagattacccaacggcttaatgatcatcaagaatatgaattgagccgaattgcctatgtggatcctcagcagaccagaaaactggtcgtggcagacaagtttcaatccctgttggacaatcaattgctggtggcggatactgactacatctctgcccgggaggccgaatactatcgggaccaagttggagaacggcagtttttaacccggattgaattggcggtcaccacccctaatgccgtcatgcggtacatgaagaatcacgagtggctgatgcgggacatttccatcgagtatcgtgataatagcggcatctcaagatttgcgggtaccgattacgcgaccaacgggaaggacttccgccgctcatttaaccggatgctgacgtatcggctgaaggaagttcagccaagagcacgcaaactgccatatctgactgatgcgatttggcagaataccttgaaataaaatttgaataaatctcattaaatgaaaattcactgttgaactgacatctcaaagtggtatgctgttaccattaaaaatttttgaggtgattgaatgacaagaaaaattggtgttattggaatgggaagtgtgggctctacggtcgctcactatatcgtgtccggcggctttgcagacgacttggtactgatcgatgtaaatgagaaaaaggttaaagccgacgccttagacttcgaagatgccatggccaacttaccgaatcatacgaacattgccgtgaacgattatgatgaattggccgacgccgatattgtgatttctgcgattggcaaactccagctgcagcgcgacaatcccagcaatgatcgcttcattgagtatccatatactcaaaaagcagccgcatcagttgccggtaagatcaaggattcaggctttaatgggattttaattgtgattaccaacccggttgacgcgatcacgtcaatttatcaggcggtcactggtttgcccaagaagcatgtcattggaaccgggacgctgttggattcgtcacggatgaaacgggctgttgccaagaaattacatatcgatccgcgttccgttgccggttataatttgggagaacatgggaattctcagttcaccgcttggtcaaccgtgcgggtcttaggcaaaccaattactgaattagctgacaaagaaggccttgatcttgataaaattgatgaagatgcccgaatgggtggcttcgtcgttttccgtggtaaaggatacaccaactacgcgattgccagtgctgccgttcgcctggccaacgttgtgttaaatgatgcgcgaactgaactgccggtatccaattatcgtgaagaactcggttcatatttgtcatacccagccattgttggtcgggatggcattatccaacaactccaacttgacttaacagatgaagaattagcgaaactgcaaaattgtgccaatatcattaaagagaagttcgaagaatcaaaagccaaggactttgcgactgaatagggacttttcacatagaacaattttcatccacattcatatttgaggatcgtcacgcctcatagtaatggccaggtcaaaatcagcaacttttgacctggctttttgtatcccaggaggtcactggattaccaattcatgatttttagcgctcttttacatgtttctcccacttttggtatatattaagattaatcgagggggaaaaatgatgaaaaaagaacgggtggaagcttttacggatgccgttttggcaattattttgacgattatgattttggagttcaagaccccggaatcgtttgcgattagtgccattttagatcaagtgccatacctgatttcctacgcaattgggtatttgttcatcggcgttgcttggtacaatcaccattacatgttcgccaagaccaattggatcacgcaaaatgtgtattgggcgaacaacttgtggatgtttaccacgtcctttgtccctgtggcgacggcttgggtcgggcgcgggttaaatgaacaggggccggaaatcttttacttcattgtctttttagcatggtcgagtgcttactattacctgtccaaccgattaatcaaggccaacgaaaaagaccactgaccgaaggcagcggaggcgattcgatcaatggtcatctatcgatatatgagcaactggaagttagtggccgctcaacttattttgtcaattgccgttttgaaattcatgccggcgcttcaaatggtcattgtcacgttaatgattatttttatcggtgcccggtttaacgcggacagcgatcggctctttcgctagtgggcaatcagggtgtagatgaagtagccgagaaagccgacgcacaagctgagcgagccaaaaatcatgatctgaacagaacagacaaaagtcttggttttaatttgttcatggttgaaaatcagggactgcttgatgatcagcggaactgccagcagaatggagaacagtgctaatgggaagacgccgacgtacatggcgtaaaataccaggaggacagctaaaacgttggcggtattaaacattaacagggaattcttcttgccgatatagtggacgatcgtccaacggtggttgacctcgtcttcttgatcatcgcaaatgttattggctaacataatgttggcaatccagaagaacaacggtgacgaagccagcagaatctggccaagcagtgaggcattccaagtgaagagctgataggaattcacgtagaccgagatcagggtaatcatgacccccatagcgaagccggacgccacttcaccatacggcgtgctggagatgggatgcggtccggatgaatacataattccgatggcaaaacagatcaatcccatccacaacagcggcaggccgattttgaataccaggaagatgccaatcaaagctgatggcacaaccataatgacgatcataaaacgaatgaggtttaaagagatgtggtcccgaccgatgatgttggtaccggttttccattcctcagcggttgaatgcatgtagtcgttatagttgtccaaggtgtccacggtcatattgaacagaatcatggcaatgaaaaaaagcgtagcgtaaagcccattcaccgagtcgagcaggtaccagctgaaaaacagtccggtaaaaaacggaaagatgctggcagctttggctcgcaactcgacgagctgggaaaaagttgataaactcatgatgacctccaagataaatttaaaataatttcaaaaacatagtctaattataccaaaggagcgggaaaatgacgctgacgaacaaaacgccggaaacaaaagttgaatcattatttgatcaaattgctgacaactatgatgggatgaactcgctgattagtttggggaatcataagcactggcgaaaattggttatgcagcagctcaacgttgaaccggggagctttgcgattgatgtttgctgcgggaccggggattggacaattgctttggccaaggcagtcgggccctccggacaagttgttggcctcgactttagtgaagagatgctgaaacttgctgacaagaaggttcgtgcagccggcctgcaggatcgggtaaccttggttaaaggggatgcgatgcagctgccatatgatgacaaccactttgacgtcgccacgattggctttggtctcagaaatgttccggatgctgaccaggtactccatgaaatgagccgggtggtgcacgcccgggggcaggttgcctgcctggaaacatccaagccaaccaatccggttatcaaattcggctggcgggtctactttgatttggtcccattaatggcaaaagtggccgtcgataaatatcaggagtacgcctatttacaaaaaaccactgccgaatttgtctcggcacaacagttggtggaaatgtttcaaaacgccggcctggttgacgttcactatcgaccattcactttcggggccgctgcttttcactggggaatgaagccctgacaaaatttcccttgattcacaagattaaaaacgttatcatgtgtttaacatattctaaggagtttttaattatgatagataatttaaacatccaaatgaatagttgccgatattacttttggtttttccgagtgtgatctgtggataagccaaaagcatttcgtaatgcatactaaaggccgcacagatcactgagttgactgtgcgggatgataccattggtgggtcctcacagtcagttcgttgactttgaggacccactttttaggaggagaacacaatgagtaaattatcagataagatgaacaaacgggtagctgcgttaacgcccgccgcaattttgactttcaaccagaagatttcagcgattccagacatcgtcaaattaaccttgggtgagcctgatttcaacactccggaacacgttaagcaggccgctattaaggcaattgacgataacgaaagtcactacaccaactcccgggggacagaaggactccgtcaggcagctgcgaacttcttgaacacgaaatacggtctgaattacgatcctgacaaacaagttatcatgactgaaggggcaactggtgccatctactcggcattgactgccatgatcaaccctggcgacaccgtgatcgtcccaacaccaattttcccactttacgtgccgatcttaatgctggccggtgccaaaccaatttttgtggacacctcggataatggctttgtgctgtcaccggaaaaattgtctgcagcgattgaggctaataaagatactgttaaggcggtgatcctcaatttccctaacaacccaaccggggttacctaccacaaagacgatttacagaaattggcggacgtcatttccaagcacgacattatttgtttaagtgatgaaatttacagtgagttgacctacgacggcacccatgtttcgatggggtcgatcctgccggaacaaacccttgtcatgaacggtgtttccaagtctcacgccatgactggctggagagtcgggatgatctgcgggcctaaagatatcatcaatgaaatcgccaaggtcagtgaatttacgatcacgtcactgaccaccaacgcccaggctgccgccgaagaagccttcaagaacggcatggacgatgccctgccaatgaagaaggagtacatgacgcgccgcgacttactagttgctggtttggaaaaagccggcttcagctgtcctaatcccaatggcgccttctacgttttcgccaagattccagctggtttaaatcaaaacagtgaggcattctgctatgacttggccaaggaagccaaagttgccttaattccaggctcgtacttcctgccaggcggcgaaggctacgttcgaatcagttacgcagccagtgaggaaaatattcaagaggccgttagccgcattcaaaaatacgttgataaacagtcagtcaaataaagggagcttgagttattttgaaaattttaatgtacaacgtccgaccagacgaacaaaaaccactggatggctgggttaagcaaaacggtgtccaggtagataccaactcggtaccgttaaacgctgacacggttgaccttgccaaaggttacgatggcattgtgattcagcagcacggatcagtctcagatccgacaatttacgagaaactccattcatttgggatcaagcagattaccttgcggatcaccgggtatgaaatcattgatttggaccaggctaagcaaaacgacttggtcgttactaacgtgccggcttactcaccacggtctgtgagcgaactggtcctggccgatgtcatgagcctgcttcgacacatcggtgaggtaggcgaacgcgaaaagcacggcgacttcagttggaagggtgtcgaagcacgtgaaattcatactttaacggttggcattatcggtgccggcaaaatcggcagcgcggttgcccggatttttagagcgctgggtgctacggtgattgccgccgacccgattcatcgaccagaactcaacgacacgttgacatacgttgatcacgaaacggtcttcaaaacggctgatatcgtgaccatgcacaccccattgactgacgagaccaaccagatgattaacgccgacgtcttcaagcagatgaagccgtccgcgatttttatcaatgcttcccggggccaagtggtggataccggcgccttggtgaacgccttggaaaaccaggaaatttccgccgccgcaattgatacctttgaaggcgagaatacgattgtcggccaagacttatccggcaagcagattgaaaacgataatttaaagaagttactggcaatgcctaacgtcaacgtgacgccacacattggtttctataccgaagtggcagtccaaaatatggttgagattgccttgaatgacgttgtgatgattttgaaagggcaaaagagccctcatgaggtaggcgaatagatgaatttaccagcagaaccatcagcacggctgaacggtcgtgaactcattatgaatacgttaaacgggctgtcggttgggatcattgttgcattggtccccggcgccttgcttaatcaattgttgaaggctttgctgccagtgtttccacaagctgctttcttcttgactttgactggaatggcggccgttttaatggcaccgattagtgcggtctgtgtcgggatgatggcgggctttggctttgccggcttgatcggaccaatcgctgcagttaatggttatggcaatgccaatctgatgaatattgtcttggttagcttacttttctttgtgattccgattacgcttggatatgttagcaattacttattcaactccaagctgagttattttgacgcccaagattttgagttggattatttataaggagtcgagaatttgggaactgaatttgccgtgctagtcctattaatctttgttggcggtgcgatttactactattacttcagtaaacaagagccttcaatgattgtggggtatcggacaaaacaaagccgcagcacaactgcaaagtggcgggcctcacagaagtggttctaccaaggggcaatcacttgtgccgcggttgttgtggtggttaatctagtaacgccattttcgattggtgtgaatttggttgttttgttagtttatttatttgtgattagttatttcatcgagcgtcgcttgcgtgagatgggagattagaatgaaaaaggcccgctgagttggcgggcttttttgtgttttagttatttgtttgttggggttagtggttttagttggggggatttgttgttttggtgattcctgtttatctagcggaaacgtgctccgatgaccctgacccctaacatgcaaaacaaggattgtatcgatgaacaaaatgcgttcatcaatacaatccttgctttacataccggggtcaacccgggtctcgtcgcactctaaatttggccccaagcatccgccgcaatcgttgggaacaatgtgaccaatcgttccagctgtgcgggttcgaatttgaacacaattgccggcaataatgcgttaatggcatcttctgcctggtcgctgatttcagtggcaccaaccaaatggttctgcttgtcataaaccagtgtgttatcgccaatttcttccttggtcacttgacggtaccagtcgtctggtaaatggttttcctttgttgtgaagccttcttttttggcatcctcaactgatacgccgactttggcaattcttggtgaggtaaagacgactgatggaattgccgggtaatcgatgggatccgtcgtgtcgccagcgaaagtatgcatcaagtaggtcgactcaaaaatcgccgttggggtgagctttggttgatccttgtcgatgacgtcgcctgaagcatagatgttatcaacattggtttggagatgatcgttgaccttaatacctttttcgctgtaatcaacaccaactttatccagtccaatgtcgtccacattaggcatccggccagtcgcgtccaagatccagttggtctttatttgaccgcccttatagttgacgataaagttatggtcgtcctgctcgaagttggcaacttcagtattattgacaaaatctacgccacgagatttcaaatcggcaacaatttgcttaacgtatggttgatagaatttccgcaaaactttgtcaccgtgggtaatcacagttaccttggcaccagccgcgttggcaatcgttgcgaattccagactgatgtagccggcaccgataattgtgatgttggctggcaggtgagtgaggttcatgaagtcagcactatcgtgagccagttctgttccaggaatgtccaaacgatgtggatgttggccggttgagatgacgatgttttcagcggttttggcttcaccgtcgaccattaccgtatgagcatcttggaatgtgccgtgacccttgataatgtcgatgttgacggatttcatcaagccgccgatcatgtccggcaagccttcgatgacttcttgcttatgtttttcattggcggtccagttaattgccaaactgccattgagaatcccctgaagtctctcagtttgacgtgtcaacgccactggtgcatccaacgtaatcttggcgttacagccacggttgggacaggtgccgccaattaagccggattcgatgacgccgactttcttgccgcgggcggccagcggaatcgcaccgtcaaaggttccatgtccactaccgatgtataagacgtcataatcataatttgccataaaaaatgcctcccatatagtctgctcggaaacgattacatcttgaactactaaaagcgtaacctgtaaacaaattgcgtgcaacgaattggtttgaaaatttacgcacagtcaaaaatgtctatgtacgacatcgaccaaaatggctatacttgaagcaaataaagggagctgatgatatgcgcagaaaagatcgggaagtcacagatattgacgaaattaagcaaattttgcaggattcccatgtgattcacagcggttttcggacggctgattatccttacgtggtccccactaattttggctacgaatttgacgatgataaccatttgacgttatacattcacggtgcaccggtgggccgcaagcgtgaattgattaaggaagacggtcggatgggctttgagattgatgatggcggccagttaatggtgcccaaagatcccaagcaaaacaccccgagcttcgcttatcgcagcgtgatgggctatggggatgccgaattggttgatgatccagcggtcaaaaagcacgccctgcaagttgtcttggcacacgagactgggcagcagttgggtgagtttactgtttcagataagacgatcgcctacgttggtatcatcaagatcactgttaaagaattcaccgccaaagcccacggtggcgatgatccggattttgaataggaatacgacgaggctggtagcagtgggggataaaataatagcagaacactaaaaagccggagcacaactaacaagtagttatgttccggttatttattctttacggtgatcgtgtttttgagcctcatgtttccaaaaccatccgggaattgaaatcaagacacccatcccaaatggaatcaagctgtaaatcaatgccgcagtggaatgatcaccactccaccacatgaagtagcatatcccaaggatggagacgatcaaacccgccaagggcactgtgattatgaggtattgaatcattcggtcgcgaagctgctgcatactcatttggattaccttcttttaatcttagattaacactaaccagtcacaaagcaagttacgaagtccgggtcaaataatgattccgggtgacgatgtaatcaattacacctgcgatcaaaagcgtgaccagacaacagccaacaaatcccatcagtgtaaaatcgccgttaatttgaattggtgtaaaagggctgttttcatggaacagtttggaatagagcagcaccgcgttttgtttgaagtcaaatgatcctaatacagggatgccggaaaagtacccaaacatcaaaatacctgccagccaaggtcgcttgagcaataaggtgaggtagtagctgacgatcacagcaatcaatgataagccaaataccgataagaactgcaacggggcttgtgccagataagattggccgtccgcgagataccgtatcaacgccagtttatttgggatgtggataaaattgttaaagcccaactggaagatgaacgaggtcagacaaatgaagatcaggctcaaaaaagtgagcatgctcaaactaatcagtttggagaggacgacattttgaatgctgttcatgctggccttgattttgacctgattatttttgagctcccgataggcaaaagaaattgtgtagatcaccatggtaattggaaagacaatgaacattgacgaccccagaatatgatcaaagctgttcctgggggccatctcgaccagatcctgcttgaccttttctccagcatctttgaggtctgtgaccacttcggctttttccccgttgctaaacgtgattggccctccggctaatatctgatcaacgtcaaccccagcgcgtttatcacgctgctggatccaaatcagactactggcgtcatttttgtaagcagtgtactgcgcccaagatattgagaaacagagaattgtcaaaacaaataacactaaatagatcgcatcagaatggagctgttgatccagttctttttgggttagggatctgagctttttcaattgtgcacgtcaattcctttcggtgaatgatgaatgcggtaagcaatacccttagcataggcattttggccagtgaagacaacggcaaaccggaaatgttcagacttatttcacacaaaattcacaaaaaattcaataatttaccaatggcatatacattcagcaactttcgttctatcataatggtaacggttccagaactagcaattatgaaagaaggatcttgtatgttctttattgatacgtctagaaatggcaaacctgtctatgatccgattgtgaaccaatctttggataactacttagtaaatgatttgaagttgccgggccacggcctgattatgtacgttaaccaacccgctgtgattgtcggggttaaccaaaatgcctacgctgaagtcaacatgccctatttgaaagaaaagggcattaaattggttcgccggacatctggtggcggcgccgtgtatcacgattacggcaacattatttttgaaaatattgtgattaatgatgaccaacattttggcgatttcaaatacttcgcccaaccaatcatcgatgccctgcatgacatgggcgctaccgatgctgaaatgcgtgggagaaatgatatggtgatcggaaatcaaaagttctccgggatgacaatgttcaaggttggcaagtcctacgctgccggcggcaccctgatgtttgatttggatatggatgtggccactgaagttttaacccctgaaaaggataaattggaatccaagggcgttaagtcggttgaaagccgggtaaccaacgttaagccattcttgaagccagaatttcaaaagttggatattgaaggcttcaagaaggccctgctgttgagattgtttaatgccaagtcattggacgatattgaaacatatcacttgaacgatcacgattggtcaattatcgatgagcgtttgaaagggaaatacgataccgacgagtggaactatgggaagaatcccggctttgattactatgtttccaagcattatgatatcggcacggtcagcttcaactattcattgaacggcaaccaaatttccgatatcaagatctatggtgactttattaccggcggcgatatttccgtgattgaaaaggcactgaaaggcgttgatctcagcaaggatgcgttagttgatgctttgaatcaagtggatattaaggctaatttgggtgacatttctgccgcggagttggcggacttgctgctggagaagacgcggattaattagatatcggctttgttttggagttctagttttgagctagggctcttttttattgatttgatcgttgttggaacgacttgttaccgacatatgtcagcctgcaagctaatccgttgaccttacccggccattcgtggaataatataacgtcataagtaatgcgacaagttaccgggggtgaacacatgaatcaagcaccaaatcagcatgacgacagcggggaacagaacggtgtgagcatgatggggatgttcaaattcgtttttggtacggttctcaaacggccgtggattttgattgtcaacgttgtcgttttgaccattctgtcattgatggactttttattgccacaattcaatcagtacatcattgaccacgttattccaaataaaagtacggcgcagctggccgtggtcgtcggtctgctactgttgacagttacgatttcagggatttttacctacgtttctacctactacatgggcgtcatgagccaaggggccatcaccaacctgcgaaatcagctatatcaatatttgatcaggttggatacccacttttttgaatccagcaaaacaggtgacttgatggtgcgattaacgtccgatattaacaacctgcaaaacctgatttcaccaaatatgttgtctctgattggcagcctgttcacgtttgtcggggtgctcggcttcattttcttcgttaactgggaaatggctttggcagtcagcctgacatttccaatgattttcgtggtggttcgcattttcagaacccgaattcgaaattcatatcaaaaggcccgtcagtctcaagctttgatgaccaatcaattgcagaacacactgactcaaatccagttgattaagagctacaccactgaagatctggaatccagtcgtttcgacaaattagccaacatgaacaaaaataacatcattgaggctactcggaatcaggcgatcttttcgccgttggtgaccttcattgagtatctggggaccgcgattgtcttattcttgggaacattgtttgtttttaaaaatcagttaaccgttgggcaattggtcgcctatctcagttatgttggtatcctgcaaagcccaatcagtgccttttccagattgttgaaccaattccagcagtcactggtttcttatggccgaattgttagtatcatgggcttgaagccggcgatcgttgacgaggacgatgcagtgggattcccacagattaagtctggagttcaatttaagcatgtcactttttcatacgcatctgatgagcccaagtcaccacacaaagctgcgattcagaatgtgaccttcgatattccgtttggtaaacaaaccgccttggttggtcactcgggagccggcaaatcaacgattaccgatttgctcgatcgattgtacgatgtcgatagcggtgacattttgttcgatggcattccaatcaaacatatcaagctcaagtcactgcggcaaaacatcgcgattgtgtcacaggatatattcatcattgacggcacgattgctgataatatccgttatgggacgcctggtgcaactgaggatcagctgtgggacgtcgccaaattagccgatattgatgcctttattaaaggattgcctgagcaaatgaagacccaagtcggtgagcggggaatccgtttatccggtggtcagaagcagcggatcgccattgccagggccctgctgaaggatgcccagattgttgttctagatgaagccactgcttcgctggataatgagtcggaaaagaccatccagcatgccttggaaaacctgatggagcaacggacctcactggttatcgcccatagattgtcgaccatccacaacgccgatcaaattttggtggtggataacggcaagattgttgagcggggaacccatgatcagttgatgaatgagaatgggtattataagcagttgtatgaggcgcagtttgaataagagcgcgacgagggctgggtggcccggtttccaagaggactttgcttgaagcccccggttttggggcttcaagcaaagtcctcttggaagttagggtcaagcccgtcggagcgtgttttaaaggccgaagggagcacacaagaagctaataaacgtgctttgggttcagacccgggagtcgcagtttctaaagaagcccccgaccagcatagacgctgagtcgggggcttcttgaatacaatagcgaaagtaatggaccggtcaaagctttagcgtgtggttgaacccttctttcagattttaacgatatcctgaaaaggatacaatgtcgagaacatgctcatttatgctagacagttgtgagcataaaaaaagaaaaccccgcttcagttttaaaactgactcgggtttttcgtgactccaataacaaaagcaatagacgagctaaagccttagcgaacggtcgaaccgtcctttccttgctaataatatataagaatttcagcctcttgtcaaacattcatcaactattaattagtttggaaaatagttgataaaacttaattagtacaggctcatgagtataataatttgcatgcttgctagcccttttcagtaatttttgcccttcttttctggttaattcctgtgaccctacacttgaaaatcgtctatgtaaggaatacaagctaacgaggtcatttactttcatatcggttactaaagatgcatcaattcccatcttcgttgcaaacatgacaaccgttgtatttcgatgttttactttttcttcagcggaaaacagattaaccataatggcattattatgtgctgatgcatttcgaatatgctttgcatacttcaacaatatatgtgcaagcttaacatctttgtttctggagcggtgatagtaaaagtctacaaacctggaaaggacaccaaatgttgcgacttccaaaaacatccagatggaggggtgatttcggtgctttacatacatatcgtgcaagtaatcatttcgctttaagtatttcatagtttgatcataacctcgctgattaaatgtactgaagtccttcaccactgaatagccatcttcttctggatccttggttataagatcaattatccgagttttaattccatgttcaatgtccaatgagatcccaagtaagtatcgccgaagttgcatatcgatcgacgccaagtcggttaaatatgcaaaatctaaattttcatatttaccatcaatctgatgaaaattctttcgataggatgtcaacttgaaataataatttttagtcgccagcatttggattgcatcaggctctgatactaattcgaatctaattcccttgcccttcatgtgtttgatcatttgtagatatgtgtactttggttttatttagttcacctcccagcttattgaaattgtctgatcagcctgtcctactatgtatatacgataaattgagcgaggatatctatatagtttgtgaagtattggggcgatttagtgatcaaatcccaaaccagttttgttttcggacattttagtttacactaatcataaatacagaaaacgggtgacaatcaatgaagacaatttatgattacaaagaaaccgaaatgagcggtaagacgattgacttgagcgaattcaaaaataaagtcgttgtgattgtgaatactgccagcaagtgtggcctggcgcctcagttggagggcctggaagaattatataagaaatataagaatgagggcttggtcgtgttaggactgccttccaatcaattccaccaagagttgggaagtgatcaagaggccgatgattattgccggattcattatggtgtcaccttcccgatgactcgacgggttgccgttaatggggatggtgaggatccactgtttacccatcttaaagaagagtccggtcatggcaagattaaatggaactacactaaattcctggttggcaaagacggcaccctgattcatcgatatgcgccaattaccaagccggagtccatggaagaggctatttatacggccctcaatcaaaaaaatgtcttgtaagaaggtggaaagttgaatacgacctatttcaaagccaccattcgagagattacttatgcgtgggggaagtttatttcgatcgtcctaatcattttgttgggatcactgctgtatgtcgggattcgggcgactggtccggatttggacaattccgccgatcagtatttcgctcatcaaaatctcggggatttgacggtgacgtcaaccttgggattaaacaaccgagatctcaacttgattcgcgccgaccccaaggttcagactgccgaacccagccatatggtgacggtgaagaaatcgccgaatcaagtggtccaggtgtattcctatgccaaatcggcaaaattaaatcaactcaaattggcatctgggcatttaccccagaaagccgatcagattgtcttggaccaaaaagctaaggactacaagatcggcgaccgttaccgtttgccggcaaccgatggactcaccactaaaacttttaaagtggtcggattcgtcaactcaccgttatttgtcagttcaaccgaccgcggcaccaccaatgttggcagcggccaggtgaattattttgcctatgcgccggccgcggcctttaaccagaaagcgtacgcggccattgccgtgcgctttaacaacacggctcatttaacggctgggaccagcaagtacaaccagcaggtggatcacgataaagccaggctggaaagcaaactcaagcaacgcccagctcaacggcgggcagagatgattgccccgcagctaaagaagattgaccagcaacttgctcaacttcagaaacagcgccggaagctggcggctgtgccaagtgcctatcaaacagcaaccaccaaagcagccgctgccaaagttgctgccggcgtcaaacaactgacccaggccaaacggcaattacaaaagacgccccaagcgacttatctgtacaacgaccgaaccgccaacgtcggctaccaggattattttgatgagtccaaaagtatcgcggccatcgccgtcatttttccgggcttcttcttatttattgccgttttgatcacctttacgaccatttccagaatgattgaaaagaaccgccgagaaatcggtctcatgcgggcgctgggctacaccaaggacttcatttctatgaaatatgtcatttattcaattcttgcgggaattctgggatcaattgccggcggcgttttgggaaccttgaccctgcccaaatttattttcagcatgctcagcaataacaacctgactcactacgtcggcgtgattccctgggcatttatcatcgaggcgctcgtggccgggttgatcgccacccttggcagcgcggcagtggttctaatcattaatttacgtgaaaaaccgaccgagctgatgcgcgagcgggctcccaaagccggtaaacggattcttctcgagcgaatcaaaccgctgtggaaccggatgaatttcaaccaaaaggtcagttatcggaatctgttcagatataagacgcggatgattatgactatcgtcgggattgcaggttgtacaggcctgatgctggctggatttggcattcgggacagcgtcaacgatctgattcccgatcagttcaatcaagttcagcactaccaggggattgtcacgctgtccgatgctgataaacaggtgcatgatccaaacatcaaagcacagactgcggcgatggttcaatcgattaccgtctcaccaaccaaaggcaccaagcgaaatgcgacggtcaccatggtggcccccaagacaccgacgaaattgaacgattatgtttcattgaccagcactcaaaccggtcagtctgaaaaattaactaatcagggtgtcatcatcaccgaaaaattggccactgatatgcacgcaaaaaaaggcagcctgctttcagccaagctgggcaataagctgctgaaagttaaggttgccggggttaccaagaattacgcgggccattatctgtacatgacccccaagtatttcaatcaagtttcaacgacgacctattcatcgacttcacgcctgttgaagctcaagagtgagagtgccagccaacgacagaagacctcacggaacctgctgaaacaaagcggcgttatgaatgtgacttatccaaggtacgccagcagttcactgggcaccgttggtttaagctcagtcgtgctgatttttatcgctctgtcggctgcattaggactggtcgtgttatacaacctgaccaatgtcaacatctccgagcggatgcgtgaattgtcgacgatcaaggtattgggcttttacgataatgaggtcacggcctacgttgccagagaaaatgttgtgctgaccctggcagggatcgtctttggctggggcatcgggttaatcctccatcattttattatgatcaaggctcagaccggagcgattttgtttccgctgaccgttcattatccagggtacatctggtcagcggtcttaacggcctgcttcagcttagcagttggcgtgattacccattacaaactcaaacatattgatatgttggattccctggcagcttcggaatgatggatgccagtgtctaaataatgtccacacacaaactgccacaaaggtttttgcttttgtggcagtttttggtgttccagtaccaacctcagtttcaaatggatgttcagcagttaacccggttatgacgcacgtccccataaaaatttgaccaacaacttatcaacctgcgggttatcgtggagcttgctgtgctgcgcctgtgggccgacgattcgcttttcctggtaggatttgacttgtggtaccagatacctcaatgatttcgaggaggcattgctgacgtcgccgtccgagtgggtgccgtcgtttttgtcgccataaatattgagaatttcaagtgttttcaattgcttgtcgtggcgcaatcccagcaactcacggtaatgaccgttgatttttgttggctcaccatccgccttcaatttcatccggttgggggcatcatccattcccaggatgccgttgaaatgcccggcgatgtcgacttgcttctcgagcttgggcagcttggtgttgccggcgttgtccagtaaataaaagacgattgccatgttgccaacggaatggccgaccatgttcatcttcttaatgccgtagcgttgttgcagcttaacgaccacatttttcgcccattttccctgggtatgatagttggggtttcgtgaattcaaatagttcacttcaacgatcgggtggaagtcatctggtttgaaagtcccaaccaaggtgactttgccgctatttgaaacgtctgcgcgaatgaccgacttggtaacgccggttttgaccgctgcgttagccatgtgcgtttcagcgtggtaactgctgccgaagccgtggaaaaatagggttggggttgcctggctggcaccctgaattttgggtgtgcctgtggctgatgtggtgcaggcgctgagtaagccaattagtaggaataagccactcagtaaggccaaacgtcgtttcttcattgtttgcctccgttattgggaaagattctttttgccaatcattataagcggattgccgccaatgagaagcaactagcagtttgtctttccgcatttttgtgagattttgacaaaaaattcggaattcattctgaagaatgtgaacgatccccgttatcattacaaatgaagcatgaaagccatttacttttgttaaacggaaggctaatataggttgtgaactaattttacgaaatcttaatattcattcatttctgagggggaattgcatgaagttgactaggaccctggcttgttgtgggctttttttggcgttgacgatgattttctttgccgacccaagcactgcacaagccaagtttcatatttatcaccagcgctcgtccgccctgcacaagggatcgctgcgcaatctgaataacaaaaaggttcattatgtcaaagtgccaaagaagtattaccacgttgccaacactgatgttgagcacacgattaaatccgaacgcggcaagaaggtcagctttcatacccgttacattttgccgctgcctggtaagaacggccagcattggggaaatccacaatcgattgcgatgaatggtaaggggtatatgtacattgtctactgcccaactgatctacataacaaggggcgaattgttcgatttaacatcaagaagctggatgcgatgggcattcggctgcatccaaaagaactgcgggatgcttatcacaagcggcatggcaaatactccaagacccaacagaaaattcacaagtatattaaggcagggccgatatttaccactggtcatggtcaatccttggcatataactggaagaaccacggtttatatatgtggcgggatgtcgaaaaggcgcctcgggttccgatcaataattggggctatatccaacacatcaaggcttcgacgttgcggccggacttcgcgatccgctttcatctgcacagccacggaacatcggtacccggtggccacgatctaacctttgaccactccggtaacgcctacttctggtcatttcctggctggggcgcctacattttcaaaggcaaaattcaccacaaatcggttcactttcgattgacccatcaagtgctgaaacatttgccggggacccgaattcaaagcatgggctataacccggttcgaaagcgcctgttgatgctgtctgatgcatcgattgccagtttccctgcgaaacggctggatggccacggccatttgaccaacggcagctttgagtggacccagtttggccccaagcgtgaatttgagggaatcgcctatgatggcagttcccgaggcaatctattagtgaaccattgtccggaagttctacaggccgatcgatcgtattagtttttatccgaaattgaaaaaattgactagtattttcacaattgagcggtacacttatgttatatcaatataactaaatatctggaggggtatgtatgaaattgggaaagttatcggtggggatcgccacagcgattctattgagtacgtcgttggtgggcacggttgatgcagcgacatatgtgcaaaaaagtaacgccatcagccaatattcaggcgccagcttacgcattttgaataatagcaaagtccagtttgtcaaagccaacgggaactatggctggtcaaggaaccccagcggtagtgagaccatcaagagtgtccatggtacaaaatggacattgaagaccaaatatctcctcccaagtacgcatatggcattggggaaatccagtcgtgatttgaccaatcctcaagctgctgcgtttggcgggaaatatctgttcgtgctgtatgcaccgcaccaatttcatgggaagggctttgtggtcagatataaccgcagtaccctggatcatatgagtttggccaaggctcaagattctctgcttaaaaagactgccggtatgaaagttggcccaatgtttgatgtcggtcacggccaatcgctggcttacaataagaagcagcattcaatttggatgtggcgggatcgggctgacatgaagccgactgcctggtcaaccattcaacgaatcagcatgtcgtcgctgaagccaaatcgtgccattaagttccacatgaataaccgtggtgcaatggtgccggccggccatgacctaacgtttgacaactcaggtaacgcttattggtgggggatttccggcggccacgttaaaatttacaagggcaagctgggcagccgttcgattcatgttcgtttagccaagcagctgttgagaaagcagaccggaactcaccagcaatctatggggtataatccgcacaacggccgactgtacctggtttccgatgactcaattcaaaccctgccggctcgtaaattaaacggccgtggcagtttgcgtccaagtgacatcaaatacactcgctttaattctcaccgcgagtttgaaagcatgatttttgactcgaccgggcacgccatgctgctatcgaaccgtaatccggaactattacgttcaacaaccagatattaataccattaaaatccgtcagatcaaggctgctgccttggtgacggattttttgaggctttatgttgacacggtgtcaccgatggggtatactcagttcataaattgatgacacggtgtcatacgcaaaggagaacaattatggtatcaacaacctttaccaatctaagtgatgagaagcagaccaaaattcgaaaagccttactcaaggaatttacagatcaaccactggcaaccgctcaagttgccccgatcgtcaagactgctgggattgcccggggggccttttataagtattttgatgatctaaccgacgcttacaaatatttatacggcgtggcgatgcgcgatattcacagtgatgtgaacaacgaggtgggaactgaatttgacccgcagttttatttggatcaagtcgaggcgttcatcaaaggtgctcgcgatagtcagtatctgggattgatcaagatgcacctaatgaaaaatgaatcactgatttcgcaaggatcaattgaccccaacacggttagttcccgggaatgggcgacgatgatcctcagtcatgaggccattaagcaaatcatgattgagccgcaaaatgaatcagtagtcatgaaaaagttttctgaaacattgaacttgttagccgggaaggggaatgcataatgtatttggcactaaaagaaattcgacacgaaaagttgaggtatggcctaattattgccatggtggccttgattgcatacttaatttttatcctgacgggtttggcattcggattggctggggaaaacactcaggcgatcaattcctgggatgccaagagcgtggtcttgaataaggattccaatattaatctgtctcagtcgacgattaccaatgcccaagccaaggacgacaaactatcggataaggaatcagtgattggatcgacgccggtggttgccaaacacaaaggtcaagaaaagatttctgcccaatttgtcggcatcaagaagagtgagttcatctataaggggttgaaaatttctgcaggacataaggcccgcaacaaccatcaagtggtggttgatgaaaagttcaagaccgatggctacaaactcggggacaaggtgacgttgaactctgtgagtgacaaatatgaaattgtcgggttcactaagaacgctaagttaaacattgccccagtgatttatggtagtctgccaacgtggaaacatttgcgggggatggaccgggttccgattgccggcagtgcgattgtgtcaaagaatgctaagtacagtgctcacaatagccagttgaagacgtattcgatgaacgaattcattaataagttgcccggctattctgcgcaaaacacgacttttggtttcatgatcggctttttgatgattatttcattagtgatcattgccgtgttcctgtacattttgaccatgcaggctctgccaacctacgcagtattgcgggcccaggggattccagcgagagctttggtgacgacaattaccagccagtcattgatcttgatggcctcgggaattatcatcggtggcctcttggcggctctgacgggatcgttaattccggtcggtgtgccgatggcatttgatattccggtgctcacctggatttccattggcttgatgattatgggcgtcattggtgcggcaattccggcgcaaaagatcgcaaccgttgaccctgtcagtgttattggaggttagttatgtcagtgattgaattaaaaaacattaataagtactttggatccggtattagcaaggtccacgttttgaaggatgtcaattttgcggctgatcggggacagttgatcctagtggttggtccctctggatcagggaaaagtaccttcttgaccattgcgggtggcctgcagacgccatcctccggttcagtggaagttgaaggtcaagcagttgagtcactcacaaaagcgcagcgagatcagctgcggttaaatcaaatcggctttgtccttcaatcatataatctggtgccgtacctgaaagtcaaagaacaatttgagtttgtggataaaatcaagcatgagggtaatttagatcagaaagaattagcagatttgcttgatcagctgggcatttctcagttggtcaaccagttccccggcgaactgtctgggggccaaactcaaagagtggcgattgccagagcactgtatgccaatccggatattgtgttggccgatgaaccaacagctgcccttgatagtgaaaaggttgccgaggtcggccgactgttcaaaaatctcgcagaaaccaggaataaggcggtggtcgtggtcacccatgatctccggttgctggattttgcggataagacttatgagattttggatgggaagattagtcttaaggataaggagcatgtcacggatcggtaaactacatgttatagctcaaagaatacctgctttatacctatcattttcgttgactaccagccggaaaatgtggcaaaaaggacgctacagtaaaagcaaataatcataaaaaagtgaacccctgcctgggttccctttttcatatttggtgattgccaactaccgggtttgtccaatgaccttttggtaggagaacaattgacaacaaaatagcatggtagttaccaaagaagttaagacttttgagcgacgttggtcaaagtaaccgtactaaaactagtgagtcgattgccattatgaatcgcaactcgccacgtttgcaagtgcccgccggcatgcaacggggtggcggttgccaccagcttgccatcaaaaaccggcagcaaatgctgagtagtgatgtcgacgcccactgcgtaatggctgttatccaatcgttcgttggcaccgattgaagccgccgtttcggccaacaccgagttgatgccgccgtgaagaattccgtatggctgtttgaccgaatcggtaacttctagtgatataataacctcagcttggctgacagagacagttttgataccaagcaattcaattaagttagacaaagtattcacactccaattttgaaaggatcgagattatgacttcagttaaatgggaatcggtaaaagattaccaggaaattatttttgaacgggccgataaaatcgcaaagattacgatgaaccggccggaaaaaatgaatgcttttacaccactgaccatccaggagatgattgatgcattcaatatctgtcgtgatgatagcacaatcggcgtgattatcctaaccggcgctggcgacaaagccttttcttctggcggtgatcagggggttcgggggaatggcggctatgttggttcagaccacattgcccggctaaatgtgctggatcttcagcatttaattcgaatcatccccaaacccgtgattgccatggttaaaggttggtcagttggcggcggcaacattcttcagctggtatgtgatttgacgattgcagctgacaacgctcaatttgggcagacaggcccgaaagtcggcagctttgatgctggctacggatccggttatttggcccgggtgattggccataaacgagccaaagaagtctggttcttaaaccatttctacagtgcacaagaggcttatgaaatgaactggatcaataaagtggtcccactttcagaggttgagtcggccacattggattggtgtaacgaaattctccagaaatcgccaaccgcgcttcgattcatcaaggcagccatgaatgctgataccgatggtttggctggccttcagcagttgggtggggatgccacgatgctcttttacaccactgatgagggcaaagagggccgggacgccttcaatcaaaaacgacagcctgattttgatcaatttcctaagtttccataggaaggttgatgaaagtggataattggattttaaagcaggcggaaactgcccctggtcggctcgcggtcgatgacggcaacacccagctaacgtttctggaactcaagcagcaggtttctcaactggctggacaattgaaggctgcctccgtgttggatggcgatcgagttgggattatgaccaagaattctttactaggctatctgatggccatggcggtcttaggatccggtaagacaatcgtttggattaattggcgtttgtctgatgatgaaatccatcgccaattatcagatagtgaaccagcggcctgtctggtggcggatgatctttttcgagaaagttttgaccaacggtttattacctttagcacgataactgatcaagcggcggttcagatcacattagttcccgaatttcgctctcaagaggtggccagcattatgtatacgtctgggacgactggtagacccaaaggtgtgatgcagacctttggcaatcacctcgcctcagcaaccgcctcagcttttaaccttggggtcatgccgggtgacgagtggctttgctccgtcccaatttttcatatcagcggtttttcgattatgatgcgtggcttgatatatggaatggcagtccgcttggtcggccacttcaatgctgaattgattgactacgtattgaaacatgaacccatttcgacgatttcggttgtcccgtacatgttaaagcaattattaaaatatcgaacggctgataacacaccatatcaggccaattttcagcgcatgctgctgggtggtgggccaattgatcgccaaacccttcagcaatgtcgtcaactccaagtcccggtggttcagtcatatgggatgacggaaacctgttcacaaatcattgccttgaactcagcggatgctgacaagcgaattggctcggttggcaagccactgtttctgactcagttaacgttaagtcaagttaatcaggaagtgctgatcaaaacgccggcattgactccgggttacttgaaccgacaggctgcttttcaagataagctaaatgacaccggctggtatcgaaccggtgatgttggtcattttgatgatgatggctttttatacattgatggcagactggatgatatgattatttctggtggcgaaaatatctttccggatgaggttgaagccgtttatgtcaatcggtcagacatcggcgagattgccgtggttggccaagatgatgccaaatggggtcaagtgcccgttgcgtttgtggtcagcgatgcgcccttagatcaggtagacctgatcacttatggcagacagaagttagcccactacaaggtaccaacgagatttattagaattgacaaacttcccaccaatgtcagcggtaaggtgcagcgattcaagctgaaacagttgttataaaatgaaacgttaacaagctcgcaatcatgagtaaatcattttactcaggttgcgggcttgttttggcttaaaagtgagttaaaccggtttacatcagcctcgtgtaacatgttaacaaaggtggaacaaactccatcgttgttctgacggcgtctagaaggcctcagactatatattttagcgcttacatccgttatattaagagcgtaaagaaatcctcgagaatttctgagatccaaacgacaaacaaaattataggagatgccaattatgaaacgagactttattgataccaacacatacacccgagaagaaatccaatacctgatcaacttaggtttacaaattaaacgcgacattaagaatggaaactatcccgacttattatcacatcggacactgggaatgatttttgaagaatcatctacacgaacccgagtatcatttgaaactgcaatgactcaacttggcggtcacgctcagtacctcgcaccaggtcaaattcatttaggttcagctgaaagtgaatcacttggcgacaccgcaattgttctttcccgcttggttgatatcctgatggccagagttgccaaacattcgacagttgaaaaattagctgaaactgccacggttccagttcttaacggaatgagtgattacaaccatccaactcaagaaatcggcgacatcatcaccatggcagagcatttaccagcaggtaagaaactcagcgactgcaaggttgtcttcgtcggtgacgccactcaggtttgtgtatcattaatgttcattgcttctaagatgggcatgaaattcgttcaattcggaccaaagggttatcaaatcaagccggaaaccttggaaatcggcaagaagaatgccgaagtatcaggtggtagcgttgaaatcaccgaagatgccgacgcagcgatgaaagatgccgattttgtttacaccgacgtttggtatggtttgtacgaagccccactttcatacgatgaaagaatgaagatcttctatcctaagtaccaagttaatgacgatttaatggctaaaggcaccagccacacaatgttcatgcattgcttaccagccaaccgcggcgaagaagttactgacagcgtgatcgactcaccacactcaattgcctgggataaagccgaaaaccgtttgactgcaatgcgcgctttgctggtctacttgatggcaccacggatgaactacaccgaaaaacaattggatgatttgaacgatcctaaattgaagtcgatgatcttaaacttagttgacgacacgactcattaatgagctgacgcaacggatgtgcaggtgaaagaaatgcaaaaagagaaaaaatttagactatttgatgccgtgctgatgtcggtggtcgttgttctggtggttgaatcagttgctccggcagccgcaatcggcccgtcgcaattcttctggtggggaatcctgttggtattcttcttcctgccatacgggttgatttctgccgaactagggacgacctatgacgaagacggcgggatttatgactgggtgagaaaagcctttggccgccgttggggtggtcgggcagcttggctgtactggatcaacttcccaatttggatggccagcctggccgttctgtttaccggcgttattggccaagtcttcccgactcatttcgggacgtggaccaacgtcttaatccagttggtcttcatcgggattgtcactttgatttcctcatatccagttgccgacagtaaatggattttgaatctggctgcgattgccaaagtgattatcatggtcagcctgggtgctttgggcatttacgttgccatgaccaaaggcgttgccagcaacttcaccgttaagacgatgctgccgcaaatggacgttaaaagtcttggctacatctcagtgatcctatttaacttccttggttttgaagtggttacttccatggccagtgaaatgcctaatccaaagaaacaaattccccaagccattatctggggcggtatcttaatcgctgtcttctatgtctttgccgcatttggtatgggcgtggcaattccaagcagcgaattgtcaacttccagtggtttgatggaaagtatcctacttttgatcggtgggaataattggttcgtcatcctgatcgcgttactgtttatgtatacgttagctgccaacctgatttcctggtcagccggggtgaactacgttgcctcatacgctgccaagaaccacgatttgccaaaggtatttggcattgaaagcaaaaagaccgggatgccaaccggcgccaatctgttgaacggtgggattgcagccgttctggtggtcatttccccactcattcctaatcaaaacattttctgggcattcttctcactgaacgtcgttgccttgttgggctcatacctactgatgttcccatcattctggaaactccgcaaaattgatcctgatactgagcggccattcaaagttcccggcaaccatttgatgattaacttgatgacttggattccggtggcattgcttgccatcacgacgattctgtcagcattcccactcaacggcagtgccgaagagcttaacaccaagattccaattttaattggaacgatcatcacaatcttacttggtgaggtctgcatcagagccgctgaaaagaatcatccgttgaagaaaaaagtcaaggcgagcagtcaccacacagaagaagccttaagtaaaaactaatttctgaatctaatgcaagaggagcaaatacgatgaaaactttacaatcatcacctaaaaaagatggatacagaatgcccggcgagtttgaacatcacaagggtgtctacattctttggccagagcggccggataactggcgcaatggtgccaaaccagctcagcatacgtttgtgaacgtggcgaaagcgatttcccagttcgagcacgtaacggttggggtttcagatgcccaatatgccaatgcccgtcatatgctgccagacgaggttgaagtggttgaaatttccagtgacgattcctggatccgagactgcggcccaacgtttgtcgtcaatgacgatggcgacctccgcggtgtcgattggacatttaacgcttggggcggcttggttgacggcctgtacttcccatgggacaaagacgaccgggttgcacaaaaagtgactgaaatggagcatgccgaccgttaccgtttggacgacttcattttggaaggcggctcaattcatgtggatggtgagggaacgctgatcaccactgaagaatgcctgctttcaaagggacgcaattctcagttatccaaagaacaaattgaaaacgtcttgaaggaatatctcaatttggacaaagtcatttggctcaaacgcgggatctacctggatgaaaccaatggtcacgtggacaacattgccaacttcgttaaacctggtgtcgttgcccttgcctggaccgatgaccaaaacgatccgcaatatgagatttccaaagaaaactacgacattttaagcaacgcaaccgatgccaaaggccgcaagattcaagttgaaaagctttatgtacccaagccggtaactattaccaaagaagaaagcgaaggcgttgatgccgttgacggcagtctgccacgtcgtgaaggtgaccgcttggctgccagctacgtcaactattacacagccaatggcggaattgtcttcccaacctttgacgatccaaacgatgctaaagcgcaagaaactctgcagcgcttgtacccagaccgcaagattgtcggcgttcctgcccgagaaatcttactcggtggcggtaacattcactgcatcactcaacaagtgccagctggcagataggaggaatcgcaatggccaaaattgtcgtcgcattaggtggaaatgccatcctctcaaaggatgcttccgctcaagcgcaaatgaaggcagttaaaaagactgccaaagagttggttaaatttatcaagaacggtgatcagttgatcatcactcacggaaatggtccccaagtcggcaacttattgcttcagcaaaatgccgccgacagtgaagccaatccggcaatgccgctggacacctgtggtgccatgacccagggcagcattggctactggttccaaaatgccatgaaggaagagctcctgaataacggcatcgataaagatgttatggcaattgtcacccagacgatcgttgatgaagacgatccagcctttgaaaatccttccaagccgattggtcctttctataaggaaacggatttgcctgagatcaagtcactgcaccctgactgggaaatcattgaagattccggtcgcggctaccgacgggtggttccatcaccgaaaccgctagaaattaacgagtacgcagcgatcaagaaggtcgttgacgcaggtatcgtgccaatcgtttccggtggcggcggcattcccgttgtcaaaaaaggcaaccgcttaattgggaaggaagccgtgatcgacaaagatttcagtgcttcaaagatcgcccaattaattgatgccgacaaattgatcatcttgacgtctgccggaggggtttactacaactacggcaagcctgatcaagttgagctcaaagaagtcggcattgacgacattcaaaagcacattgatgccaatgaattcgccaagggcagtatgatgcccaaggttcaagcagcagtcgcctttgtccgcagtaccggcaatcccgctgtgatcggtgatttggaagatgttgaacaaatcatcgaaggcaacgaaggcacaactatcgttaaggatgctgttcccgcagcagttaaatagtttaaaatgaacgaggcatggacgaaacgacggttttgtttacgcctcgttttgcgtcgattgatggggtattagcagaatgatagtgctttcacagcaaaaatgttatgattgagcgagaaaatatcgaggtagataatgaagatcaaaaagacaactccacaagaggataaatacaatgtggtccctgaatggcgtcaacaccagcaggcttacatgatgtggccggaacgcacggataactggcgggagggagccaaaccagctcaaaaagttttcagcgaagtcgctgcgaagattagtcggtatgagccgctgacaatgctggtttcgcgtcaacaatacgagcacgccctgcatgccttgccggaatcggttcgggtggtggaaatgagttacaacgatgcttggatgcgggatgtcggcccaacttacttggtcaacgcccaaaataacgttcgagccgtcagttggcagttcaatgcctggggcgggctggtcgatggcctttatttcccgtgggatcaggacaacctggtatctgggaaagtcagtgatttggaccggattgactactatgacgctgattttgtcttggaaggatccgcgtaccagaccgatggcgaagggacgctgattgccactgaagaatcggtcttatccgaggggcgcaacggccaagttgatcaggcagatgttgaagcggtttttaaacgctatttgaacgtcaccaagattatttggttgtcccgcggctacttcatggatgaaaccaatggcgatgtggacaacatggtcaactttgtccgccctggcgaagtggccttaacctggaccgaatatcaaactgatccaatgtatgaaatctgccatgaagccttggcaactctagaggcggcgaccgatgcgtccggcaggcatttcaagattcaccgggtccagatgcccaaaccattattaatcaccaaagccgagagtgaaggcgttgacccggtcaacggtcggctgccgcgttacgaaggtgatcgtttgatggccacttacattaactgttacttggcgaacggcgccgtgattctgcccatttttggcgatgagcacgaccaggcggccatcgaccaatataccaaaatctttccagatcgaaaaattgaacccgtgtacgcccgtgagctgctgcttggcggcggcgatattcactcgatcgtcctcggggttccagattagaggttttatatgaacttttttgagatcattaaaccatatgtcgaaaaattaaataaaaatgaatacggcttactcgactatgtgatcaagaatatggataaaatccaaaacaagagtatccgagaaattgcggcggcctgttatgtttcgaccaccacttttttgcgttttgtcagaaaaatcggtttctccggttatagtgaatttagcaccgtgattaagtacacggtcctcaacagcgataagcaggaagacaaggctgaaccgtttgttgaagaacagtccaagtatcgtaacgaatatctgaaaaatattgaggaaaccgtgcgggtgcttgatgagcgcaaactgttaaaaatctgtcaggtgttagaccaccagcccaaactgtacttttttgccaaaggcttcagtaagtactctgccgaatacattgaatacttatataccttgaacggcttcatcgtaattttccccaagaatcacgagcagcgccggctggcctaccgtaacgtacagctcaacgacgttgtctttgtttttgattatgaaggtgaggatgatgaactgattcaaattattcaaaatctgcaaagccaaaaggaatacgccttgctggtttcaattaccggcgcgaataacaatacgattcaaaacatgagtgacgaaaacctctatctgttcacggacgaactcaaagtcagcggagttgatatgacgtcgcacgtttctttgattgtgattatggaattgctgctgtatcaatttatggagtatgagaagtcaaaacgatagtgtgttggaagctgacagtttagttttccgtacccgattttgtttgtcttcaagcccacatatggtaaaattcaagaaacaaattgattcgaaaggaatttgagatggcaaacaactcgcaacaagagctcttaaaaacaatccatcaggctaaacctgaaaagctaaagaatgtgctgctaaaaatgggatcccttgaccccgacatggctgcattaattttggcgatttttaacgatattcctgttgatttagatatcgacgccggctttgaagttgatcatgatactgtcgaggcagatccactaccatcaaccaatccggataccgacccgcaagcgattgaagaagaaattcgccatgttcgcggcgttatttccaaccagcttcagattgcccgtgagtctgactgggactggaacggtatgaacaatttggtcaacttcttttctgacctgctaggggaagtcattgacgataccggtgaactcaaagtcccgtttgcattaggcttcccagttgccctaatggtggtccaaaatcaaatgaaggtcttttcagaggatagcctttcgccgatgactctggaggattcagttaacaatgtgttgggcgttatcatcgatttgatcaatgaatccggcagtcatttgccagtgaatgaacgtgaaaaatatttggaccaagcgctgaaactgttcggcagtccagtgttcaaagatttggaagcttttcgatatgagtttatcgatgacgttctcggtttggtcactaagcagactgccaataaagtcattaaggcctctgaaagaattatgaagcaaagtactttgtgggatgaagatcaacgcaagaaacatcacctgatgttgcggttacatctttacctggcactgggagatttgggggtcgcccaagagatagccatcgcaaatatggacgatgacgatgtccgcaaacaatggttttttgtcttgaaaagccgccatcgttatgatgaagccaaagaattggcacttgacgttccccgatatctaagaaaagaatgggacgaattgttgtccaatatgtatcaggaattgggtgagaccgacgaattaattgcgctgttgaggaagcggttgttaaaccatcaaaccgccgtctaccaacaatataagcagctgttagtcgagcgtcatgagtggcagagggtttaccctgatttgttgaaacaactggaaacaaagctgacgcgctatgaatatggtgatattttagctttggaacaggagtattcaaagttgtttgaacaactgaagaagtatcaaagcgcaccaatgatccggaattatctgcgacagatttatccggcggtcaaagataaaatgattccactgtatcacgatgttgtcttgattcctcaatcccagaagacagccgccaatgcgccaaaacagctcgagaaggatttaagcaacttcttggaaattagccacgatgccaccacagttcaaaaatgggtggatgaacttaaacagcgcctgagcggccaaaccagctttttagagggactggaaatcgttcagactcaaattaatacagttgtatagtcaaaaagttccactctaagccacctagacagcttggagtggaatttttattgaacgccacatcaaaaaggcggccgcagcacaagtctttcaacttgtactgtggccgcctttcagctttaaaaactagctcttcttttcttcaaacaaaacgcgcttacgcagctttggtgaatacttcattagctttaaccggtctgggttgttacgacggttcttggtggtcaggtattcttcaccagtttctttgttatgcattacaacatgaattctcattatcttacctcctcacgaatggtaattgttatcattacaaatataaagcactgaccgaatttgtcaagtcatcctcactggttgaactggtttgagcttcgattggcaaacaaaaatcatttagttattgtactggtaccagactgctttcccgtttgtcaccagcccgggctcttaatgcccacagaatggtcacggtatcgacgacttcctggaagagggcgccgatgatcgcggggatgacgccaaaactggcgattaacatcaaaatcgtacagatagcgattccaatcaaaacggattgacgagcaacgttcatggtgtcgtctgagattttgaccgctttactgaccaggcttaaatcgtctttgaggacgacggcatctgctgattcactggcggcagtggctccgtgagcacccatggcgatgccgacgtcagccattgccaatgatggggcatcgttaacaccatcgccaaccatcacgaccgggcggaacttcttttcaaccttttcaatgacggaaattttttcttccggcagccgctcagcgtaaactttatcaatgccaactcgatcggcgatttcttctgcgatcggttttcggtctcctgagatcatcatgatttctgtggcgcccatctgatggagactatccatcacagccttggcttccggtcgtaattcatctgagaaggccacgtacccgacatatttgccattgacggatacgtagactgccgtttgatcaagcgggtcaattgggtcatcggaaacataagccggtttcccaacccgaatcgtttgctgatcaatggttgcctggactccttgggcagtggtttcaataacgttggtggcagtcggaatttgatccggaatcgccgccaccagtgaacgggcgagaatgtggctggattgctgttcggctccggcagctagcgccaagacctgatctttggtgtaaccagctatcgcgaagacccggctgacggtcaaatgccctttggtaatcgtcccggttttgtcgaaggcaaacgttttggcattggccagcttttcgataatcgtcccactcttgacaatgatcccatttcgactggcacggctcatgccggatactaaggcaattggcgcagctaaaatcagtgggcacggtgaggcaaccaccaggacttctgcaaaccggactggatctttggacaggtaccaagctactccggcgatgacgtaagccagtaaggtgaatggcacggcgtagcggtccgccatccggacgaagtgggcaggggtgctctcagcctgtttaactaatcggatgatgttttggtactggctgtcatcggccgttttgtcagcaatcatgtcaaaggaggcatcgccgttaatcgccccggacatgacggtcgatccaaccactttatcgatggggcgggattccccggtcagagaggattcatcaactgacgtcacaccatcggtaatcgtgccgtcaactgggatgacttccccaggcttaacaacaatccggtcgccgacagtgacctggtcaattttgacgtcgaccattttgtcatctttcagcaaatgagcggattggggcgaattctccagcagtgactgaagctcagagttagctttgttggccgcataatcttccaaagtgtcgccgccggttaacattagcaaaacgatgagagcggcccaatactcgcccacggcaatcgttgcgatgacggcggtaatggccagcaggtcgacaccaaattttccggatcgcaaagttttcaccatgtcgataaacatcaaaagggcgattagtgaccccagcgttgagataacgatctgggcataaagcggcaagcgcagcccaaattgtagaaccaaggcgatcaccgcgacaattaagacgccaattagacgcatgtagttggttagtttgttcataataagccctccaatccggtttaatcttctatctagattataacaattctaaagtagaaaggcgagctataactccatgggttatcattttcaggcagaatatgtacaaaaatggcccgccatcatcgggcaggccagtgagacattattgggattatttggaaagttgactcaaagcttcaaagtcttcatcactcaatttaacattagcagcagcgacgttatcctccaagtgttgaatcgagctggttccaggaatcggtaaaatgtttggtgaacgtttgagtaaccaagccaaagcaatctgggcttctgagacaccatactttttggcgatggtgctgagtggactatcggcgccaattaaacgaccggtgtccagtgggaaccatggtaaaaaggccatcccttgggattgtgcgtagtccaccacatcgtcatccttgtggttggaaacgttatagaggttttccacagcgtcaatcttggcgtacttttgggcttctttgagttgatcaacactgacttggctcaagccgatatgcctaatcttaccttcatcctgcatcttcttgagttcaccaacctgctcagcgactgggaagtgactgtcaattcggtgaaggaagaccaaatcttcgtgatcaatccccaaagtcatcatagaaacttcgacttgctggcgcaggtagttgggctcaccatgaggtgtccagataccagggccttggcgggtttgaccaaccttatcagaaatgaaaatctggtcacggttggcggcgccctttaagccttcagccagatagcgatcggcgaaccacggaccgtaagaatcggcagtgtcaaaaaagttgattccaagttcagtcgcgtgggtaacaacatcggctgcacgggcagggtcagcgtatggaccccaagtgcctttaccagtcagctgcatggtcccgtaccccaggcggttgacgacaaattgatcatcaaatttgtaagtgccagcgtttgctgcatttagttcagtcatcaaatacacttctttctgacaataatttggtacaggtctattttcaaaccgttgctgcctgatgtcaatcaaacaaacgcgcaatcgtttgtggttagttaattttacgaaaaatgacaaaaagttgttatccaagctatacggatgggtcagcaccctgtaaaatattgtatacttacgttgataagagagatttatgaatagctgtgtttgattggggaatccatacagaaggtgaaaacgatggcagtaaagtattatggcgtgatgatggtgaatgttcagggctctgaattgttgatcgtgaatttaaagaacctgaagccactcgagcacgtcaaaaaagatattaacctgggagacgatgtctatcaggaccaacccgtgaagtacgaatccgttaatcgggtgtccgaagctttgaccggatttattcaaattttgaatgattacggtgtgaccaactacaaactatttggcagcaatgcccttcaccaagcgatcaactcagattttattgccgatcagctctttttacataccggcatgaatattgagtggctttcaacaagtgaagaaacttatttcagaaatcaaaacatttcagttgagttgacgaaggataagcaaaacgataagcgcaccacttttttggtgggcatcacttctggaaatactgccattacggagttcaaggaaggtaaatttgtcgactccaccagttttgccttggggccaatcaaaattgccgaggacttgcagagcctgcggcaaacggcacccaattcaattgggctgttgaacgattacattgattccaaattgaacgacttttacatcgggaatcctgccagcgtcgtgtccagcaaagttcccaccaagatcattttgctggggtcgctgcctttgcaacggctggtggaaaattacgagcacactaaggccagcgacacgattactgccagcgatttcactggattagtggacgacttggtggatgcttccgatcaatttttgattgaacggctccaagttgatccggactacattcccttggtgctgccggaactgctgttgaccagacggattttgagattaaccaatgcttctgaaatcgggttttccgattctggggtcgttgatggtctggtcaatcaggaagccttggaacagggctactcaaaacgggatttcacacccgagattattcgtttggctttaaacctttccaaacactatgatgttgagccggtccaccgggatttggtaactaaatttgcccttcatttatttgatcagttaaagccgctgcaccaactgggccgccgtgagcgaatcctgcttcaggttgcctcaattctccacgatgttgggaactacgttggcatccatgaacactacctgcattccgagtatattattctccattcagaaatcattgggttgtcccgggatgatattcgggtgatcgccgcaattgccagatatcacagttcgacgacgcctaatgaagacttaattcactttcagcatatctcagctgaaagccggcgattaattgccaagttagcggcaattctgcgtttggcagatgccttggacgacgaccgccagcagaagattaaaaaaatctcggtttcaatcaaggaatctaaagttgtcatcacaacgttcagcaatgccaatctggcctacgaaaactggatcttcaacaccaagagtcagttctttactgaagcatatggttataaggccgttctcaaacaaaggggtgtaaaggcaaaatgacagacaaaattgattttaaaaatcccaaatactataacaaccgcgaactgagttggctggattttaacgaacgcgtcctagaagaagcccgggataaaaacaatccattattagaacgggtcaaattcctagggatcacccaaagtaacctcgatgagtgggtcatggttcgggtagcttcactggcaaaattggttgaagttaagtgggatggcaaagattcatccggccgttctgcagaagaacagctccgggacgtcaacgtgaaagcccatgagatgttggttcggcaatacagcaccttaaaccgctcgttgttgccggcgctcaaccaggtcgacattcatttactaaaagtgggtgacttaacccccgagcaataccagttcattaaaggatacttccacgatgagctttatccagtgctcaccccaatggcggatgacagttcgcgcccgtttccatttattaataatgactcattgaatttgtcactgcggcttaacaagaaagatgatgaggagggcaagacactgtatgcgacgcttcaagtccccagcatcttctcacgggtcatcaaactgcccggtggcgataacgattttattttaattgaagatattattaagcaattcgtcgatcaattattcattaactacacgatcaaagaagtcagtgtcttccgggtgattcgggacatggacctggatgttgctgaagaagatacctctgacctgttgaaaaaggttcaacagcagctgaagttgcgtgagcacggccaagtgattcgtttggaagtggattcaactatcagcagcaagctgcgaaagcggctggtcaaggaacttcagacggccgaagattcggtctatgaagttaatggcccacttgacttgaccttcatgagcaaattagctggtaaggtgatcggtcatgatgatttgaaatatcgaccgttcaagccttatcaaccggcagctttagactccaatcacaacatttttgatgccattcaaaagcatgactggctgatgcagcatccatacgacaaatttgattctgtcgttgaatttatccgtcaggcatccgttgatagtgaggtcttagcgatcaagatgaccctctatcgggtatccggtgattcgccaatcatcaaatatctgggacgagctgctcaaaatggcaagcaggtgacggttctagttgaagttaaagcgcgatttgatgaggaaaacaacgtccactgggcccgtcagctggaaaagatgggctgccatgtgatttatggcctggttgggttaaagacccactccaagctgtcattagtcgttcgtcgagaagaaaatgggattcgccgttacgtgcacatgggaactgggaactataacgacgtgactgcccacttctacaccgatttgggcttgttgacctgcaatactgatatcggcattgacgttacgaatatttttaacatgttatccggttattcacggccgccatactttcaccagctgcatatttcaccaaatgggattcgtgaatttatcaccgaacgattggatgaagcaattaaatatgccaagcagggcaaaccggttcatgttcaaatgaagatgaattcgctgtctgatcaggatatgatcgccaaattgtatgaagcatcccacgctggcgtaaccgttgatttgattatccgaggaatctgctgcttaaagaccggcatcaaagatgtcagtgatcatatcacggtccattcgatcgttggtcgattcttggaacacagtcggatttacttgtttaattttgacggtgaacaacaagtttatcttgccagtgccgatctgatgactcggaatttgaaccgacgagttgagcagatgtttccagtccttcaaccggatttggcccagcgagtggtcagcatctacaccaccatgtggaatgataacgtcaagacaagaaccttggataagaacggtgtctacaaacgagtggacagaagaggccgtgagccattggattctcaagaattctttgcagctcaggcaactcggttgaccgaggctcagcaaggagagaatcggcccaagagtggggcccagtttcagccaatgatgagcccacaaaatcagcctgatccattcaatgatgaagatgggggcgacaaccagtaatggaaaatttggcggtgattgatttaggatccaactcagtgcggatgaccattagccgaatcagtgacgatggcacctacgagacagttgctcaagaaaaggaatatgttcgactgtctgaaaatatgggggttgagaaaattcttcagcccgaagccattgagcggactatcagtgctttgaagaacttcaaaacgatttattcaaagcttgaccatctcaacattgttgcggtggccacagcggcagttcgacaagcgaccaaccagaagcaatttttaaaacgggtcaaaaatgacattggcattaacctcaacgtgatttccgggacccgggaagcttactatgattatgttggtgtcagcgagacattgccggcaactaatgcggtgattatcgataccggcggtgccagtgccgagatcgtcctggttcaaaacggcaaagtcagcaacctgatcagtattccaattgggtcagtcaccttatcatcaaaatttgatttggctgacgacattgcggcgactgaagtctttaaagcaatgattttcgttaacaaaatttttcaaagtgtctggtggctgcgaaacggtttgaacttgccaattattggtttgggcggcagtaatcgaaccctggccaagattaatcggcgtttcaataatctgttggataccaatgatatccacggctatcaattgcgggatgacgccattaatgaaacttttgagcgcattattggcatgaatcttgacgaacgcaaaaaggttcccggaattaacaaggaacgggctgatattattgtcggcggtctgatccccgtcattttactgatgaactatttggattcagacagaattatgttttcaaccagcggcctgcgagaggggatcttgttcgaacggctgcatgatattattcaagagaatattaaaaccaaggaataattaaattctttcattcactcaaaaatgggcttgggcaaaactaactgttttgctcaggcccatttgtgctgtaattttcaatattgtctgtttaactagcgggaagcttaccgtctattttcccacactcgcggtatctgtcccactcaaccgttcaaagaacagcaggtgtttttgtgagaaccagtcaatcagtaagtcgacaaagaccagcagcagaccaaacgatagaatcagtacaacgtggagaatgctggttaactgggctttgggcgcggttgccgtcatgtctaaaagccggccgacaatctcgtaaaggccactgatcaccccgtagccaaacaaattccggattaagattttcgaccagctggctgtttggccattacggtcaatcactttgatgccaaccaggcgcatgccaatcgtctgctggcggctgagttccagtaccagaataaagatgacaaagccaatcgcgatgccaatccagtgtggaatcaggaaaatgcccaaaatattggtcaacagaccaatgatgatccaatccactgccaaagcgactccacgccgcagcggcgaaacgtttttactgagcgccattgtccgggttctgacctgttccttggttggcagaaaacggccaagcagagaagctccccaagcaccgatgatcccaccagtggtatttaacagcaggtcgtcgacatcgaatagtcgataaggacggggatagatgccgtaaagaccggagagctgggttaactcgaagaatagggataagcagaatgtgaataagatcgtctgtttccatgaccgctggaaataatagtgcaggtaaaagccaaatggcaccgttaagaagatattaaacaccggttggataaccgtgggggcttttaatgccgcaacccacgttccgggatgtgtcagtgagaatggattgtatttaatgaactcccggacgaatgtgaaaggcacgaaattgtgagtcggggtcgtcaaatgggccacaaaagattggcttggcaatgggagaatggtgagaaagtaggcacacatcatgtagaagacaaatgtgtagagcataaaaatgctccacttgggaattgcgccatacttgtggtagttcactaacaggatcggtaaggtaataaaaattgctagaattggaaaaataattgcagccgtataaatgacgtgaatgtactgtgacatggaaatctcctaaattttattttattgaatgggctcaccggggacaaaatagagtaacagcccggttccaagggcaattaaggcaatcaaaacgataattgcgatattggcgcgtttgttcattaccagaaaggcgaggtgttcgcggatgactgcgttgggcaaaaagtaaaatggcgttggcgctccaataccaaatgcggcaaatttcaacttccgggcaagcacgccggcccgcaaaatgtgatagttgttggagacaaaaatcactttattgtcgtctcggccgctgtctttttcgatgattttccgggagaaggctaagttctgttcggtgttgatggacttatcttcaaccaaggtatcaactttcgggatgccatgttccaaagcgtatttctgcatggcttcaccttcgggcaataattcgtcaccgccttgaccgccagaaaagatcagctttggatgtttgccggtggttttgatctcactccggtaaaaagaaagagcggtttcaatccggttgcctaacagtcgaccaactttgtagccgtcgatcaaaccacttcccaagacgataatgtaatctttatcttttcgtggaaagtacagtcggtataagatcatcgacgaaatcgtattccaaaccgttaataggacgtagccaatcagtagggtcaaaaacatcgtgacgcccccttgaagcggtttgggcccaactgatggattgaagaagaataacaggtcaacggcgatgacggcaatcccggtaatcaaagtcagggaactactgaggctataaccttcacgtttccacacaataaaggcgttaatgaaaaagaagatgaagcttaacgtcaaccccaagaaaaccagtaagccaaccaaggcaactgccagacctaaaatgatgccccagaactggctgttgaggaccgagataatttcaaccagcaagaccagcagaaccagcagcgataagtttgccagggtgccgatatataaggaatttctcagtttaattaagtatgtaaagaataatccgaccaggacgatgaagataatcgcggtcggtatcagtaaagtcatagaaaacacccctttgaaacattatatttcaaaggggtagtggaaaacaagcacggtcgcttcccgtaggcaaactttaactttttagctcattccgacagcctcggcatgtgccagcatatcattgagcatttctcttctggtttggcgtggcaggaagctgcggatgttttcctcactaaagccaacctgcagctgttcatcattgaagatcagcggccttctgagtaaatctggatattttaccatcaggtcaattaactgtgatacagtaagattatcaaaattgacttttaatttgcgataactgtgacaacgagttgaaatcaggtcctcagtgccattttccgacagtctgagcagttgcttgatgtcatctgcgttcaaagtttgtttggagatatctcgttccacaaaatcaatgtggtggtcggtgagccactttcttgcccgtcgacacgatgaactgccaggcgacaaatataaactaagcatggttgccatctcctttactgactgtgacgacaatgcagattgatgcaccggctcatcaacctatccccacttttatcttatcataattataactaaagtcaaatgtttgctataagaaacaggttaataaagtcttgctacatcaagggctacgactcttgtgaaaggttaagtaattcttaatgtttaatctgaatcattcaaattttaaaggagcgaggactaatgaaaattgctggatttggcgttgaagaatggttgaacaaatgggaaaaatcagcaacttatgatatttctcaaagcacgatttcatcaatgacgatgcaagaagccctggcacttgatggccagcagggggcatcattttatcaacaactggatcaagaaaagatgaactatggctggattgagggctcacctgaattcaaacaggaagtcgctaaactgtacgcccatattgacgcggacaatattttgcaaaccaatggtgccaccggggccaatcatttggcattgtatgcattgattgagccgggcgaccacgtgatttcagagtatccttcctatcaacagctgtatgacatccctaagtctttgggtgccgacgtcgatttttggcatattcatgaggaccagaattggtatccagacattaacgaattaaaatcattgatcagacccaacacgaagatgatttgcttgaacaacgccaacaatccgaccggaaccctgctggataaggcatttttgcaacaagttgtcgaattggcccggcaggtgggtgcctacgtcttggtagatgaggtttatttgccattggatgatcccgatcaatttacttccattgtcgacttgtacgacaaggggattgcgaccaattctttgtcaaagacctattcaatgccgggaattcgaatcggctggacggcttcaaatgcgactgtggccgatctctttcgcaagtatcgcgattacacgatgatttgtgccggcgtctttaatgatttgatggcgacctacattttgaagcatcgtgaccaagttctggcgagaaatcgacagctggtgatgaataatctggcgatttatcgtgactggattgactcggaacctcgagccagtgtcgtgatgccccaagcggtttcgacttcgtttcccaagttggatgtcccggaagatattgaagcgttctgtattcgcctgctcaaagagaccggcgtcttactggtaccgggcaatcgatttgatatgcccggccatgtgcgcttaggatattgtgccgatgaaacaacactcagggaaggtctgaagcgcctatccgcctttttgcgccagtacgattaaactgatttgattatgaatgtttaaagttgtttgcatttgtttaaaggtgatcgcttgaaaagccagattggtccaactttaagtttgggttaagctggcccttgtaatctatggacaatcaaataagaaagaagggatcagtaactgattgccaccatgataagtgcagccaatgacttaaagtgccaacaatgagattgaagattgtctcctccaagatatgattcttctacaaggcattgtcatttgggctacaggaaaggaagtcatctatgaagcgaaaacgtttttactttacgtctggaattgcggcgacagccattgccttagtggttgccggacgcgttttccaacggtcacgcatgattgcccatgcgaactaaacaagaaccactcctccaaaaaaatcgctgtgccacttaatcgttcaagccggttaagctgacacagcgattttttaattttgatttgctttttgcttggctaagttggaagcagcaaagactgattcagtttcctcccagattcgcttggcaattttcgacttgttcatcgtgtagagatgaatgccatcgacgccctgagagaccagatcaatgatttgatcaactgcaaaggcaatcccggcgtccagcatggcttctttgctgtcttggtaccggtccataattgcggcgaatttctttggaatcggcaccccggagatttgggtgatccgctcaatttgattcttgttggtacagggcatgatgccggcttcaattgggacgttaatgccggcaatttcagttttttccttgaaatcgtaaaacgcttgattgtcaaagaaaagctggctgattaagtgatcagctccggcagccactttttccttgagatggctaatgtcatcgacaaagtcggctgcctctgtgtggcagttgggataacaggcgctggcaatgctgaaatcggggcgctgctcatggacaaatttgaccaattcattggcatgattgaagtcgcccaccggttctttgccggggatacgatcaccacgaagagcgaggatattctttacgtggatctgatcgagacgatccaagagtgccagaacctggtccttgctctgataaagtccagggacgtgggaaactgccgggatgttgagttggttttgaatcaaatcagccactgccacggtcccatcacagtgattagttccaccggcacccaaagtgaccgaaataaaatccggctgcagtgactgaagtcgtttgagagttggcaggatcgcatcggttggtgagtcctttttaggtggaaatacttccagcgaaaagacggttttttgtttaaacaacgctgttaggctcattgatctcactcctaaccttcttggtggcatcaacgatgttcttcaggctttcaaatgactcgtcttcggaacgggtcttcaaaccacaatcagggttgatccagaccttatccaccggcagcttggcaactaattgcttgattaagccctcaatttcttgctcggaaggaattcgcggtgaatgaatatcgtaaacgcctgggccaacttctgtttggaacttggcagccaccagctgatcgatcaaagtgaaatcggcacgggaggcttcaaaggaaatcacatcggcatccaaagcgtcgatggctttaatgatgtcaccgaattcgctgtagcacatatgggtatgaatttgggtgctgggttgaaccttgctgtggacgaggcggaaggccggcactgcccagtccaaatattcagagtaccagttggactttctaagtggcagattttcacggagagcaggctcgtcaatttgaataatcttgatgtcgtgcttttccaaatccaggacctcatcttgcaaggctaaagcaatctgggtcaccgattcttttggcgtcacgtcttcacgtgggaacgaccaattgaaaatcgtgaccgggcctgtcagcatgcccttcattggtttgtcggttaaatttttggcaaagactgaggcagcaaccgtgattggtgcggttcgactaatatcaccccagatgattggcggcttaacaccccgggtgccgtatgattgaacccagccgttttgggtaaagacaaagccggctaatttttcaccaaagtattccaccatgtcgttacgctcatattcaccgtgcaccaggacgtcgagcccaatcttttcctgaattttgacgatgcggcgaattttatcttcattaaatttatcgtattctgctttggtaatttcaccgtggcggagttttgcccggttctggcggacatctttggtttgtgggaaggagccaattgtcgtggtcggcagaattggcaaattgaattcctttttttgaatcttttcgcgttcacttcgggcgggtaaacgggtgtagtcatcatcggttaaattgttaatccgttcatggacggatttattgtagggatgtttgacgttgcggaaaagggcgtcatttttttcgagcgctgatttaccgtcggcttcatcgtggtaaatggtgtccagttctttaatttcggcaagcttttcaatcgcaaatgccaagtgctgtttgacgtctgatgggaccttggtttcatctgcggcactgtatggcacgtgtaatagagaagcagaggaactcaaaacaactttggcgtccgtattcaggttgtttagcaggtcgatggttgttgcgtaatggttgcgccaaatattcttgccgttaacaactccggcgaataataccttgtcagcggggaagccgttttgtttgacgagctctagattgtatttgccttcgacaaagtcaagaccgattccgtcaaaatccaggctggtgacgtcatgatagatgtcgcggatatcaccaaagtaattttgcagcagaatcttgctggatcctttggcagccaagatgccatgatacaatttgtcaaaaagggctttttcagcggaattgacgtcgaagcttagggcaggttcgtcaatttgaatccagttacccccttgttgattcagatgctcaatgacttgtgagtaagccccaatgaggtcatcaacaaagtcattgggtgtcgtcccatcaaggaaacgactgagtttgagtagtgtgtaagggccggtgatgacggccttggcattgatccctaatttgagcgcttcgtcgacttcattaaataatttatcaccgactaatttaacgtccgtcgtcttagtgaattctgggacaatgtagtgatagttggtgttgaaccacttcttcattggcagggctttgacggtttcagaaccgttctggtacccacgggcttgagcaaagtattcgtcaagcggtgataagttgagggccttgtagcggtcagaaacgatgtttaagaggttggcggtgtctaagaccccatcaaaaaacgagaagtccccaacaggaatcaggtcaatgccggcgtcttgttgcgcctgccagtgattcttgcggatttgataagcggtttttagtaattcattttgatcaatcttgtgcttccaataatgttcggtagcaaattttaattcacgatggtgaccgatgcgcggaaagccgataatggtggttgtcatgtgtttgtatcctcctagagtgcgatttggggcggttagcaaccggagcctaaggtaacttgggggaaaatcgattttgattttgtcccaagttgccttaggtgcaggttgctgctccaaagagcacgtttcatcaaagtaaaatcagtatagatagcgggcagcctcagcaattattgaacagtacgttttaaagcgtctttgtatcaagactcattaccagataaaactgagggagccacgtcttaacaggtatgtccccaaacccctaaatcacgtgtcgttcataagggtcattggaaatcccctcagccaaaatcttcttgctccattctttggctgaaaatagtgaatggtcgcggtaattgccgcaactgtatttatcaacgccgggaacgtctttccattctactttgttggcaatttcatccaatgacccttttaaggcctcggcgacttcggtggtgctgtgtttcccccaggtaatcaaatgaaatcccgtccggcagccaaatggtgaacagtcaatgacgccatccaagcgatcccgcagcaaactggccagtaagtgttcaattgtgtgtaagccggcagttggaacggcggtttcatttggctgggtcaatcgcaggtcaaaatttgagaccacgtcgccgttagggccggtctctgtggtaattaaacgaacgtacggtgcttttacctttgtgtgatccaatgtaaaactttcaacttttgccataaatgatcaatctcccataacatttaatttgtttttaatgctaatatcaccatccgaagttgaggacacaaaaaaacatccgtccctcacatcagaactaatctgacggaggggcgaatgtttcgctttaccaccctgaatttgtcttggcctcacaaccaacacctctgaaagtaccagacttcgatactcggcgatgtaacggtcgcacccggggttcaagcgttaactcgaaaccgctattcagagttcatgttcgttagctgacgaaccatcctttttcaccgaccggattctctataggttcgttcactaattactcttctcttcagagctttaatttactagcattaaaatttaatgataatactagtcgtagttctaatgattgtcaacctgatatgccaaattatttattatccggtgaaaggcccttgaccaaaaactcgacagcttggtcaatatcccggtccaaatcgacttttcgatcaagcagaataatttgggcaccaaagccggcaccaattgagagaacgtagtccaaaattcgggaggtctcccagtccaccaagagatggcgctctttaagcttatcaatgaccttaggaatagtggtggtcaggacagccttaactggaacaatcaattctgacaataattggggatcgttggccgcctgcataaatagaattttgaggatttgtttgttttcgctggcaaaagtcagtcggttttttaaagtcggctttaagaattctgccaagctgtcgtacttgaaacgcttgaggtcttctgagaactcttgggcagctctgggaacggtttgcgaaaataatggctgaacaacggcttggagcagctgttctttggttttgaatcgcttgtaaactgtgccctgactgacacctgctttttcggcaatgtcagccgtcgtcgtggcttcaaaccctttggcagcaaacagttccaagcaggctttcagcacctgtttttgtttttggggtaaatcttttgtggaatcaatatcttccgaataaaatgactgaatcgaagttgatgccatgttaatcacctacactttccgatacttgcgcattccaatcatatttaaagcaatgaaggcgaccaagaatgctaggatagctgtaaattgtgggacaattgccgaaaagctggcctgcttttgaatgacgtcggttaacgcactggccccgtaatacagcggcatgatgtgggcgataacctgcagccagcctgccatgttggcaactgggatcaaacctgagaagaaaatttgtggaataacgacaatgggaatgaactggaccatttgaaattccgaggcggcaaaggttgaaacaaacaaccccatcgacagtgcaaccattgccaaggcaaaacagatcaataagacgacccagatgctgccaagaatggagatccctaagacatagatacagaataacacgatcaccgctgtttgaatgatagcaacagcgccataaccggttaggtagccgtaaatgatttcacttcgtttaaccggggttgccagcagtcggtccaaagttctggagttccgctcatttaaaagtgaaattccagaaattaggaaaacaaagaagaagaccatgaatcccaagaacacaggcagcatcgttgtgaagaaggtggaattactcttgccgtaaagatagtgctgcgttaatttcaggttggttggcttttggacgttttttggagcggacgctgtcggaatccgactgctgagggtcgctggcagctgctttttaatttgccggagctgagcttgcatcttcattaagccggctttggactgtttcgtggcagcaaccagctgcttaatttgaacttttatcagcgccatctgaactgatttcttgatgatcgcggtcttactctggtcggcattttgatacgtgacgactaagtggccatcagtttttttgatgaaaccggcgtagtctttgtcacgaatggtcttttttgctgaaacattcgaatccatccgatgaattttgatgtgcttgttgtcgattgttttgaccaatgaactagacacattataggtgccgatgtctgcgaccgtgttggtatttgactgaaataagaaatacatcaatgacaggatgaacagcggcgcaataaacattaacgcaagcgttcgtttatcgcggaacatttccacaaagatacgtttagtgattgttagaattctcatttgatttccccgctttcaaaaagacctgttccaaattatccacgtcgtattctttttccaaactggtgggtgacccgtgggtgatgatgtgaccttcgcgaatcatcaatagttcgtcacattcagctgcgtcttccatgacgtgagtggtgatgataatggacttgccggcttgggcatactttctgagttcatcccaaatctggcggcgaagttccgggtcgatgccgactgttggttcatccaaaattaacaaatccggatcttgaattaaactgatggcaagtgacaatcggcgcttcataccaccggaataattactgacccgtttgtccaaatcctggtttaaattgacaacgcctgccgtgtagtcaatccgttgcttcagctgctcttttttgacaccgaacaactgagcgaaaaatttgagattttccttgccggtcaaactttcatatagggcatcatcctgagccataaagccgattcgttgcaggacggggcgattgggcattcgtttaccaaaaatagtcacttcgccaccgtcgggctgttccatgcccatgatatttttaataatcgtcgtcttgccagcccctgatgggccaattaaacccaaaatctcatggcttgaggcagttaggttaacatcatgtaaaatccgttttttattgaagcttttatcgacgtgagtcactgttacaacagcatccatagttggttcctccttttgtgagtgagtgctaactcatttacgacttcagtataccccattcaaagtgagtgtcaactcacaaattgcttttcttgccggtctcacgtataatgacattaaaatttagtcctttaaatagtccagcgagtctgtcaaggaagccattagtgaacgttgtttttaccagcaatagtctgggaatgagcacttcgactcgttgtggggttgaagtgcttttttgtatgctaatgagcattttagtttgcttggaatgatttaaaggacaacaaggagatctatcatggaagacaaaagtttcggtcgtgttgagtccatcccaaaagctcatcggcatcaatcctattgggatatgtttgccacttgggtgggggcgaatgcgaataatggtacttggtatgttggcggggttatcgccgcttgtgggtttgcgacggcttcgacgactctgattatcgtaggtgtgattacatattttttactggcactatccggctatatggggtacaaaaccggtttgcccgcaatggctttaacccgagcttcgtttggcctcaaaggcagtttcctgccgtcagtgattaatgtcgttcaatttatcggctgggccgccgtgaatacgtttatcgcggcaacatcgatcagttatattctccacgatgtcctgggttggccggtatacggcaagccgggcggcctgaaagggttgatctcaggaattgtggtgatgagtattctgcatttattgagtatctcgatgggtgaaaaatcagtccggatcatcgagcggattgggattgtcttagttttcatcttggtaatctgggaatctatcgttgttttccaaaatgtgtcgttatctgaaattgtctcttggcatgcacccagtgccctgaagatgtcaccaggccaagccgttgatgtcctagctgcctttaatttagcctgggtaacggcagccagtgatttcacccgcttttctaagaagcgttccagctccacttgggcaccgttctttggcgccaatctgggattgatctggtttgcgatgatcggaatcatttcaacgatcgcgactgccattaccctgaatcattttgatgccaataattcagacccatcaacgattgccagcaaacttggcttgggtgtcttggcgatgcttgtcatcatcattaccagtaccaccgcaaatgccgttaacctgatgtctgctggatcggcactgaccaatatgactaaacgattatccttgactgtcagcattgtgctggtgaccttagtggctgtcttcgtgaccttcattcccattttctattcgactttcttaaatgttttcactgcctttctggacggcatcgggatgttcttaggacctgaaatcgccatttttctgaccgacttttatctggttgccaaacggaaatatcgagttgaccattttgcctcccggaccggtcaatattggtatactggtggtattaactggattgcgattgcttcatggctgatcgctgtcctggcatacggatacattaagacggtggccgtgttggcggactcagtcggcgcaaccttcatttcgatgttgattgctgccgtcatttattgggtcggcagtcgattgaccagccgcgggcaacttcaggaggattagagtggcaacttttaccaaacaaactttgtctttagatgacgttgaaccggacaatgaatacgtgaactgtgcgttgacggtttctaacgagctgattcggattaatgacgttgtgtttgaccactgccagttcgagcagagcaactttgacggcagtgattggggctacgtggaatttaaagggtgcgatttcttaaacgcgactttccacaagagttatttctccaactgcaaattcacgaatgtccagctgatgggggctgatttttcgatggaaaccctgcttaagaaatgtcaatttcatgatgctaacctgcactatgccaactttagtgaaactaaaatggaagccagcttctttatggactgtaatctggtcgaaagtagttttcaggcagtgaccgtcaagaaagaattatcctttaacgcctgtgaaattaaccaaatcgacttcttggacacgcgaatgaaggggatcgatttgtctaaagccagctttgacgacttaattgtgaatcccgagttgatcaagggcttaaaaatcaatccttggcaggcagggcagattgtcgctatgctgggtgtgattgttgtcgattagctttaattaaatattttctgggattccttcaatttcgagtggcagctgatgatataataatcactcagggtcaacatcgatttgaaaggggacgtccagccgtgaataaattgccgacacgaatgacatttttttatcaacttcatccagtcgtttcggcagtttatttttttgaggcgattttgagtctgctcttgtttaaccatttggcgacggcattgaccggttatgtaggattactgttggtgggcattttttataccggacaatcagcggtctggcggcaattcaagtggaatttgagcttattattgatgattgtcttttttaatgtgttgttaaatcaacggtttgggccggttctctatcagttttccgtgggtgatgtgtcattcaaactcaccttgccggcacttctatacggtgtcgttatggggttgatgttagtcgagatgctcatggcttttgctgttctgaacgtcattttaccggcgcctaaattggtatatgtcctgtcaccagtgacgccgaagctgggcttattagtggttatttcaatgaatttagtgaagacttttagccacaccctggctagtctggcgatgctccagcagacgcgaaacgttcaggctaacgctggcgggttgcttagtcgcatccggaatgctggtcgcctgttgcggattttattggaggacgcactcgcatcggggatggaaacggcccgattaatggacgccaggggattcggggttggcaagcggactcattattgggcctaccattggaaggccagtgactgggcatttttgagcgcgtcgatcttgatttttgtctgggccgtggtttcccgaattcagtcagccggctggtcgacatcagttggcgaattcacccgtggctggatgagccaggatctggttgccttatccgggctgggaggattactattattaccgctggcagccgaaggagtgtatcgtgcatggacaaattaattgaaaccagacagctcacatttacatatccggatgcttcccgcccagtcttgcaaggagttgatttaaccatcaaccgaggggagtttatcgtcatcgccggggcaactggcagcggtaaaaccacgttaattaatcatttcaaaaaagaactgctccccaatggccatcgaagcggcaaggtattgattaagcagcaagccattacggatctttccagattagccagtgccaaaacgattgggtacgttgggcaagatcccactactcagccgattatgacaacggtgattgacgagctggcgttcggccttgaaaatatcggtatcaagagcgctgaaattgaacggcggatcgccgaattagctaattatttgggcctggacgaactgctgcaccaagatatgcatgaactttccggtggtcaattgcaactggttaatttggcctcggtgttaattttgcggccggaagtgcttttgttcgatgaaccgactgcccaactggatccgctttccagccggcatttttttgatgttttggaacggattcatcaagagttgggaatgacgattgtaatgaccgagcataacttgggaaccgcattgggattggctgaccggatgatcctcttacaaaatcagcgggttacttttcaagggcaaccggtagttggcattccgaagatgatggcagatcccgatctgacagcttttgttccagctgtgtcgcggctatttttggataatcatcttgagacaaccgggctgccaatttctgttgccgccggtcaggcagctatcagcaagcaccacctggagttcaccgctcacacggaccagccgagggtcgtcgagtcgtcaacgaccatcttggcagccaaagagatctcgttttcattcgacaaacaggtaaatgtggttgatcatttgaacttgcaattacctgctggcgactggctttcgattgtcggcaagaacggctctggcaagtcaacgctgttaacgatgctggccggtttgcgagttccacagcatgggaaaattacttttaacaatcaaaaggtctggcggattccaacagcagccagaatccagcagctttcttttctctctcaaacgccggccctgcagtttggtgctgaaacggtccaagaggagttgcaccagcaagctgccgaacttcagctagaatttcctgacaaacaggttaaaatgatagttgaccgattgcacctcaacgatctgcttgaccaaagtccatttgatttgagcagcggccaacaacagctgttagggattgccattgcgctgttggccaacccgcaattgttaatcttggatgaaccgactaaggggcttgatccgacggccaaacaagctttgggacagttattgacgaccatcaaccaggctggaacgaccatcttgatggccagtcacgatatggaattttgtgcggcatactcactgcactgcgccttcatgtttgacggccatttgaacacagtcttaccaaccagatcgtttttttctgggaatttcttttttaccaccgcgattaatcggctgctgagaaggcaggtgcccgatgcaatgctggtgagtgacgttagattatctgaagggacgagtgaacatgtcgaataagtggcgagccaaagtgatcggtcaaatattgctcgtctcggtgttgatcgccgtgtttttgggattaacgctgttactgaaaaataagcattttttgttgtttagcttcatgcttttgttatgtagtattttgccggcctattggcggtttgaaagggaacccctgaagacgcaaacgttgatgtttttggcaattctgattgccttggcggttgccggcagagtgccgttcgcctcgcttcccagtgttcaggctgccagctttgtcattatcctcggcgggatttcgctgggaccggagctggggtttgtgaccggctcgaccaccgccttagtctcaaatatgtttttgggacaggggccctggacaccgtggcagatgtttgcctggggattgatgggcttgacggctgggttgattggccggactcagcttagccaccggctaatgccaatgattatctttggcggtgtctggggatttgtctacggctggatcatggatctgtggtttgccttggcatatgtcaatccgctgaccatgaagtcctttattttggcctttaccgccagcgccggtttcgatcttgtgcactgtctttccaacgttgtcttaattgcattgttgtatcgttcctgggaaaaattaattgaccgactgaatcggaaatataattttttaccaaccaaaactcattaaagggatggaatctatcatgaaatcaatcaagaaattaatcaccttatcgatgactggcctcttattggctggtgctgctgcaccgctcacaaatgtccatgctgccggcgccaagactgcttctagttcctatcaggcttcaaaggccaaggccagctacagctatgccaagaagatgctggctaagaatcgaactgggttttccggtaagacaagttacatatttagtaaaaaggcgtatccaacaaccggtgccgtctatggctactcggactttctcttgggattgaaagggttgggatataagtttaccaatgcccaacggaccaagattgctgacagtttggtattgaaccgtaagagtacggctgccgatttggcgaccgcaattattgccacccgtgccgttggtttgaacccgcaaaagctgcatcaaaccggcgctaaaacgaacttgaacctggtcagcgcgctttatcatcgttcgatggccaagcaaacggtcaacgttcaaagccaggcgctgatcgctttatcaactggttcgtatcaacgaccaagcaatgccaaattttccaaggccagcttgagcaatgccatcgttaagaatcagttgagcaataatggttgggcgtacaataaccaaactgccagtgctgacagcgacaccactgcgatggcagtaacggcccttgctcgtagtaaatcgaccagttccgccgtcacttctgcaatcacgaagggccagagttatctcaaagatgctgtctatccaaacggggcgtttggttacgcttataagggcaagaccttcccgaacgctaattcaaccgcagaagcgatcattgccttttcaaccaaacaaaagacggttaaattggtgaatagcgtcttcaaatcaggtcagacaacctcaccaatgcgggcaatgttgagctacgttcggtcaaccggctcgattaaaggagctgccactcaaacgttgggagtcggtcaggtcaacttggctaacgccgcttaccgtcaagccttagcacaccgatcggtttattcaattaagtaagattaaaggatgagtttatgaaaaaagcaattggaattgtcatcggtgtgattttggtgttggggatggcatttggcgtcagggaggtcatcgcgaatcaggtcgcccagcatcctcgaaccgagaaagccgctaagatggattctggcagtcagccaaaggccacctcaagttctcaggtgagccatccagctaaggcgaaaaaagccaaagacaaaggttcccaggcaaagcatcaatcacaagccaaaaaggccagtcaacctaggactgccgactcgtcaagtagtcaagctaccagtaacaagcccagcagttcaaggtcgaaatcacagacaaaacaggcagtaaccactaagcccaaatcgacttctaagcagtcccgaccaaagcaaaaagcctcaccagcatcaactggtaaggcttatctaaaggtttccggatacaaaaagctgttttattctggcaatttgcacattactaagaagacgactgcttttacattgctccagcaaaccaagctgaagatcacttacaccagtagcccggcaatctacgtcagtgccatcaatggactgaaagaaaacgacattaaggtcggcagcggctggatgtactcggtgaacggcaagtacgttgataagtcagctggtgataagttgattaaaccgggagataaggttcattggtactttacaacggagggattcaagtagagcgcgacgagacccggttaggacccggagcataagtgagaacaatcaatgatgaacggtttttgttcatcgttgattgttttcgcttatgtagtagggtcctgggtcgtcggagcgtgttttcaaagtagaagggagcacaaaagggaataacaaccgtgcccagagcgcgacgagacccggttaggacccggagcataagtgagaacaatcaatgatgaacggtttttgttcatcgttgattgttttcgcttatgtagtagggttctgggtcgtcggagcgtgttttcaaagtagaagggagcacaaaggaggataacaaccgtgcccagagcgcgacgagacccggttaggacccgccaagtaggctaggccgttttcattcggtcgtcggagcgtgttttcaaagcagaagggagcacaaaggaaaataacaactgtacccccagcgcgtcagaatccatttcaaagcaaaataaccctaactacaccactaaaaaaccggcagcaatgaacgaaatttgttcatcactgccggttttgtgttatcaattattatcggacttgagcagttaaagcagtcaaaaaatcggtgacatcaccaacgtaggcaaagtctgactcatcgaaaatcggggcgtctttgtcaatgttgacagagacaattttcttggcatttttgatgccaaccgtgtattgaacagcacctgagattcccaaattaatcaacaggtcggctgagaggctggcgccaccaatcccaatttgatcatcatgggtgaactcgtcttcgtcagtgagagggcgagaaacgccaaccattccgccaagcttggcagctaaatcctgtgccagttgaatattttttgcgctgtaagcgcctcggccaagggcgatcacgactttagcatcgtcgagtttggaggagctgttgatgatcgggtcagtggcgatgatttggctgtttccttctttgtggaaggtaaagctggccttaaccaccttggtctggaaatcagtcaccttttcagcgcggaaagtatttggccgaaccgttaccatttggggccgcttttccgggcagacaatgtcacacatcacgttgtcgccataggtcggtttgacctgaaccagtaggtcattttcgtaaaaaatatccaaacagtcaccggttaagccagtctggagtttggcctgcagccgcggcgcaattgatcggcctaaaatggttgccggaaacaagaggctgttggggcgattttgatcaagtacttggaataaagcatcagcgatttcttcatcggttgcgttagtaaagtgatcatcgaccaaagtttcaactcggtcgggtccataagcttgtaggctattttcagccttgattgtcgaggcttcaggaagcacggcaaccacttttctgccgtcagcaatggctttggccttggtgattaattgcaggctggttggttcgattctggagccgacggtttcaacatatacccaaatttcgttattatccatttttgtgctcctctcagtccaattgactcaagagttcagaaactgcttgagcggggtctggtgacaatgtgactgtttttttaacatccttggttggtgcataaactttggtcactttcgttggtgatccagcctggccaatttttgccaggtcaagattcaaatcggcttcagtccaaatggtaattggcttttcaaaactttctttgatattgactggcgtttcataacgcggcgtattgagttctttgcggacagtcaccacagcaggcagggtcagcttgatatcctggacggcggagtcaagttggcgtttggccaccagtgtcttctctgagtccaactccaaggtttctgcaaaagtcacttgggggaactgcaagaattccgccacaatcgggccaacctgaccagtgtcagcgtcgacagattgtctgccgaataggactaagtcgacatcgccaattgcttcgattgctttggccagcgtgtagccggtagccaaagtgtcagcgccaccaaacgcccgggagctcaccaaaacagcacggtcagcgcccatagccattccatctcgaagtgaggttgtgtaactatccggccccatactgagaaggataacttctccaccggcttgatcacgaagctgaagggcagcttcaattgcatttttatcaaatggattaataatgccttggattcctgaacgaaccaggttatttgtgtttggatcaattttaactgaatcggtttctggaacttgtttaatcccgacaacgattttcatagtgcggactcctttacttggcaatctctgcgttggtaatttctaaattcatcttttcaatggtaccttcagccaattccattgctcgggcatctctgatgaggtgttcgactggatattcatggctgtatccatacccaccaagaatctgcagggctttatcaccggatgcaacagctgatcggctgccgtacgattttgccatggcggcaacttccgcatatggcttgttggcgaccttgttatcggcacctttttgatacagcgcggtggtgttttctttggcaattgcgatatcagcgatcttttcctgagtgacttggagttggtagagcggtgtgtccatagcttttcgttctttggagtagttcacggcggtttgtagctcgtgttccataatcccggcgagaacggcgcccatcaacactcgtgcgtcagcgtgggcattgtcgccaatttccaatccttgtccgattcttcccaataaatgattatcaggaacaaccacgtggttaaggacaacttcgccgacaggcacgcccttgaggccaataaaatcttcccgcttgccgaatttgaatcccggcatgtccttgtcaacgacgaagacggccatttggtcatcctcagtcttagcgaggacgcagtagacttctgcaaggccaccattggtaatcatgattttgtcaccggtgatcacccagttatcaccctgtttgattgctcgagtggcgatgcccttgggattggagccgccggatggttcggtcatcgagaaggcaaaaattcgtttggctgcactcgggaggtactcgtcattcaatgatttattcccatatttgataaactgttcgatcgttttgaaatggccttcaagagttacggccatgctggcgttacctgtggccattttctcaagggattcggcagctgcttggtaatcaaaggctgcaccgccatattctcttggcagggtgatgccaagcaagcccgtgttaacgaccttttgaaataagccgtccggatagtcaccagcgcgatcaatctgcatatcgatcggtgccaattcgttggcggtaaactccttaatcatttgaatcagcattttagtttgatcatttgttatcgacatattgagtcctcctgtgcatactttcacaatactttatattccaaaattatatatcctaatattcccaatgtcaatgtataaatggaatatttagcaatcttatttggcgtcacattatataatatggtaatattaagttattattttatccgaatcggccaggaggcttgataatagtgaacatccaaagatttattgatcgcagaaaagaactcggttattcccaaagtgaattggctaaggggatttgtacccaggccacgatcagcaaatttgagaacaacggcaaaatgatctccactaagatcctgacgcagctatgccagcggctgggactttccttgaacgatattttccccagcgaggccgacagtgattcagccgttcgagcggaattgcggcgggccgaatttgatttaattaccactgaatatgatgatgcgttgggaattttacgatcactggaaattgatcaaattggtgataaacaaatccaaatggaatatttgtttatccgcggatatgccctggctttaagcaaacgagatgttgatgaggcgattttttgcttcgaccagattttgaatggctatgacgaggcccacacgacggtttattcaccgctggcatacgtggggatggggatttcctaccaacaggctggcaattttgacaaagctgagttttatttttccaagatgccggaaagattgaagaccaatgcgaataaagacgttgattcggtgtggaagtcattgacgatgctgttttacaccggcaatttttatgcggccaggaacgaaatcgagatcagtaatatgctgctacagtctttgattaatctcagttcggatcggcacgtaactttttacgtggctcaggctcagtatcaattggcggataacgaatattcggtcaatggcaaaacccagcgattctccgaacttattagtgacgcctttgcgttcgcccgatttaatcggaatcggaatttaattaagcagattgatttgtatgctaaaaaaagagtgtagagtgtgaaagaggacgtttagcaattgaaatttaagcgccgctggacggaaaccgagtcaggttttcggctggcggcgcttaaatttcaattgctgtcctctttcacacgtttaatcaaaataacagtaaaacaccaggaaaccgagtcaggttttcggctggcggcgcttaaatttcaattgctgtccttattcacacgtttaaactaaatagcagtggagctaaagagaggcccagacataacttacaattagttgtgtccgggcctctcttttcgtcaaatattgttttcgcaattgctgaatatcgtgattcgacaaatgcatttgctgatgtaaataatgcttcattgtgccatcacagtggtaaatcgctgaataggcggcattcaaataggctgatcgagcggtttttgaacgtttcaggttcctgagcacggttgggttatgcgtataacgggccatctgtcgatattctttggccgtcgttttcttcagataatggttcgatgccaaatagtttttcataatggtcgttttgggaacgccaagacttgaaagaatcagcatggtcgctacaccggtgcgatctttgccatatgtgcaatgatacagaatcgcaccggatctttgcttgagcagataatgaaacatcgtgcgataagccttaacacagtggggctcaagaaccattttctgataaaattgttccataaaatttggctgtttggcggctaactgaccggcatactgagaagtcgtgtggacgccgaaatttgggctgctcatgacggataggtggagatgacgaaccccagaaattttggcgtctggtgttcgtttgatttcaccacttgagcggaaatccaagatgaccttaacgtgctgcttcttaagtagccatttatcgtgatgatttaatcgggttagcgcagccgatcggatgagtcgattttggcgaatgtgctgaccatttttcgtccgaatcccaccgagatcgtggacattgggcgtcgtcgtcaagtgaatggtggcgcctagggaggaagtggtgttggcagaacaaaccgcaaaattagcagtgagtatcactgtcactagtaatgtccgactcatgatttggctcaatgacttcatccactcacccccaacattcattataggactgggcagtcatcatgacagaaatttttggatgtgggccaaatccgcctggcgcttttgtggtgattcatcttcagcgttgaagttgtgccacttgattttcttgagaccgatctttttgaatgtgcccgtggccaaggccttcataatgggattaccatatttgagtttatagagaaacgttggtgtgccagcaattgtgaagatccggatgattggattcttttccaggaccactctgggatgcatggataccgcccggttcttgctaaaaactttatcaatgaaacccttggtcatcgccggcatcagctcccaccaaattgggaaaataaaaataatttcatcggcggtttttaggcgttcgaaataacggtcaacttggtcattaatcggtgtccgtgttcgccaggcactcaggtcttttgcgtgcattaccgggtcgaagtgatcgtgatttaagtcgatgacatcaacgtcatggccttgggcagttaaataattgatcgtttgtttggcaaccgctgcactataactgcgatggtggggctcgttatttgcggccgacagggtgtaagggtggtcaaatataatgacatatttcatgttagaaacctctttttaaaaattgacagtttgacttttcaaaatacattccaaggaatataattagtataagctccaatgatgaaaagtcaatatatattccgaggaatttaaaatgaaaaagaaaaatgcaattgaacaaatcaagaaccaactagaaatatttagaagtcatgatgttgaccgtgagatcctggcagccatcagacaaaacgatcggttaaacgctgctctggccaatggcatcaccattaacgatctgcatattattcgcgctgctgctgccaaggatggtgtgaagatttccgcgattgtcgaccaggtaccgatgacacaaggagccgtttccaaagccgttaacaagttggctgaaaggggtctgcttcaaaaatcgcaccaccctgataaccgcaaggacacgtttgtagaactcacggcgcctggggaaactattaatcaaattcatagcgactaccatcgtcaagaagagaccaaactggctgagttagccgacagttattcaaaaaatgaactggagatgattgcagaatttgtcaccagcctcaatcaaatccggcaaaataattccaaattaaagtaaccggtttcttctttgctatatcaaaaactcctgtctactgcttataaaaagaaagttaggtttccctaattaaagatttacaagtctagaaactatgctaccattagatttgtacagaagataaggaggtaatgggatgtcaaaagaaaaaaagtcccaaaaggaacatttgattcattacgccaatgggccttcactggaagaaattaacggaacggtggttgtgcccaaaggcaagggattctggcgtacgctatttggttattccggtcccggcgcgttagttgcggtcggttacatggatcctggtaactggtcgacttcaatcaccggtggtcagaattttgaatatctgttaatgtctgtcatcttaatgtcgagtttaattgccatgttgcttcagtatatggcggctaaactgggcattgtgactcagatggacttggcccaggcgattagagcccggacaagcaaatcgctgggatatgttttgtggattctaaccgagctggcaattatggcgactgatattgccgaagtcatcggtgccgcgattgcgttgtatctgttattccacattccgttggtcatttcagtatttattaccgtatttgatgttctgctattattattgctgaccaaaattggtttccgtaagattgaggccattgttgtttgtttaatttgtgtgatctttgtggtgtttgcctatgaagtgatcctgtctgatcctgactggctcggggtctttaagggcttggttccaaatggtgagaccttctcttcgtctcctcaaattggcggtcaaacgccactgactggtgcacttgggatcattggagcgacagttatgccccataatctgtatctccactctgctgtttcacagactcgtaaggtggatcacagtgatgaagaagatgttgcccgaaccgttcgtttctcaacttgggattctaacattcaattatcaatggcattcttggtgaactcactgctattgattatgggagttgctgtcttcaagagtggggcagttaaagatccgtcattcttcggactgttccaggcactttcggattcttcgaccttaagtaatggtgttttgattacggttgccaagtcagggattttatcgattttgtttgcggtcgctttactagcgtcaggtcagaattccaccattaccggtaccttaaccggacaggttatcatggaagggttcatccacatgaaaatgccgctttggatgcgccggttggtgactcgtttgatttcggtggttccagttttgatttgtgtgggtatgacgggtcgtgaaaccccgattcagcagcacgaagcgttgaacacactgatgaataattctcaggtcttcttggcgtttgccctgccattctcgatgctgccgttattgatgtttaccaataactcgttggaaatgcatgaccgtttcaaaaactcgtggattgttaagattcttggctggttctctgttatcgccctgacgactttgaatatgaaaggtcttcctggccaattcgaagcatttctaggtgatcatccaacccagagccaaatttcaatggctgataatgcctcgtacgtcgttattgtcttggtcgttgctttattggtatggatgatttgggatatccacaagagcaacaagcgttttgaagcagcagctgccgaagctgaaagcaaagcagccgaggcggagaaataatagtataataatcaattgaaagagatttcttttgtacccaaataattcatcatcaagaagggatgttacaaaatggcaaatactgaaggcggtcaaaaattcgatcgaattcttgtgggtgttgatgattcggaagatgcccaattagcatttagatatgcaattcgtgaagctcgtcaatccaatgcacgtttgatcattacttcaattttggaggacgataacgttaacgttttccaagcattaagcaaagattttgttcatggggagcgttcagcgcttgccaagcatattgaagactatcggcaattagctttgcgtgccggcgttaagcaagtggatacggtcatcgaagaaggcgatcccggcgagacaatcgtcaaacgggttattccggctaccaaagccgacttgttgatcgtcggttcactttctaagactggtgttcgtaagtactttggttcccaagcagcctatatggccaagtactcaccaatctcagtgatgattgtccgttaattggctttaaaaatgattttaaaacaggatcgggaagaatatttccggtcctattttgttagacactagggggaataatcttggagttaacagaaaaaagccgtaggtggttcattgccacattactgctgggaacatttacgatgtcaatcagtcagtcgtcactatcgactgcctatccgacatttatgaggtattttgatctgccggccagcacgattgcttggctgacgacggggtttatgctgatcatgtcggttgtcatgccattatcaccatggttgatgaagaactttcgatttaagccattatatctttcattattggtaaacttcgttgttggaaccttgattattatctgggcaccgaatttcctggttatgatggtgggtcgattaatggaaggattcagtgttggggtcttatttccatcttatcaatcgatcatacttgaaatcacaccaaccgatcatcgtggtagcgtgatgggcactgtggggttggtcatgggatccgcactggctgttggacccatcatctcgggggtcttattgcaatttttcccgtgggaagccatctttgcgttcttcttgattattctgacggtggtctttctgttggcactcaagaccgtcattagtccgttgaaaattgaatcaactcagtttgattttgtttcagtcttcatgtcgctgggacttattggcttattgtactttatcaacgaaatttctcatatgactgccactagctactggaactgggggattttattggtttccttggttctgctggtcttatttgttcgccgacaattgcgcatgccacagccattattgcgactggatattctgtcgatcaccaactttgatttgggagttttattaacttcattgtcctatatgtccttgatcacggtcaccattatcatgccgctatactaccagcagatactgggattgacgccgttatggtcaggcctggcactggttcccgccgcagctattttgtcctggttaaatcgacggagtggccggctggcagatcgcattgggtttaagccagttattatgattggttttggattattcatcgttggctgggcaggtttattgttgctatcagggttgaaaaatatttggattgccattctatgttcgattgtaattgaatctgggaacgcctttgccatgatgccggccaccacgctgggagccaattctttaaccaacgatttgattccccacggctcttcgattattgcgacgattaggcaaattttggggtcgaccgcgattgtcattgcgacagttgtattaggagaccggaatttcaacggcgtgttcctcacctttctcattctggaagtcattgccattttcttagttttcaaaattaaggatacgcaacaacaggcgggcaaagcttaatttggctttgtgaaatgaaaactattttcacgagtgatatacgttaactgttgcgttcgttaaccactttgaaaatcacaatgcattttgttgtatctgttttcatggcatgatatcctatatctggatgtaaaaatgtctaggatagctgaagacgttacagatttatccaaattttaggaggtcatataatggcatatcggactgtaaacccttacaacaatgaagttgtgaaggagtacccatttgcgactgaggacgaattacaatcagccttggcaacgggtcatgatttatacgaaacgatgaagaagcaagatatttctgagagagctaaaattctgcataacgttgctgcgaaactgcgtgagcactcagatgaattagctcgtgcatgtacgattgacatgggtaaattaatcggtgaatcaaagggtgaagttgaactggttgcgatcattgctgactggttcgcagatcatggtgaggacttactgaagcctgaaaagatcgataccattgcaaccggtgatgctgaaattcaacatcacgcaaccggagttgttatgatggttgagccttggaacttcccttactaccaaatcatgcgtgtgttcgcacctaactttatggttggaaatccaatgatcttaaagcacgctgccaacacgccaacatcagctaaaatgtttgctgacgttgtcgccgaagccggtgcccctaaaggttcgttgactaacttgttcctttcatacgaccaagtgactgaagcaattgatgaccctcgtgttcaaggggttgccttaactggttccgagcgtggtggtacagctgttgccggcgccgctggtaaagcacttaagaagaacaccatggagcttggtggaatggatccatttgttgttttaggtgatgccaacatggatgatgtcaatgacattgcatggcgtgcgcgaatttacaacactggtcaagtatgtacttcatccaagcgattcatcgtgatggacaatgtttacgatgaatttgtggagaatttgaagaagaagtttgctggtttgaagcctggcgatccaatggatcctaagacgaccttagcaccaatgaacaccgaaaaatcaaagaacaagttgcagaaacaattggacgatgctatcgcagctggtgccaaagttgtttatggtaatgaaccaattgacttacctggtcaattcttcatgccaacgatcttaacggatattgacaaagataacccagcatacagtgaagaaatgtttggtccaatcgctgctgtttacaaggttcacagtgagcaggaagcaatcgacttggccaacgacaacccttacggacttggtggcattgtctttgccggcgatgctgatcacggtgcagaagttgcctcacaaatcgaaactggaatggtctttgttaacaacttcatgtccaccttacctgaattgccatttggtggggttaaactttcaggttacggccgtgaaatgagccacattggtcagatggcctttgttaacgagcagttgatcgttaagactgacaagcctaacatgggtaaccttgccggtggtttggttgcacttgatcctcaagaataatgaacgtgaaataaattgactgaaaagtaaagaagtcgggagataacgttttgttcgttatctcccggcttcttttgcgtgccattgttattttgtttaaatcctaggatcaagattcttcgtgcgatgctcttggcacaattacctgtaaaaagtcacttttggttgtgacggtaattggcagagacatcgctggatccccatcgattctggcctgaatgtcgcgttttgacaggttatcgattttaacggttttggttttaaaatagcgaaccccctgggcatttttgagattgccggtgatgaaataactcaagtaggtgagtagtttcatgggagtgaagctcttcagcaagaagacatggagataatcatcgtcataagacgcatccggattaaaggcgatgaacccacctaccgaattggtcgtcgtgatcagtagaatctgggcccgcaagacttcggagcgatcattggccgtgatttttaatttgtaagaacgattggtgaacagctccttgaagcctttgaccaaataaatcattttgccaaagcgcttcttttcgtcgtccttgacgtttcgagcgatatctgccaatcttcccagggtgaggctgctgaccattggtgttttccccacagccccgaggtcgacctctgctggtgagccatccaacagattgttaatggcttgatcggtgttcagggggatgtgaagggctctggcaaaattattgatcgtgccgccaggaatgattcccagcggaattgattggccagccttcaagaagccctcacaggcggtattgatcgatccatcaccgccaatcgtaatcaggcagtcatagttttcgggtgatttttgggcctgtttgaccgcatcatcacgtgacttggtttgactaagggtcaccgacttgccattactttccaataaggattgagcttttttggcaatcgcttcgttgtcgcttttaccggcactgccattataaataattaaatattttttcatgttgcacctcctcaaaggaatgattcggatgacaactttattatattacgcttttggggaatggtcgtctttggggattatggttaatgatccgttcatgaccggtgatgttgcatcaacagtgtggaggtccgtgaaaatttgaagaaatttcatgaaactttcagctgtattagcttcattgaggtcctttaacggcagccaataattttgaccttcctcagactgcttgagggttcctgagaaatgactggtgcggtagagaaatccgagtcggcggtaggcaggactttcgttgaaccattcgacagttccacaggattcgagctgactgaccgtcaggccggtttcctcaaatacttctcgaaccatgccgtcgtaaagactctcacctttttcaacgtggccgccgggaaaggtgtggccaaatttccagtcgacgtcggttttatcttccaccaagacctcttgagtggctggattgtagatcatgcacatatttaccaattcgattgattcggttctggaataggtcatttggctgcctcccgctcaacttcttcgttgacactgaattgtggagtcactttaagggctttgatccgattctcgccccattcatacatctgattggcaatgggcatcagcgattgaccgagctcggtgatttcataggtcacctttgtttgagatcccgcgttgacgtgcctggtaatgaggccgtcttcagccatttcccgcagctgattggtgagcactttgtgggtgactttgggcaacagccgcattaattcgttaaagcggtaggcgccgtcagttcccaagtgaaataagatgaccaatttccatttgccgctgaacatcgataaagtgagctccttggaacaggtgtagtcaccgtttttcagacggtctttgacatcttttctgatgacatcagtcatttgtatccctccaagattttaggcacctgaaagtgcgttattgtatcattttgatacctagtataaagtagatagtatcttggaacaagaaaggatgaatttgatgagtaaagtagctgtcatcgtgaccaacgatgttgaagatattgaatacacatcaccggttgaagcactcaagaatgccggccatgaggtggtaaccattgaaaatgaagctggcaatcaaatcgtcggcaaacacggcactaagttgactgccgataagggaatcggggacgtgaagccggatgagtttgacggcttattgatccctggcggcttttcaccagatcaactgagagctgatgatcgatttgttaatttcgtcaaagactttttgatggacgacaaaccaacttttgcgatttgccacggtccgcaactgttcatccaaaccggcttgacggctggtcggacaatgaccgcctacctgaccgttcgaccggatttgtattatgccggcgcccgcgtgaaagaccagccggtggtggttgaccgtaatttggttaccagccgcactcctgatgatttagacgattttaatggtgccatgctggctattttgaagaagtaattgaatttaaagtaacttgactgcaaaaagaccggaacaaggcgattttcaacgcctgttccggtccttttgctttttatgttatgaatgtctaactcaatgcaaatgagggtccttattcgtatccagtccacctaactggcctctgaattctttggaatacaggttcaaatctgaacggtaggcgtcaagattgtcgctcatgtcaacggtataatcaacttcttcaccgtgctcacctttatccaaaccaagcttttcttctttacggtcaactcgcattggcatcactaaactcagtaatttgataatcactgaagccgcgatggtaacaaagataatcgttgccaaagttgcgacgatctggacggtaatttgatgccaaccgcccccataaaaggcgccattgtgggcaacaatcgggttgacgctcttggtagcgaacaaaccggtggcaatactgccgatgatcccgctgacaccatggcagccaaaggcatccaaagcatcgtcaacaccgattcgatctttcaaatagttaacgaagaagtagctggcgaaagttgagaacatgccaatccaaaatgatccggcgattgttacaaagccacaggcaggggtgataccaactaacccacaaagcgttccggtacaaacaccaaccagggttggtttgccgctgataatcatatccaaaatcatccaggtaaccattgcagtaccggttgacatggtcgtcgtaatggttgcctgagccgcaatgttgtcaacaccgagtgctgacccggcattgaatccgtaccagccaatccacaagatggtggcaccaagcaatacccatggtaaattgtagtgggtgtgagggatgtcgccgaatttaacccgtttccctaagaaagcggaaaggacaaaggcagtgacaccggcattaatatggacaacggttccgccggcaaagtccaatacgcctaatccataaagaataccgtgtgggctccaaaccaaatggaccattgggtagtaaatgataatcgaccaaagaatcaagaaaaccaacaagaagttgaatttgatccggccaacaacggcacccacgaataaggcaggggtaataatagcaaacatcatttcaaatactgaaaaaatcccagtcggaatcttggttgcagtcaatgaagtcagatcaacgccattcatgaaaaagttcttcacggttccaatgactccgccaatgtctccggaaaatgataacgagtaaccaatcacgatccaaagaacaatggcaacaccggtcataatgaaaaccgacagcatcgtgttaaccacgttgcgttttgaaaccaggcccccatagaaaaacgccaatccgggagtcatgaataagaccaaaatactggataaaatcatgaacgaagtatttgcagcattcataacatcgcttccttctcttttaatgtcataaattctaacatcatatttttggaacgtccagcactttttgaaattggttagaaaattagaatgaatttaatgttgatggaaacggtgccaatggcgttgattaaagcatctttgtcctattaacttccatcaaaaaagttaagccgactaattggtatatgtaattaaaactaacattaaagggccgaaacacaaatgtttcttcactgtgtttcggcccttatgttataccctggattgcgataatctttattaattcaattcattaatggcttctggaatcggttcatttccagtgctcatctcaatgacttctttgatgccggcatggttttcgactaaaccaattaatacgtcggcgacattatcgatactattttcgttggtgctataggctcccaaagtcactttgcctgacccggctttttcaaccagcgcggttggctggaggattgtgtagtccagattggtgttgtgaatcaaccattcatcggcatagtatttggcgatcaagtaattctcaagcggagagtcggcgaattcgtctggtgacaatgatcccttggaactcagcatgacaaaacggctgatttctttttcttcggctgcctgcatgactttgacggcaccatgtaagtcaattttaagcaggtctcggccacccgatccggcagtgaagataattgcatcggcttctggtaaggcctctttaatctcatccatcccgttgttgagatccaatttaaatggcgtcacattctctgatgctggcactttttccggcttgcgggcaccagcatagatttcgtctgcagaatttttggccagtttggcgacaacgtttgaaccaactcggccagttgcaccaatcacgataattttcattgttggaatcctcccttatccttattagctcaattatggtagatataaggccggaatgcaaaagaaagattgacattggcttaatctttcttttgcaagtctaacgtcccaagcggggtggatgatttttaaagccatggatagggcgacaactggaatcacgacgactaagcagagttcgatcgctgaaagtttaacgatcgacatgctctctggaaacgccgttatcacgaaccacccaaaaatccaagacaatcttcgccatcaattacccaaacaaaaaattcaaacttgatccacgtcaattccttatcggccgaaccaccatatactaaaggcatcaattaagaaatggagcgggagattatgaaattccaaagatatattaatcaacatacaaatcaaattacactgataacggcagtattaattggcgtaggcctcttggggaaagttgttgacagcgatatggtctacacggtttcattcatcgccgcttcaattatctcagctgtgccgatcgttcttcgggcagtttccgcactccgatttaaaacgatcagcatcgaattacttgtcagtattgctgtgattggcgctttcatcattggcgagtacaatgaatcagcgatcgtcactttcttgttcttatttgggacgtttttggaagacaaaacgttggccaaaacccgccactcaattaaagatttgacggaaatggcaccgactaccgcaatggttgtggatgatgacggcaacactgaggagattgatgttgactttgtcgacgttgacgacgtcgtcttggtcaaagccggcggtcagatcccggttgacggggaaattgtggatggatccggtcacatcaacgaagccagcattaccggtgaatcaaaattagtcactaagggcactggtgatcaggtattctctggcaccatcttagacaacggaacacttaaagttcgggcaaccaaggttggcgatgacaccacgtttggcaaaattgttgaactggttgaggatgctcaagacaccaagtctccggcagaaaagtttattgacaaatttgcgacttattacactccggcagttttgattattgcgctgattgtgggcttggttaccaaagatttccgattagcgattaccgttttggtcttgggatgcccaggggccttggttatcggcgccccggtttcaaacgtggctggaatcggtaatggtgcgaaaaacggtgtcttgatcaagggcggtgaagtgatgaacacctttgccaatgttgacacgttggtattcgataagacagggactctgactgaaggaaaaacggcggttactcagttcaaagactactcaaaagaccagttggccttgcaaattgctgcggcggttgagaaacagtcggatcatccgttggcacaagcagttgttaaattctcagctgatcatcatattccgtttgacgacgttcaagttgccgatgctgacacagtcaaaggccgtggcgttaaggcaactgccaacggtaagaatgttttaattggtaacttgagaatgatgaacgatgaaaatgttgatttgacgtctgaacaacgtcacgacttggaaaacatccaagacgaaggcagttcaacggttatcgttgccttcgacgggcaaattcaagccattctgggtatctcggatgtgattcgtcaaggcgttaagcaaagcctggcgacactcaagtcactcggcatcaagaagacagttatgctgaccggtgataacctgcagaccgccaatgccgttgctgaacaaattggtattgatgaagtccacgcagaacttttgccggaacaaaaagtcgaatacgttaaacaatttcagcaggaaggccacaaagttgcctttgtcggcgacggtatcaatgacagtccatcattggtgaccgctgatatcgggattgccatggggagtggcaccgacgtggcggttgaaacctctgatgtcgtcttgatgtcatcaggactcaatgaattgatccatgcatatggactttccaaaaaaacggtcatcaacaccaaggagaacattttcatcgccattgcgacggttgtcgccctgctgattggcttgattctcggctttatttacatggccagcggaatgtttgtccatgaagccagtatcctggttgtcatcttcaacgcaatgcgattaattaattatcaaccaaaaaccgccaaacttgatccagatcaattatcagttggcgaatatgatttatcattaaaacagtaaatgagatggaggttatcaatatgagtaaagcaattttacaattagacgcgctgtcatgcccgtcatgcatgcagaaaatcaagggcgcacttgaaaagcaggatggtgtggaaaacgtcaaagtcttgttcaatgcagccaaagtcaaaactgattttgacggcgataaaatttccgcagacaaattgtcagacacggtaactgatttaggctatgaagttcaatcaatgaaagtgaaataggtgaagaatatgacaacagcaaccccagaaaaattatttgaagcagaagttaagcaagcagatatcgaccaccataccccaacggctggtgcgatgaccggccacatcgttgccaacttggaagttttatccaacaagctccagatggcaaaatggtatgtgaaggggatgtccgcccaacagctgaaagtcctattcggcgacttacttaagcaggcgtacgaccaaaaggatgccttgggcacggtcttaatcgatgaagcgttaatcacgccaagtacccaaaaggaattcacggagtacaccatgctggaagaaaatggccagaataaatatgaatctgcagagtggctggtcaacgacttcgtccatgactatgacactgagaacatgtttgtcacccgggcaattaagttggctgaaaaagaagaccgcccagttttggcacaacatttgattggcctactgcgagataacaaccacaacattgctactttgcaggccttgcttggaaagacaccacgagagggcttggacgaggaagacgacgaagattaatcattaacctagatacgaaaaaagttccgaggcaaatttgcttcggaacttttttaatatcatttttttcgaattcaaacattcaaacaaatcagcacgataacacaggcaatcgtacttgccaggatccaccagccaacccgataagctgtccgctgataggttgaaatttgctccaaactcaatttatcaaaatccggcatcttaagtgaggcattttgaaacatgctagtctgcagcagcgtaaagtcttttttgatcagaagttgataacaataccagggtcaagccgatgagtgccacattgattgagacaaatattaacaggacgcagataatgatcgcactagtcagtataatccgccgagttctcattttcaccactccttcagggcacactacttcactggacgagtgatggcagattgccatcaagaacaaattaccagagatattcaactggatttttgatgtgttgatcgtaaacgtcacggacaatttgcatctgagcatcagtcaaggcgggcagatccgctgcagtggtgttgcgctcgatttgagttggattgcttgcaccagggatgacagcagaaacggcgtcatacatcaagatgaagcgcaaagccattgcggcaagattatcggttcccaagcgttgcttcagttcggcagcagctttaacgccggtcaggtagtcaacaccggagaaggtctcgcctttatcgaactgttcaccatgccgattagttgtcctgtgatcttctggcgcaaacttggtgtccgcggtaaatttcccggtcaaaagaccacttgccagtggaacccgggccaaaatgccgacgttatttttcttcgctaagccaaagaagagatcggcaggacgaaggcgaaacatgttgaagatgatctcgacagccgagatgtcataactgagggctttgatgccttcttcgacccgctcgacactgacaccgtagttctgaatttttccagcttgcttgagcttgtccagttcaaaaaaggtttcaggcatgtagtaattcatcattggcgggcagtgcagcagcaccatgtccaatgagtcgacacccatgttttgcaatgactcatcaacgtaccggtccaagtgagtcgggtcaaagtgcttaatatccaagggcatttcttttcggccaattttagtcgtgtagtgaacatcaggatgattcctgacaaattcacccacggctttttcactttggccatcttggtagccatcagctgtatcaaagaaattgacgccacgatcataagcttcctcgagtgtgtcccgagcatctttagggtcaaacggggtgccccattttccacctaactgccaggtaccaagggaaacctcgctgacactataaccagttttaccaagtgttctgaatttcattagtgttacctccaaatagcaatccacttgtttcaatcataacatctcggttgatactttgactaagcgtatttggtggtggacaggtccacggtcgttaaaaatagtccatcttttgaaacttggacggctccaaacacgtaaattaatcaaatatttttggtaaaagttgcaatatatcgttttaaacacgaacaatggcgttgacttccatgatgatggcaagtatcctatagacactaaataaatttgaaaaggtgagtggttggaatggcaaacgttgtcggtgtggcaatgggatcaatttctgattggccaacaatgaaactggcttgtgaacaacttgaaagtcttggaatcccttatgagaagcacgttatctcagctcatcggatgcccgatgaacttcaagaatttggcaagacagctagggacaagggcatgaaagttatcattgcgggtgctggtggcgcagctcatttgccgggaatgattgcagccaacacgacacttcctgtcattggagttccgatgaaaacacgaacattaaatggtgttgactcattgctttcaattgtccagatgccatttggggctccggtcgccaccgtcagtattggtgaggctggtgccaagaacgccgccttattggcagctcaaattttaggaacaactgactcagctatcgcgaagaagttggctgatctaaaagaaacccagagagtggaggccaaaaacagtgagcagcagttcgattaaaactatcttaccgccagctacgatcggcattgtcggtggcggccaactcggacagatgatggcactgattgccaagtcgatggggtatcacgtgggcatcttagatccaacacctcacgctccggctgggcaagttgctgatttccaaatcgttgctgaatatgacgacgttgactcattgatgaagttggctgaacaaagtgatgtgttaacctacgaatttgagaatgtcgacgaagattcgctgctcaaggcaaagaaggtggctgagcttcctcaaggcgtcaacttacttcatatcaccgggcagcgattgaatgagaagaattttatcaaggattgtgggattccggtaaccaagtttgccgctgtttcagatgaagcgtcacttaaagctgccgttgacgaagttggctatccagcaattcttaaaaccgtttctggcggctatgatggtcacggtcagatggatattaattctgccgctgatctcgctgaagcgtcgtcactgtactccaaagcggaatgtattttggaagcccgccaagacttcatcgcggaagcctccgtcatggttacccgggatttgaatggcaaagtgattaccttcccactggttgaaaatcgtcataagaatcacattcttcataccacaattgccccaggcagattttccaagaccgtccatgccaaagcaaaacagtacgccgaaaccatcgctaatcagcttaatttatatggggttctaggcattgaactgtttgtaattgatgaccaagacgtcatggttaatgaactggcaccgcgtccacataactccggtcactacacgatcgaagcctgcaacatctctcaatttgaagcacatattcgaagcatctgcggcttgccgattcctgaaattgttcaggaaaaacccgcagtgatgagaaacctgttaggaaccgatttaacccttgcccgcaatctactcaaggaacatccggaatggcacttccacgattacggcaaggcagagattcgaccacaacgcaaaatgggccacgttaccgtcgttggtgacaacatcgaccagttactgaaatcaaccgacattttaaagggagaaaactaaaatgactgaaattgtgaaaaaagatttgttgtataaaggtaaagctaaagaaatgtacacgaccaacgatcctgacaccatgtgggttcactacatggatcaagtaacggcttttaacggcaagaaaaaagttcaaatggcaggcaagggtcaaaccaactgtgaaatttcagccttgatcttcaaggacctcgccaatcatggcattaagaaccactttatcaagcaaatcgattccaacaatcaattggttaaacgggtaaagattattccattggaaacagttgttagaaactttgcttccggcagctttgaaaagaaatttgccgttaagcatttaatgaagttcgataagccggttcaagaattcttctataagagcgatgaattggatgatccattcattaacgatttccaagctgagactttgaaggtggcaactgaagatcaaatgaatcagatgcgggcgattgcacttaaagttaatgaccgcctcaaagaaattttctcagaaatgaacattgatctggtggacttcaaagttgaatttggcattgattccgacaaccaattgattttggccgatgaaatttctcctgacagctgccgattaattgaccgcgatacgcaaaagtcacttgataaagatgtcttcagaaaaggcctcggtgctttggtaccagtatataaggaaattcttggtcgccttgaaaaagtggaggatgttaaataatggctcttgcgaaagtttatgttaactacaagaaatcaattttaaatcccgaagcagaagccgtccataaagctttgaagcgtctgggttacggtgatattgaagacgtgaagttgggtaaatactttgaattaaccattgctgacggcaaatccaaagcagagattgataaagaaattaacgaaatttgtgacaaattgctcgctaattacaacatggaaaattaccactatgagattgttgaaacggaggctgcccaatgaaatttgctgtccttgcttttccaggatccaactgtgaaatggacctctacaatgcaattgaagatatcatcaaagaagatgttgaactggtttcttacaagaacgattcacttgccggctttgacgctgttctgattcctggtggtttctcatatggtgactacttacgaagcggtgccattgcccgcttttcaccgattattcctgcattacaggattttgccaaaagtggccgaccagttctgggaatttgcaacggatttcaaattttaaccgaagccggattactgccgggaagcttgcagaagaacgtttctgccaagtttatctgcaagactgaacctctggtcgttaataatgaccactcgatgtttagctcagcctatcaaactgggcagttgatcagtttaccgattgcgcatggtgatggcaattattactgtgaccaagatactttgcgggaactggttgccaatgatcaaatcgttttcaagtatgccaataatccaaatgggagcgttgataatatcgccggcatcaccaataaagccggcaacgttcttggcatgatgccccacccggaacgggccgttgaagcaatgcttgggtctgatgacgggaaggggatcttccagtcgatcgttaatcacattaaaagtcgaggggtaatctatgaatagtgtaatggatcaaacaactgaagcgacaccagaacaaattcgtgataacaagttgtaccaatcgatgggattgacagaccacgaatatggtttgattaaagatgatgtcttgcatcggctgcctaactacaccgaagtcggtttgttctcaggaatgtggagtgaacattgttcttacaaaaactccaagccggttcttaaaaagttctttaccaaaggcaaacacgttgtcaaaggaccaggtgaaggtgccggtattattgatattggcgataatcaaggagttgttttcaaagctgaaagccataaccacccttcagcagttgaacctttccaaggcgccacgaccggcgttggtggtattttacgagacatcttctcaatgggtgcccgaccaattgccagcatggacagcttgcgatttgccgaaccgaaaaccgatgcggacaagtattttattcaacaaattgttgccggcattagtgcttacgggaactgtattgggatcccgacggttggcggagatacagcatttgacgatgcctacgcccacaacccactgattaacgtgatgtctgttggcttgatggatctcgataagattgaagttggtgcagcagccggcgttggtaacagtattatctacgttggccataaaaccggtcgtgacgggattaacggggcctcgtttgcttctttccaatttgattctgaacatgaaagtcaacgttcagccgttcaagttggtgatccatttgaagaaaagctggtgatggaaggctgccttgacgtcatcaacaatcattcggacgccttagtcggaattcaagatatgggtgctgccggattggtttcatcttcggcagaaatgggttccaaggctggcggcaacggaatggaattgaatttggatttggtcccacaacgtgaagccgggatgtccgcctttgaattaatgctttcagaatctcaggagcggatgttgctgtgtgtcaaagccggtcatgaagatgaagttttgaatgtctttaaggaccatggcgttaacgccgtcgttattggtcacgtgactgaaggccataattacaaacttcttcaccacggtaaagtcgttgctgatgtgccggttgattccctggcgtctcaagcaccggtttatcaccgtgaatcagctgtaccagcacacttgaaaaatgccgatgagaatcagtatcaacctcaaattagcaacccaactgaaaccttgaaagatatgcttggccaattaaccattgcttctaaggaaagtatctatgaaacctatgatacccaggttcaaaccaacacggttgtggctcctggatccgatgccgccgttgtccgggtgcgacaccacgacaaggccttggcaatcacaactgatgttaatggtcgctacctctacttgaatcctcgagtcgggggtgccatggcggttgctgaagctgcccgcaacattgttgcatctggtgccgtaccgttgggaattaccgattgcctgaactttggtaatcctgaaaagcccgatcagttctatgaattggatcaagcagtgatgggaatgagtgaagcatgtgaaaagtttgaagctcctgtcatttccggtaacgtttcccttaacaatgaatacgataatattccagtctatcctacgccaatggtggggatggttggcctgatcaaaggcctggaccacatcacgactcaagactttaagcaagccggcgacctggtttatgtagttggtcaaactgaaccgggatttaacggttctcaaattcaaaaaatgcaaaccggaaaaattgccggcaagctcttcaattttgatttagattatgaagtgaaaattcaaaaattaattacagctgccattcaacaacatttgttgaattcagctcatgacatctctgagggcggtctgattactgctattgctgaaagtacttttggcaatcagcttggcgttgacttgtcaggtaacttaaccgttgctgacttcttctccgaaagccaatcaagatttgtcgtttcagttccacaagaaaagcaggccgattttgacaaattagttggcaatgacgcagaaaagcttggaaaggtagtcgatgacaatcacctatttgtccaagccgatgatggttactttgatcttgatgttgataaagcatttggtatttggaaaggggcattgccatgccgtctgaagtaaaaagtttaaatgaagagtgtgggatttttggcgtttggggaacgcctgatgctgccaaattgacctacattggcttatttgccctccagcatcgtggccaggaaggtgccgggattacggttaataatgaaggccatttgaccaccaagcggggatttggtttgttgaccgacgtcttcgattcacccaacgcggttgatgaaatgaccggtcaagctgcaatcggccacgttcgctactcgactgccggcagtaatttattggaaaatattcaaccgctgccctttaactttagcgatacccaatttgcgcttgctcataatggtaatttaaccaacgccatttcaattcgaaagaacttggaagaccgcggtgcgatctatcattccagttccgatactgaaaacctgatgcatttgatccggttgagccaagaagacaacttggacgaccagatgaaagaagccttaaatatcattaagggtgggtttgcctacttggtcatgactaaggatcgcttatatgctgcccttgatcccaatggctttcggccgctcgttgtcggtcagctgccaaatggtgcttacgtcgtctgcagcgaaacttgcgccttggatgctgttggcgctgagttcaaatttgacgttcaaccaggtcagttaattaaaattgatgcttccggcatcaccgttgataaatataccgacgatactcagttggcgatttgctcgatggaatttatttatttcgcccggccagattctgatatttacggcgttaatgtccattctgccagaaaacggatgggggctcgcttggctcaggaacagccggttgaaaatgccgatatggtgattggggttcccaactcatccttgtcggcggcaatgggatacgccgaagaatcaggtttgccttatgaaatgggcctggtgaagaatcaatattctgccagaacattcattgaacccactcaagcacttcgcgaacagggtgtgaatatgaaactctctgctgttaaaggggtcgttcggggtaagaatttggtgttggttgatgattcgatcgttcgtgggactaccagtcgccgaattgtcaaattactcaaagatgctggggcggcttccgtgcacctgcggattgcatcaccgccgctgcgctatccatgtttttacggcatcgacatccagcatgttcgcgaactgattgccgccaacaagacgattgagcaaatgcgcgaaatcttcggagctgattctttgggatttctgagtgttcaaggcgtaattgattcagttaatttgaagaccgacgcacctaataagggtctctgtgttgcatattttgacggcaaatatccaaccccgctttacgattacgaagaagaatacgatcgcgatcaagcccaactacaatcaatgagatgaggtaattcgaatggacgcctataaaaaggccggtgtcgatattaacgccggttacaagttagtcgatgatattaagaatttatcaaacaataaagaccttggctcattcggtgggttgtttcccttgtcgctgggtgcctatcaaaacccggttctggtttctggaacggatggggtgggaaccaaattgttgatcgctatcaaagccaatcaacacaaaaccattgggatcgacctggttgcgatgtgtgtcaacgatgtgttggcccaaggcgcaaagccgttgttcttcttggattatctcggagttggtcacctggataacgaaaaagccaaagcaattttagccggcgtggtcgaaggggtttctcaggctcaggcaaaattggttggtggcgaaactgccgaaatgcccgatatgtatactcatgggcattatgatttagctggatttgcggttggtattgctgattccgataagcttttgagccctgacaatttgcgtgaaggggatgtcttgttgggacttgcctccaatggtcttcattccaacggtttcagtttggttagagacatcttgttcaaacagaatgcttattcattaaatgatcagctgtccggctgtgagtatgatttgaagcgtgaactgttgcgcccaaccaagatctatgtcaaatcagtgttaccggtgatcgagcagggcaagatcgcatcaatcgctcatatcactggtggcgggttaccagaaaatgttgccagaattttaccggataacctttcggcagaatttgagtatggcagttggcaggtgccggcgatcatgaaggatttgcaagagattggccatttatcatttgatgacattctgcacacctttaacttgggccttggcatggtgattgccgttcatccagatgatgccgatgccgttgaatcacaattaaaagcagctggcgaaaccgtttcacgggttggtaagctcatttctggcgacaaacaagtaatcattcgaaaggatcagcaatgaaatctgacgtaaaaaacatagcgatatttgcatccggtgagggaaccaatttcacagcattgacggaatctttcaaaaaagaacacttaccgctcaatgtgaagttgttggtttgtgatcattccaacgttcacgtcctcgaccgggcacataaagaatctgtttcaacatttgtgattaacttcaaagattatcccaataaagctgccgctgaaacggtgattgcccagaagcttgaggaagcccaaattgacttcatcattttggccggttatatgcggatcatcggccccaccttgttagccaagtatgaaggcaaaattattaatattcatccggccctgctgccgaagttccctggccgccatgggattgaagatgcctatcaagctggtgtcgatacgaccggtgtcacggttcactgggtggattccgggattgattccggaaaaatcattgctcaacgcgaggtgccagtccacaaggatgaccagttgagtgaccttgaacagcggattcatgcgacggaacacgtgttatatccaagcgttgtcaaacaattattagaaagaggagaaatttaatgtcgaaaagagcccttttaagtgtttctgataaaagtaatttggttgattttgctaaacagttaaaggatttggattttgaaatcgtttcgaccggcggcaccaaaaaagccctggaagatgctggcgttgaagtaaccggtgttgaagaagtcaccggttttccagaaatgcttgacggccgggttaaaacccttcatccaaagattcatgccggaattcttgccaagcgtgacgatcccgaccatatgaaacaattaaaagatgccggcattacacccattgacttggttgccgttaatctgtatccgttcaagcagacgattgaaaaacctgagaccactcaagcagaagcaatcgaacaaatcgatattggcgggccatcaatgctgcgggcagccgcaaagaactttgccggcgtgctaaccgtcgttgacccagctgactatcaaccagtgatcgatgctctgaaggcacacactgatgacgccgatttcagaaaacatttggcagctaaagtgttcagacacactgccgcatatgacgccctcatttcgaattatttgacggaagaagaatttccagaaaaactgactttaacttacgaaaagcaacagtcattgcgttatggagaaaacagtcaccaaaaggcagccttctaccgcaaggcgttaccatcaaaactgtcgattattcccaaccagcttcatggtaaagagttatcatacaacaacatcaaagatgctaacgctgcactgaatatggtggctgaatttgatcaaccaacggttattgcgatgaagcacatgaatccatgtggggttggtgtggctgataccatcgaaaaggcttgggatgaagcttatgaatcagatccgatgtcgatctttggtggaattattgccgtcaaccgagaaattgatgctgcgacagcagaaaagatgcacaagattttcttggaaattgtaattgccccatcatacactgatgaagcatttgaaattttagctaaaaagaagaatattcgtctgctgaaagctgatttgagtcatcgagacgagcctgatcgctttgaagaaattactgttagcggcgggatgctcattcaagaaagcgaccatgaaattgatcagattcctgacttcaaagtggttaccaaagtccaaccaactgagcagcaattgaaggctttgcaatttggccaacacgttgttaaacacgttaagagtaacgcggtggttgtaacaacggacaccaagactttgggtgtcggcatgggtcagcctaaccggattgactcagctaagattgctatccaaaaggcaatgccaaaggacggttacgaaaatgctatcatggcatcggacgccttcttcccaatggatgactgtgtggaatacgcagccaagcatgatatcaaggccattatccaaccgggtggcagtatcaaggataaggattcaattgcgatggctgataagtttggaattgccatggtgatgaccggggtaagacattttagacactagaagcagagggcgacgagccccgggtgtccccggtgtgtaaggcggaaatttaaaggatgaacgggctttgttcatcgtttgaatttttggcttacacgttagggggcaggggcgtcggagcgcatttcaatcagagcgcgacaagggctgggtgacccggtttccaagggtactttgattgaagtccctgggtttgggactttaatcaaagtacccttggaagttaggggcaggggcgtcggagcgtattttaaaggccgaagggagcacctaggaacctaataagcgtgcttcaagccctcgttgttgctcagtggagcacatttgactaaaattcttaaagcatcaaactatccataccgttcaaagaaaaaatcaacaatgtacaacaacgcacaacaaggctgtccatcagccttcatacataaaccatccatcaacaatcaaaaaaggagatcaaatcatggcaaatgttctggttatcggatccggtgcacgtgaacacgcaattgcagcaacaatgttaaaaagtccccaggttaccaatgtctattgtgctcccggtaatcctggaatgaagaaggataacattcaaattgtggatatcgatgaaatggactttcccaacttggtggagtttgccaaagagcatctggttgatttgacgttcgttgggccggaagtgccgttgtccaaagggattgttgatgccttcatcgccgctcgtttgcgggtattcggcccagatgagtctgcagcccgactcgaaagtgacaagacatttgcgaaaggattcatggcccgaaacaacattccaactgcccagttcaaaacatttacgacctttgatgatgccgaaaagtacgctgagagtttgtcattgccactggtcgttaaggaaaatggtctggccgccggtaaaggagtcacaattgtgaaagactcagccgatctggcagcaaccatccaacacgcacttgataaagccggtgaaattttaatcgaagaatttctggaaggtgaagaattttcactgatgctgtttgttggcggtgacaagaaggtggttttcccaatttcacaagatcacaaaaagatttatgaaggtgaaacgggtccgaatactggtggaatgggtgcttattcaccggttccacacatcacccaagatgttttggatgtcacagttcaaaagattgttaacccaacgatggctggactggcgaaagaggatttggagtttgccgggattatttacatcggctgcatgctgaccaaacaggggccaaaagtgatcgaatacaacttgcggctgggtgatccggagacccaagttctattaccccagttgaagagtgatttttaccaaatgacctctgatttgatcgaccatcaaatgccaaaagttgagtggcaggagggtgagttctatcttggcgtcatggtttctgctccaggatatccaacttcgcccaagcaacatattgcgctgcccgatgatttaccacggaatattttttatgccggggtgacagaggaagatggaaaattgtacagttcaggcgggcgaatctttacgttgtacaatcatgcttcgactctggaatgtgcccaggcaaaagtttacgctgagttaagccggcttgatttgtcaggattctattaccgaaaagatattggctttcgagatttataaaactatttgaacaacacaaaacgggtatccagagtttggatacccgtttttgatttttataatttgagtgtggctggccaatcttactagctttgtcacagtcagtgagcggacttatcaaagtgatttcaagcaataataatggcaaaaaagacactgaagccactgggagtcggtgcctcaatctggatcaatgattatttgcgcagaaaaaccaaattgtccgctgttgagtcagtttcactaaaccgatagttgggtgaatcgaaatctttcaggtcagaaatttgttcaacctgatgttcggccatgaaccggaccatttcaccacgcgccattttcgcaaaggttgccctggttttgatgttgccgtcaaccaaatgaccaaaggtgatattgatgaaacgatcggttaactttaagaatcgggtgacggttttggcgtattcttgggatgccaaattgataattggctgatcgtctgccagagactggtagatgcgatcatcccaaaattcgtacatatttttggcagggccaattgataatcttgaatccatatcaaaacggtagggagcgacgccatcaaagggtttcagaatgccataaaatcccgagagaatgcgtaaatgttcctgcagataagtcagtgcggcttcactcaagaggtctggtgccatgtactgatactgaatcccggagaagctgagaatcgccggggttaatcgatgatacaggtcaatgtcctgtagttgtctgtaactcgcctctgtcagttgatcacttgcatgccacaactttttgagctggtcgtaactcagctgatgcaatgcatctaaaattacagtcgtctgtttcaaatacaccggcattccctgcacatcaaaatcatcttgattgacgaccattttcttggctggtgaaataatgactttcatcgctaatcattctcattaagccagctgtcaagaacgttgatgaattcatcatgttgatccagcaaagccaggtggcggctgttggcaaatagatgccacttggcaccagggatatgatcataaaccgtcttggcgattaacggggtgcagaggtcgtctgtgccgttggtaaccaatactgggacatgaatattcttcaagtcatcagtgacgtcaaaatcgctaatggtgccattctcggtgaactcattggggccttcagcgatcaaactggcttttttaccgttggttggccggcggagtggttcaggcgagttttcgtctggatcatcccagcagtacatttccatgtaacggtcattggctgcggcatatttggggccagagaagttcccagtccgctctgcctcagcgattgcctggcgatcttcgtagctgagatacttcaagaggcgatgctgttcttgaatccataacttgattgaagatggggaaccatcgatcatgacgcttttaacaccttcttggctataatgagtcaaataaagcatttctagcatgccaccccatgattggcccagcatatgtacttcatccaagtgaagatattttctcagggcaattaattcttctgcccacgtctctttaacgtagagggattcgtcgtctggaatcgacgatttgccgcagccaatttggtcatacatgatcaattggcggccagtctcggcataatcatcgagtaattcgaaatagttatgtgatgaacccggcccaccgtgaatcagcagcagtggggcttttccaggtgttttctcgccaacgatccggtaatatgttttgtagcctttaaatggcatgtaaccttcttcaattttcattcaattatccagtcctttccagtaaaaatctttgattggcatccattatacgccagttggcagtcaattattagaggatttatcataattaagacagtgtggaaaaataaacgcttagttgccagaatataaggaaactgtttatttttccactatttggctgggtaacataaaagccggggcaaagcattcacttttgtcccggcccctttgtaagtcgatttaatcattgattaatttatctcgtaattgatccactgaagtataaacctcaccgggattaattttctccagctctttgtgtttggcattaattgaccaagcagccgagtagcatttaatcccggcttgcttgcaggcgacgacgtcggttggagcatcacctatgtatgccatatcgtctttggtggcgttaaattgtttgatcacgtcactaaattgttgtgctttgatcgagccgtcaggagatcctgataagacaggggagaatgcatccgccaatccaagtgagtccagactgacttggaggctttgctcacccttgccggtaatcattggcgtgatcacatcgcggtcgtggagttccttaatgagcttttcaattccctcaaacggatgccgtaattgcaaatgcgcccgccggtagttttcgtgaaagctttccaagacctcatcggaataatccgggatcaactcctttaacatcccaacttcgtttgctccaaaggtggcgaggatgacctggttgctgatccatttgccagtataatcgtgaacggttcttctaaacgaatcaaagattaccgggaaagtctcggcaaccgttccatccatatcaaacgcaataattttttccattactatttttgacctacctttcgaagtgcatgaccaggattccctgtcggatgtgcacttcatgacagggttcctaaatgagcctatacaactattatctgctactaggcacaattattcaaatgaataaaaaaatcgccggcttgatgtcgacgatttttgaaaatattcattgagttatgcccgctttaaactcatttttttcaatcctggtaatgtaatcattgtgatgaaactgatgacgtagaggattgagagaaagcccatgacaaccgtcaatgagtagttgtccattaaaattccaatgacaactgatgagaagccgccaacggcacggccgatgttgacgatcacattgttggctgtcgaacgaatttcagttgggtagaggcggctgataactgccccgtacccgccaaacataccgtttgagaagaagccgacaatggcgccgatgataagaagtgaaatggtattgtgggctaaggtaatcgtgaagaccatggcagccgaggcaatcaggaagatgccaaatgctcggcgtgggccaaagtaatcaaggattgagccgaaggtaatcattcccaagctcatgccgatgatagtggaaatcatccacagtgatgaaccggaaacgtttaagccaagttgtttttgcacgatgattggcagccagttcatcaagccgaagtaaccggcgatttgaacggtggtcataatcattaaggcaaaactttgataggctaatttgggtgaactgaacatgtacttgaagacggcgctggtcgtggattctttcttctcggcttcaaccttcttggctgcgacaaactcttcagtctcgctcaagtgacgacggacaaaataagttaaaacaaccggaacaatcccaaccaggaacaatgcgtgccagcccagacgtggaatgacgattgcggcggtgatcgctgccagaatggcaccaatttggccaccaattgcggcaaccgatgtcattttgccgatttgatttttgtggaaggattcggcaatcattgagatcccgacgccatattcaccaccggcaccgattcctgccaagaatcttaatatgtaaatcaatgtgatgttattggcgaaggccatcattgcggtggcaaatgcaaagatgaagattgtgtaggtgaaagtcttaacccggccaaagcggtcaccgatcagaccaaacatgatcccgccaaataacattcccaagttggtgattgaaccaatcaatccggcagcgccaccgctgagatgaagttggccaatcattgagctcattgcaaaagataaaaatagcacatccatattttccagcgcgaatccagaactggtagaagcaataacccatttctgattcttcgtaaaagtatggctgtgcgtaagtgctgcgtttgtattttccatgttcgttcctccaaatgaatgctcgctgacattctttatttttgctgttcacattattacatggatgttttggaaatgcaagttggtcaattaaggatatctgtgattgtttgcttagctcggacaaaagatggtgtatcaagtaggctcacaaattctgcatgatgactttgaaagtcataagtaaaaaattgaagtggattcacaaaaccatcaattttttcattattaactctgattaaaaagccactttctcgtaaggagttattcattgcatgggttatgggagcaaccactaccaagtgagtcattcgactgtacccttgattgcttaaaactagagcagggcgtcgctttctgatttcatgaccgacggatggatcgaaatcaatgtagatgatgtcttgttgatttgggacgtatgggctaatctttggggatttctctgccaactaatttacccccaaattcttcttgctgttttaaatcgtgtgattctatgaacgcttcattgtggaatggattatcatgctttgggacataaacaattaccccatctctaccctgaaaaacatcaaactcgtgtgcgattggcttgatactgtttggtacagttaaggtattcgagttgccaactttgcgaattttaactgacatgaatatcacttccttctttcgtatacatgaagtatacacataatgtatctgatgttcaacaaatatgatcactaagtttcacttgaacaacctggtccatcgtgataaagttataaacaaataaaagagctttaatttggttcagagaggccaaaagcggacgacaattaatctaagagtccgtgattttgtgggatttagtacagggatgtactgaataatacacagtctcgggctctttttctgtcattaaacaggagggtaattatgcgaggaccactaattgtatcacttgatgtttggaatcgagaaggcttgttcaagatcattgaccagtttccaaccgacgaagggatgaccgtcaagatcggcatggagctgttttacggcgaagggcccacaattgtcaaagagctgctgaacaagggcttcaaaatcttcctcgacctcaagcttcaagatattcctaataccgttaagatggggatgatgcaaattggtcggatgggtgttacctatacgacggttcacgcattgggcggctcggaaatgattgcggctgccaaagagggcctcgagcttggcagtgaagaagctggggtgccgactcccaagctgctggcagtgaccgagctgacttcaattactgaagatgctttggaaaatgagcagaactgcaaattagatatggttgaccaagttgtctccctggcaaaattagccaagcgatcgggtgccgatggcgttatcacttccccgttggaagtcagttcactgaaagaacaggttggtaatgacttcctatatgtgaccccaggaattcggccagccaatttccctaaggatgaccaatcaagaaccgcaacccctaaacaggccgcagaatacggcagctcagctttagttgtcggccggccaatcattcgagctgaagatccggttgctgcttatcacaaaatgttggaggaatggaattatgcaaactaatcaaattattcaatcactgattgaccaccaaattgtcagtatcaatcttgaaaaacccttcagatacgccagcggaatcttatcaccaatttacaccgactttagactaaccatttcgattccttcccttcgagatatgattgccgacggtttggcagaaaatatcaaagagaattatcctgatgccaccgtcatcggcggggttgcgactgccggaattccccatgctgcttgggtagccgaaagattgaatctgccgctgatttatgttcgggccaagcccaaggatcacggtgccggtaagcaaattgaaggtcgaattaccaaggacgataaagtggttttgattgatgatttgatctccactggcggcagtgttttgggtgctgttaaagccgttcgcaacgaaggcgtcaatgtcattggggttgcctcagtcttcacatacggcttgccggacgccgacaagaattttgccgacgctgacaccaaattagtaccattattgagttacgctgatttaattgcccaaggccacaaagaaaataaattctcagacgaagagtattcacgcttatcaacttggcacaaagccccttgggactggacaaaacgggaggaagcaaatgcaaaataatatctcactcgccgctcacattggtgactatcaattcgataatttattgttaaacgcagctggcgttcgttgctcaaccacagacgaactgaataagaccctggattcaatggcaggtggctgtgtcactaagagtgccacaccagaagaacgggccggtaacgaaagcccccgcatgaaggcattaccgctgggcagtattaactcgatgggcttgcccaatcatgggatcgattattatttgaaatttgctgaagaaaatcagggcaagaacggtaaacaagtgatcttatcgattgccggcttgtcaattgaccaaaatattgagatgctcaaaaaagtccaggaaagctcattctctggattgactgaattgaatctttcctgcccaaacgttaaaggcaaatcgcaagtgggatacgattttgacgccgttcgcgacgtcttaacttcaacctttaagttcttcaagaaaccccttggcttgaagctgccaccatactttgactttaaccagtttaatgggattgctgaagtcttgaatgatttcccaattacttatatcaacgttatcaactcaatcggtaacggtttagtcgttgatccggaaaccgaatcagtggtgatcaaacctaagggtggctttggcggcctcggtggcgattacgtcaagccaactgcattggccaacgtgcgggcccttcgccaacgtttgaacccggaaatttcgatcatcgggactggtgggatcaagtcaggcatggatgttttcgaacatgtgctttgtggcgctaatttggtgcaaattggtaccgcatttggttatgaaggcacaccgatttttgaacgaatttcaaaagaactcaaagatatcatggacaaaaagggttacaggacgctcgatgatttcagaggaaaactcaaaacaatttaagtatgattcaaggtcaagccagcaatggtttgacctttttatattcactaaagccaatggtgcggtaaaattgaaacaacaccattttgaaaggagtcatcctatgccagcaagtaagcttcccgatcatattgaagtgattggtggaaaagtgaataatttgaagaacattaacgtcaatattccgttacataaatttgtggcagtctccgggttgtccggttcaggtaagtcatccttagccatgggcattctgtattcagaaggtgcccgccgctatttggattctctggccacctacacccggcgacggattagccaagttggccgggccaatgttgactcggttaagcatattccatctgccttggcattgcggcagcggccaactattcccggtgcccgttcaactgtcggcacaatgaccgaaattttcaacgtgctgcggttgatgtattcccgtttgggttcgccaaaatgtcccaacggccaccaagtcccgccaaccattaagattgcggaagccatggacgtcatgggcgaccaaatgggtgtgattacctgtccaacctgtggcgtcaagttccacgcgtttggtgccgaagactttgcctttaattccgacggtgcctgcccagagtgtgaaggattggggatcaccaaacagcttgatccggacagattgattggcgatgaaaccaaaaccatccgtgatggggcagttgctgcttggcgaacaccgggcagaaactttatgccgattgttgcccaggcggctggtgtcagaattgatgtgccctataaccaattaacagaaaaagaaaaagagatggtcctgcatggtcaacagaaacattacgccatcgatattcccagtaagaatggccgggtttttcacatggacaacgcattgtacgaaaatgcctataacgccattgaggacagcatgaaaacgacgaagagtgagattgccttgaaacggctaaatcgtttttactgtttcttcacctgcccaatgtgtcacggaacccggatgaatcccaatcgtcttggacaactgattgacggcatgaacattgccgaagccagccatatgccacttgggaagctgccggcctttgttgaccgaatcaaacaatggttgccggacaatatgcagaaattggcccaaaacttgacgactgaattgctcaatcaaacgcaaccattgatcgacctggggttggattatttaaccatggatcgggctggcgcatctctttcgaccggtgagcttcaacgaatccaacttggccggacgttgcgaactcagacaactggagtgctgtatgtcttggatgagccctcggtcggcctgcaccctgacaatgttgccggtctcatcaagatttttcaccaactggttgaccagggaaattcgttggtggtcgttgaccatgaaacggcgattattaacgcggcggattacatcattgaaattggcccggggtcgggtgtcaatggcggccaagtgattgatcaaggaaccccggctcaaattcgccagagtcagcattcattaattggaccgtttttgactgggaaagcgcagttggtgacccgaaagattgccaatgacgatgtttttgccaaagggtctgtgacactgacaatcaaccagcggtttaacttaaacgatgttaccgcagaatttccggttaaccggttgattgccgtcaccgggttctcaggtgccggtaagacgacactcgttttggatggtttacttgatgccttcactgcaaagtttcacaagcattcattacccagttatattagcaagtttgaacccggcaaaatgaagcatatcgtcagtgtggacgcgactccggtcgggaaaaacgcccggtcaaccctggcaacctacaccaacattatggacaatctgcgcaagaagtttgcccagctgcctgatgccaagaagcatcactataccccaagttatttttcctacaataataagcagggggcctgccccgcttgtgggggaaccggtgaaatatcgctggatattcaatatctgcctgacatggttgaaacctgtccaacctgcaaaggtcgccggtttaaccaggatattttgaacattaaatggaatggcaaatcgattgctgacgtccttgactacgacgttgatcacgccattgacttgtttaaagacgacgaatccattttgaagaccttggaagtcctccagcagatgggactgggttatcttcacttgggcgaggccactccgagtctatccggcggtgaggctcagcgattgaagctgacttctcatatgaagagccgccaaaatgatacgttatttatctttgacgaacccacagtcgggctgcacccactggatgtgcatgtgttgttaaaagtcttttcacagttgattgaccagggggccaccgttttgatgattacccatgatcttgacctaatggcgaatgccgattatctgattgacatgggcccccgtggtggtgatcagggtggtcggattgtcgccaaggggcggccggcggacttggttaaggatccgcggagcttgacgacaaaatatctggcggaacattttcaaaaatttcaaaagtaggtaaacaccagcctactaatcaatcttgcggattggtgctgagttgattgaaattgtatgtaggccttcacaaaatactattgacaccgttagatgaaaattgtaaattgatttagatagttggttttttaaaacaactttgatgctacaaccaaaatatggtatttaatctgaagtgtcatcatcgtaattagtgccttcgtgagaatatagcggtatctcgtggctcagtaaggttgattgttgaatttagtgataaaaaatggagggaataattcaatgactaatgcaacgggtagggagcagcttcataagcgaaacttgaatctagttctgcaacaaatttttaacaatagtattatttcgcgaattgatatttcacacacgttaaatttaaataaatcaacggtatccgctttgtataatgagttagacaaaaagggtctgctgcaggaagtcggttcagggcaatcaaccaatgttggtggtaggaaaccggtcttagtcaagattaatgagcaatatggatatacgatcagttttgatcttggtttccgtcaccttcatgtgatgggcaattatcttaatggtgaggtcttttactatcaaagaattgagcttggcagtagagatattcaaaaaattctgggaatgattgatcatcagattaaagtttcaatgcaaaacgatcagaccaagcgtggactactcggaattggtttttccattcatggaattgttcaagataaccaggtgatcaattcgccttttatcgatatgaagggtgtggatctggtcggacgatactccacaaagtatcgagtaccggtccttcttgaaaatgaggcaaatctttcaggtgtttatgagcgcgatttcaatgacggcaaggataagaataatattattgccattagtattcataaggggattggtgcaggcattattttgaacaggcagttatacagaggggttaatggcgaagcgggagaaatcggccgctcgttgatgtttaccgaaaattttactggcagtaaaaatgataaggtcgaagacttttgctcagaagatgcaattattgagcaagtagaagttcagactcatcagaaaaatttaacacgtgaggatatcgtacagagaaatcgtgctggtgataaagttgttcaaagtgaacttaaacattttacttatgcaatttcgcgggttatttataatgttgcaattagttttgccccccaagaactctacttgaactcaccattgattgaagatattccaacgttgtttgatgatatcgttgataatgctcagaagcttgggatgaagatacccattcggctaatcccccattcaggctatgcaacgcttttggggtgttgctcattgttgacacatcgggttttggacatggatgagtataatttgacatttacaagtcagaaataacaatataatatggccagtgatttgcttgagcaagtagtaggttagtatattaaaaagttgaccaatattgaaagaatactcttccaaaaaggtcaacttttgatttatccagagatgtaattctcttggatcgccttatcatatttagtcactttggatgacttgcgatactgtgctggtgtattcccggtgacgtctttgaaattacggttaaaggtccttagattttcatagcccacgttaaaggcaatgtcggtaactggtaatgaagtgttctttagtagttcacgtgctttggaaatacgaaaactgttgaggtatttagtatacgaaaggttgattgttttctgaaagagtttggataagtatacatagtcatagccgattgagtcagcaatttgcttgagtgtgcatgattctgtgtaatggtcattaattatgttaacaatctcattgcgggtgaggtggcaattcagtcggtcctcaatcggacgactccttaccatcagccacattcaactataataaagggttatgcctgtgtttatggcggagatgatcgttattttaacaatttgtttgtcgccgagactggcgtatcagaagacgacaatcacattggaactgcagagtacgatggtagtccaacatcaatgaaggaatatattgccgcggttgagcaaagactaccgggtgatgttgagttgtttgaaaccatccgacaaccagtctatatcaacgacaatgcgtatcttggcgatgctgatgcattttcgaaagaacaaaacaatatccgattacgtaattgggatgcaaagttgaagctaaccagcgtagactcgcatatcgtgttacaactcaacgttcccgaagaattgttcaacacttgtgttccagttcagaaaacgagttcgctcgggaaagtgcgtctggccgatgcagtttttgataacccagatgggtctgctttaactattaataatggcattgataaaaagaccggattaagtaagcgaattattggtcctttttctcagctacatcagggagtcaatcaaatcgtattatttgacgatttggagcctgattgataatagatatataacataagtgaaagtaagtgggatgtgtgaactgaaacccacttactttttttgtttatcgataatattccaaactaattgtggcgattttgcgcaaactaaaatccagttttaaatattagatgacaaataatgtccaataaatgtcaaatacaagcatatcggtaagttcgtttaaaagataaactaaccatgtacttaattaaggatcaactttctgaaagcgcttcaagtaactgataatgaatgcactttttaaggtgatagcgttctgacctaattgcatatgtgatgattcgtgtaccaaagataagtggcggtgacgaccgttagtgattgttgcaatcagctaatttttttgatgaaaatgtaagcggcttcaagtgtttgttttaagacaacaaacgattattgaagatattctaatgaacggaaaaggtgaataaaatggcacaaaatgaaaatgttccagaatggcatggcactgttttggatagtgaacaacctaagaaaccaattaaaattgggattgccactgggattggcgcactgctgtggttaggaccctatttgggtgttaatggggttttgcttccagcaaaagttcagcagattattcctaatgaaaaagctcaggtagttgctttacttgcttctgctgccatgatcgcagcaacgttagcgaatattattattggcggattctcggatattacgcgatcaaggtttggtcgcagaacaccgtggataattgctggatcggttggaagtttattaacactgctgtggttcaatatggtaacgacagtgccaatgatggtggttgcttggtgctcgtatcaagtttgtttgaatgcgattgttgcgccattgcttgcttttttacaagaccaagtggcccctaagaaccgcggaacgatttcttccatttatgcttttggatatgtgattggacaatatggtggtcaagttgttggggctcaatttctgagccacgttggtactggtattgttgtgatggctttcctaacattactttcaggaccaattgctgcaattatcgttcgtgagccttcaagcttgggaatgcctaagaagcattttacagcgggaatggttgttcaaaactttgttttcccgttacatcaagcaaaagatttttacttagctctatttggaaaattgttgattaacactgcaactacagcaattatgggttaccaattgtacattttgagtgattacattcagttaaatacgggtggccaacagaagtacatttccatcatcaacatgatgctgatggtaactgcgattatcatgtcaattactgctggacctgtatccgattggatgaagagccgaaagatcccggtatttattgccgcattcttggttgctgttggggtggccttcccgatgttaagtaataatccttggactatggtggtttatggattgcttgccggattaggaatgggaattttcttcgcggtcgaccaggcacttaacctagaagtattaccaaacccacaaacagctgctaaggatttaggaatcctgaacttggccaatactggttcacaaattattggaccgattgtggctgctgcaattgtcacagcttcacacggtagctattttggaatcttcccagtatgtgcaggtcttgccctcgttggtggtattatgattctcttcgttaatgaacatcgtgatgttaaggttcaagaagagaatgccaaataaggacagttttaacaatccttggcccttagtccttatgaaccaaggattactctaattaatgtaaggacaaatatacgatagaggtgaaaacgtttatgactgctacacaaattgaaagtactcaagattcaaaactggttgagagtcagttgagcaccacgagtgagaagctccataataatctcgaagttggcatcgagaaacgtcaagaaatttggggctttggtcaaacatttaacgagttgggctggcaagcactacaaagcctatctgaagaaaagcgtaacgagatattggacgatttgttcaaacccggagagggtgaaaattatcgaatttgccggatccccgttggtgccagtgactatgctttgaattggtattcattagatgaaacacctggcgattatgagttaaaggatttctccatcgagcgtgataagaaatacttaattccatatatcaaagctgcccaaaaacggaatccagacatcgtcttttccgcttcaccatggagcccgcctacatggatgaagacaaaacccgtgtacaattatggaatcttgaaacatgataagaagactcaacaagcatatgcgaattactttgtaaagttcattcaggcatatgagactgaaggaattcacattagccaactgttcccacaaaatgagcctcaacgagatcagaaatttccttcatgctactggactggtgaggagttacgtgacttcatcaagaattaccttgggccaacttttgaaaaagcagggttgaataccgacatctggttaggaactatcaactcgccgctcgaagatactgaaatgaccaaggatgaaaccaccgactatccagttattactgaaacggttctttcagatcccgctgcttatcggtatattaaagggattacctatcaatgggcaggtaagtctgtccttcaacggactgtacaagcattcccggaattgaactatttccagtcagaatctgaatgtggtaatggtaacaatacttggacttatggggaatacgtctttaacttattccgtcactatatcagtaatggtgtgaacgcttatatgtattggaattctgtcttacaagatggtgaaagcacgtggggttggttacagaacagcatgatttcggttgattcaaagactggtcagacgacctataaccctgaatattacgttatgaagcattacgcacattacgttcgaccaggtgctcacttgctttcgtatggcggccacgctgctggggaagcaactgcttatgagaataccgatggtagtgtcattgtggtgatgtctaatagtatgaaccatgatcgagacatctcgattgatgttaagggcaaaacatacgaggctcacttaaaagaacattcattcaacacattcgttttctcttaacgaggttcggtgttaaaaaacggctggatggatttaaatattttaaaagagcttgaaaaagtatttgcgacatggtaaatttaaaatgtaagttggttgattgaactaactaactaataaaacctggaggcttgcttattatgagttattggaacgtagataaaattaagtatgtcggtaccggagagaaaaaatcaggattaggatttcaatattataatccggatgaagtcgttggtggtaagaaaatgcgtgattggttacgctttgcggtcgcttattggcacacatttgaccaacggttagtcgatccgtttggtgatggaacggctattcgcccatatgacaagtacactgacccaatggatcaagcgttggctaaagtggatgccgcatttgaattttatgataaattaggcgttgactttctttgcttccacgaccgggatttagctcccgaaggcgatacgctccgcgaaaccaatagaaacctggacaaggttgttgacaaaatcgttgaaaaccaaaaaacttctggaatgaaagtgctttggaacacatccaacttatttaccaatccccgttttgttgagggtgccggtacttcaccatatgctgacatttttgcttactcagcagctcaattaaagcacagtttggaaattggtaagcgtgtcggatcggaaaactacgtattctggggcggccgtgaaggttatgaatcactttggaacactgatatgaaacgtgaacaagaacatgctgccaaattattccatatggctaaagactacgccaacgaaattggttttgatgcacaaatgctgcttgaaccaaagccaaaggaaccaaccactcatcaatatgattttgatgctgccactacgattgcctttatgaaagaatatggccttgataaagacttcaagcttaatttggaaggtaaccacgcgaacttggccggccatacctatcaacacgaaatccgagttgctcgagaagccggtttgctgggctcattggatgccaaccaaggtgataagctgatcggctgggacattgacgaatacccttcaaacttatacgagacgacagcggcaatgactgaagttgttgaaaatggtagtattggacctcgcggcggattgaactttgatgccaagccacgacgttcttcatttgaaccaaatgacttgttctatggccacattgtcggaatggatagctttgcagccggcttgagagttgctgttgcaatgaaaaacgacggcgtccttgatgacatcgttaaaaaccgctatagttcatttgactcaggaattggtgcagatattgaatctggaaaagcaagtatggcagatcttgaaaattattcactggataaaactcaaaaagatcttcgcgatgcaactcattcggatcatcttgaagagattaaagatacaattaaccattacatcattcagactttaaagtaacatcctgatcaaatacaacaattaatgggaatgggattaattttccattctcatttttttcgaggaggagaagatatgactgaatgcgtacttggtgtcgatctaggcaccagttctgttaaagtaacagcggtgagtcggactggtgaaatcattgcccaggaaggaatggatttcccactacaacagccacaaccgggttacgcggaacaagaccccgaagactgggtcagtgccgcgaccgtttcaattgttcgactcattttaaaagataagctcacccccgaccaaattgtcggtatcagttattccggtcagatgcatggactcgtcttgctcgatgacaataatgaagtcctgcgtccagccatgctttggaatgacactcgttccacccaacaacgccaagaaatcatggccaaaatgggtagtcggttcgtcgacatcacccataacaagccactggaagggtttacgctgcccaaactgttgtgggtaaaagaaaatcagcccgagatctttcagaatgccaaaaccatgttactgccaaaggattacctaaggttcagaatgactgggcaattggcgattgattactcggacgcaaccggaaccgtgatgtttgatgtcgacaaacagcaatggagcaaggagattttagatgcatttgatattcccgagacaatttgtccgccattagtcagatccattgatgagacggggaatattaatgagtggtacgcagaatattctggattatccacccacaccaaaacctttggcggcggtgctgataatgcttgtggcgcagtgggtgccggcattgacggacccacaaaggtgctctccagcattggaacttccggagtgattttaaaatatgaacccgaaaaggaaaccaattatgatggcgtgattcaatacgaggaccatgccattcccaatgcctattactcaatgggcgtcaccttggccgcgggattttcactgagttggttcaaaaagacctttgccgaaaacgaggactttactgcagtcgtggatagtgccgccaaatcaacagtcggcgctaatgggttgctctttgccccgtacattgttggtgagcgggcgccatacgccgatgcggacatccgcggcagctttatcggcattgacggaatccatcagcgccacgattttgttcgcgccgtattggagggaattatcttttccttcagagatattttggatttgtatgaggcgaaaggaaaccaatttgagacagtcatctcgattggcggcggggccaagagtcccctttggcagcagatccaggccaatattttcaatgtcaaagtggtctccctgcaaaatgaacaggggcccggactgggagctgccatgctggctgcggttggtctgggctggtatcatgacatccccgagtgtgccaagacctttatccagttcaaagatgtctttttacctgagccggataacgtggaaaagtatcgtcaattacatcaaatttatcgaaaaatttatccaagtaccaaagaaatcacgcatgagctggttgatttccgacgagatcatcagcgttagcaaccattcaatggagcctcgaaactaaaggttccattttttagttaagaaagatgacacgatgtcactgccaaaaaaacaactcaaatttatgcaggaattcatcatggatatcaaattaatcgtcgcaatcatcaccatcacaatggcgctggtcttttatacaattggcgtgttctctgaacgaaagtcggacgcgcttaaactgcgccacctactattgtttggccttgggttggtgtttgacaccactgggacaacgatcatgtcatcaatcgccaacacctcgggggctgccacgcctgtcctgcatttggcaactggtttagccgcaattgctctgatggcctttcattttctgtgggctggttacgttttatggctgggaagtgaaaagtccaaacgcaatttccacaagttcagtttactggtatggctgttctggctgatcccgtacgttgccggtttggtaatgggaatgagcaactaagcacaggacgcaaaagggtccgaacaccattttgatgatgttcggaccctttgacaattagtttgaatagactattttgacgacaaatatgaaataaacaccgatgccatttttcaattaatcattttgagcttcggcaaccgccaaactgcgttgatgcaggtaggttacaccgccgaagacaactgtccagatgatggcaccgaccgcaccgataatatcttgtgggatgaagaacaaggtcacaaagataatggcgaagaaagcgatggtgagtggactggtgaaattgtaccaaggcattttgaagccatttggcagaaagtcactggattcacggtatttccgatgagccatcattgccaaggcgtataccaggatatacatgtcatttgaagaaccggcaacgatcgtaaagactgaagccgtggcgttggtgagactcatcaacggggtaatcaagaggcacagtgcggaaaagccaatcgcagcggctggaaccccatttttagaaatcttggcgaaatggcggttcataaagctgtccttgggcgtttcagttgccagctgatagaagtgacggccagccgagaagatgaagctgttcaaagaagatgaagctgacgtcaaaacaacaaagttaatgacggcggctgcagccgggaagccggctaatttgaagacctgaacaaatgggctgctggcaggcgtcaaatgggtccatgggatgattcccatgatcacgattaaagcgccgaagtagaagatcaaaattttcagcagcgtttcgttaacggcttttttgatgattcgatgcggcgtttcggcctcgccgatggtaatgctgacaaattcaattccttgaaaggcaaagaagaccattgggaaggcagagataaaactcaagccgccatgggggaacattgagaagttatggaaaatattttgaacggaagcgtggccaagtggggtggtcgagtgcgtgaacatcatgaagaccccggtggcgattaaagcgacaatcgcgatgattttgattaaggcgaaccagaattcagcctcaccaaagaccttggcggcgattaagttaacagctgccagcgttcctaagaacacaatttgaatcagccacgatgggatatttgggaaccaaaactggacatatgtagagatggcggtaatttctgccatggcacaaaatgaaagccccagccagtaggtccagccggtaaagtggccgacggtgggtcctaaatatcgggtaatgaatgagacaaatgtgtgttgtgacggatctgaataaagcatttcaccaatggcacgcatcattaagaagaaaaagatacctaacactaaatagactaataaaattgatgggccggttttactgatggtggtcccggaacctaagaataacccggttccaatcgtgcctccgatagcgatcatctgaacgttgcggttgctcaaggagcggcgggtgccgtctgcgttttcagttacttctgttttttgcatgaataaacttcctctctgttgttaatgatgaatcaaattagaggcctctaattaatttgtcattatactaacaccacggtgtctaaatcgggcattttagagaggaagttttcagatgattttgtgattttgattattttttcatgaaaaaaaggcaggattgccggtttgcctatgaaaataaaaaactttttgcagctcttgactattcgtcgtcttccggcagtttgagtgggcgagggccaatattcgttgtgaaggcaacgtttgtgtgactgtagccgaactctttaagagacgcgttgaattcattcagttcggtcatggttttgtagaaaaccttcagctgaaccgaggcgtctccggtgatgtagttgcattccaccacattgggaatttttgaaatgaagtcaacaaacttaggcatttcaacgtaactcacgtcaattcggacaaatgctttgatcaaatagcccaacttttcgtaattgacattggcagtatagccgttgatgaagccgtgattttcaagattttgcagacgaacggacgcggatggcgcggagatgaaacatttttcagcgatgctcttgatggatgcgcggccgtcttcttgaatgatatttaaaattttgcgatctaatttgtccattcgttttctccttaaaaatagtttgcgtatattataccattcaccattttgaatggttttgagaaagctcgttggtaaatgcgtcatggtattaatgataattgccacatacaatgagaatggctataatgaattttgtatctaaaattcgaatttagtaaggtcttgaaaaatgatgaaatcgaaaacaccacaatggaagaaaaacatgtgggcgctttggttcggcaactttgccaccggtgccggcgcgagtatgtcaatgccgtttctaccgctctttatctctgagatgggcaacttccccaagtggcagttaacattatatgctgggctggcattctcaggcgtgtttctgagtcaggcgattgtctcgccaatgtggggaaatctggctgataaaaccggtcgaaaaccaatgctgctgagagcggcgatcgggatgacgattagtgccacactgacagggttgtcgccaaatgtctggttcctgatcattattcgttttatccagggaactttctcgggatatatcaataatgcttacgcgctgattgccagtgaagttccaactgaagacagcggtaagacgatgggaactttgatgaccggaaatgtcggtgggcaactgattggaccgattattggcggatacctatccggtatttttggctaccggctgccattttatatgtttgggttcatgatgtttctggcatcactgtcgacttggttctttgttaaagaagacttcaccccaattaaaaagggtgccaagacgggaatgaaggatgcttttcgagggattgctcacaagcgcgtggtctgggcaatgatcatttcatcaatgctggtcatggctgccacgacctccatcaacccaattattagtttgtttgtcaaagaattaatgcatagtcatggaaacgtagcctttaccagtggggtgatcgcggcactgcccgggattgcgacgatttttgccgcaccttatctaggtaggctgggcgatcatatcgggcctgaacgaatcctgctggctgggctaatcttctcggcggtcgtcttcttcccaatgttctttgtgactacagttgtgatgttgggagtgctgcgattcttgattgggatcgccaatgcggccctgctgccgattactcaaaccgtcatgacactggaggcgccggcccgttcggtgagccgaatctttagttacaaccagtccttccaagccatgggcgcggttgttggccccatgctggcgtcgggggttgccgggattttggactatcgatacgttttcttgatgaccacgcttttggtattaatcaacattgtggtggttgtcgttgcttataagaaggatcatgttaaggttgttgatgtttctaattcataaatgtggtgaaggcattcctgttggggaatgctttttattgtgtagaggtcattattatatgccatttctttaaccaactgatataattaaaaagtaaatgaagccaattgttttgtgttatacgagggggcatttcatgattaacaaattagttcgattggttggtatctccgttttgatgcttttggcggggttcactgtattgtcacttggaaacgctcaggtggatgccaattctgtcatttacaatggtgctaatccacaaatgacgcctacaattggtggcggaactagcggaactggcgggactccggctggattggaacactatgtttatgtgactgttggtaatgaaaagtccaattattcgtctaatggagccttacaagatggaacaaatggtcgtcaatcagtaattgattatcaaaaatataaggatgctgggtctcctgaaattattgaacatatgtacttaaagaataccaacgctgatggcactaaagacatctcatttcaacgggctttcaggtatcctgagaatattccgttgaatcaaattggaaggccaatcgtagaagaacaaaaggaagatttgaagcccgatgttacgagcaatagtgacgaggcaaagcaaaaagttaatttctgggcaaatggtgcccacatggctaatgcctatgtgactctcgcacctggccagtgggtggatatatcaatgcccctcaagattaccaatttggattctattaattatcaaaaggggactgcattccaagtttacgaaggcgagcagtattggactggtggtacgaatctagtagttagactagcagaacaaatcgatccggatacctattcagattttcaaaaaggccagtatttaatcacttatttggataaggacgggtactatcagcaggcaaaagatattcaatcattaatgccaaaatttgatttggctcgtgacattacatttagtagtttgaacacgccgttcggcacttctgattcatctctttggacaggcggaacatattttgttgatggcaataaaatggtcgcaactgatgaaaagggacaatcattaaacttcttggatatgttatacagtcatggctatgcccctgtttggagaaacggtcgattgttaacatatgaatcatttaatgcttacgagggatcaaatactcccggtaacccagattactttaagtatatgagagacgttcttggccacaatggcatcggcggtattaactggcaggttgtaaaagtactggtagctgataatgccaccgtcaatcgcggggcaaagtgggctccacttgatcacgtaactttgtttgacccaaagcaggaaaagaatggttcggcctcagaagtccctgtgaccaaagataatgttaaaatagcttctgataatggtcggatcaacgctgatgggacgttggataccagtaccccgggtgtttataacgtcacctacacctacgaggcggtctattcagattctgtccgccgaaccatcagtaaaaccatccaggtaacggttcccggaaaccctaacggcggtggcggccaggccccatcctcgaatacttcagacaacaatgccaatccgacgaataacaacggtggaaataacgcttggaatccgactaatccaactgattcaaacggcacggggctgcccaattacgcagctgtgaaaggtgctgcggtgtacgcaaccaagcgaatctatctgtatcagcacccaactttcaagaaatcacaacgattggcgacttatcccaaagtcgcccgaactgctcggccgatgtttgtggtcatcggctacgcccgctccagcaacggtgccctacgatacaaggttcgagatgtcaatcatggtaagaagatggctggtaagatcggctatatcactgccaaccgaaaatttgtcgtgaatgtttattatcaatcgttaaagggcagccacaatattatagtgatcagcaagaaaggcattcacgcatacaagcatgttaatctgactggtaaattcaaaacctacaaacgttggaccccacttaaggttaagcgactggtccaccacaacttaacgacgcgctatcaattgaaaaacggtgactatgtcacagccaacaagaaattagtttttcaaattgacggtcacttagtcgttgtgcgcggatatcaaactaaataagaccatcaaaaaagttggagttcgtctccaactttttgtgtcccttgagttacaaccgcgagtcgatttggttaattcccccgagaacagtaccatattaaattgcaaaatggtaatatttacttaatacaaattgtgcgacaaaaggatattgaggagtgaatttcatgattttgagtttcaaaaaatcattgtatcttggcctggcagcaatcgcggtagtggccgcagttgaattaacaaccactgatgccagtgccaaatcatatgcgagaatcacatccaaccaagtgatgcagacagccccgcagaaccgtaacgtgacgaccaacgggacgaatgcgctctacaccaaagcgggtaccttgcgcggtgcccggatgattgcgtctaagtatacgttgcagcgatatggcagctccaagctttccagccagtatttccgggcttaccgggtcgctacgactaatcggggtgcggtttactataaggttgtttcattcaatggtgtttaccgtggttggatctatggcgggcgagtaaacgggacctttgccggcggcttgaatccggccaacacgatggcaaatgcgaatttacctttgcaaaagaccggctacacgttgaccaatccacagaaatacacgctgtgggtggatcccaaatggtcacggtataaggccaaacaagttgacatgagcagctatagcgccaatgacacctttacaattactgatgcggctgttaagacgcgcgaacaatatttatactataaagtcattgatgataaaaattccgcgattgtcggctgggtctattcaggtggcgtggcagctcctaattcccaacaggcaactaaagataacagcgtcaagattaactatgtaaacccagccggccagtccgttggggcttacacatggattatccaaaagacagatctaaaagccggggctaacatgaccgatggagccaagctgggggatattctccaaaacagcactcaactaagtgatgtggccaccaagaacgtgccaaccgggtataagatcagtgccacccaaagcccaaccaatcaaccggcaaatgtcaccgttggatcagaggactatctggtctacgtggatccgatcaaggccaactttctatcaccggttgcctattatttgaccaacactggtcagcaaattagcccatcccagctagtgggcaatacctatccgattttgacagacgcccagatgacgattttctcaagtcaaacccagggaatcgtgccagccaaagtctttgataacgcgttgtttgcagaccctaacaaactggcttccttgaccggcgtttcggtgaagaatgccgacggtacgatgactacaccaatttattacttcaacaagcaggcgacgattgccgccaacacaacagctaggtatggcgatactttgaagctttactatacgttgccgcagagataagctaagatggcattcaaattcattgacgaatttgaatgctatttttatttataagctcaaaataccagttctgaaagctttttgcttacttttttcacctgattagcccataatataactactctaaaaagtaaagggaggcatttggatgtcgattttaactgatacctatgaattaaataatggcattaaaattcccaaagtgggcttcggtacctggcagattccaggcggccaagacacctacgacgctgtcagcacggcccttcaggctggctaccgtcacattgatactgcaaaagcctatcgaaatgaaaagagcgttggcgaggcaattcttgattcggatgtggaccgggaaaacgtcttcgtaacatcaaaattaccagccgcaaccaagtcctatgacggggcgattgcggattttcgttcaacaatgaaggccttgaacctatcttatttggatttgtacctgattcatgctccgtggccatggggcgaacggggatcgaccaactatgatgaagccaatgtggaagtctggaaagccatgcaggatatttatgccagtggtgaagtgaaggcaattggggtttccaattttaatgtccatgatcttcaaaacattttggctcatgctgatgttcagccgatggtggatcagattcgctacttcgtcggctacaccgagcctgaaacaacccaatttgccaaagataatgatatcttggtggaggcatattccccacttgccaccggcggcattctggagaacttagacattaaaaagattgctgacagatacggggtgagcgtcgcgcaattagccattaagtttgttctgcaaaatgacgtgcttccattacctaaggcaactcacaagaaccatattgaaaataatacccaattagactttacgattagtgccgaagatatgaaacttttgaatgggctcacagcaactgatatgtaatatagagaaatcttgaacggatcgcacatttgcgacccgtttttgtttgaaatttgttacagtggagttgaatcctaattgaaaaggggaaaatcatttatggcaaatgtattgattttaggtgctaatgggcaaattgcaaaattggtcgaaaaacaattgctcgatgaaacagatcaccagttaacgttgtttctgcggcaggcgaaccggatcacggtcgctgatcccaaacgtgaaaccgtcattgaaggggatgccaccaatcgacaggcaatcatcaaagccctcgacggcattgatattgtttacgcaaatttgagcggcaaaaacattgaagatcaggcgaaagcagttgtcggcgccatcgatcggaccaacgttcagcgtttgatttggatttcgaccttgggaatctatgacgaagttcccggtgcttttggcaaatggaaccatcagcagctcgacggtggctatcttgagccgtacaccgcagcggccaaggtagtcgaaaattctgatttggactacacgattatcaggccagcctggttatcgaataaagacattgtgagttacgaaaccaccgaaaaaggtgagcctttcaaagggaccgaagtctcgcggaagagtattgccgacttggttgttaagttgattaaccatccaagtcaggcaattcgccactctttgggtgtcaaccaaccgaatacggatggggacaagcccagttggtactgattgtctcgatttgcgtctgaatgttatctagtagaactgtgcgccaataagcagcttccagtgtataagggaagctgcttattggcgcacacttttttgttcaaaacttacaactctctaaaaaggtttgcgattctgttaaggaaagtgcaactttgtcacttggtttgcgtttttaagttgcgtttaagctgccaacgataatctagtgacaatcaataacgaagggagcaatgccaatgccacatcaaccattcaaacgcaggtaaatcatcaagcagcacttcaacgaacatttcaacttaacaaaatcgattcactaaaaaatgaaaccaaaaaggagatcatcaatatgaacttaaaaacaatcttatacgcaaccggtgccgcaatgggaatcttcacaacgagtgcagtgactggcgcaactgccaacgctgccgttaccccaaccccacaatctcaacaagctagtaaaacaaataccaacagccaaacagctaatggcaataagacccaatcgaacaaccagtccaagagtaacactgatcaagctgctaagaagacggatcagaataaagctgcaacgataacgccagccaaaacgcaaaccacaccggccaaaaccggaaaccaaaccactacgccagccaagtcaaattcgagcagcaatcagcaggcgaataattcaactcctgccaaaactacgaccccagctaagacaacgaatagtacagccactgcgactacgtttgatcaacgagccccaaggctaaccggttcagcttataagagtgaaaatgccgggtttaaaccaactgtccaaaataagcacgctaataaaaatgtgactgtcaaatactcaattaacacctacgaatctgacggttcagccagctccaagccgttccaaattaagatctacaaagacggcagcctttacaagacgattaacgcatcttctggtaccgcaactgggtcattcagcgctcctaaaggtacttacaccctgcgtgtctacaccagccaatcaactcattacactggcggtttatcagttgaataaaaaaatcaaataaattttagccatttaagcttcgtttaagttggctgaggtaatctatagacaatcaaataagagaggagggaaacaccaagcaagcacatcaaaccaaacccctaatatgatttctaatcagctcccagatgactgtctatgcgaaaggaaggatgaactgtacatgtcaaaaaagacccttttaaaacccaagtttaaatacgcatacggttccaaccagcatcaaagatttgtggtctggagctgctactaaaaccaagtaccgagttaattcaagaccgagcgctggaactcactaactcattgaaaggactgatgccatggagaataatcggatttactagcgtatcacaatataatattcacccctcaaataattactaagaaatacccaacaagattgacaagattcttaacttcatgaaatacccctcaatatgaattgaataagaattacccctcaatatgaaatataaaattcccttagaaagtcctgtatgcgagcagggctttctttttgtcttcattcaaatttttaacgtgcatttgattgttggaaaaagcgaagttgcgtacaattagtttagatgttttaattcctaacgaaaggcggtgacaatcttgaagtcgagtgctgaatggtcaaccaggtggcctgaacggatcagctatgggttaagcgatgccgctgacaacctgatttttcaaatgatgacgacttatttgctgtttttttacaccgatgtctatggtttgacacccagtgcggtcgccatcttgtttgtggtcgcccgagtagctgatgtcgtcgaaagttttatcatcggtatcatgattgaccacacccattcaagatttggtaagagtcggccgttctttctgtggtattcggtgccttacgtggcttttgcgattctgacgtttgtcacaccgaatttctcctatggcggcaaactgatttgggcttacgtgacctatcttggtctggggttcttatacactgccgttaatctgccaatcacttcaattctgccgacgatgtcacagaatactcgtgagctgacactgcttggggttatccgccagttctttggcagttcagtccaaatcatcgtggcagttttcacactgcctttagtttggctattcggccacggcaaccagcagatggggtttctgggaacgattatcgtgtttggaatcatttcactatttttgattatcaacaccttcgtgcacgtgcgtgaacgcttctccaatccacacattgcccaccaaccggtcaaggttgttttgaacatgttagcccacaaccagccgtggattatcatgtcgatcgtgatctttatgtattggctggtcacggcgattaagaatcagacgaccatctattacttcaagtacacccttggcaatgaaggtctggttccctgggcaaatggctttactttggcagcgttaattggcgtgttaatgattattagactgactgatcaccaaagtaagaagaaaacgatgttacatgggatcctgattgctttaaccgggcaggcgattatcgctgccggcgtgtatggtaaatggctgctggttttgtttgccggtgtctttattaactcaattggaaacggcattatcatcggtctagtctcaattatgattgccgacactatccgatacggtgccagcatggggattcaggcagaaggtattttagcttcaacggatgattttggggttaactttggtctgggaattggcggcttgattacggccggcttgtttcacgtgtcgggttacgttgccaatcagtcacagaatgcggcgactttatcgatgatcaattggaactatgtttggattccactggtgatctatgccgggatgtatttggtgttgagtttatatgatgaacagcgaattattgatgccattgaaaaataaaattatggtgaaagtcgatttgataccccaatccaaccaaacaacgcacccatttccacgtcagaaatgggtgcgttgtttaattggatgacctgttccggaaacatttatgaatgcggcgtcctcaactgcatattagcattgaaaaattgtggatacgccaaataacacgatatcgtactgccgatgctggtggccgccatgagcataaaggtgaccatgatctggtacataatcgccttcgtagggtcgacaccagcaaagatcagaccagacatcataccagggaggctgacaatccccacagtttttgccgaatcaatcgtgggactcatcccagtccgaattgcttctcgtacgaccgtaatggcggtttggtaacgcgtcgctcccaaagccaacctttccaacaacccttggcgctgatcatggaactggctgttcaagcttcggtaggccaaaccaatcgcaaccatcgcattgctggcaatcataccggaaaccggcacgatttgactgggaacaaaggcaatcgctttagccaaaaccagcaagccaattgtaacccccgtggcaacagcaatggcaagcagactgatcacaaaagcatggggaatgcctttggcacggcctcttgcattccaagccgcgttgaagacaatgatcgctaccatgagaagtgtcagccaagctcggttaactgagatgatataggtcaggacgtaaccgacaattgtcagttgaataacggcacggatgacgccggttaccaagtctttttcaagaccaattttttctttgaggctgataaaaaatgcgaccgccactaaggcaactgcaaaaaataaagcggtcggggtaacaatcaggtgattcatgctgtcacctccattctgccgtcaacaatggtgataagccgatcggctgccgccaattcagactcatcgtgcgtgaccgtgataatcgtgacgccttgtttggtgaagttagccatcacttgatggacagtgtcttttgttgctgcatccagcccagttgtaatttcatctaataacagcacttttggcgtgaagatgagattgcgaatcaacgcgacacgctgcttttcaccaccagaaagttccgtaatgttctttgtcagcatatcggcagggagattcacatctgccaaagcttttatcatccgatcgtgattgaccggcttttggcgaatttggaaaggaaaggccagattgtcttcaacggtctcaccaaaaagactgggttgctgataacaataagataccatgcgacggtacgccgtcgtttcatattcttgttgtggctgacccgaaaatataatttggccttctgtgggtgtgagcaaggtggctaataataacagtaaggtgctcttacctgacccggaaggaccggtaatggtcacaaattctcccggtgccaccttaaaagaaatattagccaatagcgttcgttgtgagactgttaaaccaacgttttgtatgttaaaaattgcctctaccatttttgattcccccatttttttctattattgattgtagaggattgcaaatacaatgtcactgataatgattattaatttataatcatactaaattagcttgtgagtcgggcgtgacagtcgagtgctcgccgccatgacctaagttgaacgctaagaaaaagtgccccaaatatcatcgtaaaatggtatctggggcaccttgatttggacattattatttattctttcgcaccagctaattcaaacagctgagccattttggcggacccatcagcgtggaagctgaaggcaacttcactgtaagttgcccaattgtttaactcggtgtctcggtgttcggcatcgcaggtcagcagttcatggctggctgtttgggcagtctttttatacgatacataaccattggagttgtacaccagaattgcgccttggccggaattgtaagtcgtgatgccatatggtgtgaaataagtcggcaaaacggccatacactctgcgtagccactccccgaggcattataggactggccatttggacgaacgtgacttagcttggtccacagttctttggaacgaacgatagttttagctttcagtgaagatcgatgcttaaaagccttgagtcctttcgtcaatcgataagcattaatttgtttcatgtactgtgtgtcaaccttgcgagccaatgttgattcctttatgtacttcacggttagcgagcttggcatgctggcataggtgtaattctgctgaatcttgtggggtaaatagcccttgattgttttgacatagccggacttagtggccggataaccgctggtcgtatacgtgtaggtggtaccaaacgcattaataccatttgaaatgcgggtatacgtaatgggcgcccgtaatgtttgccccgatgttgaaacgtaattaaccgtcatagttttggcggctttagcgttgccgccaaatacggcagccgaaaccagtcccaacgtcaaagcgatgattgataacaattgactgcttgatttcatctatatccccccaatacggatcgaaattattaagaatttcttaagtgtttgcaaattcattatagcaaattatgccggagggcgttcaagaaaaaatgaattatttcgtgattcttcgagtccggatgaaattaatgattcgggcactcgtggtaaccgttgtccgcagcgcaatcccgatgatcaccacaatgaggaagtactgcggtgcaaagtaagaaatcagcaggtatagcagactaaatccgagcatgatctgagccgatctgtattcttcgcggtcatgagccgacattttgatcccatctgcttcaccgatttcaatcacttcgtggaacatgattgcctgggtcaggttcaccaagataatgatgactgaataagccattgttggcagctggtggccaaaatcgtcatttaaccaagaggtcgcaaacggcgtcaaactgatgaaacagaggtaataaatgttggtgattgtaattaaagacgttgtatgctcgatgcgactaaatagttcctggtgataaacccaatactgagaaacaatcccaaaactaacaaaataaatcaccaaatgtttgatcagatccagcattggtccttgcgctgtactgattggcgttttgatgtccaagaccataatggttagaaccacagcgaatatcccgtccgaaataccaattaagcgtgattttgaatagtgaaacaccccgatcatccccctagattagtgtatgagctcattttacagctctttggtcggagagggtagttcggttatgaaataaatggccggttattgttcttttaatttgcaggcatattcaattattgatctgcaatgtcattaacatactgttatcaatatcaaatcaaaatagttatgtttttgaggatagtgtgataatattattttgtaaatcaaacgggaatggaattcatataggagtgatacttatgcgtgttttaggaaagcgttcatttattacacggtttcaacaggtgtgtatggccgtggtagcattcttcgcagttttaacaggccttggattttcaacaacgtccacggccagtgctgcaacaccttcaaaggatattttgcgaccgacacttgcgataactggtgatgacgttaatgggaagcagcagacgattgcttcaatccaaagtgttgctgatccaacaactactcatgccttgctgaatgtcgataaatattcaaacatatatgctcggtattcagttacaaatgacttagggtattcattgccagtttggaattttgtccatcttccgtggttgtttgatcacaccgcaaataacccaaaatccttagtttttgacccaagccgaggaaacccggaaatgaagtcaattgggtttgccagcgatctcaaagaaccaatgatggaatcatggtcatattctcaagacagcagatatgttttacaatatacaccatcagaagacttaacaagtattttttatggtggaatgactgacacaagtagtgtttggccaattcagatggctgcaaatgcaagagttgagatgacagttccattgaaactggcaccggattttgactttaatccatcacgtgtcgctcgatttagaagtgaaatgcaattctatacggacaataccagcgtggataaggtggtaaaaaatgaaattacactccaaattacccgaacccttgacgttgccgacttcgaatccgacacctacgcaacgttaaccaacgctgataaattcaaagggatcaatcatacgtttgatgccgatgggaaggaacagccggacaagaccaaagccgacgccaagatcaccccaactgatcaaaaaggcgtttacgatgttgcctacacttacgatggggttaccaagaaagtgaaggccactgtcaaagatcaatcaaccatcgaggctggcgactttaccatcgctcatggcagcaactgggacactcagaagtttaatggaattaagagtttgactgacgctaacggcaataaggttaaatcgccaggtaacgtgaagattaccaatatcaaagacgcagccggcaaggatgtcgacaaggtggacaccaacgccgcagagaaaacctataccatcacttacaccaatggtggcgcttctcaaagtgtcaaagtaaccattggcaaacgggccagtgtggtgacaccacctgccagaaatacaggttcgacaagcagcacagtgaaggttccgggacgaccagttacggataactccaaagctagcggtggcaatactgctggcaatacccagacatcaaccaaccagcagcctgccaacaattcgcaaccagaaattcagtcttccccaggggtcgctaagaaaggcgctgccgtgtacgccaagaagacaatttatctgtacaagggcgttaatttcaagaaagcggaccgactggttaaatatcacaaagcacaacgcgttgatcgaccgatgtttgtggttacaggatatgatcgctcaagcaaaggcgccttaagatataaggttcgggatgtgaaccataccaagaaatctgatgggaagatcggctacattacggctaacactaagtacgttgtcaatgtttactaccagaccatgccaaagaaaaatcagctcacagtgatctccaagaaaggcgttcatgcctataagaacgtcaacctgactgggaagacaaagacttataagaacggtacgcatcttcgggtcaagaagattgtcaaatatcatttaacgactcgttatcaacttaccaatggcgattacatcaccgccaacaagaagttaattattcaaggaaatcactaaattattttccagaaaaagtcctggcatccgctgctcaggacttttttgatgggtaaaattctcattacaaccgatttgcacacaattgtaagcgctttgtacttaagtgatcgacttccccttacataatagttatgtaataacatattaaacaaattagtactaaaagcaggaacaaagtggtactatgtgggtggagtggggaaagtatgaatatcaaattatgagggagtgtttatgatggatagtcgaattagcaactcatcaaatttgaagtttcgaacaaaacacagacggatatggaagatcctaaccgggatggttaccacaatcgcagtcgcgtgcggattgggatttatgcacgcttctgccgatgatgtgaccaacgttatccagcggaccgatgaattcaatattagtaaagtgaatccactgcaatacacatacgtccatgagagtctcagtcacttgggagggtggcagggggcagcttatgccgccgcaattcctaacgatgccaagggaactgatccgaagaccggcaactcgtacgttagtgaatggatgccggatcctggacttgagtatttcatttggcaggcagcctttgccgacaagtacaaaacggcggaaagtttttttgccaacttttcaaaaaatgatttgaaggatcttgagtcactttatagcgaaatgggcccacaaaatgccgggaccgactcaaatccaaaaccatcccagtattatatggctttaatgggaatgaattctcttgagggactgcaatatgcaacgaaactcaaacagattaatttggatcccaacgtctctgtcagtgcggtaacttatggaacagcgactaaaaatggtaatttatgggatatcagcgcgctaaaaaatttgaatcaattacagtcagtgatgatccaaatgttttcgattaatgatatttcagcgctggccaacaagcctaatttgaccaatctttcgttgaattacaatcaaattgccgatttgtcacctctggcaactaacaaaggtaacaaggggctgaatttgaagaccggattcaatcaccaacacattcttttggaaccggtcactttgcggggcagtgccgctacggctgctcaaacgtcgtttacgactccgtcctttatcatcaaggatttggaatccgccaatttaccggtgaaggcgtttgacatcaaaagtgaaaaatctgattatcccagtttgtacccaagcacctctgatggcggcaacatcaatcccaccactttgacgtggacaaacttcttaccagacaaaactaacttgtatggttcgttgtccagtcactggaccgatcccaactctgattttgaaggctggatcatggtgccttatcagtttaaccaaacggtcggcaatgtctttgtgaactatcagctgctgcagtccaatgggaatcaactgcagttggcaccgaccagcacaatggcgggaaatgttggggatgcctataatattggcaataatccaaacacggcttacaccctgaataaattaatgggagaagacaagcgggtggcaattggcgtgtttgatgggaccggcttatatgccgatttcaaagccaataacggcaaagccaacgcggttggccagtccggaacgtacaccgatcttcctcagactcggacgattgtgtttgcatcggattcatcaaccgtcacaatcaactacgaagatcaagacggcaacaagctccaagattcaacggcggttacaggaaaaaccaatactgtttttaccttaccgacaattccttcaacaatcaccaaagatgatcaggtatacactttgaaggggctcaaggaaggtcaaacagtgccagcgaaatttgattttatggacatgtcactgacctacgtgtatgaagtcaagccaaccgaaagcaaaccagtcaccgttcgatatgttgacaaggacaatatgcctcatgagattgggccgcaaaaggttttgactggcaaacgggatgacacctttaatgtgaacagtgatgattacaagttgaccattccgggctacacattcgcaggtattttaggtgatgcgacaggaaaatttggtgacaatgcgcaaacgatttacatgcagtacaccaagaatcctgcccagccaaaatcagtgaccattcggtacgtcgatattgacaacatgcctcacgagattggccctgaaaaagtgattaccggaaaaatcggtgacaactacaacaccactgaagcccagtacaaacttgcaatcgatgggtatacctttgtggatatccaaggaaatgcgacgggtcaaatcagtgaacaggggcagacggtctactatcgttataaacgggatcaagcgaaaaatgaggctaaaccgattataatccgttacgttgacgcagataacatgcctcatgaaattgcgccaaccagaaccgtagccggcatcattggtgacaaatatgatgtccgtgacaatatgtacaaactcagcattaacggatatacctttaaagatattcaaggggatgctaccggaacctttgacaccactggacacacggtctattatcgttacaccaaagataaagccaccccagtgacgccgccggttaacccaccagtaacgccggtaaccccaacgccgacaccacagccgacgccacaaccaactcctcagccgaagtcagaaccgacttcacaggagacggtgacggcaccaaatgaagccggcaagattgccaagaaaggtgaagcggtctattcactgaagaagatttacctgtatcggcacgctgatttcaagaagggcgaacgacttgccagctatgccaaaaagccgcgggtaaatcggccgatgtttgtcgtgagtgattatgccaaatcaaagaatggcgctctgcggtatgtggtgaaagatgtgaatcaccacgccaaatcagatggaatgaaggggtatatcaccgctcggtatgcttacgtccgcccagtatattaccacagcaagcaccaagttctgacaatcattaacccaaccggcgtcaatgaatataccaaccgaaatttgactggtaagattaagaatttcaagcagggcactcaactcaaagtgaagggatttgtcaaacataacctgactacccgatacctgctgagtaatggacactatattaccggtaaccggaagctggtatttgccagcaagttggttcaaccaaccaagattaaggttaaacggtcgatttacttgtacaacaacgtgaacttgaataaacgattgaagcacatcaaggcaggaactgttttgaaagtgaagaagtgggattactctcatcagtattcaacaacgacctttggtgctaaacgatatcttgtcagtggtggatatgtcaccgctaatgggcattttgtgaaagttgtgaagtaaggccatattaaaagcttcggtgtcagtagctggcatcgaagctttttgatttggacggagtcgttattttacaaattcattgatctaatcacgattttaaaactggaacttccagcgttgaatcgtttaagttcaatgtgtaagtgatggcttgattaccgtggacagtgtagaccaggtcactggcatagattaccaaccccaattgatgacctttgagtaagtgccaaaaggttggctggaaggcaaaccgtaattcatagttcgtacgcggctgcacatcatcgactcgataagaattttggcggttctgcatgttgatgtgagcttcggtgattcgtttaaagtcggttgggtctgtctgaggaagaaattcttttaaatcatgctttcgccaatggtaaccttgcaaaatcttttgggaaaccagcgtttgagggacttcagttaatcgttgcgcctcaccgtagtcgacaagggcaacgctgatttggccgacaatggaactggtttgggcaactaaagagatcctcggttggccatcaattgtgagatcgtgtgtcagtgggtcggacaagagccgaatgcagtggttgtccatggcggtgccttggcgtgaatataaatcattgcgccagtcattaaggtgctgggtgtaatgctcgaaaacctgttttggcagctgatctgagaaactgagattaccattgatgttattcaaactggcgagcgagaaagtgcgcttagttgattcagatccgccccagtcaggatagtcatgccacgtttctgcgtgggcgttgtcctgaacgattacatctggcatcacgtcgtcgacccgattttgaatcccaaatagtttgttggacagccacaggtttaccaaatcggtgtaatcaaaggagcgaaaattgttgagatactcgtgctggccttggtgaaggatcaatttttgcgtgatatcccgggtctttaacttattccgggaattccagacttgtccggtcttgacgttccaatcattcaaaccgtgaaccagtagcatatccgccttggtatgattatatttggtaatgtttcgggcgtcccaaaactggttgaagctgccggtatcgtgttcttggtcgtgggtcatttgttttaaatgtttcagccaggcgtccttgatttgagcataatctccagcagttcgttggcggctgaaagtccattcagccaacacatcggcatcatcaccatcaggggcaaccaccaggccgttttcccgataataagggtagtaatcggataagccggcctccacgatgctgatttttaacccgtcaacgccagtaaacgcggctgcggtggcaagtgttcctaaataagagcggccagtcatcccaacgttgccgctagtccaccaagcatcaatcgcaatttgatcggagcggttggtaaaggcagcgcgcttgccgttgagccactcaatgaccgccgttgcgctaagggtctcagccttggtgccggtggttcggaacccatcggagtctttggtaccgattcccgatgagtaaacaacggcgaacccccgagccagaaaataatcattgagagaatacgaccaaaatttggtaaaggtttcgccggttttagtcgtttggccgttaatttttcgcggcttaggtggggtaacgttgctgggttgtgcttcaacatcttgataggttaggtgatttggttgttttcgcttgagcggacgtttgttgtcgagggagaatttctctgaccatttttcattcatgccttgggcgtatgggtcggcagtgaagataaccggcgcttggtagccctcgttagtttcagcaggccggatgatattggtttttaacagatcccgtttaccgtcgtggtccgagtcaagggatgattcgacgtagatgacttcacggattaatttatcagtattgaaaacggcttgggctttgccgttgaagaatagtggtattttgaaatcggaatcgttgagaaactgctggtaataccctttgccagctatgtagtcgatcaggagttgaccgtatttgttccgggtattcaacaaccgataccaagcgtcgattagctgatcacggttcatcgttgactggttcagcggtttcggtaggcccagttgcgtgacggccttgaatgggtctttgagggaaaaatccaatccgtctaagaatccaagtaattggaggccaatattatagaacgctttagcggaccgggaccagttgccttggtgaatgttgctgcatcaatcgtttctgttgccattaagttgtgaatcttttccagtcgagtggttagggaagcgtgctgggagaagtattccagcaaaaaattgcgatagagttccatcggatcgcttatcttaagattggtcggattcaaaaaatgaatttctgtcagttcattgattatttgttgatggttggtggggacatacccgaattggttgattttcattaagtgacctcctgaatgtaattaatgccattatacatttgcggcttggcactgcaaaattaatttaaaaagcagcgattccgcttggtggttaaggaatcgctgcttggttattctcaagttgttgatgaagctaatctgaaatcaaatcggctggttggaaatcttttaacctgggatcctgtgctactcttcatgcttttcttggtcggactggtcagcgtcatggtcagtgggtttggaattttgacccggctcatatgattgagctttagcctgcagcttcttttgcttgacctcatgcttggcatcccggcgttctgctcgccgttgggtgcgtttttgatgctcaagaattttatcttcttcgtgggcagcccggcgcttggcctttgcctggcgttcaatatctttggctgcctgtttggcagattctttatcagcttcctgttggcgttcggtttccttggcggcttgctttgaggctttttcacgggcttcacgctgaatttcggcttcttttgcagcagcttcggcgtcatgcttgcgttgatcttgctgctgttcggcttgtcgtgctgcttgtttgacggcttctcgattggtattacgctgttctttacgaatttgctcagctgcgtcacgatatttcttggaaccgtcacggatttgcttggcaaattcttcccactgtgcttggcgctcttttctgacttcaacactgtcaggattattgctgggagcgtgtgggttgaccgaatggccggcactgtcggtggcgaccgggtgatcaagccaaccgctaaacccatgttggggatgactcgcgtttgacgttgttccgtcagttccggttgctgcctggtcctggaccatttctctaaattgattaatggcgttctgcggcaacttcaagtattcctgtcgctgctcggtggtcaattgcgaagcatcgtacatttgttgacgatcgcggctgcttaggatcatatagacgattggatagggaaggtagaaccacaagacaacctgcgggaaaaaataggccaggacaatcaagacggcgttgaaaatcaaatagtattgattgtgacgcccatagattttccgatacagctggcgcatttttgatttgtcagtgtactcaaagtgcatgactgatcttgcaagcaggcgaaatgatgctgaaaccaaaaataacaggagaccgtatgccatgaccggaatccgggtggtgttgctggccatcatgtttgtggccagtggtgtcagtgatagtgggattaagaagataaaatcatacaacatgattcgataactcatatcgtcaatatcattgaacaaggtggcatgctggtaccacatgttggccacaaaagcgaagctgataatatagatgccaatttgtttgcttaaaaacaagtaatcattcaagttgtcccgcaagactggtgttagatccaaaaccataattgtcaaaataatggcgatcaccgcatcgctaaaagcgtccagccgactcttcaactttttcatttgttttgccccccagaatcgatttagtagtatgtattatgctttaaatgtagcacagtggccgtcaataaggtgataaattgtttaagaaattttatcagtctcacaaaataattgggtggcgatataataaaactaattaaatgattgtgaaagaggtggcagtatgtttccttacttgggtctcaaagccagtaccaaccaagcccaaattgatgaacgattaaaatatcaccctgaagtatttgaatttttcaccaccgatcaggatgtgacgccaagtggcctgaatcacttgaaggcgatgattgaacacgtgaaggccgctggggtcgacagaatgtcatgcaccacccgatgaagattaacggccaacacaatgaagtggcagttgaccgattgagcaatccggatgcttaccactttttaatgcagagttctgaaaatttgattcagctggccattcagactaacacgcaagttttgattcacggggcctacaactcaccggtttcagatattctcagcaactatccttcgattgattccgcccgcaaggtggtgttcagccgattggaccattttaaatcactgggcggggaccatgtgatgttcgaaaattccatttcaccgttgtttgattacggcgatccaaaaattgaaaacctgatcattgagcatcaataccggctgtgctacgataccagtcatgggttcattgtgctgcacggcgataattcgaaactcaaagccagtatggcgcatttgcgagatcaggttgtccattatcattttgtggattcaatgggccagttccacgacagcttggaactgggaaagggcgcgatcgattggcagcctttaaaatcggtcgtcaatccggacgccaccgatatttttgaaatcaatctcaaagaccaaatgaacagtcaagaaatgcgtgccagctatcagtacctaaaagcctcttggcaaacatccggttgattttgttgtaagatggaagtagttggtttgggggagttacatagtgaaatttaaaaatgtctttgcatttatcattgtttcagtattcatcgtcatggccttggccgctgctcaacattcatttgcagttcggaaggcagcaacgccaagtgatagtcagaccaccactcaaagtgtgtattggaaagcgccgtctgaagacaaagcttatccagaatggtccaaaatgagcaagccttggatttatgtgagtgttaaacaacagaaagtcttcatccatggtaatggcaaggttcaatacattatgaactgttcgactggcatccccagcagcccaacgccacggggaacgttccatatccaaaaggaacgcggctattcattttataacaagcgctcacacgaaggcgcccactactgggtttcctggttggatcacggcgtctacttattccacagtgtgccgaccaacgcccacggtcagtacgtggtttcagaagctgagaagttaggcactcccgcatcccatggttgcgttcggctatcaatcgctgatgctaaatggatgtatcaaacggtgccgtttggaactaaagttgttgttcactaatgaagtcatatcgtctttattcgatgaatgaggctgagacaaagagctaatctgtttgcctcggcctcatttaattagttaaaaaggctgggatttccacgctgacgaagaatgatcagacgttctaaataattgactgaaagaaggttctaacatgacattgcataccattttaactccagagtggattcatgaagccaaattgattgccgccgagaatcctcggctggagggctttgttcccagcgagggcggccttcatccacgaattctcttgttgggtgaagcccctggtgacaaagaggttaagattggccgcccatttatgggcccatccggcaaagaactggatcgctggctggcatcgctggggttaacccgtgaggatatctacattaccggagttgtcaattcccgtccattttcaattgggaaaacgggtcgaaaaagtgaccggcgccccaatcagaaggaagttaagcgctcggctgcgatgtttgactgggaactatcccattttcctgatgtcctcttggtgccaatggggaatgccagtcttcagcggttattaggtaccaaggccaaaatcggtgatttacatggccagttgttggaacgcccaattcaaaaatataaccagcagacagattcctttgaactctctaaggaaaaacatcaaatctttcctttgtatcatccatcgtattcgaagcggttcaagaatatgaagcccgtggtcgatgcggattcgcaaaagctcaaacaattactcgaacagcaatcaaaccgtcattgaacgccgaatatgggctggatggtgttagtctataatcaaatagtgttttgaggaaggtgaggatgatggcaaaaccgttaaatggcgttgatctctatcattcattatttggcactgagattcacgatccacgcgtgttgtttgaaatgctgacggtgaacgtttttcagccaggactaaattggcgggtggctgccagcaagattccggtgtttgataaagtcttcaagcattttgacgttcacgaaatcgccaagttcgatgaaatggatcttgaagctttggaagccgatccggagatgattcgaaatccccgcaagattcgggcggtcgttcagaatgctcaagcaaccttaaagctgcagcctgaatttaaagacttggcggactatttgtggtcgttcgagccaaaagatgatgtggttcgcggatcattgcagcgggattcccatggcttgggagctgagctggccaaggatatgaagaaacggggcttcacgttcgtcggtccgaccacgatggagttgctgctgattggcagtggcattttgaaacatgaacatgattaggaaaccttcaagcagactaaaagagagcggatcgccaagtaggctaggcaggctttcagccggccgtcgttgcacgtttaaactagataccagtggaactgaagaaaggttgaaacataacttacgattagttgtgtctcagcctttttttgcgatctaatgctcagcatcaggattaatatagttccacaatccagtttttgtcttggtcactgtcatccaaatactccggatgatcgatcaaagcagtgttaattttagccactttaccggcccttggtgaatggacttccgtgactgctttagccccttcaaaggagaggatgacgtcaccttctgcaacttcactgaggttctttgggaatgccgcaaaggaaatttcaccaatttcacctcgcgccaggtcatttaacccaattcgagtatgtgaatcatcaaccgttgcctgccagagatattttgaatcatcaattttttgtgccatattaatcttcctttcaatttgtaacgttagagtgacgagctttattgttatggtagcctccgggttgacagatgaaataatataattcatctatcaatctggaggcttttgttatgccaagaagcaagtaccgtgcagaagaaaaactggactttataactaagtttcaacaagaagatttaagtatcgaaaaatttattagtaaatactctgtatccgtttcacggcccacctttagtcactggctggattgttatactcgtgacggtcttgatggattaaaagagagtaagaagtggcaacattattctaccgagttaaagcaacaggtggtaattgattatctatctggtaaaggatcctttcgttcaatagccaataagtatggattacggtcaaaacgtcaggtggaggtatgggtttccaagtataatgggattgagaaattgacagcaactccgtcacgaaagccaggtcccgataatgacacggaaaaccacgtttgatgaacgcgtcaaaataactgaatatgccctagctcatgatcgtaattacaatgaaactgccgcgaagtttcaggtatcgtaccagcaagtgcgatcctgggttctgaaagttgatcaagggggttttcctgcccttaaggaccaccgtgggcaccataaggcgccgtcagagctggatgaagttgataaactaaagcttgaggtccgccgacttaaggctgagctcaatgataagaaggcaatcgaggctttcgcaaaaaaattgctcgccctgaaacggaaaccgtagaagggcgtcaggctaacttcgatgcctatcaattaattaaaccgatttcaaaaaaatacggctgtcgcaaggcaattcttttaaagatgatgggtgtctcacgacaggcatattggaaatggttaaagcgttctgctagtgatcgagaggctttcaatcacatgttagaagagaaaattaaggttttagatagcgaaaatcggcatacatttggcagccgccagctggcatttaatctgaatctcgatccagaagtgactgaacatattggccgtcgtcgggtaactagattgatgcgaaaactcgggattgagtgttgtgtccgaaggaagagacataatcgaatgaaacaatcagagcagcatatcaaggataatgtgctcaaccaagaattcgatcaagctaaacaaccagatcaagtttggctgtctgatttcactcaactggcctacggttcgcatggtgaatacagtgttaagctatcaggcgttttagacgtctatagtgggtacttggttgcccatcacattagtgcgacagaaactaaggaagccgcaatcgaaacctttgaaaaagcctttaaagtcgctggtaatcccagtccactagtgcatactgaccggggatcggcttatgtttctggcgacttcaatgactttatgtttcagcataatgtccggcgcagtatgtcgcgccctgggacaccctatgataattcaatgatggaacgatactggaatgaatttaaagtgtgctggatcaggacacatccacgaccaacgacttaccaggaattagagagtttaattgaatcaggtatcaactatttcaattcagaacgacgttcggcaaaaagaaatggccttaccccggaagaataccggaataaagccatttctaaacaagtaactgcatagttaattttatattatttcaaatgtcaacttgacaggccacagtgcatatagagcttgagaatctgttctgtttttgaaatggcattgttaaggtggccgtccggcctcattagtgtgtcaaggtcatcggaacttaaatacttggcaatggtgggatcggcgtaaaacaagtcccttaaagtggcgtgttcacgatcagcttggtcacgcagtttcactagtaatcggtgggcgttttctctgcccatgtgcttggcgagggccatcatcaatgatccggagtacattgtgccatcgtcagcggataagttctgtcgcatgcgctgggcattaaattggccaaatttaagaatattaatggcgtagttcaactggccggaaaggtacattgtcatttcagggagggcaacatataaatcacgccacacggtggtgtccttctcaccatcaactgacattgtgtcgtacatcagacccatctcgtttcgaatgaccgttgccaaattgacgaccgcttcgaccatatatgggtttcgcacggtgggcacaacagttgatccttggcggccgggcgcataggtttcctgaaattcaccaacaattgtctgactcatatagagtaaattcttgcctaatcggcccagtgcctgggcaatcatcgtttcgacatggcagtattcagtgaatcgttcccgctgcgtgtgccaatacatttccggttttgataatcccaagcgatcacaaaaatcctgttcgatctgatcatagtcatcacccagcattgaagatgtcccgtcggcacccgctaagctgccagcgaaggtaaatggcgccagtgaatcaagcttgcgcatgaggtagtccaattcattcaaaacaatcccgagcttgaatcccagcgtggtgggggaggcgtatgttttgtgggcgacggcagcagtgacagtgctcttgtatcgttcacacaagtcataaaggaccgaaccaagttgatcaagataatccttcagcacccggtcagactccttaagttgaagaacaaacgcggtgtcttcgacatcctcactggcagctccatagtgaatgtattgcccgctgtcgtcatcaaaaagtgactgacaaactgtgacaaatcccgccagaaagtgtccagctctggctgactcaatttttaactgcaccctatcaatattttccggaaccaatttggcttggatttcttggtaggctttatcagggatcttaccgtttttggccattgcgtaagccaccgccgtttcaacttggcaaatgactttcactcgattttggtcagaccagatatttcgcattcgagccgttgaataaccattttgattgtacagcgaacctagcatttcaccactcatgttagttcacctcctgaaaattaggattaagcattaggtcggccatttcagctgctgaaatggggccaatgttagctgataaatttgtcgttctgaaggcttcttccaggttgtctttcttaaaaggcgttccgatcagcttatcctcgattactttcaagtgaccattggcctgattaaagtcgccaaagatgcgtgcatgggtcacgatgccatcatctactgaaaaactgatttcgaccgtgccgagaccatcaaagtgattcccgtggaagaaatcatcgtcgcgtttggttcccataatgaaatccggatcggtgaacttgttctgagcgatttgttcaacctgcagccaatcctcttcagacattgtgtaggtgggaatagttgtcaagtcagtcgtttgaaagacttcttgaagaagcagccggcgcatttcatcaaaagtgatttggcgatattgtggtaggaaatactgacgaatgttggtaacccggctgtgaaccgacttgattcctttggaggccaacttggttttgggtggggttagcgcttctgcagcctgatccagatcgacgtctatcattaatgttccgccgcacgagaatcggttgccgattttgagcgatgacatccccgaaaactttttgccgtcgactgtgaggtcatttcgaccggtcatttccgcgtccaccccgagcttatgcagtacatgaatggctggtgttgcatattttttgaagttgaggtaattcgtgccatcgtcattatcgataaaggcatatgtcaaattacccggatcaacgtaaaccgcaccgccaccggcgccacgacgcgccaaacgaatatcgtgggtcttaatataatctaaattaacttcggagtatgcgtcctggttgacgcccagaacaactgatgcggccgctggttgtgaaaaatgaaagatcgtgtcggtaaatttaggcgaagtgataaaaaacgtcgagagactgccgctgactcccgggtcgcgcaaatgccgttgtgaatttggatcagataagtcgacaaaaataatgattctcagtcccttcaaaaaaattcccctgttaacgattacatagaaaagtatagcacgtccgggttaaaataaaaaagagcggaatagcccatcacaatggctatttccagctccctattgaactaaaacgataaaccgattatttttaaaaaagttccacaatccaagttctatcccgattatcctcgtttaaaagctcgggatgctcaattaaatccgagttcactttggcgaccttgccgctcattggtgaatggatttcagtcacggctttggcaccttcgaatgacagcattggatcgccgacacttaattcagtcatcttttccggaaattcggcgaaggtaacctgaccgatttcactacgggccaagtcgtttaagccgattcgagtgtgtctttcactggttttttcttcccataaatatttggaatcatctgctttatctgtcatgataatcatcctttcattatttaagatcgtacttctcttttaacattaaatctgccatgtcaggtggcgttattttgccgatgttagcttcaagattgctgattctaaaggcctcttccaagctgtccttggcaaatggcacgttggtaatctgattttcaatggctgccaaatcaccattgggattgttgaaatcaccatagatttttgcgtgagtcacgacatcgtttttgactgagaaactgatttcaacagttcccacgccgtcaaaatgacgaccgcggaagtaatcatcattgggtttggtgcccatgacgaagtcgtcaccggtataggcttgatcagcgatttttaagacatccttccaatcatcatcagtcatcgtataggttggtacatcacgaatatcggtgactctaaagacggtcagcaggatacgtttttccagttcttcaaacgtgatatttttgtatttcggatcaaaatactgacgaatgttggtgacccgactatggacagatttgatgcctttggattgcagttttactttcggcggggtgagggctttggccgctttggccaggtcaacatctgccatcagagtaccgccgcataaaaagcgatccccgatttttaatgctgacattcctgagacctttttgccgtccacggttaaatcatttcggccggtcattttggcgtcgacacctaatttcttcagggttgaaatcactggttgggcatagcgtttgaaatcgccgtaatttgagccgtcgtcgttgtcaataaagacgtacgtcaaattgccgggatcaacaaacacggcaccgccaccggcaaaccgtctggagagttgaattttttgatcacggataaagtttaaattaacctcggaataaacatcttgattcaacccaatgaccactgatgcctgtgggggcctggaaaagtagaaaatcggttcagtaaattttggactggtgatgaagaattttgagagactgtcggtgatgatcggccggttcaaatagtctttaccactggaaatatcaacataacggataataatcagctcctctgattgaagtaagcggttacaaaagaattcaaaaaacaatgcaaccggaccttgactctgtctaattgcattgtaacccattattgggggagttgctcgaaagttaactgaaacgtgcgggtcacccagcccacgtggcactgtggttgaaatgtgctgcgagcaactgacactgcgatctaagtcactttgattcaaatccaaacccgggatttcaatcaaagcgatcttagctctctgtgtcaaaacgttgctctccgcactctaatcaaaatgtgctccgccgagcagcaacctgcacctaagccaacttcggacaaaatcaaaagcgattttgtccaaagtcagcttaggctccggttactaaccgctcggctccgcactctatctcatgtctaatggttgtttagatgttggctttggaaattcaacatccaattgagccaactcattatcagttaacgtaatatctgcggctttaacattatcgaccgcatgcttgggatctcccgattgagggatggccaaggtattgccatcacggattgcccaggccaaaataatttgccaggcagttgccgaatggttgtcggcaatttgtttgacgaccgggtcattagtcaaacgacctcgggcatcaccagctgcaacaggtgtgtaggcaatcagtggaatatgccgttgcctcatccaaggcagcaggctgtattcaatgccccggctgccgagattgtacagatcttcattggcggcaacctgatcggcattcggcaaatccatcagttcttccatatcagaaatatcgaagtttgagaccccccaatgcttaattttcctttttgctgcaattgttggagcgtcgcgatggtttcactcaaaggaacggcaccacgccaatgatacaggtataaatcaaaatagtcggtcccaactaatttcaggctggtatccaggctgtgttccattctggaagctgaggcatttgacggcaggactttgtcgatgataaacaaatcatcacgctgcatgtccttgatggcctcgccaactaagcgttcgctgcggccgttaccgtacatttcagcggtgtcgattactctggcaccggcagcaataccatcttgaattgctttaatttcatcagcccgggtgctggcactgtctcccatgtgccaggttcccaaaccaattgcgggtactgttgaaccacctatgttcaattctctcatagactgtcatacctcctaattttcattagttaatagtataaccctgataatggcattcatcatctaatttttaaccactcaaaaatttgttggccgactgcttcgggtaaatagcgaatttcaatcagttgattgccattgccatggcggacgttgactctgatatgcgctaatttggtatgggtcatccagattgattggacaaataaaaatgactggatattcttgtggggaatcacgtattgcgagcgggtgaagaaatggccatcttggagaatcagctggtcgttgacaatcttccagccggtattggcagctgaataccagcccatcaaagccgcgatgacaaccaccggcaggctcagtaatccccacaatttaaagagatatagacaaggcaggacgatcactaggctgatcaaagtggcattgcggatgaaataccagtaagctcgtttcgctaaatgatccaattggctgaagtgagtgggcgcccaattgacgaacggatgcagggtgtcaaatacgcgatcggttttcaccacgggtaagatcattaaatcattgcttttctcatcatcccccgccgatgacgccgccagtgcttggacggttgaaatgtgacaccactggcgaatcacgttttgtttaattcggagcgcttgaatccgggcaatcggaatagtgactgaattgcgttggaatagaccctgctcagttttaagctggtcgtttgtggaattcagccgaaaccgatagtacttttgaacgatggttaaataggaaccggcaatactgataatcacaattaacaagccaatggcgcccagaatgattgcagactgatgaattaatttggcggtcaacgaatcaattaacttttgcggaatggcttcttgaattttgccgtagaccgcaaaaccggccccaataatcgggaagacccccagtgaagtcagtgcgaagatgtttagttcatgcgggttgatttcgtagtcggcatgttcagggattggttttaactgttcggttaagtgttcagctgcaggtgcaggttcggcgtttccggtgcgctgacgttcaatttctgctctgacccgttcgttaactaatggcaaaaccgcttccgggccgtgctcatcgtgaccggcggtttcaatttgaagcttttccagatgaaatgggaccaaaaagaaccactgagtgtgctgaattgtttgaatccgggtgtatggaatgtgcgtgtgccgtttgacgaagatgccgctgttaattgtcagcatgtccgagtcgatttcaaatgtaaagcacaggtaacgaacggtatgccaaagaatgatgagcaggacaagaacactgaatcccaggagtggcgcgatcccaatggctgttgaccagcgggtaatcggcccggatccaataatcagcagaagcagcgtatcccaagaatgccggaagataaagtagatgattgacaatgggttgagatgctgttgattagacgtcattgttccgcacctccaccgccaacttcataatttgtttccggagttgttcgccaacttccggtttgacaccatcaattttgtgggacgttgaggccgtggtgatgcggacttcttgaagcttttgcgactgtaaaattggcccggcagaaagggtcacgtcctggacgcgggcgatgggaatcgatactaacttgcgaaagataaatccggaccgcagttcgacggcatcatcggacaaggtgtacagccaaaaagaataccgatacggaaccaggctcatttcgaccacaaaatcaatgatggcaacgacaaaaaagaatccggcagcgtacagtagccattgatagttgaaaaaatagtgaatgatgaccccagcgaccccgacgccggctgacaacagtgtgttgaagatggccgagattcgccaaacggttttgatttgggcgggtaaatgatttgattcattcatgtgatttgcctccttaacggggaatacgatatgtcgtgtgttaagtttacaaaagaatgacgacaattaccatccgatgagttttgaataagggaatcaatccggtagacataacgcggtttatagcgttatacttacttttatgcttttcacgaaaatcgaaagggggctatcaattgtcgaaaaaagttagaaacgcgataattgtcctgatatttggaaactttctggtctgtattgggatgagtctgatcttcccggtcatgccatttattaagaacgaactgcatttatccgccaccgatatggggatcatgaactcgctgtttgcaatcgcacagttggttgcctccccaattgttggtcaaatctcggataaaattggtcgcaaaccaattctggttgccggcctgctattatatatggtttcagaaattctctttgccatgaccaactggttgtggatgtttgatatttcccggacaatcgggggcctgtctgccgccatggtggtaccgaccaccaatgcattggctgccgacctgaccacgccacggcagcgagcccgagtgattggtttgttgtccgcggcatttagtggcggcttgattttgggacccgggattggcggtattttggccaagtttgattataaaacaccattctggttcgcagccggattaggtttcttgagtatgctgtcgttgtggttaatgctgccgaacgaaaaagaaattgagaagattgctgccaaccatcaagttcccgcgcaaagcaggccacccaagcgggcgtcttggactcaggcaaagaagctgtttgcagggccgatgggactactgtttcttctgattttaatttcttcatttggattagttggcttcgaaagtatttatagtctgtatgtcaacgaagtttttggcttcacaatgggcaatatcgctttggtattgacgttaaacggactgacctcgctgacatttcaagcgttgctgttcgacagactggtcgtttggctgactgaaaaacgcttgattcgctactgcttcttactctcgtttctgggtaccggctggattattctggcgcactccaaattagaagtgattattgcaactttaatcgtgttcacagcgtatgacttgattcgcccggcgattacgactctgctgaccaaagcaagtgccactaaacaaggtttaatcaatggcgttaacatgtctttgaccagtgtcggcaacatcgttggcccaatcgtttccggcgcgttgttggatgcaagttatcacctgccatacttggtcgtgatcgtcttcctgttcatttcatggatcatgacgtattggattcgggatcatttctcagttgatttgactgagactaactaggcttttcctgctgtgagtgggagaagcctttttttgctgaacggaatcggtagccaacttttttgaaatttagacgacattttcctatcatcgcctctcataatcagttacaatgaaagcgcatactggatatgcacaaatgattttcacaaatggaggtaacaattatggcaaagcaagttgcattagttactggagcaggtcagggaattggtgaagccatcgcgactcgtcttcacgatgatggattcaatgttgccgttgttgatttgaacatcgacaatgccaacaaggtagccaagaagctttcaccagatggttctgaagcgattggcatcaaggccgatgtttccgaccgtgattcagttatcgctgctgtaaacaaagccgtaaatgaattcggcgacttcaacgtaatcgtcaataacgctggtctggggccaacgacaccaatcgatacgattacccccgatcaatttaaactcgtgtatggtgtcaacgtaggtggtgttctgtggggcatccaagctgcacatcaagcatttaagaaattaggccatggcggcaagattatcaacgctacttcacaagctggagtggttggtaatccaaacttggcattgtactcaggcaccaagtttgcggttcgaggcatcacccaggtggctgcccgtgacttggcagaagaaggcatcaccgcaaatgcttatgcaccaggaatcgtgaaaacaccaatgatgtttgatatcgcgcatcaagtcggtaagaacgccggcaaggacgatgagtggggcatgcagacatttgcaaaggacattgccctcaaacgtttgtcggagccggaagatgtggcagcagctgtatcattcttggcaggtaaggattcaaattatgttaccggacaaacgctgatcgtggatggcggaatgcaattccagtaagagcgcgacgagccccgggttgaccccagagtataaggaagaacggtcaatgatgaacgtactttgttcatcgttgaccgttctttcttatacggccgggatcaggggcgtcggagcgtattttcaaggcagaagggagctgttagtaaaataagtgcctcaaaacctgtagccttttcgctaaagtaattgtgcagctcaacaaacggtcaatgatgaacgggctttgttcatcgttggccgttttttcttgtacattagggccctgggtcgtcggagcatagctcaaaagcagaagggagcagaaaataaaataagtgctgccaaacttgtagcctctttgaaaaggtattagtggagtcgaaaaaaggaccagtgatgaacggtttttgttcatcactggtccttttgacttgtgtagcaggggtcaggggcgtcgcacacggggctaggcaggctttcagccggccgtcggagcatgtgtataaggcagaagggaggcgtaactccaataagttcattcaaagctgtagcctctcttaagcaccactgctatcgagcctaaacgtgcggcaaccggctgatcccggccatttaagcgacgaaaacgcctcgtcccagaaacaggaataactcgtttcgtcgcttaaattctgggatgaaaacgcctcgtcccctactcagggcataatcatcttaataaaaatcggcgtaatataagtttccacgatcgcagccacaaacagcagcggcatcaccaggaccagcgtatccgtcagcgtctgcttcagcagctcaatgtatttaatatcctcgcgtttacgttttaagaatttattcatcccataccatgccaaccgtgcactgatcgcagcggcaatcacctgggcagaaatttcaaaaattccgtgtggcaggacaccaccgacaaacatcaggaaaggactaccaacgatcgaaatcaccaaaccgacactataggcattttgcaaaacataataccaataaatcggtaatggaatcacacccaaggcgatgacaacggcggcaccagcgaagttccagaaaaataatggcaaaaaattagttttgctgggtgctgtcttatcgattccattcgtaaagtgatggactagactgccggtgtccatgaagttcttggcatagatcaacacgatgatccagacgattgccatgacgatcagatattcaacggctttcttaaaatagatgcttttaaaacgatcaatacttcctctaatcataacctgtcccccttgttttctataatgaaagtatacagttaaattgtccacaaaccaattaatgtgtcattgcaatttcccttcaacaaatcattttcattggccgcgggcggtatggtatgctaaaggagtaccaacattaaagattggagatgtttgttcttggacggattacaatcaacaattaaattaaataatggtgtcgagatgccacgcttaggtctcggcgtttggaaaaccagtaacaacgattcacgagacgcagtcattacagctatcaagcatgggtatcgggcaattgataccgcacgtgaatatgggaatgaacccggtaccggtgaaggtatccgtgaaggtatgcaacaggctggattaaagcgtgaggacatgttcgtcaccaccaagctgtataacggtgaacagggcgactatgacaaggtttccaaggtgttggacaaacagctgtccgacttgggactcgattatgttgatttatatctgattcactggccggttgatgccacttatttggaaagttatcatgcacttgaacgcctctataaagaaggaaaagttcgggccattggggtatccaacttcgataatgaccgcatgagtaaattgctggaagaatctgaaattgtcccggcaatcaaccaaatggaatttaacccgacccaacaagaaaaagacattttgaactttgacagcagccatggcattcaacttgaagcctggtcaccacttggtgctggtaaagcattgaagaacccggttatcgacgaattagccaaaaagtacagtcgttccgctgcccaaattattctccggtgggaatggcagcgtgacattgtcacggttgtgaagtcagtccatgaaaagcgaatcgtcgaaaatagtgatatttttgactttaagctgagcgatgaagatgttcaacgaattaatcagttggatgaaaataagcgtgatctttggtatgacgactttacctggcataatccaaacgggcgttatggcaatgaaattgaaaaggttccggatattcaaaagtagcccgaaaccagatttatcaggagttttcgactcctgattttttattgtttaataatgactgcgtggttattgactccccagtcatttatgatagacttaaggcgaatttgaaatagcaagactttggctgctcgaaaggagtgggcatcatggaaaatcaattaatcttagatgtacaggggcttaaaaaatcatttggcaaggtgcaggcattaacagacgtgaatcttcaacttcatcgtggtgaagtattggggtttattggacccaacggtgctggtaagtcgacaacaattcgggtgattttggggctcatcaaggaatcgggcggatctgcgacggtctttggtgaagatgcttggaaagattcggtcaaaattcacaagaacctcgcatatgtaccaggggatgtttatctgtggccgaatttaaccggcggccaaacgattgatatgctgctgcatatgtctgggcaaacccatactgccaaaacggacgaattaatcaaagaattcaagctggataccagcaagaagaatcgaacctactcaaaaggaaaccgccagaagatcgccttaatcgcggcgttttcaaccgatgttgacctctatattttcgatgaaccgacctctgggctggatccgttgaacgagctcattttccagcagcgggtagccgaactcaaagatcatggtaagagtgtcttattgtcgagtcatatcttatctgaagtcgaaaagatgtgcgatacgattgccatcattcgagaaggcaaagtgatcgaaaccggttcactggaatcgatgcagcacttgacccgaaacgtggtggcaatcacaactgcttcaccaatggacgggctggacaaagctaaaggcgttcatcaattgaactttaaaaatgatcagcataccattgccgagtttacggttgattccgatgaaatcggcgctgtgatggatctgctgaccaagagctcaatcgttcaattgaagacgacgccgccaactttggaagatctgttcctacgttactatcattcagatgcgggtcaaaaagtaggtgagtaagatggcacaatacacacaaactttaacgttattaaaggccaatttgaagcgggactggcttaaaatcacgatttggctggccgctctggtcggcgttttcgtggcagtggctgctaagtttgaaggcatttacggcaccagtaaacaaattgccgccattggatccactttgcggtccaaggcgatggtcgctttgatcggcagcgttccagacggtcagctgacgacagccttgattttcgcatcggaaatggcggtattctggggattgtttatcattatcttcaactattcattagctgtcagcgccagttgcggtcaagaggaatccggcttgacagaaatggtcctcgggggtcatccggttggtcgcttggcaccactattggcggcagctttggaattgctgattgccaatggcttgtttgccctgattaccggcatcggcacaatgattgccgacatgccggggagtgatactaacggcacttggctgtcggcagttgccattgccgctgttggttgggcgtttggcatgattgcactgatattcgctcagctggttgctgacagccacaacgtttcgatgtacaattacgccttcttgggaattgcttatctcattagaatgatggctgacgtctccaaacctgattacacctggatttcaccactaggctggctggaaaagactgaaatttacgccaacaataattggtggcctgtcctgatgcttttggccttgggaatcctggcatttgctgccgcagttgccttaaacagcaaccgggacatcgatgccggggtcatccacgtcaatccgggcagtgaaaagagccatttcctccgtggaccggcaaccttattggtctggaatcaaaaatcattgacgatattctggattgttggcatggccattttgggcgccagctatggatcggtcttcaatagtatcagtaaaattttcaacacctcaccgaccattcaaaaagtcttgggtcaaagtggcatccgccatattgagcagacccaagtattgtcgtttgtcggtttgctgggaatcatctttagcttgctggcagtgattgctggagtgatgattgttaatcacctgataaccgaagaacgtcggggttatctccagatggtcatgaccaagccacaaagcagaccttatctgctgggagtttatgtggccttcggcttgattttggcagcactcctgcttttcgtagcgttaataagtgccatggccgccggaaatgttgtgatgactcatccaattgcttttaaatacttctggcaaacgttcgtcgctaatttgccgtcaatcgcattgtttatggccttgatggtgggcttgattggtgtttacccacgactgcggacactggtctgggcttatttgggcctttcatttctcattacctactttggtaacctgatggatctgccaaaatggacgctcaaaatttcaccgttttattggacgaaaaaagtcccgatcgacgcgattaataccacgcctttgatctggatgctggtaatcgctgccattttgataatggttggctttgttggttacaagaaccgcgatttggaaagttaaggaggactaatatggtgaaaagactgccacgtgatccgaaaaaagaacatgcaattttgaacgccgctgtggtccagtttggcaaggacggctttaatgccagtaccgataagattgccgaagcggccggtgtttccaaaggatcggtttttagatattttgataataaaaagaaactctatgtagctgccgttaagcaggccatggcaacactggttgagacggtcgatttgagtgtgtggaccgattcggacgatttggtgaccatgattattaatgcgaccaaatataaaacagagctctcccatcaatttccaaacgaatttgccttgttgacccgcgtgtatgcccaggataatttgattccccaaaaggtgcgtcaggaagtatttgcgattttcaccaaatggcaggcagaagtagaagataccgtcgtgacccgcgtagttgataagatgacaattcgcaaagatctggataaaggccaagtaaaaaaatatttgacgctggttctaggaacgatttcagcggaggtccaaaaagaacttgaggagcatcctgaaatgaaacggattgaggatatgggcgacctgattgccaccgtgaagaattatctggaaatggcggagtttggcgtcgttgaatctagacgggattaaatcggttagaggaatatttgaaacacgtcacacaccgtcttttccggcaaacaacgtgcgtgacgtgactagttactttggtgaatttaacgttgtctgccaaacacttaccaggacccagcaagcaaatggcatggcactaaggaataatccaataaagattaatccaggggcgtcgccggacttggcccagatgtaggcaaacgtcagactggtggtggcgatgattaccgtgataatgccaagcagccattgcaagcgatgaacagcaagcacgacttgttggggtcgttgaatgagccgccagagaatgacgatgccgaaaaccgtacagaaaagaaccacccagccgccacctaggaccaggattaacgccaagttgatcttggtggttaagaccaggaggactgttgcccagatgcccactgttaagagtgcgaggcacagcaatgccaggctggcgtgcagaagttgatggctttggttagggttagatttcattttgaagacctcctattattttgagtttagactattcttgttgggggaggttggttgttgggtgatctttggaaaaacgtaaataggtatgtggatgaaaaaataccagctgggccttctttttggaggctttgctggtattttttggttgttgtttgatgatgtttttctattatctagtggaaacgtgctccgagggcctgtccctaacttctaagtaagctttggtcaaaacccaagttcagggttttaaccaaagctcacttagaaaacgggtcacccagccctcgtcgcactctgattgaaatgtgctccgatgaccctgacccctaacatgtaaaacaaggattgtatcgatgaacaaaatgcgttcatcaatacaatccttgctttacataccggggtcaacccgggtctcgtcgcactctacggcattaccaaatcataatgatttcccacgatcgctgtcccacggtcatggaccacgccttcaccaagtggtgtttggacatgggtgccaaatgggacgtttgatggggctgccacgattaagtagccgtctgcatcgtagccgccatgattagtggtgccatccgcaaatgctgcgcccgtgtagtacgtccactttttaccatcttggtaaatcacaccttgtgattggaaggctgccggtgttgtggttgcactgctggttgcgtcattggtggagttgtccgaccctgattgggaagtgacgacagctgcatgggcggaaccctttttgattgaagttgatgtcttgaaatgttttttgttaactttcttagcggtcgttttcttagcagatttgccaatttcaagtttttgaccgaccatgatcaagttcttgtcagcaattttgttttgcttaacaagcgtgtcaacgctggagttgtgcttagcagcaatttcagccaaagtgtcgccggatttaacggtgtaagtacttgcgctggcagcgactccggtgaaacctaagaaacctgcaacgacggataatgttaatagactctttttgattgtaataaccaccttttagattactgtgtctagaattacgttcacgattgaaacgaaagcccgacttccaaaattgataaaatgattgcttgaatgttaatgtgtgtgttccggaacacaacttggaaatgttgagtgaattttggaagatgattgattagtaatgtgaacgtggaacaatcaatcacgcaagtataatatcagatctgaactaaccgtcaaccgccattacaaataagacaaaagtgtgacaatgaacgtccgtggtaattcagtaaatgaggcagcatgttacaaacacgttaaagttaaaagagactgtttcccattaaatgaatgtaatgattgtgtaaatggtgaataaatacctgtatatgccaattaacttgagtggagtggtgaatggcggaacttttatataatcattaggcgaatttgaggttcgccggtataatgaaattaacaagaaaagtgagtggtgaacaaaatggttaaacaaggcagatttgccagatccagtaaaatgaagcaaattaaagcgattcgcaaacgaatgcatcaaccggcgggacggacaattcacccggaccaatttcaagattttgttttggtccgttatgggctgacgctgaagaaacgattgacggggattgataaagaaacggttcaacgatttattcaggagttgttggtggtgacgccgattgatcagacatggcaattgaaccagattttgcgggacacgcttcgaagtattggcaacaaagtcccatatcaattttatcgaatcgtgaccaacaactggccggagattcagcacttcctccagcgagaaattccggcggttccattggctaatcggatcttggtgaccaatccggtttccgatagtcaactgcaggaaattgtctcagccgaactggcgggaaataccatgattgaaatggttcatgagaatccggcaatggagaaaatgattaccgacgagccgtatacgacactgcagacaaatttactgagtgatgggaaaattgattggcaaaaagttgccgctgttttcacgcctgttcattttaatcccaatattgctgaagacgcgggcacgaaacaatggctggaagccttaatcaaggaatagtgaggtcatgacgatggatttacagcaagcattagaatgcgttaatttagtaccgatgtttcagtcacttccggaagatcaaaagaccgaggttgccaaattggtggtccaacatcactatccaaagggaaccatcatctatctggctggcgacaaagtcgggcacttcatgatcctcgaagcaggccaggttaaaatttctcaagtggctgccaatggtaaggagcagctgttgaaagtccttcaaccgggtgattttgatggggaggccgctttgtttaacggcgatcagagaaacatggcggcgaccgccttggtggactccaacgtctgtcaaattgagcaggatgcctttcaaaaattactccagaagagtccccaactctcggtgagtctgctggcaaccatgagtcagcagattaatagcctccaggaagaaaagacgctttcgtctacggcggatatggccggcaaactggctaagtacctggttgaaaccggtgcggccctggatgaaaatccatttaaacttccattaaagaagaaagatattgcgacctatttagggacgaccccggaaacgatcagtcgaaccttcaagcagctcacgagcaaagggttgattgaagctaaaggatctcaggttaaaattatcgatgaagacggcttggacatgttagtctaagctttttctttttagtaaatatttattgcataaatttagaaaagaattgatttatacgtacgaatattttacaatgagagagtaaacgaaaactaaacgtagctacgttggaggaaaaaacgatggacgaaagtcgagtacgaaatgaaattgtaagcggaaacatttcgttgggaattgaactgggatcaactcgaatcaaagctgttctggtttctgacgatttccaaacaattgcttcaggcgattatctttgggagaacgaattagataacggcatctggacttacccacttgaaaaagtttgggatggcattcagaccagttatgcaaacctggcattagaagtgcatgacaaattcggggttgatatcaagaaaattggttcgattggtgtcagtgccatgatgcatggttacatggcatttgataagaatgatgaaatcctggtaccgtttagaacttggcggaacaacattaccggcgacgctgccgaagcattgaccaagctgttcaacttcaacattccagaacggtggagtatcgctcatttataccaagctattttaaatgacgaaaagcacgttaaagatgttgacttcatcaccactcttgcaggatacgttacctggaagttatctggcgaaaaggtcattggagttggggatgcttcagggatattcccaattgacgaatcaaccgtcaactacaataaggaaatggctgacaagtttagttcattacctgacgttaagaaatatccgtggaatctactcgacattttgccaactgttttacctgccggcaagaaagccggtgagctgactgatgaaggtgccaaattgcttgaccaaagcggcacccttcaaggcggttcactgattgcgccaccagaaggtgatgcgggtactggaatggttgctaccaacagtgtcaagaagcggactggtaacatttctgccggtacgtcagccttctcaatggttgtccttgattcaccaatgaaggccgttcatcgtgatatcgacatggtaacgacaccggatggtgcaccggttgccatggttcataccaacaacagctcttcagacatcaacgcctgggtcggcttgtttggtgaatttgccaaggcattgggtcttcaactaaagccggatgatctctatggcacattgtttgccgaatccgttaagggtgatcaagatgctggtggattggttaacttcgcctatctttcaggcgaaaacattaccagaatgcctgaaggccgaccattgtttgttcgcaagcctgacagcaagctcaacttggccaactttatcaaagagcagatttattcagcctttgccccacttaaaatcgggatggatattttgcttcgagaagaacacattaagaccaacgttttggttgcacaaggtgggatcttcaagaccccggttgttgcgcaacaagtcttggccgatgccctgaacaccccaattgccgttatggaaaatgccggtgagggtggcccttggggaatggctgttttggcactcttctgtgttaaccgtaagaatggcgaagctttggaagattaccttgccaaccgggtcttcaaagactcgacgacggcaacgttgtatcctgaagaagccagtgttcaaggttatgacaagtttatcgacaactacaaggcagctttgcctgtagaagccgaagctgttaaatcaatgaaaatgaaaaactagaggtgcgagagaatgttagaagatcttaaaaaagaagtttatgacgctaatatgcgtttaccccaacttggtttggtaacgttcacttggggaaatgtttccgcaatcgatcgtgacaagggcttattcgttatcaagccttccggtgttgaatacgacaaaatgaagccatccgacatggtggttgttgatttggacggtaaagtcgttgaaggggacatgaacccatcaagtgacacgccgacccatacttacctgtacaatcatttccccaatattggcggcattgtgcatacccattcaccttgggctgtgtcattcgctgcagctaaaatggatatcccagctgtcagcacgactcatgccgacactttctatggcgacatcccatgtgcccctgctttaactaagaagcagattgaagaagcttacgagttaaacactggtaaagtgatcgttgatgaattcgaacgtcgcggtgttgaccctgacgctgttccggctgttttggtcagccaacacggaccatttgcctggggcccaacagctgataaagctgtctataatgccaaggtattggaagtctcagctgaaatcagttatcacgctttacaattaacccgtgatgaaacccatgtcccacaatacttgttggacaagcattattaccgtaagcatggtaagaacgcttactatggtcaaaataatgctaaatcaaagtcacatgctgaacatgaataatctgctttaacgaatagggcagtttattaagaagagaaaagtcgagacaaaaccatccgttttgtctcgacttttttgtagtcttcatattacttggcggaaaagtgggaaaatcagtatgagcaaactatttgcgtcggcctaacttcagccttatactcaccaaaaagcaattttggaggcgattacattggctgagaatccattaattacgatttccattccggcgtacaacttgggatcatacttgtccaagactttggatagtattttgaaccaaacttatcaaaattttgaggtcattttggtagatgatgcttcaactgaccacaccccagacacaatggccaaatatgcagataaagaccaacgcatccacacccactattttcagtcccatgaaggggtctcaaaagcccgcaattacgcgattgataacgctaaaggcgacatcattgtctttgttgatggcgatgatttattggagccgcaatatctggaagtcatggcccgcgggttggctgatccgtcggttgatttagtggccgttggctacaactggggctggcgcggcggcagcggtaccggcaaccagttccgcgaagtttccaagaccaacgcatatgcctcaatcaatcgccgaggcggcgattttggcggctatacctggaataaaggattcaagatgtcaattattcgcgatcatcaaattcaatttgacgaatcgttggacttggcagaagatctgctgttcacggcagattatattttcgtgtcccatcgtttcctattctacccaggggcactctacacaaaagtcagtcgttccaatagcatcattcactctgcgacttgggagatgcgaagtaaagagcaggttgttcgcagacacatcgatgaaatggcaagaaagatgcagccgtaaaatttatgtaaagattgtggataagcttccatttagcagtcagtttgaggtaatatagcttcatctgaggaaatctatttttggaggttactctggtttgccaagttttaccaaatctcgccagcaaaaattaaataaactcattttgttcatgatgacgcttgtttcgatcctgacaatgagcgccattagtgtgtccgcaaagtcagccaatcaacaaaagtttcaggccaaagaggcctatgtgatggatgcagaaaccgggcaggttctctaccaaaagaatgggaacaccaaacggccaattgccagtctgtccaaactgatgaccctttatctgaccaaaaaagcaattgataatcaccaaatcacttggaaccaaaaagtgccggtggacgaccaacttcgtcgaatgagtaaaagttatgaagttggcggctttcggatcaagcgttccaaggaatataccgtccgcgatttgtacaaagccgcattaattgcgtcgtccaacccttcagcgatcgccttggggaaattagtcggtggcggcaataacactgaatttatcaaaatgatgaacgaacaggcgcacgcctggggcatagatgccacttttgtcagcagttccggcctggacaataccgatttgagcaagtatcattaccaggttccccacacgacatcaaaagctcagaacatggtgagcgccaaggccatttcgacggtggctgccaaggtgctggcgatttttcccaccattacccaatggagtaagcagccctcgatgaaggttggtacccaagtgttggttaattctaatcgcctgctgccaggctcggcattttatcacaagagtactcatgtcgatgggctcaagactggttttaccgtgaacgccggcctctgtattacggtgacgtactggcatgacggtcgccacttgattgcaacaattattgacagtaacacgctgtatacttcgatgaataagctgatctcgacggtcaaccagcaatatcagcccaccaaggtcgccttaaagtcgcatgctttctcaattgacggccatcagttgaccgccacacctaaagaccctgaagcagtcatttggcagcgcaaagggaccgatggctcgcatgtgaccaattattcagcaaccaaaacggcgttgccgattaccaaaggccaaccgattggcaacgcgatcgtcaaactggcagataactccagtacggctgtggtgccaatgctggcagcgactagcattaagcagccagctaaaaaagtgaaacatgcgactcacaaaccctcgttgctcaaacgcatttttggttttgtcggcagtatttttggcggcatttatcggctgtttgtggatttcgtgaagtttatgacgccataatcatttcgtacacgttccagctatataaaatgagacaagtaatggaggccggaacataaatcgtaaagatggctgtcattgcaactttgattaccacttgtatattgataaaacttgcgacaaacggctgatcccagaatttaacgcataaaaccagtcattccaaaatccggaatgactggttttatgcgttaaattctgggatcaaatcgcctttcgtcccaatctcctttgttttccatgccaaagttgacgtatgataggggcaaatccttggaggcaaccatcgtgaaaaattatcaaatcgttcaaatatcagacacccatttaacaccacagaatgcgcaacctgcgaacaaccaacaaattgatccgatgctcaagctgatgcaggtctttcatgacatcgaggcaactcaagttcaccctgacatgattgtaatcagcggtgacctgattcatgaaggaaaagccgtagattatcgccaattcaagacgctggtcgaccgagaacaagtccgatttggtgtgccgattcaagtcctactgggtaatcatgatcgcacgtccgccttttataccggctatctggataaaccagttcagccccgatattattacagtttgtcagataacggctgggatttttactttttggataccaaatgcggagacttggaacccggctaccttgacgagcagcagttgcgctggctgaaggagaagctgggtgaatccaatcgaccagccttgatctttatgcatcacccactcctgggagcacccttggaaaacatgaagtacagtattttgcaaaatggcgatcaattgcaatctatcctaaagggcagccaagtcaaagcgattttcaccggtcacgtgcattttgccaatatgttcatcaaaaatggcatcttaaatgtgtcagctgattccaccgcttatcatattaattgttccaatcctaaacgccatctaatttcagaaggcaccggctataacgtgatcactttgtctgaccaacaaacgagtgtcgaacaacgaccgttattgctgggaaatacgaccatcaaggcctttaacattccgtcaaccgacttcgttgacccccagattgttgcccaggaaatgaaacgggttttccggtaaactttcaagtgtttttaatagtctgatgggccatcctggcgtacactaatacagaatttaccttacaaaaaggggtgagctgtatggataagcaaccagttgaaccaattggcccatatgaaagactgctcagcgggtcactattggttatggccgcaggggtgctggactcgtacacctatctgcaggatggcggcgtcttcgccggcttgcagacgggaaacttaattttaacaggattgaggatcggccgcggcgattacgccagcatcggccaagccttggtgtcactggtaatgtttgcggttggcgttgccatcatccgggtgattcagtaccattatcccagtgagcgggcagtgacacgcaagcgggtgacgttagtgtttgaaattttaattttgatcgtcgtgagtttgattgccggccgtgtatccattttggtcacaactgggctgttggcgctggctgcagcctcccaactgcaagagttccgccggatgaagaacgccccgtttaccccactgatgatgaccggcaacgtccgcaccttatctgaaagtgtcttggactttgttgcccaaggggatatgaaggcactcaaaaaagccggtgacattgtgacaatcatcggctccttcttcattggtgcgctgttaaatggctatttaattcagtttttccatgggcagaccattttaatcgctgccgttattttgttggcaaccatcttgtttgccaagtaagctattctgatttgagttttgaatacatggccacgtcatggaattgaccattatataagagatattcctttaaaatgccatcttcatgaaagcctcgtcgtgttgccacggcgcggcttttgttgtttttaacatcggcgattaactccaggcgatttaacccgagttcagtgaaggcaatttgttccacatgggccaagcagagcgtcatcacgcccattccctggtattgatcagctagccagtaaccaatttgagcccgctgattttcatggctgaattcatggaggtcaatcatgccggccggttcattgtcgaccagaataatggtgaaccaaaaatcaccacgagccattttttcgattccgtattgcagaaatttttgctcgtcactgactgctaccatccctttggcccatggcagccactccgccagctgcatgcggttgctgttgatgagatccaaaatgccgttcgcatcggtcgctgccggtaattttaaggaaatatggtcgttcacttgatcaataaacatagagtccctcctcgtcaaactgttacaattaagtataacctttttgagggaggaagacttgttgaatgaaagacatacgttggaattgcccgacgcgctaaaagcacagttgggcgttaaatctggtgagcaagtggaggtccgaatcggtgctgatgaattgaaaatttccactcctagaccagtggaagtcaaaaagcggcgctgggggatgatcattttaaccttcgtaatgagctgcgtctttttgggatacttcatggtccgaaaaatctatcaggtttccttggtcggtagtgaatcagtggcgacaatggtgttactattgacgacactcagcggcctgatgagctttatggtcgtcttcgtccggttgaaacggcagtctggctcggcagtcgaagccgtttcgtggcgaaacctgccaacggtcgcgctggcatttgcgctgatcagcttcatgctgatggcgggattgttttggattgccggtcgactgtttaaaggtgccagttttgatttggtgacgtcaacggcattatttgccttgatgaccagtgttgaaattcaagctatcaatagtcttgttcctcagctatcttcacgccttttgaccaacatctttattgccgtgattgtcagcggagtcattttggcgatgatcagtaatcaaaacttgtattggtggaaacacaatctcagctttttgggtaccaacaaagcggttgattcttgggagtttaacctggcactatttttttcggggttaattttgttagctttggtggattatttatttgcttctttgaaacgaatcttccctaaaagccggcagttgctggtgttaagaatcttattgactttgctggcgattgatttggggatggttggagccttccccaacaacttggaaatccattcgttgcatactcggctggccggctatttgattttcctgatattaggactgatttttggtattcgctggctgctgcctgatatttccaccgattttcagcacatctcctggatgattgctgcagcattgctggctggcgagatattatttcaggtggttggctatttgtcgctgacagcgtttgaaatcatggcgtttttactggcctttagttggctggtgatgctgtttgaacgtttgaacgactatctggagccaattcagaatcaacggtatgtcattaaataattgtgaggttatttcgatgtttcaaatgaaagcaaacaaggcaaatcaggcacccatggcaagatatatgcggaatcagtttcattttcttggcctcaaaacaccacagcgaaaagcggcctcgaaagcctttatccaggcttccaaaaccgttcctgttgctaaaatgatggaagaaattgctgaactctatgaccgtgacgagcgtgagtaccagtacgtggcgattgatgttgctgatgccaatgtgaaacgattatcttttaaagacgtcaagacgttaactaagtatattcaggtgaaatcctggtgggatacagttgacacttggcgaaaagtgtttggggatttcgtggtattgcatccggacgaaaagcgggcggtctttgatttgttctatcagcacgacaacttttggatgcggcgagtcgccattcttttgcagttgctggagaaggacacgttggataccgagctgctggccaaagccatcgaatatgatattgacaccgatgagttttttattcaaaaggccattggttgggcattgaggaattatagtaaattcaatcctgcttgggtgcgtcgatttgtggctgagcatcatttgtcgaagttggcggttagggaagggacgaagtatttgtgaggggtgtgggtgtttttgagatcattcattatcgagcaccacttttacttggaataaacgtgctgcttacggctgatccctgctatttaaacaaattgggcaattattccaaaaaggaataactgcccaattcgcttaaattctgggatcaaaacgcctaaagcaccactctaatgctttgaagccaaatgatgatccgtgaatctgaaaccagtgacgacaataatagctgcgacaaggaatgaggacaagccgaggatcatgttagtaaagccgatgcttgccaagattgatgcaaaaattgtaccaaacactaaagttaacaaaccgatcaaagtgatttttaaattctcatccatgagatcgcgcccccatactattaattgttgtaaaaatcgcaagcaattctttgtcaaatcagtggttatatttagtagtcattagcaaattgtttgcgctttctttacaacttcattgtaacgtactcaggtttaaaatacagcttttttctcatatttaaatcgttttatttcgagggaataattaggggcatgaatgttcaaaatgaccggtgctggacaagttatgaattgtgtgtaaaaatattggtaacagaaattcgaaatgaaaaggaagtgaagcccattgaagattgcaaatcgttaagacagaatttgataatgaatcactgttcagaacaggggttcttctgtgcgattttgcaattttagtgggttttaagttcgatacttttagtgtctcagaacacccaattagtttatcaaaatcgcctgcgtgccgatgtgcacagcaggcttttatattgcgcaggaacccatctgaacctttaatgaggtgagattatgggaaccattcagattaaaaatttatcgtttagatatgacgggatgctgaccaatctttttgatcagttgaacttaaacattgatgaaagttggaagctgggattgattggccgcaacggccgggggaagactacttttctcaaactactgttgggaaagtatacctaccagggagaactaaacagcagcgttgactttaactattttccacaaagaatcccggatcctactcaactgacaaagcatgtcttattgaagattgccggacttgatgacagtgagttatggcgaattcaagttgaaatggataaactgcagttgactgacagcgtcttggggcggccatttgagaccctgagtcccggcgaacggaccaaggcactacttgcagtcatgtttaccgataatcagacttttcaactcattgatgaaccgaccaaccatctggatattgaaggtcgagaagtggtcgctgactatttaaagcacaaacgcggctttatcgtggtgagccacgaccggcactttatcgatcaggtcatcgatcatgtgctgtcgattgatcgcgcaaaaatccaattatttgctggtaattacgaaacttgggcggccgagtatcaaagggaaaatcagtcggaactcgctgaaaaacatcaccttcaaaaggaaattggccgactgaaggccaccgccaacacaatggaacgttgggcgggtcatgcagaaggcaagaaacagaaaagccgacaaagtgaccaacatgctaatatcgataagggattcgttagccataaagctgccaaggtcatgaaacgctccaaaaatacgctgcggcgcactgaaaaagatattgaggtcaaacagtctttgctgaaaaatgtcgatgaagtcgcgccactgaagttgaatagtattcaaccaccgcaaaaatatttgctgcaagtggaagatttgcaggtccaacgagccggcacaattttgaaccaacccctgagcttcgatttaaagcgcggccaacgcttgatcctgtttggccctaatggaatgggcaaaacgaccatcgttaaagtgattatgggcgacaaagagttgctcgctggcggaacagtcaataagcccgccagcctcagaatctcatacctgagtcaaaactttgaagatctcaatggatcgattcaaagctacgccgatcagtttggaattgaattaaacgacttactgaataccttgagaaaattgggctttgagcgagcggcatttgatgaagacttgaaggatttaagtatggggcaaaaacgtaaggtctcgttggcaaggtcgctgtgtgagccagccagtctttatatttgggatgaacctctgaactatctcgatgtgatcactcgaaagcaaatccaagacctgatcttgcgcaagcagccgtcaatgcttatcatagaccacgatgaggcctttattgaagcagttaaaacggcgcccttgttaaaaattacgccgattgattcacaataaggtgtacttattgatgactttgttataagatgtgctagatattgttgtgaatttttagaggggttaagatgccaaaacattcattgaagaaacattcggtcaatcgatcgttattattgagcctcggggcaattatcgttgtgggtttgctgatggttaccgtcggcaaagtgtcccagggcaacaacagccattcgacggctacccgcagcgccaagcagatcaaaaaagccaagattgccaagctgaatgctaagattcatttgacgaagcgcgagaagaagattgccagtcattacaagctgaccaagctggagacacgaacagcctccaagacctatatcaccgcgattggtgattcggtgatgattgacgttaaaccggatgtcaaacgagtctttcaccacagcgctgtgagtgggtctgtcggccgccagttttattcgctgccggggattgtccgccacttgaaggcgactggtcatttgtccaaatacatcgtcattaacttggggattaacggaccgccaacccagcacgatattaattcagtattgaagaccctgggtaagaaacgacaggttttctggattaataccagggtgccacgtcattggcagaacacgactaatcggatgatcgccaagacagccaagaagcattcaaacgtgcatttggtgaactggtatcaagccagccgtggtcataaaggttggtatgccagtgatcgggttcatttggatttgaccggtgaaaaatactatactcggacgctggccaaacgtgtttcggaaattttaaattagtcagaaaaaacactttgaatcaagttaatagctcaaaaaaatcagcagtcgcatttttgcgattgctgattttttagtatgctgtgtatttgcatgccaataagacacgtatttatttgatgagttgcttgagttcctcaaaaacgatcggcagctgcttgtccttaccggtatctgtgaaatggtgaccggatggcatcaaaacaaacttggcgtgtaggtgccgggctagcgttaatgtgtacgggtacggtacactatcgtcattaatagctgaaataaccgctaccttacggatctttggcagaattccagtataatccaccggatgttccgtgaaggaatcaagttccggcagtgtccaaatgggttcgtcaaagcctgatactaataagacattgacgttgtggatgtcgtgctggtcaaggtagtggaggacttgaatgcagccgaggctgtgaccaacaagggtcatgccgtcctctgggtcaatatttgcgtcacagtactggtcccaagcctgttccaccggatggtcggaatccggaaagttcagttttttaaatggtcggtggagttctgtttccactcgattttccaaccaaggaaaccaatgatcgttggcattggacgtatagccgtggaacatgtagatggtcatctatgctaccttctttcccagtattaaagcgcggttaccattgctcatgcttgtaagccatttcccaaaagtgcagttcgaaatagctgcttcgcaaaaacgccgtctgcatctgttcctgttcttcagcgtcggcagcctcaccaagttggtcgacaatggttttcattttgtcagttgcagtggtaaatgcggggctgtcataagtctcaataaattgctgataaattttaattggtgaacctgcttttatcaatcgctgaccgatctcattatataaccagtagcagggcagcaatgccgcggcggcgcgagaaggggtgccttcattgagttcatggtacatatgggtcacataactgtaggcattgggggcaatttcagtttgatcaatctctttttgggtgatgttcaactcttggaaaaattcagtccggacttctttttcgctgtcattgaagcctttggctccagcatagagaaattctttgatatccggatcgtccatttgatcggcaattttgccatggagggcggcaaaattctgcaaataataacggtcttgtttgaggtaataacgaaatgtttgttggggaagtgatccgcctgaaagctgcttgatgaagggatggttaaaactggcttcccaaagtggttctgattgttcacgcattgtgtcggtgatttttgccattacgcttaactccttaggttagttagggacatgtttgagataattttaccatgattattaagcgataacgacttgaattggcaacttctaaggttctggaactttcattgttcgatccactcgtgagcgaccagtggcataatcaaactggatgccgggctgaacattgaacaaatagacgttgaagttcagtgtccgatccgttgaaattgcttcaaggtgaatgccgcgggccattaattcatttccccgaaaaattggcttggcaaagaagatcactttgttcccacgtcgcagggattctctgattttactttcaaaaatcgtttgaacccgctgattggagaagctggtctgggtgaataggttcttgggattgttttggtcgcctgacgtgtcggttggattatactggccggatgaactgataccaccggagatcgaataggcaattaaatgaccgcgattgataatcggctggccatcgaggaatttttggtgccaagcggttggctccacatactgacggacccggttatcgtcagaaaccacatttctaggttccaagtaagccaaattgccggtgctggtccgattaaagttgtccagatcggaataaatcaccttattggttttccaagaatttggatccagctgtgctttattgtggttcacaaagatgcagctgggatctcctgaatgataatccagcttcgccagttgatctgattcgacacttttgttcgaatggaacaaagaactggtcagattgttgaccattgaagcgaggttactaggctgttggtcgacccccagccacatgccgacaaggatgattgccaaggcaaagattgtctttagaccggtgttgcgtctttttcctcgagattttctgggatattttttatgttgactcatgatcatgcctcaattctatatgtaagctctgccttcaaacataccagaagggaatggatgaaggcaagagtataaggagagtatgcacacctgtgtgcaatttgccggggaaagcaaagatggctttgcggccatcactttatatatacggtgaaatggttggagaatatttttattttttgaaattttttggaaaaggtttttattttacacttttatctaacgaaaacgtgctcaaagacccaggacccggccacacaagcaattaaagccaacgatgaacaaaaggcgttcatcattggctttaattgcttgtgctctgggtcctaaccaggtcttttcgcactctgattattaaataaatgctcaaaagctaaccggtttggtccgcactctgatctttatggcaaatcatttcccgccgcgaagaacaggtcgtaccactcctgctttgtgagttcgacatctgctccggctgcgctgtccttaatgtgttccgggttcattgttcccagcagtacttggacctttgccggatgtcttaagatccacgctgtggcaatcgcgttctttgaaacgccatactttttgcccagctcttccaatttatcatttaactttttgaactttggatcgttgatgtacatgccggcaaacaaaccataattgaatggtgaccaagcttggatcgtcatgttcttacgacgtgagtattccataatgccgccatctctcatgatgctggcatcgtcgatcatgttgacgtgcatgccttctttaaccattccggaatgaaccacgttgaattgtagttggttaatcaataagcgttggctgatccaggattggaccatttcaacttgttggggattaaaattcgatacaccgaagtggcgaacttttccttcccgctgcagggtgtcaaatgcatcggcgatgtcgtctgcttccattaacggatctggacggtgcagcaagaatgaatccaaataatcgatacccattcgttgtaaaatcccgtcaaccgagtcaatcaggtgttgtttggagaagtcgtaacgttggccgaatactaagccgtcatgacttctggccggatccaaaatgatgccgcctttagattgaataaataatttatcccgagaaattccagaagctttcaaggcttctttgaatttggtttccgattgtccgtcaccgtagatgtcagctgagtcaataaaattaatgccagcatcaacagcggcttccaatgtcttggcagcgtcagcggtttccataccagccatgcgcataattcccaaggcaactgcggaagcttcaaaatttgtattaccaatctttacagttttcatgatcgtcctccttcattgattaccttaattatacggcattctgagggcggttccaaaggtcttgtaaaaaagaatatgttataattcgaatacttacaaaacgaaatgaggaaccaatttgagcgaaaatacaattactgaattaattaatcagtatggctacctcggcattgcttttctaatcgcaatcgaaaatatttttccgccaattccttctgaactggtgctggtcttcaccggttatttaaccgttaccagcaagatgaccatttgggggtcgattctggctgccacggctggcgcactgatcggggcaatcgctttatatggcgttggccgtttgttgagcgtccaacaaattgaaaaattggtttctgggcgatttggcaaaatcatgcggttgaaaccggcagatattgaaaaagcggccaggtactttaacaaccatgggggtaaggcgatcctgcttggtcgctgcatcccggttgtccgcagtttgatttccattccggcggggatgaccggctatccgtttaatcgattttgtttactgacgactaccggaacgctgatttggaacacgattttgattctgatcggccattttgccggtcgggcttgggatcagattctggggatgatcgatcagtggctgatgatcattttggtagtgattgttgtgatcgtgggatgttatttgtattatcgattttctcggaaggcggattaagatcgggcagctgtttgttgagtattgatgtttttgcctaataggattactcttccttgggtgtcattttacctagcggaaacgtgcaaatgaaggctgatcccggccatacaaaggacttactcatttattccaagatcaggaataaatgagtaagtcctttatattctgggatcaaagcgccttcatttgcactctcttttacttttccttaaaattccccaaactttccaataaactcctaacaaacttcacaaattactcggcaaaatttgttatgatatttataagtaatgcaccacgacagctgaacccccacaaggaggcccactatgaaatggtacagtcatgaagcagaaacaatattacaagaacttgatacaagtcggatccacggtctgagtgaagcgcaagctcaacaacggcttgccgaatttggacccaacgagttggccaaagaagaacgcgaacccgcttggaaaatgttgctcaagagctttaaagaacccctgatcattatcctgcttatcgcgattggtctggcattagcaagtgccgcctatgacttttttgttagcggtgattctgggcatgcgatggcttctgtgtacgaagcgattgccattgtcttaattgtaattatcaacagcggtttgacctttcatcagacccggaccgcgcaaaaatcactggacgcgctttctgatatgcgtcagcactacatgaaaatccttcgggacaacaactggacgtcggtggctgccaatcatttggttcccggcgacatcgtcagcgttaagtctggtgattttatcgaaggcgatttgcgctggctaaagacgtcagaactgcagattaacgaatctcatttgaccggggagtctgatgccatccaaaaaaataccgtctctctccctgaggataccgagttggcagatcgtaccaacatgggatactccggttcgatggtggtcaatggaaatggaattggtgtggttgtggcaactgggatggcaaccgaactgggtaagatttctggactgatgcagcaggttgacgaccaaaagacaccgattgaaaaatcagtccacgggttgagtaagaaattgatgatcatcgctgcagttatcatcgccgtgacgattggctatgacttagtaaaacaattaattcaggtcggcagtatttcaatggacagctttggcgggatttcagccacggccatcgcgattgctgttgcctcaattcccgatgcaatgccggtggtgctgtcaactgtgttgacgatcggagccaagatgatggccagccaaaagggcttggttaagtcgttgagcagtgtcgaaacgctgggctcaaccacctatattgcctcggataagacgggaactttaactaaaaatgaaatggccgtgacccgctttttggcaaatggccaagtctacaatgttgaaggaaatggctacacaccaattggcgatttcatcagggatgatggcactccaagcgattctaaagattaccagcggttcttagaagtcgctgtcttaaataacgaagctgaaattaaaccggataccaagcaaaattggcggccgtttggtaatccaaccgatgtttccttagtcgtgctgggagctaaagataacgtcaaacgcgacgtgctgttggaagataagggtgatcgggacatcgatattgtccgaattctcccatttgacagtacccggaagatgatgaccgttgtgattaaagaaaatggccggtactacagtttgaccaagggcgcaccggatgtgatcaagccattgaccaaatcggcactgattgatgggcagccggttccaattgcttcggtggccgcaaatattgaaaaaacgatgctggcgtttgccaaggatgccttacggacgatctcaattactcaacgtgagatttgcaaagaagatgccttgaatgcatccagtgccgaattggaacgtgaactgacctttcttgggctggtggggatcattgatccgccgcgtgaggaagtcaaagcgtctgttcgcaaattaactcaagcatcggtcaacgttgtcatgatcacaggtgaccacgcgatgaccgccaaggcaattgccaaacagctgggaattatcgactccgatgatgcccgggtgattaccggccgtgacttggaggaaatggatgaccaacagctggcagacgtggtgttggacacgcgggtatacgccagggtaacgccagaacacaagcagcggattattaaacagctgcaggcccatgagcaagttgttgggatgaccggtgacggcattaacgacgctccggcactgaaagccgctgatattggtatcgcgatggggatcaatgggaccgaagtgaccaaagatgctgccgatttgatcttgctggacgataaatttaccaccattgagaagtcggttgagtcgggtagaacgatttttgccaacattttgaattttatgaggcatgagttgacgaccaacgtagctgaagtgctgtcattattgctgggagtcttcttgattacttcttccattggaaatatcaccgaagtgacaccaactctgacagcgttgatggttctgtgggtcaatatgatcagtgattcactgccatcgtttgcactgggctatgatgaagccgaatcagatgtgatgcagcagcgtccccgtgatactaaacaatccattttggcaaatgggatgctgcggcgggttctgttccgtggtggcgtgatgggcgcaatggtctttctggctttcatttgggcagcttcacaaggctatacggtggctcaaagtcagacgattgcctttctaacgttggtattcggacagttatggcacgtttatgatgccagaagtgtgaatacgttgtttgatcgaaatccgttttccaactccagattaacgttggcggttgggtttgcggcgacatcctcaatcctggtaacgttaatgccatttttcaataatgtgatgggaaccgcgccattgacgatgacgatgtacgtgttgattatcttgatttctgccgtaccaacttttgtgatttctggaattaagaaattcatgggtcgaaatcgtaccgaatcagtggctgttactcaagcaaattaatatagaacaaaaaacaatctaagattaagtctggtaagaaagctgacagccgtcagtttctcactggaactaatcttagattgtttagattgagatggaaatgattttaattttgtaagtgacttgcggcgcggagacagtgacaatgtcgccggaatggtggttcagtagtgccgaaccgatgggagaggcgatcgaaatcttaccgtggtcaatatcaacttccggagtgccgacaatttcatacgtttcagttgagtggtcatccagaaattcaaatttgacggtcttgccgacttccacggtatcgttgtttgagggggtgtaaacctgagcgtactggagttgttttcgtaagaatcgcaatcggctctccaggtggcgaaggtctcgcttggcggcactgtactcggcgttttcggaaagatcaccaagcgctcttgcatccgccaaacttttgatcttggcgggccgagaattttcgagctcacgaatttcagattcaatttgttcgtagccaaacttggtaattttgttgaaatgaggttccatgaatgtatccctcctgacatttttaagtatacaacatgtctaaattatagccaattaaactaattacttataaaaatcggcgaaatttccaacatttttattgaaaataacggcgatttagtcgcaaaattgccgaactgaaaccttgatctataagcgtttgttgatgatatgttatggaaatattaccaaatccctatttggtttaacaaggttgtaattttctggacacgtctctgtaaataggttggagtatatttttcactgttgattaaacacgaaaggaaaaatatatttcatgagacttaaaaagatcattatcgcattaatgactgcattaactttctacggcacaatgaacgttgccgcatccactgaaatcgctgaagctaagactactaaagtatacaaatcaaacttatcaaaggctaaccaaaaagccaagaactggatcgcctaccacgaatcacgcggttcataccatgccagaaatggtcgttacatcggccgttaccaattaagtgcttcatatcttcacggtaactactcaaagaacaaccaggaaaaagtggctgaccattatgtcagccaacgctacggcagctgggtcaatgctaagaagcattggaaggcttatggctggtactaagctataatacgaatatgttaagagatcaaacaatgaacaacacttgttcattgtttggtctttctttttgcttattgattgaatttgagctaccttcaaaattgtaaccgctgtaatgaaccattattcggaatctccgttgtgattcctcaaaattcatgttaatataaaattattgttttaaacacgaataaaaaggagaacataatggaaaatgtttctgttccaggcaagaaatcacctgttcgtaatgcaattttaggttttcaacacttactcgccatgtattctggcgatattttggttccgttattaattggtggggcactgggctttaatgccgctcagatgacctacttggtttccatggatattttcatgtgtggtgtggcgacattacttcagattcgcagaacacagattaccgggattgggttgccggttgttctagggtgtgcagtcgagtacgttgcaccgctgcagtcgattgggaagaattttggcttgggttatatgtacggcggaattattgtcgctgggttatttattatcctcattgccaagccatttgcgcacatgcgtaagtacttcccattggttgtgaccggttctttgatcacactgattggttttaccctgatgccggtggcttttcaaaacatcggtggtggggatgccactgccaaagcatttggtaatccgacgcacctattccttggcttcttcacagcgcttgtcattattgtcttaaacatttgggctaagggatttttgaagcaaatttcaattttaattggtatcttggtgggttcaattgttgccattttgatggggacggttgatttcgcagccgttggccaagctcactgggcacagttgccacagttcttctactttggtgtgccgaagtttgaatggtcgtcgattgccaccctgattttggccgccttcacctgtatgatcgaatcaaccggcgtttactttgctttaagtgacattaccggccggaagttggaagaccgcgatcttgaacacggttaccgttcagaaggaattgctgccattttgggtggggtcttcaataccttcccatactccaccttctctcagaacgtcggaattgttcaactttcaggaatcaaaaagttaacgccaatttattactcagcattcatgctgatgattttgggactgatccccaagtttggtgccattgccactctcatcccagcatctgtattgggcggcgcaatgctcgtcatgtttggaatggtgggtgctcaagggatcaagatgctctcacaagttaagctcaacaacaagaatctgctgatcattgccgtttcgattgggcttggcttgggagttaccacgcaacccaatttgttccagtacttacctgcaaccgtccaagtgatcatgagtaacggaatggtggtcggaagctttaccgctgtgattttaaacatcttattgaatcacacagctttgagcaaaaaagttgaagaataatttaatcaaatcaataataaaaggccagcgagttaatcgctggtcttttctgggttaacgactgtctcagaaattatcgttttggaacgtattcttcgacatattcagaaatgatattaagcaaatcagtcactggttctgacgtctgcttgttcttgatgaatgaaataccaaagttggctgtcaggacatccgttggaatctcgatgacgttgatgtgcttcttctgttcatcagtcaaacgacgtgggttggcaaatggttccggcgtgatgattgccccgacatgttccaatgcgagatcggaagccaagtgcagatcgggaacttcgacgctgatttcagctgaaacgccaatgtcgttcaggaagctggtgaccaatcgttggtagttatcttcctgcggtgtaccgataaattcttcacctgacagcttggtaaggtcaagatcctcataattcaagaagactttatcaggatcatacagcttggaagtttcaggaataattaaaaccaatggtaactgagcgattggtttgtattcgaccttgtggctttgaagtgcatggccaatgaaaaagtcgagggttcctgacaagagccgtttttcggcgtctcgactggtcattctggtgatttgcgcatgaatattagggtacttgttatagaaccggaccagaaccggtttgtataagtcgttggtcacaacttcattggaagcaatggttaagtggccgtatttgaactgtgacaggtgcgtcatttcgcgatccaagttggctcgcagtcggttttcttcctgtaaaaaagccagaagtcgttcgccggcgtacgtcagctggattggatgagatgatcgatcaatcaatttaacgccaaagttcacttcggcatttttgataacccgactgatataaggctgggtaacaaataatgcttgggcagctttggacatatttccttgtgccttgatttcttcaagaaacgaaagtaatttgctgttcataatgtaattctcctttgaagacctctcgcctttagtttatcttctaaccagattatatgatattctagtaatatatgcatgaatagtgacttctaatgttggtattccacaaaaaagctacaaccaagtatagcaattccccgtgcgccagtaaaggacatgaaccttttagcccgggtattatagtaatcttaagatttcatcatttatattaccattaggtactagtacccaatcgttatcagtgaagaaacaaatcatgcttttttctcgttgaatggtaaaatagtgtcataacttttatcccttaaatggatacatagcctactagaagggagttatcacattgagaattgaacaatcacctgaatttcaaattcatttacaaaccttaagaagcaaggaagaattatttctcgaaactatttataatgtcggcaacggtcactttggcgtccgcgactccaatccgctccagggaaacaaccatgattatattggctccccgggcttatttattaatggcttctttgattacgaagaagtcgcctatggtgagaagtatcgtgggtacccggacaataaccaggtaattaaccggttatttgatccacgctttattcgtatcaaggtcggtaacgaagattcgttgaccgatcatttcaaagttgaaaatattgataagaacctggacatgcagactggactgctgcacgagcttttcagcgtcacgactcctggcaaccggaattttaatctggtggttgaaagctttgccagtctgagcaagctgaatgtatacggagtccgatattctgtgattccaaccaacttttccgatgaaatcgaagtgatcaaagttcatgattacgtcaaccaaactgttcaccagcaggatgaagatgtccgggtcagcactgatctggggcaaatgcagctggactttattccagataatggccaacccagttacttggtaaccacttttcgaagccaacagggggcgattatcacctatcaagccagtgagaattttgccccgaatccgccgattgaatacttcagagacgacaatcaccactatggctaccggagtaaatattacgccaaaccaggcagtgccaaggactttgaatttttatttgcgatcggcgatatccatccactcgtcaatgccaatatgtattccgatcagtacctgtcatcgctgaataattacattaatgacaccacgtttaaatcagaattgatggcttcggcacaagtttggcagactttttggctccacagcgatgttgaaatcgatggcgatcctgctttgcagctgtgcgtgcgcttcaatttgtttgagcttaaccagtcagctgggcgagatgctttaaccagtattccagccaaagggttgactggtaatggctatggcggtcatttcttctgggacaccgagatctttatgctgccgtttttcacctacacccaacccgaagttgccaaggatctattgatgtttcgctatcacacgcttcaaattgccaaggagcaggccagtgactttggccttggcaaaggcgccatgtatccctggcggacaatcaacggttatgaatccagtgcatactggctggcaggccaggcgcagttccacattaacgctgatatcgcctttgccgtcgaacaatattatgagattaccagtgacgatgactttatccgtgattatggatttgaaattattttggaaactgcccgattctggatggagtacggcaactatgccgaacttgacggcaagcgccaattcgtccttaaccgggtaaccggtccggatgaatatagcgccctagttgacaataactactacaccaacgtattggcccagagtaacctccgtttggcagtcaaatatgttcgcaagttcaagggcgacgacggcattttgagtcgacttcacgttactgacgacgagatcgacgctatggaaaaggccgccaatgccatgtatctgccttatgacaaggagaagaacgttaagctgcagttccaaaactttgaacagctgccgaaaatggatatttctgccattgatcaaagcatgttcccattgctcttacactatcacccattaatgttgtaccgtcaccaagttaataagcaggctgatacgatcatggttgattttatgttccctgaaggcaacaccttggatcagctaaaagccgactatgaattctatgaaccaatcactacccacgattccagcctctctaaggcgatctacgcgattatcgcggctcggatcggtaaggatcagcaagcctacaacttcttctctcaggccgttcagacggatctgatggatgttcatcataatactaaaaatggcattcacgctgggagtttgggcgctgcatgggaagggatcatgtacggcttcgcaggaatcgtcaataatgcgacgagttttagcctcgagccccatttaccatccacttggaactgcctgaagttcaaggttcatctctatgggaatgaatttaaatttacgatttatcaagactcggttgaagtcgagctgctgagcggtgaggggacggacatcaccgtttatagccatcgcaaacacctcaccccggacaataaccgggaaacttggcaatactaaatttttttgaagaaagtctgaaatattaacgtcttttttggaaaacaggcgaactttggtttatgatttgttatgatagtgttatgcaaattcatcgttgattgctgaatatttaaacaagcccttgatcgttttgggcgagtcaatttatctgatgtgaaagggatgcactttataatgaagaaggaagctcgtcaatccaaaattgagcagattattaatcaatataccattacaacacaggacgaactgatggagaaactgaaggtggctggtattagcgtcactcaggccactttgtccagggatatccgcgagatgcagattgttaaacagccggatagttcaggcaactcacgctacatgatttttaagtcgggtaaccaaaatgaaatcgagcggatgtatcggatgattaacggcacggtaaccgacattcgccagattcagtttgtgaacgtgattcacactcaacccagttatgccaatccattggctgcggtgatcgatgatctccacatggaaaatgtttccggaacgttggccggctacgataccattgtgactttcagcccgtctgtagactctgcccgtgagattaatgatttgtttactaagcacgccaatccagacttgctggtttcttccattcaggatggggaataggcattcataatataaaaaataaggctttctcagctttgaggaagtcttattttttgtgctggtaattattttgcgaattgtcgataaatgcgtcgaccaatcgccccaatcagaaatgctagccaccaaatgatgccgactgcggtgaccagtttgccaagcgcgagtcccggcgtttgatatttcagtgaaacaaagtggcggccaactgggattctggcacccacaaagccgtgattgaccttgaagatgtctccggcctggccatcgatctttagatgccaaccggtggagtagggaattgaggtggtcaacacgcgggtgcgctccgttgcatccgtatagccactcaccgaattattggtgactttttggctggtcaaaccagctttttgaagttgttggatgcgggtgttgtactgccggttaaatggtacggccatcaacttgacactcttgaacttcagttgcttaacgccattaaagtgaatcgtcattgatttttgcagcttgttggcgtaacccagattcaaaacaatgtgctgtctgtcctcgtaatcggagaggttgttctccggtaattgacggacgtaagtgaaattgttgggggcttgaaccgacaatgtgtaagcaccgagatcgggatgctgcagagcagttctaatgcgatcaattttttgcagtttggaaaccggggtgccatcaataatcgaatcggcagtcaggctgttcagtctgtctgcagtggaatgagtggtgtgggagataccgtcgatcaccagatacaactctgaatgacgatatttttctggctgattaatgtttaattgataggaaagatggcgtccctgcgcatcgttatccatcaaatgaaggccgttggcatttgcggcctgattttcggcaacgatccggtgattcttagccagcacactttgaagcggcttggcattgggattaatgccagtggccttttcccagatcctgactttgttagccggtaaagtggtcttatatttcttcgcggtatcccggtagcgggcgtttggtgaaatccgcagccgatccaagacagccttgacggggttattggcgatatgttcgtcaaataatcgagtcgtgtacggcacgttttgaatgttgttctgcggttcggtcatcgaaacgccatcaaccggcttttcaaccacagcccctgataacatagcctgttcacgttgaagcggtgacatgttgcggtagttggcagctgaaatgacatatttttgtgtatagactaacggcaaagccaaattggattttaacaaaatcgtcccggaatggttgcttaacccgctcaccggttgttccgggaagtcgacaattttgccgtttttcccgcgaacataatggaaaccatatggaatggcttggggctttttgacaatatccgttttggcaaacatgtatttaacacccagtaggttcagcagggtggttctaccatctgcttcaccaagcacggagttgaccaccgcctgtgaattatccagtgatctgctgaattgaaacaggctgccgttttggatggagtaataagcccctaagtcatgggttcccagcaccatcgggatgttgttgccggcggttcggtgaggatagtagttgtggatggtggttgttcgatagaagccgccgttttttgccaacccattttgagcaccgtcataatacttgtggagccactgttcggctgacccggatgccaggttggaattgatattcttactattattgggactgaaccagccttgtccggcactaatgacgttaatgaagacgagtccgaccaaaatggtgccaacgtgcttgggagatattttaagcgacgtttgacaggcaaacaatagtagaaaactcagcaataatccgtaagataccaaatcgttttgcggtagtttgagggtaaagcctttggtgatccacacgagcacaatcaagccggcactggcaccaatcaaccagcgcaaatcgttttgagtcaggttcttgagttgatcaaccagaatcatcgttgccaagctcattggcaacacgatcaggaacaaccagcgattggacggtgttgacattgcgttggccaccgcactaaactgcggcagcatcaacgcaatgatcgtcaacgtgataatggttgccagtgatcggtagcgtttgaaatgtctgaggacatacactgctccgagaaatgtcaatccgcagaaattcagtaccagccaataatccttggtggtggtactggtaatcagttgattgggcatcgccagatagtatttgagtggataaagaatcagcccgttggcaaacttggcatggtaggcaattcgagttgattggaaaacggccaataaagttggaatcaagatgacgccggctgtcaacaggccagtcacgacaccttgcaccaaaccatagataattctgccgtttttcaactgttcggggtggttgtgacggatgttgaagtatctggttaataggtagacaaacgtcccgattgccagcatataagcgaagtaaaagttactgatgagggccaaggcaacggcaaccgccaacggcagccagttctgcttgtggagaaccttttcaatccccattgccaacagtggaaacagaatcattggaattaagaaaaatgggtgatgcatcgagacatagaagttgtagccggaaaatgtataaatcaacgtcccaatcaatttactgtgagtgctgaaatcccgctcattggcccaagccagaaatgacagcccgacacagtaaagacgaagcaagattaagacttgaaagccgagctccagcttggcagccggaaaaagagcaatcaggtagctgaatggatcaccaattatgtaaaaggcaaaggtggtgagttgatcggcaccagccccaaggttccacgaccagccactcattgcctgatgggcggttccttgaagcattcgctgaaattgcgccataattggaaaatgttgggcaatgccatcgacgttccagatcaaagttttgccggccagccagggaatcgtgtaggtggcgaggcagacaagtagaaaagcgatggaatagatcaaataagttcgaaactgaaaagactttctgcgagtatcaattctcggttccatgaaattacctccaatacatatcccattttgcctgcattgaggccgatagacaaggctattgacagatttttaatgtttgtaacattgatgccctcaagttgaaacaatgtgcatgaacattcatcgatgaattttagtaagctgagtaaaacgcttacataatcaatggtttgtctaaatccagtctcagcaaaagtgaattttcttttaccaaactgtgaatattttatgaagtcgaaacatatttataccaaacagatgagaacaaagtatgaatgttgtgaagaaagtgttatagttagagcattcttaaatctaatcaaattcttatgttctaatttaaacattttattttgcataattaaccgctaaaagccttttgtgaaaggaataattagcaggataatttataaaatgaaaccgcaatcattttcgaccttaattgtgtgagttttttcacgttcacaatgtccaaaaatgtacggtaacctttttcaaaggggttatgatgtacttgtattaatggaagaggaggtaacaaaatgacaagtccaattcatgtaacatcggaaatcggtaagttgaaaacagttttactgaaacgtccgggtagagaaattgaaaactttacacctgacatgatgccccggttattattcgatgacattccatatttaccaattgcccaaaaggaacatgactactttgccgatactttacgcgacaacggtgtcgaagtattgtacctcgaaaaattagctgctgaagctttagacgcagctggtgacaaagttcgtaatgacttcttagagcaaatgctgactgaatccggatatgcaacaggtaccattcatgatgcattgaaagaatatctcggcagcatgaacaaccaagacatggtcaacaagatcatggaaggtatccgtaagaatgaagtagatttcgtgccaacagacttagtaagtgctgctgaaaccgagaactacgaattctacatggatccaatgcctaacttatacttcacccgtgacccttcggcatgtatcggtgaaggtttgagtatcaaccacatgacattccctgcaagacaacgtgagtcactctttaacgagattgtcatcaagtatcatccacgttttgctgacaaaggggttcatgtatggcgtgaccgtaaccacgatacccgtatcgaaggtggagacgaattagtcttgaacgatcacgtaatggcaatcggtgtttctcaacgaacttccgctgacgccattcaagatattgctaagagcttatttaaagaaggtcactttgacacagttattgcgattaagattccgcataaccatgcaatgatgcatttggatactgtgtttacaatgattaactacgatcaatttacggttcatccaggaatccttggtgagggcggccatatcgacacttggacaattactccaggtaagaacggcgacttgaacttggaccacagaactgacctcaagcaagtcttgaaggatgcgcttaagctggatgatttggacttgatcccaaccggtaatggcgacccaattatcgccggccgtgaacaatggaacgatggttcaaacactttggcaattgctccaggcgttgtggtaacttataaccggaactacgtttcaaatgacttactcagaaagcacggcttaaaagtgctggaggttatctcaagtgagttgtcaagaggacgtgggggtccacgttgcatgagctgcccaattgttagagaggatatctgaatcagagcgtgacgagggctgggtgacgcggtttctaagggtactttgactaaaatccccggttttgggattttagtcaaagtgcacttagaagttagcgtcaggcccgtcggagcgtgtttacgaagctgcctcgttcagaaggctgccaaaaaatatccaaccaactctacaatccagtgtaccgtacccaaaaacaatcatcatcaaggagaattcgattatgacaaaagatttcaagcaaaacgtatttcaaggacgcagcgtattagccgaaaaagacttcacagcagccgaactcgaatatttgatcgactttggtctccatttgaaggcacttaaaaaggctggcgttccacaccactatttggaaggtaaaaacattgccttactcttcgaaaagtcatcaactcgtactcgttcagcatttaccactgctgcgattgaccttggtgcccacccggaatacttgggttcaggcgacattcaattaggtaagaaggaatcaacttcagacactgccaaagttcttggcagcatgttcgatggaattgaattccgtggcttcaaacaaagtgatgctgaaattcttgccagagacagtggcgttccagtatggaatggtttgaccgatgaatggcacccaactcaaatgttggctgacttcatgactgttaaggaaaactttggcaaacttcaaggtttaactttgacatttatgggtgacggccgtaacaacgttgccaactcattactggtaaccggtgccatcttgggggttaacatccacatcgtttcacctaaagaattgttcccaactgacgaaattcaaagcatcgctaagggctttgctgaaaaatctggtgccaaactgttgattaccgacgaccttgatgaaggtatgaagggctcaaacattgtttataccgacgtttgggtatcaatgggcgaaagcaactgggaagaacgcgttaagttgttaacaccatatcaagttaacatggaagccttgaagaagaccggcacacctgacgatcaattaatcttcatgcactgcctgccagcattccacaatactgaaaccgaatacggcaaggatattgaaaagaaatatggcattactgaaatggaagttactgatgaagtgttcaccagcaagtatgctcgtcaatttgaagaagcagaaaacagaatgcactcaatcaaggctatgatggccgcaacacttgggaatttgtttattccacgtgtataggacaaagtaaaatttcagcctagtacccaccttgaaaaatagctcaacaatacaagggactggcaacaaaacatttgttttgtcccagtcccttattattttctaagacggaggagaattattatgggacgtaaaattgtggttgccctcggaggtaacgccatcctatcaaaagatgcttcagctgccgcgcaacaacaagcgttgcgcgataccgccgagcacctggttaaattcattgaaaatggtgaccaactgatcatttctcacggaaatggtcctcaagttggtaacctgttattacaacaagctggtggcagcaccagtgataacccggaaatgccgctcgattcctgtgttgctatgacccaaggcagcattggctattggatgcaaaacgccatggaccaagtgattaaagaaaaaggcttggacaagactgttgcgacagttgttacccaagttgaggtcagtgctgacgatccggcatttgccaacccaaccaagccaattgggccattcatgagcgaagaagatgccgatctcgctaagaaacagaatccggacttcagcttcgtggaagacgccggccgtggctatcggcgggtcgttccttcaccaaagccgattggggtcgttgagacaaaagcggtcaacgccttggttgacgccggcatcgtgccgatttcagttggtggcggcggtgttccagtagtcagtgatggtagtcgactggctggtaaggaagcagttatcgataaggatttcgccagtgaaaaacttgctgagttggttggtgctgacgcattgattatcttgaccgcggttccaaatatctttgtcaacttcaacaagcctgatcaaaagaaattggagcatgtgtcagttgctgatttgcatcaatacatcggtgaaaagcaatttgctccgggaagtatgctgcctaaggtgcaagcagcaattgactttgttgaagcaaccggcaacgaggccgttgttaccgctctggataacatcgaaggatttattaatgatgggtcggggacaattatttcggcaaaataacacataatcccgattttgtccttaaaatcatcttagactttgtttaatgtacaatctggttatttgaggtacacttctaatgagaacacaattatgtaaccgtttttgggagtgtatttatgattttaaagaataagagtgattatgagtattatgctaaaaaactgcgccgccatcctgaatttagtccgctgagtgataagtatatcaatcagctgattgatgagatgactgttaaaacctatcatcgcggtcaaatcttgtttgaccagggagacacccgcgatcggttctattatttgatcgatggtgtttgtaaatcctttcactgggacaaagacggcggcgaacagctgtatctgtatattcgacccgaaaaggcattcccatatattggtttgtttgaagacgatcgctatgcatacacggtccagacaatgtccgaggtcaaattagccgagttcccgatgccgatttatgaggaaattttgcgtgagaaccctgagttgatggtcaatgctgtcaaagaaatgagtcaaattatcaacacctctgagactcagcttcaacgcatggtgaccaccagtgcaaaatgccgggtttggaacgcaattctcttcattggtcaacaaattggtgattatcaagaagatgagacaatccttgttccgtatccaattacattggttgaactgtccaaggtgagtgggacaacgagggaaacgaccagccagatggttcagcagttggttgccgagaacaaggttcaatataatcgcaaatatttcaaaattttagagattgacgatgattcatattaattgaatattattcaagggagtgagctaaatgaaagagcatgatggtaaattagggctgctcgaactgatcggattggttgttggatcaatcatcggtggtggtgtgttcaacctgatgcacgacatggccgtaggagccggtgccggtgcgatcatcattggttgggttattaccgccattggaatggtgatgttagccttgacgttccagaatttgaccatgaagcgtccagatctggatgccggcgtctatagctacgccgaagccggttttgggaagtacatgggatttaattctgcatggggctactggttgtccgcctggcttggaaacgttggttatgcgacactgttaatgagtgccgtggcctactttctgccggtatttggggatggccaaaacatctggtcaatcattgcagcatcatttattttatgggcctgccattttatgattttacgcggggtcgaatctgcatcgtttgttaacacaattattaccattgccaaattgattccaatcttcctattcatcattatcgtattgtttgcgtttaagatgaatatgtttaccagtgatttctggtttacaccaagtgggaaatttgaatttggcagtgttatggcacaagccaagagtacgatgttagtaactgtttgggtcttcatcggaatcgaaggggcggtcgtcttctctggccgtgcccggaaacgttctgacgttggtaaggcaacagttcttggaattatcaccgttattttgatttatatgttaatcacattgctatcatttggtgttatgagccgcgccgggttggcacacttaactcaacctgcgatggccgaattgcttcaaagcctggttggcaaatggggcgcgatggttgttaacggcgggttaatcatttccgttgtgggtgcctggctgtcatggaccatgttcgccggtcaattgccatacgaagctgccaaagaaggatcgttcccgaagatgtttgccaaggaaaataagaatggggcaccaattacctcattgaccgttaccaacatctgtgtggaaatcttcatgttctcgtacctgattacggcttctgcttataacttcttctattcaattgccagtgctgcaattttaattccttacgcattttcagcattctatcaattgaaatattcattcctggaagatcatggcaaaggacgaaccggcaacatcattgttggaattatttccagtctgtatgcctgctggctgttgtttgctgccggagccaacttccttctcttgatgtcgctgctctttgctgccggaattccagtgttctggatcttgcagaagaaggacaaccacgccgagaaggtctttggaccgattgaaatgttgctggcaatcttcattgtgctggctgcaatttatgcgatttatggattgattgttggacaaattactttctaattgtaattcgtgacggagaatgaatttgaacagccgtatatttgtaactaagggagcagctcaaatgagccgctcccttagttattgattcttttaaaaataagcagtcacaaacaaatacccagccaaaccaaatgcagctaatgaaatcaaaatccgcagcaaatggatgtttgaatgacggacgatgatcggtccggtgtagccgccaattagtaggccaaatccaagcgggatcaccaatagccaatcaatccgggacttgaaaataaaaatgaccgtcgcaatcaagttaccgccaaaggcaatgacgttcttcatggcgttgaccacggtaaaacgatcatcagtgatgattgataaaattgcgaggaagataacaccaccggcagcaccaaagtaccccgtgtaagctccgactaggacaattccggtcaggctgatcagtgatacccagaagtgcttggttggcgtttggtgtgcctgcttcaatttggcagtggaaacgtccttttttcgaccggacatgaataacagaatgcccgcgaagaggatgaagaaggggaccactttttcaaacgacgaagccggtgcaatcagcaacagcacactaccaccgatgcttccgattagcgaaaggatgacgtagagagtcaattttttccaatgccctctgagttcctttagcgaagaagccgttgcaccgattcctgagaagatcagggcagtggtattggtaacattggcaataactggcggaagccccaccgccaacaaggctggataggagacaagtgaagccagcccggcaactgaggcgagcaatcccgccgcaaagccggcaatgattaggaaaataaatgtaagcaccatgagttgggctgacctcttttcaattttttgatacttctaatatactacattttacaaagtagtcgaattcatcttgtgaggggcttgatttctgatgcccaacccttgataatatttaactatcaactcaagatgaaagcaggttacccatgacacaattattttttgactttgacgggacgatcgccgactcggaagccggcattctcaaatcgctgaagtacgcagtcgacaaaatgaaattgccggaactaacacatgatcaatacttgaaatttattggcccggcactcaagaccagcctccaaaaattttatcctgaactgtctgaagctgatcagatgcagactttaaaatactacgccgattattatcgcagtgaggggatgttccaactcgatctctaccccggtattgtccaagagttgcaggtcttgaacgaacagggctacggcgtcaatatcgcctctgccaagccggaagatttgattcatgaattgacggatcaactagatttgacgcaatactttaccggtcgatttggtgcggggactgacgagaaaacccggatgaccaagacagcggttctcaaatatgctttggaacaaactcatgccaacgccaacgacagcatcatgatcggcgaccgtgacaccgatatgcttggcgggtatcacaatcaggtcaagacactgggagttacttatggatttggcgacgttgccgaactgttgggcgcccatgcgaatacgttggtggataagcccgagcagattcaaggtggagtagagaaattaatcagctaaatatactaaaacggatcgaggaaatcttcctcgatccgctttttgttagttactggatgttcaattggaaaagcgtgctcccagataacgacgatgatcgttgggttcactttaaggcttgatataggcaaaaccctgttcctgcagtgaaaccaaatcagcgacaccggcagcgacaatttcaacgtttgccggtaactggttttccttaatcgaatggctattcatcgaattattgcaggcgtggaatctaaccccttctcggctgaattgctcgacggcatttcgcagatgttcgtccaaatagcccttgatggcatcgccgttgactaagacgacaatatggtattcttccttattcacgcgtccataatccagcaggttactaatattgctcagtgtgtgatcccacttatccaattcatcaatgtgaaagacaactttatgcatcattattccctcgtttcatccgcgtccaacgaatccaaaaattcctggtaatcctcgtggacctgttttgaatattcgtttgcccaattaattaaagcggagactaatttcttcttggtgccgacatacccgtgaacgattgcggcggtcgggctttgggcgtggccccgtgccagcaggagcccacagattttagcgtaggtagcaaaatcatcggcatctaatttgtccaagttaatcgattctttcatatcccagaactgacggacatagaagctgcggccggtatcatcgttgtgatagaagcctagcagtggatcggatgcccgctgcaaaatctgctggcaggtgacgattcgctcaccattatccggcttgctctggctaaatggggtcgtcacatcaaagcctctaaaacgccgagtctgcaaggcctccttgatttggagaaccaggtggctgccgtcaatcgcggttaacaagaccaggtagcaccgggtgccaaaactaccaacgccgacgctatggcggacaatatcactgatatgaaattgtgagaggaggacagtgacgtccgggctgaccgagcgggtgtaactccgcaagtgctcgcgaatttcgttgaagcggcgatcactgacatggacggtccgtggagcgttttctttaaagacaagatgtccccgggaatccaatgtcgtgaattttttgaccactttacccgagttccgttgttcggcactatcccgaattttgcgccaaacctttggtagtttgtgatcggaatcctccgactgcaggaaggattcaacttctgtggagaagtagtagcgttccattgctgagtgatcatcaaaacattggctgagaatctgctggtaggtttcaactgctccctgcataatctcgttaatttggtcgctgtctagtcccagctgctctccttggaggacaatgctgacaagcaggcgccggaggtcccagtcccatgagccgatggtggattcgtcgaagtcgttgaggtcgaacagaagttttcgctcaggagacgcataaaaaccaaagttccccaaatgagcgtcaccggaaatgaccaccggaatattggtggaagtttgtttcgacaggtcgaaagccatcaattcgtccgtgccgcggaaaaatgcgaaggccgaggcagccagacgcttgtggcgcagcggcattaaatctccgatcatcttttcttcaacgtgagaaattccttcaaccacgttacgcttaaccgggacaaattttcccagctggtcaaatgagatccggtcacgaatcttttttccgtcatcaatcagttcgtgaatcgatttattaatattaattttacttaagtcgtagtgcaagcccgtggtcgttcgggtaaaagtcttgctggtgtctgccatttaagtcggctcctttattttgacaatctataatatcattgtggcaattcccggtccgtgagtcaagcgaagccaactcatccgccggcttgatatgttacaataatggaaatagacgatttgtaggtaatggagaattagatttatgaaaaaattgtattgggaaagcatcgaagtgaataatcaaaaattcttcttcacagtcactgaaaaagggttgaactttgtctccagccccgggaagtacttgtctgagctttttgatttttaccctgatcgttatgatgaccaatttatgtacgacgactcggtgaccgccgattatttaactgaattcaccgattactttgatcaaaaacgtcaagactttgatttgccactggatttagagaatatcggcaccgacttgcagcatcaggtctgggcagaaattcaaaagattccatatgggcagacagtcacatataagcagttggccgaaaatatcggtaaacccaaggcaattcgcccagtggcccatgccgtggccatgaatccggacctaatcgtgattccgtgtcatcgggtggtccgcagcagcggcgacatcggcgagtaccgtggcggtaaagaaactaaaaaagcccttctcgagttggagaagaagccgattgaaaagcatgctttgattagcaagttaccgttgcctaagcttagtcaactaggtaaatctgatctttaattaaatcaaatggttggtgatgtcggttcagctgtttggcagtctcgggcttgataaaatgggcttgttgccagaaagctttggagtcggtagcgccatttttttcgccgataacgattaattccaaatcgttgtcggcttttctaatggcattgaggacgtcgacatcaatcgtttgtttgtccggtgaccagctcatgataacgtatttcacctggctctgatatttggcgattgcagccagcgcatccagcttttcgacgcgaatcagctgatgcttgccggtttgattttcgtcaacccactcaagactgtcggttgggaagacttttacgccaagatcattcagtcctttggaaatatatccgttgccggccatcacttccaacaccggtgagtcaccgatgtagtcggcgagatccttgataaacggggcagagatataggcccacatcccgtattgactctctaagtaatcccggaatgagcgcaattgtttatcaagtttgggcagcgcatccgacagttcgttccaaagctggtcgccttttggatcaccgggcttgaatcgaccgttgatatctttgaaaatttgatcttggatatcatcggggagcattaattccggcaagtcctgcggtaggagtccttgtttgattaaatggtcactttcaatgacattattgatgagaaatttaacctgtggataggcagcaaattgatcacggaattttagcatctgggcgatatagttagattcagccggttgggtagtggggtgctttttcttgagcaactttttcttttgtttattggttagcatactggactccttttgagtttcttttttggttagcactaaatgtgacggtacgtaaatacgctcaccaagccaacttcgaccgcattatccaataacaaggctcgatgctcgaaaacacatcaaacctcgttattgaataaatcctcagaagttaaaccgcttgcttgatacattaaagatctaattctccttgttccgtccgtggcccttgatcatgcggggcattgcttcttccgtggacgtaacctgagattaactgatagatttcatatcggtccttggaactcaaatcttgaccattaaattgcaaggttttatctgaaataaatagtcgcgccaagtcataggtattattttcagataaccccgtcaaataatccatggtcgcgtcgaagaacttggcaaggcgctggatttcgatgtagttgggcgttctgatgccacgttcccagttaccgatttgagatccggtactttcatgctccttatcagtcggggaatctttgttgatcgcgcgggctagttcttccaaagttaattgttgaccttttcttaatgctcgtaatctttctggaaacatgtgatcaccgtcctgttcgttacttatattatacgacttttttgctaatcaccaaatttcggcgttaaaattcagaatgtggtatatttatcacgagaaaaattgaattggtgggatggatgaatgaaacgaaaaacaaaagtctttattgggttggcttctgcagtggtgattatctgcggcggtctatttggtgccgggatgtatttttacaatgttgccgtggtaccggctcccaaatcatttttaagcaagactgagccaatcaagcccggcaactcgcgctatccggcctacaaatggtatcagggggctgacaagcagcattggtttgaaatgtctgctactcggcaccttaaattagatgccaattacatatcagctgacaagaccaccaagaagaccatcattattgctcatggcttcatgtccaacaagaaccgcatgttcgactatgcctacctgttccacaacctgggctacaacgtcttattgccggatgcccgcggccacggcgacagtcagggaaactatatcggctatggctggccggatcgcttggactacgttaaatgggtcaaaaaggtcatccaccacaccggtcagaagtctgaaattgcgatttttggaaccagtatgggtggtgcgacgacgatgatggtcagcggagtcaaaggtctgcccacccaagtgaaggcgtttattgaagactgtggctacacggatgtttattccgagattgcctaccaggccaaggaaatgtatcatttgcctaaattcccgttggtcgacattgtgagtgggattaatcatgtgaaaaatggttattcgttcaaaaaagccagcgctttgaatcaagttgcgaagaacaaacggccaatgctgtttattcatggtgccaaagaccaatttgtcccgaccaaaatggtttacccactgtatcgggctgataaggggccaaagcagctgctgattgttccaggagccgctcattcacgttcatttagtacccacccgaaactctatacggataccgtcaaaaagtttttaaatcgctatttgaactaactataaactttggcgacttcaatcagtgagtatgttaaactactattaggactgtttttagaaaggaggtccgcacttgttactaatcataattctaggaattttggccgccatcgtgggtgttgcttgcggcgtgcagctgcaaaagcgtcacttccagcaggagattcaaaatgcgaaagccactgctgaaaagctgttgaacaacgccaatgaagacgccaagaaacaatctgccaagattattgccgatggcaagcaacaaacgattgactaccaggattcaattgaagaagaacttgacagctaccaagccgataacgttacccgacagacccgaatccaacagcgggaaaccggtttgaagcaaaccgaatctcgtctggatcagctgcattcaaagctggctgaagaaagtcatgaaattaatcagcaaaaagctgaaattgaacagcttcaccacaccgcaaatgatttgtcccaggaacgattaaagacgttgcaggaacgcggctcaatcagtttagccgaggctaaacaacaaattctcgatgaattgaagacggcgttaaagcgtgaaaaagatattgaattgaaatatcaagatgacgaagcacaggtcaacgcgccaaagatggccaaaattttggctgacgacgccatccaacgcggacccgtcgacatgccgcgtgaacacattgagcattcagtgcaaattaacgacaacaataccaaacagaagttaattggtcgcgaggcctctaatattcgctacatcgaaagtttgacgggtaccgatttggtgttcgatccagatgatccgcatctattacacgtggtcacccaagatccgctgagaagagaagttgccaagacggtgattaccaacttggcagtcaccaagcagattaatccgcaatcaattgagcaccaggttgagaccgctcagttggatttgatgaacgagcttcggcgcaccggtgaaaaagtggtcggttcgcttcacatcggctggatgcatccggatctgttgaagattgttggtcgactgaagtatcggaccagttatggccaaaacgttttgaatcactcgattgaagtcgccgatatttcagggatgctggctgccgaattgggcttgaacgtcaagattgccaagcgggccggcttactccatgatattggtaaggcaattgatagagaagtagatggtacccacgtcgagttgggtgtcaagattgccgaaacctatggcgaggacccacaagtcatcaattccatcgcctctcaccatggggatgttgaagtgacaaccccaatcgctcatctggttgcggctggagattcaatttccggtgggcgcccaggtgctcgaagcgagtctgttgaagagtatgtcaaccgactcaaaaatctggaacgcattgccagctccaagcagggtgtcaaagaaagttatgccatccaagcgggccgggaaatccggattgtggttgatccaaagaaactggacgatcaacagaaccaacagttagctaatgaagttaaggatgagattgaaaatgagttaacttatccaggtaagatcaaagttacttcaatccgtgactttaaagcggtggcttatgttggcgctgagaagaaaaaagtgcataaacgattgaagaaagcataattaaaaaaagacggggacaagggaccttttgattcctaccatttaacacaaaagtgcaatcattctaaaaccaagaatgattgcacttttatgttaaatggcaggaattggcctattgttccagtttcttttagggtgcgatggaacagtttctaatttcatttaataaagtttgtcgctaaggcataaaccaagaaaagcagaacaccgacaatactgatattcctgaccaaacgcgggattttgtatgccggaacattcctgtacggtggcattatttcgcttgcccatagataaaagccaatgatagcaagaaagcaaaatgagagttgatatgaaaaacttaggccaatccggacgagcggcatgaggacgaatatcaaaccgcaaaacaccagatataatctaatttggattttaaatgatcgattgataattacagaccctttcttcatttagttggggttataagagcattttaaaaataacaggagccttttgatcttgccgaataaattaattgcgcttctcagaatcagaaataatttcaaaattatgattgacggtggcttcaatcaccggatgcttctgtaagtattccataatcacgtggctgattgtcatatcacttgatttgacgatcttatcgctggtatacatgggatagtggccgccgccgcttgctcgataacggttaagggcgatggtcaggacttgatcgtcttggacatccttgccatgatacttcaatcgggtgactcgatgaccaaccggtttggaaatattcagggtataatcaatcccttcatacatatcgtagttataaaaacgttcctttggaaaaacaaatttctcgttcaccacgacgtcaccgtgccggaccgtgaagtattgagcggtcacttccaaagcgccgcgcaaatcggcgccggtaatctttgaggcgaccaacgtgtttggatacacgtagttagtaatgatgttgcgcatggtaatgggatcttcaaatccgtgggcctcattgttgtaaagggcggttgccgaaaggtcagttcccatcttatccatttgaattttttggattaattcgataaatgctgattcgtgaattcgggccttgaatgggtcatcgaaagttaagctgcccttgattcgtgaaagcggcttgtccagccacgcttccaaatgtttggataaatccgtgactgttgatttgattgtctggtcgggttcactgtctttgacgttcagcagttccgcgtcacttctggtgaccgtgtggttcttggtctcaatcgaaatcttggccacatattgcccgcgagaacctggctgaacaattggcacgttaaataattggctggcaattttgcggtgttggtgcccagagatgagcgcatcgatcccagaaatattctttaagatatcgtagccgcggttttcgcctgggttgatatcgttccagttaccggtatgatcacgttcaaagccgccgtgatacacgacgacgaccacatctgccttcttgcgcatttccgggacgtagcgtctgcacgcgtccaactctgaaatgagattaaaatcgttgagatcattgacgttcttccattttttagtggaagtggttgtcaggcccaagaaaccgattttgacaccggcgacatccataatcgtgtatgggtcggccaacagcggttcgttattgttatcaacgatattggcgcacacaaaatggcggtctgaattcttcatcatgtagttgagataatccagtccgtaatcaaattcatggttgccgatggtgccgagttggtagccgacttggttataagcagtaaaaaacgcttcctggtcctgcttatctgctcgcttagccacgtaataagccatcggtgatccctcaagaaagtcgccgttatctaacacgatgatcttttcatcgggatgggtcttttgataatttttaatcgtcgaacacgccttctcaataccgaagggtttatcaagacctgaatcaacgtagttggtaggttcaataaacccgtgcgtgtcgctggtcgctagtagcgtaattttcatattttcacccacacaaaatcaagtatatcgtcaagtatagtcaattatgccatgattgtaaattagggttggccaaagtagttaagccaacaggaaatcggttccggatccctgctccatgtaagccatctgatcagtggaaatactttggctgagctggtctgacaggcttctggaaatcttaccggctttgaaggcatctgccacgtaggcgtattcatattggaatgatttaatcaacaggctatttctgtcactggtttgggtgtcacctgcagaacggctctggcggaagctgtacgagctgcggacgaagttgactgcattgctgttttgatcgtcttcaatttggtctaaatagctgttggcactggtaaacatggcgtctttgatcaatagattagtctgttggcgctggtcatgaatctgctggcggttttgcttaggaatggctgcttggattcgttgtttgatttgtttggttttcttccgcgacttaaatcggcgcagttggtatttaaaaatatacttaacccttgtccaaaagcccaagtggttgctgggtgcagtgatcatccgtcgtgaaaacaaattggcaatcttttggtcgattttgccctcggcggctaaatcaaccactgcctggacgctgacttgctgggcaccggccataatttcctggacctgtttgcggtcgacttccggattatttttctggctgttcaacatgtcaatgacatagttgcggtccaaaagtgcgatcgtcgagtcttgcttgacctgggaaatggcgtagttgaccatttcaccacggtattgattgaactgaccctgatcctcaacttgctttttcggacataacaggggcagggtgattgttgggacaatcaggcttaataagatgacaattgtggcaatgtagatcaactggtcgcggaatggaaacggctggccaagggacgtcagcggaattgacagtgccatggccaaggtaatcgttccatgaaccccaccgatagcactgaccagggcttcgcgtgtcgttgggactttatcttggacgccaaacagattggtccgcatccaaatataccgaatgagtaacataaccagataaattgccagtgcatcaaagaccaatttgataattaaggtatttgaatagggaatcattcgtttgatgactttcggcagggtaacgcctaagaggacgaacaccaccccatttaagaggctggtgatcacaccccaggtcgcattggtgaccagccgcacactggtcgaagtgagctttaaacggctttgattgatgccgtagatgatgccggcggccacgactgccaaaattccggaacatcccagttcctcggaaaataaatagatggcaatcggggtcatgatactaaatggcacgatcacgctggcagtatccattgatttattgaccaatagcgtttgaatttttacgaagatcaaacctgcgactgcgccaaccaccaggccgccgaagaagctgatcaaaaaccgcgtcagcccctgagcaaatgagaagtccccagagataaaggatgccagggctaaattgaagataacgattccggaagcatcgttgaataaggattcattttccagtgcaccggaaacgtttgtcggcagttcgatatctttagtaattgatttgaaggccacagagtccgttggggtcacgattgcggccaccgcaaagcaaagtgccagaggaattagtggcagcagcaagtgggcgactaggccaatgatgacggcggtcaccaccgccaggatgactgccagattcagaatttgtctgattgaatggcgaaaatagcttgcgctcgtgttttggccgtcattgaacatcaacggcgcaatcaccatcagcatgaaaatttccggctccaaagaataattctggaagaatggcagtaatgataataagaagccgcaaccaatttgatagaaggtcaatgggaggctgggaaagattgtgtacaagatgttcgcaatgatcgcagccacgattaacagggtgagtgaatagaagactagcatttttttctcctttaaatgattttaataccaatattatagttgattgagtagataaacggtgtataattaatttcacaagtaagttactataagtaagtaaccgtattgacaaatattgtcagtatgataatatagtaatcgaaggatgttgtttctcgtttgtattttttgttactgagcaggggggaattgtaatgctgaatttatatgtagcacaaagcagcgcttcaagtcggaaggcacgtgcatggttgaagagccatcacattgattttaaggaaagaaatatcaattccaaccctcttaacgctgatgaggtaaaacaaattttacgtttaaccgaaaacggcagtgaagacattatttctacacggtctaacatctacaagaagttgaatttggacctggacaacttaactgtttcacagttggttgatcttgtcgttaagtaccccgatttgattaaacgtccgattatatttgacgatcatcgtcttgaggttggatttaacgaagaagaaatcagaagattcttgccacgaagtgttcgtgaagcagaacttcgtgaactggaatcacaaattagttaattcataaaaataactaatcagttatacggatcaattgaggaacttgggtaatatcttactcaagttccttttttagtttgtgaaatcggcccaaatcattactctcccacgcggataaaattatcgataactttggggcaaatttaatttgtacggaacaacattaaaagcaattaaggaactgtttattattctcacataatgtaaggacgacggaaaattcctagtgttgtgtttcacgtgattgttgcttaaaatcaaatcagataaacaaaggagacggacaagttgattaaaatggtcgcacttgatttagatggtaccttgttaaccagtgacaaaacaatttccaaaggcaatgagcaggctttaaaagccattcatgacgccggcgtgaaggtggtgctctgcaccggccggccgattaatgccatttggcggttcattgaacagttaggattaactgaagacaccgattatacaataactttcaacggtgcactagtggttcataacaatgataaggccgagttggcaaaaagtgggattgagaaggccgatttggtgccgctgcacaattttgtcaaagccgagaatgcaccattagacatcttggacttccagcaggtctatccaatgaccgacttgaagccatcgatgtatcagcagcagttcaagggaaatattgactttgttccccgggccttttctgatttgagcacgactgatgaatactccaaagccatcgtcagtgacaagcctgaattattggatcagtatcagagcgccattgatgacaccttacgcagccactaccacattgtccggtcacaaccgcagatcatggaatttttggcggccggtatggataaagttgtcggcttgaaggcattgttggctcactttgacatggacttcagcaatttaatggcctttggcgatgctgaaaatgatctgggaatgatcaaaaatgccgagatcggcgtggtcatggaaaatggccaagacccagtcaaacaagcgggggatgtcattaccggcaacaacgacgctgacggggtggctcagtacgttaatcactattttcactaacctgaaccagctcccggtaaaatgtttaagattgatctgacagtcttttttcgatttttcatttgtattatgataaatgtaattcaaatcaacaatcatgaatgggggaatcgttatgaaacaaagacaaggcatcatgacattaatttttgctgcggtcctttcaatcgggctgctcggcggctttacttcgacagctgacgtgagtgccaagcagaccgtcaaagtggtcaaagttcagaaggttgcgaccaaagcttatcgggcaaccaagggttacatgtataattcacccaagctcaccaagaaaattcataacttaaaaaattatccgaagacgactttttattctaaaaagcgggtcaccattaagaccaccaataacaagaccgcatactacacttacgttgccaataagagcggcaaaatcaaaggttatgtctactcgaaatacttaaaactgtatcagccaaccaagacgacatcgaccagttcatccaattctcaatccgataactcgatttccactccccaagtcatttccaaatcgtcattgtcgtccttaattgcggcttctccggacttggatccgacgggagagttactgagtctgacctcagctgattacaagacctatcaatcggttttcaataagaatttcaatgttgggaactatgccgatgagggtgtctttacagatgatcaggcctcaatttatgtcaaatcaccaaccctgcagccttacgtgcaaaaggcaatcgacaaatggaacactgctttgggcaccactgtctttacacttgggacggcacaaaaccacagcttgacgttgggatttggtaacggccaatcagaaggctgggatggtgtctttgacggcgacagtgtccaggtcgattattacgacttccacgatcggacttatccatatggtccgatgccattgtcctcatcgcaaaccatccagattaaattgtcgactgatgataccgatgttgacggggccgctgaagggatggcagcaacccgtgtcaaacagtcagctgccactcatcgtgatactagcgcccattatctgaccaccacagtcagcggtacgccaaccgaactgttggaaaattactgggtcggcgtgattacccatgagttgggccacgctctcggtctggatcataccccatatttccaagatattatggcagctccggccagcaccgaagatggccagagccaggaaaatgccaaatatgactggacgacttacaaagattccgacaacgtccaaggtggcgctttaaccgcgacactgagtcagcgagacattgatcgtgccaagctgaccaagctactagggtattggtgagatgaagttaaatgcatcatcaattagatcattcggttcatagacacaaacaaaccgcttattcctgtttggggaataggcggtttgtttgtgttaattatcaaggcgcttcatttttgcattaatgtttactgaacaatccagtcaagtgcgtcatgaatgcatccaggtaggctggaacatcagcattgacagccactttgacgttggtgtttggatcatccagtcttgccgggtctccggtcgttcggccgtaatacttttcgtcggtggtgacatacatgttcaaatcgatggtttggacgaagctggggttaattgccacgccaaccgcaaacggatcgtgaagggcacagccgtgaagatcggggctggtgacttcataagccttgatgtagtaatcgacgatgtcggcgaaggcttcaccagatttggtgtgaagatcacgccatttctgggtttctttgtaagttaatagggttctgagggtcacgtccaagccaacttgagtcagtggggcctttctaaaaacgtgatcagcggcagttgcatcctgttgaatgttagcctcggcgacgttggtcacatttccaggaaccgtaacagcgccacccatgatggtgatattgccgatttccttggtaatttccggagccttcttaatggcagcgtccaagttggtcaatggaccagttggaaccaagatgagatccttgccgtattgcttaacggcatcaataaagaaatcaatggcatcgcctttttcaggttgacgtttgggatcgggtaattggacatcgccgatgccgttttcaccatgaatctgagcactaaccggcattctgtcgaagtgatcggattcggatgagtgtgacagtccttgataaaccggaacgtccgttgcgcccaagagttccaaaatcttcagtgaattttgaaccccgtcttcaacgtacacattaccgtaggaaccgataataccaattaaatcaacatcgggatcggcgaccgcataagcaattgccattgcgtcatcaataccggtgtccaggtcgagaatcatttttttctgagccattaagaactacctccgtttgtgtattatcaaggatgaaaaccctttacctaatcataaccgaattttattggaaactcaattccgcttcgaacttgaaaccgattaatttgtaagttacgcttaatggtatcaaccttaggagtaaattatgaaaaaaagtgttaaaacaattggtagtcattttttctctttggtgtggaccggtgttcgtcgaaattatgataatttggatgataacatcgccaaacatctgggagagtccgagcccaacagtccggttgagattcatttatcacggatgttttcggaagtctttaaacggcattccagagacgaagccgaccgtttattcatcgtcggcactaaaacaacgactcccagcctgcggaaagtatccagccggccggtcacgccgtggttttttacccgcgtctttttagttctggcagtcagctttgtcatgttaatggccttactgtttgtcttcaaaagtaacaaggtcattcccggaattatttttatcgggtccttggcagtgccattctcacttttgatgatgttctttgagattaacgtctatcaaaatatttctgtccggcagaccatggtgatctttttagtcggcgggattctgtcattgattgtaacgatgaccttttatctcatcctgccgattcgaaccgaggttagtattgaatctgctttgattgttgggattgttgaagaactggctaaatgtgtcgtcattattttgttcattaatacctataaagccaactacattttcaatggcgtcttaatcggcgcggccattggtgccgggttctcagttttcgaaagttccggttatgtcagtgaatacggtctggccacaatttttacccgtagttttcaagccatcggcacccatgcgatttgggcggcgattattggtggggccgtgattctcggcaagacgcggaaaaagcaatttaccgtgcgggacttctttacgaaacccaaatttttcatattctttctcgtggtcatctgcctgcacacattttgggattgggatatccccaacaccggaattggcgtatcattactgcaggaattaattgatattgcgatcgggtggttcctgatttttgtgatgatcgatgccgggttaagagaagtcaagacattgcagggacaacagattatcattcatcgaagtaaacagaagaagttcgttaataaacgctaggaggatcctgatgacagaagttgattcattttatgacattacgattatcggcggcggtccggcggggatgtttgccggtttttacgccggtttgcggaatgccaagacccaaattatcgaaagcttggcagaaatgggtggtcaggtgacggcattgtaccctgaaaagacgatattagacgttggcggctatccaaacatcaaagccagaacattagtcgacgaactggaaaaacagctcagcggctctgatacggccgttaaattaaatcagacggtgatcgatgttcaacagattgacggcggctatcaggtcaccaccaatcaagaagttaccaagacgaaatcaattattattgccaccggggtcggcgcctttaatccccgtaaggtggcggttgataacagtgaagattttgagggcaagagcctattttatagtgtcaaacatctggatcagttccgcgaccaaaccgtcttagttgccggcggtggtgactctgccattgatgaggccctgcttctgcacggtgtcgccaaaaaagtgtacctgctgcatcgccgcgataagttccgtgcccttgagcacaacgttgaacgattgatccagtcgaccattgaaccggtgaccccttatctgattaaaggcttaacccaattggataatggtcaagtggaagttgaagcaaagaaaatgaagactgaagagatcaagaagctgaccgttgacaagattgtcgtcaattacggctttattgctcaagatgatgccttgaacaaatggcaggctcatccggaaatcaaccggggcaccattgaagttcaaccaagcagcaaaaccaatttacagaacgtctttgcgattggggatgtttccaagtacgaaggcaaacagccactgatcgccacagcctttggcgaggcgcccattgccgttaattcgattatgaaaagcttgtatccggatcgcagaggtccgattcacagtacatcgattagaaaataagacacataaagacggttatcctcaattttgtggatagccgtctttatgtgtcttattttctatctaaattatattgtttcaaagcctgaccagtccgagattgtgattcttgttgggaatcttttggcaatccggagaacaaaatccgaccaccgtaaatcccggcatccggaccaacgtcgatcagccaatcagccttactaatgacttccaggttgtgttcgacgatgatcagggtgttgccggctgccaccagctcatcaaacagtttgatgagcttggcgacatctttcatgtgcaggccggcagttggttcatccagtaagtaaatggttccggtttggttcaattgaactgccagctttaatcgctgcagctcaccaccggacaatgttgtgagcggctggccgagggtgaggtagtccaagccgactttttgcatgttgattagtttgtcataaattttggtcgtatctttgaagaaatcaatcgccgattcaattggcatattgaggacttcactgatgttcttgccttgatacaggtagctgagagcctcgttattgtaacgtttgccgtcacacatttcacatttttggacgactgggtccatgaatgccatgttggtgatcgtaacgccttttcctttacagcggggacaggcgcctttgccgttataactgaacagactggtggaggccccggaaactttggcaaaaatttttcgaatatcatccaaaatatcgaggtaggtgacaggcgtcgagcggatattcgttccaattgctccctgcgccaagtcgatatacggttcgtggagctttggccgtaaggcatccactaacgaactttttcctgaaccggcaactcctgaaatgaccgtttcaacacccagcgggatgtcgacgctgacgtcttttaggttatgagttgtaacattttgcagtggaatagttgatttaaatggtcttggcttccgatatgtcagtggttgtttcaggtattcaccggtcatcgtgtgcccattgagcagttggtcataagtaccggtaaaggtcacctgaccgcccccacggccagctttgggaccaatttcgaccacataatccgcaattggcatcaactcggggttatgctcaacgaccatgatcgtgttgcctttattcttcaaattgatcagggcatttttaatcagctgaatgtcatggggatgcaggccgacgctgggttcgtccaagatgtagaccatatctaccagtgaactggtcaaaaatttggcgattttaatccgttgcgtctcgccaccagaaagggtttcggtgctgcggtccaaagtcaggtagcccaagccaatgtcgatcaacgactgaatcttggttgcaacttcacgaatgacgtccgtaaccaacggaaccttgatttcgtggagaaactttagtgcatgaaccaggtccattgccaaaacatcggcaatatttttgccgttgattttgcaagtgagcacctcaggacgaaggcgggtcccatgacattcaggacaaggccttctggtgacaattttagccagggcttctttgtggtgctgagcttcctttttgccgataattgatcgacgaattctgggaatcaagccttcgtaaagagcggttcggtgccaggcggctggtgcgtccttcaacgtttgttgaggtgcatacaacaaggtatccatttcttttttagtgtagtcttgcaaaggcttatcattgtcaaataggccgctgtccgtgtaccgccgccagcgccaagtgttgggaccaaagctgacaaaagtgattgccccttggttcagtgacttttccgggtcaattaacgcattggcatcaatatcatcaacgtagcccaatccctgacatttttggcacattccttggggcaggttaaatgaaaaagtgtctgaatagccgacaaagggttgaccagcccttgaaaacagtaatctcaacaacgagtaaatccccgtgtaggttgaaagagtcgagcgggcatttttaccaatgcgcttttgttcaatcacaatggcaaccggcaggtgctcgatacttttaacgtgcggctgcccatattttggcagatactgttgggtaaaactgggaaaagtttcgttcaattcccgccttgaggctgcagcaatcgtatcaaataccaacgaggatttccctgatccggacagaccagcgaagactgtaatggcgtacttgggaatctttaggtcaacgtgctttaagttgttttgataagcatcgtgaacttcaattgcaccatgttcgaacatataaatttatgacctcctatttttttgatgatttttagcagttgggagctttttgggaccggcttctttcttaagttctttttgcagctgattgacctgtctggacagccgggtgacttgtttggttaaatctttcagcgcatcggtttcgtcattgtgtttatcctgagaagtgaaaaagtcggtgatggtggaagttaacaaaccaataaaaccgattccacccagcatcaggacggccgaaatgattttgccgccatcggtcttgggggtaatgtcaccatagccaacggtggtcgccgtcgaaatggcccaccagagtgaattctgcagtgaatcatgctcaaaagacgcaaagattagcgagctgaagatgaggattaccagactgattgataacaggtagataaagccggtatcatagagaaacttgtgaagggcgttggttaatttgccagagagaccaaatcgccacagcaggttgtaataccggacaatcgaataaatcctggcaatccggaagaagataaaaattggatgcgagggaatcagcgcaatcaagtcaaatagattggagattaggaaatctttttttgacttggcccgtttgaaacgaattaaataatcgatcaggaaaaagagccatatgagtccaaagatcactcggtatggcccttcattgagggtgattttagtcacgagggcaagaactgccaagacaaaggaaaccagtgccaatgaaacgacaaggatattgtaaagcaaaattggcatgttcttggtggcttgtttcatctcagatttcccccttagcgactgctgtcgttgttattcgcatctggattggtaatcttgattcggttgctgtcggttgtcttgtggtgaatttccggcgcatcggtgaagtattctttccaagtcgacttgtcaccgttcttggaatagatactagtggacttcttacccaaacgtttttcaatccgcttttctttttgataaaggtcggcgtaattgtaattccgtggatcaattgccttaaagccctttggatggtagaagcgcaacagattcttttcgttcaacgaatctgataatgaaagctccgtttgaacccgctccttatccttcttgacttgagcctgttggcgtttggttaatttcaacagttggccggtcttattggagtaaatgccgccactcagggaggtaaacgccgggctgacccagtcctgatttctgaaggcaacgacttgatcgtgctgcttggataaaatgtcggtcccaaattggacgtagcgcttgctgctgatacctaggagatgcatcaaagtcggcaggacgtcaatttctccggcatattttttcgaaacgaagccgttcttttggccgggcacatcaataattaacggtacccgctgcagctgggcgttatcaaaatcgtcccagtcgtcaggattcttgcctaatgccttggccaaattggtgttttccgaattggaaatgccatagtggtcaccataaagcagaatcaaggaatgtttgagcaggccggttttgcggaggtagttgtagaactcatggacggcctggtccagatagtgggcggttaagaagtagttgtccaccacgtcatcaccggtattggtggtcttgaaattagtatcttctttatccaaatcgtatgggaaatggttggtgaccgtaatgtatttaacgtagaacggctgttggagattctggaggtatttgaccgaatccctgaataacaatttatcctttaaaccatagcccaaggagcggtcaccggtggtgttgtagtaactggcatcaaagaagtattgataacccatgttcttgtaaacgttattgcggttccagaaactggcaatatttccatggaagaccgcagaagtatagccacgacgctgatttaagatagctggagcggcttggaaggtattgtcactgccaagttgggcgaacaaggatccctgcggcaaaccgtaagtgctggtctccagcatgttttcggcgtcagaagtttttccttggccaacctggtggaagaaattcttgaaagcataagaggatttactcttatagagtttgtttaaaaatggggtcacttcttggccgttgattttcttgccaatcaggaattgttggaaactttccaagtgaatgacgatgacgtttttacccttggcaatcccatagaactttttattcggtttggcataatgcttgcgggtgaacttcaagacgtcgtttaattccgatttggtagcggtggcccgtaaatcattgttgtgctgggatttgaggccatcgtagactgtaaaggcatccaggccgaggtacttcactatgtaagcccgatcaaatgtccgcgtcagcagctgcggccgatccatttcggccagtgacaggttaacaacgaaaaaaaggaccgaaaacgaggtcactgccaggccaattcggcgattcagcggccgggggtcgattttgattttgcgaaggaccaacagcaaaatgatgaccaccagatcaatccagtaaaagatatcgtggaaattggtcagggcaagtgagctgccgctgagcccttggttgaccttggagtagccggtcattgtgctgacggtcataaaatcggtgaactcacggaagtaaatcacgttaaggtacagcaaaacggtgtttaaaattgaaattaagatcgccagcggataaaagaaccgactttttttgaaataaagggcgatactgagtaacaaagtcgtcgttgccaacgggttaattaagacaatcaggaactgaaagggattggtaattcccagcccgaggtcgacaaaataggccaacatggttttggcccaaaagcaaacaattaataaaatgatgaagcccttgcgagtgctgcatttttccaggacccaattaatatatttcaaaacagtgtgctccttacaataattacttgctttatcttatcaaaaaaacgcgcagaaataaccattgtcaagagattttgcagaaatcttaagttgattggtgtgcgcggattctcaaaaaattgttatactttagatattaagggtaaaggatgtgtcatcatgagtaaatttaatttgtacatggttcgtcacggtcaaacctactttaacatttataacaaacttcaggggtggagcaattcgccactgacggaaaagggcattcaaaacgcggtcgataccggtgagaaattgaaggacaccaagtttgcggctgcatattgcagtgataccaccagggcggagcaaactgctcaaaccattttagatgaaaatgacgcctcggatattgatgcgccgattacgtcaatgtttttccgtgaggagttttatggctactttgaaggaaatgatatgagccaagcttggtatttggcaggcgccccacacggcttgccgaccttccgggatatcgttgaaaaatattccattggcaaagcgaaagattacctaaaagaagccgatccgttccatcaagctgaaaacaatcaggaatactggaaacgtttggatcaggggtttgacctgattaaacagaacccagaaatcaaagacggcgacaacgtcttattaatcagtcatggtaacacattgctgagcgttgtggaacgctatggcaatggtcaatttgatgtgactgagcggccagccaacggcagtttgaccaaattgaccgttgacggtgatgacatccatgtggtggcctttaaccaacaataataacaagttaggcgggtatgaatttggagattaaattaactgatcaattggatcaaatttatcaagacgcaagaaccattcgccatcatgtcttcgttgaggagcagggaattgctgaaaccgacgaatttgacggtactgattccgacgccattcattttgttggctatgtgaatggggaaccggtggtaactgctagaacgaccgttaccaaaaagggcgttcatattcaacgagtggcaactgaaaaagccgcccggcatcaagcttatgccaagcagctcctggaatacctgctggaccaaccaatgtttgaagacgccccaatgttttatttgggggcccagaaaacggcgattggcttttatcaaacgctgggatttgagaagtatggggagccatttgaagaagtcggcatcccgcacgtcaatatgcggcgaacgcactcagccgccgatcaccacgatcgataaaatgatagttggttgtatgtaaatattaacagagagatccaagcggaattcaggtaccgcttgggtctctttttgctttgcggtccgtggtcacacaaggccatgacattaaagtgacattttacttgacaaaattggcagataaaacagaataagagtgattaaatgaacgattccaggggggattggcatggatcaattaatggcccgttcaatgaaagcctatcagagcaagtttgcccgtgtgattcaggatactttggcgctgctgtttccaattatgttactgggaagttttgctgaggtcctgaaatattctttcttgacgcccagtgggtttgttgccaccgtattcggggtgactaagtggctgcccgctgcgaggcagatttcacagttattggggctgattgtccactgtacggttgacatgattgccttatacggcgcttacgggatcacctactgtacggtaaaagcctatggtcgccaaacatcggcgatgtcaggtgctatcggcctgctggcattcttgatggctgcctatcagccccatagccacgggcgattgctgtttaacagcactttgatgggtcagggactgttaattgccctgataattggctatatcgttggacggatcattgttgccttcgagaaacgccgggcgttacgatcctaccaaatcatttggcccttgctgctggtggttgtgttttcaattgtggtcaatgttgttgtcagccttaccagaagtccggaggttcaatcgttcatctcgtcaactgccttgcatgcggttcaggccagcgcgctttcctatgttatcggcatgggattgttgacggatctgctgtcttggatggcggttggcggaccgttttctgcgagtccgacctttaccgatccagccgcgttgaccaatttgaatcacgctctcaaaacagggtcagccttcaatgcgccattcaaatataccgatgtgaccctctttcacagttttgccaattttggcggcaatggtgcggtactggcgatgattattgcgattttagtcttctctaaacgacagcgctttttgaccgtctcgaagtggtcaattttcccagcgctgtttaataataattacgcgatgatgttggggatcccaatcgtttataacccgatttttctgattccctttctgctggcaccactggtgaacatgctggttgctgcttcttttctggcgctcaaatggattccggcagccgtttatccggtaccttcagggacgccggggcctttgattggtttcttgggcaccaatggcaattggttggcgctcattctcggagcggttctgattttcgtggatgtgctgatctatatgccatttgtcaaactgtatgatcggcttgatcgaaaccggggtgagcaatgatgaaacggacagttaaaatctggttatggagtcttcttgcggtgttgctgtcagttggcttgattatcgcgtcactccagtggtcacaccaaaatgtcagtgagttaacccggcaccacaactctcagttatcgccagtcatcatgattccggggagttcggccaccgaaaaccgctttgatggtttagtcagtgagatcaaccacaaccgcacgaatccgcatagtttattgaaggttaaaattaccaacgatgacaaactccacttcaccggccgtctgagaccgggggacaacgagccgttcattgtggttggctttcaaaataacaaggacggttatagtaatatcaagcaacaggcccgccaatttaacgtcattttccataccttggtcagtcgattgaattttaataattttaaggcgattggacattctaatggcggcttaatttacactgtatttttggaaaattattttgaccaatattctaatgatgttcggatgactaagttgatgacaattgggtcgccgtttaacttcaatgaacggtcgattgataataagacgcaaatgttatcggatttcatcaaaaatcgcaacaagttgcccaataatttgagtgtctactcagttgccggcaccaagaattacacgtccgatggattggtcccgctggtaagtgttgctgctggccggtatgtttttcaaggcgccgttcgtcactttacaacgatcacagtgtctggttccaacgcccagcactctgatttaccggaaaacaagcagattgttgatttgattaaccgatacattctccactcgactcgggttccaagagcaagacaaaacgaaccacggttacattaaccgtcgtcgaaaatgtctgttaagccacgaccagctttggtgaatcgtaatcgctgaggcaaatgacagtagccaagttccaatgtagacggagaaaatgcctaaaactggttggcgactcatcaacccttggccaaatgttcgccaaagcagttgattccaaaagacgttggacaaaaaggctggataggcaaagttggccaagcggtgaatcagatgagtgaccgggagtttccgcgtaagttgggagtcgcctaaagcagcaatcaaactaatgatgctgaggtcataaatggtcatcgatggtttgtagtatggggcgttagtcagttgaacggggaacttgaaggcaaataattcatagttaatccaaacgaacgatcccagagcaaaaacggttatcagcccgtgtttttggagccagcgatgggccacttggcgatactgccaagccagagtcccgacaactgcatataataagaaactgacaaatagtctgtccagcaggtaccagtccttggcatgtgggccgtgaaagacttgggtgtcatagaaaattaaccagaccaactggaccaccgaagtcagcagcagaaccaaccggccacgctgttgattatggccacaccaattggccagccaccagaaaagcggcatcagaatgatgaattgcaacatcatcgaattgtaccaaaggtggggtgcagcattcccgttgatgaattgccaggcaaagtcgccaatcgtgtggtaatgctcgacttgctggacatttggcatgattaataagtagaccagggtccaagcaatggtggggatgaatgacgcgtgccacatttgctggagatagccccggtagcttaaattggtgtcgtgagtgactcgcatggtcgtatacaggatcccggtaatgaacgcgggtgccgtgaatttgatgaagttgtaacaaatgccaatgccgatctggatattgacggtcggatgagtttgcagggcttgaccaagaatgatttgcagcatgacggccgcgcaggcaaataccttgaggtaatcgcccatgtctggggtactgggagatttgattttgcgatccatatctgtagctcctttgaagaattatctactaccaatataccaagtgaagccgaaattacaaaaagaggctggaaacaaatgaatgtttccagcctcttcaggtgatagttgattgaattgttgttatgttgctatgtgttaaaaagattaatcgtcggtagcgtcatctgagtcaaagttaacgatatgagcggaaccaacgtaattccaccatggggctttgacagtttcggtgatgacaccgcggttttgagcatcgatcatcttaccgttgccgatgtataaaccaacgtgagaaattgatgctgcgctccaaccgaagaataccaaatcacctttttgcaggttcttgtatgacaccttctggccggcgttgtattgtgcttgggcagtacgaggaagggtgacactcgcagcctttttgtaaacgtaactggtaaagcctgagcaatcaaatgctgaaggaccagtggcaccataaacatatggcttgccgaggttttgcttggcaactttataaacggctgaatatgaaacatcagtgtcggcagctttggatgcttgagcatcttggaaaccggcaaatgataatgtgaagaatgctactagcgtaagtaatatttttgtatgtaatttcattttttatcaacaactccctatcaaatctacagtgataacaataccaatgaattgttgcaaaagtgtaacaaacaatttgcaatgcagttaaatgtcatatggcagttgaaacattggtaacctggcttgtgaataaccgtttccacaagctgatttgagggtgtttataactgagcaattaaaaaagccacccaatgtgaattgagtgacctttttgaaaaatatccccatgatttggattaaatttgtctgaagatgacgtggcaaaaatagaaatcttaataaattatttatttattcttcaaaagattgtctttattgggcaaggttacggccaatttacccatcgaagtgacgatcatcggcaagatcaggtagtagacgcagaccgtgtaaatgacgatcaatgccgtttcaatcattgcaaacgatgcaccaaatgtgaggccaattgccaaggcaatgacgactagcagaatgtagcggacaatcttgccgtaactggccatggttggccgaatccattccagcagtgacaattccgtgtatctgaatgacaagcccaacgcaatgatctgccaggcggcaatcgcggtcaggatgctgattgcaagaattggcacctgccagtcaaattgattggtgcccgtgacataatgcatggtcagataggttaattgaaagccggtgatcgcagacatgataaacgcaacggtccaatacagcggttggagaatcgaacgactgacaacgaagacagtcaccaaaatcccgataatcactattgccaataaagtaatgaaatgatggttaagtttggactggttaatggattgtgtaatcggttcgccggtgaaggcaacctggtctgacgacagcggagttccccgcagctgcaagccaacttgagcttcgagcatcttaacctgcttgaggttggttttgctggatggggcgttgttcatgacaacttgaatggtggtaatcttcttgtcctggctggtgtagttaagcatcgtctgtaggaagtcggtgtccaccagctgcgctttggtaatgtaatagacgttggccgcaccggacttttggagaccattcaaataatcatagatgttgtttaactgatcggtcgaggaattaacctgggaactgacctgttttaattgcttttggacttggctaatttgttgactgtaactctcaagattattggcgctgttttgaccataattttgaatgaccgatccttcggcgttcagttggctgatgcctgacgaaacactttgtaaggactgattcaattcgttaatcttctgttgatacatgcggactctgcgtgaagcaccctgctgaacggcgacactggagttggcagcaacactgttaacttgtgaggctaagctggagctgtcttccacaatttgattactctttttaaccaggctctgcatgtctttgacctgttgcttgaggccggacaaattcaggttgctgccgctggtttcgatcccattggaggcctgtgaaagttgcccggttgcctgcttggcgtttagtccgatcgattcaagttgattggaaacgtaatacttttcgatcggcatcccacttggctgcgttaatgaataagcggcgctaacccctttggtatgctgaagtttagtggttaactggtccaaatgctgcaggtatttttcattatccaagggctgatcgtttttaaggtaaatcgtgatcggcgttgctttaccctgtgaaaaatgtgcctggagaacatgggctcctttaacggcttgattagtctgcgttaggttggtcattggagaaaaattcaggctggtatggtagaagtaaatgaacggtagggtcagatataaaacgaccagaaaggcggcaattggctgccagagtgaaaagtcggttgcccggttccagaagtgggatttcatcgcactcaatggggcgctagacggccagaaaatactttcccctagagcagccaggaaaacagcgttcagggtcaagacggccagcattaagacaacgtaggtgatgccaagaacccacagtgattgtaattggtcatagttaatgaagccgcagcaggcgaagatgatagctaaagcactgccgacaatggtgattggaaagcgtaggtcggcaattgtctgctgggtggcataacgcgcttctcgttggagggccagcacgcttctgagcttgcggtagatgtagatgttccaaatggtgccgatcaccacggtggcaattccgatttcaagtggcgtgtattgagtgaaggcaaagttaaaatgtttggccaatgccgttgagatactaaatgaagtcgtaaatgccgcaaataatgtaatgaaagaaatgaccggtgcaaataacgaccggaagtaaattcccacaatcagcattgaaaccacaaataatgtgatcaaaatgatgttggtaacttgcgcggttttttcattgttgacgtcgcggacaatttccggactggtgacgtaggactttaatccaggcacctggacttcaccaaccaattcattggtcaaaacgcgcagggtactgcttttggcgtcgatatccaagctggcaatttgagtagaaccatctttggacaacagctgctgtttgccggccacgttggtgttgatggtgacgatcttcttgatactataaaatgattgatgggctttgagtttattcaaggcattgtcaatcttcgtctgctgcttagcggtgatcttgccgtttgggttcgtgtagaccacgttaatggtagacgcttttcccagattgtatccccaatcatttcgcagctgctgagcctgcgccggttgtgagtctttggaaaaggtgggctggctgtatgactgcagtgtatcggtcacgtttggagcggttataattgcaataaatgtaataatcagccatactaacagcgtgaataagcgatttttgtgtaattttgcgatagtttccttcattgattcgtcccctaaatatgtatgtatgaaaaaggctcatatattaagagtttaccattttataaaggctagtgcgatacgttttgggcgttttgtggtatattgggaaaattgttgtgaaatttagtcgaccatttttgatgggaggttcttaacgtgtgtacaagtatttttcaaattggccaagaagacggcgcccatgtgttgtcacggacgatggactggccgcagctgggagctcatcccgtctttgtgccccgcaactacggttggcactcggtatatgacgacaaacgttacgtcactaaatatgcgacgcttgggtccggccaccagcacgctaaacgaattgatatgtctgacggggttaatgaatttggtctggcggttcaaaaattgacctttaccaacggcagccagctggtcgaaacgccgggtgagaacaaaatccatctggcaccgtttgagctgtcgttctttttgctgtccaattatcgatcagttaaagacatcgaggaccatattgaagaaattgaattgatggctgacaagtacagcttaatgaagtatggacacagcgaattgcactttgctgcctgtgatccgactggtcgaatcgtcgtcatcgaaccggtcaccaccccaattgaaatcattgaaaatccattgggaatcttgaccaacagcaatcattttgatcggcaaatcgataagttaaataagtatttggattttaccccggattttgtcaacggaacggttcccctcaatacaccgcgggtgactaccggcaatgtgtccggcaagtcaattccgcccggctcatattcaccaggatcgcgatttattcgggcagcatacctgaaggaaagaattgacatcccccaaaatgaaaatgaggcggtggataattgctggcacctgttggactcagtgaatgttcccaagagtaaggagcaccagccgacttattccgtctaccgggcagccgtctgctgtgagagccggaattactactatcagccatatcacgctaaatcagttgccaaaattcaattgacggatgacctgatcaaatcgaatgaagtaaagtttttcaaagtagctgatcaaatcaccttcaatgagttaaactaatgtattgaggatatgagcggggagaaatcaagttgcgaaaacaaagttggcgggttattgtcatattattagtgacgtttgcggtgttgatcgtgggcgtttccctgcgtgggcagttaagtcaccatgcacagcgaaattccgtgccaactttggttcaaaaaaggcctgatcatttctcgactcgccaaaaacgaagctttatcaaccgcgttggcacgccggctgtcaagctgtacttgaagaatcggcaagtgttaccgagcgtcgtgatcgctcaagccattttggaatctcagtttggcacttctgaactgacaaccaccgccaataatttatttggcatcaaggggacttaccacggtcagtcggtccagttctatacccgagaggtcgagaacggtaaatcaatcaaagtcctggctcagttcagaaagtatccgaatttggcgtcctcaattgctgatcacaatcaactggtcagcgagaagtttatcaaagctaaaaatattttgagttatcgaaagtcgacgcgcttgctgcaggccaatgggtacgcaaccgatccccattatgccgccaaattaaaccgcctaattgtcaaatatcagctgagccgttatgatttaaaagcaattaatgaacgtgtgtgaccagcgattacattgttgacgcacgtttaaatgaaaatttgttgaggtgaatgccacattgttgaattgggtttctaatttatatggtccattttttgatcctcataattgggaaacggtgattaccagcggtagtgactggctgattattctgtcactagtcacgattgagtgtttgctgtcggtcgataacgcggtggttctcgctgcccagacacaggcgctgccgactaaagttcagcgggaaaagtccctgttctatggcttatggggcgcctacctgttccgtttcctgatcattggggtggggacttacctgattcatttttgggaaattaaagttattggctcgctgtacttgttctatctggtttaccaatttttccgaaaaaccaagattgttcgaactaagaaattggccggcagcaaacgccacggcatttcactgttctggtcggtggtcgcccagattgagttcatggatgtggtcttttcaatcgactcggttctggcttcactggcgatttcgtccaacccggtgattgtcctgcttggtgggatgatcggaattctggccatgcggggcgtcgctgaagtcatcatgaagttgatggggattatccctgagcttcagccgatggcctacgtgttaattgccattattgccttgaaattattcctgtcgattccggcaattgacattgaaattccagcgacggcttttggcgggatcgtgatagcagcggttatcattactttgattattcactatgtaagaaaaaagcggaggattaacgatgagcacggaaataacgccgaataatttagcggccgaaaccaacaatccactcaccgtgatcgatttctgggcgccttggtgcggtccctgcaagattttggaccccatattggccgacttggaagcagattacggtgatcaaattcactttggcaggatgaatgtcgacggcaaccaggaaattgctgagaagtaccatgtcttaagcgttcccagcttggtcattttcaaaaatggcaaagctgctgaaaaggtgagtggcatttaccccaaagataaactaagaaaatatttcgatcaaaaaatatcagaagttcaatcaatttgacgggcagtctaccgaaatggtttgatgcccttttgttttgccattggtgtcaatttggcatttaggatgtccaagccttgaagcggaaagttaaatatcggcgcgataatggctcgtttggcaggatcgggaaccacttggctttctttgagattgggcagcattttcgccaagtcggtttgggtgagatgaagtgccttgctgtaatgcatgactcgctgaaaaaccagatttttgaaccacaggtagtagatgattccagcggcggcaatataccaaaagattgtccaagtgatgccaattttggctggggacaggatattggtgaagaaagccaagataataaaggcacaatatgttaaaatgctaattatggttagtttagattttgttgacatgattgaccaactttcataacgaaatttgtgataccatttagatataattatagacaagttggaaaaatatagatagtgagatgaaattgtgaaattttcagtagagacaattgatcgcaaagattatgcggctgtacgaggtattatcgcagatagttatcaaaatgacggacccaacacagatggtgacgaggttgatatggttgatcgtctgcgcggcagtgaatcctatcatgatcaatttgaagtggtggccaaagatcacgatcatcgagtggttggccatgcattgatggtccccgccgaggtccgttccgcgacaggcaaatttccaattgtttccattgttgagattggcgttttgcatggttatcgaaacgacgggattggtcaggaaatggtcatcgaattagaaactcgggcccgcttagccggctatcacgctgtcagcgcaattgatcattctgatttcttctttaaaaacaactatgtgcctgctgacaatttcaatatcttgccaacggtggcggttgatttcaatgataatttgatcaagccactgttcgatggggccctgtatcaaaagggcggcaagatttactatcccgaagaattctttgggattcgcagcaccaactattaatttaatcattcaacgccacatgaagtagttcattcatctgagggtcagaaagccggtgggagatgcgaatcggtcaggatggattgacgaaataccgtggcggaatttaacggataataactagagccgatatcatctagtgagtgagctgtacatgtgcagttaatctgggtggtaccgcgctgaagcgtcccttagtctatttttggactgagggacgcttttttatatggaggagtatatgtaatggaaaatgatgttaaagaaccaacgattagtttaaccgagggcattgttgttctactgatgatgctattgattatgggcttcagtgtgatcaagctgcagatttcaccgcaaattccaattctgtttgtgattctgctgttgattgcctgggctaaagttcgccgcttttcttgggactctgttaatcagggcatcatcaacgggatttcaaccgggattattccgatgtttatttttattctgatcggggcactgattagctcgtggatcgctgccggggtgattccatcactgatggtctatggttttcatttgattagtgccgagtggttcctgccatcggtctttctggtttgtacgattgttggtaccgccattgggagtgcctttacggttgtctcgaccatcgggatcgcctttcttgggatggggctcaccatggggattaatccggccatgattgccggggcggtcatttccggcgccatctttggcgataagacctcgccgttgtcggattcaactaacttggccgctgcggtagtgggcgctgatttattcagtcacattcgcaatctgatgtggtcaacgattccggctttcttcacatcattgattgtcttctttttgattggccgtaccaatgcgcaactcaataccgcttcaattgaccgaacaatcaacgttttgacccagcatttcagcatttccttgtgggcatttgttcctattgtcttgatgttcttatgtgcctggcgaaaaattccggccattccaacactgtttatcaatattttggtagcggtcgggatgctgtacgtggagcagcccaagaccaagattcaagcagttgtcaacacgttgaccaatggctatgtgtcccatactggcaataaaaatgtcgatcaattattgactcgtggcggaattgccagcatgatggcgaccattgccttgatcatttcagccttggccctgggtggtttgctcatgaaattcggcgtgattgatgctgtgatggggccactgtcacggaagctgcagtcaaatggctcgctcattttggccgttatcctcagtggcattggtgtcaatgtctttgttggtgaacagtatttatcggtcattttacctgggaatgcctttaaatcaacttttgataaggcaaaattagcgccggttgccctgagtcgggctcttgaggatggcggcacggtgattaattacttgattccgtggggcgtggcaggtgtttttgccgccaatacgcttcaagtttccacgatttcttacctgccatttgcgatatttagtctttcttcaccaattttttcgatcatcagcggcttcaccggcatcggtttgaaacatttgaaaatgcatgaaaacggttagcattgctactttaacaacgttttacctaaatactggtcattcttaatttaacaaacattactcactcgttacattagttacgcggagacggtttttcttaatacgcgtgatattggatggtaacttcgtaactatacactatgtattgttgatcgacgaggtcaacaaaaattctagacacagaacacagatataggagtgtgtaattttgaaaaaagtattatctatgatcttcgctacttcagccgcagctattggtttattcttcgcaggatccgcatatgcttcagcaagcacagtagttacagttaagtcaggcgacaccgtttggggaatctcacaacaatataattcctcagtaaaggctatcgagagcgcaaacaaccttcaggatgcaaacgtcattcaagttggtcagcaattaacaattccttcagctgacaccgcatcaaatactcaaggtagtgcacatgcagcaaccgcaacgactcaacagactcagagttacagccaaccagctcaaactcaaaccaaccaagcacagactagccaagcatcaacttcaactagcactgctaccagcggttcagttgctgaacaagcagctcaattgatggaacaaaagactggtgtttcagcatcaacttggatggctatcagttaccgtgaatcaagaaacaacccaacagcacaaaacccaagctcaactgctcacggtttgtaccaatcactttacacaacaagtaatgactggcgcgaacaagtaaacgacgcagcacggatttaccattcacaaggaatgggtgcttgggcattaaattaagagcgtgaagagccccgggttgatcccggagcacaagggaaggcggccaatgatgaacttgttcatcgttggtcgtcttttcttgtgcagtagggatcaggggcgtcagaacgcatttccactagatagcagtggtaaggacctcaatggcgaacttgttcgtcgttggggctttttctttatacgttaggggttgggctgtcggagtgtatttgaacaaggtggcaccagtacaaagtcaaagatgccaatcacccaataaaaaagatatccgcagtgaggcggatatctttcctacataaaaattcaattatccccgtaccaacaactcgatttgacctttttgaggcgcgaaattaattccgacaagtggttcgcgcaaaatctttccatactcatccaaaacatcggatggcagtggggtgtgggccttgagggacgcaaccacgtcaccggcatcgtgagcttcagataagtcgatgaataaattgactttgttaaccacgtcgcggaacaggtcggttaaaatcccgttaggtttcccctcaacatcggtgataacgacctgcgaagaatcgaacgctaaatggttaaagcgcaccatttgtaaaacgtcaaacaggttatccattgacaacaagtcccttcatgatgattcatttaatattaagtgtagccgtttgcatattcaaaaggcaagtattatatcgttctgttgataaatttgatctaaaaaaggtgccgtgacgcagccattcagctgtatcacggcaccttattaccatctaaacggtgttagtcaccattcatgattgaatttttaacgatcacgtaatcaactttggtaatatcattcaacttgcggccaccggcatatgaaatcgacgactgcaggtcctgttgcatttcgttcaaagtatctgagatgtgaccacggtaaggaaccaacatttgtcggccttcaacgttacggtaggcacctttttgacgctcagatgctgaaccccagtattgcttgtatttcttgccatcaatactgatcaggttaccaggcgtttcttcatgaccggcaaacaatgaaccgatcatcaccattgaagcaccaaaccgaacagacttggcgatatcgccattgtaacgaataccaccgtcggcgatcattggttttcgagctgctttggagcacaaccgcagtgcagctaactgccagcccccggtaccaaacccggtcttgagcttggtgatacatgctttaccaggtcccacaccaattttggtagcgtcagcgccggcattttcaatttcgcggacagcttcaggtgttcccaggtttccggcaatcaagaaactatctggtaattgttccttgatgtagtgaatcatctggataacgtagtctgaatgaccgtgagcaacgtcaatcgtgatatattcaggcttctcgttgtcggcaaccaacttgtcgatgaattcatattcttctggcttgattccaacactgatagaagcataaagatcctttgaatgcatcattttgatgaaaccttcacgcttttcaggttgaaatctatgcatgatgtagaagtaaccgttttgtgccagccaaacggccaggtcatcatcgataacggtttccatattggcgggaacaacggggatcttaaatgtcttaggtccgaattttactgaagtgtcagcttcactccgactcttaatgatgttcttgttagggatgagttgaatatcttcgtaatcaaatacttccatgatttacctccgaggttttaggacagctccgtcaggtagcaattgttgctacagtttataagcgcctgactcttcttgcgactttaggacagctgcgcaaagcagaagtctgcgcctaagcacctctaacaaaattctaaaagcgggaattctgttagaggagacttaggcactgacttctagccgcttggacccgctcactgttttttaccaaactttttccacgacgttcgtctgttctctgtcaggaccgactgagaaggttgcgtaagggactccgactgctttttgaacatggttcaaataattttgagcgttggttggtagttcatcaaatgtcttgcacttcgtgatgtcttcgtcccatcccggcaattcgtcgtaaacaggcttgcaggcatcgagttcttttaaggttgcgggataatggtcaatcttcttgccgtttaattcataagcaacgcagattttcaaagttttaataccggttaggatatccaaacagttcagtgccaaatgggtgtagccgctgacacgcgctgagtggcgtaaaaccacactgtcgaaccagccgattcggcgtgggcgcttggttacaacaccatattcatggccaacttcccggatatgatcaccaatctcatcgtggagttcggttgggaagggtccttcaccgacacgtgaagtataggccttgcagacaccgatcacgtggtcgatccgattagggccaaccccggttccaacggcggcaccaccagcacttgggttcgatgaagtgacaaacggataagttccgtggtcaacatcaagcatgaccccttgagcgccttcaaataaaacatttttgtgattgtccagcgcgttgttaataatataggaagcatcaacaacgtatgggcggatgcggtcggcgtattcgttatattcattgaagatcggttcaaattctaatggttcatggtcatagattttagtgagtaattcgttcttaacttgtagattgcttcgaagtttttcttcaaagatatccttatcaagcaaatcggcaattcggatgccaattctctcgtatttgtccatgtaagcagggccgatccctttgttggttgtcccaatcttagaatccttcttttgctcctggagaccatcgaagagaatgtggtatggcatgataacttgagcacggttggaaattctcaaattatcggtactgattccatcctttttcaaattgtccatttcgttgatcagggatttggggttaacgacaacaccgttaccaattacactgtacttttcctgatcaaaaatacctgatggaatcagttgtaaatgatagctgttgccgttaaatacaatggtgtggccggcattgtcgccgccttgatagcgggcaataatatcagcactttgaccgaagaaatcggtaatcttacctttcccttcgtcgccccattgacttccaacaatcacaatagatgacatatgaacacctctaaattttattgccaggaatctacccagcatttttaataataccaacttgtattccattaatcaaccaaaaggctaataatttttacaagtaaaacgtttaatattcgactttgaaaccgaatacgaacgaaaggtaattattattctcataatatagtcaaaaagtgaacaatatggtattattatcctgtcattatttagtagaaaggactcgttatgatagatagatattctttacctgaaatgagcaacatctggtcactgcaaaaccaatacgcttcatggctcaaagttgaaattgccattgatgaagcctggtccaagctggggaagatccccgctgaggacgttgagaagattaagaagaacgccaagtttgacgttgatggcatcgccgaaatcgaagcggtgacccatcacgatatcgtggcatttacccgcgacgtctccaaatcacttggcccagagaaaaaatggatccactatggggttaccagtaccgatgtcgttgatactgcctggggtgtccgaatcaagcaggccaacgaaattattcgaaaagatattgatgcatttattgatgtgattgccaaacaagctaaaaaatacaaggatactgtcatgattggccggacccacggtgttcaagccgaaccaaccacctttgggttaaagctggcgcgttggtattctgaaatgaaccgtaacaagcgtcggtttgcgactgcttctaaggaactggaagccggccaaatttccggtgctgtgggaacctttgccaatgtgccgccgtttgttgaacagtacgtgtgtgactcacttggtttacgcgcccaggaaattaccagtcaaattctcccgcgtgatctgcacgccgattatatttcaaccttggcactgattgccaccagcttggaagaatttgccactgaaattcgtggattgcagcgttccgagattcacgaagttgaagaacatttcgatgccggccaaaagggctcttctgcgatgccgcataagaagaatccaattggatccgaaaacatttgcggattggcacgagttgttcgcggccacatggtgactgcttacgaagacgttgctttatggcatgaacgagatatctcacattcatcagctgaacggatcattattcctgacaccttgacactgttggattacatgctgcaccgcttcaccaggatcctggatcgactaaccgttttcccagaacggatgaagagcaacatgggcctgacctacggcttgatttacagccagcgggtgatgttgaagttaatcgatgccggaatgacccgtgaacaggcatacgacttggttcaaccattgactaaacaatcatgggataagggcattcagttccgtgacttggttgaaggcgataagaagatcactgatgctttgagtgaagatcaaatcaacgatgcttttgattaccattaccacattcgccatgttggtgaaatctttgcccgagttggcttggaataaccaacggacggtgattttaaattgaattaacctgaaatcgattagtgctaaatgacaagggcttggacaagacgatctgttttgtccaagccctcgtttagttttttcacttttacctagcggaattgtgaaaaaataagcgcttattttttcacactgatatttatggcagaaataccaatcgattatcgccataatcattccatttttcagcaatctgactgagtgggaaagcggtcaacggcaccgcgattttgccatcagtaatcatcttcaataaggccggcatatcgtccgccaagttggctgcggtgaacgagccgaagccactgccgattaaatggaagtcaatacttcgaaataagctgcctttcagcggggagctctggccggccatggagccgatttgaacccaggttaaagtgtgctgcggatcttggcgctgggcaatcatatcggtaatcatagtggccgcaatgtcgccccataaatagtccaaaaccacgtcgacgtcgccaatcttggccaagtcagcttttagttgatcatcgttatcagttaatttgatggttgaggtgacaccaaattggctcaattttgctagtttttctggattgcggccgacaccgattacttcggtcgcaccaaaactaatgctgatggggatagcaagttggcctgaagcgccggttgcgcccagcactaagactcgcttgccgcggatcttgtcttcgcccaagcgttccttgatcgccataaacgacgacattgccgggttagctgtagcggcgacaaccgccggatcagcggtattatcgattgggaacagtgctcgtcggttgacgactgctttttcggccaaagtcccataaacgttattgctgctgttgaagtagacgtgttcaccgtcggccgtttcaccaacggcatctacgccggggacgatcggtagggtgctggctgcggaatagtgagtgccgtttgccctggcgcgggcgagttggctgactgcggccgccaagacgtggacctcaacttcaccatcttcgactttgggatcagggaaatcgccgtactccgggccacgagtaaaatcattaataattgctgctttcatgtgaatgctccttaattgtcatttaaatggaatcattgaatgtgtgctttcaatatggcctttatgatgattgatgacggttggttttgcaacgatattgactttcgaattggcgggggtcgatttggcgcacgttccagctaatcaaaacgcctctcattccactctcaactatatttcaccatggcggccagtatccaaaaagcgcactgtcttgccgacaatctcataaattaataaccaactgcccttgatgaacagagcccgttgaggctttctgctcttaatgacgtgatcatcatacttttcggcaactggctgaccacttaaaatctgctcctctactgttttgaaatcagcctcagtgtatcggttggcgcgaatcatattttgataatgtttcttgaatctggactggtacttgggttgatatttgcgcattaattgactccctctcgaatgatgatagcttttattatagcttttttgactggatctggggacagaaaaaaggcccggcgggggagccggacctttcagttcaatattctgaggggaatatgaatatgataatctggacaacaaatcaatggggggattgatttgctgctcaatgttattggggggtgagtagaaataaatctcgtttatctcttgctcatggttataatatacatgataaatataaaaaaagttggacgaaagtgtgaactttttgtgaattttagcaaacttattttggcggataaaaaaggctgcggcgaaagtttgtgaccttcgcgacagtccattttatacctaatctttttttgagggggagataaggtttaaatcaaattgattttatcatttctgacaaatatgaggtgaagagaagccttaacttctattcgaaataagcatacaggaaaagttaggctaaagtatgaattaattgtgaagattttgtgaactttttcaatcggttggcttttgggtacaaaaaaagataagacacggggatgccttacctcaagttacctatattctaggggaagaatatgaatacaaaagtaataaattaaagggggatttaatttattgccacataaaatgacgtatcactttatgtttatatctacactatatagaatgaatatgaccaaagtttgaaaaaagtgtgaagattttgtgaacttttgcgaatttcaccacaatttgtccgataaatttccaaaagattaaaattgaccgtaagaaaccgcgagatgaggaggattttaaatgagctttatggctaaacggtttatcaagaaatttagggctgaaaactacaagaaaagcgtcgcccacagcttcttgaagcctaatcagaagatcaatatttttcgtcaaagtgctgatcagtacaaaattcgtccggtcaaaaatggccagttggtcacaattcaaccaattcaaaaccccaccagccagattctctatttccatggtggggcatttacagtgccgatgaatgaagaccagctggaaatgattaccaagattgccacagaatcaaatagtctgatccaagtggctgattttccactgttgcctaaacacagtgcagacgaaatcctacaatttgcccaggcggcatttgacttggtgattgaatcggaactgccgacattcattgttgccgattcggctggagcgaagatcgctttgcagctgctggtggataatccaggaaaagcagctggcagcagtttcatctcgccgtggttggacaccaagttgaccagcccagcgattgccgagcgggctgatgaggacatcttattggatctaccaacattgcaggagattggccgttggtttgaccaaggggccacgcctgaaaaatgggtcgattatactgatgctgctcaattaaaaggagtcggcccagttcaaatcttctatggtgaaaatgaaatgctggtcccctgcgatcttcagttcattgaggcattacagaatgccgaaggtgccaatccagaagtcattgcctttaaggatgggtaccatgattacaccctttggttcaaattgtccgaaacaaaaaagacctttaaacgaattgctgaattcattaaagatcaacgtggtgcttaagcttggggaaggcatgggtgtcggaccatttcatcattgtgccttggaacagtaaggcaaagatggttccaaaaccaattgcataaagtttcccggtaaataaataggatgccgagatgatgacgaccggtggaatgtagctcaaccactgggataacacggcactgccgtgaatgtatttgaaacggatgatgtaggccaagtcatcgttggggtgcataatcaagttggcccgagcgtacatcgaaactgccatggccacgcagtacaggccgatgatatccaaaatgaggcggacgtagaagtccattgccgggactcctagtgaattaaagatgaatgtgaacagcgctaccaggtaactgaacggcacggtgtaaagcaggttggagaaaaaccggcggcggtcaaaggaccccagtagtaactgattgctcaaagtaacaatgatgccgtagataaacagcgtcgttcccagggggatgttgacccatttggaaaggttaacagcggatccggtccataccgcgcttcccaggtttgaggaaattgccagggcgtttcctgcagagttaataataattgacagccccaggtaataaaggcgctgcttgaagtctttcattttagccattatgtattcaaattctccttcaattgatcatgaattccattgtataatatttaatttggtttgaacatctttactgaaagccccctcggtcaaattgatactgttctttcacaaatcgtgttaatattcacggtagaggaggcggtcttgtggaacgagaatattcggaagtagaagctgagaagcatttcgaaaataatcgtctgtggtttcggcgattccaaacaacccgctcatttcgaaagttaaccaaacccgaaagagcagcagctggatacattactcaggcatttgttggcttagcatataaatatcaattacgaagtccgcgccaatattctgcaaagtcggtcaaagaagttgtcatggatttatttccggaaaaaattgcagcaaccaacgtctttttcacatccgttatcccagtgatgcaccgctactttgtgttcctgggcgtgcagcacaaaattagcaacgcaaaaacgctgatcaaagcgttggaaagcatcaaggtgcgtcagctgttggatggccatcgggatgccagtaactgggatgcccacaagaaactgggcatgcaggtgctgatgggctataagcaggatgtggatcccaagaaggtctcggcgtacgaagaagattataatatgggcgttccactgaggttctgtttcgacttcagcgtcaaccggccgccaaagaatattattttgctgacggagaagttaagaaagaaattcgaaaatgtgatgtatgagaacaacaaataagagcgcgacgagccccgggtgaccccggagcacaagtcaaaaggaccagtgatgaacggttttcgttcatcactggtccttttgacttgtgtagcaggggtcaggggcgtcggagcgtattttgaaagcagaagggagcagtagataaactaagtgctgttactctgtcgcatttaccatatagaaaaagtgctctaggaacgaattttgttcatcattggtccttttgacttgtgtagcaggggtcaggggcgtcgcccacaggactaggcaggctttcagccggccgtcggagcgtattttcaatgctggtaggcgcagatgataaacgagtggattcagttcgtgaatttcggcttaaccaaacaaactcagcttgccgataaacccacatcgttttatcctgaaattaatatcagttttaggagatgaacagaatcaaaaaaatattaatcataaccacatcactcgtcctactggtaggctcgtacttcttatggacaatggtcactttcgatgagcatgctgaaagctacatccaaagagatctcaacaagaatatccgcgaccatcaataccacaagctaaggaaaatgagtaactcggccgcctatgaatggctgagaaaagcaaatcatgtgaaattaacttttgctacggataatcaaggaagtggaaatttatattattatgctgcaaggatcaatcaccaatacaattttttcgtcaccttcaaagtgaaatcatttattccaagtcgattcacgttgactcggatcacctattatcctaactatcatccgcgctgattcaattcatcaaacaaaaaaagccctccgcagccaaccagccgcaaagcgcccacaaaaaatattcttcaaacaacaactaatttaaaacctgaacgtgatcaatgctccccaacttgaccaccgtgacgcctttagcaggacgttcgatgaaagcctgatcgtcattaactgcagcgacacttcctgtcagcgtgccgtcgccggtttgaatgcgcactaattttttattcttataagcattcatcaattcatttgaaatttcttttgtcgcaatagtcaacattgtcacctcttatgataaaattaattatagttcacaattctgctggatgtaaacaatttttctcacaagcataagcttaagaataatttattaacatttttttgcatttagcgctaaagtggatatataggtaagtgaaaggggtattgaaatgactgaacgccaaatgattcaagaaattttaaataccgttgatgttatttatagttttgtcaacaccgacgatgacaagaaggaatacgaaattgtgatcaaccgccaagacggagataatcgtccgcttgagaacgtcaacaaggaaatcaaacattacttcactgatgccaactttagttatgatgaagagctcaatgacaatggcgacgacattcacgtgcaggtaaaacgttaattggtctagttgagtattacttcacaaaaaagtgattgaaccagcaatttgaattgtaatgcacgttatggtatagttcataatgtgcttttttaatataatcaaaaggctataaattgatttgaaaattcgagttaccgaaaaaattttaatggaatatgtaatcgctttctagtgtttggagggaatctaatgttaacagacagaccaaaatatgttttatcaattgatcaaggtacgacttcgactcgagcaatgattttcgatcacagcggtcggaaagttattgaagcttcaaagcccgttaagcaggcaatcccacataatggctgggttgaaacagaccccaatgagatttggacatccgttttgaatgtgatttcttcggcgttcattgatgccggcattcatccagaagatattgagggaatcggcatcgttaaccaacgtgaaaccacccttatttgggacaaggagaccggtgaaccaatttataatgcaattggctggcagtctaagcaaaccgccgctttggcccgaaaattaaagaatgacggctattctggtatgattcacaagaagaccggcttgattattgactcatacttctcagcaaccaaggttcgctggattttggatcacattgatggtgctcaagagcgtgccgaaaaaggtgagttgatgtttggaacggttgatacgtggctggtttggaaactttccggtggcgagtatcacgttacagactactcaaacgccagtcgtaccatgctgtttaacatccacacccttcaatgggatgatgatattttaaaattgctcaacattccaaaggcgatgctgccggaagtaaagacttccagtgaactatatgggacgacgaagaattatcagttctatggcattgaagtgccaattgccgggatcgccggtgaccagtcggccgctttgattgggcagctggcgtttgaaccgggcatgattaaaaatacttatggtgatggtgccttcattatgatgaataccggctccaaaccagagatttcagatgataacctgctgacgacgattgcctataatttcaatggcaaagtcacttacgcccttgaagggtcaatctttgctgccggaacagctttgtcctggctggcagatagcctgcagttaattgacaacgttcccgaatcccgtcaggcggccatgaattccgaagacgatgatgaagtctatgttgtcccggcattcaacgggttaggagccccctactgggaacaagatgttcgtggggcggtctttggcttgactcgcggaacgaccaaggacgactttgtgaaggcaaccttgcagtcgatcgcatacggtaccaaggacatcattcagaccatggaaaaagataccagcatgcacatccctgaactgatggctgacggtggcgcttcacggaacagttacctgatgcagttccaagctgatattttaaatatcccaatccagcgggccgctgacgaaaacaccactgcatttggtgccgccatcttggctggactggcagtcggtttctggaaggatattgatgaaatcaagagcctccaagaacctggccgaactttcacgccgaacatggaagattcacgccgacaaaagctgtatcgcggctggcaggctgctgtgcaggctactcgggggtatcgagttaaaatttagacttacagtttaatagcgtacaaaaatagaccactcagccaaaaaatcactttttgtctgagcggtctatttatattattcatttttatcctttggttctttccaataattagcgttactgagcagttccttggaccgttcatccgcgggaacaaagccaatgttgaacaggtgcttgaagtacatcatgttatagatcagcatccaaacgatgccgagaccatatgagccaagggtgtaggcaacttggaacggttggcccattccaagtgacagcgccattccggcaataatttccactccagccatacacaacaggttataccagtctgatcggaaaattggcacccagaggttgaatagaagggcggtgaatgacggaccaactttggcgatccgaatctgaccgttttctttgttcacgacagtagcaaagttcggtggaatcgggagtccagttggattgttaggatcattttggttattgtcatcattattgccattaccaaatgggttttgcatggggagcctcctttcgaactaatggttacttcttcttgaatttaacaacacattcacaacgggaggtttgcggcatcaaatccactgattgaatatattcaacgttatacttctcagttaattttactaaatcctgcgccaaagtcgatgggttacaggaaatatagacgaatttcttcggcacgatatctaaaatcgtgtcgatcagcgaatccgctaaaccagtccgtgggggatcgacgattaatgcggttggtgtccagccgtcgtcaacccactcgggaagcagttcctcagcttcaccgacttcatataaacagttaaagatgccgttacgcactgaattggcgttggcgtcttgaaccgcttcggcaatcgtatccatcccgcggacttcgcggacctgctttgccaccgaaaggccgatggtgccgacacctgagtaggcatcaaccaatttttcgttgcccttgagatccagtgctttgaaggcctcatcataaagaaccgaggtcatttcaggattggcctggagaaatgcccgggcagacaaatcaaacttcaggccgttaagcacttctgtgatggtttcccggccagccaggtgaatcatttcatcgccccaaatcagtgaggttctgccaggattaacattttgcatgactgaaacgacttccggtaattccgccttgatgcgttccaatagctggtgcttcttgagcagtttcttgctttgagtgataaaggtgacctggacttgatcggttgcgatggcggctcggacaacgaccgttttgatgatcccggcgtttttctcctcatcatatgcggggatgcccagttcatcaatcatcgtcacaattgcccgcatgactttcatcgtcaatgggtactgtaatgctgaggtcttgaggtcaacaacgtcatggctgcgggctttgtacaagccggcaatcgtgttgccgttctcgtcgtggcggatttggaatgtcgccttgttccggtaatgggtcggatcatccataccgatggttggcagcagcttaaagcggcgataaccggtgggctggtatttttccagcgactggcggacaacgtctcgtttgaactccaattgctttgggtaggccaaattttctaactcaaaaccgccaacgtcatttgcgtagtcgtccactggttgaatccggtccttactcttggtcaaaatttcgacgagcttggcgcggataaagttatttaaatcattggtcacttcaacgatgactttttcggttgggagcgcaccgggaacgaaaaccagtttgcgttcgtagtaaccgatgccttcgccgttgattcccattcgtttaatttcaattgttaattgttcaccttcgttaacgtgaaccgtattattatcgttatacattgaaccgtccttaatattcttagttactagtatgatagcacatcacgagggctattcgcatgtgaagcaggcggacgcgaggtgtttcgtcaaagaatttaaggcaatcaatcgattatccttaattgtggacaaaagattgattgccttaaatggctggcggccacagttaccgccgattgggggtaacaaaagtggcgcaccaaatgaattgatctttttctaaaataaattctgaattgaatcaatcgacttaccaggttgcagtatcaggatcggttgccaaacctgcttgaccatggaagccgtcaatggtcttcatatcggtatttgacaagttaaagtcgaagatatcggcattttctttaatgtacttctcgtggattgattttggcagcggcaggaatccatgctgcagtgaccagcggagaaccacctgagccggcgtcttgtcatactttcgaccaattgtggccaattctggaatcttgaaaatttcaccggttccaagaggactgtaagcttcggttaaaatatcgtggtcatcattatattccacgaccgccggctgcatgtccgaagggttgatgaacatttggttcaccattggcttgactttagccgtttccaataacgcatccagatgcttgggccggaagttggaaacgccgattgccttggcagtcccggctgcataaaattcttccatggcccgccaggattcggcgttggcttcctgccagttgtctcgaaaggcaaccgggtttggccaatgaattaagtagagattgacatagtccaatcccaatttctccaaggatcggccaaaggcttccttggtcttctcataaccgtgatcagcattccagagcttggtcgtcacaaataaatcttcccggggaacgccgctatctttgatggcttgaccgacactttcctcgttgccgtaagctgcagctgtgtcaatgtgacgatagccggcgttaagggctgctaaaacggcatggtaagcttcatcgccattggcggattgccaagtaccaaagccgacttggggaatcttgactccgttatataaggtgtacgtatctgttaatgacatattctggcctcctattgtgtctctaacactattttatagaaattaaatatgaagtacaaagaatttatccattgaggagtgctcaccgttattcaggggatgccccaaatcggtaaagccgtattcagtgtacaggtgaattgcttctttcaaagcgtggtgggtttccaggtagaccgtctgatagccggcccccttggcaaacccgaccgctgtgtccaacaatctgtagctgagatggtggccgcgggccgagtcagttaaatacagtttctgaagttccgccacatgattggcatgatcgaactcagcgatgccgttgccacccaggacgttgccggcgtcatcgacagcaacgaagtattcccggtcatccttttggtcatagaagctgctcaaatggtcaagttctttgtcgaaatatgcggtccccggaatgtccagtccgtatgattttaaaattgtccgaataatttttgccagctcgaagtcatcttgttgtttaatcggccgtatttttaccattctatcagctcctgtccttaacgtttgattagcatattaccacttttggaattgcagagtaaagcccatgtgaacgctttatcgtgatatactggaactaatttggaacaagttcgggagggatcactatggatcaaagagttgcgattgtgacgggcgcttcatcaggaatcggcatgcagattgccaagaacctctatcgaaacggtatggaagtctatgcactggctcgcagagtgtatgcaatgaacgagctggatgatttgggtatccacaccatgcatttggatgttaccgaccacgatgaaatcgatcgggtcgtcagtgagattgtggccaaaaccggccggattgatgtcttagtcaataacgccggcatcgggtcgtttggctcggttgaagaagtcaccttgacggaaggcgagtacgaattcaaagtcaacgtctttggtttagtcaaaatgattcaagcggttctgccgattatgcgaaagcagcacagcggccggattatcaacatgtcctcaatggccggcaagattggcaacatgctattaggcagctggtacatcggctccaaatttgcggttgaggggatcagtgattcactgcgacaggaattgaaaccatttggcattgacgtagcaatcatcgagcctggtgcgattcagtccgagtggaaggatggtgccatggatcggatgatggatgcgtccggcagcggcccttatgccaaattggcccggcgatcggcagctttctttgcgatttcctacaagtttgccgctgcaccaagagtggtagccagagctgtcgaccgggcagtcttttccagacgaccgaagaccaggtatgcgattggaacgggcgctaaaccggcaatgttaatgaagcgcttcatgccggacaagtgcctggacgccttctttgaggccttgaataagtacgctcagcaagttgtcaaccgagaaacgggtcaaaacagatagcaattgaccactgaaattaaataaagtaccattaacttagaaacactgggggaactgctatgtagcagctgagaccgacctgaaccaggccgaaaccctttgaacctgtcagctaggactggggtagggaagcagagtgcgatcaggggcggttagtgaccggagtctaagggactttggacggaaatcgagttagattttcggccgaagttccttagatgcaggccactgccccttggagcacgtttccgctagataacagcagaaaccaccaaccaaaaccaatcacccaggagctgcagacaccaagtgtctcagctcctatttttgtcaacaagcaaaacaacaaaggagaacaatcaaatgaaaatcgatttattaggcacattacgaaagaagaatcccatcgcttttaacatctccaactttgtgaccgtccaagatgttgccaatggcattaatgcgttgggtgcatcaccaattatgtctgaagaaaagaatgaagctgagccaatggtccaaatggctgattctgtgacggtcaacctgggtgcgtttaccgagggtcagttggaacagatcagtgcggtaacgactttcgctaatcagtacaagaaacccatcatcatcgacccagtggccgtgggtgccgttgactaccgcaaggaacgctgcaatgaattattggatcagattgatgtcgcggtcattcgtggtaacgcgggtgagattgctgcattggcagacgttgagtggaatgccaaggggattgatgccggtgaaggcagcggtgatctggaagaaatcgctaagaaattagccaagaagcgcaattgtgtcgtggttgaaagcggcaagaccgatatcattaccgatggcgaggcagtggtccgaatctacaacgaaacggatttgttcaaactccatgttggttccggggatatgctgtccagtaccatcggctgtttctgtggcgttgagcacgactatttcgaagcagctcagactgccacggcggtctttgatgtggccggagaagtcgttgccaaatcaatgcccaaaccactggccggatcatttggtgttcagttgatcgatgagcttcatttgattgataccaagaccgttgagaagtatgcgaattttgaatgatacagagtgcgacgaggcccggtttgaccccggagtgtaaggtggaaatttaaaggatgaacgggctttgttcatcgtttgaatttttgccttacacagtaggggtcagggccgtcggagcacgtttccacaaagtataatgcatgtgaaaaaatccaagtaatcacaagctcaacaaagaaaggtaggactcaaaataatggttaacgaaacagttcaaactttaacaatcgctggaactgacagtggtggtggtgccggtgtcatggccgacattaaaaccatgcagatgcgccacgttttctcggcggcagtgattgtggccgttacggcgcaaaacacgattggcgtccaggactttatgccgattcccaagaaattgattgatgaacagtttgcctcagtcgccgatgatttgaaaattcgcgcttgtaagacgggaatgttggcggatgtcgccacggttgaagcagtggttgagaatttgaaaaaatatgatttggggactctcacggttgatccggtgatggttgccaaaggtggtgcccgcttgctttcagaagatgcgattaagacggttcgtgagcagttgttgccgctggccgatattttgacacccaatttgcccgaagcggaagaattaaccggcatgaagattgaagataaggatcagatgatcgatgccgccaagaagctgcaggatctgggggttaaaaacgttttgatcaagggcggccaccaaactgaatcaaaagagtcctcagacttcattctccttgagagcggcaaatcattctgggtcagctcaccgcggatcgacacggttcgaactcacggaaccggcgatacgctttcttcctgcattactgcagagattgccaaaggcgccgatgttgaaacggccatccggattggtaagaagtacgttcaagcaaccattgccaatgggattcaagtcggtcatgggcatgggccactaaaccactgggccacatttgaaggggacggtgactaagatgggcatgcaatttgaaccggggatgctgcgagcttactttattgccggcacccaagatgtgaaggataaatctaagacgctgcaagaaattgccaaacaagccatggaggccggcatcaccgcctttcaatatcgtgagaaggggcccggctccttatctggtgccaagcgggacgaaatggcagctgacttgcgggaaatgtgcagtgattatgagatcccatttatcgtcgatgatgacgttgacttggcaatcaagacccatgcggacggcattcatgtcggccaaaaggatgagcgggtcactaaggtcatcgaagcagttggtcagtcgatgtttgtcggcttgtcctgtgatactcaagagcaggttaacatcgccaatcacattgacggtatcagctatcttggcagcggcccagtctttccaaccgggtctaaagccgacgctgatccggtgattggcgtcgatggattggcaaaattggttcaagccagccagctgccggtggtcgcaattggcggcattactgagcaaaacatcgtcgagcttccccaaaccggagtagccggcgtttcggtgatttccatgattgcccaaagtgatgatatctttagaacagttaaagtaatgaacgaaacctttgaaaagtaagggcttcgcaatcagttgaaatagacaattaagcgggtagcgcactcctgggattttccaggattgtgctatccgcttacgtgctgctattgagtgatgctggacaattattccatgttaaagccctcaacggttgcgtggggcaggtggttaacttcgccggtcatggtcttcatgacgtcggtattgttgcgggtgtaatacgagacttgataagggccgggaccacttaccttacccttgtaggtttccagaaccggttgaacaaaaccggccacatctttgctggtgacccgtgccaaattaacgtcgctggtgttgggcgttccaaacgccttccagtcagtcgtcgacgtcgggccaaagacaaagtagctgccggaccgatcataagaagtctggtcagaatgaattttgacactgtgcttaccaaaataaatgttagattggttgccataccaggcaccgcgaaatggttgggccacttcgcttggatttgaagccgaggcatcttctcgatggtgggagacgacacctgaaagcccgatggtgcctacaaaaatcagcgttaagataatcgtgattgtcgattttttcatgataaacgctccccaaatatgcttatctattaccatctaaagggtactccggcaatgtaaattaagtgtaaacattgggtatcaaatatgtacaaaattgatattactcgaagattacctccaagttacaattattaggtttggataaaatccatgcataaaacttgtgattttggcggaaagccgttttaatagaacatgaacacgtttttattttcaaaatatttaattggggtgagattgaatgaaaggacattttaagttagcccttgcggctgcgttcctgttcgtgtccgccggcatttttggtgtcgctgcaccaactgccagcgccgacgtgatcgccaatcctgggactgcgggttcgattccgcaggtcaatgcagggaacgtattgaaagactacgatgagaattcactcaacgtggttaacaactcaacaccgcagggtaacacaagcaagaagtataccaagtattcattggatccaactggttacaactacggcaactcgtacaatacaattgccggcagttcacaaagcaatacatttaagacgaagttcttcttaccagatggcttcaatgtttccaactatcaacatggtaacttccaaagtgtcacacttgatggcgatggcaacatttacttcatcgaatcaaatggtaccaacaccaaccagggggcaattgttaagttcaacatggctaagcttcaacagttaggcgttggatcggatgttttactgttgtggcgggcatttgattacttcaacccgtacacgacagacggtcaagctcataatgatgagtacaaccaagtcaacgcacaattacaaggtgcatttgacaaggttcagactttgacgacgactttgaaccagaataagtcctggcagaacaaccagaacaactggaagaagaacgctcaaaagtggtattactactggaagaacaagaaagccaagtataccaagatttccaagtcatataagtattcttacaatacccgggccaaggccaagaagactgtgaagacagctacttcaaagatggccacttggatgaaatcttatcagtcacacaaggctaagattgccaagtacaataccaagatcaatagtattcaatctcaaatcgatacttatcaaggacaaattgacgacgccaaggcgcagaaccctgacatgttcaaatacgttgatattgcccaaacagcgcagttgtctccagaagttgatattggccatggtcaaacattgtcatacaacccacaaaacaagcacatttatttagctgaagataacacgttgactgatttggcatcacgggatgataacaacacggttcttgaaatggatccggataccttgaaaccaatccgtgagtacaactttaagatgtatcatggtgactccgctaacctgcagctccacacattggcatttgacagtaaaggaaatgcttattggggccgtaagttgaacggtggttacatgttcttctacggacgtcttgatgaaaatggtgtcagcttccaggcttcatcatcaatggtcggcaagcgtggcggttccacgaaccaaggagttgccgttaaccctgccaataaccgcttgtacttcgtttctgatgatatcttgacttcagtgccaacatcaggcgttcaaagcggaaacttctcggcagacgatatccactatcaagccttcgattccggtcgtgagtttgaaagcctagcgtttgaccaagacggttacggatacttgctggcattgtggccacctgagttgatgcaatcgactaatccattgaattaatttaaatagatgagagcaggaatttcctgtttgatgcttttgagtagcagtcgcgagtttgcggctgctattttttgttgggacaaaatcgtcatctcaaaggttacattaccactcagtaggtctaatttgtcaaaacaattaaataggccgccaatcaaaaaaagtcacgagccgaaaagttcgtgactttttattactctgcgtatgcctgagccaaaccggcaatgtctgccgaagtgatgtcgttgtcggcaaccgtgggatacatgatgctgtccatatcctcagaatgctgcaatcccaatgcatgcccgagttcgtgctcgccgacgtggactctttctgtcgtcgtgtatgtgaatagactgcagttattggcgtaaatcgttgaggtggacggcgccaataagaacaaattgttcttctgtttctgataatacttgacggtcgtcatcccagcgtagtccaaattatccgtattatcaacggctagcatgatgtcaggatcctggcttgctgcaattaaatgaacaatgttggtatcgttccacttgttaatagcctgttgccaaacgttttgataatacgctgacccagtatcaatcttatatgtaatggtcgtgtccgcccaccgatatttggcaggtgtggtgttggaatcgttggtagccatgacggaaccttgggccgatgattctgtctgctgggttgtcgttttaacacgtttgacgtattcaatggccgtgttgatctgcggggtgtcatcggtggtttcggccacaactggatgggaaagaccaaaggttaaagtgacggtgaacatagtgagcagtaggatgatcgttcttttcatgagcatttctccggattaaaatttgtaacctgatatatcaaaacagttactttaatatagcattatagcatcatattattaaaacacaatactgctataacgataaagtgataatcaaacaggtcatttatcaatcaccttctcaatcaatgatgcctcaaagtgccagcatacaccacgactaatgcggcatccaaaaaagggctgcggcacaattttcattctgtcgcagcctgatgactcgctattcaatttggtaatcagaagaaataccagtcagccagataaaggcccaagacactggtcaacgcgaacacaaccaccagcgtccagacgatattacttgccaggttatgatgactcttgcgggcaaagccgatttccaataatgcgatgacggccaggcccaagatgaccttcagactgcccagcaccggatctcgtggtacccgataaagggccagcatgaagccggaaaccaggatcggaatgtacagcacgcgggtaatcatcatgaaaatcattgaaagcttatctttcagaacaaatgccaaaattgcggtaatcattaataggatccatgaaatgagatggatattcatataaagcaaaatgtaacctcctcagttgtgtttctattttagtatagtattttgccgacaaaaagaaaaagtaatttcttgattaggttctgcaaataggctattttttaggtagttgaaacaatcgaaacgagggggttgtcatcatggacgggctgaattatacccaggaatttgtgctgtgcgtgctgaatcaaaagccaaaattgagtgcattcaaggaccgtaaagtcgctgcgtgtttgttattatcagaaattgtcgaactgttgcgtgctggggcgatggaattgacgcctgtcaatcgaatggtggttgcccaagtgactaaggcaccggcggattatttagtgccgctcactgaagacatcaagaaacggcagccggagtcagtcaacaattatgttcgcgacgcggttctgtcggtccggaaacgccgggtcaccaagattgccgaagcgatttgtgactcattggttaaagcaggctatctggaagttgaccacaagacctattacgataatcaaacactgacggatcgcatcttaacgcaactgtatcaagatgcgatcgctaaaaaagaaccgtcggagaagaattccatgttggcaattttgctcgtcaattcgggtttggtgcaccaaatttttcccaagcaggaagccgaaaccatcgaactgcggcttaaagaagtcatgaagtccgatcagtatcatttgatttcagatgtgaccaaacggatcaataaagatctggctgggattattgacgcggtctcatttgccaggtgagatcaatcaaaaacactgcatcatataacctaaaaagtcgagataaagttttctttatcccggctttttcgtgtttattatttatgtgaatattgcgcctgcagtgcattaagcgctgtgacgtagttcatcgttggcaagttgccggccttgaaatctgctagtttgtcgtcatcaattgccatcactttgaaagcatccgcctcagaaaccccggcactttcccttacttcattgattcgcttcagtaactcagccggtgtgaggctcaacaggtaaagacgtttgatctgcgtcaaagtctgctggtaagcactttccggtgcggttccagcgtagtaggccttgatttcgtccgggtcgaattcgacgatattgaaaagataatcgtctgccaagtgtagttttgcttgatatgatttgatttcagccaacatttcgttaattgtcatgattcaactccattgcgttattttcaatctttcctatctatgatatgacaaatcaacgcagaattctaatcgaattaatatttggcagccaagttagcgtattcctgtggggttaaggccatgatcgaaccgtgacgcttcttgagttggccgaagtcatagtctggcgcgacctcccagtcggtgggattgctgctggtcagatcagacgtcaaaatcggcaggtagccgcggccattgtgaaattggtcgacgtagatgcaccatttctgctgatcagccagccaaacaatttccgggccttctaccgtatcgccttgaatgcccaagtccaaatcttggagagcagtgacatgctgccaattgccattgagtgaaggtgactgttcaattggaattgttccgtcacgggatgcacggacgaattggccgccagctttgaccatggtcatgtcgatcaaatcattttttggattcttggcaacggcgtaagttgcggttgattcgaagtgctggaagtctttagtgtatgcccgccagatttccattttgtgggtttgctggttgggggatgaccaaaagacaaagtaggcttcatgagccggatcataaattgcttccggtgcccaaacacagccggtattctcgccgaccatttgaatggcgcggggagctgaccagtttactaaatcagccgaatcccagaaaatcaaatccttggacccggtggtagtggctttggcctgaccccagccgccgcgatgataaatggacaggtcggtggccatgatggtaaagtggccgtcttgccggcgcatgatgaagggatccctgacgccgcgctcaccaatcgtcgatgttagaaccggctggccgtgattgatgtcagtccagtgaagaccgtctggacttaaggcaaagtaaagttgttcagcggatgggctgtcttctgttccagtaaaaaatacgaagaggtagccgccgttggtggattgattgttcaatgtcaaatgctcctttttagcttgttttagtaaaaactcgttgtgaataatatagcgcttacaggtggggatgtaaatgctgttttgttgtgtgaggttgatgcctatggtaaaattattgttaccatagagtaacggatggaattttgaaaatgcaatttaacagagaatatgcaaaattggcaatcaatcagattgaaagtgcatatcgtaaaggtgatattttaaggcgccctggacgacatggatacggacctcattctgagaagacagaagcttacttgcgagaccacggaattacctttcaaaaggcactaaaagatgctgttcaggctctgagtacctcgaagttaacaagatttcgtggcccatctcccagttattttccgggacaatcaggtggggttgtgtatgactttttggggccgctttatgattctaatatgtacatcaagttttcactcgtcgtccgcaatgatcaacaattcataattttcgaatcatttcatgagtctgatagaaacgactttggaaattttattgagttgaatgtatgacaggggaggcaactaatatgaatcctgtaaaagtaaattcagtcattactgaatatgatccgatttctgaccaaaagatcaaatatcagaaaattcaaatttctgaatccgtgactgtgagaaatatatctttcaatagtccacactactaccttgtcgaagaagggatggacattcatgatcctcagaactttgaagtcccatttgacaatcctgatgtgaatttgcgggctgattatcaggtctatcgtgaaaaagctggtttcctgcaaccaaaagagattaaaaaaatcagagaacatctgagattgagtttacgtgaagtgtcagccattttaggaataagttatagtacattatctgaaattgagaatggattagtattacattctcaaattcaagatacactgttacgaatgcttgaacacacctacactttgtcgacgattgtcgaacagcataaaggcttgattattaacagtcatgggctgaaagcgtaccagcgaattattgacaagttaaatgctgagaaaaattgggattcatgaagattcgatgtggctttatttttgcttaactgatgtaaatcatttcccggatatgatacgatgaaagcgtagtacattcgaataaatataaggtggtaaataaattggcagaaaatgataattggcagttaatgggtgttcgtttggatggtttgagctttgacaggagtaattttaatccgcaaaagggcccgcagatcaatgctgaaacccgtttggcattgcctaacgacccggcagacaaatcaacaatgagtgtcgttcaagttgtctcgactttcaaattgtatgacgatgaactggcaaaaagctatttcacggcaaccattgccggtgtgtaccaggtgccgggcagcttgacggataacgatgctattcaaaagacaattgacgatgacaaaaacttgcgagacagcttcgctcaaccggttgtcgattacttaatcgcaaccctggcagacttgagcttaaaggcatttggcacgccaaccattttaaagcgcgagcaattgattgatactttgtttggtgcaaagcagcagtagtaggcgactatctcaatattaaaagacaaatcaacagtcggagcaaaggtgaatactttgcgccgattttttgcactcataattaccactatgaggaatcacactgtattcaaagctagtaaattgcgttagaatgtacaaatatgttaaatgaacgtcacgaattggaggaccacatgagctacttagagctgcataacattaaaaaatcctattacctcgccaaccaggaattcccggttctgactgggatcgacctttcctttaaccaaggggaattcgtctcgatcgtcggagaatccggtggtgggaaaacgacgttgatgaacatcatcggcggcttggacagtaattatgccggcgacgtcgttttgaacggcaaatcgctgcgccacgatactgccaagcaattggatgcctaccggagacaaacgattggctttatttttcaaaactttgatctgatcagtcacttgactgtttttaacaacgtcatggtgtcactgcagatgaccaaactcagccataagcagcaggaggcccgcgcccgtcagctgttggaacaagttggcttgaaagaccacatgaaaaaatatcccaatcagctttccggcggccaaaagcagcgggttgcgattgcccgcgcgttggcatcggatccggaaattatcatcgctgacgagccaaccggtgcgttggacagtcaaaacacccaagagattctggccttgctggaccaaattgccaaagacggcaagctggtgatcaccgtcacccactcggagacggttgccaaccacgggacgcggattgtccgcctagctgatgggaagatcagcgaagacaccaccttaaagccaggttatgagaagtctcaagccaatgagctggcaactcacaccttgagatttggggcaaccttgaagatggccttggaaaacatgcgctataacctcaagcgaaacctgctgattgtctttggcgccgccattggaatctttagtgtgattgtcatgctgggactgggaaatggcgtccagggatacatcaaccatgaaatatactcgcaggtgaaccccaacgccgttcaggtcactaaaaacgtgtcggctgatgccagtaccgatccaagcaagattaacgtgaccaccaaggacaagaatcgattcaaggacattaagaatgtgaagagcatcgacgatggttactttgtccagggtggcactcagctgcgccgtgggcataaaacggcttcaatctcatttatgcagacccataataaaacgatgctgactaagagtattgccaaggggcatgcgccaaagaacggcgagattatgctgaccaaggaatacgccgaaaagcttaataaaaagcatccgtattcgctgatcggtaagcgggtcacattttatcagaacacgcttaataagaagaagcgtccggttatgctgacgaaatcactgaaggtcagcggaattgccaaagcaaataccgggtcgacctcggtcacatacagcacgatgaagtcactttacagctcaaagggtatcaagattcagcctaattttgtgaccatcgaaatcgccggcaacgttaagaacgtcaaaccggtcgagaacaagatcaaggcctacaagaacgacaagaaaaaggccgcttatcaaatcaccggtgtcggcggcttcgttgatacgctgaacacctatatcaccctcgcagttaatgtcttggcaacgattgccggaatctcgctgttggtatccgccatcatgatcattgtggtgctctacatcagcgtctccgagcgaaccaaagaaattgggattctccgagctctgggatcctcaaagggaagtatccggaacctgttcttctcagaagccttcttcattggcttgttctcatcggctttggcgattgcgttggcggaactgctgcaggtagtggccaataacatcgctcagcggggaatcaattattcaatcatgcaaatcaccccgggaaatgtcatcttcggttttgtcgttgccattgtcatttccttgctggcagcactagccccagcggcctcggctgctcgattggatccaattgagagtttgagttacgaataatagtttgaatgacaatttttaagtcctcctgcgaacaaacgggagggcttttttcgtatatcatgaatgtgctgatcgaaccatcctcatgttataattatgttataacatcagttgggaggagatcgaatggctaaagttaaggttcgaaaaattggcaactcactcggggttcttctacctaaggaaagcggtgtccacgagggcgatgagttggagtatgctcaagagggggacaagatcattttagacacacaagaagcgcaaaacgcgagagttagagagattgttgaaaatagcttcaaagattttgaaacaggaaatgttttgactgaagatgatatggtccggatctttggcaagtacggttggcataaataatggatccatatgaattgtcgttctcaaacgattttcaaataagcctaaaacagacaattgccacttgggagagcattggaattgatgccagcaagattcagacctttgtatcagacattaataccgcggtggcttcactcaaggtatttccaaatcgttttgccaacgttgatgaaaaatatcgcattccagtaccgactaggcaaattattatcggcgaccattacgcgatcttgtaccgagtaaaggaagcgacacacacagttgagattgggccaatttataatttgaaacaaatgggtattactttttagattctcctgagagatcagcactttaagaggcgtggaaataactgattgtcagtcatttctgcgcctttttgagttccactgccttctagcctaaacgtgcagcaatcggctgatcccggtcatgtaaacgccttgtgctgcactctggtattgacaacccacgcatgtagtatacaatactacatgaatagtattgaaaactacgtaaatatcaaaggagattcaaaatgtccgaaaagattgccattctcgctgattccggttccgatgtgccggcagaattgctgaaacaatatgataatattgaagttgccccaatgctggtgaccatggccggcgaggaataccgcgacaatgtcgatattacccccgaagaattttatgcccgcctcggccaagccgatcagtttcccaagaccgctgcaccaactcaagggagtgtggaagcgcacgttgccagcttgaaggaacgcggtttcaatcgaattatcggcatcaccgtttcggcacatctctcaacgacatttggcattttcaccaatgtggctagggaaaacaccgatatcaagatggacgtgatcaataccagaaatattgggattggcagtggcttgttcgcggtctacgctgaagaaatgattgacagcggtcagacgtttgacgaaaccatcaagtttctcaagcagtcggttgaggacagccggacatttttctatattcccagcttgaaatatttgcgggcaggtgggcgtatcggtcgagttgccgggttgatcggttcggtgctcaacattaagccggtgatcgcgaccgactctgaagggatctatttcccggttgccaaagcccgttccgagcagaaagccatctcgaaaatggtccagttggtctctgatataattgccagccacaagagtgtccgggtcggcgtcgctaatggtgccgatgtacccttgcaggaaaaagtctatgaccgcttgcactcggccttcccacaacttagaatatatcgaggaagcgtttcgcctgcgttaggggttcacaccggtcctggattggttggggttggcgtgcaggtaggcgaaggcgaataacgaaggaggggttcgatgccaaaaacgaccaccgagcttcagattagactgccaatgtgggaagaattgccggcattttcgctgcacttggaccagctgctggatttaactaacgagtatctggaaccaatcatcggcgataaaattaccaagacgatgctccacaactatttcaaagctaaaattctcgtgccgccggtcaaaaagaagtatcagcgtacccagctggccggtgcaattgtggtggggctgctgaagaatatttttacgttaaatgaggtgaaggccggcttgatcacactcttgggaaatggcacgcccaagaccggctacaataattttgtagttatgtttaacgagcaggctgccaaggccggcaaggaattgtcggatcccaccagcttggaattggcttcagccggccagccaactttgatgcagtatgatgccgtccagtcgattttgttttggctgtcggcgaagaatcgattacatgaaatgatggatcagcaagaccgtgatggcgcttaggcgtttgtcacggttttttattatagcgacatctactcataatgagttagtcaataactttattacaaatgtgtggaaatcgagtttgccgtgaactaagatagtcgtgtatgaattgaattcgttttcaattattattgaatgtttttggaggggtaaatttgaatagtaatcataaaatgttattgagggaattctctattggggcagcagttctggcagcagttgcattaagtacacccaccttgacgaccaaggcaagtattccaaataatcaaaacatgtcaacgttaaactcaagtacctcagctcaatctggtcattacaccgaagataattccgaggacaattatcaatttgactggtctctcagtgatgatggaacattgacgttatctaatgcaagttttgtatttggcggtaacaattcgccgattaattcccacatctctaatcaattacctgccgatgtggtgagtgccgtcaagaagattgttctgactggtagccccgttgcaagtgggaatatccaatacttgttttgtaactttgccaatgttgacaatattgatgttcacaatttgaatgtttctggtgtaaccagcatgcaggccttgttctgtgaaaatcaaaagctcgattcggtgaacatctcatcatgggataccagcaatgtttcaaacatggctacgatgttctgggaagaccctatcacgaccattactggtttgaatgatttgaaaactggtcaggttaccgatatgcatgaactttttgcgacaagtaactctgcagacaactcgaaggtgactcagctggcccaaagttttattaacactgcagatgtacacaatgtaaaaaactttgaaggattattcgataacagcaacatgaccaacctggacatcagttcgtggcacatggacgctgccactgacacctcaaacatgtttggagattaccaaattgccgttccaagcccattggcaagttacaccggctctaaaatgaccactttaactttgggacccgatgacaagtttgtaccggtttctgagccaactgctgttgtagcaccgacctttaacccctttggatccacacaaacatacgttccaattaacttgccttcaggaacaaccatcaacatgcctgtcgataaatcaggtaactggcaggccgtcggtagcggaacagtaacgaatccacaaggtgccacttggacaagtgctgattttgacaccaaatacgctccaaccgccacaccgcgccccgccaaggaaacctatgtctggaagcacacggcaccaaagctcaacatcaatttgaaatcgccagttactttgaaacagggcgccaaatttgatgctgacagctactttgtttccctgactgatgctggtgaaaatgccattagtgccccgattaccagtcttaaagacgctgaagcattggggatgaccatttctggcgctgacaaagtcaacactaaggttccgggaacttacaacgtcactttcaagttaggcagtcaatccgcaactttaaaggttacaattcccggttcttcaagcaacggtggcaattccagcaacagtagctcatcaactaccccaaccaacaccaccccaagcaccaacaactcatggaacccaacgacaccatcccaagccaccggcaacacgggcttaccgaactacgcggccgtaaaaggtgacgccgtttacgccaccaaagccatctacatgtacagctcaccgaccttcaccaagcacaaccgaattgccaaatacaccaagaaggcccgggccaaccggccgatgtttgttgtgaccggctatgacaagtccaacaacggtgctttgcgctacaaggttcgcgatgttaataagggatcgaagacttatggtaagaccggctacgttactgccaataacaactatgtcggcggcgcttattatcagactatgcccaagaacaagaagcttaccgtgattgctaagcacgggatcaattcctatcgctcagccagcttgaccggcaaatccaaacactacaagaagggtgctcgactgcacgttaagaagcttgtgaagcataatttgaccacccgttatcagttaaccaatggtcattatgtcacaggcaataaaaagtttgtcattcaaggaaattactaatatctgaacgcaaaaggacttgaagccaaattggcttcaagtcctttttgtatctgatttatttaattcgcagcaacaccaaaccatgcccggcaatcgtccagagcgccggcatgtgctgaacggccctgggaaattgatcccagtggcctgctggactcttcaatttgtcagttagtgcctgatcagctggtgttaaccgcaggtgccttttgtccacattgtcgattgtgtagagcatgtacaagtcaaattcgtttttggggatgttggtctcgccggtcatcggatcatactggtaggttcccggttccacttctacgtcaaattgcggggtggcgccctcatacaagcggggttcttcgggcgcgtggggcttcatggggtcctggtcgccgctaatcaggctgaaacaaattaacgccagtccaaaacagccaattgcgatgacaaataatagtccatatgtttgcatgcccattcccccaagtgttcattagtccttaattatagaacaattcgttggtaaatagctaactgactttgacaaactggtttggcaaggtcaagtccgccatttgaatgtgcataaaataataccgatccgagcccattcccctagggtaataaaaccgaggtgaatcatgcctaaacccaacagccagttgaattagagaccattatccatcgcttttgcctgtaggactgatataatataatcggcattaaagaaataacatattcgttgggctatggaggggattcatatgaataacttaaaaattatgggcgcacttgcaggagcatttgccattggtacaatgatccttacaactcaagccgacgcagctaagaaggttaaagtgacgtcaaacgtgcctattacggcaaccaaagtcaccaataggaacgttgcaattaccggcaagaacaagatctataacaaagccggcgtcttgaaacacgccaaggcggtaacatccaccaaacagattaagcaactcggcaattctcagcggtcaaaagacttcttcaatgtctaccgcatggcaacgaccaacaaaggccaagtttactacaaagtcgtctcctttgaaggcaaatggcggggctggatctacgggggaaagaccaaggccgactatcaaggtgggatccgcagcgttcagaccaccaaagacgtccagttaccagatgatgttaaaaacgctaaatttaccctggaaaatccaggcgtttcggggacaaacaactcctggacggcgattccgtggtctcagtacggtgctcgcttaaagacgacagactccagcccatacgctaatgatgaattgcgggtgacggccgccaaacagctcaccagacaatactacggcactttctactatgtggttgatgacactcatcctgagttcagtggttggctgaacagcagcagcctgaaagccgtcgcaaccccaccaaccaataccaccaccgtcaccaattatgtgcaatcgccgcctgaagtcgtgaccaacacggtgacaaatacggtcacgaaaaccgtcgaagtcccagccaaaaatccattgacaattaattacaatgtttatgagttgggaacctcccagaatcaagccgtttcaaatcaaattttgaagatgtatcaagaccagtacgccagccccttgagtgaattgaccaagaatcccgataccgcggcctctaagctcaaggatcttggtgacgggcagacgttgaaatctaatgacccaactccgatgaactatgcctcaattgcagttagttttgataaagacaagaatgtgatcacgatcactttgaattgggttcaaccaataatagttgccagtgatgctctgtttcatgctggggacgattatgatccagaaagttacctctggtctgtgactgatggaaccggtgtgagctatccgagaggggattggttggatcgagttcaaatatctactgacgtaaataataatcttcatggaacgttccacaccacatatactttcaaactgatggacggcatgaccgccacgacaacggcgactgtcactgttatgaagtgacctgtcatcttcctgaccaggggtattaaattcccggttgtattccaccctgaacccgttataatcaaaactgtaacacaatataatacgtggtctggggtgccccaacggctgagatgatacccatggaacctgatacagttaggactgtcgcaggaagaccgatccaaaatgtttttaataacgcaaatgaggatcatcaaacacgcaaagaccaggggcaatttagctgccgctggtctttttttgccggtccccgccacgacaggaggaaataccatgtcattatcccaagatatcttgtttgaagctcaaccctatttgattgccaacgagaaacacccatttgttcaaggaatcatcaaaggggagttgtcaccggaacagctccgttactacgacaagcaggacatcgcctttgagtataacgaagttgcggtcatcaatgcgctgataaacaacagtacgaccaccgaccaggcactgctgtttcacaaacggcaggacatgcagctgcatatgctggacgattggctcaaacgggaaccggagtcgatgccccacgactgggaatcactgaagcaaacgaccattcagccgattaaccaactctatcgccagcacatggcaagcaccattcagacccacagcgtcctacagattttgccgtcgtttgcggccggggagtggatgtacgttgaattggggaaatttgttgcgactcagaccagagttaaagaagaacccttccaaagttttctttcaatgagtggggatgattttctggggcctaaaggctatatccagcaattctttgatatcatcgatcacgaagccgagtcagcgaccccacgtgagcaggagcaagctaagcagacatttttgaagagctgcctgttggagtggtatttctgggatgcggcttataagctgattacttgggatgactggaagaaaaatgcattaggtggtaaaggcggagtgacgttgtaatgaagcagataaattgcttgacgatatgtgtgaatcgaatataattattgtaagacgcaggtattacacaatcaaaagaggtgatttcattggcagtggatatgaagaataagacaatttctacccgagtcaacgaaaaaatagcagaaaaggcaaaacaaaatttagccaatgtcggaattacagtctcggaatatcttcgattggcattgatctcagccgcagaagatggtgtgagcgatctattgaactccccagaagcaatgcaagcgaagtttgaagctgaacacggtcagaccctcaacattggaagtgttgaagattacaaacggtggtcggaaaaattgtgactcaacttcaaattaaggcaactggacaatatgtacgaagtttaaaacgattgaaaaagaagcattatcctgttgagttgattgaggactgtctccgtgcaattcttaataaagatcacgatactttgatcaaaattcacgatcatccattggttgggcaatggcgtgggtatcgtgagtttcatcctgcacgcattggaaaggcgagtagtcaacttgataagtgggtcgtggtttatcaaatcgatagcgatgaattagtgcttatcttgattgaaacgggcaatcataatgtgctgaaatgattcttcgcaaaacctttaaaacataaaaatgagctgtatctcctaatggtaattggaggtacagctcatttttagctggtcttggtgctattaagttggctcggaatgcataaggccgaaaaggtatttgactaatgctcaaagtctaaccaatttactacgcacgctatccgttcacatgcccagcgaaactcggcataaacgcactactgatcgtctcaacatcgacattctgtcctggttgcggtgcggcgacgaattggttattgccgatatagatggcaacatgatgcgtggcaccttcatcaccccagaataacaggtcgcccggttgtgcttcagagacagcttccttggtaacgtggctttcctgagtcaccgtgtagtggccgaggctgatgccggctgctttttggtagacatagtcggtcaaaccggagcagtccatgccttggagcgattcgccgccccagacataggggatgttttgggttgccagctgcttggccaggctaaccacggcgtcggctcttgaatcgttgctgttgaccgttgccttgggtgtgccggcatttggattgtaatagttggtgctggcttgttggttgtaagttgcattggtgttgttgtaagtatccgcgctggcggttgtcgcaacgccgcccatgatggcaccggctaccgcaaagctcagaatgaatttcgtgaatttcaatgaagacacctcgttattagatttggtagggtcatcataagcccgcaacttttcaggaaggttacaggaattttgtgatctattgacgaaagatgtcaggctgaaatagtgttaaagatttggtagcgaaaggttaaagaattttctgggagcgttgactttgttggttgagatccgctgggaatcattaaaataaccaggttgggttataaaatatactcaaatctttatactttttactaaaattggtgaataccaccccaaaagtattgattatcagtaagaaaacgcttacactataaaataaatttaactggttactatacttttaacaaagagggaaatgtcatggaaaaaagtaggttcaaagtactcgcagaaacgggcatcatgtcacggccggcaacccggttggtcatggctgcccaggaatatacatcagacgtcacgttaacgtacaacgaccgcacggtgaatctcaagtcaatcatgggtgtcatgtcactgggaattccccaggacagctacattgaaattgaaattaatggcgatgatgaaaaagaagcgatggcaggcatcgaggactacctccaaaaagaagggatcgtcgaaaaggtcacgatggacgcggacgcataacgtcgattagaatccagcacttccaatccagtggtcggacaatccagtttgtcgaccactttttatgtggcttcaaagactaaattccagtaatcaccgcactggattggtataataaatgcatactatattaaaagaaaagagtgattcatttgaggggaaagcaaattgtgatcacagcgttaagcagcctgctggtactgggtaccgggttggcaatcagcgccgatcaagccaaagctgccgagaagaaatcggttgtcaacgtgacctttaagcccagcgatgagaacgagctgaccgactacgtctacaacacggttgatccaaccagcagccagtatcaccaatatttgacaccgagtgccttcgcagacaaattcggccagtcagacagttacatacaagcatttcaagattatttagccaaatatcacgtccaggcccaggcgtttcctggcaacctgtcgatgaaattgaccgggacttcgaccaacctgcagaaggctttcaaggccaagtacgtcccagccaagaagaaggggtatcatccaaccacgtcgtacaaattaccgggacagttgtctgataaagtcgtggctgtgattggcctgtattcgacgaacccaaataagaagactaagaagacgaccaagaccgcaaccaaggccaagaagaccactaagaagtctgccacccacagtgacacgaccactttatcgacgaccgacgctaagccgaacatcaagtacaccggcaatgccttctcgaagaagtacggtgctgccaaatttgccaaggcttaccaagtcgatgatttgtacgatcaaggtcttgaagggtccggtcagcgcatcggaattatcaatgatagtgatgtgcgggatgctgacatgctgacctactggaagcaagccggcgttaacgacgacatcagccgggttcaccacatttacaccgtggcgacccaggctcaggcccaagctgatttgaataagtccatcagtgccgctcagatggaagccactttggatgctcaatctgcttcagccattgccccagaggcccagatcgacctttacacggctgttcagtacggcaccaagacgactttgacatcagccttttacaacaacttcatgaccgcggtttcagacaataacgacaagcagattaccaccagtatggcgccggcctttgaaaccaaatccaactggcctgacccaagtgcttcgctgagtcaatatagtcacgcatttaatctcctgctggaacaggcggccgttcaagggattaccgtgtttaaagccagcggtgaccgtggcccatatgccctttcaggtgccaaagagaaccacatcatgtccacttcaccatacgaggttgaagtcggcggaaccactttgccatatcaaaagattatcgatggcaatctgatctccgtgaacaaggaacgggcttggggcgacacttactccagacctgcttatgataccaaatacagcagctttgccggtggtggcggtggcttctcagacatcaacccaactccgagatatcaaatcggtgttccaggtgtcaacacctttagagccatgaactatctgacattcaagaatggtaaatactcgatcaccaagaatcctcacgtcatcacaggtaccaagaccggccggaacttacctgacgttgccggtaacgctgatccattgactggttatgcctcaattgtttccggaccaaagtacactttcaaccctgagactaagaaggctactaaggccaacggtattctgtggcggatcgatggtggaaccagcttcaccgcaccacaaatggccgctgcgaatgcggttatgaatagtggccgccagacgccaatcggtttctggaacccacagatttacaagtacgcccaagagtccgacagtccatttaacgtccttgacgacgcggacttcaacgacaacttgtactacaccggccaaccaggcaagctgtataaccaggcaaccgggcttgggacaatcaacttcgacaagctgtacaacaagttcaacaataccaacaattaggcggtggcttgtcgcaatcacttgattgacctatgatgaaggtgattgattcaatattttatgaatgcgggatgtgagatacatgcaaaatgaagatcacagtaaaattgatcgcaaacaattagcagaaatcgtgccggatctaaccaacgttatcagtgaccctgacggcaccttctcagtctttgactggggccacggggaaatcattggggttatccagcaccaccaggattatcctgacacggcacttgaagaagtcttaaccggcgctgtgccatctggtcttggttattcctacgacccggtagacgagacccacttccaagttgacggcaaggaccgccgattggagaagggcatcattgcctcgagaaacgccgctgtcctggtggcgccggatgtgccggaaggaattctcgattacttgggcattgacatgattaatactctccagataccaggcgttcattatgagtatccagatatcttggattaagcgaaattaaaaagtctagcgtcaccttcgattgaattcgaatggtggcgctagatttttttgattgatgactcagaaatcagtgggagatgttattcaatcatcgtcggcaccttccccatggcggccaacaccttcaccaaatcagcataggacatcaaaatcgtcgcggtattgacattcggatgagcagagatttccggcatcgtctgcagtgacttgttaatcagcaccttcacctggtcgtccgtatcgtgcaccaacgccagtggggtgaccatcccggaaacgacgccgagcagggattccaattctttctcgctggcgaatttcagtcggctgtggcccaaccccagttgctcagccaacgacttaaagtcgacccggtgattatcgaccagatacaaatagaactgatcgctctttcgatccttcagcagcagattcttcacctcaggcaggcctttgggcgcattgggatcatccatcgtccaaatggcagggtggtccacccgccgatagtgcacgccaacccgtgccagcaaatccaacgcttcttgttccgtcgccattttcatccaatcacctcgttgaatacatattatacgcaaaagttgctataagtttgccttttagcaaaaagtcaccagcgccaaacatagccaaattccacaaacccaggattaccaggcgctaagatgccaaaatctcccgcgttgttccgtcaccaccttccatctatactcattgcttgtgacattggccaatggatcaccaatctaatcaaaggtggattcataatgaaacgtaacaacaagcaaatcgaactgtaccaagatgcatttgacttcctattagacggcgaccatgagctggtggtctatggggtgctgaagaagctgcatattcgccgggataatccatattatgaggatctggttcaagaggggatgatggccttcgtcgagaaatacattcaggcaatcaacctcaaaaaagaaccgggttcctacctgctattcatctatcaaggagtctattggtacattctcgactgtctccgcaaagaaatgcgtcaccgagccggcatcgaagaaccaaccgatgaaaaagatctcatgcttgaactggaagataagaagaaatccgtcggcttctacgatgcgcacatcatttctgatgaattaagaaaccagttatcccaggaagaggcccgctatctaaccttggcctacgactacgggatgaatatcagcgaaatcgccagggaatgccacgcttcacggacgaccgtctacaagtggcgccgcggggttatcaaccaattccaaaaataatctgaacactttggccccttcgtttcgttactattacatgtaagggttggcgccaacgacttacaaattaagcagaatagaggagaaagacaatgcaaaaagattggatgaaatcaaatgttacctatacgttggttaatgaggatcacaagaagggcgttaagcactcttttgcgtatgttactcaaaatgtaaccgcagaaaaagtggccgctttcggcaagatccttgaaagcctgatcgacggtaacatcactgacgcagccgtatcttcaaccgaccacgttgaattaagcgacgcaccaaaagccccggccgcacctcaagcaccacaagcgtaattatcacggactaataggaggaaacacagatgcgtaaattagaattggtattcaagacttcagacgagaagcttaagaccctgtccatcaactatgccaacggggaattaaacggcgacactgttaacaaagcgatgactgaaatcgccaaactcaagatgtttgaccgcgacggcatcgatccatacgccacaccaattgccgctcagtatcgtaagactgagatcgacaagttgttcgacacacgcggagaataattgcataagggtaattagctacagttaccgaccaggccgacaatgggaaactttcccgttgtcggcctttttgtgcatcgtttactaaatgtagaagtcaaggaactcacttacaaaaagttactgacaaacgcctgcatgatgcttaacggcggtacttgtgttacagaattgttgcaactatttcaattaaaagttatcagtacaattatgttgcgatatcagttataagaagctatcattaggactgtagaaagtttaggttagctctgcttgaagcacctcttgttatggggtaaactaagggtacgggttacataaacctagtgaactacaaaatattttattcatattggaggagacgcaataatgaaatctagtttgaagaaatcattatttgtaggcttagctgctttaggcttcgtcgcagttgcaggttcagcaaacgctaacactgcatcagcaaagagttatgctaaggttacatcgaacaaaacattaactactgacgctactactcgtaacgttaatgttaatggaactaacgcactttatactaaggctggtaccttgaaaggtgccaaaaccgttgctaccaagagtactttagctgctcttaaagactctaagcaaggccaaaagaactggcgtgcttatcgtgttgctactactaaccgtggttctgtttactacaaggttgtttcatttgatggtgcttaccgtggctggatctacggtggcaaatcaactggtgcatttggcggtggtgttgcgcaatacaacacaaccactgatccacaagcatcaactgataccagttcatcagtgaactcaagtgcctcaattaacactcaaggccaaacaactggtttgagtgctactcaaaaggctgcaacctataagattgccaaccctggtacttcaaacgatggtactgaagtaacttatacttacccagcatggactcaatacaagaagggccgggtaattaccgactcaacaccttataaggacgctactttcaaggtgaccgatcaaacaactcggacccgtgaaggcgacctttgggttaagatcgaagcaactgacgctgccaacagcaaagctaatggttggattctttacagtggcttgaagcaagctactcctgctacaccagctgagaactttaacgctgatactagtgttaagattgcttaccgtgatgctactactggtaagacattggataagactaatacttggaccactgcttctactggtaccaagcaaggcaatgccgttaacgctttagttaacagtgctggttacaatcttactcaatatcttgtaaatactggtgcaccatcgggttatacctttaagaacctgtttagagtctcttgaggagtaatgccagaaaagccagcaccaccatttgtagactggtattaaggtgacgttcgcagttcttccagaggcgccgacatttatccagccagctgaaggagcgttcaataatccagcgttgcggcatcacggtaaagttatgtaattcattgcgtttagcaacctgaacggttgcttttaaattcgttttaacatcaatggcgaagttggtgccggtataaccaccatcaaccaggacactacgaacattttttaaatgatcggcatgaagagccaacattgcgctggcaccgtcccggtcagaaacattggctcgagtaatatggatggcttgtggaagcccgttaatatcaacggctaaatggcgcttaatcccagagattttcttaccgccatcatagcctttattttgagcagtatcggtatttttaacactctgagcatcgacaataataaatgaggttagcgccgagcgatcctgttgggatcgtagggtaaagacaatttttttaaaacctgttccaacaaagattcttgaaagccaggccctttagctgaccaaattcggtagtaataataaaccgtcgaccattttggaaaatcgtgaggtaattgacgccattgacacccagtttttagtagatacaacagtgcattaaatacttgataaaggtcttgggttcgaggtgcggtgcgtttccgggctgtttccaattcaggccgaatcatttcaaactgggaacgagagatttggttaagataattagtcatcaaagcgggtctcatttcttttttatcaagattgtagcaaattattcgggcctttgtaagactctaaacaggttctaagactactgatggcaaagatgtagctaaggatgcttctaacttaacaattagtcctgttatcactggtgccaagtttggtgatactttgactgttgatgttacaccaacggctgctcaaactaaagttgctctctactacgaaacaacttcaggatctgctatttcacctttgactgcaaatgactttgcatatggttatccagcaatgactgccgatcagcaagcaaaggcacttccagacactaagactaacccagctacattcaatgtttcaaactacttcgatgattatgatttaggtggtaacaataacgcccaatttatcaatcaattcagatctgcaacaaatgcttataccgcagctcctggccaattgactgatccaaccaccggtagaacaactggtttatcaaagactggattctttggccaaccattgaataatggtactcaacgttacttctatgtatttgatggtgctgctaccaaagctaacaacgctgatcaacaaactaagggagcaaccgttaaagtcgttatgcaacgatttgtaaccactcttcaattaccagctcaacaaagtaatgccaacgctaacaccgactacattgctaagtaatcagtattagtagtttcacttgattcatagttttacccattccagctctacaaacttaatatgtaatgtcgaccaaagtgatttggccgtccgctttatggaatcaccgttccgtcaatatgatttgtagttgcacacaggtaacgaataaattgctgggcggaagagatacttcaagcatatttcttccaggcaatttgaaaataaaccagcgatccgatttacttcgggtcgctggttttttgtctgaatacagttaagggttcatttgattgattctgtgttcgatttggaattttccaataaattggtggagttcttttaattcgttacttttctccaagggttagtcggtatggaaaaacggattgggattggccgttggacccaaaaactcgtaatctgtatatagataaggaacgttattattcatattgtgctcgatgccggcgttgtagactttccagcgcagttcgtcgatttccttcattattttgtcgtaatctctcaatgacaaaagaaccccgagcatttggtcgtgtttgataacaaacacaccggtttgattccactttgcccgttggaaagctttagttggtgactttttcaattcggaaacagatatgagtggcgtatttaaaactgtcattgtatccctcctcgtatttgttcttatgatatcaattttccccaagagatactagtttggtggctctcgatcaatggacaagaagatgctttcatgggctgaatacaaaaaatgcctgaaacataaattaacagtcatgtttcgggcatttttcgtagttttagtaatcagcagccgttttagtagaagtcgttttcttcgtagcggttgtcttactggtggtcgttgtcttcttagtagaagtggtcttcttaatctgatcctttgggaaattatcaatcataaagttggcgatgtctctggccatcagttgataagtcttggcagccggatgcaagcggccgtcgttaaagcggtcgatgtggttggcgtcggtgatcaaattaggatcgacgtcctgccagttgaggtatggcacgtcattttgctgatagacttcagcttcggcactcctcaactcgttcatggtgtagccgccttggccgacaacgtcatcagagttctggttgttgtcgtaacgggtgattggcaaaatgccatagatgatcaggctcttattttccgctttcatctttttaatattggtatccaaagtgttcttgatttggtcaatggtcgaatcggtatgaccgtaatcattggtcccataagcgatggtggccacgttgtatttggcaaaattggtatcttcaaccgtggtggttaagtcccccggtgtcgacatgtcgccagcgtcacacaagaaggcaccgttataggcggcgttatcaactttcacattcaggtaacgggccagccaggtcgggtagccggcatccaaggtctcgtagccgtcataaccggcggtaatggagtcgcccatggtgatgagcttgtctgatttgaagtagtcactatttttcattgcgatgtcaaacgttccttccgaaatatcttgtaagttgccgcgccagacccagccgttttgtttgccggaaccactcttcacgtaataccaaacggagttgcctttgccttgggcggatcggtcgatgacagcttttttataagtgtaccaggttaccttggcaaagtctttagcagatcccaaagtcttgttcaaaccggaagtcgtgtagacgtagccgccctttaaatggtagggaagtggttggtcgtagtcttcggtagaaacaatggaagcagctggaatcgtttttttagtggtgtcattagttgatttggatttggtgcttgatgaactcgtggaagtcggcgtcgttggtgtcgttgtggcagcactggcaggtgccatgatcgccgcgatccccaaagcggctgtgatggcagtcgttatgtaaaaacgtttattcatatcaattatctcctcataatttcgaactatgtattactttagcatgatattgttacgaaacccttacatgccgcttacactcaaatgaagagttcgtgcacaacttgcttatttttagtaaatcaattatgattacttttagcaagatactaatagaacgatttgactagaatgcaagcgggggagtcaataaatgaatatcaaagtaaaatgcaggttaacactgttattttcattgatggtttttggcggtttggggatgaatactcaagtcaatgccgccactgatgattcaaccacggctgcgcctcagattcaatcagtcagcaaagccgattcatcggtcacggtgaatccggctgaggggacctcatccaacgtttcggtggatgagtcaagcgacagcgcagcggcaaagattgacgattcaaaagtgaacaaggattctggcagtagcgtcacaactacatatggggatgccaaggataaccaggttaaggctaacagcgatagtgataaggatgcggctaagggtgactcttcaacggctgcaagtgacacctccactgatgtgtctcaggattcatctgctcaaaaggatagttcatctgaccagaatgccaccagtgattcgtccagcccaaccgatgatgccattgacaccgatactgacatggcggacgtgactgaggatactgactcgagcaaggttgtgaagccagcctctgccaaggcggacgctgatgcggataaatccagcacagatgctcaaccaacaacggctgccagtgacgctgatgccccggatgatagtccagcggtcttggaatcactgacccaggatgcatccaaagccgaccaggcgccagagacactggttgtgccggatcaaccgattattgaaagccaaaatgttcacaacgatatcgttggggatacatttgccgacaaagtgacgaagagtgatcccaaggcagttaaggaagcaaccgcgattgccaataacaagaccaagctgttgaccttcaatgccttctcggacaaaatttaccgtcacgtattgaagacagctcagaagccggggacggtcacgacgacctctggccataaagtcaccttgaccacgcctgttaagcacgtgaaatacaccgagcatgattcaacaggggtttcagagaccctgccagtcatggccaccttggcgattatcggggtagccggtattacgtttatagcgtttgacccgcttagatttctctttaaataaatgattagacgaagcacggtcgggtttgtcggccgtgctttttgctgtctaaaggcgcgtcaatttaacgtttagaaataagttcaaaaaagagtatttaatacttgcaaacgcttacagatatgatattatatagtcaaggaagggaaaagaagttcgaagcatagggggtttcagcctactttgaatgttcttcgatccaagattaatatgttgttatgtcacaggattattttcaaatgtttcacgtgtagaacgcatagttgtttattttaagttttaagagtttgaggttcacgattcacagaagcatggatgtttgaataaatgatgttttatttagccgattgtttcagagattcatagagtttcaaattgttacagtttaaaataacagaaggttaattcaggtgattaagtgtttgaatataatgttatgagtcacacatgttcaaatatgaattcgatgattcgctattgaaaacctggtggagtaattgaaaagggttatgtacagaggtcacttgtagtgaatctgagagattcattcgaatatcaaattgatgtgatatcaagttgatgaaagatccaatgaaataggttaaggttcacaggttttaagtaccatgcaccttaggtttatgtatcacgtatcaagcagttgcaccaagtatgatagtttcacgtagaaccaaaatgttgaccacacggcaaatttatcaataaagtaaaaacgtgaaaatgattaaagtttgcggcagttggatcaacaaatagttagattgaggcgataagacattaaagttttaatgaagtgggtattaaccccaaagttcccttccgtataggatttaagcttgcagtacttagatgcgagtttgaatcctatttttttgtagagtgcgacgagcaacgggtgatgcggtgtgtaagagtgcggactggggcggttagtaaccggagtctaaggtgcttcgaacggaaatcgagtttgattttcgtttgaagttccttagatgcaggttgctgccccagggagcagatttccactagagaaaagggaaccacaaaataaccaatacataaaagaaagaccaccaagaaggacagccaacaagcaccaccaccagccaccccggcaccaacccaaaaccaaacaaattccataaatcccccacggtcgaaaattccctatttacgccagcaaaacactttgatataatgaaagcgcaatcaagaaagtaaaaggtattacttaacgccatttcttgatttctatttacaggactttctgcaatgaggtattctattcacatagaatatttttttctgagcaaagttttgatctggaaaggaagtttctcatgaactttcgtcgtgtcattgtacttgatctggcatctttgggtgtcggcgaggccagcgacgctaatcgatttgaatcggttggcgccgatactttaggtcacatcgcaactcttgaaggaactgactttcaactgccgacattaagtcgactggggttgggcaacatccgctacagcgacccggttgtcggtctgccgccagtggaggaaccgatcggcttttttggcaagattagaagccagagccgggagaattcgcaattaagtggtttgcgggagatgtttgactttcagacacccacccgaacgaccagcgtgattgacggcatcgtcggccttttaggggttcactcgattttgatcagcaattaccagagctacctttccaatcagaaccaagcggaagtcattccggtcaatacggatgagggtggcttggagcagcttcaccagcaggtgattgcgccgaataacggcctgctttattttcgggcattagggttgtccgaacacgcacaaacggggaaccgcaaaggctgcatcgattcacttaaattggtggatcagcatttggcacggttgatgcgggaactatacagcaccgaccttttaattatcacgtcttcgtatgccaatgatccggccatggacgttacgccaacgcgcgaatacctgccgttgattgcctacacgtcctcacttcctgagggcaaggccttgggaattcggcggacccttgcagacattggggcctcaatcggggagatatttggccttgaagtgtccaatgaatccattggcagcagttttctcggcgaattgaagtaagtcgccgcattatttagggtttaattcataaaaccaattccattacagagggggatagctagccatcttcatcgttgtttagcaattattgtcgttaaaattcagaaaagaggatttcagaatatgcaattatcatatttactggtcaatattctgggtgtcgccgtataccttggaattgctttcttgttttcaaataacaaaaaaggtatcaactggcgttcagttggtgttgttttagtaattaaccttgttctggcatggatattgactagcttctcctggggccgtgatgcggttaaagccgctgccgacggatttaactggttggtccaagtcgcttaccaagggatcaacttcgccctgcctaactgggttaccccacaatttggcggaactgccaaatcaatgaactttgtcacgagtgcgttattgccaatcctgatgattgttccattgtttgatacgcttacatatattggcgtattgccatggatcatcaagtgggtcggccgtggactttcatttgttaccggcgctccaaagttcgaatcattcttcgccgttgaaatgatgttcttaggtaacactgaagcacttgccgtttcatcactccaattaaaacaaatgtcagcaaaacgtaacctgactctggctttgatgtcaatgtcatgtgtcaccgcgtcaatcatcggggcttatacccaaatggttcctggccaatttgttttgactgccgttccactgaacgtgttaaacgccttgattattaccagcttattgaaccctgttaaagtcactcctgaagaagatacggttgctaaaatgggtggctcaggttccagtgaagccgctgttgaagctggcgacgttcaagctaatggtaaacgtgaaccatacttctcattcttaggcgactcaatcttgggtgccggtcgtttgatcttaatcatcgctgccaacgttatcgcctttgttgccttggctgctttgattgacaagattttggctttgttcaacccatggttgtctttggaacatatcttaggaatcatcatgttcccatttgcatggttaatgggtctggatgtcagtcaggcattccaattcgcccaattcatggggatgaagttggttaccaacgaattcgttgttatgggtaagattgccggcaccattcacaacctcagcatcttcccagctcactaccaagcacaattaacagttttcatcacttcattcgccaacttctcaaccaccggtatgattatcggtgccttcaagggcttggttgataaggaaaagaacgatttgatcagtaaaaacgttggtaccatgctgctttcaggtattctggtatccttaatgtctgctggaattgttggtctgtttgtttggtaaaatcagttctagaaagttaggttttatgtttggataagttacaaagagaagaagaggcggctaaccggctgcctcttcgtgaggctatacgggataaagccaccgtcaaacgggaaatcattgctgggatcaccggctttttcgcgatttcatatatcatcattgttaatccaatgatcttaaaagatgccgggattcccactgatttgagcgtctttgcgacgatcatttcttcgttgatcggctgcttgattatgggcttttgggccaatgcaccagtaattttgacgccgggaatgggcgtgaatgccttcttcacttataccgtggttgttgccatgggtctgtcctggcaagaagcgctggcaatctcgattgtctccagtatcatttatgtgattatcgcattcacgaagttgagtgagattttggccaggggaattccagagactttgaaagcggggattaccgccggcattgggctgtttttagtcgaaattggactggagaaggcgcagttgattcagcaggggaagaactcgattctggctctgggtgatttaaccaagccggcgacgctgctggcgttgtttgggttactgctcacgctatttctgttcgtccgcaatgttaccggcggcttctttatcggcattttggtcacgtcggtggtcggaattctgtttggcatcaaagatcaggcctcaccgtcagttggaattggcgatatcactcgttactcggggattgtcgccaaaggaaattttgacaacgcgttaaccattccgttcgttctggcagtcttctcaatgaccatgattttggtatttgaatcgatggggctgctggaagggattatgcctaatcccggcaagtttaagaaggcgtttcaggccagttcggtgaccagctttctttccgggattcttgggaccagtcccacggttgctgcagcggaaagtgcttcggcaattgaaagtggcggtcggaccgggttaacatcgattgttgccggactgatgtttgcggtttcgttgttctttatcccgttgctggcatttgtgccccaggcagcgatcgcacccgtgattatcattaccggtgcgttgatgatgaaccagctcagccgcattaatatgtttgatttttccgattggttcccggcatttctcatcgttgttctgattccatttaccagtagtatttcgactggtttggcgtttggatttgtcgcttacccaattttaaaaattgccgctggcaggcaacacgagctgactgtcgcgacatacgtcttaggatttttattcttgtgtgatttggtgctcagtgcactattatagaagtaacaagcgggcggacttcaggttcgcttcttgttaggaactaattgtaagcgtttgatattaacaaatattgtttggaaaggaacttatcatgaccatcaaaattattatggataccgatcctggaattgatgatgctgctgccttaaccatggcgttgaacgatcccgagattgacctgaagttgattaccagtgttgccggcaacgttaccgtggacaagacgactaagaatgcccaaaagattgtccgcttcttcaataaaaaggtgccagttgcagccggtgccaagcagccgttgatcaaggaatttgaagacgctgccagaatccacggtgaatcggggatgccgggttacgatttcccggaggatctgccaaagccattggatgtcagcgcggttgaagctttaagagaaacgatcatgagcagtgacgaaaagattaccttggtcccaactggttcttataccaacgtggccttgctgttcagtgaatatcctgaagtgaaggatcacatcgaacggatcgtcgcaatgggtggttcacttggtaagggcaacatgacttctgctgccgagtttaacgtcttcaccgatccggatgccgcacgaattatgtacaattctggaattccgattacgatggttggcctggatattaccatgaaggccctgattaccccggattctctcagcaagcttgagcacatgaacgagaccggcaagatgctgcatgacatcatcattcatgatggtgataacagcgctgaaggaattgccatgcacgacgtcaacaccatcttctacctgcttcacccagaagcgattaccaccaagaagatgtggatcgacattgttactgacggcccagccattggcgaaaccgtcggcgatatccgtggtgcttaccatgatggtaagaccaacgctaatgtttgtgtggatattgacgctgaggcctttaacaagtggttcttggatgaagtttctaagattaataagtaaattttctaggcagtcagatattttttctggctgtttttttgttggacggctgtaatagtttttctgcaccctacgtcttgacactttcccagtagattggcataatgaatctaacattaaaaacacatgagaacaatgcgatgacgagaagagtagtgatcgaggcgatctaaagagaagggccatttggtgagaggcttgattgtcaagatgatgaagatgagctccgagcaggtgaccggtagaagccggtgatccgtcagcaaacgttattttgccgggtatcgattttaaatggtaccgtcgaggtgtattttagatacacgaagatagggtggtaacgcgcatgagcgtcccttagtccgtaaccgggctaagggacgctttttgttttctcataatccaacatacattgcaaagtaggtgaaatcattgagcaaaataactgattatgattctaaattaatcgagtcactgttcatcaaatatgccaaagtcaacacgagatctgatgccaacagtcacacagtgccaaccactgtcggccaggtcaaactcgccaagatggtggaaaaggatcttcatgacttgggaatcaaggatgccaagtacgagccggaaaattcttacgtgcttgggagcttgccgagtaattctgataaggatttgagtgcgattggatttattgcccacttggataccgccgattataatgccgaaaacattcaacctcaggttcatccaaactatgatggcggcgagatcgtcttgaatgccgagaagcagatcgtgttgagcccgaaagaatttccactgcttaagcactatgtcggccagcgggtcatcacgactgatggcaccaccttgcttggcgcagatgacaaggccggggttgcagccatctttggcgccctcaaatattttctaacccatccagatgttgaacatggagaagtgaaagtagcgtttggccccgatgaagaaattggccgtggcgctaaacggttccctgccaaagaatttggaacggaatttgcctataccttggataacggccagccgggacaaatcgaagcggagacctttaatgcttccgaggccaaaattgatatccgcggcactgcagttcatcccggggatgcatacggcttgatggtcaatgccgttaccttggccaatgaaattgtgagtgcattgccaaaagacgaggttcctgaaaagagtcgcgatcaccaaggcttcattttggtcaccgacatgactgcaacagtgggggaggcccatctcaatctcattattcgcgagtttgatacgcagaagtactatcgcaatttggcactgttacatcagattgttgacggaattaatgatcggtatgattctccaagagtcagtctgaagattaatgaacagtatcaaaacattggcgatacggtcaaacagcatccatacatcgtcaatctggcattgaacgtctatcatcagctgggaataacgcccaacattacaccgtttagaggcggcaccgacggtaatgcgattaccgctaaaggtattccaactcctaatctatttaacggtggtgacaattttcatggcccttatgaatatgtcagtaccgaagcgatgaccaagactgcccaggtggtcagcgagattgttcaggaacacgtccgcgaatatggacaccgcgacgagagcccagttaaattaaattaacaccagacatcagcaaccagtcaatccgactggttgtttttatttgcggattgatcaggttgacaacttcaataacctcgatttacaggtgaatttactaaacccaataaattcatggcaaaacatgttaaaatcttatatgtatgcaaccgacaaatgtctttggacaccttgtcagtcaagctattttaggttaaagtataataagacgtgaaacagattgtttcacatatcaggagaaatcaagcatgaacaatgatcaattcaaaaaggcgcttttggataaaggtatcgaagtcactgatcagcagatggatcagttcgatgcctattttaagctgttagtggccgttaacgaacacgttaatttgaccacaattacagaaaagcctgaagtgtatctcaaacatttctacgattcgattacaccagccttttttgtttcacagattaaaacagcgccattgtcgatttgtgatgtgggagcgggagctggatttccatcattaccgttaaaaattcttttcccacaactcaaagtgacgatcgttgattcattgaataagcggattaactttttgacaaccttggtcaaagaattaaacttgaccggagttgagctgtttcatgcccgcgccgaagaatttggcggtaaaaaatctgagcatcgtgagcagtacgatctcgtgaccgcccgtgccgtggccagattaaccgtcttgagtgaactttgcctgccattggctaaagtcggcggcaaaatggttgccttaaaggctgccaaagctgaaggggaactatcagatgctcagccagcgattcaactgcttggcggtcaggtctcgggggactttgaattttcactgccggtttctgacgaagaacggcacatcattgtgattgataaggttaaggaaacccctaagaaatatccacgaaagccagggacacccaatcgtgaacccctggatcaaatcaaacgatgaggagggatgaaagatgacatacgtaatcgcgcttgcgaaccaaaagggcggcgtcggcaagaccacgacggccgtcaatttgggtgccgggatggcttcgatggggaagaaaattctcctggtagatgccgacgctcaggggaatgcgaccagtggagttggcgtctcaaaggcagacatcaccaaagatatttatgatgtcttggtgaatgaagaaccgatggcagaaacaattgtccacacctcacatgagggtttggacattgtcccggcaaccattcaactgtctggtgcagagattgaattaacaccccagatggcccgagagacccgtttgaaggccgccctggatgccgtcaaagaccaatatgatttcgtattgattgattgtccaccgtcgcttggtttgattactatcaatgctttcacagccagtgactcgattctcattccggtgcagagtgaatactatgccctggaagggttgagccaattattgaacaccattcaattggtcaagaagcatttcaatccaaatttgaagatcgaaggggtattattaaccatgtttgacgcccggaccaatctgggcgaacaggtcaataccgaggtccgcaaattcttcaaggatgaggtttacgacaccattatcccaagaaacgtccgcttatcggaagcaccaagctatggtctgccaatcatggattacgacccaaagtcaaagggtgctgagaaatatatgaatctggcaaaagaggtgctggcaaaccatggctaataagaaaaaactaaccggtcttggcaaggggattgaagccttgttccaagataataatgtcgatacgagcaaagaagatgtcgttgacctgaaagtcagcaccatcaagcccaacccgtaccagccccgccaccgttttgaccaaaaagcgttggaagatctggccctttcaattaagaactccggtgtcttccagccaatcattgtcaggcagcccgatccggaagttgactcatttgaactgttaactggagaacgccggctgcgggcatccaaaatcgccaagcaggagacaattccggccatcatccgcagtgtcaatgaagagcagatgatggaaatcgctgtcatggaaaacctgcagcgagaggatttgaccacgcttgaagaggcggaagcctataacatgttaatgagtcgactggacctgactcaggcacaggttgctgcacgactgggtaagagtcggccgtatattgccaactacttaagaattctgggcctgccgaccgaagttaagaaaatgctcgaagacaagaaactctcaatgggccaggccagaaccctgctttccgttaataacaagcaggagcttattaaattagcccgcaaatcggtcaacgaatcgctaaccgtccgccagctggagcaggctgctgccaagatcaacggtaacaagccggccaaaaagaaaaaggcccccagaaaatcaccatttgtcagggcgtcagaaggtcaactccaagaaaaatttggcacatcggtttcgattgtcaattcatcacgcaagaagggtaaaggtaagattgaaattgagtatacctccacagacgatctcaaccggatcctggaaatgtttggggtcgatttggactagtcacgttgccgaaaggagacttcatttatgtatgatttaaacgatttagttgaaatgaaaaagcctcatccatgcggcaccaaccgctggcagatcattcgaatgggtgcggatatcaaaattcaatgtaccggctgcggccacattgtgatgatgccccgaagagaatttgatcataaattaaaaaagatccttgaaaaagctgaaaaataaaccagaaagaagcgtttaagttatgtctttaacagcaggaatcgtcggcttaccaaacgtcggcaagtctactttgttcaatgcgattaccaaggccggagctgaaatggccaactacccatttgcgaccatcgaccccaacgtcgggatggttgaagttcccgacaagcgccttgaccgaattcaagaattaattccagccaagaaagtggttccgaccaccttcgaatttaccgacattgccggtatcgttaagggtgccagcaagggtgaaggacttggtaacaagttcttggaaaatatccgtcaagtggatgcgattgtccacgttgtccgtgcatttgacgatgacaacattaccacggtctccggcaaggttgacccactggacgatatcgacacgattaatttggaattgggcattgccgatctggactccgtcaacaagcggttaggtaaggttcaacgcgctgccaagggtaatgacaaggaagccaaagcagaattggccgttcttgagaaaatcaagccggttttagaagatggcggttcggttcgttcaatcgactttgatgaggatgaacaaaagattgttaagggtctattcttgttgaccagcaaaccggttctctacgttgccaatatcgctgaagacgacatggctgacccggagaactccaagtatttcccagaaatcaaggaattcgctgccaaagagggtgccgaagcaattgcggtcgctgccggtcccgaagaagaaattgctcaattagatgatgacgaaaaggctgaatttctggaggctgaaggcgttaaggagcctggtttaaataggcttatcagagcctcatacaagcttttgggcctgcagacgttcttcactgcaggtggtaaggaaacccgtgcctggacctttaagaagggtaccaaggcccctcaagctgccgggatcatccattcagactttgagcggggcttcatccgtgccgaagtcatggcctttgatgatttggacaaattggagacaccagcagcagtcaaggaagcaggtaaattgcgccttgaaggaaaagactacgtcatgcaagatggcgatattgttgaatttaggtttaacgtttagacgttattttaaggagtgaagctagtgagtagcaacgatgacacacagcgcaatgccaacagcaaagcgcgtcagaagaatgcccaggtgcatcaggatcgggatcatgcggccaaaattgtccattcccagttcgataacatcgggttaactaagcggaatgctgagtacatgttcaagttcaatcaggcacttggggctaccaaactgtctgcagataagaagaacgaagccgtccagacgatggttcaagaattgctggagggtcaaaagtcaggcaaaactgccagaaatatgtgggggactgtcgaccaaaagattgaaacgacggttcatccaccggcaagacctgctgatccacgcagagactattggaagaatgccgggtacaatgctgtcctgtttttgacgatcttcttcttgatgtatggggttctgtggttcctgccaactaagggcggccaacactcaccaatgatgggcatcactggaattctcattagtgcggcagttgccggcttggggattccaattgtgacgatgatgttcacaccaggtgttaagcatcgattctcaatttggattcgcatcatcctggtcgtcttgttcctgatcgtgtggatgggaatcttcacgctgtcatcaattctgccgccagttttgaacccagtcttgaatccaatcgtctacatcgtgttgggtgtgttgtcaggagtggcagccttcttcgtcaagcgccgattcaacattaccggtggtgtgttctaaaactaataatgcatttaacgatatggtttggtcagatgagttgtcatttgatcgagccattttttgtccatgctccaaacacgaacaataaaatgtaaatttttgaaataaatgccagacgacgaaaaaagatgaacaatggtctttatttattcggaagagtcgtgtataatcaatacaatttcagaaaacgatttgcttaaggggcttgtcatttttatgagaagcgtatgagaattctttcagatacgttgaataactaaaatgaaaatgataagttattagacaatcaacatttaaaaggagcgagatagatggttagttgggatgaaaaattcggtaaaaaaggtttgacgtttgatgatgtgctgttgattcctgcagcgagcgatgttttaccaaatgatgtggatttatcagtacaattggcagacaacttaaagttgaatgttccttttctaagtgccggaatggacactgttaccgaatcgaagatggcgattgcgttagccaagcttggtggcatgggtgtggttcataagaatttgagtattgaagatcaagccgctgagattgccaaggtgaaggcagttaagaagactgctgacactcctaaagctgcggtggatgacaacgatgcgttgttggttgccgccgctgttggggtttcatccgatacttttgaccgggcatccgctttactaaaagccggtgccgatgcgatcgtgatcgataccgcccatggccattcagccggagttcttcgcaagattgctgaaatccgtgaccactatcctcacaccactttaattgccggcaacgttgccactgcagccggaaccgaagcccttttccaagccggcgttgacgttgtcaaagttggaattggccccggctcgatttgtacgactcgggttgttgctggcgttggggtccctcaaattacagctgtctatgatgcagccagtgttgcccgcaaatggggcaaggcaatcatcgctgatggcggaatccagtattcaggcgacatcgtgaaggccttggctgccggtggtagtgccgtcatgctcggcagcgtcttctccggaactgacgaagctcctggtgaagtctttgaagatcatggtaagaagtacaagtcataccgtggcatgggcagtgttgctgccatggaacaacaacatggttcagctgaccgttacttccaaggcggtgtcagtgaagccaacaaattagttcctgaaggtattgaaggcgaaaccgaatacaaaggcagcatcaacgacatcgttttccagatggtcggtggcctgcgttcaggaatgggttacactggttcagcaaccatcaaagatctcaacgacagtgcccaattcgtgcaaatcaccaatgccggcttgagagaatctcatccgcatgatgtcaacattactaaagaagcacctaactacaaaccagaagattaatgcatctcaaacacctgcaggtcaaccgctatccgcgattgacctgttttttgtcttcaaactgagtttggttaaaatgtcgccgggttccagttcaccggctccgcctgctgtagtggcttggatttcgagcctgtagtctcgaaatgccaagatgctgtaatcacgacttgcagtcgtttcaacagcatggacactacagctggcaatgccggtaaactggaacccggctactggcagcatatctatgagtttggataaaagtgattgaaagggaactgcatgattcgcaaatcaaacggaatgaggccgaattttgctggtttggcattgacagccatagtgaaagtgttgttgaagccgatgaaatcggcaattacaacacctttgtatttcaagactacaggcttgaaatcaaagccactatggcaggcagagccaaaccagcaaaattttccacttaagcagcctcttagcacttacaggacgagaggaatgctaagttttcatcaatatcgacaacaattatcatttttattactaaataggagtattatgattctgttagcaacattaatcatcaaggcaggaggcataccgttggactcacaaaacattcttgaacggccatttatcaccatcactaatttaatctggagcttcgaccacgccaccaatcgggtcaatattctgctggtcaaacgcgataacgatccttacaacaactactgggcattaccggaaacctttatgcgctcccaggaaagtgccgaagagactgcgttgcgcctagtccgagaaaagattggcatggatttgtcaggcagtcacactgaacagctggcaacctttaccaatcctctgcggacacctggcgatcgggcactgtctttggggtacatgacatttttacctgataaaccacaactcaaggcggggtatggcgcctccgatgcccggtggttcaccatgggatatactgataaaacatacacctttagcgattcggatcatattttccaatccaccgattgtccggttcaacggacgtactatgcagaatttggcgggaccaacgctgatcctgacaaacacttggcatttgatcatgaatggattttgaaggttgcctgtgagcgaattcgcaacaaactggattatcagcctaatatcctgttgatccttggacgtcaattcacactcaaagatgctcggcgagtctattcgccatttttaaaacttcgggttgaacaaattgacaactcgaatttcaagaaaagtcaccaagatctctttactgacattggttccagcgagattaacggtcccggtcgtccggctcggttgtacaaattagcccatttgcgggcgtaaacgcttgaaatgttatcggagtcgttgtaacgtagaataaaagtttggaacacttttattttaagaatataaaagttaaaggtacttttaatcccaatgaaaagagtcgaaacataatgagtaacttatcaatgttgacagatttatacgaattttcaatggctaacggctatcggcagacgattaccgacgagcagggggtctttgatgtcttcttccggaaagttccggataacggtagttttgtgattgccgccggcttggagcaggccgtcaaagcgctgcagaacttccactttgacgatagtgacatcgagtatctccgatcattgaacctgtttcaagagaattttttgacgtatttaaaagatttcaaattcgattgtcaggtatccgccattccggaagggacgcctgtctttccacgagagccactgctgacaattcggggacctttgctgcaaacgcaattatttgaaacgatgattctcaacattttgaaccaccagtctctcatcgccactaaggcccgccggattacctattctgctgatggccggccggtgatggagtttggtgcccgacgcgcgcaaggccccgacagtgccacgtatggtgcccgagctgctgtgattggcggctgttccagtacctccaacgtgttggcagccgaagcctttggtatcccggccgccggcaccatggcccatgcctggatcgaatcgttcccagatgaattgacctcttttgaaaaatgggccgaagtttatccagacaatgctgccttactggtcgatacctatgatgtgctaaaatctggcgtgccgaatgcgattaaagtcttcaaagaattgaaagccaacggccacaaaccagttggtatccgaattgattccggtgacatcagtcaactttccaaggctgcccgcaagatgctcgacgatgccgggttgccggaagtcaagattacggcttcaaatgccttggatgagcacgtggtcgcttcactccttaatgagggcgcgccgttggataactttgggattggtgagaagctgatcactagtgcctcttcaccggtcctcagcggggtttacaaacttgctgccgttattgagaacggtaaaatgattcctaagatcaaagtcagtgccagccgggaaaaggttaccctgcctggtctcaagcaggtctaccggctttatcaaccgggaactgataaggcctttgcggatgtcatcgccctcagtgatgaatccttggatcaaccgattacggtggtgaaggctaacccactagctaccaaacgggaacagcgaatcgagaagtttgacgccaagccactccaaaatgaagttttggccggcacagatttgaagatggcttttccaagtgtctttgatattcaaaagtattccaaacaaaaactaaccgagattccagctgccactcagcggttggtcaacccggacgaatttccaatctatgtgaccaccaagctggctgccttgcaggagagtctgctggaagcggatgctcagtagttgcatgacattttaataaagaattagagctgttggtaaagttggagctttgccggcagctttttttcacatatcggtccgggtaaatttgaccctcctgaggtgggatgggtttataatacccctgtaaacggttacatgacggatgtgctttagaagggggcatatttatgtattattctaatggcaattatgaggcctttgccaaacccaagaaacccgcaggtgttgccaacaagtcagcctatttaatcggttcgggtctggcgtcactggcagccgcagtctttctggttcgtgatgcgcaaatgccgggggaaaatattcacgtcttagaagaactgtcactgccaggtggcagtatggatggcatttataatcctgacaagggttatattgtccgtggcggccgggaaatggaacagcactttgaaaccttgtgggacctgtttcggtcaattccaagcttggagaatcccgacgtctcagtcttggacgaattttattggctgaacaaggatgacccgagtttctcacatgcccgagcaatcgagaagcgcggccagcgaattccaactgacggcaaattcaccctgtccagaaaagcagtggaagaaatcgccaagttagtgatgacgcctgaagaccaattggataatttaaagatcaacgacgtcttttccgatgacttcttcaagtctaatttctggctggattggtcaacgatgtttgcctttgaaccatgggccagtgctgcagaaatgcggcgctacctgatgagatttgttcaccacgttggcacgctgccaaatatgtcgtcactgaaattcaccaaatacaatcagtatgagtccctgatcaaaccgatggtcaagtacctggaagatcggggtgtcagtttccagttcaataccacagttgaaaatgtgattgtcgacactactgatgggaagaagaccgctaccaagctggagattattgaagacggggtggagaaaggcattgatttgacgccaaatgacttcgtcttcattaccaacgggtcgattactgaaagcacgacctatggagataacgatcatccggcagctaaggagcatgcggttggcgcggcttggacgctttgggagaacctggccaaacaggatcctgcattcggtcacccgaagaaattttaccagaacattcctccggccaactgggtgatttcagccacgaccacatttactgatgatcgaattgtgccatacattgagcggattaccaagaaagatccgcacagcggccagttggttaccagcgggccagtgtcgattcgggattccaactggttgatgggcctaacagttagtcgtcagccacacttcgctcagcaaaagccaaatgagctggttgtctggacttatggcttgttctcagatttacctggaaactatgttcaaaagaagattgccgactgctcagggattgaaatttgcgaggagttcttataccacattggcgttcctgttgatcagatcgaagagattgcccaatcagccaacacgattccggcccacatgccgtacattacctcgtacttcatgccgcggcaggcaggcgatcggccgctggttgtcccagccggttcaaccaacttggcatttatcggtaacttcgctgaaacaaagcgcgacacggtctttaccactgaatattcagtccggacggcgatggaggcggtctatcaactgctgaatgtcgaccgtggtgttccggaggtcttcgattcatcatttgatattcgatcaattcttagttctgtgtactatttgaatgacgaaaagtccttattggaattaccgttgacaccaccggaaaaaatggttattcagcgattactgaaacatgttaagggaacttacttggaagaaattttgaaggatcaaaaactcatctagggagatggcaggtatgaaagcaagatcagtcatttgcggtggtttattgtttgcagtcggcgtagcagcggggatgcacgtggatcattgggcacatgaaatgcaccatatgcatcatcacggccatggtccgcatatgggtccgggtcatttccacgaccaaccttttgaagatattggtgatctaccttatgttcgcgagacgcggactgatgggggtggattgaggaatgaagtttagagtgcggaacaagccgtttagcttttgagcattagtgtgataacgggcgttaacgctggtcctgcgttaacgcccgttatcggactaagcggagaaagctggcttgtggagcacatttctgctaggtaagagaagatcttaaaagagaatcgtcaacatggtagaaccaccaaataaacccactaagtagcctgaagcctacttcctggaattacttggtggtttttgtttgaggatgattttactgtgctattgtccttgttttctagcggaaacgtgctccaagcaactgatgcttgtatattaaagatgtcagcaaggtaacattaatttgtactaaactgatattaagcgctgtggattagtccatctgaggtacggatcctaacggatactggttacgttagactctaaccacagtcttttgttgtactgttgattagtttgataacacatatcccaagatatgatgtttcatttaatgcaagaatacagggcaagagatttgtggagcacagcgttaattacatacgtgaggagcggtaatgatgatttatgctggaattgatgttgcaaaatatgagcatcatctatcaattattgatgaccagggaacggtactattagctgatctggaatttctaaataatcgtgagggttttttgacggctcaagcgacacttgacaatgcgcggacggctgatggtcaagtccaagtgggattagagaataccggccattatggttataacttgatcagctatttgcgacagcacaagtttcaagtgtttgcttacaacccattactaatcaaaaagtatatccaggccaataccttgcgtcacacaaaaacagatccacaagatgcgttggagattgccaaaaagctaaggtcagataccactaaggttagctttgaagcagacgccgatatcattgaattgaagagtgatacccgctatctggaaggacttaagcgtaaacgagtaaaaaccaagctcgcatttacaaatgtcctcgaccaagaatttcctgagttggcgccaaatctagggccagtatccgcaaagtacagtcagtggttgttggcacttttgaagagatacccgtcaacagataagttggctcatggacgaatcaacacgatgacaaacatcattaccaaatactccatgaagcagcatggcgaggaaatggcaattaaagttcgtgaactggccagagaaacgattggtcaagcatctgatagtctttcatttcaactcctgcagttgatcgatgcgctacaatttgagacccagcagatcaaggaagctgatcaaaagatccacaaaattatgaatcggattaagacgccgctcctatcgattccaggagttggagaaacactagccgccattattttagccgaaattagaaatgtgaactactttcaatcaccaaaccagattctggcatttgccggtgctgagccctcaatcattcgctctggtgaaatgcaaggtaactacggtcacatggttaagcacggttcaacgcagctacgctgggcgctctttcaagcagccagactgtgcgcaatgtattcgccaaccatgcgagcgtattatcagaaaaagaggtctgagggcaaaccatatttggtggcattaagccatgtagtcaagaagctagttcgaattatttaccacattctaaaatacaatgacccatggtctgagacggtgattagagattaaccaagcctaaaaaccatgtaattatcaaattcaaaaaataactatttttgaagcttatttcttatacgctcaaaaatggggtaataaacttcaataaagtcattatttttccttgacgtaatatagtttgtctaacgtgtaagagggacagaggttaaaatccgggttcaggattttaaccactgtccctcttacacaccgcatcacccgttgcttgtcgcactctcttttttaagttccccttaagcttcccatgctaatcttgtaaacgttgtgcaaacgccttacagtaacatttcagacatgcttgttgaatttattaaaaaagtgtaaaatcaaaactggatgctaattgataaagccagacacataataatgataaaataatagtaaatacagacgataatgaggttgattacactatgaaaattttagttgtcgatgacgataaagaaattgctcagctcctggaaatttatattcgaaatgaaggctacgagcctgtttccgcttacagtggccaggaagccctgacccgcttacggactgaatccgacattggtttgatgatcttagacatcatgatgcctgggatgaatgggattgaagttgtcaaagaagtacgtaaagattctcagattcccatcatcattttgtcggccaagaccgaagacatggacaaaattcagggcctgatcagcggtgccgacgattatgttaccaagccgttcaatcctctggaagtcatggcacgggtaaagtcgctgctgcggcggactgaagagcacgtcactaacgatacgcccgatgttttggacattggccccttaaccatcaataaagattctcacgaagtcaaaacgatcactggcacgccgattcagctgactgccttggagttcggtattttatacctgctcgccagccatcctaaccgggtcttttcagctgacgaaatttttgagcgggtttggcgacaggaaagcattgtctcggccaaaaccgtcatggtccacgtcagccatctgcgtgacaaaattgaagaagccactaacggcgagaaagtcatccaaactgtttggggcgtcggctataagatcgagtcccattaggccaagtcaattttgaaatgggggatgccgcatgaaactgacaggtcgtgagaaaactgagctgtttctggaaggtgtcgtaacagtcattttgcttttgttgctcaacctttcagtgatcattttaattaaccaatcaatctccaccaacccagggctgcgggacggaattttcattatcaaacgatcgattttgattggccccgaccacatgcatctttggagctgggagaacatttttattgtcctcctgctgctgtttgatggtgccgtggtttattggcggctgatcagacgttaccaccaaattcagttgcgccacatcatcagtgagctgcattacattgccaatggtcatttgaatcaccgaattccctttaaactgagtggtaatacccaatcggtggttgaaagcattaacgccttggttgacagtgtcatcaagtcaatggatgaggaacgggcaattgaaagttccaaggatgaactgattaccaatgtcagccatgacttacggaccccgttaacctctattttgggctacctgggtctgattcgggataagcaatatcacagtcaggaagatttgctgaagtacaccgagattgcttatttgaaggccaaacaaatgaagtccctggttgacaatttattcgaatataccaaggtcaaacagaccggaacgccactttccatcagtaagattgacctcaatcaaatgatggaacagctggtggccagttttgagctggaagctgataaaagcgggctggcaattgctgctaaagaaacggacaagcccttatacattgaggccgacgccgaaaagctgggccgggttttcaataacttgatttccaacgccatcaaatatggcaagggcggccaccacatttatttgagtgccgcagtcggccaacccggcgaagttgtcattcacgttgccaacgatgggccggagattccgcaaaagtcgcttgatcagatttttgaacggttctatcgggtggagagctctcgcaataaggataccggcggctccggcctgggactggcaattgcccagagtatcattgatttgcatggcggctacattaatgtcagctctgatgaaaagttgacgacctttgcgattcatttaccggttcaacatggtgataaattaagcaaaaagccccgccaaaaaattgctgaataaaaggagaactttatgaagcatcgaatcaaaattttaacggccttaatgggctttttttgcgttttaacactgtcgatgacggttgatgccaagtcgacagttaccccggaaccagctatttatgccaaatcagcgattgctgtcgatgctgacagcggtcagattttataccagaagaatgccaatcagccgcgggcaattgcgtcgatttccaagttaatgaccgtctatatcgttcatcagcaaatcaaggccaataaactggcctgggatgacaaagttaaaatttcatcggaacttgccaaattaagcacggcctccggtctcaccaacgtaccgctgaccgccggcaaagcctattccgtccgccaattaatcaatgcgactttggtcgaatccgccaatgcagccgccttggcacttggccagaaagtggctgggacagcaaccaaatttgccgcgttgatgaacaaaaccgcccggaagataggcatttccgacggccacttctacaatgcttccggtttgaccaacaagttgaccggtaaattggctttaccacatgtcagtgccaatgcggaaaatcgattgtcggcaaaagatgttgccttgctggctcaaaagctgctgcaaaagttccccaaggtgaccaatattaccaagcagacgacgtcaacattttatgggaccaccatgacgggacataatcaattgattgatgatcacaatttgggtcaaggtgttcgcgttgatggactaaaaactggaacctccgacaaggcaggggcgtgttttgttggttcagccacgacgaatggaaagcatcggattatcacggtggtgttaggtgccagaaacaagtccgccagcgatcctgcgcggtttattcagaccgccaagttgatgaaatgggtttatgccactcatcaaccgattaagttggcagccggagcgacaattgccggggtcggtaaagctaaaattcccgatggcaaacagacgaccatcttgccggttaccaagacgacccactgggtttgggccgacaaaggcacttctgccaagcagatttctggtcagtatgttaatcagcctgccaaactgacatcgccgactaaaaagggcactgaggtaggtcacgctcggctaagcattgacggcaaacgattgcaatacattggccactcggctggcaagctggtgatggtgaccaatcaatctgtgaaaaaagccaatttctttgttcgcctatggcgcgcgatattacggctgttttaaaattcaattacacaaaaggtgtttattaattgagtcatatcccatataattgtatttggattgtgtttacattatttttacacacatgtcacgaatgtgtgagatgggtttagatggaggaatccttttgggaaaagctgtcgcaaaatctagggagaagctgccatattggcgaagaattcttgacgcttctttgcctgtagatttgagttatattccaattgggctggcatgcggtattttattgaacgcttccggctttaacgtttggaccactttaatggtttcaatcatggtcttttccggtggggctcaattcttgattgcgtctcttctggccactaatgcgccgatgctttcggtcattttaatgatgttctttcttgaactacggtacgcattgctggggtccagtctttccaagtatctgcatggagaatccttggggtttaccgcgctgtttgcggcgtcaatgaacgatgaaaactacgcgttgaactatttaaaattttcaactgataagaagtttacccctcatgaagcactacatgttgaacacatgacgctgatcttttggacaattagtaacattatcggcagtctaatcggatcggctattaacattgatttaacaattgtccattttgcactgaccgcgcttttcctgtacatgattgtggttcagctgaagaatgggttgattattgtaatttgtattttgtcaggattcttggcggctttctttatggtccttaccaaatccacgttggggctggtcttatccactttgacagcatccttcattggttttttggtcgaagcgacgatcagaaagtacaaacccaagagtggttggctgcggccgatgaaaaaccctgccggatcgcctgaagacgccgacgaagacgctgatgactaggagctatctttatggaatggaacacaacacagcatgtatggttaatcttggggtgtttttgtgtggcttttgcgccgcgactgattcccctgatgtttttccgtacccgaaaaattccagattggtttaacgaatggatgagatatgtcccaatctcgctcttcacggcgttggttgtcaaggacattttcatttcacctgaatataccgtcaccatcgtcaaccgggcaccggagatgattgcggccgtcattgtgattgggattgcttattggactcgttcaatggcaatttcggttgttttggggctggttgctgtttttctcttggcgatggtagtgtgatgagcgacaagttacatacaaaaaggtcgagggaaaggtgattttgcctatctctcgacctttttatttgtggtcattaatctagttgcactatgtgggaatctatttggattaaattcttacagtaaaattcttcttttaattttctcagtcggattggcgactaccaggccaaagtcgtcgggactcaagcgttggtcgacccgcatcccgttttgcacgagaatggtgtacttgtaattttctttaatcgcaatgtccatgaatgggtcgatcaagtcctggtccatccggccgttgatgtagagacggtattccggatagttttttaagatcttagtgaccatttccgccgtgccggcttgctggagctggccgatcgtcagcgctaaggcgactcgttctctgaagttgccaagaaatgcccgtttctcgtccggcttgatctgaggattgccaaacatgtgctgcttaatatattcttctgaactgtcagccatttgcgtgctcctttcaaatctttaaaattaatataacaaatattttgaacaaagtctcgatctgtcatttgttataatagtctctaatgattgtttttccaaatatcgtgaatcttggcatgccagtgaaaatgccaattagggaaaaatgttataataaatttgaacaaattttattaggagggcttcaatttgaaaaaatggatctggattgtaatcgccatcgttatcggtgcatcagttggtggttacgcatatgcccgtcatagccaaaacgaaaaaatttacgctgaagctatgcagcgaggccgccttcaaatttcgaatgaaaaatacaccgctgctgaaacatcgtttaccaatgccttaaaacgcaaaccgaatgatgataaagcggataagatactgaaccaaacgcaatcgtttatttccgccaacgatttatttgacgaccttaaattcggtcaggcaaagagtgagtatcagtcagtcgttgacaccaagaagggcaatgaactgttgtctgatcgtgccaaagcacaaattaccaagattaaaggcatccaaaagaaccgtcaaaactacaacaagatttataatcaagccttggatcaggccggtaatgggcagtacaccgagtccaacagtacgctggataagattttctctgataaatcaattcatcaaaagtactatgccgatatcctgaagaaggcccaaacattacgagataagaacaatgatgccatcagcggcaatgcttccgctagttccaacagttttgactccagcacatcagacagtaacaccagcaataatcccaacgtttccggcgctaagggtgctagtttgacgtcgtctgagaagaaagctgccgctgcctacaagggctcaaatgaatacactgtgaccaagggcgaccgcgatcttgacggcaaaccgattacggctgctcagatcaccagtgccagaaagcaaatcagtgctgctggtgtcgattccaacgcaatgagcgaccaggatgtcagaaacgtcatcaaaggtgctcacaagaatggcgaaacaatcggccagtacgtgaaagcccgatattaagattcggtaaaggggttgtgacaaaactaacgttttgacaacagcccctttgcttgtttcattttatatagctggaacgtgtgccaaaaggccgcttcctaggcataacctagaataactttccgagctttcagctcaaaaagtcattctaggttatgcaacggaagcaagaccgccttttggcacactccctttctgtttataagtaataatacttgtgagaaaccgttttctaagagtaaaattaattttaattagaaatcacgagggggttgggtatttgtcaatttgggcaaggttcgtcaacaacgtaccactgagaagatttaccgtgttgatgctggtcatctttgtgctttatgtgacccggagtatgatcagcacagtgctgttaacctttatcttctgtttgttggtggttaaattaaccaatgcaatccgcaggcacatcaagattccggcgggcattatcgtcacgttcgtttacctgttggtaattttggggttgtactttgcagtgaccaaatatattccaaaaattgctgatcaaaccattcgaacgacacaggatattattctcttttacaccaaccccaagaatctaccggatgataccacgatgagttggttgaatgaactggttaagcaaagcaatattatggctcagatgaaaaatggcgtgtcgctggtttggaaatacgtgaccggcgttggaaccatgggaataacgctgttcttgtcgatgattttgagtttcttttttgccattgaacagcgaaccatgaccagattttccaagctgtttcttgaaagtgactttggctggttcttccaagatttgtacttctttggcaagaaatttgtcgcaacgtttggtgttgtgattgaagcacaattcttcatcgccatctgcaacacagtccttaccaccatcgtgatggccttcatgcatctgccgcagctggcagccttggcattgatggtcttcatcttgagcctgattccagtggccggcgtgattatttcctttgtgccgttgtcattggtcgggtattcagtcggcgggtggaatgatgtcttttatctgttgatcacgatcattgtcgtacacgcgtttgaagcttacattttgaaccccaacttcatggcctccaagaccaacttaccgatcttctatacttttgtcgtcttattgatcggcgagcacttctttggcatttggggattaatttgtggggtacccattttcaccttcttcctcgacattttgggagttaagaagcatgaaggcaaactcgacaaagtcccaaccaagccgggggaaccatagaaaccggattcactttataaaagtttcacaattaagctgaaaaaattttccatttggtgtaaaatcaatctgatagagataaagaaagaggtaattatattggcaaaacttgtgttaattcgtcatggtcaaagtgaatggaacttatctaaccagtttactggttgggtcgatgttgatttgagtgaagaaggggttaagcaagccatcaatgctggtaaattaatcaaaaaagccggcatccagtttgactttgcatttacttccgtattgactcgagcaatcaagactttacattatgctttggaatactcagaccaactttggattccggaagttaaatcatggcgtttgaacgaacgtcattacggcgctttgcaaggccacaacaagaagaaggctgctgaaaagtatggcgacgaacaggttcatatctggcgtcgttcatacgatgtattgcctccacttctgaaggccgacgacgaaggttcagccgttcatgaccgtcgttacgccaaccttgatccacacattatccctggtggtgaaaacttaaaggttaccctcgaacgggttatgccattctgggaagatgaaatcgctcctaaattacttgacggcaagaacgtgattattgctggtcatggtaactcattacgagcactttcaaagtacatcgaaaacatttctgacgaagacatcatgaaccttgaaatggctactggtgaaccagtggtttacgattttgatgacaaattaaacgttgtcagcaagactaagttggactaattagataatatttgaagcactgttgttgggtaatcctgataatagtgcttttttgttgcttaagattcacccaactctaatggtaaatggggaaactaacgcttatcaacggatgaaccggtttcaattttaatggagatttaaccttgttcctgactcttgttggttaattttaataatggcatgctattctttagtttgatttttaacaatcaccagaattacatatttcaaaatattataattggggaatctagctatgtcgaagaaaaagatcacgttagttggtttaatcttaatgatttttaccacgatttatggttttgccaataccaccgttgcttatgagcaaatggggtatgcaagtattatttggtacgtattggccgcaattttgttcctgctgccaactgctatgatgttcgccgagtatgggtcaaccttcaaagacgcccatggcgggatttattcctggttagccgggtcaattggcgaagaatgggcctttattggtaccttcatttggttatcatcctggattatttggatgatgtccactgcttctaaagtctggattccgtttgcgacaaccttattcgggcacgatacgactcagagctggagcttctttggcttgagttctaccaagacgattggtctgctggccattctttggatcatcaccgtaacatggtttgcggttcgcggaatggactcgatttccaaaatttcttcggtgggtggaatctttgtttcgctgctgacggtgatttttgcaattgccagtgtcaccgttttgattttaaacggcggtcatttggcccaaccggttaccgggatgcacagctttattcaatcgccgaaccctgattttcagtcaccaatcgctttgatttcatttatggtttatgcggtctttgcctatgccggaactgaaactcttggtggtgtgaccgataatatgcatgaacctgaaaaaacatttccacgcgggttaatcatttccactttggtaatcaccgtgatgtattcactttccatcttcctctgggggatcactgccaattggcattcagtccttggaaatggtcacgttaacctggggaacattacctatgtcttgatggccaacctgggtgttgtgctgggccagagtctgcatctttctgcagctgccagcaccatcttggggacgacttttgcccgctttgccgggttgagtatgttcatggcttatatgggttcgttcttcgtgctggtctactcgccactgaagtcattcatcatgggatcaaatccgaatttctggcctgccaagatgactaagttgaacaagaaggggatgcctggatttgcaatgtggacccaagcggtcattgttgcggtcctgatcttcttcgtgacctttggtggttcaagtgccaagcagttctacgtgattttgacgaatatgggaaacatttccacttcattcccgtatatcttcctggtggctgccttcccattcttcaaacgcaagcagaacctggaacgaccgtttgagatttataccaaacggtggatgaccgataccatctcaatcattgttttgattgtcttgatcggcgggattgggtttacggcagtttacccaattttggaacacgattacgtcaacgccttctggacgatcatcggaccaatcttcttcggtctggtcgcttgggcattcttgacttatcaatcacacaaacttcgtaaaaaagcgcattaatattttagacaacaaaatggattcggccgttatttggccggatccattttgttgtctaaaataaatttgatttgagatgaatgtcatcgtccgcagtaattgttcgaatgacccgacacggattgccgaccgccagggaattagcggggatgtttctggtgacaacagaaccggcaccaatcacgctgccagcgccaattgtgacgccaccaatgacaacaacgttgctggcaagccaacaattgctttcaattgtgatcggtttggcgtactcgtcatcgtattcagatccgtctgagcgctgtttgagattgcgatcttggtagcggagtggatgcatcggggtggccaaggtaacgtttggaccaaacataacgttgctgccaatcgtgaccggacagtcgtcgaggattgtaaggttggcattaccatagaagtggtcgccaatcgttgtataaatgccgtaatcgaagaaaattggcccttgaaggtaaatacctttatcggcattggggagcagctcagccacaattttggcccgttcttcggtgtcctcgtcaaaggtatcgttatatcgtttggaaagtcggtgcgcttggtgctgttgagcagctaagagtggatcggtgggatcatatatttttccggctaacattttttcttgttcagtcatagtgtcctccaaattagtgttatacccagtatagcgtatttaactgtggtagcgctaccacgaccgaaactgttatactgattgtagctgattttaggaggtgtctccatgattaatccggtaccactttacaaggagatgttccaacagatggggccacagcactggtggccggccgattcgaaaatggaaattgtgatcggtgccatccttgtgcaaaataccaattggaacaatgtcgatatggctctgacaaatttaaaagatgagacgcatttggacgtgaaacagattttgaacctgccaactgaaacactgcagtcattaatccgccctagtggcttttacgtcaacaagacccgcagcctccaagccgtcctcaaatggtttgatcaggacgattgcaactttgccttaatggcagataagtataaatccgatttacgtcggacaatgttaaagctgccaggagtgggggaggaaaccgctgattcgctgctggtctatgtatttgatcagccggcgtttattgccgacaaatatgccagaacgctttttacggatctgggatttcgcaatcttggcaattattcgaaacttcaaaagagaatttggctgcctgaatcatttacatatcaggatgcccaggaattccatggcttaattgacgagttcggcaagcggtatcttaagagtcggcgtgattttgatgccagctttttgggtggttttgataagcaccagcttgatcggccatgacagataatcttgcgaattagatataggagttggttagatgaatgtactgttgatgttgctgccggcagttggctgggggcttttgggaccagttgttgcccgcatcggtggcaagccagcaaatcaaatctttggaactgccgttgggacgctcttggtggcagcggtgatgacgcttttttatcatccacacctttcagtgccgacatttttagcggcagtcctggctggaagtttctgggttattggtcaagtcggtcagttcattagttttaaaaatattggggtatccaccaccatgccaacttccaccggattccaattaattggcacttcactggtcggtgtcgttatctttggtgaatggtcgacgatgatggaaaaactgctgggtgcaggggggatcctaattttgattgttggcattatgctgacatcggtcaccgataagccactggttgcccaaaggacaccgcaaaagaagctgccaactattctgatgcttttgatgacgaccttgggatacgttgtgtatatggccattcctcggggactgaatcattcgggactggcgatcttcttcccagaagcaatcggtatcctgctcgcggttctggtctatgttttcgtcactggtcagcagcggattattaaagagccagtcagctggttgaatattgccggtggactggtcttctccctgggcgcaatttcttacattggttccgttcaggcgaatggcgtcaattcagcttttgtggtttcgcagttggctgtggtcatctcgacgttgctggggatgatttggatgcacgaaacaaagacgcctcgtgaactggcgtttacaatctttggtttgttgctgattgtctccggtgcggttataacgacagttttttgaccacaaaaaaatgcgctggaaccggaattccaacacattttgggcaaaataaaagaccctcacaggggtctttatttattttgatttaattattcaacaacagtaacgttagcagcttgtgggccacgatcgctatcttcaacgtcaagggtaactttttgaccttcttcaagggtcttgtaaccgtcagcattgatagctgagaagtgaacaaaaacgtccttgccgtcttctaaagtgataaaaccgtaacctttgtctccattaaaccatttaacagtaccttgttccataagaatgaaacctccgttgcgcatagcgcgataaattttgcatttgaaacttgaaaagtaaggagtcattcttattagaacgatggaccttgtttcgaagctaaatacattatctacactttaacaggtcatcgtagaaattgcaaatataaacgctcatcgactctttttacagagaacttggcttgagtgggctataatgaaattaacgttaatgtcgaaaggggatcgtcttatgagcaaatcagttaattggaaagccgccttaattgccgggggtgttgccggcgttatttccggtctcgtcaaattgggctgggaaaatgttttgccgccgcggacacctgaacggaataaaaccaacccgccacagcgtttacttgagcaggccggaattcctgaacaggtgactcacgcaacttacacctattccgatcagcaattaccatgggtcagctacatgatccactttggtttttcaacttcgtttgcaatgttttacagtctggccggccattatgttccggtaattaaaatgggcgacggcacattgtttggtctcggtgtctggggtgcctttcatttgggcatcatgccggcaatgggcacggttccgtctgccaaagatcaaccggttgaggaacatgtgtcagaggctttgggccacgttgtctggatgtggaccaacgacttaattgccgatgaggtttatcacaagttaaccaaataagtttaattcaacgggtcaacacaaaagaggtcggatcataggcaatcaatgcctacgtccgacctcttttcaatttaatgattattttgattctgctaattgttcttttggtgcatcagtggatttaatttcttctgaatcttcagtcgcttcagagacttttcgattgcccattaccagattaataatgatggcactcaaagcggcaatcgtgattggtgaaccgagcaggtactgaaccatttgtggcgtttcgctaaccaccttggctggcaggagaattacagccattgtcaagacgattggaatccctaaaacataaatggaactttcatcagtggccagattacggataacgttcaacccattcagcatgatgatgacacaaatgatggagaagattccgccaatcacagcggcaggaacagctgacaggaaggctgataatttaccaaagaacccaagaacgacgaaccagatcccagctgagacgaagacacgtttgctggcaacaccggtgatcgaaaccaccccggcgttggttgagtatccggtcattggggttgtcccgagcagggcggcaaacagacagctgagtccttcaccaatgattccgcgattccattgtttcttggtgatcttttcaccgacaacggcactcattgcgaaccaggtaccggtggtttcagttgtcaataccatataaatcactacgaaggttaaaattgccggcagtgagaaatgaatcccgtaatgtaatgaagtaaagtggggcagactgatccaagccgcgttgttcacgactgaccaatcgaaacggcccatcatcgaagcaacgatcgtgccgacgatcaaagcgataatgattgaactgactttgaacaatcgttgaagttgggggatgcggatgccgattgtaatagcgaccaacattgccaaagcggtgatggcagcaatttcaatgttttggttgacgtttccggctgccttgaagatattgtcattcaaagcggatggtaataacgacaggccaacacaggtgatgatggtgccgccgacaattgctggaaccaatgtgttgataatcttttggtagacgcctgaaacgccaagcagaattaataacaatgctccgacaatcaaagatcccaggacagtcgccatcccgccgttagcggcaccgtttgccaagtagaccccggcaaccgcaccaattggcacaaatgatgggccttgcgaaacgggcagcttcatgaagtaccgggtttgaagaattgttccaatcccgcaggccaagaaagccgcctgcaagaagccggtcttctgtgccagactcattgacagcagcccggcgatgatgatcggtggcacgtaaacatccatggccaacacatgctggagtcccagtaatcctgattggaaatatgaaaccttatcatctggaccataaagcaaaccgttatcattgcgtttcattaagaattctcctcaatttgttaaatttcggctaaacacgaacattaatttaaaataaaaataaataattcgcatcgctagttaatgtttagtataaacactagctttgtaattatcaacaataattcgaaattaatttttgactttaatgttcgtgtttggagtccaaaattgaacacgcaagatgatgattgtcatagtggggatgaaaccgttatccgatcaaataatcattgaccaaattatcattttccacattaaaaaagctgaaattcatcattgaatttcagcttttaatattgtgaagcattatctggcaagggacttgaccaacgcgtcgatgatgtgggtgatttctcgctgctccagaggttgattaaacaataggtaaccaatgatgacgccaccgacaaccgaccaaatgattttgagaatttccaagttctcccagttgacgattaaatggttgtctttgagttgattcaaatttttattgatgttgtgccaataaaggggagggaatttagtcagcagttcttttctgacagtctcattatataagacctcggagacaaaaattttgaggacggctgcgttgtctttgagaaattgaattctgtcgcggaccaatgaatcaacaaaggcatgtaaagtgacaaattgtagggggagctgatcagtcttaaattcggtgaggacggcgggaaaaatcgagttgatcaccggttcgatgatggcattcagtaacccgcgtttattcttgaacttactaaaaatatttccctcggaaacgcctgccttggtggcaatttctttggtgcttgcgttggcataccctttttctgcgaatacttcgattgctgccaataggattttgacctgcttgtcggtcattgcatttagcacgttggcatcagcaaataattttaattcggtaccattcagcattcagtgtggctccttactgtgcattgaatttaaatttcagattaagtatacactcaatctagtattttaaaagtcgcttagctgattttcatgtaaatttttgataaatgccatgaaaacggcttcttgaaaacttttgagagtaatggttgacctttatatctccgtgtgtataataagtgttggtaattgactgagtaactactcaaacaattgcccgaattcaaaccaatgaaagagggctaatacatgcgagagagtgtggaaatgaaagaacctaagaagaagtttttcagtagtacagaagatgctggcgacagcaagagcttagatgaggttaacggtagtatcatcgtgccgcaagatgcaggattttggcggacgttgataacttataccgggcctggaattctgattgccgttgggtatatggatcccggtaactggatcacatcaattgctggtggggctcaattcaagtacagcctgttatcagtggtcttgatctcaagtttgattgcgatgttgttacaatccatggcagctaaacttggaatcgtgaccggaaaagatttagctcagttgacccgtgaacgtaccagtaagcgagttggatttatcctttggatcatcactgaattagccattatggcaacggatgttgctgaaattattggttcagggattgcgttggaattactgttcaagattccattagtagttggcattttgattaccagtgccgatgtgttgatcctgttgctcttgatgagattaggcttcagaaagattgaagccattgtggccaccttggttgcagtgattttactggtcttctcatacgaagtattcttggcaggaccgaatatgcctgaactgttcgccggctatattccttcaacatcgatcgtcacgaacaagtcaatgctctacctggcacttgggattgttggtgcgacggttatgccccatgatttgttcctgggatcatcaatttcccagacacgtcgggttgaccggaagaatcgcaaggatgttgccaaagcaatcaagttctcaacgattgactccaacatccagttgtcactggcatttatcgttaacagcttattgctggtattgggagctgccttgttcttcggtacgaacagttcagttggtcggttcgttgatttattcaacgctttgcaggattcacacattgttggcgccattgccagtccaattctgagtatgctgttcgccgtagccttactgtcatccggacaaagttcaacgattactgggacactttcaggacaaatcatcatggaaggtttcattcatctaaagatgccactttgggcacaacgattgattactcgtctgctttcagtcacaccagttttgatctttgccatttactatcatggcaatgaggctaagattgaaggattactgacggcatcacaagtgttcctgagtattgctttaccgtttgccatcatcccactggtcatgttcaccagtaacaagaagttgatgggtgagttcgtcaatcatacttgggtcaagtacgctgcttggtttgccaccattgtgctggtaaccttgaacgtttacttgattctccagacggttggcttgctgaaataaccgtttaaagacctttataaaaaataagtaggtttccgttatattctttataaaagtgtttagcagttgggagtcgttgacaatttaaaaatttgtctgcggcttcttttcttttagtctaaaatagaggttaataactaacagggggattactaaatgatcaaacccgaaaagacaatcaatggaaccaaatggattgaaacgattcaaatcaatgccgaagaacgggcaaccctcgaagatcagtatggcatcgatgaagatattattgagtacgtcactgataaagatgaaagtactaactatgtttatgatatcaatgaggacgaccaattattcatctttctggcgccgtatgccctcgacaaagatgcgctgagatatattacccagccatttggcatgttgcttcataagggtgttttattcacgtttaatcaaagccacattcctgaagtcaatacggcgctttactcggcattggataatcccgaggttaagagcgtcgatgcatttattctggaaacattgtttgcagttgttgacagctttatcccaatttctcgtggcattaccaagaaacgcaactatttggataaaatgctgaaccggaagacgaagaacagtgacttggtttcactttcacatcttcaacagacattgacctttttgtccagcgcagttcaaaccaatctcagtgaactcaatcgtttgccaaagacccattttggtgtcggtgctgaccaagataaaattgatttattcgaagacgtgcaaattgaaggagaacaggtccaacgaatgtttgagattgaaactcaagtcgttgaccgaatcgatcacaccttcaacagcattgccaacaataatctgaatgatacaatgaaatttttgacaatttggtcactgaccatggctgtgccaacgatcattaccggattctatgggatgaacgtgaaactcccgttagccgggatgcagtatgcttggatgctgacgctggggatttctgtcgctttgattgtggcaatgctgattatgctgaaggtccggcggaagatgtgatgggtgagtggtttattgctgggtggaggatttttttggagtgtgtatagttgagcagttatgctattttgagcacccttcggcctttaaaacacgctccgacgccccagggcccggccacataaacaaaaacttccaacgatgaacaagaaccgttcatcattggaagttttcgcttatgttccgacggccgaaaacggtctagcctacctggtgggccctaaacgggtctcgtcgcgctctggcgcgtttgtcatgctatcttgagctcccttcggcctttaaaacagactaagcttgtgatgaattaaaacccgacggggctttagttcatcactttttggtataaagtgattgtgaagttagtaatgccgtgagcatatttggcgctggacgccgtctctaaaactggctaacttcactgttcttatacaaatctgctctaagtctgttggcgtttaacgtcgtgtattgaaaattagattatataagacttgaagcaacaactttaaaggtaaggtgatattttatgcgagtaacgtttggaattgatgtcagtaaagcaacttcggaaattgccatagtcgttaatgggcaagcggttagccattttaaaattacaaataatcagccgggatttaataaactccaaaaaagtttgaatgactttcaaaaccctgagattgtttttgaagcaactgggttatattcaaggagattaagagtgttcctagatgattatggttaccgctacactcaattgaacccattagcctcaaagaagcagcttgatcgactccgtcctaataagactgacaaaaatgatgccttacacttagctgaaactcagtttgagatcaggcgtgctttaacttatcagcaagatccaatataccagcagttacttgattggagtcgcttttatgatgagattacttgtgactcagtcgcaaataagaaccgacttcataaagcccttcagtgtacatttcccgaagctgaaggcgttcttaacagtccaacagggcacttatattggcaccttttacaagcgttcccgattgcgagcatggtgcgacaaagtagttcaatggaactaagtcagcatatcagaaagttctgccagttatctgtcccaaatagccaagctttagccgctcggctacgtcaattagcctcggagtcctatccttgtgttggggaagactctggagtggttatgcaggtccgttatttggcaaccgagttacttagattagatgacttgaaaaatgacatcattcaaaaaatggctcgattagctcaagacttgccagaattggccattttggaaagtattccaggtatttccgttaatacagcagtccgcctgattggagaactgggagatatccgtcggtttacgagtgccaacaaactgaacgcgtttgtcggcattgaccttagacactttgagtctggcgaatatatcgccgtcgatcatattagtaagcgtggtaatccatatgcccgcaaaattctgtatcgaacaattctcaatatgatggtaagtgctcgcacaaagccatcccacatcaatgattattgccgggaaaggaaaaagcaatcttctggaaaggctgatttcaagaagattgccatgggtgcaattagtcgtcttaaccggactatttaccacttgatcctaaataaccagaaatacgattatctcaaaactcgaccaaaagctgagtcataaatctgattacgataatcataccagccttgtaaaaaatattaaattgttaaggcttatttagtttaccctcaaagccactttacctaaccagaaaaacaattaatttacggcacagccatgcccgacagaaaaagaatggtcttaaattgccggtataacttgactataggtagaaaatacgctccgacgaccctgaccccagaacataaggcagaacctccagtaacgaacaaaacccgttcgccactggaggttctgccttatgttctggggtcaactcgggtctcgtcgcgctctcatttttaccatttctttaccgaatcaataccaagcaaaaacattacccttctatactaaaagtgttacattggaagttgcgagattgacaatgttgggagggttttacatgaaagaacaaaatgaatcatttgccgcttcggccttatcagaaggagcaatccccgctgccggggaggccaccaacactttttccgttagtcagcctgctttgcgaaccctgaaaagtgtgaaagaacatgaaatccacttgcaaggggctttcaacgtccgcgatatgggcggctatccaaccaaagacggtctggttgttaagagccacttactcctgcgatccgccaggttgaatgctttaacctccgcagacgtcaacacacttattaatacttataatttgggcgtcgactttgatctgcgtcgccccgaagaagtcagtgagttgcccgaccgttttttgccgggcgtgaaatacattaacgattccgttgatacccgtgagacttactattatcacattaatgctgaaaacaaccggaagcactaccggacttatgtcacgtccgaacatgcaagaaaggtctatcacaatttatttatggctttactggagaagcctatggggaaatcgctcctctggcactgtgcatctgggaaggaccgcaccggtgtcgctgcttctttgatcctctacgtgttaggcgttgattccaggaccatttttaaagattacgtggcctccaacgattttctcaagccacggattgacgcccgaatcgcccggctcaaagaaaagggtgccacccgttcagaaattaagtttgcaaaagtcgatggcggtgttgatttgtcctacttgaaagctgcgatcgatgaagttaaacgtgattatggctcggttgctgatttcatcacaaatgggttgcacattaccaaagaacaacaggcacgactacaagaaatgtacttggcataacaattgaataggtgttgaatcaggctattgggcagttatcgtccgatagccttttactttactaaaaaataatgaaagaataaccgatcttttcaggaagtacaataaatcctaactgacatatcaatttgcaaacctatgtaaatcgtccacactaaataatataagcgcatacaacgttgttccaatgcaggaactaatggtatagggaattaaaaccttttgccaaaaatattttagtaaaagttaggaaaaacatattgacagcgctttcctatgacgttattataaagtcactgatatataagtgttcaaattttctcaggacgttcaaaatctttgaatgtcgcaccggcacagacatacagccatttattatcaaccattatcaattgctgggtgaactttgggaaatgaatgcttttatatttgaagtgaaatgtaagcggttaatgccgttccaccgactaatcgcttatcgcatgattgaactgaggaggcgtgaccagtaagtgattgattgaagtttgcgtaaaacttttggtaccacaataatattttatcgggagtgaaattcatggctaagaaagatgaagaaaaagacgctgtcaaaacaactgttggagttgttaccaacgccaaaattaaggatgaacaacaacccaagctaccttggatgatttcatccgcaatgtttttagcaccgctttgttggtatggtccaatcggatcaactcgaagcgtgttaattccgcaattgtttgctcaattggatccggcacataaagtttgggcagttggtattttggcaacgattgcctcaattaccggtgcggttaccaacttactgtttggtgccctttcagatgttacccggacacgatttggtaaacggaaaccatacattgtcttaggaacgattgccatcgcgatttcgttggtcttaattgccaacatgaaatcaattgttgccattattgccatttggatcgttgcggcagcggccgaaaacgcaattgccgcggcgatttacccgcagatttctgatcgggttgcgccaaaatggcgtgggacggtttctactttctacggtgttggctttaccattgcccagcaagggtttgcgttgttagcggcccagttcctcggcaacgttaaatttggtatttacttcatggccggatgtaccgttattttggccctgatccacgagctgctgattcaagaaaagggtaatttggacgagcctaaagtcaagtttgacaaggacagcctgaagaaatatttcttcttcccaacccatgatgcccgcgacttctacctggccttatttggtaagttcttcatggttgttggttcaaccattgtcacgaccttcctgctgttcatctttaccgactacattggtcaaagtactggccaagccggaacatcaatttcaatctttagttcgatcatgctcttcatcggtgtcttctttgctttggttggtggcccacttgccgataaacttggtcgagttaaagccccagttgtgattgccaccttcgccttgggtgctgccgcattattcccactctttgtcaaagaaccatgggcaatgtttgcttacgctgttatcgctgcgtttggtaatggcttgtacaactctgttgatggtgccttgaacatggatgttttgccatcatccgatactgccggaaaagatttaggtttgattaatttggccaacacattaggtcaaatgcttggtgccatggttgcttcagcaattgttgaagcctttggttacggcgcaatctttatcttcgccattgggatggaactgattggtggaattgcgattgccatgattaaacgggttaagtaatcactgtttgatgaaagaaggataaataatgtctgttaattcagaagattggaaacaagctttacagtccaaagacgcgttcgccgattttatttacgattacttcaaggaccacaaagatttaaccggaaactatgagactcccagctattacgagtactacgttgtcactttggatagcaaggaaggcttgattatcacattgaagactgggttaaaccaaaatactggtgatatcaatgcgccgctaccattcaaggatgttgaacatatttcagtcgaagacttccgtcaactggtcttgaacaagaaatttgaagatcaaagcgagagtttgactgacgtattctccaagatgttagcttcagagcccaacgcccgctttaaccgcggtcaagatgggaaatagctttgctcaaatgaattagaatcaggtcccgtattttggggcctgtttttttatgaccgattaaatatttagtaaaattaatgaaatgtttaatgaataatctaaatgtttattgacaaaatactgtaaagcgcttacattagaattagtgttcagactaagcaagaggagtgtgataaattcatggaaccagacattaaatggttagacgatcctgaaactttcagggtcggtatgctgccagcccacagcgatcatcaattttatcagagtgctgatgagattcgaaatgatcacagcagttacgtgcaaagcttgaacggccagtggcaattcgcctatgccaaggatccaatgcaccggatcaaaaacttttacgctgctgattttgacagcggtgactttgatgcgatccaggtaccacagcatattgaatttgccggttatgacgattttcactacattaacacgatgtatccctgggaaggcaagatataccgccgtcctgcatatgcacttgatcaaaatgatcaggaagccggtcaattcagtgaagcagtcgacaatcctgtcggccactacattaagaaattcactttgaactcagcattcaaagataaaaaggttcgcgtccgttttgatggcgttgaaaaggcgatgtatgtttggctcaacggccatttcttaggatatgccgaggatagttttacaccgtcagaattcgatttaaccccatatcttcaagacggtaagaatacgttggccgtggaagtcttcaaactcagcacggcgacatggctggaagatcaggacatgttccgtttctttgggatttttagggatgtttccttgattgcccaaccagaagcccacattgaagacctgtccatcaaaccaaccttgagcgacaatttgaaagatggcactttgaatgtcaccacaaaaatgacagttaacaaatcgggtgccaccgccaaagtgtcagttaccgatgcagacggcaatgaattgtacgcggattcccagccggtggatgacgccatcactttgagtgatgtttcatttaaaaacgttcatttgtatgataaccacgatccatatttgtatcagttgacgattgaaattgatgatcaagatggcaacgttttagaaatcgtgccttacaaatttggctttagaaaaattgaaatcaatcaagacaaggtcattacccttaatggtaagcgcttggtcatcaacggcgtcaaccgccacgaatgggattgtcattcaggccgggtggtttccgttgacgatatgaaagccgacattcgaactttcaagcagaataacattaacgcggtgcggacctgtcattatcctgatcacacgctgtggtatcacttgtgtgacattaatggaatttatgtcatggccgagaataatttggaatctcacggtacttggcagaaactaggtgcagtggaaccatcttacaacgtgcctggatcggtcccgcagtggaaagctgccgtgatcgaccgcgcccgcaacaactatgaaatgctgaagaatcacgccagcattctcttctggtcattgggtaatgaatcatatgccggcgatgacattgcggcgatggaacaattctacaagcaggctgacccaaccagactggttcactatgaaggggttgttcaaaaccgcaagtatgaagatgtgatctcagacgttgaaagtcggatgtatgcttccccagacgaaattcaagattacctggatcataatccgaagaaaccattcctcttgtgcgaatacatgcatgacatgggtaactcacttggtgggatgaaatcctacattgatctgattgacaagtatccaatgtacgctggtgggtttatttgggactttatcgatcaggcaattgaagtcaatgacgaagtcaccggccaaaaagttctcagatatggcggcgatttcgatgaccggatgtctgactacgaattttccggtgatggattaatgtttgctgatcggaccgagaagccggcaatgcaggaggtgaaatactattatggacaacacaaataaacaattgcacttggtatatggcgatggtggcctcggcgttggcggcgccaatttccattacatcttcaattacacccgcggcggcatggaatcaatggtcgtcgatggtcgtgagtggatgtatcgtgagcccaagccaactttctggcgggcaaccaccgataatgaccgtggtaatggtttctcgaaacaagctgttcaatggtatggcgccgatatgtttgccagtgccgataaagtcgatattaaaattaacgaccagttgattgaatttcccagtgcaccgcggaataatcagtattccaaccatgaatatgccgacaaagtggaagtgatttatcattttgcaaccctgacaattccaagtacggatgtcgaggttcattatacggtgacaggtgatggtgtgatcagcatccatgcccattatgccggtaatgatcaattgccggatttgccagtctttgggatgcgcttcattttgccaactgccgcaaccggctacgaatatgctggcttgtccggtgaaacctatccggatcgcatggctggcgggattcctggcgagtatcgaattgatggcttgccagtcaccaactacatggttccccaggactgtggggtgcacatgaagactgactgggtcacagtgacccgcaacgccaccaaagtcagctcggatcactcggatacgccgtttagcattaaattcgaaaatgatggcacgccgtttgcctttagctgcctgccatatacggctgaagagctggaaaacgccactcatcaagaagaattgccactgccaagacggacagtcgtttcaatcttgggcgcagttcgtggtgttggcggcattgacagctgggggcgggatgttgaagagcagtatcacattcccgcaggaaaagatattgattttggttttaagattacgaaagcttaattgtttgtagagtgggactaaaggcgttttgatcccagaatttaagagcacagatcgattattcctggttttggaatgattgatctgtgctcttaactggccgggatcagccgattgccatgtaggctaggcaagcatgctggccgtcgtcgcacgtttttgataaataatatgggatcacaagaaatagaggccgaggcgaaagtgtatacttttgtctcagcctctttatttaccataaagcacaattgaattaggaaaatcagtgccaaatttacttgtgttttagtaaaatatgcagtatgattaacactgtaaaagcgctttcaaaatacaatgatgaggtgattttaacattgaaacgaaaattatttaatgaacaaattaaagacaacccactccgcagtaaagcggatgtcaaagctgccttggtcgacattttggcgcctgccatggaagttttggcgcaacaaaaacgaaagggccgcttccggatgagtgacagtggggccgtttacctccaagacaagaccgaagtggaaggtttcatgcgcctgctttggggcttagggccattctttagtgataaaaagcgggtatacgaacgtccagactggtacgagttggtgacgcaaggcatcttagccggaactgatcctgatgatcctgattactggggcggagatcttggtgactatgaccaggtcttcgtggaaatgggcgctttgactgccttcttgtatgaaacaaaagattatttctgggataatttgaccgttaaaaagcaaaaaacgattgtgaaatggatggatcaggtgaaccacaaggtgattccaaagaccaactggttattcttccgtgcgatggtcaaccaatttatcactgattctggttacatggataattcagagttgatcgatgctgattatgcgatcaccaataaacattacctgggtcatggctggtcctacgatggttatgtcaaccagatcgataactacattccgtttgcctaccagttctttacgatcctaacggttggcttggcacacactgataataagcaaagtcaattattgaaagaacgggcccagaaatttgtcccaagttatgccaactggtttgccgctgacggggcggccctgccatacgggcgcagtttggattaccggtttgcccaggcagccttttgggcagcttatgcctatgcgcacgttgatatgcctgaaggctatagcctaggtgatatcaagcacttgctgttgaacaacctgcgttggtggttccaacaaaacatcttccaaacggatgggttgattccaatcggctatgcttatcccaatatgaattttgctgaaggttacaacgggccggcttctgcttactgggctttgaagacctttatcttctttgccttacctgatgatgatccattctggaccaccaaagaaagtgatgacttcaagtttgaagctttgaagaagcagccggaacctagaatgctgatcgctcacagtcaaaatggtttggaagttcaatcattcaccgccggccagcactcccacgaacatgcccatggtgaagccaagtatgagaagtatgtctactcaaccacctttggtttcagtacgcctaaaggatccgttcttttgaaacagggtgcttatgataataccctggcagttgccgaatcggaaaacttctggcaaaccgccttcaagtacgatgattacgcaatccacgacaactacgtctactcagactggaagccgtacgatgatgttgaaatcaagaactttgttgtgccggcaatgccttggcatgtgcgggttcatgaagtcaatactggccgagagcttcatttggctgaaggcagtttctcagcccctgatagtggagcacctgacgaatatgaaatgaaaactggagtggataacgccatcttctatcattcaagagtcggcattaccggattagtcggcttatcaaaggaattgacaactgaattgtcaacgccggaacccaacaccaatctctacttcaataagaccaagattccgctgcaaaccggtgtcttggcgccaggtaagtacaccttgatctcattgtatcttggcgatcgtgagcttgagagcctggatgatgatggcaatattgtgattccagaagtgaagttggatggcaataagctgacaatttcatttaatgatcatacggttagcgctagtttcgatgaattttaataataaatattgaacctgatgggcttcagattttctggggcccattttttgattacgggtaactaaccaacgtccactatgtcaccgcaaagaaaaccatagttatccaaaaatagttaaatgaaccaaaatgatttggttggttatttttatgattttttgggaagtggggttgtacattttgtactttgccccatggaacgcgtttccgtttattcccgatctggctacattggtgacaggaaggaaccgggccggcctgtttgcctccgtgatgacctttgttaatcaaatcagtgtcggtgttgccggtgtggttgccggatatttgctggactttgcctattttcgggagtcggcaagcggggcagtccttcaaccccagagtgccattaatatgattatctttatcgtatcgggtggcgttggcttgatgatcgtcttggcaatgctgtttgtcggccgctttcatctcagcaagaagacattcatggttctttctgcagaacttgttcgtctgcaaaagggcggtagtatgagtgatgtggatccacacaccaaggcagtctgtgaggatttgaccggcgttaaatatgattcaattgaggtttggaagaaagatgaccaaccgcaaaataaatcacggggttagccgtttttgggattaaatctcctcaagtcgatttgattgaccacaacctgcttcgggtagatacttttgttgaaataacaagttatctatttggggaggattcacatgacaaatttagtgattaaaaaagacgttgaatatgattctgttaaccaccagttaactgacatttattatgatggtgaaaaagcccaaagcaaaggcgcaatcattgatatccatggtggcggctggttccgcggcaacaagtctaaagatgaggattcctcgatccggtttgtggaagccggctacctggttgtaacgccggcctatcgaattacgccagcggctttttatccggcacctttggaggatatggatcacttgtatgaatggttaaagaaatccgacttgccgttcaaccacgaccatatcggcgcttttggctcctctgccggtggcaacatgaccgtcgaattggcaatcaaatatggcattccgattgcctcgctatcgggcattttggatattgataagtggttgagcgaacatgaagatgtggttgctgcagaaggtgacaccagtggctttaactcaaccgccagctcgaatattaaccagactggggccaacgatccgttttataagtggtttgtgaccaactactttaacggccggaccgaccaatacaccgaagccactccggttcatcgagtaaccgaccagactggtcagatgtatttggccaattcactgaatgaattcgtgccaaccagcggagtcttggatatggcccaagcgctgaccaaacaccaaattccttatcgaacccgaatgttaaccggtagtcgtcacgctaagggatacctggatgatgtctgggatgacgtggttgggttctttgctcaaaccttataatgcggtacacttaataggagcgcggtgacagctgtttacctggatgaccaggttcagctggtaactgacgtcatcacgaaataatcagtgtacgcaaaagtggccgaaacgaaagttttgcttttgttcggccacttttatacataatgaaacggggtcacaatggatgattaagaatagaatgtcttggggaaaggaattctggttggcagccctttttctggtcctcttgatgggtgtcgacttttcggtccggggggcaggtccgctggttcgcggtggtgcccgactgatttttgccctggtcgttgccggaattgtcttctatgtactgggaacgatgaaaatttttcagactaaaatcaaattggggacttttgccaaaatctggggattcatttttggcatttgcttgggtggattattcctattgattagcattctcggtcacacggctttgatgatgcatgccaaaacggtggttgccgataccatgatggcattgtcagcgggaatctttgaagaattcttgtgtcgggggttattattctcggcattcctgtcggcctttaaacagaccaaatacaaatttaccgaggccgcgttggcttccggaatcttcttcggcctctttcatttcatgaatttgatctcaggacagggctttttaccaacccttcaacaggcgacctacgcttttgtgattggcgcgatctttgcatcaatcaggttgacgaccaataccttaacctgggtggtcctcattcatgcgttaatcgattggcagccggggatttcggtgactcatacggttagttcactggcgtcgtggctggtttttctggcagtttggggaacgattctggtcgtgaccgtgatttttctgatttcgtttgatattagttctaaacgacaactgtcgttaagttgacgacataataaaatgcggctgaacaaaaggatcaccttttgcccagccgcattttgttgaggaaatttttaagctgctttgatctttaccaataacccaaaaccttggttaacttggcacgattaatatctcttgaggataatttatcctggaaaatcgcgtaatcatcgttgacgactttggattgactccacgagtacttggcgtcaccgctcttagttcccgaatcagcttccataatatcattggaatacggggtgtgatccagacccaggctgtggcccagttcatgggtgatcactgatttccagtaggtgtcatagagtgcctggtaatctgcactgtttggctgatcagctgatggcagtgcatggccggtctctgctttgtagacggccggcaggtacttggtgttgtcgaagaaattatagttgatgtaaagcttgctggtaatgtaataaccatcccagctgccctgaccggttccagcattcttaaagcccactgtaatcgtgtggtcggctttggtgcctaatttaaacgctttggttttgagggccttgttccaattctgcatcgcggcgtaggtataagacttcaatgattgattggccacgtagacctttgccgtatgatttttgaagatgccctgggcactcattggctggacattgtaccagcggtcaaagacctgccaatatttgtcatagatataagcggggtatttgcggacacttgatgttggattcaaatcaggggtgcttttaatggccttggcaaccgttttgccggcaatccgctgagttgatttggcataagtaatcggactttgaggcatgttcaacgtcaatggcaccgttaaagcaaaggtggcactggcgactgcagcgagaatgaaacttctttttttcataaggaaccctctcttgaagttacataaaatcattttgcctgaataatagcattccaatcaagatcgttcaagaaatcttgcttcaaaccaagcggtcttaatgaaggcttatgaattattgcaggggatagactaaattgtaccaagtttccccggcatgactggatgctgaaatgccttcgttttgatagtcattgctttcataaaatgggatcaggtctgccagacaggtcagggtgatggccactcttccctgcgctttggcaacctgagccaattcagctagaagctgactgccaatgccatggccgcggaaatcgggatggaccgccaggctgaggaccgtttgatacggatcatctcgacggttggcgtgggcctgttcaaatagttcatctgtcagataccgttgtgaaaatgccggaccgacgatgtaaccgactacttgattggcctcatctgttgcgacaataaatgtgtccggatacaaccggattctttccgccatcgcagttttggtggccgcttcggccggagaaaagcccgcttcttcgatcaccataattgctgctaattcatccatccttgccggttgataatgtaatttcaattcggacctccattagcttgtggtatcattaattgcgtaccattttattaataataattatcataacacgataggggtcttcacaaaatgaatcattcaaatatcgggcatcgtaatcgcggggtgatcctgatcgcagtctttatcgcgacgttcatgacttccgttgaagtgaccatcgtgacgacggcactgccttcaattattagcgaacttcatgggctggcttatcaaagctggattatgagtgcctatctgttgacgactgcgatcacgacaccaatctacggcaagttggccgatacgttgggccgacgaaaagtatttcagtggggtgtgaccgtcttcaccatcggctcgcttttaagcggattgtcaccttcgattttattcttgatcgtcgcccgggcaattcagggaattggggcgggtgcggtcatgccactgacgtttacgatcatcgccgatattttttcgtttgaacagcgggcaaatgtgctggcactcaataatacagcttggggactgtcagccctggtcggcccgctaattggcggttttttagtggaccatctttcctggcactgggtattcttcgtcaacgtgcccttgggcatcatcgtcgccctgctgatctggctggggtatcaggaaaatattgagctcaagaatcagctgatcattgattggctggggattatctggctggcaatttcactggtgagcttattgctggggattcaggcattggacacgctgccgttggttgcaggcagcctgttggtagtgacgattgtggcaacttggttattccttcgccatgaaaagcatttcgcagacccgttaatttcaccaaaaatgtttcattccaaaacctttacgattcaaattatcacagcaacaattttgagtggggtcttaattggttatcaaatgtatttcccaatttggctgcagtcgttgtatcgggtatccgcaaccactgccgggttagtcgtgacctccagctcaatcatgtggctggtcgcctcgttttttgttggtaaattgattgcccgctttgttcccaaacaaattgcggtgacgttgattggtgtgatgctgctcagttatttatcactgatctttgccagtcaagcatttccggtctgggcattttatgtgattgccatgattaatgggattggtatggggatcgttgtcagtatgaatacgattcttagccagcatttggtccccaatgaaatggtcggttcggcgacttcagtcctaacccttggccgttccttgggccaaacggtgatggctggggtgtatggtgcgatcttgaatttagtcattcgattgcagttgcatggcggaatcaccttttcaagggtcaataacgtcattagttccaaaggggcagccgtggtggccaatcggtcgctgattgatccaatcatcctgacagcccttcatatggtgtttgtcggggtggtcgcgatgttggtagttgtcttggtaatcaatattttagatcctaataaaaaaattattcgttgatagttgtggaaattagcacgaaaaaagaggtcggacatttgttccggcctcttagcgtattgtgccgttcaaaagcaatcggcgttagcgggcaatttgatttgcccagcttattttgtggatcctggcaccccggcaaccgtctgaaagacgtcagccaatgaggtatgcatgtcagcgaatttcttgttgaggataagctggcggaattcttcaaccgagatggtttcaacatctttgaaaggaattgtcggcgcatcggcgttaaccgtcggattaattgagctgaccagggtgatcactaggcccttttcactgttcaaggtgacagtatagtactcatagtatgaaggtgtttcgtaattaccggtcagttccttgtggtccttaaaatagttgatgataaaatcgttgaatgcctttggtgattttaatgatgctttccaatctgtgtttgtcatagtcaaacttcctttcgtgtctcaatcaatttcaaaatggggtaagcggcggacaactaacatattagagctgatttttctctcttgcttcaattgttattctaaacactcctcaaattaatacaagtgaaaacatcaatgaaaacgttgacagttatgcatttgttttaatttgttgattggaagcgttattttcgccggaatgagctgaatcatcaaaaaacaccactgatatgttagtatcctgctgggagtttcatagatcaatacgcgattggcttgctttgtgagccgttttgtaagaacataacagcatagattcagattttttcgagaaagtggtgataaaatggcaacaggctatattggtcggattcgaaaacgcgtgggccacatgcctttaattttgaatacggccgctggaatcctattaaatgatcagcaccaagtactcttaaatttaagaaccgatagtcataactggagtttgccgggaggctacatggagttcggtgaaacttatgcccagacttgtgtgcgtgagtatcaagaagatagcggcgtaaaagttgagattgtccggccgctcggattgttcgaccagggaatcttcacgtatccaaatggtgatcaggtgcagacgattgatcggttgtttttagttaggaaagttggtggccaattgttgtccgctgagactgacgagaccattcgactggattatttcgattttgatgacctaccgccactgctgaatcagcagacggaaaagatgctggcatttgccaaagaaaatgcatagggggacttgatgatggctgataaagtactcgttccggctcaattgcatccggacggaaaacgttatttacgtgagcacggcctggaagtcgtggaattgatgcgggctaacgctgaaaatattttgaagaatggcaaggatgctgccgcactgattttatttttggatccagtcggcgagaatgtcatttctcagatgcccaatttgaagattattgcccgtcacggcgtcggctatgacagtgttgacttggacgccagcgccaatcacggtgtttgggtgaccaacacgcccaatgccaatgcagcaacggtagcagaaaccactttggcagaaatcatggacgtgtctaagcacatcaccaaaaactcgatggaaatgcgggatggcaactttgcatacccgttggctcatttgggattcgatcttgaagggaaaactttggggattcttggttacggcaaaattggccgtctggtggccaaaaaagccagtgcgctggggatgcgaattttgattcataaccggaccccgcgggaatcaccatacggggaatttgtcgctctcgataccttagtgaaatctgcggatattttgacgctgcatctagctgccaattctcagacccgacacgtcatcggtcgaaaacaattagccgagatgaagccgaccagtgttttgatcaacttgggtcgtggtgctctggttgataccgctgcgctgattgatgcgcttaaaagcggctcgattagtggtgctgctcttgacgtctttgacgaagagcccttaccgatgaacagtgagttattcaaattgaacaatgtgttattgacaccccacattggttccagtacggttgaaagcttttccagaatggccacggatgcggcaagtgaagtggttcgggtcttgaatggccagcagccacagtggccggttaaccaaccccattagttttctggaaaatttggataaatacattgtacgcaacctatatagcgcgtatagttaagttggatcaacaaattatacaagggaagcgtttctcatgacaaaaacatacaaagcagaaattacttcattgaatggcgacaagattggtactcatccaactggtgaggcaacatttacgattgatggcgatacactcaccgttgaaattaccatggatcatacgtcaccaaacacccaacactggatgcatttccacggtttcccagatggcaaggatgctcaaccggcaacgattgctcaagacaccaaccatgacggctatgttgatctgccggaaaccgaaccagtgtccggaacgacaatggtcccgtttaacgacgccccagagaagatggatatcccaactgatacctacccaacttctgatgcggacggtcacttccactacacgaagacagtcccgttggctgaaatcagcgagaagttcaaggaagtctttaatgacgacgacctccaccttgagaagcgggtggtttacattcacggggttccccagtcgatggatttacctgataccatccaaggtgccgttggtaaatatgatcaacatacgacgttaccgattgccgttggcaagattgttgaagcctaaattaattaagatctattcagaagttgaaatgattcgactactgaatagatcttttttgattgcttcctccagccagcagcaagtctgccatttacgatcgttttggcaattgatgcacaggtatacaggcttaagaatgtttgagataataaaattgatcatatagaaaagagcgccgattatggaaaataaattcaatcttactctcaaacaaaatcgctttcttacgaaaaagaatcttgtcaacatggtgtattccaattcaaaatttgagggcgttaatacgaccctgccgcaaaccaagacgattattgacggcatgagtgtcgctggtgtttcgattgatgatattcagatcatcattaatctcaaaaaagggttggaatttgtattaagtcacagtgaaccatttcgattagatatttgtcggcaaattaatcgaatcgtcgcggccgaagatgccctcgtccccggacaaattcggactggaagtgttcagattggcggtgttcagtacgtaccgccagttccagaagccagtaatgtcaaaagcgcaattcaagaaataatgggtgatgatcagactgccactgaaaaagcgcttcaaataatgtatgagattatgcggcagcagatcttctgggatggtaacaagcggactgctattttgtctgctaattatattttgattaatgccggtgccggaattgttaatatcaatgaaaaccaattagaaacctttaacacattactggccaattatgacgaaactggtgatttacaggccatcatgcagtggacatacgataattgtttatatggcattgaatttcaataactgtcatttataaccaattcagccccaatcaaaaattcttcgggatttttgattggggctgaatgatttgattattcaaataagtagttagttggcggctttaaattctttaatcccttgttgcagccggttcaagccatcttcaaccatggttttcggactggcaatattcatccgcaggaagtggttgccatcaccgccatagacgtcacccgccgaaagatacaggccggtttgggttcggatgaaggtggctaattttgctgagtcgtcggtcagttggctgacgtcgatccagaccagataggtggcggttgacggaactacgacaatttcgtgaatgtttgcctggcagaatttgacgaccatttcgtaatttgcccgaatttggtttctcagttcatggacccagtcgcctgccttggtataggcagcaatggtgcccggaattgccaagaggttgggctcgccgagttcatcggtgttaattccccggttcactttgctgcgcagggcttcgtttggaacgatgaccgttgcggcgtgcagggcggcaacattaaaggttttgctgggtgagacgcagacgatgacgttttgcagcagatcacttggcaacgagaataccggcgtgtagtcagcgcccttaaacaccagatcaccgtgaatttcatctgacagtagggtgacgctgtgtttgaggcaaagctgattaattttaacaagttccgctttggtccacactttcccaattgggttgtgtgggttgcacaagatcatcatggtggtcagcggctcggcaagtttggtgtccaaatcatcccaatcaatctgatactggtgggctttttgatcatagaccagatcggatgacaacacatggcgaccattgttcacaatcgaattatagaaaatattgtaaaccggcgcttgaaccaggacgttatcacccacattggtgacgcggcgaacagctgaggatatcgtcggcacaacgccagtcgaaaagaacatccaatcccgtttgatagtcgcatgatgttccgtttggtaccagtgggcaactgcatcaaaataatcggtgtgcggttcctcgtatccgaagatgccgaagtcgactttttgacgcattgcatcgagaatttccggggcgactttgaagtccatgtcggcgacccacattggcagctcattaggtttgacatcccatttaactgaatcggtattgcgccgcgaaatcattgaagtaaagtcatacattaggctgtctcctttttagaagttttgttatcagtaatgatagtcgttttacttggatcgactttggtagggtcaatcataacctcaccgattgaacgggcgtgaatggtgccgctgattgggttcttaacactcatgatgttcgagttgatttctgcgtcaatgtcagaacagtattcaaatgccaaatcggtccgcagtaagcggcagttacgcatcgtgaggtgatcgatgtagcataacccctgatcgctttcaatggtacagttgatcagcgtgaggtttttcgtattccatgccagatattcaccgttaattgtggaatcgacgatcttgacgttttcgcagttccagaaagcatctttggacacgagagttgaatgatggacctcgacatttttggcaccgtcaaagacatagttgccaattagattcagatggtcaacggaaatgttttcactattcatgccaaaataatctccgttggcctggacgttgttgatcttgatgttttgacagttccaaagggtttctttggcgtcggaaaagtggtcgttattcagcgtgatatcactgcagcgcctgaaaattttgggtgcctgaatcgcactgtcgttgatttcaatgtcgtgagtgtaccagattcctgaacgagccatggtttctaagatcgagtggtcaaccttgacgtgtttgctgtaccacagtgggtatttgtaggtaaaaattgaatcggttaagtgaatgttgcgactttctttgagaggggattccccggtgccaaatgtggtgccggaaatgtccgcgttggtttcggcaaacagtggtcgttcaccgtcaaaatattgatttgtgtattgtttcattatgactccttattagtttgattaattgattgttttctgaaaaggacttaatttcagtatactcgtttccaacaaattggtgaccgggatttaaatgggattggtttcactataaactttgaagtggactctaagtcaagggcgtttcagcgataacttttgattaatgtcatcagtaccaataaccactgctataatgtaagtggaggtgcagattatgacaacaatttatgttgacccttccaaaaagaaggaacagatcgttaaactgtctgatggcacgtttggtttgatgaaagctgaaaagcaaaagtctgggattggttatgagtttgactttaccagccacatgcaccccagcttcagaatcccgcatgcaccggttaatggggatgaagaaaccgttcattcgattgacggcgagcagcagtttaagattcagtggttgagcaagtgatttttcagttagcaggcagcttggctgacagatttaagggactaaatcgattatttccggcttgaaataatggctttatttgcttaaatactgactggttgtcgaactcgacgttttaactgagaatccggctgaattgaatcaattctcactttcagggaggctgagacaaaagtatccgcttttgcctcggtctttatttcttgtgatcccatattatttatcaaaaacgtgcgacgacggccagcatgcttgcctagcttacatggcaatcggctgatcccggctatttaagagcacagatcaatcattccaaaaccaggaataatcgatctatgctcttaaattctgggatcaaactccgttatcctcactctcttttttacgaccattttttcatggttcttattcctgttcacttatcgttttggccttataatcaaggtgttaagaatcagctatctggatgggaggcattattatgcgagcagcatatattacacaaaatggcgaggcaaaggacatcaagattggtgagttgccgaagcctgaaattaccaatgatgaagtgttaattaaagtgaatgcggtggccgtcaaccatgtcgacacgtttgtccgttcgggatcttttaaaaccgataccaattttccgtttgtgatcggcagggatgccgttggtcaagttgaagaagtcggggctgacgtcaccggtttttccaaaggcaactgggtttggaccaacagcatgggctatgccggccgccaaggagtgaccagcgagtacgccgccattcccgcggccagactattccatgtgcccgaacacgttgagccgactcaattggtggccgccgttcattcagcagcaactgccgcaatcgtgttgaccaaagtgtttggggccgtctccggggcatcaatcctggttgaaggcgccgccggccacgtcggaaccaaatttgtccagatggcccacatcatggggctcaaggtggtcacgacttccaacaccagcgactttgacctgctggaccgcttggggagtgatcaatgtctgaattacgataagtcattaaagaaacaactctccaaggctgaaactcaaaaagttgactatgtagttgatacctctgggcaagttcaactccaggataatttacgggcattgaagccgggcggcaaagtctgcttgattaccgcaccaaagagcaatcaattctcgtttgacgtccgtcagttttacacccagtcaaagacaatcagcggatttgtgatcagcaacgcaccactggatcaaattcaagatgcggctaagtttattaatcggctgatggctgacggctatcttctggaggacccggttttggagaagtcctacgaggatgcagcgtgggctcacaagaagttggaaaagaatgccaagaagaaaaagattctcctcaaattttaataagcaaaacatttaggaaattaaaataaatcagttatactgtacttgtagataggaaacgcttacaaggaggtatgacatatggggaaattagataacaaagttgcaattattactggtgcatctcaaggaatgggtgccagtcacgccaagatgttcgttaacgaaggcgctaaagttgcgattaccgatattaacgcagaaaaagggaacgctctggctgatgaattaggcgataacgttatttttatcaagcaggatgtttccagcgaagatgactggaaaaacgtcattgatgagacggtgaagaaatttggtaagctggatattctggttaataatgccggaatcagttttaacaaaccgctttccgatatcactctcgatgactacatgaagatctttaagatcaaccagctttccgtcttcttggggatgaaatacgcagctgaagccatgaagaagaatggcagcggcagtatcgttaatatttcatcaatgaacggactggttggtggtgcgattggttacaccgataccaagtttgccgttcgtgggatgactaaagctgcagcattgcagttggccggttctcacatccgggttaactcggttcacccaggggtaatttccaccccaatgattcaccaaggtgatagtgaagaagtcatcaagcagtttgcaaaatcaattccgctacaaagagtggcagaaccagaagaagtttccaagatggtgctcttcttagcatcagatgacgctagctactcaacaggatctgaattcgtgattgatggtggaatgacagcgatgtaactgaatgcggtcgtgttgggatgttaacatttaactggattcaaaaaagccgttggacaaaagaaaatcaacttttgtctcaacggctttttagattgtttaatgaccaaacttcaaatgcaacgtataaatgaatttatacgaacgcatcttttcagctctggaatggactgcgtggccgaataaaggctttttggccggttccagttgatgcagctctaacagcattcgagcctcaccatcaccatgaatggcgcgatacttcaattcgttttcagctgctttggcgaccagtgcttccgaccagcaacgcggactgagccgtgtgtataggtcataattgctttcattttccatgattatgtagacgctcccccgaaactcaactatttgtataatgaaatcactatctataagattatgattttttcgccaataagtcaattggggtttgtaccaattcaaaaaggatcaggcaatcattcctaaagggaaataattgtctgatcctttactcaagatgctgcatccacatagtactaagccagattctggttataaacgtaattcatcaaggaccgggtttcggtaaactcgttttcgtcatgcaggacaaccgtgataatccggtcatggcctgacttgcgacccgttccaacgaagcagtaaccggccggatcggtgtaaccggtctttaagccgtcaacgttcagggacttttgataatactttcgtcccgggagcaggttattgtagttgtgaagcgtttgaccatcgaccttcattgatttaactgaagcgtcggtcaaaatatcgttgtaatcaacaacgaagtgacgggaaatttgagcaatatcgctggctgaaacgtaattggcattcttggaagcaccaatactgtaaccataaggagccaaactattctgttccatcccggaagccgaaacaaatgatgagtgcttcaatccccattccttggcttgattattcatcatgccaatgaattttttgttgtaagcaggcgttgaaccgccggcaacccattgtccaagggcaattgcggcgttattggatgattcaatcagacctgccaggtacaactgacgaacagtgtagctgttgtggttgaatttaaagccgccaaagacattggatttacctaatttcttcaaaccggcattactcgtggtgaccttactggaccaagtacccttgccttgagaaatcttttgacgaaccaggtagagggtcatcagtttggaaagagaagcgatgggtcgagcagtgttggcgttcttcgtccaaacgttattattggtattgacatccaaagcgacggctgacttggcatatttgagaccaaatggtgaggtgccggcctttaagtacttgtgccaaacaatgccagaaactgttccggaaccatttttcactttatagtagagtgcttttgaactgccatgcttcaaagttaccttggccgtcgcgtaccaggtggtgtacgggtaggtctttaagtttgcaaccttcttggtgtgtgaagcgttatacaccgcgcccttggtcgaacttttgtgatagggcgtcttctttatcgctgtggttgagacagttttataggaacttgaactggcgttgaccgtcggcgtctgcccccaaagtcccatcccaattgtgattgtggttgcacaggtaaccagtgccagccgcaaaaattgattcattttcatatataatctcctcctcattcaataaaaagtgtaacattcaacctttgcccactttgtctttttaacagaactgtaaaagaactgtttgatcggagtaattctgtgagttctaattaatattggtgaaatagtctggaaatttatcaagcacggattgttgttcactgagcattaaattgagatggctataaaccagttggtgtacctttgccgcatcgtggtcactgaaggcattgataatatctcgatgttcttgggtcagtctgttcatgggcaggttggcgtcataaactctgagcagccgatagcgattcaggtcggtactgaaactgattagccaattccaaatattttgtttgttggcaaactcgtaaatcttttgatgaaaatggttatccatttgaaagaatcgttggatctgatcacgtttggaggccgtttgctgttcttcgaccacagctgacagctgatcgatttggtcatcggacacagtgctaccaattgacttggcgatgtctgattccaacaattggcgggcatagcgggcatccaatgattttttcaggtcaattcgagtgacgtaagtgccgctttggggaagcgagtacagcatgtcgtcccgccgcaaacggagcatggcttctctaacaggggtccggctaaccccaatttcttcttcaaattgtttatcggagacttgttgaccagggtacaaatccagattcatgattttggtatagattgcgttataggccttatcttgtaaactttccatgtcatctcatctttctttttttaaaatcgatccactgagaatatgttaccatattaattattttcctgaatcgtcaaagtgaatgaaatggggcagcagcgactttgaccgggaattttaaaagtgatatattagtagcacattaatggtttggaaaggacgattgtcttgaaaatggggttcagatggttcggcgagcagaatgatccggttcaactggcggagattcgccaaataccaggggtttctcaggccgtcacggcactttatgacgtccctgtcggtcaggtgtggccaaaggatcgaattgctcagctgaagcaagcggtcaccagtgccggtttaggttttgaagtgattgaatcggtcaatgttcatgatgatatcaagactggacaatctggacgggatcaatatattgaaaattatcagcagaccatcaagaacctggctgaagccggcgtgaaggtgatttgctacaattttatgccggtatttgactggctgcggaccgatctaacctatcagttgccggatggctcgaatgccatggcttaccagcctgaaatgttacctgatgatccgaatgaactgattcaccaaattatgtcgggctccaagggctttgaaatgccaggctgggaacctgaacgtttggctcatgtccaacaattatttgccaaatatcggcatgtggacgcagaccaattacgggcaaatttgaaatattttctggacgccatcatgcccacttgtgagaagtatgacgtccgaatggcaatgcatcccgacgacccgccatttctattgtttggcttaccacggatttataaaaaccgcgatgatatgctcaaaattgagcagctgtacgaatcaccctataacgccttcacgatttgtaccgggagcctgggagagaatccacaaaatgatgtgccggcaatcatccgcgaatttgtccaaaaggatcgggcgccgtttattcacgcccgcaatatccgcttcatgaaccagacaaaaacagcattccatgagtctgctcatttgtcgtcggccggatcactggatatgtatgagattgtcaaggcgctggcagacaacgattatgagggttatctccgaccagatcatgggcgaaatatttggggagaacagggacgtccggggtacggtttgtacgaccgggcactgggagtgacctatttgaatgggttgtgggaagcaatccggaagaatcaataggactttggacagatgagcttaattatatttgttttaactatgaacgaggatatattaaaggggttgccggcaaaatggcgaccccttttgttttctgtaaatgtatatcgatttcctggccgaactgtgggaaaatacgcagcttccggccatataaggggattatccaaagatccaagcccgggatttttggataatccccttatactctggaagctaagcgcgtattttcccacgcttatttttatctattaactggattcttccctttgccattgttagaaatcatcgccgccttgatctcggcatctgaagaaaggttaaagtccccagggatggtcagcttcaaaactgcagccgccatcgcataatcaagctgatattgaggattgaaattgtggccgatcccgtggacaatggctgcgccgaatgcgtcaccgccagcgacttctgggagaatctcgacatcgtaaatcggactctcatagaatcgtccctgatgattcatgattcccatccattggctactttggggacgttggatgtttcgtaagatgctggcgacggtttggatgttaggatatttatccgtgaggctggtcattgcctgttgaaaggtagctttttgatcaattgcttggcgattggccgcctgaaaggctttgatgccaaaggcctgctcaatatcttcgtcgtggaccagacaaacatcgacgaatggcaatatccgcttgttaaaggcaacggcttgagccgacgtccacagttttccgcggaaattagcatcgtaaacgacttgaatatcgtgatggtgacagaactcaacggcggatagcaaaaccgcttggagttcggcagacagggcagcggtgatccccgaaatgtagaagacatccgtctgatccagtagttgattccacggataatcagccgcttctgatgttgcaaaggcactggtcgcccgatcataaatcacgtcactggctcgttgaccgacgccttgctggagaaaatacagaccgattcggctgccgccgcgacgaatgcggctggtgtcgacgcagaacgcctttaattttgaaatggcggtgtcgccgatttcgttgttggggagttgggtgataaaggccgcttgatcccccagcaaagccagtgaaacggcaacgttggcttccgcaccgccataattggcattaaacgaagtcgcctgaaccaacttctgattatccggaaccgtcagccttaacatgatctctccaaaagttgtcacccgcatcgcaaaaatctccaatcgttatcattacttgtatctgtataataccatattaattggtgccaaaacgcgcgactgatgcggacgttgacacttttaaactgattgtgacagaattaattgagataataaaaggtccggccactcagttagagaaggccggaccttatttagatggttattgatttgatgagttatccgaatcgtcattggattcattgtcggattgatggcttgaatcgttggtggttgtgggttgatttccagaagtggctgccggtgtaacattgattcgatcggcttcttgatggacctgcgcttcgtgttcatccaccaactcacgatagaaattggcaaaactgagttgcatataaggctgaacccagatggccgcaatccccagggtaatgccaaccagcaagccccagccaatgaagctgagggccattacaaaataatcccacttatggccgtccattaattgacgactacgggtaatggcatccaaataactgattttttcgccccggtcaacggcatcgcggtagatgtataatgcctgggagtaggcgacggctttaataagcccaggaatgattaacagaatcatccaaagaataatcaaaacctgctcaatgatgtaaatgacaatggttcccaagaaatagtcaacgttgtttaagatggtcatcgacttttgcaggggctgatcataggtcaacttttgtcgcatcgcgtcgatacagataaaggcgacgccaatcgcgaccagagacccgagcagaattagaatcatgccgaaagtctgagcaccggtccagattggttcaccgttaatatcgtaaagctcttcttttggcgcatagatatagccgccaacaaattcaagaataaatactggtaaaaatagcaaaaagaaaatttaaaatgagcatttaataggctcttagagtctagttttaacgcttttctatccataatcacaacccccgtcaatttaaaatatctttacaagttaattatagtgcaacctgttgaattcacttagtaaaacgtcctttatgcttgcttactcgtctggataagatcatccaccactaatttgtacagcagtgacttaatcgccattgattggtactgtttagctgacaaatgatcagcgtccacatcagtcagctcctgattgaacaggtcaatgaactgatcataagctttgggggcggagtcgagtttgagggcaattttcattgcctggtcgatggtatccagcgataaaattggtttgagcagactcaccaccagtattttggccaagtgaacccgtgagtagcgcttcttggtcgggcggtcaaccaggccttttttaacgtaactgttgatcatggatttggtaatctcagtgtgggtgattggtgccaaatattggttgacctcgtcaatcacttgatccatatacaaatccaaattaggtaaatcttcaaagtgcggcatggtcatcgccgctaattttttggtaaaattatctttagtcatggtattccccttcgaattgaatactagtattattgcataggatagttgaaaaataaagtacgtagactttaaaactatgttatcttgacttagaaaatagaatagcttattatgatgctaaggaggcatcgtgatgaatgaattaatggctaaaaggcgtcatcaacaaattatctatgaggtattaaatgctgtcacccacggtgtttcgttttttgtggcgatttggttgtccattttattagtgaacaaagctttacgtgatgggctttcaatgggggcaattgtcagcttgatcatctacagtgcgacagttctctcactctatttggcatcaacgttgctccactgttttgttttcaccaaagccaaacgcgtctttcagatcttggatcatagcaatattttcattttgattgccggaacgtacactccttattgtgtcatttttgtccacaactgggctggcaacattctgttggccagtgtctgggtgttggcaattggggggattatcagccacgtggtctttcatggcagatttcagaagactgaaaccaccatttatgtggtgatgggctggttatgtatgttcttgggcaaagcgctatatgacaatttgagcaccaacggtttttggctgctggttgccggcggcgtgacttttaccgtgggagcattgatttacagcattcccagagttccagggatgcacttaatctggcacttcttcgtgatgggcggcacactgaccatgtttctctcgattttctttaatatttagatattatcaaattaggcttgacttatttctcagtggtggtaaattacatgtatcaacaaattaaaaataaataataaacatgaagttacgattagaaaagtaattgcttaactcacataaagagagccccgctggtgagaaggggatgtgagtggcagtgaacacacatctatgaactggttagctgaaccaagtaggctatcccgctagtgagcgttaccacggctactgtaactgttctccaatttggacgactagttacgagcagcgtaaggtcgtttttgtaagaaaacgatgaacgtgaggtggaaccgcgaaagatcgtcctcagatattgcttcggcaatgtctggggacttttttatttcataggatttgattgtaatgaatgtttggttatctgaaatggagagtggcttatatgcaaattattgaagattccttagaccaattattgaaacaggttgccatcaggacgaacgccgttgccaaccgcgaagaagttgaaaaatcagtgcgggaaattatcgccaatgtcatcaaagatggtgatcaggcagtgaaaatgtacgaacagaaatttgataatgtcgagctggagagtttgaaggtcacccagcgggaaattgacgatgcctatgaagcgactgatgacaccgtaattaaagccttggaacttgccaaagccaatattacgtcatttcaccaaatggaagtggaagatagttttattgatgcgaaaaagaaaggcgttattcgcggcgaaaagattgccccactggcagctgttggactctacgttccaggtgggacggccgcttatccgtcttccattttgatgaacgtcattccagccaagattgctggggtttcacgaattgtcatggttacaccaccacaaaaggacgggttaaataaagcggtcctggcggctgctaaaattgccggcgttgatgaaatttatacggttggcggtgctcaagccattgccagtctggcctacggaactgaaacggtgccacgggtggataagattaccggacccggtaatgtgtttgtcgcaactgcgaagaagcaggtgtttggtcaggttgacatcgatatgattgccggcccctcagaaattggcgtgattgccggttcccaggcggttcccagccaggttgccgcagacttgttgtcccaggctgaacatgacaaattggcccgaccaattttagtcaccgacgaccgttcactcgccgaagctgtcagcaaggagatggatcgtcaagttgatttactgcccagaaaggaaattgccaaagcagcgatggaaaatgaaggcttcattgccgtcgtagacgatattgacgatgcctttaccctgatgaatgccgttgccccggaacatttggaagtccaattacccgatgccattgaatacttgaaccaaatcaaaaacgccggctcggtcttcctcggattttcagcttccgagcccttgggcgactacctcgcaggccctaatcacatcttaccaaccgggggcacggcacggttcttctcgccgcttggagttcaggattttgttaaacggacacaatttgtttcctatactagggatgccctgaaaaaagaaaaggatgccatcacgactctggcacgggttgaaggtctcgaagcccacgccagagcaattgaaagccgctttgacgattaaagtgtaaaaggttgtcgtgagttcgtaacattgtttacaaaaatagtcatctgccggttgattcagtgaaaactgatcaaacaaatagtttcccaattcagtgccctattgcctttgacagaacctttttgtcaaaggctttttctgtaaagtaattgtagtcggatggaaaaataacttttcggtaatcgatgatatacttgttataactcatgggaggcggaataatgaaacaattcaaaatttttatgtttgcactggcaatcgttttcggaattcagttagcagctcttccagccaaggcggatgccagcacttcaaccacgacccccaaagcattgcggggcacctggtacgaatatcgtggcagcggtaagtttaatgtcatcaagattaccacgcacagtttcaccaccaatggcaaatcttacaccccttcaaaaaaggatgaccgtaagcttcaggtcagcaaatggggatcttggtacctcttcaataaatcaaagtcttcgaaaaaagacctgggtcagtacaagaccactaagaagttgattggcggatcctacaagaaagtcttaatcaagtatcatggcattggcacttatcatgtgtttccaaaccataaatatgaacacaaatattcctacactgtcttagactgatgagacggtctcttcgaagcggtttgttagaatttcgttacctgatcatttataataaagacagatattataacaaacgacttcgttaggaggcccgcgtatgaaaaaagcacttaccaccgggttgctgttattcattctgccgttgggattgtttggctgttcgaatcagtcaaataattcgagcagtgaaagttccagcagcacgaagacagagcagtccagctcgacgacttcttcaactactaattcggcatcgacttcgacgacgattactcacgccaagcgggcagtcaaagtccgctatgaaaaggccaattttacaaccaccttggaccgggagtatcgggaagaatatttgtatcagaatgtcccgggaactgttgattcaaacaaagtttattcgtgggataacttaaacgtttcagaaaacaccaaggttcacgtcaatcaaaaggcgattgcgaccttcaaagatgacgatgataacgagtacgatcatgaggatttctatcgaattacgttgggcaatcagtccggcaagcagtattgggtaggcgatgatgtcctgcaaaacgatcatgaaaatgactataatgactgatgattcaaacagcttgcattttattttgattggttgtattctattaccaatcaaaaaaggaggtgatgctttttgaatagtggaatatctcttaaggcatcagctgtggagaacgaattaaaatagttgatgcatttgagaagggaactcgcaaatagtgtgcgggttcctttttagatcgtgacgagccccgggtgaccccggagcacaaagaaagccagccaatgatgaacgatctttgttcatcattggctggctttctttgtgtagcaggggtcaggggcgtcggaacgtattttaaaagccgaagggaacaggaaataaaataacaaatcttcatcccggtgaatcaaacacacgttagacaaactatattacgtcaaggaaaaataatgactttattgaagtttattaccccatttttgagcgtataagaaataagcttcaaaaatagttattttttgaatttgataattacatggtttttaggcttggttaatctctaatcaccgtctcagaccatgggtcattgtattttagaatgtggtaaataattcgaactagcttcttgactacatggcttaatgccaccaaatatggtttgccctcagacctctttttctgataatacgctcgcatggttggcgaatacattgcgcacagtctggctgcttgaaagagcgcccagcgtagctgcgttgaaccgtgcttaaccatgtgaccgtagttaccttgcatttcaccagagcgaatgattgagggctcagcaccggcaaatgccagaatctggtttggtgattgaaagtagttcacatttctaatttcggctaaaataatggcggctagtgtttctccaactcctggaatcgataggagcggcgtcttaatccgattcataattttgtggatcttttgatcagcttccttgatctgctgggtctcaaattgtagcgcatcgatcaactgcaggagttgaaatgaaagactatcagatgcttgaccaatcgtttctctggccagttcacgaactttaattgccatttcctcgccatgctgcttcatggagtatttggtaatgatgtttgtcatcgtgttgattcgtccatgagccaacttatctgttgacgggtatctcttcaaaagtgccaacaaccactgactgtactttgcggatactggccctagatttggcgccaactcaggaaattcttggtcgaggacatttgtaaatgcgagcttggtttttactcgtttacgcttaagtccttccagatagcgggtatcactcttcaattcaatgatatcggcgtctgcttcaaagctaaccttagtggtatctgaccttagctttttggcaatctccaacgcatcttgtggatctgtttttgtgtgacgcaaggtattggcctggatatactttttgattagtaatgggttgtaagcaaacacttgaaacttgtgctgtcgcaaatagctgatcaagttataaccataatggccggtattctctaatcccacttggacttgaccatcagccgtccgcgcattgtcaagtgtcgcttgagccgtcaaaaaaccctcacgattatttagaaattccagatcagctaatagtaccgttccctggtcatcaataattgatagatgatgctcatattttgcaacatcaattccagcataaatcatcattaccgctcctcacgtatgtaattaacgctgtgctccacaaatctcttgccctgtattcttgcattaaatgaaacatcatatcttgggatatgtgttatcaaactaatcaacagtacaacaaaagactgtggttagagtctaacgtaaccagtatccgttaggatccgtacctcagatggactaatccacagcgcttaatatcagtttagtacaaattaatgttaccttgctgacatctttaatatacaagcatcagttgcgtcggagcatagctcaaaggccgaagggagctgaagctaacagaacaaccgcaagctctattgaatcgatgcaaatgcaccaaacatcacgtacgaactttgttcatcgttggctgtctttttgtgtagcaggggtcaggggcgtcgccgagtaggctaggcagcctccaaatgcaaaccaaaatattacaaccacattaaatcaaacatcctcagaacttttccctgaaaaacgctagataatttctaccaaaacctgtagtatgaaaaagttgtgcttttcagaaatcaataaaggggatgagaaatcaatgaaaacattcaagtttcaaagcttcgttttagttcttattgcatttgtattggggttcagtgaattcctaattgtcgggatcctggatgacttgagtcaccaattcaacgtgtcggttgcgactgttgggtatctggtcacggcatttgcgattgtctatgccattagtacgccgttcattacaatcctgattggaagattcaatctattctgggatttgatggtcgcaatggctgtcttcacgtttggcaacattttaagctttttggcacccaacttcttaatgctgacggtgtcacgagtggtcactgccatggtggccggcgtgtcgatctcacttggcttgacctttgccggttatgtagcgccaatggctaaacgcggctggctgttatcttgggtattttccggtttctcaatcgcctcggttgtcggcgtaccgcttggaacctggatttcaacccagtttggttggcggatctcgtttctaacggtcattgtgatctcagttttgacgatgggcctcatttttgtcagcctgcccaaggacttcaaacaaaagaagagtaccatttccgggcagctggcactgttgggcaatcaccggatccaaatcggtatgctgctgccaatgtttaacctggccgcaatctacgtcttctacacttaccttcggccaattattaccaatcaactgcatttttcagtctcaatgctgaccattttgctggccgtctttggaattgccaacattattggtaaccgtgccagtggccgcttaagtgaaggtcctgggatgaaagggatgccgtttgtctatattggccagttcattttaatgatgctgatgccattagtcttcaacttcagttggccgggagcactgcttttgacgctggtcatcttcaccataccgttgattaattcgccaattcaattattcttcttgcaaattgctgaaaaggattatccacagtcgattgtgttggcctcgtctctgaattccattttttctaatttcgggattgccttgggatccgcgactggtggggtgattgtcagtaacctcagccttgacgcggttggccctggtggcgcagtctacgccgttgtcgctcttggactggtgttgtggttgaaccacttgacctcgaaagggctttcatctcgctccactaacctgtaaaatgtgattgaatacaaaaattttggtgggtgagaatatgaatggatttatcggtgagctgtttggaacgtacgtgttgattgtgctggggactggcgcttgtgccggtgccaaccttaagcaaacttacgccaaaggctcaaactggacgtttatcagtgtggcttggggaatggcagtaacgatgggggtctatgtggcctcgtcactggggtcgctgggtcatttgaatccggcagtcacgattccttatgctatttttggcctctttccctggaatcaggtggtgccgtatttattaggccaatttctcggcgcatttcttggggctgcgacgatcatgatgatcttttatccacatttcaaaacgacaacggttgataatggcaacacagtcggcatatttgcgacccgaccagccatctattcgccggtttccaattatctatccgaagttgtcgcaacctttgtgtttgtctttgcgctgctaaacctgggagattttacccaggggctgaaaccgttagttgtcggcctattgatcatggtggttggtcttggcgttgggacgaccaccgggtttgcgctgaaccctgcccgtgattggggcccacgatttgcctattcagtcattccggtgcccaatcgtggcagtggtgaatggtattattcctgggtaccgatgtttggtccattaaccggtggtatcattgcggccggcctccaagttatggttaaatagacagtatcaattattttggaggtatttatggatcgtgttggaatgaaattagaagccaaacgtataattggcagtcattttccgttttttgtcttattgttcctgccggcggtgattattcagctgggatactcagtggcttattcggccaaccctctgcacgaggctgataccaaccaggcctttaatcaaattattcagggaactgcccactttggcagtaatgaactgttgaatttgtggctgatttcgactttgatctcaatcatttccggccttctcttgtccggaatgatgtttgtctgtattgacctaattcgtaacaaagtgccgtttgatcaaccagtaaccaggtcgtttaccattttgaatcatggccaatacttcatcggcgcgattatgattggcattatcacgactgtactgacactgttatggtcggtactgttgattgttcccggaattatcaagggttttgcctattcgcaggccttgaacatttaccgggattcagtggatgccggcaaaccgattgggtatctggaagcaattacccggagtcgaaaaatgatggtcggccacaagatggattactttgtcatggaattgagctttattggctggtacatcctcaattcgttcacctacggcattttgttgctgtggctgcagccatactaccagttatcgtttgccaatttttatgtaaaaatcgctcaaatgaaccaaactgaacaatgaaaaatcctcatcattccaattgctggaagtggtgaggatttttattatggctcactaatattaattatcgaggtgccagactgtggcggatcagtccgaaacgcgacttaatcacccagggcttgggtcaaatcgttggccaaatcttttgggttctccaatcctgtcgacagtcgtaggagttcatcggtaatcccaagttttagacgatcttctttggccatgtcgctgtgcgtttggagagaagggatggtcagcagactttcgacaccacccaggctttcagcaaatgaaataattttgaggtgtttaaacagccggtcaacttggtccatgttttgtagataaaagctgatcatgccaccgacgccaggatataggactttttgaacttggggcaatttcttcaaacacgctgcgacatatttagcgttgctggtgtggcgttccattcgcacggccaacgttttgaggcttcttaacagtagccaggaatcaaaggggtccaaagtgacgccggttgtattgaaattgaattccagttcactggcaatttcttctgacttggcaatcacacagccggccaacatgtcgttatgccctgaaaggtatttggtggcactgtggacgacaatgtctgccccctcacggagtggctgttgatacacaggcgttagaaaagtattgtcgacgcagaccaaggcgttctgattggccgcatgaatcagatcagccactttttgaatatcaattattttcatggtggggttggagggtgtctccagccaaactgccttggttttggcagtcaccaagtcacttaacttttcgtaatccttaccgttccatttactgaatttgacaccgtagtggtctgccaggtaatcgaagtaacggaacgagccgccatacaaatcgtctgaggtgatgatttcatccccagacttgaataacgaaaagaccagttggatggccgccattccggaactgaccgcgaatgcattggcaccgccttccaggtcggcgagggtcttttgaaggacgcttctggttggcgtcgataagcgtgagtaggagtactgtttgtgcggatcaaaagtttccgcatcctccaagtcgcggtgccgaaagtttgacgtgagatagatcggggttgaaaccgagtggtactgatcgtggttatctcggttcccagcttgtgcaagtaatgtatcgatatcaattaatttgtcagacatatgctcattctcctttaaattatttcatcaaaaaagccttcatcctaaacgatgcgtgttaacgctgttcagggtgaaggctatttcactttaccacctggcttcactgagatttcacaacctcagcctcattaagtacgccatcttgatggatgggatacttggcaaagtaacgcttgctgacgtcgaattagccaaaccaaaataacttggtgaccgattcggagttcagagatcatcttcacatttttaaccagtcttctctcaccaatcgaagctctctttatcagtttaaaaatgctactcttctcatcaacacttaagtaaattaaaatttacataattgtagaatatatttcgttaaaggtcaacggtctatcgaaaatttatggttagatatttcacaatctggacagttttacactacctgttcacttaaacgatcgcgacaacgaaaatgaagccctgaaatgaagcctttatttacaaaggattgtgggttaatttaaggcttaaaaaaggtcaaacttttttgttgagcctatttacatatttttcacaaggtgttaggatgaaagcggtttaagaatatgaatagtcattggaggaagaactcatgaaagaaaattttgattttttaatgcctagtgtgaacttttttggtaaaggtgttattaaaaagattggtgatcgtgcgaagatgttgaacatgaagaaaccgttaattgtcactgacaagtttcttcggggaatggacaacggtccggttgctcagacactggattcattggatgctgccggcgtttcatacgtgatctttgatggtgttgaaccaaaccctaagattcgcaatattcaagctgccaagcaagtatatttggacaatgattgtgacagtattatcacggttggtggtggttcttcacacgattgtggtaaaggaaccggaattattttgaccaacggcgatgatattaccaaattggccggaattgaaaccttggagaacccattgccaccattgatggctgtcaacacaactgccggaactgcttctgaattaacccgccactgtgtgatcaccaacgaaaagaccaaattgaagttcgttgttgtttcatggcgtaacattccgctggtttctttcaacgatccgatgcttgaattggatgtgccagccgcaatgactgctgcaactggaatggatactttcgtccagtcgattgagccatatgtgtcaaccaaccgcaacgaaattaccgatggtcagtgtattgaagcaatcaaattatgtgaggaaagtttgcgcgaagctgttgccaacggtcacaaccttgaagcccgaaccaagatggtcgaagctgaaatgttaggcggcatggcctttaacaatgccgaccttggctatgtccatgcaatggctcatcaactgggtggtcagtacgatgcccctcatggtgtctgctgtgcaatgctgctgccaattgttgaagagtataacttggtggcatgcccagaaagatttgctgaattggcaaaagcgatgggcgaaaataccgacggcctgtcaacacgtgatgcagcagagctggcaatcaaggcaatgcgtcaaatggccgatgatgtccatattccacgcagtatcaaggcaattggtgccaaaccagaagactttgaactgatggccgagaatgctctgaaggacggtaacgctttctccaacccacgaaaagggactaaagaagaaatcgtccagttgttccagaaagcttatgacatgaagtagagtgcgacgagacctgtttagggcccggagcataagcgaaagcttccaatgatgaacggtctttgttcatcgttggaagcttttgtttatgcagtagggccctgggtcgtcggagcgtattttcaaggccgaagggattacaaaatggcataataaacgcgccacccgcgacgagatccggttagggcccaccaagtaggctagggcgtttccattcgcccgacggagcatatttcgaggattcaaaagttgtcttccggatccacaaacccaaaaaccttccaacaatcttcacactttcttcacaacttggcgagaatattaagataaaattatggtgtagataagatattacccaaaagaatcagaatcaattttcaatattggagggcgtttattatgaaaaagtttgatctggccgatgcggcattgctgctacttattccattgacgatgatcggcttctccgctagtattcatacccgtgatcgcgatatttctaccaccaaggccgcccaggtgaataagattggtgaaaatatcgatacagaatattcaggtgattccgacttaaacaagggcaacatcagaccgctgtattttcagccgtcgcgggtttttagtgtcaagtaccggacggttagttttaaaacggttttggacgaagactatcgggaagaaaaattatatcgttatgttccgggggctaagaaaaacaatcgcacttatcgttggtcaaccattaaggcccgcaccggcaaacgggtttacgttgataaaaaagcgaaagcctactatcgggacgatgacggcgaacgcgaaagtgaagatttctaccggatccgcgtttccgcgaacaagcatgcaacgcgttactgggtcaatgaagatgcgattgacgactgatttttaatccatttagttgaatcgggatgagtaatctttgccaaaccaactctcaaaaaatgaccaattatttcattttgaaatggttggtcattttatttgaatcatgaatcaatttgtggctaattatgataaattagatgtataaaatcgcttaactggaggtgcaatttgaagatattagtaactggtggtgccgggtttattggatcaaatttcatccattatctactcgaaaatcatccgactgatcaggtgatcaactttgatgccctgacttatgcgggtaatttagcaagtttggcagatattcaaaatgattcccgataccattttgttcagggaaacatttccgatccgcaggcggtcgcacaagttatttcaacctatcagattgattcagtcgtcaattttgcggccgaatcccacgttgaccgctccatcttacatcccgatgcctttgtccgaagcaactttgtcggcgtcagcacattactggatgtggtgaagcaacagcgggttaacaagtttgttcaaatttccaccgatgaggtttatggcagctcacgggggcatgagcagttcaatgagtcggcacacctcaatcccagttcgccgtattcggcgactaaggccggtgccgacctgctggccctttcgtactacaagacgtacggcatcaatgtgtcaattacgcgatccgccaacaattacggcccgtttcaattcccggaaaaattgatccctttgatggtcaccaatggccttcggggaaaatcactgccggtttacggtgacggcaaaaacgtccgcgactggctgcatgtgtttgataattgtcgcgcgattgatgccatcttgcgtcatgggcggccaggcgggatatataacattgccgctcacaattacgaagaaaacattcaaattgttgcaaaaattgttaagcagttggaattgcctcagtcgatgattgactacgtttccgaccgaccggccaatgatcagcgttactcaatcgatgatgcactcattcgcaatgaattaggttggcagccgaccattgattttgatcagggcatttcccaaactgttgattggtatgtgacacatgaaaagtggtggcgaccgctgttaggcgccgtccacaacagataatggggtgaaatcatgaaaatcggttttattggtactggtgtgatgggcactgggatgattaaaaatttactcaaggcgggctacgacgtcacggtctataaccgtaccaaggaacacgccaaggatgcgcttgatgcgggggccgcttggctggatacaccagccgaagtgaccaagaacagtgaggtggtcattaccattgttggctttccaaaggatgttgaacaagtatattttggtgacgacgggattttaggggttgcccacgctggccaaacgttgatcgacatgacgaccagctcaccacgccttgccaagcagattgccaaagctggggaagccagggacattggggtccttgatgcacccgtttccggtggggatgttggcgctgccaacggaaccttgacgattatggtgggcggctctgaaagcacatttgagaaatcaaaacccgtgttatcggcaatgggcagtacgattacccggtttggcggggctggtcaaggtcaaaatgccaaaatggccaaccaaatcatggttgccgggacaatgaccggaatgatcgagtcacttgaatatgccaaacatgccggcatcgatttgtcgcagatgattcgaacaattaatggcggggcggcagcaaactggagcatgactaattatggcccccggattcttcagggggacttccagcctggatttgctgccaaacattttttaaaggacctgcggattgcgttggatacagctgatgaaatgaacattaatttgccggcgactaaagtggctcgggacctctacgagaagatgactgacgagttgcatttaggcaatcttggtactcaagggttgctcaaggtttatgaaccagataacaactgagtgattttgatgcggccggaagctgcttattggcgcacagttctgctaaataacattcaggcgcaaaacggggctggaacaaaatttttagttttgtcccagcccctttctatccgttcgattatttttgctgatttttgcgttcttttctgctttggttggcagaaaccaggttgatgataactgaaaccaacaaacaaattcctgctaaaataaccaagccgattttgacatcgtctggaaatgatgacttttgaatgaagaaggccaatgcgattgaaatcacaagggcagcatctgccacgatcagtttcggcgaaaatcccattgtactcacacctttcaaaaagcattataacaaatcggctgtccttgtcacggttatttgaaaattttgtctggcaggccaaagttgatataataagactataaatgaaggttaggtgaagatcatggcagaattggacagtaacgacgcatttattgatacgaacaagttaatatttggcattggccaggtgcaacagatcaccggggtttccggaagacaattgcgttactgggaagaacagggctacattcaatccatcagccaaaaaaagggtgcagcacgagaatattcgctgcacactttattctttatctttcacgttactcgatttctgaataacggctttacccttcaggcagccgttgacagagctaaaaaatttgatcgccaattgccggtcctgcgacaattcttgcgcgctcaactgcaaggcgtcaacattgatgatgaccaaagtgtcttggatttcggctacgttgattcctcacacacacaacgaatctatggggtcgttaaagatggtgagacgttctttcgaattgaaaatgttgattaagcatcacatcacttatcgaagcgctggctgtggccagggctttttattgtgcgctcaatcaatcgtcttcgttatcgaatttcttatataagccaatgattgtcttatcttttaattcgactggcttaccatccaacgtgacgtcgacaattttgtaatagtcttccaggtcagggacctccaaacgctgattggccaggaagtcggctgcagacttgtattcaatggactcggtgccgccgccgttttcgtatttgatttttaacatgatgccactttctttctatatagattaaccttattgaacaacttaattttagattgaacatttttgaaatacaactaactgcctttatgaaatttctgtgaagaatgtttgccttttttgagactttaaattcgactgaaaaattgggccatgatatattattgatgaggggatggctgtcgtaacatcctaaaatttaatattgtaatgacgacgtttaattagggggaattgaatgttgaagtttaagcatatttttgttcttgtgttaaccacgttgattttagtgattggtttttctgcattaggcagtcaatccgcttcagcacaaacaatcaaatttaccagcgcgatgcacaccagcaagaatttgacttacaacggcacaatcaagtactacgttaaagcggacgcaaaaaaatattcacctgaaatcacctatgcaactcaaaaatggaataaagcccttggcaaaaaggttttccaacgtaccacctcaatcagccgttcccgattggtcttcaccggaactaataagcttaaccggaattacgcgggggtcgcagaaattaacagtggcgtgattgcattgaacacctcatggatgaatcgatacaatcagcagaagcgccgagcagtgatcattcatgagcttggccacacgtttggcaccaaggatttgtacaattatccaaatggggcactgcgaagtttgtttaagcagcagacgatcatgggcggtaactatgccaccagcattaaatcgtttgatgccaaattagccaaatggacgttgagaaaaaccagaagcatgtcccaaaccgagtttcgccactatcgttcgaatgcgggactctactaccaacagatgcttaacggacagctttaatttctgctgagagaccattgacaagcgattgtccaaacactatgattaacttattgttttatggacgttgacgcagtccggtagtcaattaacttgagaagtcagaaactcagcggtagatgtgagctgagcggttaatcgacgaacatacagctgctgagtcttcaactatgtgagacggatcatctcgttatcgatgaattgagtggttggcgatttttcgccagtaacttgggtggtaacgcggaaaacttttcgtccctgacaattaattttgtcagggacttttttatttaggaggaattatggaatgaacattttggaagatttgaaatggcgtggcgccatcaatcaagaaactgatcatgaaggcttaaatgaattggttaatcaaaagtctgtcgggatttacgtgggaattgacccaaccggcgacagtatgcatattggccatttgatcccgttcatgattttgaagcgattccagctggctggtcatcatccagtcattttgatcggaagtgggacgggctcaattggtgacccaagtggtaagaaatctgagcgggtccttcagtcgatggataaaatcaagcgtaatgaaattgcgctgactgctcagatggaaaaattgtttggagaagacggtaagtttgagattgttaacaactacagctggctgtccaagttgtcactgcttgattttctccgcgattacggtaagttgttcaacgtcaacactatgctgaataaggaaattgttgctagtcgtttggaagtgggaatttcgttcactgaatttacctaccagattctccaggccattgattttcttcacctttaccgacacaatgatgttcagcttcagttgggcggggctgaccagtgggggaatattacctccggaattgatctgattcataagatagaaggacccgatgccaaagcctttgggttaaccattccactattattgaagtccgatggtaccaagttcggtaaatcagagggtggtaatgtctggcttgatcccaaaaagaccagtccatacgaattctatcaattttggattaaccaagatgataatgatgttatcaaataccttaaatattttactttcttgtcacaagatgaaattgccgacttggaaaagaaagttcaaactcaacctgaaaagcgtgaagctcagcgtaaattagccgaagaagtgacggagtttgttcatggcaaagaagccgttaagcaggctgaacatatcactgcagcattattctcaggaaatgtggctgatttgacgacaaccgaaattgaacaaggcttcaagaacatgccatcagttgaggtttcatcagaaccgttgaacattgtccagtggctggtagatgcgactaagattgaaaagtcacgccgtcaggccagagaagacattaccaacggtgccatcagaattaacggtgaacgcattgaagatgttgattacgaaattaatccggcgaagaagtttgatggcaaatttgtcattgtccgtcgtggtaaaaagaagtactttttagcgagagttaaatagaagcaaagacagatcgaacgatgatctgtctttttttagttgacaatgttcatcaaagtcggtatattatttagtgcggcttttgcgagaatgacttcttcgcagagttacaaattttaaaaagtcattgacacacattgcgcgtcatgataatattaaatagttgtcaaaagcgagaaacaagcgcttccgacaactaagtagacctttgaaaactgaacaaaattttcgacaaacaaatgtgcagggcgtttcaattcttcggaattggaaccaaacatttgcgaagtcaattcgtaaaaacaaataataaatttaaatcatgagctatcacaggcttatcattttaaacaatttaagatgagagtttgatcctggctcaggacgaacgctggcggcgtgcctaatacatgcaagtcgaacgcgtctccgttaatgattttaggtgcttgcacttgaaagatttaacattgagacgagtggcgaactggtgagtaacacgtgggtaacctgcccttgaagtaggggataacacttggaaacaggtgctaataccgtataacaaccaaaaccacctggttttggtttaaaagacggcttcggctgtcactttaggatggacccgcggcgtattagcttgttggtaaggtaacggcctaccaaggcgatgatacgtagccgacctgagagggtaatcggccacattgggactgagacacggcccaaactcctacgggaggcagcagtagggaatcttccacaatggacgaaagtctgatggagcaacgccgcgtgagtgatgaagggtttcggctcgtaaaactctgttgttggagaagaacaggtgtcagagtaactgttgacatcttgacggtatccaaccagaaagccacggctaactacgtgccagcagccgcggtaatacgtaggtggcaagcgttgtccggatttattgggcgtaaagcgagcgcaggcggttttttaggtctgatgtgaaagccttcggcttaaccggagaagtgcatcggaaaccgggagacttgagtgcagaagaggacagtggaactccatgtgtagcggtgaaatgcgtagatatatggaagaacaccagtggcgaaggcggctgtctggtctgtaactgacgctgaggctcgaaagcatgggtagcgaacaggattagataccctggtagtccatgccgtaaacgatgagtgctaagtgttggagggtttccgcccttcagtgctgcagctaacgcattaagcactccgcctggggagtacgaccgcaaggttgaaactcaaaggaattgacgggggcccgcacaagcggtggagcatgtggtttaattcgatgctacgcgaagaaccttaccaggtcttgacatcttctgccaacttaagagattaggcgttcccttcggggacagaatgacaggtggtgcatggttgtcgtcagctcgtgtcgtgagatgttgggttaagtcccgcaacgagcgcaacccttattgttagttgccagcattcagttgggcactctagcaagactgccggtgacaaaccggaggaaggtggggatgacgtcaaatcatcatgccccttatgacctgggctacacacgtgctacaatggacggtacaacgagtcgcgaaaccgcgaggtcaagctaatctcttaaagccgttctcagttcggattgtaggctgcaactcgcctacatgaagttggaatcgctagtaatcgtggatcagcatgccacggtgaatacgttcccgggccttgtacacaccgcccgtcacaccatgagagtttgtaacacccaaagccggtgaggtaaccttcggggaccagccgtctaaggtggggcagatgattagggtgaagtcgtaacaaggtagccgtaggagaacctgcggctggatcacctcctttctaaggaaaaacggaatcctgcacattgtcgaaagttttgtttagttttgagaggtctactctcaaaagtggttacgctttttgggcctatagctcagctggttagagcgcacgcctgataagcgtgaggtcgatggttcgagtccatttaggcccatccacggcctgatagttagctatcaccggagtaacatggggaattagctcagatgggagagcacctgctttgcaagcagggggtcagcggttcgatcccgctattctccattgacacgagagtgtcagacttggttctttgaaaactagataatattaattttctgtaataatttttttgaaattgtatttatataatttcaaccgagaacaccgcgttattttgagtttgttaactagaaaaaatcgcaaatactcaattaactttgcatcacgtcgtgatgtacaggttaagttaaaaagggcgcatggtggatgccttggcactagaagccgatgaaggacgggactaacaccgatatgcttcggggagctgtacgtaagctttgatccggagatttccgaatggggaaacccagcagttttaatcgactgttactatatagtgaattcatagctgtatagaggtagacgtggggaactgaaacatctcagtacccacaggagcagaaagaaattttcgattccctcagtagcggcgagcgaacggggaacagcccaaaccaatgagcttgctcattggggttgtaggactgaacatttgagttaccaaagttgttgataatcgaacaatctgggaaggttggcgaaacagggtgatagccccgtaggtgaaatcaatgaccctcagttcaggatcctgagtacggcgacacacgtgaaacgtcgtcggaatccgggaggaccatctcccaaggctaaatactctctagtgaccgatagtgaaccagtaccgtgagggaaaggtgaaaagcaccccggaaggggagtgaaatagttcctgaaaccatgtgcctacaagcagttagagcccgttaatgggtgatagcgtgcctcttgtagaatgaaccggcgagttacggtaacatgccaggttaaggtttaaaagccggagccgcagcgaaagcgagtctgaaatgggcgttttagtatgttgctgtagacccgaaaccaggtgatctacccatgtccagggtgaaggtgcggtaaaacgcactggaggcccgaacccgtgtacgttgaaaagtgctgggatgaggtgtgggtagcggtgaaattccaaacgaacttggagatagctggttctctccgaaatagctttagggctagcctcggacgtagaatcatggaggtagagccactgtttggatgaggggcccgtcatgggttactaagttcagataaactccgaataccattgatttttatccgggagtcagacggtgagtgataagatccatcgtcaaaaggggaacagcccagaccaccagttaaggtccctaaatatatgctaagtggaaaaggatgtggagttgcatagacaactaggatgttggctcagaagcagccatcatttaaagagtgcgtaatagctcactagtcgagtgattccgcgccgaaaatttaccggggctaagcatattaccgagactgtggacttgaccttcggtcaagtgataggagagcgttctaagggcaatgaagccagaccgtaaggactggtggagcgcttagaagtgagaatgccggtatgagtagcgaaagatcagtgagaatctgatccaccgaatgactaaggtttcctggggaaggctcgtcctcccagggttagtcgggacctaagccgaggccgcaaggcgtaggcgatggataacaggttgagattcctgtactagttgatgatgtttgagcgatggagggacgcaggaggctaagttgtgcatccagttggaaagggatgttcaagccacgagtcagtcaaagagttaaatgctttttggcgggttgacaagtggtgatgaggaccgaaatttaagtagggaagcaaccgacgtcacactgccgagaaaagcttctagtgagtcatcaactacccgtaccgcaaaccgacacaggtagtcgaggagagaatcctcaggtgagcgagtgaactctcgttaaggaactcggcaaaatgaccccgtaacttcgggagaaggggtgctgtgcgcaagcacagccgcagtgaaaaggcccaggcgactgtttatcaaaaacacaggtttctgcaaaatcgtaagatgacgtataggggctgacgcctgcccggtgctggaaggttaagtggatgagttagcttcggcgaagcccagaaatgaagccccagtaaacggcggccgtaactataacggtcctaaggtagcgaaattccttgtcgggtaagttccgacccgcacgaaaggcgtaacgatctgggcactgtctcaacgagagactcggtgaaattaagatacctgtgaagaagcaggttacccgcgacaggacggaaagaccccatggagctttactgtagcttgatattgggtgttgacacagcttgtacaggataggtaggagccattgaagccggaacgctagtttcggcagaggcgttggtgggatactaccctcgctgtgtgaacactctaacccgcgccactcagcgtggcgggagacagtgtcaggtaggcagtttgactggggcggtcgcctcccaaacagtaacggaggcgcccaaaggttccctcagaatggttggaaatcattcaacgagtgtaaaggcagaagggagcttgactgcgagacagacaggtcgagcagggacgaaagtcgggcttagtgatccggtggtaccgtatggaagggccatcgctcaacggataaaagctaccctggggataacaggcttatctcccccaagagtccacatcgacggggaggtttggcacctcgatgtcggctcatcgcatcctggggctgtagtcggtcccaagggttgggctgttcgcccattaaagcggtacgcgagctgggttcagaacgtcgtgagacagttcggtccctatccgtcgcgggcgtaggaaatttgagaggagctgtccttagtacgagaggaccgggatggacataccgctggtgtaccagttgcgccgccaggcgcaccgctgggtagctacgtatggatgagataaacgctgaaagcatctaagtgtgaaactcacctcaagatgagatttcccattcctatatggaagtaagacccctgagagatgatcaggtagataggttggaagtggaagtgcagtgatgtacggagcggaccaatactaatcggtcgaggacttaaccaagtagaaatggtgttcaagggcagaaaattaatattagctagttttgagagaacgaagttctttcaaggaaaaatagtgtggtggcgatagccagaaggatacacctgttcccatgccgaacacagaagttaagcttctgcacgccaagagtagttgggggatcgccccctgcgagggtaggacgttgccacgcgattttatggaggattagctcagctgggagagcatctgccttacaagcaggaggtcacaggttcgatccctgtatcctccattccttgagccgttagctcagttggtagagcatctgacttttaatcagagggtcggcagttcgagactgccacggctcattacaattgaatattattaagcgcataatatttgtatgccgacttagctcagctggcagagcacctgtcttgtaaacagggggtcggaagttcgaatcttctagtcggcattttgcggaagtagttcagtggtagaacatcaccttgccatggtgggggtcgcgggttcgaatcccgtcttccgcttgttatgccggggtggcggaattggcagacgcacaggacttaaaatcctgcggtcagtgatgaccgtaccggttcgatcccggtcctcggcatattatgcacccatagcgcaattggatagagtgtctgactacgaatcagaaggttgtaggttcgactcctactgggtgcattgttttaacgggaagtagctcagcttggtagagcacctggtttgggaccagggggtcgcaggttcgaatcctgtcttcccgattgatagcataactatcatttttcatcgcggtgtagctcagctggctagagcgtccggttcatacccgggaggtcgagggttcgatcccccctgccgcgatataggtcttggacctttagctcagttggttagagcaaacggctcataaccgttcggtcgtaggttcgagtcctacaaggtccatcgactcaattatatactggagtttttatacagcttttatggaggattacccaagtggctgaagggggcggtcttgaaaaccgctaggtgggtcaaaccacgcgagagttcgaatctctcatcctccttattatcgcgggatggagcagtctggtagctcgtcgggctcataacccgaaggtcgttggttcaaacccagctcccgcaattttggttcgttggtctagttggttaggacgcctgcctgtcacgcaggagatcacgagttcgagtctcgtacgaaccggttttggctcggtagctcagtcggtagagcaatgcattgaagctgcatgtgtcggcagttcgattctgtcccgcgccacttgtttttaatattatttttgcgggtgtagtttagtggtaaaaccacagccttccaagctgttgtcgcgagtccgattctcgtcacccgctttttcatataatgggcctatagctcagctggttagagcgcacgcctgataagcgtgaggtcgatggttcgagtccatttaggcccatattttggagaagtactcaagtggctgaagaggcgcccctgctaagggtgtaggtcgcgtaagcggcgcgagagttcgaatctctccttctccgttttaaatgacccgttggtcaagtggttaagacaccgccctttcacggcggtaacatgggttcaaatcccgtacgggtcattcaagagaatcttattatattatcgcgggatggagcagtctggtagctcgtcgggctcataacccgaaggtcgttggttcaaacccagctcccgcaattttggttcgttggtctagttggttaggacgcctgcctgtcacgcaggagatcacgagttcgagtctcgtacgaaccggtggaacatcgaaagttttcaagttacttaggtagcttgtttttttacagaaaattctgatccaacacaaaaaccgttaatcagtgaagtcatttgcacttcatcaattaacggttttatttgaatgaacgttttattgagtctttttggtcttagctggtgtgtaataagcttcatgtgaatagaagtttggtgaatcacggtactcttttggaatgaattcatcagaactgttcttccaaagttcgaaatcggcgtaatcatcccaagtccccaaaatgattcgttggctgatgtccttgtgataattaagggaataaattgaatgcatgccatcgggaaggccatttgttcgcagcttgttgattcgcgcatcaaaaaccttctgttgatcaaaattcaaatctaatgtggagaagctaatgaagccgtcccacttatcttcaccactgtgacttaaaatatcatagaaaaccggtgccttgaagactgaatctttacctgaatggtccagcagcataaattcacctggttggctgagagcctggtacatcattaaatcccgatcaggatgcgctgccttgagttctgttaaaattttttcatttccaaatgtaatgacgatctgttcgttcatttgacccacctcctatatacaattttattatactttctttcaatattggaaccaaacatttaccccaaattagcgtaaaatataaattggataaagatgaaagaggaggaattcttttgaaactaacagtgattggttttcttggcggctatccggatcatggtgatgccaccagcagttatcttttggaatcgggtgattttaaattactgattgattgtgggagtggcgcactgttgagcttggaacaggttgtcgaccctctgaaactgaatgccgtcattttgagccattatcatcacgaccacacagccgacgtgggcgtcttgcaatattattggcaattgcatgaaaaacggtacagcgagcccgtattgccgatttacgggcacaccctcgatgagaccaacttcaagggacttacctggccgaaatctactaaagggatcgcctatgatccaagtcaagcactgactgttggcccgttcacgattacatttttcaaaacccatcatcctgttccggcatttgcaatgcgtattcaagaatcatcaactggtaaggtactggtgttcactgccgatacagcttatttcccggaattgacccaattcgttcacgatgccgatcttttgatgactgatacgaacttctttgcggaaaaaaccggccagaaatggcatatgacatcgactgagtccgggcaactcgctcatgacgggaatgttcacagattgctgctgacccacctacctgcagatggcgacatcgagcagttaaaggcggaggcccaaacgaccgctggggaagccatgccgattttggttgccaaaactcatctttctgtggatatctaagccaaatttgcccaaaataaggtctttgtttgtctattctgtgaatcttatgatttatataacaatttccgatataatcaaagcatcaaatgattactaggaggattcacattatgacagtcaatttattaacaacccccagctgcacttcctgcagaaaagcaaaacaatggctcatcgatcacgaggttgattttgtggaacgaaatatttttgccaagccactttctgaagttgaactcaaacaaatcttgatgctgtctgaaggcggtacagatgatgtgatttcgacccggtcatttttgtacgaccagtacaaatcaaagatgtcttcaatgaccatcagccaggtgatttccttgctggcaacccatccagaactgattcgtcggccaattttagtggatgccaaacggattgaatttgggttcaatgaagatgaaattcgttgcttcatgccacggagcactcgaaaatgcgaattggaaaagatggtcaaaaaagccttatagtcttggaatcttaattgcttgttaatattcatgtttagccgtattatttacttagacaataatatgatacaatgttattattaattaccctcagatattgaaaggggtggctaaatatggaaatggaacggattaatgagaatacgattcgtgtgttgattggtaatgatgatctcgacaagcgtggcattaccgtgcttgacttgctgggcaaccacaagcagatcgaaagcttcttctacagtattctcgaagaagttgataaagaccatcaatttcaaaataacgatgccgtcactttccaagttcttccaaaccaaaatggcttggaattgtttatcagtaaggatgtagatatgtctgataacgacatgttcgatgcaggtgactctgattcagatcaccctgaaaaacgtgatcgggtttccaaatatatcgcagaacatgccgataataacaaaccgcaacctgtaagtgataaaaagactaacgatgaatttggtcatcaaaagcggactgtgattcttgagttcgaccaattagatgattttgtgtcgctcgccaaggcattgcgacttgaaaatggcacatcggatttgtacttgtatgaaggaaaatactacttgaagcttgaactattcagcaatgaccccgttgacatggtcgtcagtgatgaagttgcaattgccaatgaatatggcaagaagactgctgttactgaagaggttctcaacgaatacggtcagcagttgatggaaaacagcgcattagagttaagcaggtactatttcaaataaagttcaaccaactaaaaacgacagccgttaatggctgtcgtttttagtatgccgattattgttgatacgcacgtcccttgatcgttgttcgatagtacgtttggcgactattttgactttgtggggtgcgaaaccccaccgttttggaaacgatatacagtggccgtttacgtgatgcctcaaagactcgataaaggtaggcgcccaacatcccaatggtcaatagagtgatgccgaccattaagaatagcgcaaagaccgcaaagtgaatggtatccatcgtggtaaacagcgaggtaaccaagtagccaacactaaatatgattgacaaggttcccagccagttggccaactggaggggaaatgatgaaaacgaggtcacgccatccattgccaaacgaatcatttttcgcaacgggtatttagaagtcccggcaattcgctcttgacgttcgtaagtgacgtcggtctgcttgaaaccgacccagctgaccataccgcggacaaagggatcggcctcattcatttgtcgcaattggtagaccacttgcttgtccattaaccgaaagtcaccggtatccagcggaatattgacgttagtgattcgttttaaacctctgtaaaagagggctgccgttgcctttttgaaaacactttcgccatttcttgaaagccgcttgccataaacgacatcgtagccttcatgccatttgtcgatcatatccacaatgacggcggggggatcttggagatcagcatccattaccacgactgcctcgccttgggtataacgaatgccggcagtaatcgcgagttgatggccaaagtttcgtgaaaattcaaccaaccgaatattattgtgcttggcttgctgattggaaatcagttcgacacttttatcggtggagccatcatcaacgaaaatgaattcaaaggtctgcggttgattggcagcaaagttttccaaggtgttgatggtggtttcaatgccttgctcttcattgtaaaccggtaggacgattgaaattaattcctgttttttgtccattaaatgacctcctatttataaattgacgacaagtcatacagcacgcccgatgaacccattccgccaggaccttgcatggttgtctgtttctgggtagacttactgttcgattgaccagctttttgagtggattttagtttgggattgctcttcgttgaaggcttggttcccggcttaccagttggctttttcttgcccgacggagctcccgttggtgcctggttgctgttaggggctttggcttgtttggtggacttggtggtcgtcgtagctcctgggccacccatgccggcttgagaaccgttgctgcttgaagattgatacaagctggttttgactttggtagcgtgtttcttaatccaattgataatcttggtattccccgatctgccggagtaatagaagtactttaagtcaccgtttttgacgagtttcttgaattgagacaaggtaattgccggatcagttccgttaaagccacccatcgccatgaccgccttcccggttttgatgatgtaaggcgctgcggttgtcgaatcactggtggcaaacagatatttggcgtttccttgatgtttttcaacataattgagcagtttggtgttgactgagctgttacccatgccgccaccgccacccggcatgccgttactgctggatgtgagcagcgatggcccggcggttggaatcatggctgattcagcggcaatcgttggtgttagcgaccaccaggttggagctgccatgatggaaatgagaccgccaaccaacagtgcctggaatgctcgaccccgtggtaaaatcgccatcccaattgaaaagccgattgcggcaattagaatcacccaggtgagccatggatagtaactgtaaacgtaccaggactggagtgccgctgtcgccacgatcgcaatcgggagcagatagaatttccagcaggttcgtaaactgtttttaaacaggccgaccagcgcagtgacgccagttccaaatagtgctgcgattggtggggccaacatgatcatgtagtagggatgaaagaaactggcaacgctgaagaaaccgtagaccggaatcagccagctggtccacaggatcaactgtttttgctgcttggacaggctaaaccaacgtttgcgacggtctctaaagaagactaagccgccaattaagccaaagagggcaaatggtaataaccaactgacttcaggcccgagggctgattggaagagtctaaacggtccggcagtgccgatgttgaaggcgccaccgccaccaccgccgttacccatcttgccggggccacctttgccgccgtttggctggcccttcatttgcttaccgccaggtggggtttggtgtttgccggtttgcttcatgccggtaggggcttgaccacccggcattccaccaccttttttgttggtcgttttgctgttcattccggcaccaaatgtcccgccggttccagtggtttgaccaagcagtcgttcacttccgttatagccaaaggccagttccaacaaggagttggtttctgaaccaccgacgtaaggtcggctgctggcaggggtcatgtcgacagaaattgggtaggccagggtgaagactaagagcgacacggtggccaacgttaatttggtgattttctttttccaggtttcgttggctgccaaccagtaaaataaatacatggctggcagaatcatgaacgcttggagcattttgacgttaaaagcaattccaattaacgcaaagctgatcaacaatgaccaaattttgcggctgccaatggccttttcaagaaagtaaagggccaacattaagaagaaaactaacgtggcatccatgttattggttcgcgaatcagccaccacgatcggtgtcagggttaatgccaaggcgctcagacgagctgcgttttgaccaaagtacggctggatcaatcggtacattagatagaccgatccgactccgaaaagaaccgatggtaagacgatgctccagccgtggagaccaaagattttggcactgattgccatgaaccaaagtgcgactggcggtttatcaaccgtgatgtaaccggccggatcaaaactgccgtaccaaaagttgtggaaactttcggtcatacttttaatggccgcggtgtaaaaggcgtttgcagaccccgccttccagatttgccagccgtagaggaatagcgcaaggacgaggattacgcctaaaatccagtcaaacctgaatttgcgttgataacgattttgggtattttcaatagatagattattggttgccatagtggcggacctcctttaagtgatgttggttgaatacccaaaactttgaaagcaaaaaattggtgggtacggtgatcatcaaactgacgataggaattagtcggctgtcaagaatcggccaaccgctggcaaaatgagcgaacaaaacactgatcagccaggtgaaaatgtaagtggcgtagtatttccatgcaaccgttttaactgaagcacctgtctgaaacacccagcggttatttaacgccaaccccagcagagaggtaatgccgtaaccgattgccatggcaatggttgcgttggttggatgaagcaataacagatagatgacataggtcagcacggtgttaatgaatccggtaatcccaaattttaataattgctttgtactagtaatggatgactcactcctttctgaattgatgaaatgagtttatatgtttaaccataaaacaagcttaaaacatttgatttatgataaattgtgaataactgagttgacggaatgcgtaaaaacctttaatttagtgtcaacgacaaaaggagaacattcaaatgaaagacttacacatactaataattgaagatgatgaggacctggcgaagagtctgcagctgtttttgggcgaaattgcgcaaacgaccgtctcccacgatggctttgaaggccagatgctggggcaggagggaatctacgatctggttgttttggatttgatgctccctcaagtcagcggctacgacattttgaaacactggcggaccgaggaccatttgagcatgccggtgctgatcttgaccgccaaagacaccctggacgacaaagtgcacgggtttgaacttggagccgatgattatttgaccaagccctttcaccgtgaggaattgctgatgcgggtgaaggcccttttgaagcgaagtggccaccttggtgacgacaataccctgtcagttgggccatttaaagtgaacttaagcaatcggattgtggaagttaacggcaaagagctggcactgaatggaaaagagtttgacctgttggtctacttcattcaaaatccggataccatcattaccaaggaccagatttttgatcggctctgggggtttgagtctgaaaccgcgatttctgtcgttgaagtctatatgagtaatttgcgaaagaaaatcaagcagagctcatcgcttcagccaatcaagaccttaagaaacgttggttatatgtttgaaacggaggaatcggattgaaaaaaggtgatccgcagcaaaaacaacagctgagccttttcctaaaggaattggtggggttcgcactgttgtttgctgtacttggtttagttgttttcttcttatttcaccaatcgatttataaaaatatcgaccagggattggtcacgcaaaagcaaaacgtgttaagtaaccggaaagctcctcaatttcggacgggcggcaatgcgcaaaatccagccccggccaaacccaataatggtgatacgccatttagaaccaacattttagtttttaacaaaaaagggcagattatcaatgctcaaatgctgggcaatcggatttacaatctatttatcaataccgaactggataagtcgcaagtcaacaaggtccgcgaagtaaccttaatgtcaaccgacaacaccttacattatttccgaaccctgttgattaaggtgcccaagtccaattccaatccaatttatgccggtaactatgttttgattttggaaaatattgataccgatttgatggcggttaacagttttaagcgctcactgctgacgacactggttttcttttggatcgtcgcgattgcgattgcttatttcctatcccgatcgagtatgaaaccgatcctggacgcctggaaacgccaacggcaatttagtgctaacgccgcacatgagctgcggacgccgctgaccgtcatccaaaatcaaatggagtatatgttaaccaaacccaagaccaaggtcatcgaccaggtcgatccaatctcaacttctttggatgaggtcaggcacctgcaaacgttgaccaaccggctgttgatgctcgcccgatcagattctgggacaattgaaatcaacaaacaggaagtggatttgaaaccttggttcagccaaattctcaaaccatacgacgatatcgccgccagccaacataaatcgatggtgacggtccttaaagccgatggtaagggacgcctggataaggatttgattcgccagctcttaatcattttgttggataacgcgatcaaatacacgcctgccggtgggacagtcactgtgatgacggcattgaaccgtgatcgattgacgattgaagtgcgtgataccggaaccggaatacctgatgctgacaagaaacgaatttttgaacgcttctatcgttctgacaaatcacgaaattccaagactggtggtaatggcttgggattggcgattgctaaatggattgttcaacagcactcggggaccatttccgttaaggacaattatccaaagggaaccgtgtttgatgttttgatcaagctgtaaaatgataaagtaattactgtgcacaaagaaagctcggagtaaaagtgatttgacttttacctcgagcttttttgtgattgggttccactagatcaatgattgatcctgcttatcggccttgttaattcctggaaataattcgtgcagatattcaagcggttcaactttaccgactttgtcagtgtagacgacttgagtcacgttgtcataggttaaggtgatcagtgactcaccgtcttcatctttgacaacataataacggataccgagttggatggcgtaaaagatcaaccgttgggcatcaaatgagattttgccaattgatggcagaagggtcgttgcgcccaaacgttgggcccgccagcgcttggcgaccgtggttccgaagtccatcaagctgccatttttgatgtgttttaacaacattgccgaagctgttagttccgggtgggtgaccacttcactgaaatcgtccagtgcctggagctgttcggaatgggcatgaagtgacttagccatttcaatcaactgatcaaagatttggatgccttcagccattttgaaagtcggctggttggggttctccaacgccacctgattgttatcagtgaaagattgttttaaatcagcggcaatattttcatggtcaactggggtgactaagagatacattaagaagaattttaaaaagtacattgcgtgacgactgatgccattaggggtaaacggcgtgttatccagtactcggaattccagataagagatgcctttagtgcgataatctttaatgtcgtcttggccgcgaagtcggaccggtccataaaattcagctgtggaatatagataatggtcgtcgattgcatgattaatgccgtcaatgtaatgatccaagctggtataaatggtggcgtcaacctgatcttgtggttcgttgacatagccataaatgctgttgcggatacttctgaccggatgggtgagttgtttttgatcctcagcggataaaaagcctttctccgcaattgggctggcaccgaacaaataagtcagcagccaacggtgaaggacaaaattttgagctagctggaagtacaatgcatttttgaaggccaccaaggtactgaactggtcttggtagtggacataaagccgattgatgaccggttcggggatgctgaagttgacgtgaacgccagtaatgatttttctggcgaccccgtacttttcggttaagtaatcacgatatttggcgtaggcgggccgaccaaaatggcctttaatatagttgacatcatcttcgtccattgctggcggcatactcagcggccaaaaggattccgatttatcaatcgaccgatataaaactgtctgcaaagtatccaattgatccaacacgccgccaatattggggttgggatcggtaataatttcgctcattgattcggaaaaatctgattgcaaatagggatgataacgtctggaacccagattttgcggatatggcttgcggcttaatcggccgtggtcatcgattcggtgttcttcgatttcaatgccgattaggctatggtaaagctgttctgcaacgcgttcttcttgaatgtgttttaataaatttttcagcatagtagtcccccagccggatttagttatacataattataaacaaaaatcggcagaatggtagtcatacggccgttctgatgaaaacgtaaggttatttttaacttcttgaaaatcattgccatcggtttcgtatttaacccatagaaggtgatgaaatgctgatagcgatgattgataatcaattagtgaatgcggctgaattcaaaggccaaaagaatttagccaatcgactggtttgcccgggatgcaggcaaaaagtgatattcaaacgcggcaagtaccgcattccccattttagccataaatccaatcgggtttgcggtagtttcagtgagaatgaaagtcaggcccacctccagggcaaactgacttttcaacggcagctgcgagccatggcgacagaggcggtgttggaatattatctgccaacaattgagcagcgggcagacgtttatttaccgtctccaaagctgattttagaatatcaatgcagtcccatttcgtttgccgaactttctcggcgaacggtgaattaccagtcacttggaattgacgtggtctgggtgctgggggatcgccatttaaatgccgccaaacgattggatggggttgccaagtttgcccgttttagcagccaactgggcttttacatcatcttttattctgctaaaaatcagcagttccgaattgattttcagattcgcgaagttgccggtaaactcactagtcatatgcgactatttaaaactttggccgagttgaagcgattcattgaccacccgccttcagctcttcaacggtattcagtccgggctactaatacggcgattttgcaccagctcaaccggattcagcggagtattgttttgaaaaatcccacttacctggacatggtcacgcgatgttatcaacgacgaaaagtctttgtcggctgccctttgatttgtcatggaaaagagggtgagggatggccgatctttcggcggactgctttgtgttggcgagtgtggattgttttgcagctgtttacgggcagtaatcgggaaatttccaatcaggagttaaatcaggttttcaagcaatcggttcaactttttggccaacaatttgcccaagtagatgattacgttcgtttctttcaaatggcctttaccagttttatctttagcctccgggccggcggctatcttcgacacacggtagccggcgtgcaaatcattaaacaaccggtgtggtttgccgattatgatgaaaaacggcaatatatcatgaccgccaagccggaggtgtgctaacctattggtaactaactatttgaaggaggacgttatgccaaaaccacaagaattaccgcttagaaaagatgttccagaagaactgacttgggacctgacgacgatttatccaaccgatcaggaatttgaaactgactatgacgctgttcaaaccggtgccaaacaattcgctgaattagccggaaccattgagaagagtgcggcctcactgctgacagcaactgagcgtttgatgaccttaagtcgaaagcttgaaaaagtctatgtctacgcccagttgaaaaatgaccaggataccagtgaagacaagtatcaggccatgtattcccgtgcggaatccttgggggctcaatttggggcggcaactgcctggtttgaaccggaactcctcaaaatttctgacgatcaaatcaagcagttttatcaggatgaacccaaattggccgattatcgacggtttttcgatcaaacctttaaacgccgtaatcatattttaagcaacgatgttgaagccgttctggccggggccggcgatattttctcgtctggagagaaaacctttggcattttggataacactgatctttcattcccagcggtcactgatgagaatggtaatcaggtgaagttatctcaaggtgtttatggtattttattggaatcgacaaagcaaagtgtgcgtaaagaagcgtttgaaaaattgtatcaagtctatcgtcagttccagcacacgctggcggcaacactgaccactaatgttaagaatcacaacttcaaagccaacatccgccactataacaatgcattggaggccgctttggctgataacgaagtgccgacagacgtttataacaacctgatcaaagtggtcaacgagcatctcgatctgctgcacaggtacgttgctttgcgtaaaaagattctgggccttgatgaactgcatatgtacgatatgtatacgtccctagttggtaaaaaatcacccaagtatacgtttgaacaatccaagcaaatcgccttggaggctttgcaggtaatggggccggattatgtcagccacgtcaaagaggagttcaacaaccgttggattgacgttgttgaaaatcaattcaaaagaagcggcggctattcctccgggacttacgataccaatccgtatattttactgaattggaaggacaatttggataatctctacacgctgatccacgaaaccggtcatagtatgcacagctactattcccatcataaccagccttatcagtatggggattactccatttttgtggctgaaattgcgtccacgactaacgagaatatcttgacggattatctcttgaataaattcaaagatgacgatgaaatgaagaaatttattttaaattactatctggatggatttaagggaacggtcttccgtcaaactcagtttgctgaatttgaacaatacattcatgaacaggatgcaaaaggtcaaccattaaccgccaactttatggatgattactatcgcaatttaaatcaaaaatactacggggatgccgtgatttctgaccctcagattggtcttgaatggtcacggattccacatttctattacaacttctacgtttaccaatattcgaccggctttgctgccgcatcgacattggctgatggcattgtgaacggcggccaggccaacgttgataaatatttgaattacctcaaatcaggcagttctgacacgccaaccaacgtcatgaaaaaagccggcgttgacatgacgcaaccggaataccttgagaaggccttccagatttttgagcagcgtctggatgaatttgagcgtttgtacaacaaatagtttcgctaataaataagcgtaaaaaataccgacatttgggagttcccagatgccggtatttttgtggattaaattagttgaatcgtaagtttgatttgggatacggaactgtcgttggtttctttgaagcctgctcgaagtgagcagccgatcccagactcttggcacaaaagccaaagagagaattgtaatcaaagtccttgatacgaatgccactgtcagcaacgtcggaattaaacaaaacggtggttgatggatcgcggacttccatttcgtggaccactcgctgatcacaacgaaacattttttctgccaaatcagagcggcggtctgccatgaacatctcgacatccaaaccatttcgttcagcgagcttggcaaccagttcatccgagtatggtactgaattaatcagaagttctttttgcaggtccatcaagaagcgtcggccaaacttctttccctgaaatgaagctgccttgaaatccaaaatggtatcgtagggcaggttgtgatcaagatggctgagttgctcattctttgaaaagtcgtgcagaattttgatgttgagcatcgaaacaaagcgcacgctgatttgtttgtttaatttttgtgaaatccgttcaatcgttttttcggcgtcgtaacaatgtcgattaagtggatcaacgaataaataaatctcaagtaccattattgcccctccatgtgtaaccgacaacaaaattaatatactaattattttctccattaagaataccaaattttcacgtaaaaacaacaattttgcttgaagtgtgtatgattgattgggaaaggttgttgaatatggtaaaattaagtctgattgaattttaccttgaagcaatagagcgttcggatgagcgcaacagattggaagtgttagcttggttgagaattgggatgactttttagttccttacaaacaagctgttgatgaattaaaagtaaaattacgtggcatcagagcgcaattcttaaaaattgatggtcgcagtccgattgaatttgtgaccggtcgggtgaaacccgtcgacagtattaaagaaaaaatggtcagaagacacatttccgaagaccggcttgaagaagatatggaagatattgccggtttgcggatcatgtgtcagttcgttgaagatatttatcaagttgtggatttgcttcgcaaacggactgatattaatattcttgaagaacgggattatgttcataacaagaaaccgagtggatacagatcataccacattatttttgaatatcctgttcagatgcttgacggtgaaaaagtcattttggccgaaattcaagtgagaactttggcgatgaacttttgggccaccgttgagcactcattaaactacaagtatcaaggcgaatttccggatgatttgaaaggccgactggaacgatctgccgaagccgcctttcatttggatgaagaaatgtcagaaattcgtgatgaactccaagaaaccaacaagcatgagccaggcaaagatgtaaggaagtcgtctgatgaagatagccatctacagtaatcttggtgagtcgtcaaacattgtggcgacttcattaaagaaaaaaattgaagaatcacccgatttaagcatcgacggactgaatcctgaaattgtcatttctgtcggtggtgatgggacactgctgtctgcatttcaccactatcaagacattagcgatcgaatccgattggttgggatccatactggccatttgggcttttataccgactggcgggattacgaagtcgccgaactggttgacagcctagagcacgacaatggtcaaagtgtcacatatccactgctggatatccgggttaattatgtgagtggcggcccagctgattatggcttggcgcttaacgaatcgaccctcaaacagattagcggttcgatggtggctgacgtctatattaaggacacactctttgaaagttttcggggtgacggtctttgtgtctcaacgccgagtggctcgacggcctacaataaatcagttggcggcgcaatcattaatccaaccctcaatgccattcaaatggccgaaatctcctcgattaataaccgggtctttcgaacgctgggctcaccgttgatcatttctccagatgagtgggtgaaaattgttccgaagagttccaaccggacgattttgacttgcgatcaccaaatcatctccaacgaagccgttgaatcggtcgaataccggatttctaaacgccggattgcttttgcccagtatcggcacacgcagttttggcggcgggtaagcaactcgtttattggtaaggttaatttagatgactgaatttacgtggaaatatacaggccaggccccgatcaaggtccggacattcattatgagttacgggatcacccggacattgttgaaaaaaattaaatatcatggtggaaagactttggtgaacggtgaagcctcactggtcaaccgaatgcttcaaaccggcgatacggtcaaagttgtcttgccgcctgaaccggagaacgaccatgttagcgtctccaacgttccaattgaaatcgttcatgaagatcccaactttttggtggtcaataaaccatacggggtggcctcggtaccggcgcacaaccatgttgattcactggttaatcgggtgaaaggctattatcagcgccagggctatgccaatcaaaaaatccacattgtgactcgactggataaagacaccagtggtttggtgatttttgccaaacaccactttgctcattcagttcttgataagcagttgaaggaccggacaattcaaaagacgtacctggcgattgtcgctgatcgaatttcaacgccccactttgaaatttatctgccaattggtagagccgatgattcgttcgtcaaacgccaggtcgttgattccggcaagatgtcggtgaccgaagcttggacagtgcgtcgattagctaaacaaaccttgttaaaagttcgactgcacaccggtcggacccatcagattcgggtgcatatggctgctattggtcatccgttgattggcgattggctttacaattcagatgaccattcaatgaccaggcaggcacttcactgtgccgagttgactttttatgatccatttgccggtcgcctgcttcattgcgaagcgcggctgccggaagatatgcagtcctacattaatttgcataaactttaattgacgttcaaccaacagcttcccacaaaacgtgtttgagaattttggctaggaagcttttttggttggctgctgtgatataatgaactgcgtttgtggaggattttaagtgaaaaagattgattttggccaaaaatttatgaagcagaatttacagttattccgttgtcctgtctgtcaaacaccattcgatgaggtggtgggatatagcttaagctgtccccatcatcatacttttgacatctctaaaaaagggacgctgtttttcctcaccaaacaggcaaacaacgaatatgacaaatcgatgctccaggcccgccacaaaattttacaggctggtcttttcgacccgattgtcgatgcgatcgcaacgtatttgggcccggaaccagaaaccattttggatgtgggctgcggtgagggcacgccgctggcacgcttgctggcgcttagagatggcaaagataccgcaatcggctttgatatttccaaggatgggattaatttagcaacccaacagccagccgacgcttttttctgtgtcgcggatttggctcggctgccatttaatgaccacacaatttcgaccatcattgatttgttttcaccatctgcctatgatgaatttaatcgggtagccaagactggcggccgattgattaagattattcccaacagcgactacctgcatgaattacgagtcgctttatttggcactggtcaaaagaacagttcttattcaaataacaaagtatttgatctgttcatgacgcactactccagtgccagcattgataagcttacatacgaattttcaattcccaaagggatgcagcaggatcttttgacgatgacgccgcttcactggggcaagggacggcaagataacgcccttcaactggttaatgcactcaagacgattaccgttgatgtttcagtgatggtcgcagacttttagaatatttggaggaaacaatgactaatcatatcgtactatttgaacccttaatgccggcaaataccggtaacattgcccggacttgtgccggaaccgacacggtccttgacttgattgaaccgctcggattcagcattgatgataagcacctcaaacgggccggactcgattattgggataaggtccagatcaattatcatcaaaacctgcctgaatttttgaagtcggtcaagaatcccaaaaacctattcttagtttctaaatttgccaaccaggattacaccgatccggattattctgacccaagtcaagattactatcttttatttggtaaggagacgaccgggttaccggaaccatttatgcgccaaaatcctgaaaaggcgattcgaattccgcaggatgacgacaacattcgggcactgaacctgtctaacacttgcgccattgtgatctatgaagtactgagacaacagaacttcaacaatttggaacgaacgcatcaatatgaacatgataagctgaaataatcaacagtcattttacgggaaggggggaacagcatgaaaaccaagcgaaccaagcgaaccaagcaaaccagcagcaagccggttaaaaaacgcggccgtccacgaaagacgaccaagaagactggcggccagtcgagctttcttcagaaatatacggttaatgtcatcggtggcgtcgttgccattttggccttactgggattatttcaagccggaattgtcggtaccttaatgatcaatattgccaaactgtttgtcggcagtctttatccggtctttcttttggttggaatcgttgtcggcgttttcctggcaggcttttcccggttccccaaaattccagccaagtatacttggggaacggccttgattttgctgggcgttcttctttggctgaccttaattgaatacattcaggctgcccagccggttgactttatcaattttaattggcagaagctggttgatgatgttgtttcatctaacagtgattccaacatcggtggcggcattctggcaacgattgtgttttatcttgcccacgtactatttggcaaaatcggcaccggaatcgtcgccagcctgatcattttgatcggtggttttattctatttgatatttcatttgcaaaaattttcatgggtctgcggacttgtttgacatttatcaagactcgggctgcagccatccgacagcagacggaccagaaacggtctaagaagccggctaagcagccttcatcggcaacggctgccaatcacccacaaactgtggaacagcctcaaaatgatgattctgagccaaataagttgtcggcgtcagcgatcacgatttctggcatgccagtgactgatgaagctaaacagtcacgtaagcctgtctctaagccgacacctcctaaagaatccgaaaaagcggacgattctgccgacgttaacctggtcgacgtcaaagaagatgatgcctacaagttgccgacaaccgacttgctgacgcaaatccctcaggatgatcagtcaagcgagttgcagtcaattgaccataacgctcaagtccttcaaaagacgttggacagttttggggttaaagccgaaattaagcacgtcagtttaggcccgtccgtcaccaaatatgaattgcaccctgatattggtgttaaggtgagccggattgtgaacctggctgacgacattgccttggcattggctgccaaagacatccggattgaagcgccaattccgggtaaatctttaattggcatcgaagttcccaatcgaaagattgcgacagtttccttcagagatgttgttgaacatcagcctgataaccatggccacgtgctccaagtgccgcttggaaaggatgttaatggtaatgtgattacggctgatcttaccaagatgcctcatttactgatcgccgggtcaactggtagtggtaaatcagttgcaatcaatggcattattaccagtattttgctgcacgccaaacccagccaggttaaattaatgctgattgatcccaaaaaggttgagttgggcgtttataacggcattccccatttgttaagcccggttgtttccgagcctaagaaagccgccagagcactgcaaaaggtggtttccgagatggagaaccgttatgaattgtttgccaaattcggccaacgaaagattagcacttataatgattttgtcgcgaaaaacaatcgtgaaaatgacactaaaatccagccgatgccctatatcgtcgtgatcgtcgacgaattggccgacttgatgatgaccgtctccaatgatgtcgaagcagcgattatccggctggcgcaaatggggcgggctgctggaatccacatgattttagcaactcagcggccatctgttgacgtgattaccggcttgattaaggccaatgttccgtcaagaattgcctttgcagtatcaagtgggattgattcccgcacaatcatcgatactaacggtgctgaaaaattgcttggtcggggcgacatgctgtttttgccaattgattccaacacgccgattcgagttcaaggggcctttattcccgataaggatgtctccagagttgtcaaattcattaccgatcagcaatcagctgattatgatgaatcgatgatggttagtgatgaagagatcaaagaagaggatcaagaagattccgaagacgatttattcaacgatgctttggcctttgtggttgatcaacagaaggccagcacgtcacttttgcaacgtcacttccggattggctataatcgggcagcccggttaattgatgatttggaaaagcgtggctatatcggaccacaagatggcagtcggccgcgtcaggtctataaggaaaaacaagaataagtttgaatgacaaaaaagaggctggcacaaaagctttcacttttgccccaacctctttaagtcgtttgtttataagaatgtcatgattgctgaaatgaccagtgaactgatcgttgcaataatcatgatccaaacaaataccaatgtaattttttgaaatctggttctctttttacgcgccaatatttgcaccactttctcttgtattccatacacagtttaactatcattatcgttcaatgcaatatgttttgtcaaaatcaggagggtaactcatgcatatttctccttggatgactgacacggtaacctttataacgcaatttctgattctatttgcagttgccgggttcttagttgttttaagaaaaaatcaatttttcaggtcgaaggtgccgattaaaccactcgatttttggccgccaattttgctgtacttcattcacgagattagtaaaaagggtttgtcggggtcattcattcccgaagtggtgattgtttggttagggctcacattgattgtgttgatctggcaaatttttgccaatccgaatctaacctacagaaaattttttatcactttttggcgattcagtgatttatttttattcggctgttggatcgtcgtggggatttatgtcatttttgagtctatctgaatcaataactgttcatcggatcaaagcagatttttatgctttggtctttttttgtgcagaaatgggcaaatctccccaccactttctcattgccgtcagatcagtcctggacggatttttagttgaatatgaaaacggtttataacaaaaaagtgacaaattttgaggaggcgtggttgatagtggtggattgtggtagaatgtgattgtaaactgaaattgggggtgatgacgacatgttcatgggtgaatatcaacacaacattgacgccaaaggacggatcatcatccccgctaagtttcgccaggatttgggcgacaaactcgttgtcacccgtggaatggatggctgtttatttggctatccgatgagtgaatgggaaaaggttgaacaaaagatcgacactttgcccgtgaataaaaaggatgctcgttacttcacgagattctttttctccgctgcagttgaatgcgaatttgacaaacaggggagaatcaacatccccgcaactttgagggattacgcaaaaattgagaagaaatgtgtcgttgtcggtgtctccaatcgttttgaaatttggagtgacgatcgctggaacgactttagtcatgacgccgaagagaactttaatgaaattgctgaaaatatgattgatttttagataagcagacatgctggaaacgggggtgatcgaatgtctgaatttaagcacgtaactgtcctcttaaacgaggcggttaaggggttgaatattaatcctgatggtacatatgtcgatgcaacattaggtggtgggggacataccaccaagattcttgaacagttaaccaatggccatctttattcttttgatcaggacgaagaggcgattgcttataaccaacagcacttggctgaatacattgaagccggtaaattaactttgattcacgataatttccgtcatttaaaatcagctctccaaaacgttgatgtttcgggaattgatggaatcgtttacgatttaggcgtctcgtcacctcaatttgacgaagccggtcgcggattcagttatcgctttgacgcccgccttgatatgcgaatggatcaggataatccaatcgatgcctggaaaattgtgaatgaatggccttacgaaaagttggtccggattttctatcgatatggcgaagagaagtttgccaagtcaattgctcggcggattgaaactgttcgacgagagcatccaattgataccactaacgatttagtcgaagtgattaaagagggaatcccggcagcagccagacgccacggcggccatcctgctaagaaagtctttcaagcggttcgaattgctgtcaacgacgaattatctgcgttggaagattcactggaacaggcgttggatttgttgaatgtcaacggccgaatcagtgtcatcacttttcaatctttggaagatcgcttggttaaaaccatgttcaaagaaaaaacgtccttgccggaattaccgcctaatttaccaatcattcccgaaggcatcaaaccaaaatttaaaagtattactcgaaaaccaattgttccaactgaagctgagttagaagagaatcatcgatcacatagtgccaagttgagaataattgaacgaattaaaaactagataaaggaagagtacatattatggcacaaaataatttagctcgtaacttaaccgaacaaccgcaaccgtatgtttccagccctgatcaggctaaagtaaaacgggtgagcattgcaaaagccctcaaactttcgtcctttgaaaagctgttaattgtatgtggcagcgcagtcttaactgtgttaatgttagtagttgtatcgtcaaaaattgccttgtctaattcacagcatgaacttcaacatttagacaaccaggttgtgacggttcgcaccagtaatactaatttaaaacaacagattggtgagctgcaaagcagtacccgtctggacaaaattgcacacaagagcggcatgtcactctccaatgcaaatataaggaatgttactaaatgaaagagccatctgatcgttccgcagacaaactgaatgcccgaaaaagccggaaaattgttggaataagtttgttccttgcatttttcctgctttttgcatttttaggcagtcgtttacttgtcattgcggttgggaaaaatgttaaaaatgtcaatttaaatgaccgcgccgaaaaactttatactcaaactcagaccctcaaagccaaacgaggatctatttatgatgcaaacggtaatccaattgccgaagacaccagtacatattcgctatatgctgttttggacaagcagcaaaaagggttgaatggcaaaccactttacgttgtgaataaaactaaaactgccagagtgctcgccaagtatttacctatcaccgaaaagaaggcattgaaaattttatcccccaaggataaacagcccttccaagtggaattcggcagtgccgggaccaatatttccttactgactaagaagaagattgaagcagccaaactgccagggattgactttgtccaaaagcaagcccgcctatatcccaacggcgtcttttcatccaatttaattggggtggcggtttctgaaaccaacaagaagaccggtaccgccaacttggttggccaaatgggcattgaaaaagccttcaacaaaacgctagccggacagaatggctttaaaaacgctcagtacgatgtatacgggtacaagcttcccggtaagcagcaaaaagaaaagccggccaaaaacgggaataatatttacacgacgattgattcgcggattcaaaccctgctggagagcgagatgaactctgttcagtcacaagttcatccggctggaatgaatgccgttttgatggacgccaaaaccggaaaaatcgttgctgcttctcaacggccaactttcaacgcggcaacgctgaaaggcatcggttcggcttggaccaacacgttatcctccgatatgtacgaaccggggtcaacaatgaaagtctttacgctgtcatcggccattaattcgggtcattataacggcaccgacacctatgagtctgggcgttattcaattgacggcaagattgttcccgattggaatcctgccggatggggctatatcacttataacaaaggatttgccttgtccagtaacgttgccatggctcatttggaacaacaaatgggtcccaagacttggaaaaaatacattaagcgatttggctttcttaagagcaccaatagtggccttccgggagaactcaccggcagaattcagttcaattatccgatcgaacaggctgacacctcatttggtcaaggaattgaagtgaccactttacaaatgatgcaggctttatctgccgtttcaaataatggtacaatgatgaagccgtactttatttctaaaatcacaaacccggcgaataataaaacgattaagcaatacggcaagcaagttgttggtcatccgatcactgctgcaaccgccaaagctgtcagaaagcacatgcaagacgttgtctacaagtcttacggaatcggtgccgattacaaaatcaagggctaccgggtggctgcaaagactggtaccgctcaggtcagcaacggaatgggcggttatgcttccggtgacgacagctatctctactctgtggccggaatggttcccgccaataatccacgctacgtgatgtttatcacgatgaaacagcccaaactgactgggaccaagacagctacacaattgctggcagagattttcaaaccagtgattacccgtgcgctgcagaactcgaataccaaacaggcaaccgtcaagcggcaggtaccaacggtgacctatcagacaacgacctatgccaaacgggtgatgaatgaaaaaggctttaatgttgtgacaattgggtctggcgattcgattctcaaacaatcgccgagcgctggaacaacacaagccgaacaaaagcgggtctttttactgacaaataaagactggaagatgccgcgaatcatcggctggagtaaagccgatgttgaaaagttttgctcgctgacaggcttaaagctcgagtctactggtagtgggtacgctgacagtcaaagcatcaactttgagaagtcaattgatacgggcgatgttttaaaagtaaattttgaataatgaaggatggtaaatggcgactatgggtaattggttaacacctttattgagtacatttgtgataacggcaatttttatgccaagtttgattaaatatttccgaagccgacatgaaggtcagatgattcgagaagaggggccttcgtggcacgaaaagaagtctggcacaccgacgatgggcggcattttgttcatcgttgcgatcgtcttatccgacttggccttcggtggggcaaaagggatgttgaacccgacgcttctcatcttactgtttgtcctgatcacctatggtctccttggaatgtgggatgacagtattaaactgtttcggcgtcagaatgaaggattaaaggcctggcaaaagatgctgggacaaattgtggccgccgtgattttctcagtggtatacatacacgaaggctttccaatggcgatcaaaattccgtttggcggcgaccttcgattaggctattggtacattttgttcattgtcttttggctggttggcttttccaatgctgttaatttgaccgatgggttggatggactggttgcgggcctggggacgatttcctttgcggcctacggggttattgctgccgttcaaaagcagccggaagtggccgtcttttgtttctcggttgtcggtggtttgttggcattcttcattttcaatcacaaaccagccaagatcttcatgggagatatggggtcgctggctctcggcggagctttggcagccgtttccgtgctggttcaccacgaattttcactgttgatcattgggatcatctatgtgtgcgaaacggccagtgtgattattcaggtggggtcgttcaaactgactggtaaacgggtcttcaagatgacgccgattcaccatcattttgaaatgagcggctggtcagaatggaagattgatatcgttttctggctgattgccttggtggcatccgccattagtgtgatgacgatagtatagaggttgggacaaaacggctggttttgtatccagcctatttgactattcatatgatgaaaaacgagggaataaaatgaaaaaaattgatgattataatcataagaaagtattggttttgggtgctggtaaaagtggcacccacgctgctgaactcttaaaagaattgggggcaacagttgttttgagcgattccaaacccagttctgaactgcctgaagtcgctgaattgcaagattccggcattcaaacggtcaccgggaaacaggatccggctatcttggacgatggttttgacattatggtaaagaatcctggtattccatacgacaacgcggttgtagccgctgccgtcgatcaccatctaccaatcattactgaagttgaactggcttcacaaatcaccgatgccgaaatcattggggtaactgggagtaatggtaagaccacaacggtcaccatgataactgaaatccttaaccaggaacgtgccaaagggcatgcctatgctgccggtaatattggcatttctgcgaccgaaactgccaagaaggcgacgaccgacgatacgatcgtgatggaactttccagttttatgctgctgggaattaagactttacacccacatgtggccgttttgaccaatattttctccaaccatttggattaccataaaacccgggaaaattacgtgaatgccaaaatgcggatcaccatgaatcagacgcctgaagatttctttgtggtcaactttgattctgatgaatggcgcggcttaagcaaacgcagtgctgccaaggtcgttccctttgccagaacaactgagattgacaagggtgcttacgagaagaacggcaagctgtattacaacgacgaattcatcatgaatgccgaggatattaaagttcccggaaagcaaaacgttgagaatgccttggcggcaattgcctgtgccaaagtgctcggcaaatccaatttggcaatcaccaatgtattggaaacgttcactggcgttcgccaccggcttcaatttgttcttgaagccaacggccgcaagttctacaacgattccaaagcaacggatatcgaagcgacccaaatggcccttgaaggttttgacaaaccagttgttttattggctggtggacttgaccgcggttatacatttgataaattgattccgcaatttaaggaacatgttaaggctgcagtcttatttggcgaaactgccgatcttttggaagattccctgaagaaggcgggcattcaaaatattcaaaaagttgataatattgatgaagctgttccagcggcatactcatttagtgatgaaggcgacattgtgttgctttcaccagccaacgccagctgggatcagttcaaaacctttgaggagcgtggcgatcgctacattgcagatgtggagaaattgacgaataagcaggaggggcactaatgcgtttaatcatttctggtggcggtaccggtggtcacatctacccggcactggcaattatcgaggatttacttaaacaggaacctgattcagaagttctctatgtcgggtctcagcgtggcctggagagttccatcgttcccgagcagggaatcaagtttgttgccttggaaattcaagggttcaagcggtcgctgtcattggagaacttcaaaacggtggcgttgttcctaaagagcgtgcatgaatccaaaaagatcattcgagactttaaacctgacgttgtcattggaaccggcgggtatgtttccggggcagtggtttatgccgcggccaaagcacatatcccaaccatgatccatgagcaaaatagtgccgttggattaaccaacaaatttttgagtcgctatgtggacaagattgcgattggctttcatgaggcggccagtcaatttcctaaagaaaaggttgtcttcgctggcaatccccgcgcccagcaagtggctaatatgaagagtactttcaagtggtccgatgtggggctgcaagacggtgaaccgaccgttctcattttcggcggcagccaaggggcaccggcaattaataaggccgtgatcggcgctgtcagcgagcttaacaaacgtcagtaccaagtggttttcgtcaccggtcaaaagcgttatcaaaacgtgatgaatttgctggataaaacgcggatcagcagtaacatcaagattctgccgtacataaacaacatgccgcaagttttaccgaaagtttcactgattgtcggtcggtcaggagctaccagtattgctgaaataacggccttggggattcccgccgttttgatcccaagtccatatgtcacggctgatcaccaaaccaagaacacgatgagtttggttaaccgtggcgcggcattgatgatcaaacaggatgatttgaatcctaaaagtttgttaaaggccgtcgatcagttgatgcacgattcaacggcacgtgagaaaatggcagagaattcaaagcagctcggcgtcgttgattccgctgacgaaattttgaatttagctagaacactgatcaagtagtctgataatcgggggtagagatcgttgggagcacaagaccaaaatgggaagaatcacggaggattgtttcgcgatttccaaaataggaacgtcaaaaaaatgtggccgttggtgatgctgattaccatcattttgttggtcatgatctttatgatctcgtcatacagtcgcgtgaaaaaggtcaccgtttccggtaatgagattgtcagcgatcaacaaatcaaggctttttcccctgttaagaagggaacgtcactgtttgctgtctgggggaaaacggacaagcttgcccaatcactcaaacaacgcagcagacggatgcaatcggtgaagatgaagctggtcaactttaatcaggtgaagattaaagtcgaggaatatccaacgatcggctatctcttcgttcacggcggctatcagccaattttaaagagcggcgtgattattaaggggaaagttttgaatcccaaggccggttttccggttttgaagaaatttcaaaatcctaagaaactgcggcggacgatcaaacagtacagacgaatcagtccaccggttcgcgcagttatgaacacgattagcttttcaccgactaagagtaaccccgatcgaatttttattcagatgagtgacggcaacaaagtctatgcttcaatcagtacatttggcgacaaaatggactactatccaagcatcagttccaagctgaaagtcaaaagtgtcatcaatttggaggtcggcgcctattcgtacccaatccccaaaaagcagacttcaacaaaaacgaccagtgtgcagggctattagagctaattaatctttttcgttgtttatgattgtgttaaacttatgttatgttcagaaaatattctagatgtggaggttccttacatatatggataattcgggtttatatgtgggacttgatataggaactacctcaataaaagtaattgttgcagaaaaagtaaaagggcaattgaacgttattggtgtgggaaatcagccttcaaatggattgagccgtggtgtgatcgttgatattgaccaggctgcagacgcaattcggagtgctgtaaatcaagctcaagaaaaagcaagtattgagattaaagacgtgattgtaagtgttccggcgaacatgttacggattgagccatgcaatgggttaattactttggatgatcaatcacgtgaaatcactgaggaagatgtccgaaacgttgcggcatccgcacttggcaccagtttgccacaagaacgagagataattgatattcagccggaagaattcatcgttgacggattcgacggcatcaaagaccctcgggggatggtcggcgttcgtctggaaatgcgcggtaagttaattaccggttcaaaaggcattatgcacaacctgcaaaaggccgtgaataaagccggcttgaatattatttcaactgttttaacgcctctggctgaaagccacgtggtgttaaatgacggcgaacaggactttgggacgattattgtggatcttggcggtggacaaacaaccgcttcagtcattcatgaccatcaattaaaatatgccacaacggatcccgagggcggcacatttattactaaagacatttcaattgttttaaatacatcaatggaaaatgctgaaaagatcaaacgtgattacggttacgccgattcgctccaggcatcggcggataatgaatttccagttgaagtagttggccaatcagaaccaacttacatcgacgagcgttatctcgcagaagtgatcgaagcgcgtttaagccagatttttgatcggatcaaagatcgtttgaatcagattcaagcgcttgatttgccaggtggaattgttctgactggtggtgtggctgcacttccaggaattgccgaattagccgctgaccaattcaacactaatgtcagggtctatattcctgatcagatgggattgcgacacccatcgtttacagctgcactttcactagtgtcatactttgccgatctggcagacgttgatatgattgttcgatcggccgttggtgcaacattgaccaaagcgcctaagttgagtcagcctgagcagacaccaatgcctgcagctgggaagactaagaagaccaaaaaaccgacacagaagaaaaaacgcggtgaaggaatcaagaatttctttagtgatttctttgattaagcacttaaacggagggaaaagacaattatggaatattcattagattccaccgataaccacggtgcaaacataaaagttatcggcgttggcggtgggggaagtaatgccgttaacacgatgattaactcagatgtaaaaggtgttgaatttatcgttgccaacaccgatgttcaggctttggcaacttcaaaagccgaaaccagaattcaattgggacccaaactcacacgtggcttgggagctggctccaatccggatgttggtgccaaagctgctgaagaaagtgaagaagcaatcacggaagcacttgaaggtgccgacatgattttcgtgacggccggaatgggtggtggtaccggtaacggtgctgcaccaattgttgctaaaattgctaaagaccagggtgcactcacagtgggtgtggttacccgtccatttagttttgaaggacctcgtcgggcaaaatacgccgatgaaggggttgctcaactaaaagagaatgttgatactttaatcgttatttccaataaccggttacttgaaatggttgacaagaagacaccaatgatggacgcctttaaggaagccgacaatgtcttacgccaaggggttcaaggaatttcagacctgattaccagccctggctacgtcaacttggactttgccgatgttaagaccaccatgcaggatcaaggttctgctttgatgggtgtcggcactgctaacggtgaaaatcggactgccgaagcaaccaagaaagcgatttcttcgccattgttggaagtttcaattgatggtgctgaacaagtattgttgaacatcaccggcggaccagatttatcattgtttgaagcccaagatgcttctgacattgtgtcacaggctgcgacgagcgatgtgaacattattttcggaacgtcaattgacgaaaccttgggtgacgaggtccgtgtgacggttatcgctaccggaattgacaagaaaaaggctgaacaggatcggatgtcaacgcgacggacccgttctgctcgtccacagccaactgcccggccacattcagaccgtcaagctccagaaaccaatcaatcacaggattcttcaaatgctaagagtgatccacttggtaactgggacatcagaaaacaaccagcgccaactcgtcctgctgctcaggatgaatttagcgacgttgagaaaaaggattttgatcctttccaacctgatgttaattctgacgataccagaccagataccagtgatgattcacaagacgatattccaccattcttcaagcaccgtcgtcggggcaagtaacatcagctgaccggtgcggatgtttggtgaaatgtgaaaggacacgaaatgccaaaatttaatttagctaatttttttgggatggatacagaccaaccagaaaatcaaattgataagccggcggacaacgttgtattgatgaatcgacaagaaccagaaaccagcagcattgttgtttttgaacccgttaattataccgatgttgacaccatcgcccaaaaactattggaggacagtgcggtcatcatcaaattggacaaattggataacaattcagctgcccggatggttgatttcttgaacggtgttttgtttgccattcacggatcaatcaatcggctcggtaggaacatcttcatttgttcaccgaagaaatttcaagtaactgagtaatctcgagaaaataaggagcaacctattggtcacatttgttatgtatgcagtttggtttatcgacaaggctatcaacatttatatgctgtgtattgtcgtgtatgccctgatgagttggttcccgaatgcttatggaacagcaattggccgatttttggcccggattgtcgaaccatttgaaagcttgtttaattttgccacgattgggatgattagtctcgctccgattgttgcattagcggtgctgacgttcgtccaaatgggcgttaactatcttggacaattgttaatcggctactaattggggtatggacatttcagccagagggggaaatatcttggtagactcgaatgtttcgcaacactatcgacaggctgaattgccttttttagagtcaatcgacagtttgagcggcagggttgcgaatgaatatcgaccgatccttactgattttttaaatcctagacagctttatatacttgaaacaatcgtcaacagatacgagggtgtctcatttcaaacttttggtgggtatccctcagctgaattaaaacgagcggttgcctttccggattactttgttcccaaggccgatgattacaatattacggctttccagattgactatcccagtaaatttgccacgttatctcacggacaaattttggggtcgattatgggaagcggcattgatcgggatgtcatcggcgatattgtcaccgatggtttgaattggcaatttatgtgtgaatctgagatggccgattatgttcaatcacaagttgaccggatcggcaagatcaaaatcaagctgaaacaaattcagcctgaggagattattgtgccggttgatgaaggtgaagaattaacgacaaccgttgcttctttgcgggtcgacgcactcgttagtgaaggattccacatttcccgtcatcatgccaaggaattgatcgaaggcggcatgattcgaatcaattgggaagatgccaaccgaccggatcttgaaatttccattcaggatattatttcggttcgcggtttcggcagactagttgtgcaagatattgccggcatgactaaaaaaggcaagattcgaatcggattaaaagtatataatcgaaataaataggaggattgaatcattatggtattaagcccacaagatattcataacaaggaattttcgacaaaattacgaggttacaatgttgacgaggttaacgattttcttgaccaagtcatcaaggattatcagatcgttttgcaggagaacaaggatttgaactctcagctaaacgaagccaaggacaaactttcctactttaacgatttgaaagattctttgaaccagtcaattttagttgctcaagaagctgctgataaggttaaaaccaattcgaagaaggaagctgaaattaccagccgtgaagctcaaaaaaaggctgacgatattttgaacgctgctaacgaaaaagcggatgctgttcttgaagaagcatcaaaacgtgctaagaagttggcaattgagactgatgatttaaagaagaacacccgggtattccggcaacgacttcaagtcatgttggaaagccagctcgaagtcatcaaagggtctgactgggatcgcttggttgaagaaaagccaaccacaacttacgaagatatcgaaaaagttgttggtagccttgacaacatcgcaaacccaggggtacaatctgaaactaaacagagtaatggtgctgcagatgttgaagaaacaccggctactgtggatgattcaaaccagaccgtcgtgatttatccagatggtcgcacacaaaatgaataattaatcgattagagaaaagaaagttattggctgaaacaacagcgagctgaagatagtggaagttcagcagtcaccaaccggtaaatcgatcacctctagtacataaatcgattatctgaagagatagaattttaaattctaaaattgggtggtaccgcgaagacttcgtcccttgtgacggggtctttttttgtagagtgcgacaagagccgggtgatgcggtttctaagactactttggttaaaaccccgattttgggttttgaccaaagtagtcttagaagttagcatctgggtcatcggagcacatttcaactagtgtgggactcgctccgttaattgccgtgagtcgcgttttatcaataccgcccaaacttcatccaccaaccaaatttctcaacaccaacacatcatcactccactaaatatctccatgaaaggaagtccagcaatgcgggtaaaagatacattaaacttaggcaaaacaaagttcaaaatgcgtggtaatcttcctgttaaagaagtcgatcgtcaaaaggcttgggaagataacgatgtttatcaacaaagacaaaaattaaacgagggcaaaccaacatttgtccttcacgatgggcctccatatgccaatggtgacattcatatgggccatgcgttgaacaaaatttcaaaggatatcattgttcgatacaaatccatgacaggttaccgggccccttacgttccaggttgggatacccatggcctgccaattgaacaaaagttgacgcaagccggatatgaccggaagaagatgtcgaccaatgatttccgtaagttgtgtcgggattatgcgttgaaacaggttgaccgacaaaaagaagaattcaaacgtctgggtgtttcaggtgactgggacgatccttacctcactttgaagccagaatttgaagcccaagaagttcgcgtatttggcgcctttgctaagcgtggcttgatttacaaaggtaaaaagccagtctactggtcatggtcttcagagtctgccctcgctgaagccgaggttgaatatcatgacattacctcaccaaccgctttttatggtgaacacgtcgttgacggtaaaggtgtcttggatgacgatacctacatggtggtttggacgactacgccatggaccattcctgcttctgaaggaattaccgtggatgccggatttgattactcagttgttcagcccgaaggtgaaactcggaaatttgttatcgccactgagttggttgacaaagttgccgacctcattggctggacgaatgttaaaacgatcaagaccgttaaaggccaagaccttgaaggcattttggcagaacatccatttgatcatagtcgtaaattgttaacgatgttgggcgatttcgtggaccttgaagaaggaaccggattagtccataccgctcctggttatggtgaagatgactttaatatcggccgtcaatacggtttggatatttttgcaccagttgacgataaaggctacttgactaaagaatccggtgaagactttgccggcgttttctatgatgatgccaacaagattgccttggataaattaaaggacgctaagttgttgcttcactacatgccgttgaagcatagctatccatttgactggcggaccaaaaagccgatcatcttccgggcaacgcctcagtggtttgcatctgttgataagattaaagatgaaatcttaaaatcattggacgatgttcaattcttccctgattggggtaaggttcgactatccaacatgatcaaaaaccgtggcgactgggttatctcccgccagcgggtttggggtgtgccactgccaatcttctatggcgaagatggtgaagcaatcattactgaagagaccgttaaccacgtagctgatttgttcgaaaagtatggttctgacatttggtttgaaaaggatgccaaggacttattacctgatggtttcacaagtgagcattcaccaaacggaaagttcactaaagaaaatgacatcatggatgtttggtttgattcaggttcctcccaccaaggggtgcttgaagaacgtaaagagctgacttatccggctgatatgtaccttgaaggctcggaccagtaccgtggctggtttaactccagtttgattaccagtgtcgccgtttctggtaaagccccttacaagcaagtcgtttcccaaggatttacccttgatggcaatggccataagatgagtaagtcacttggtaacaccattgcaccaatcgatgtgattaagaagatgggggctgaaattgtccgcctgtgggttacctccgttgatacttcagctgacgtacgggtaagtaccgagaacttcgtcaaggtttctgattcttataagaagatccgaaacacgatgcgattcttgttggccaacacgtcagactttgatcccaaagaaaatacggttgcctttgacgacttggaatctcaagatcaatacatgttggtgctcttcaataaattcttagccgataccagaagctatatggaacgatatgacttcctggactggaacaagaaggttgttggatttattaccaatgatttgtccgcattctatctggatatcgccaaggacattgtctacattgacaagcaggacggtcacaaacgccgttcgatgcagacggtgatgtatgagattgccgttggcttaaccaagttaatgactccagtgttgcctcataccactgaagaaatttggggattcctccacgaacccgaagaatttgttcaattaaccgatattccggaacccaagaagtacgaccacgattctgaaatcctcgccaactggacgaaattccgaagctatcgtgatgacgttttgaaggttcttgaagaggctcgtgacgccaagaagattggtaagtcatccgaagccgctttgacgatttacgcaaccagtgaagtggctgacttgatgaacagtttgcagactgatttggcaactgttttgatggtttctcaattgacgatgaaggactttgccgatgcgcctgatgacagtaccaaatttgacagcgacggcttggcattatcagttaaacccgctgaaggcaagacctgtgaacgctgccgtttggttcgccaagatgttggtgcagacagtgactacccaaccttctgtcaatcctgtgcccaaattgtccgtgaccagttccctgaaaccgcaactgaaggttttgaggaaaagtaaagcggcctttgagacgttgatcgtttaaatttcatcaaaagctgttccaatcttcatgattaaacattaaaatgagactatgacttaaatgttgtagtcttatttttgtattttaattaattgaaatgtgctttggctcacagattgtgccaaacacctgggaggatattttgcttaaaggaaaaattaaaagttacaacccacaaaatgcatttggtttcattacccaagacagcggtgaagacgatctgttcttcttcaaaaatgcctttcctgaagatcaatacggcaccattcaagttggcaagccggtagaatacgttgtcgttgccggacaaaagggaccgcaagctgccaaggctcacgtgatcgaagattagccgtcttgattgcaatgacccggtattatttgtagaatgagagtattaactaaaaaaggtgatcgagttggactttgaagaaaaagtaattggcacagagaagatctacgatggcgcaattatcaacgttgaaaaacagacagttaagctgcctgacggacagacatcatttcgagaaattgtccaccattccggagcggtcgggatcttagccctcactcacgacaataaaattattcttgagaagcagtggcgggcaccggctaaaaagaccaccattgagattccggcgggaaaagtagacggacgggatgctaattttcacgataccgtcattcgggaattgaacgaagaaatccgttatgttcctaacaccgtcaaagaactctacggcttttattcctcagtcggcttttctgacgaatacatgaaattataccttgccgaaggattaaaacccgttgccaatcaattgccgcgggacaaaggtgaattccttgaagtgtttgaaaaaacgctggatgaagctgtggcaatgattgcggatggcgagattcaagatgcaaagaccattactgccattcaatattggcagttaatgcaaaagtaggtgaccatttaacttggcgatcgatgataatcacaaaaatgacggaaaaccgttaacgcgagaacagtaccgaaaattaaaattacagcaggaagcagactttgaggcccgcgacaaacggcgggttcaagtcgaacgcgaatatgcaagaaaacaccaacagccggtttccgaagcgacgcctgaacctcaggaaacgacgcgggcacatgaaaatcatccagaagatgacgatttcaaaacgccgcgttggcaccggattaaccgcaaactgaattggacaatcacaatcttaattttactgatggtgatcgtttttttagtgttgttttttgtaaattaaggagaatttgaatgacttacggaattatttgtgcaatggacgaagaactggcaatcttaaaagaagccttgtctggcgaagaaaccaagcattacggcaatgctgattattatttgggaacaattcacggccaaacactggtcatcgttaaatcggggattggtaaagttcaagccggcatcacgacctcaactctgatcaatgaatttcacgtggacgccgtgattaactcgggttcagccggtggcattggtgacggtttagcggttggtgacatcgttgtttcgaccgagacagcctatcatgacgtggatgtcaccacttccggttacaaaatgggccagctgcccggctttcccgcccgctttaaagcctcggaggaactcgctgacaagattgtcaaagcggcccaacaaagtggcgtgactgcccacaaggggttaattgtttccggtgaccaatttattgccgattcaagcaaaattgcccaaatcaagcataattttcccgatgccttgtgttctgaaatggaaggggcagctgttggccaagtggcctatcaaaacaaagtaccatatgccgttattcgggcaatgtctgacgttggtgatgaagaggcggaagtcagttttgacaaatttatcatcacggccggtaagaagtccggtcagatgttgattgacctctttaagaacgagtgactttaaggagtgaaaataatgaaagagatatatcttgataatgctgcaaccacaccggtttcggatgaagtgtacacagaattaatggataagtataaaaatatttacggcaatgcttccacgctttacggcttggggagagaatccaaagccgtcatggagaatgcccgggatgtgattgctaaaagcattaacgctgatcctgacgacatcgtctttaccagcggcggttctgaaagcgacaatacggcgattacccaaactgcgattgcccgcaagtcactgggcaatcacattatcacaaccgccattgagcacgaagccgttatcaggccgtgtgaggccttggagaaaatgggctttcgggttacctatcttcccgttgacgagtatggcaacatctctttagacgactttaaggctgctttggacgatcagacgatcctggtttccatcatgactggaaacaatgaggttggttcagttatgccaattcatgaaattggtgaaatcttgaaggaccatcaggcttggttccatacggatgctgtgcaggcatatggtctgttggatatcgatgttcaacgtgaccatattgatatgctgtcgacatcggcacacaagattaacggtcctaagatgattggttttctctaccggcgtaaaggggtgaatttccccagtttgattaagggcggcgaccaagaggaaaagcggcgtgccgggactgagaatgttcctgcaattgccggatttgccaaggcggtccaaacaatcacaccagaagagaaggcgcaccgccaagccaagtatttgaaatttaagtattatatcgccgataaattgaagcaaaacggagtcgagttcgaggtcaacggtcgaatcaccgaggataatttgaaccacgtcttcaatatctggctcaaaggcatctcgacttacgtgatgcaaactaatctggatctggcaggaattgcggtttccggcggatcagcatgtacggctggtagtatcgagccatcgcacgttttggtggcaatgtacggcaaggatagcccaagaattagtgagtcgattagaatcagttttgggcgttacaatacgactgaggacctggataagttggtagatgcaattaccaagattgttaatcgggtcaaaaccaagggggtaaagatgtaatggcattcgcaaaaacaggtaaggttaacggtgatgatacggtgtatgaactaagggataacgttaaacggttcacactgcgtgatttgggctttattgagggcaagaccggtgtcttttcactggaaaagtcattggacccaacgtcgccgtataatgccaattataaattcaaaatgaaggttgataaggatctaagtggttttagaatggcgatcaccacgggaaatggtctggaaaaagtcaacatcttcaagaatccggatacccaaccaagtgttgagcaatatcaatttattattaacgatttgattgatagagatgtgctaaaaagaagagtgtgacgagagccgggtgacccggtttctaaggccgttccactttaaaccctggttctgggtttgaagtggagcggccttagaatttagggtcaggctcgccggagcacgtttgatgagagtgtgagccaagctggttagcctccgagcattaggtgaataaacaggtttgacgctgcctttgcgtcggacctgtttatttggctaagcggaggaggctggcttggagaacacatttcaagaagagtgtgacgagacccggttagggcccggaacataagtgattaaggtcaatgacgaacgctttttgttcgtcgttggccttaattgcttatgtggtagggccctgggtctcggaacacgtttcagctgagtaacagtgaactaaacactatatgggaggaaaaggccaaccaccaatttaaacaagtaattgtacatcacaatcaaacaaacccaatttgcaacattcaatcgttgggcccgggcaaaactaatccttttgcctgggcctttttacagtctgccattctacctagtcgaatcttgcccccatcagcagcttccggccatataagcgggggacaccaaatatccaagccctggatatttggtgtcccccacttatcctctggaagctaaccgctgattgaggcacactgtttttttccaagattaacattgacacgtccacgtaaaagcgataaattagattataattaagatatgatgataaacggataagtgatgatcttatgaacaactcgtgtttcacgttcgtctgatgatttcttacatatctgaattgtagaaaccatacttagttacaacgcttatcacctgcttaatcaatattttaaggaggacacatatacatggcaaaacaaaagttagaagatttagattggaccaaccttggattcgcctatcgtgatttaccatacagttacaacgaggaatttaaggatggcaagtggcaaaacggcgggttaaccaccgactcaacactgactttcaacgaagctgctgaagatttgcattatggtcaggaagtttttgaagggatgaaagcctatcgtaccaaggacggccgaattcaacttttccgtcctgacatgaacgccaagcgctttacgaattctgccaaacgtttggtaatggaaccatatcccgaagacaaatttgttgaagctgttaaagaagttgttaaagccaacgctgattttgtgccaccttatggttcgggcggctcgctttacatccgtccgttcatggttggaaccgaaccactggttggcgtttcaccgtcgtcaacttacaccttccacatctacgccaccccggttggtgcatacattaaaggccttcatccaatgccatacatggtcagcaaatacgaccgggctgcttacgctggtaccggtcaggctaagactgccggtaactatgccggaagtttgttagcagctaaggaagctaaagataacggctttgccggcgaactttatttggatcctcgtcaacataaatacgttgatgaatttggcggtgccaacttctatgcaattggcaaggacggcaagttctacacaccaaaatctcattcaatcctgccgtcaattaccaagaaatcaattctgcaaattgccaaagacttaggattagatccttctgaaaccaacatcgacgtcaatgacttggatgaatacaccgaagccggtgctatgggaaccgctgcggttatttcaccggttggctcattaaccaacaatggtaaaaagcacgtcttttacagtgaaaccgagccgggacccattacacaaaaactttatgatacattatttgggattcaatcaggtgatgttgaagataaatacggctgggttgttccggttgaataataaaaaaagttggccgtcgcacctcgcgacgccaactttttttgaccgccgaatcccttggaaagtgtttgacattttttctggcaaacattagaatattagaaaatggttagaccgatgacaactatttactacatatcctcaggagggacactatggcaaaagcaaaaccggcaacagaaattgattgggaaaacttaggcttcgattatatggacttaccgtatcggttcttagcgcattatcaggatggtcagtgggatgaaggtcaactcactgaagatggtactttacacatcagtgagggctcgactgggcttcattacggtcaggctgattttgaaggcttgaaggcttatcggactaaggacggcagtattaatttgttcaggccggatcaaaacgccaaacggatgactaaatcctgtgcccgtttattgatgccggcatttccggaagataaatttgtggcagcggttaaaaaagtggtcgctgccaatgccgactatgtgccaccatacggaactggcggaaccctttacttgcgtccgctgatgattggtgttggtggtaacatcggcgttcatcctgctgacgaatacatcttcacgatttttgccatgccggttggggcttactacaagggcggtctgaagccaaccaatttcacgacttcatactatgatcgggctgctcctcatggaaccggtcaaagcaaggttggtggcaactacggcggcagtttgctgcctggtgaccaagctcacaaagccgggtattctgacgtgatttatttggacccggcaacccataccaagattgaagaggcggggtcagccaacttctttggaattaccgcagacaatgagtttgtcacacccaaatcagattcgattttgccaagtatcactaaatattcgctgttgtatctggcggaacaccgacttgggttaaaggccgttgaaggtgacgtcttcattgacgatttagatcgattcgaagaggccggtgccatgggaacggccgcggtgattgcaccgattggcgggattgaatataaggacaacttgcatgtcttttatagtgaaacagaagttgcaccgattactaagaaactctacaacgaattaaccggcattcagtttggggatgtggaagccccagaaggttggattcaaaaagtcgaggtttaatcgattaacaaatgattgcaccagaaaagcgggctgggacaaaacgaacggttttgcccagcccttcgtgttttaattggtgatccccggcccgtcaggttagtcgattgtctatgaaaggatggtcattgtgatcaaacgagaaggtcattcccacacagaattttgtcctcatggaagtggggatgatgtggaattaatgattcaaaaagcgatcaagctgggttttcaagaatacagtattaccgaacatgccccgttgcctgatggattggccgataagtatgccgggaaaacaaccgggctgactgaggcttcaatggcggccactgatttggacgcttattttcaaaaagccaaccaaatgaaagccaagtatgcagaccaaatcaaaatcaatattggatttgaggttgacttcctgcctgactttgtcgattggactcgcgactttttgaacgaatacggcccgcagacaactgataatattttgtcggttcacttcatgcaaggagcaaacgataaattctggtgtgtcgatgatactgtgggagatttccaggccggattgttgaatcaatgtcccgactcacaagtcctatatgaacattattttcaaaccgttctggcctccgtgaatgctgacttgggtccatacactcccaaccggattggccacatgactttgattaaaaaattccaagattattttggcttggatcgtcacttttctgaagacaatctaagactggttgatcaaattctcaaggcggttagcggccaacaccgtgaactggatttgaacgctgccgggttgtacaagccttactgtaatgaacagtacccgtcatattcagttatccagatggcaaaatcgttaaacatcccatttgtttatggcagtgatgcccatagtattgccgaagtcggtcagggttataatggcgtgatttcattagttgaataaatcgcttgacaatcgatggtttggtgataatatatgaaactaaataaagtaaaagttaatataataaagttttgattagaaaaagtaactagtagtaatttaaaagagagtgccattgctgagaaggcacattttacgctggcgaacacacatctatgaactaatcggttgaaccaagtaggccggttcgcatgtttagcgttatcagggttaccgtatctgttatcagaggatgactagatattggcaacgtaaggccgactactgtgaggtagcggcaaattgaggtggaaccacgactttaaggcgtcctcgaagactgaatacagttttcggggactttttttatcgaaataggaagtgacagttatgaaaaataagaatttaccaagcggcacccgtgacgaatttggcacggaagcggaagtcaaagaaacgattcaaaataaactttttcagggctttcggcggcggggatttcgtaagttaaccaccccggttttagaatattcagatgtttttcaacctctgaatgccgaaaattatcgtccctaccaattattggacgagcaaggcgaaccactggttttacggcccgatttgaccctcccggttgcccgagtcatgagtacgaccggcattgagctgccagtgaaatggtattacggcggcgacgttttccgagtgaagaagcagttatccggaagttataaccaattaactcaggccggaattgaaattgttgggtacaagggcttgaaagccgattgggagtgtctggaagttgctttagcaggatgtcgggacatggccatcgaaaatgtcacgattgaactgagtcacgccaagtttgttgatgtgctgattgatcagctggatttgccggaacccaccaaagctggtttgaagcaagcgttgttcgccaaagatctcagcaagtacaaccaactcgcacagccactggcagaaacaccgttttcatcgttcatcaatgaatggccgtggttgtttggcaattttgatgaggtgatgaaagtcgttgataccttaccgccgattgaggagctgaagggaatcgttaatcacttaaagtcaacggcggccttcatccaacagttattccccaaagtcaacgtcaccttggacttaagcattccttctccacagagctattacaccggcatggcctttcgcggctttaccgataaatcctcaggctatttattcagtggtggtcgctacgatgacttattaaccaatttccaaaatgtcaaaacgtctgccgtgggagtggcattcgatgtcgatgccttggtcgaacggactagcttcccagacgacacaccgaccacgttgatcttctttgaggatgaccaatggcaggaggcagaagcggctttatccaagttcgccaatgcgaccctctgtctgaccgacgattttgaagatgccaaacggctggcagccagcaccaatagtcaactcattgatttaacaaaagcaggtgaaaaatgatggaacgaattaaaattgcccttactaaaggccgaaccgaagatcaagtggtcccgttactcgaagcagctgggattaactgcgaggggattcgcaacaagcaacggcggctgattttcgatgaagatccccgttacgaaattatcttggttaagggcccggacgtcctcacataccttaacagtggttcggttcaaatcgggatcgttggcagcgacatcctggccgaacaggaaaatttccaatacgcaatgttggatctcaatgtcggcaagtgccggtttgtcttggcatcaaccaaagatttcaatccccaggcccatcggcgaaaaataattgccaccaaatatcccaacattaccaaacgttatttccaagggattggcgaagacgttgaaatcatcaaaattgaagggtcagttgaactggcgccattgattggcttggccgatgcgattgtcgatattgtcgaaactggcaacaccctgcgtgaaaacaatctccaagtcttcgcaaaactacagccggtcaacaccaaagtcgtggttaatcgattggcacttcgccagtatcaacctcaaatcaaaagcttaattgccagccttgccaaggccgacgatcaactgatccaatccaaattaattaaggagtgagtaaaatgcgaacagcaacgatttctcgcaacacaaatgaaacccaaattgaattaagtctcaacttggatgactattcaaagattcaaattgataccggaattggctttttcaatcatatgctggatgcatttgcccgccacggccgcttcgggttggtggtcaaagccaaaggagatttagatgttgacccgcatcacaccacagaagacgttgggattgctttgggactggcactcaaacaggcgttaggcgataaagcaggcatcgaacgatttggctccgccttaattccgcttgatgaaactctcagtcgagtggttatcgatttgtccggccggtcttatctggtatttaaagccgaatttgccaacgatcacctgggcggctacgataccgaagtcaccgaagacttcttccaagccttcgccttcaacgctgaaatgaatcttcacgcagaagttttatatggcagaaatacccaccataaaattgaaacacttttcaaggcactgggcagatcccttcgagcagctgtgaccatcaatccagaaatcaaggggattccgtcgactaagggggttatctaatgatcacaattattgattacgacactggcaatacccgcaacgttaaaaacgccttggacttcttgggcgttcccaatcaattatctgccgatcccagtgagatcttgacggctgatgggttgattctacctggtgtcggcgcctttaaaaaagccatggattctttaaatgaacgtggcctggttccagtgattcaacaggctgccgatgcagaaatcccaattttagggatttgcctgggaatgcagatcttgtttgataaaagttatgaatttggtgaatcgaccggcctggggttaattgccggcgaagtggtgccgattcctgagaatttgggggtcaaggtccctcacatgggctgggatcaaaaccagtctcagcagaccgatgcacttggagatgggtttgacggtcagttcagttactttgttcattcctactacgttcaaacggcggctgaaaacattgtttcgacagtcgattatggcgtccagattccaagtatcgtgcgaaaagacaatgttattggttttcaatttcatcctgaaaagagtggtgaagttggactgaacggtttggcaaaattcaaggagatggttgaaaatgcagattattcccgcaattgacttaaagaatcaacaaagtgtccggctttaccagggtgatttccagcagacaaccgttattagcaagtcgcccttacaacaggcattggcaatcgattctgccggcttaaaaaatttgcatctcgttgacttggatggcgccaagtcaggacggccggtcaaccggtccctgatcgaacaaatttgcgcccaaactgatctcaaagttgaagttggcggcggaatccgctcactctcccaaattaatacttacctcacatcaggcgttaaccgcgtgattctggggtcagcagccctgaacaaccccaagttggtgcagcaggccatcgaacaatttggtgccgatcaaatcgttgtcggcattgacggcaaagatggtcgggtggccgtttcgggttggctggaacaaagttccgtggaaatgggtgaactgatggcttcaatggtggcctttggggtcaataccttcgtggtaactgatatttcccgggatgggacgatgactggtcccaataccgctcagctcagcagtctgcaggccaaattccctcaagtcaccgtggtggcttccggtggcatccgtaacgtttccgatcttgaggatttgcaaaccgctgggattaaggccgcaattgtcggtaaagcaatggctacgggtgatttgccgctcgatgtcttggcggaggtgaataccagtgttagctaaacgaattattccttgtttggatgttgaccacggccgagtgaagaaaggcgtcaacttcgtcaatttacaagatgttggcgatccaaccgagattgcggctgcctatcagcagcaaggtgccgatgagctggtgtttctggatatcaccgcgaccaatgagaagcgtaaggcgattgttgagaccattgaaaaagtcgccagccaagtcttcatgccgctgacagttggtggtggcatccacagcgtcgacgatatgcaaaatctgctgaaagccggcgccgataagacagccgttaattcagccgctgtcagcaacccccaattaatcacggccggagctgaaaaatttggcgctcaatgcgttgtgttagccattgatgccaaatggaatccagaatccgggcagtatgatgtctacgtcaacggcggccgtcaacgcacgaatttaaatgcgattgagtgggccaaaaaaggggttgcgctcggagccggtgaactcttagttaccagcatggataaagacggcaccaagagtggttatgatattaacctgtacaaacagctaaccgctgccgtgaacgtaccggtgattgcttctggtggctgtgggcaactgggtgactttgctgaagtctttgaccaagcagatgttgacggtgctttggcagcctcggtctttcactttggtgaactgacgattgctgatgtgaaaactgatttacgcaaagacggggtgatcgtacgatgaaacctgattttgaaaaatattcagatggcctggtaccgacaattgtgattgatgacaataccaaacaagtgttgatgatggcctatgttaatgaagaaagtttcaatttgagtatgcaaaccagacaatcctggttttggtcccggagtcgtcaagaattgtggcacaagggcgaaaccagtggcaatacgcaaaaaatcgtgtcaatcgatatcgactgtgatgaagatactttattgatgaaagtgattccggccggaccggcatgtcataccgggcacaccagctgcttttaccggaccattttaccggaaccaaccaaggaggaataatatatgcaagatttagacgaactttatcaattaattctggaacgcaaaaacaaccccgagaagggctcatacaccgattatttatttaccaagggtctcgataagatcctgaaaaaagtgggtgaagaagcaaccgaagtggttgtggctgcgaagaatccgtccgatcccgactttattttggaagttgccgatttggcctaccatgtcgaagttctgatggcccaacgcggaattacccccgaccagattaagcaggagcttgccagccgtgaaggcaaaaaaagcatcaccaaggatcgtaaacaaattaaggagtggtaggaatggtcaaagaagccgtcaaaaatctgaaaccgtacgttcctgaactcactttggaacagctgaagaagcaaaaggggctggataagttagtcagaatgtccgccaatgaaaacgcctatggcacatctgccgatgtggccaaggcactggacaagtggcactatcgcgatgccaatctgtatcccgacagtaacgctgatgagctgcgggaaattattgcttcccagtttgatatcaacgccgacaagctcatctttggcaatggcttggatgaaattatcgaattgctgtcgcgggtgattcttgaacccggggatgaagttttggatccggcaccaactttttcagaatatgcactccatgcagaaattgagggtgccaagattaaatcggttgggttggacgactccggccggattgatttaaaagcaatggcccgctcaatttcttccaagaccaaaatgatctggatttgtaatcccaacaatcctaccggaacttttctggaggctgatgccatccgggcatttgtcgaagatgttcctgaagcgattacagtaattgttgacgaagcctacattgattttaccggcggcatccatgactcggtcatccagttgaccaaggaatttaagaacctggtggttttgcggacattttccaaggcttatggtttagccaatttcagggtgggctttgccgtttgctcagacccattaattggctatctgcaagcagcgaggttaccgtacaacctgagcacctttgctgaaattgcggcaaccgcggcctttaaagaccagtcattcgtcgacaataccgtcaaaaaagtgattgccgaacgcaaaaaatgggaacatttcttaatcaaagccggcttgccgttttatgattcggcaaccaactttattttcttccaagtgaagggtggggatgctgatgcgcttcatgaatatttgttggaaaatggttatctacttcggaacggtttacgcaaggactggctgcgagttaccatcggcagaccggaagacaatcaagccgttcaaaaattgattgccgattatcttgcttaaacatttacttacaaaaagtagcattcatttcgagaatgcgttaatattagttttactggaaattacgaccttcaactcgtggattctccagaatctaattgaaatgatggtggttttatgcaagacaacagtcaaacacgtgttgttgttggaatgagtggtggtgtcgactcctcagtcgtcgcttatctgctcaaacaacaaggatacgatgtgattggcgttttcatgaagaactgggatgatactgatgaaaacggcgtatgtactgcaactgaagactataaagacgttgctaaagtcgctaacaagatcggcatcccatattattctgtcaactttgagaaggagtattgggaccgcgtgttcacttacttcttggacgagtataaaaagggcagaacccccgatcctgacgtgatttgtaataaggaaatcaaattcaaagccttcttggattacgctttggaattgggtgccgattacattgcaaccgggcattacgcccaattaacccgtgatgcagacggtcacaatcatttgctgcgggcatccgatggcaacaaggaccagacctacttcttgagccaactttcagctgaccagctggaccgggttatgtttccaattggtaacctggttaagccggatgttcgaaagattgcccgcgaggccggcttggcaactgccgacaagaaagactccgttggtatttgctttatcggcgagaagaacttcaagaacttcttaggccactatctgccagcaactcccggcaagatgatgaccgttgacggtaaagttaagggtcaacacgatggcttgatgtattacaccatcggccagcgccgcggacttggaattggtggcgatggtgttgataaccagccatggttcgttgtcggcaaagatttaaagcaaaatattttatacgtgggcaagggttatcacaatccattgttgtatgccgattaccttgaggcttcagatattcactgggttaataacttggaccgcggcaaggacttccactgcaccgctaagttccgttatcgtcaaaaagataccggcgtgaccgttcatatcagtgatgacggccagtcggttcgcgttgattttgacgcaccggttcgtgcaattacaccgggacaagccgttgtcttctatgatggcgacgagtgcctcggctctgcgattattgatgcggcttacaagcaggctaaggaattacaatatgtttaatctgaaaaagttgacgattgccgtcaactttttttgtggacagattgcgcttgtcagaaaatacaactgtgactcctggataatcgttatcatcagttgttacttttagttgagctttaaaaataaaacaaatttttcattataaatttcgttaggcttttgaaatcaaaccgttttcctgtcataatgtaagaagctaacagcagtttggaggaatgtcatttgactaagttgtactttgttcgccacgggaaaaccgaatggaatcttgaaagccgttaccagggtgccggcggcgattctccgctgctggctcagagttatacggaaatggatctgttaggcaaacattttcagaaaaccgattttgcccacgtttattccagtccgatcaagcgtgctcgggtgacggcggctcgaattgaccgcaaattaaagagccatccggatatttcactcttatccaggttggaagaatttcacttggggaaaatggaaggtcaaaagtttgccgatgttgagcaggcttatcccgaagagtttgaggacttccgcaaccatcccgatttgtacgatccaaaggccatcggtggggaaagttacttggatgtgattaaccgcatgacgccggcaatcacttcaatcgttaaggcctacccgggtcaaaatgtgatgatcgtcagtcacggggctgcgcttaacgctgagatcaatgcgttgctgggtgtgggactgcccaatttacgaaaacgcggcggcctggcaaacaccagcacgacgattttggaaagcacagatgaaggacaatcctatcaactgattgattggaacgacaccagttatttgaacaaaaaattagacccgacagatttggtataggtgacaatatggcaaataattcagataaaattaaaaaattacaagcaaaaaatcaagaaaatcagcgtaaatatactaggaagcgcgaggctgaagaggcgaaagccaaagccacgatccataagctagttgaaaaagtggatcacgaacccaacaattatcacaattactatgatttagccacgttcctggtcgaagctaaagattacgagcaggctgaagagcttttaatgaaggccctcggcttatttgacaaggccagccaagccgtcaaagatactttgaaatttggccttggaaatgtctactatgccgccgcagaatacgataaagcaattaaaatcttccaagaaatcgaagacaaaaagctgcaggccgaatcttacatcatgctggcccaaagctatatggccaagggtgacaataagcgggcgatggtctttgctttatctgctcaaagtgctcgccacgatgaccctgacgtcaaccaaatgattggggacaatctcttggccctgggcaactttgctcaagcgggggacttctacgatattgtcttgaaaacagagcctgaaaacggcaaagccaactttaatcgcggcctggttgccatggtgaatggcgaagattttgaaaactattttgcaaaagccaagcaggctgatccggcttattttgaaaagggtcaacaaaagttgaaagatattgaaaaagtgatccagatcaacaaagacaagccgaagaagtaaatgtcagcatgagtaaggaggaccgtcttggaccattcaatagatttatttggctcagaacagaataatcacgaaccacaatatgtcgatggccgattaaaggcgatcttcttttcgagtaatgacagtttttataaagtcgtcttagttgaaattacggagaccaatgtcaattggccggaagacgaaatcgtcgtcaccgggaactttggcgatttggttgaagaaaacagctatcatttcaccggaaaactggtcgatcatccccgttatggcaagcaatttcaagccagcaactacaccagtgtgatcgccactaccagagaaggggtcgtcaagtatttatcaggcgatcagttccccggcattggtaagaagactgccgaacgggtggtggatgttcttggcgatgatgcgattgaaaagattaccgcggataaccgtgttttggatgatgttcccattagcgccaaactgcgatcggcaattattgaaaatcttgatgccgatgataacttggaaaagaccattgttggactgaacagctatggtttttcgagtgcgattgcttcggccatttaccaaaaatatcatgaagatgctttgaaaatcatttctgataatccctaccaattggttgaagacattgacggcatcagcttcaagaaagccgatgccattgcccttcgattggggattgtgccggattccaacgaacggattcgggccggattgatgtatgcgattgatgaattatgccttcaaaatggggatacatatacgacgacggccccattgattcaaactgcctcgagccttctggaggggaatgcccagcagcagattcctggaaaaaaattggccgagagtttggttgagctggctaaagaaggcaaggttgtcggtgaagaagaccgcatttatttaacccggctttacaatgccgaagttcaaattgccgatcatttgaaccgggtaatcaaaaatcaggatgatgaagatcagctcaaagaagatgcgatcaaaaagcaattgcgagtcgttgagaagcagttcgatattaattatgatgattcccaagttgccgcgattgtccaagcgatccagtcaccggcatttattttaaccggtggcccgggaaccggaaaaaccaccattatcaacggcattgtcaacacatttgcccgactacatgagtattcactggatattaattcctataaagacaaaccgtttccaatcgtgttggccgcaccaaccggtcgagccgccaagcacatgactgaatccactgggttgccagccagtaccattcatcgactgcttggtttgaacggccgtgagtccaatgacaccactggtaccaaggatattgaaggtgccctattaatcattgatgagatgtcgatggttgatacttacttgttcaggtcgttagttcgggcaattcccaaccatatgcaggtggttttggttggtgaccaggatcaattaccatcagtgggaccaggccaggtattccacgatttgctggtttctaagcagattccggccatgcagctgaatacaatttaccgccaggagaagggctcatcgattatccaattggctcacgatattcatcgggggcagctgtcggaaaatttcactcagaaccaatccgaccgctcgtttatcccgtgcaacgaataccagatctcttcggtcattgaacaggtcactaaacgtgccaagcaaaaagacttcggcttgatggacgtccaggttctggcaccgatgtatcgcggtcgagccggaattgacaggctaaatgacgtggttcaagacgtttggcagggtgatccaactggtaaaaagtcggttacgatcagagaacacacttatcgaattggcgacaaagtgctccagctggttaataaccctgaaaataacgtcttcaatggcgacattgggatcattgtggggatggacgcccctaaaggacagcaagtccccaataagattacgattgattttgatgagaccgaagtgacctatgagaaaaatgagtggacccaattcaccttggcttactgcacttcgattcataaagctcagggtagtgaattcaagatggtgattttaccaatcgttcgccagttctcccggatgcttcagcgcaacttactgtatacggccgtgacccgggccagcgactttttgattatgctgggtgaaaaagaggcctttgagcaatgtgtccgcaacgtgtcggttaaccggcagaccagtttggtcaaacggctggtcgacgcaattggcattcagccgcaatcaaaaggcacggacagagagccggaagctgaggatcaaaagcaattgccgactgacacgcaaccagcccaagagactgatgatgctaaggccgataatctgcccgatcatttaaccacagcggttatcaatcaaaatctgattgacccgatgattggcatgggggatgtcactccccgcgatttcttgaagtcataggtttatcagtgaattcttaacaagttcaggccgaaattatggtagaatttaaataaataggtaaagaagaatacttggaggaaatcatggccgaatcaaaaacgcatcccaatcttaaattattttctttgaattccaaccgccacttggctgaggaaattagtaaagcagtcggtgtgccgcttggcaagtcaacagttgaaaagtttagcgatgacgaaattaaaattagcgtcgatgagagtattcgcggcgatgaagtttacatcatccaatccgtttctgatcccgttaattctaatttgatggaattattgattatggtggatgccgttcgtcgggcaagtgccaagtcaatcaacgtagtgattccttattatggctattcacgtgccgatcggaaagcgcgctccagagaaccaattactgccaaattagtcgcttccttcttagagatggacggcgttgatcgcgtggttgcccttgatctgcatgctgatcagatccaaggcttcttcaacattcctgttgaccatttgaaggcggatacgctgctggcagactactttgttaaaacccacaagagttccgatgttgttgtcgtttcaccggaccataccggtgtttcgcgagcacgaaaattcgctgaacttctgagtgcaccaattgcgattattgacaaccggtcgccggaagatgccaccacggttcccgaatcagttatcgggaacgtgaagggcaaacgggcgattattgtcgacgacatgatcgatacggcatttaaattgacaattgctgccgaaaccttaaaaaaggccggcgcaaccgatgtctttgcgattgcaacccacgctgtcttttcaggggatgcccaacagcggcttcaggattcacccatcaagaaggttattgtgacagattcaattagtatttccaaagctgaccaatttgaaaaactggaagtggtttccgtgggtcaattatttggtgaagccattaacttgattcataatcacaaatcggttggtaagctgtttggaagataaaatattttacgaggtggtttaatttatgtataaggcaaatgacgatcgttatgaaaacgcagtggtacgcagagctgggaattccgggctccaactgccggcactatcattcggattgtggcatagctttggcgatgacgccaactatggcgacagcgagaaagtcattttgaaggcctttgatttaggaatctttagctttgataatgcttataattacggcccaagtgccggcgctgctgagcggatgttcggtgaagtttaccgtgccaacctcaagccgtaccgcgatgagctggtgattaccactaaagccgggtttaatatgtggcccggaccttatgggaacttctcatcaaagaaaaccttggttaatgcgcttgacggcagtttgaagcggatgggcttggactatgtggatatctattacagccaccggtttgatcccaataccagccttgaagaaactgctgaggccttggatgagatcgttcgttccggaaaggcgctctacattgggatctccaactacaatgccgcccaaaccgctgaaattatcaaatatttcaaggaactccatacaccattcgttgtgaaccaggcatcgtataatatgctcaaccgcggtatcgaagaagatggtctgctggatacattgagccaaaataataaggcgctggtcgcatacggaccattggctgaaggcctcttgaccgacaagtatttagacggaatgggtgatgacgttaagattcactggagtaatgaatttgtcatcaaacatggtaaagacgagttggtgaagaaattaaatgagctcaatgacattgccaagaaccggaaccaaaatctggctcagatgtcattagcttggctcttgcacgatccaacggttgtcagcgtggttactggggcctcgaagattaatcatctggaagataacctgaaagcactcaacaatcttgactttacgtccgatgaattagctcagattgataaaatcgttaaagaataattattaggttgttcatacatgtttgaaataagcattaaattgggattaaaccggtttaatgctttttatttggtataatctaatcaaagacatttgcccgtgaatggagaataattatgacaaagaaagtgacaattactgatttagccgctcgtgcccaggtctcagtgacaacggtttcacaaattctcaatggtaaggctgcccgttttagcagtaagaccgttgagaaagttaagcagttgcaaaaggaaatgggttacgttcccgactttaacgcgcaaagcttgattcgtaaaagcggtcggacaatcggtgtgatcatccccaacatgaataaccctttctttagcagagttttacttggcattgagactgaggcaattaagcaggactatgtgccccttatttttggctctaacaacagtcagtcacaagagacgcactatctcttcgaatctgttcgaagggccgcagacggcatgataatcgcttcagcggtgtccgacattaattatattgataatatcttgaatcaaaacggcattccctatattttaattgaccaggcaccggtggttaagggtgatcgggttgatgccaataatcaaaagggtggggctttactagccgattatttaatcaagaatggtcatactgatgtcgcggttgtctgtgccaccaaaccaaccctcaatcttcaggaacggctggctggatttgtggaaacctacaaaaacaacggcaccccaattcctgaagaccgaattattacgactgagatgaccaaaaaagggggttacgctgctacgaaagcagcgttagccaccaagccaactgcgatttttgggatcaatgacgaggttgccattggggtctatcgtgggcttgaagaagccggcttgaaaattccaagtgacatttcggtggttggatatgatgacattgatttgggagagtacatttcccccaaactcacaaccgttcatcagcctgcttttgaaatgggaaccaacgccgctcaaatgatcatcaagcgaattgaagaccataatgagccaatccaacaggtttccctgccggtatccttggtagaaagagatagtgtccgggcaattaactaactgggatagttgttaaatttcaggaaatttgatagaatttggttaaaggttttaacacactatactaagggatttagaggagcttattatgacaaataaagtggttgtgctcggaagtctaaacgttgatacaacattgcacattgaccaaatgccaaaaccgggggaaacgattagtgccaagagtaaaaccaattccgctggcggtaaaggggccaatcaagcagtcgcagctgcccgttccggtgctcagacgagttttattgggcaagtgggtgatgatagcaacggcatctttatgatcgatgctttgaaacttgacggcattaataccgatcatgtgggtatcaatcaggttgatgggaccggttctgcggtcattcttctggacagccagggtcaaaacagcatcatggtttatggtggggccaaccaagccatgaaaactgaagtcattgccgacagccaagccctgattaaaagtgccgatattttaatttccgaatttgaaacaccgcaggaagtgacctacgaagcgttcaagttggccaaacaacacggcgtgaccacgattttaaatccggcaccggcttcaaaaatcatttacgggttgctcgaagtcaccgatttaattgttcccaacgaaaccgaaagtgccacattgaccggtatcgaagtcaacgatactgattcaatggatcaaaacgccgctaaattcagcgagatgggtatcgacaacttgatcattactgtgggcgatcgcggcgcgtactatcatactccaagtgacagtgggtttgtgccggcgttcaaagttaaggcaaaagacaccacggcagctggtgacacatttattggggctttcagttcacaaattgacaaagatttatccaatattgaagccgctttggtttacgctcaaaaggcctcatccattacagttcaacgtttaggggccttaccttccattcccacggccgaagaaatcaaagcagaatacaaataaaaattatcttaagtattagtttaatttttcttccaaactgttttgcgagtagggtgttgctttctcgaattttatctggtagtatatccagacgttagcaggaaatgttaaaaaattgataacattcccacgttagaaatcaggattgacgattcgaaattcaaatttcatgttcaaaggagtttatagctatgagtaataagttagaaattctgagagaataccaaaaggcatcctcgaagcttgatcaattaaagtccgaagaagcagacaagatcaagtctaccccagtgaatacgagttctaccgaagtaatcacaccacagtttggcaacgaaatgacgcatttgaatgaagaatgcatgcagttaaacatgatcttagaagcaatggatgcttcggaagactaggtcgtgtgaacgcgggatcgtctattgacggtgccgtttttttgttacaatccagtgcccaactggtctacggaaagccaaaacaagagcgtgggccaataagcggttagcttccagagtataaggggattacccgaatatccagaacttggatgtttgggtaatccccttatatggccggaagctgcttattggcgcacagttctgctagataacattcaggcgcaaaacgaggctggaacaaaatttttagttttgtcccagcctcttgttttggccttcagtttttattttttgaattttaatgggcaacagccaatcggcctcaaaaattgtctgatagtaacgccactgacaccgcacttttaatctgatttcttccctggagctttgacagccagttttcagggaacgtcaccggcgcaaagagtagtgatgccagcatggaagtaattgaaccgatagtatcggcgttactgccaagattgacagcctttgacacggcaacgttatattgttccgaattcatcaggcaccagaaaacggcgttgagggtggcgatcacatcgctggagggccttaacttcgtactcgactgtcggaggaagtgagactcctctaattgctcaaaaaacggcacctgagcggcgaattgatcttttgagcggtaatagtccagggattccttaacggctcttagcatggcgtatttgttgggattttgaatcaggcgaataatgacgttggttaaaacgccggaaccaataaatgtcttgggggttcggttggtggtagccgtgtaatcatgaaccatgtcggcaacggtttcattaaaggtgtactgctggttcttcgttaaaatataaaaggctaacggcatcaaccgtttaagggcagtattgtcattgtctgaatccaaagtgccgccggacaaaaccggtggggtgccggtatcaaagcgttggatggctgctttggtggtctcatcaacgtcgtatgcataattaaagggcgtgtaatcaccaaaatggacccattgcgaataacgtgtcatgaggtcataaagattatatccaaacgttaagctaactaaagaagcaattgatagtgatgtatcatcagaccaagtgccggctgggatttgattcgtccggtgttcgaccatctcatggattggatcatcgaaggggttcaggcgggtatcgtgttgaatcggatatccaagcgcgtcacccagggcaactgctgttaatgattgaaataaaaggtagctggtggaatacatagaattacctcgtcgttagtttttcgcggtactgaaacttaccgaatccagaagggatatttaaccgtgtcaagcttcaggttaaaagtccgctcgccaagttcttcgccatcgatttgacccaaacgattaccatttgtttttataaacagctctttttcatgataatgatgaataaatttaagccgtaagtgtctctttaaaaatatcatagatacaaataaaatcaattgccaaaggctgggtttttcgaccactactaaatccagatggtcgtcgaacactgatgcgctgggcatgatgttgatgcctccgccgaaataaggaatatctgttgtggttaataaaaatgtgttatcgaatgtgactttaggcatatttcccgggagaatttcggtcttgaaccctttaaagtggatgatcacgtttaatatagccgccatgtatgaaaattgtccgaagaattggtgactttttaaagaagaatgatttgcgaggtgcacaacagtggcgtcaaagccgatgccgaaattgttggtgaagaagccttcggaatgatgatcaaggtctgtgtagtggccgacattgatggttttagcagctgattgggtcaaaatgtcagccaatgctttttcccagtgcaaaggaatctttaatccccgcgcaaaatcatttccggaaccgaccggcaaaaaggcaattggaactggatgatcattttgatggacgcggtagtagtgctgacagcccaacagtgtttcgtgaagggtcccgtcgccgccagctgcaatcaacacagcgtcagtttggttggcggtgtcaatttcactgagagcttgttcggctagttcaacagcatgatttgggtaggcggtatagagtgtctgataatctgcatgtgcagccgccagttgtttttggatatccggccaaacctttttggcgttatcaccaccggcatgcaaattgataatgatgaaatatttcattggtgaatgagcccccaactcagatggttttatgtaaaaaacttgagaatcgaatataaaatctatccgcttctcaagttttcgaattagtcacgtttagttttgttaatctttaccattcatgatgagcattggcaaaatcattggatggcgttcggtcttgtcgtaaaggaattcttgaagatcatcaataatcgcatttctaattgaagactcggttgcttttttagcacgcatcgactttcgaatggtcttaaatacgcggcgtcggccttcatccaaaagttcaccggattctcgcatgtagacgaagccacgtgacaagatatctggaccggattggatttcctggttggccaagttgattgttgcaacaaccacgacaataccttcctcagaaagcagttgacgatcgcgcaagacaacgttaccaacatcaccgatgccgctaccatcgatgtaaacatctccggcagtgaagtgaccagccatacgagcattatcttttgaaagggcaaggacatcaccattttgcatgataaagctgtgatcaagcggcacgccacattgttcggcaagctcagtatgaattttcagcattctgtactcaccatgaatcggcatgaagaacttcggcttcatcagacgcagcatcaatttctgttcttcttgaccaccatgtccggaagtatgaatgttgttcacccgaccgtgaatgacattggcgccggcttcttcgagcttgttgatgacgctgttgacactggtcgtgttaccaggaatggggttacttgaaaagataaccgtgtcaccaggctgaattgaaatctggcggtgggtaccgttcgcaatccgtgaaagggcagccattggttcaccttgagagccggtacacaagatcaaagtcttgttagctggcagtgactgcagctcatgtgcatcaacaaacgcatcatcaggaatatcgagataacctaattcgcgtccattcacaatcgctgcatccatgctgcgcccaaagacggcaatcttgcgaccgtgggccatggcattatcacaagcggttttaatccgtgaaatgttggaagcgaaggttgcaaagatgattctgtcttcaatattatcaaaaatgtgggcaattgaagttccaacccacttttcagatttggtccaaattggcttttcagcgttggtgctgtcagacatcaaacaaaggacgccttctgcacccaaacgggccatttcctgaagatcaggcggctggttggtcactggtgtgaggtcgaacttgtaatcaccagtttccacaatcacgcccaccggtgtatgaacggcaattccaaccgtatcagggatcgagtgggtggttctgaagaatgaaactttcattttttggaacttgagaaccgacttgtcactaatttcgtgtaattcaacggaattcagcaagccgtgttcttccaatttattcttaatcagcgccatcgcaagtggtccggcataaatagggacgtttaaaaccttcatcaaatatgggacaccaccaatatgatcttcatgaccatgggtgatgaccaaagctttgatcttatccttattttcaaccagatactgatagtctgggatcacataatcgacacctaagagatcatcttcggggaacttaattcccgcatcaatcaggataatttcatcctgaaactggatcccgtaagtgttcttaccgatttcacccaaaccaccaacgccatagatagctgcttcgttattcttgacgtttagttttttcatttattattaaactccgttactttgtaatcaggactactttgctcatactccaagtgctttccttggaggggttcgatgaattcaatatcataatcagtattgtcttcaactaacgcgtgagcttcaacctctgtgtcggcctcaacatagagtgaatgagtcgtttcccggcgagggctttccttcttgctgggttgatataaaaccttccaaatcataaaaaaactcctttaaaattatacaatttttttgcagaaactcgaggtttccttacggacaagtggttgtgaaaacacaactaataacgatattctaccataatctaaaaaataagtatataaacatgaaagtaatcaactcgcaccattgcatggtaaaattaaatcaatgaaaagaaatggggctcagttatgaacattgatttgattattcaaattatcatcgggttggtcgcagcatttgctgtttacaatttgattcattatatctttgtaacgagacccggcagaaaacggctggcgttggcacagcggattgccaatgaagctgtgaaaacttcgattaaccagctggttgaccaaaaggcggttttgccctttgatgaaagtgattttaaatctgaagatattgccgaagtgtggggcagaggtgtgatggcatttgaatatcatctgcccaaggcaaaaattgaaagttcaattcccgatttccgaaaggccttggcaacgacgcttgagcaatacggtgatacacaccacatgcacgcgcataccgatcaggctgatcggccggcgtttatggtcaccgatgtctggcagctggatgatcgggtgcactttgatgttgcctacctggtgaacgtgacgacgattgaatatgtggatgacttaaagcggctgcactgaaccattatggactagtcaacggcgtttgcttttcgatactgtttggccagtcgcttgcgtactttgatgattgcaagtagattatgatccactggcggggaatatagattttcaacagcgaccagcttggcaatcagtgccaggccttttttctcactgccaaaatagagctgccagaccgcggtgatcaattgttgttggaatcggccattccaacttaaatccagggtgttgacctgacggattttgtttagaatttcttttgccgactgatattgagccaagttgagctcgatttgaaaaagagaaagataaagatccattaattcatcggcaatatgaaatgggtcatccactgcttgaaggtattgtcgacaattgttttcaaatctgcgaacaatctcggaaataagcttttcttgatgccggctgaccgcaattggcagtaaaatttgggcctgcctaatttcttcaagtgtccaggtctgtgatgcaaaaagggtgtcccagagattttccattgccggagtgactgtgaatgtttttgaataataagtgacgaccaatatttgacccatagcagcaaccgatttgtaactgaggcggctgcttttttgcgtttcagcgatgatttggcccattgtttgaaggtcgtggccgttataggcccgtagcaggcgccttttcagtgatgttgcagtgggttcgtgataatcgttttgaataaaacggaattcgttggctgaaatggacagattatctaaaattttaaataacttggcggcactgatgtcgttctccccattttcaaagcgatgagcaaatgaacgtgacatcacgcctgagtacacttcgctttgagtgaatcctttaatttgtcgaatcattttgactgtctgcccgattgttttcatgattgcctcccaagctttgaatgtggcatatacgcaacacattttacatctatcgctttaataatggtagtaggcttcagttaatcaaaattaaagcgggtgctgacaatggaaattagtgatcatgagtcaaatatgcaggttataaaagatgtatcgagcaacttcaccagtactttttgtggcgacatgttttcatttgctctggggctcatgctgctgcgggccacggggatgtcgttaagctttggactctcaatgattatcatgccgattgtgaccttgatcgggttggtgccgattggcaacttggtcgacacttatccccacaaacggcttttgattattagtctggtcgtccggatcaccgcactattcatttattcgatcgcaattggtcacttcgatggcagtggtaaattaatcccaacgattgggtttttgatcatcaattacgcatctgtcaatctttcgaattccggctacatggcatcggttcacgaattagtcaacgagggtcatattcaaaaattgaattctttgagccaatctgcggcatcgtttgcctcgaccttttcgccgattgtggccgccggattgtatgtgatagttggctttaggctgtttatcgtctttcagctgactgctcacgtgattgccctgataattcttttgacgatgaattttcattatttgagctatccaaggaaaagcagtcagacaccgcaggaatcccagtgggcaaaattcaaactggggttaaattatttgatggcccacggctttttacggtatctcatctgtattgccctgtttttgaattttatttttgcggtcattaacgttggcctgccatttatgattgtggaacatttacatttgggaaacgtgacgctggggattttgaattccgccgatgcccttggcatgctgatcgggaatttgatcatcagtgtctcgaaagaattgaggcacttggcaaaaatattagctgtcacgatggtcatcattggtacggggttggctggagttggcgctttattgatggctgctcccgaacaattagtggtccaattggtgggctcgttgatgttgtttgcagtggggatgtcactggcttttatgaacacgccttttggtatttacatgcaaaaaacagttccgactgaactgatgggcagagtctcgtctaccgaaatgtctttgaatatgatgtcaattcctttgggaaccgtcttttattcatttgttttccaacagattccaagtggaattgtgttcattatatctgggatagctctgattgctgtcacgggattgacgatgccaacttttatgcatgtccagatgccaaagactggtcatgccacccaaaaggcggatcgtcagcgtctctaagttgagtttgtcgggtaatatgtctataagtaaaacggtttgttacaaattcaatgaaaaagaaccagcaacttacaaaaagttcatttgatatttgttcacaaggcataaccaaacagatctaattcaggaaaggccactcgccacaattaaattggataagaaaaaaaccgggcaaaagtttttccttttgctcgattttttaatatggatgcttattgaaatttcttagatcggcatatgaacaactgatttggtgcaccgatcaatacacaaagatttcgtcatctgttttggcaaatgggttgtccttattaatgtgatcataaaagagtgttccatgaaggtgatcgatttcatgctggcagacaattgccgggtaatttttcaatcgaaccttgtgctctttgccgtcaacgtcttggtattttaaggtaattctggcagcccgagggacatagccgggaatgtccttatcaacggacaggcagccttcgccctctgtcaatgcgccacgctgaaccgaattcgacacgatcaccgggttaataatgacatctttgaaaaccggttcatctttttcatcctcgtcttcacttggaaccaacactgaggccatcatttcagagacaccgacctgtggggcagccaagccgacgcctgcacgcagacctaacttttcacactgttccggatcctggctgacttccagatattccatcagatcatgagccagttgtttatcttctttgctcaaagggaatttgaccttttgagcttgtttgcggagaaccgggtctccatctcgtacaatatccttcattaaaaacacgctaaagacctccgaaaatattttaagcattaattgaataacttctattctaacttaattttaagaaaaaaacactattcacaaagtgggtgaaatttcacaaagtatactcccgcaagcggtttcaacccaaaatttgtcaagtgaaaattatattcaaaaaagttggtttcatcacaatgaaagggcttgcaaacgttgctgaaaaatgctaaatttaacttgtggtttagaagtgatcagtttgtacatcacaagtctagctttacaggaaaggaaagtgttatctatggcagcaaagagtaagcatgttgttgattttgccaagatcaaatcaacgatgagcgatccatataagaaaccggttcaagttattgatgaaagcggtaaaatagttaatcaagaattatttgaccaattcagcgatgacgaactagttacgctgatggaaaagatggtttgggaacgtgcattgcatgaacaaacaatgaacttttcacgtcagggtcgattaggtttctatgctcctacttacggtgaggaagcctcagaaatggggattgcccacgcaatgaagaaacaagactacctattcccagcatatcgtgatttaccacaattaatccaacacggtgcaaccgttaaagagggttacttatggtcaaaaggtcactaccaagcttatgactacgtacgacgcggtgtacgtgcatttatcccacaaattattatcggtgctcagtatgttcaatcagctggtgctgcattaggaatcaagaagaatggtgagaaggataccgttgcttacacatttaccggtgatggtggtacttcacagggtgacttctatgaaggaatcaacttcgctagttcattccaagctccagaagtattcttcgttcaaaacaacggctgggcaatttcagttccacgaaagactcagaccgccgctgaaacccttgcacaaaaaggtgttgcttccggtgttcctggtgttcaagttgatgggatggatattttggcaacttacttggttgcaaaagaagctcgtgactttgttgttgccggcaatggtccagcattagttgaaaccttgacttatcgtttcggtgcccacagttcagccggtgatgatcctagtcgttaccgtactaaggaacaagaaaaaccatggttcgaccgagacccactaattcgtttgagaaaagttttgactgacaagaaactttgggatcaagacaaagaagacaaattagttgctcaatacaaagatgaattcaaggaagcaatgaaggatgccgaagctgctcctaagcaaaaggttagtgacttcttgaagaacacatttgaagttccaaccccagatgtagcagctgacattaagaaatacgaagcaaaggagtcgaagtaatcatggctaaaatgacatatattaaagcaattaccaatggacttgaccaagtattacaagacgatcccaagactctgatttttggtgaagatgttggtaaaaacggtggtgtgttccggacaactgaaggacttcaagataaatatggtgaagaccgagtattcgataccccacttgctgaatcaggaattttaggaatgtcaatcggacttgcattaaccggctggcgtccaatcccagaaattcaatttatgggattcacaatggaagctgttgattctgtcggtggtcaaatgtcacgtaaccgattccgtttctcaggcgacgttacgatgccgatcacaatcagaaccccatttggtggtggtactcatactgccgaacttcacggtgactcacttgaaaacttgttcattggcatcccgggactgcgggtagtaactcctgcaaatccttatgacgctaaaggaatggttatctcagccgttgaaaacaacgacccggtattattcatggaaaacctgaaactttatcgttcaatgaaggatgaagttccagatggccactacactgttccgctagacaaggcaaatgttgttcgtgaaggatctgacattaccgttgttgcttacagtgccgaagttaacgaagcacttaaagtagcagataaattagaaaaagagaacatctcagttgaagttattgacttacgttcattatcaccaattgacgatgaaacaatctttgcttcaatcgacaagactcacaaagtagtgattgcccaagaagcacaaaagatggctggtgccggagcaaaagttgcttcagacattgctgaaaacgacattatgtcattggacgcaccaatcggccgtgtttctgctcctgacagtatcttcccatttgctatggctgaaaatgattggcttccaaatgctgatgatatcgaagctaaagtacgagaaattttaaactactaaaattctaatttgttacagaaaggaagttagatcccatggcttataagtttaaactaccagagatgggagaaggaattactgaaggtgaaatcgctacctgggatgtaaaagttggcgataccgtcaaggaagacgatccgttagttgaaattcaaaacgataagtctgtccaagaaatgccatctccagttgccggaaccattaagagtattgaaaagcaggaaggagaaaccgcagaaaagggcgacgttttagttgtcattgatgatggttctcctgatgaacctgatgatgccgcaccagcagctgcacctgcaaaagaagaagctgctccagctcctgctaaagaagaagcacctgcaccggctgccgcaccagcacctgccgctgctccagccgcagtaactgctgcaccagctgcttcaaatccaaacgcaattgtcaaagcgatgccatctgttcgtcaatatgcacgtgacaaaggcgttgacattactgctgttcctgccacaggaaatcatggtcagatcaccaaagctgacattgacaacttcaatccagctgccgctcctgccgcaccagctgccgctgcaaccgctgctgcacctgctggcgaagcaaaagctgccgcaggtcaagctatcaaaccttggaagtctgatcaacctgatcttgaaacccgtgaaccaatgtctccaatgcgtaagatcattgctaagtcaatgcgtacgtctaaggacattgcgcctcatgtaacttcatttgacgacgttgaagttagtgcattaatggctaaccgtaagaagtacaagcaagcagctgccgaccaagatattcatttgacattcttaccttacattgtgaaggcattggttgccgttatgaagaaatatcctgagttcaacgcttcaatcgatgacaccactcaagaaatcgtttacaagcattacttcaatgttggtattgcaaccaacacggaccacggtctgtacgtaccaaacatcaagaatgctgattccaagggtatgtttgagattgctaaagaaattaccgagaacacccaagctgcctatgacaacaagcttggcccagatacaatgaagggtggttcaattaccatcagtaatgttggttcaattggcggtggctggttcactccggttatcaaccaacctgaagttgctatcttaggtgttggtaagattgccaaggaaccatatgttgatccagaagacggcgagattaaagttggcaatatgctgaaactttcattgagctacgatcacagattaattgacggtgcccttgcacaaaatgctttgaattacatgaatcaattgcttcatgatccagcaatgctgttgatggaaggatgatcgaataatggctgatgttgaaaagaaagaaacagtaattatcggagctggccctggtggctacgttgccgcaatccgtgcatccgaattaggacaaaaagtaaccctgattgaaaaatcagatacacttggcggtgtttgtttaaacgttggttgtgttccttccaaagctttgatcgctgctgggcatcgtctgcaggaagctaacgatgcttcgacgtatggaattacaactcaaccagctacaatcgattttgctaaaacccaggagtggaagcaaaagaaggttgtcgaccgaatgaccagtggtgttaagatgctgcttaacaagcacaaagttgaaatcattcatggagaagctgttcttgacagtgatactcaattacgagtaatgcctacaggaccacaacaattcatgagtgccgataccggaaccacgattcagtttgacaacttaatcattgccagtggatcacatccaattgaaatccctggtttcaagtttgacggtcgggtgattgactcgactggcggcttgaacctgccagaaattccaaaagaatttgtcgttatcggtggtggctatgttggaaccgaattagccggtgcatatgctaacctaggtgcccatgtaacaatcattgaaggattggattccatcttgaatggatttaccaaagacatggtttcattagttgttaagaacttgaagaagaagggcgttgatattcataccagtgctaaagcaatttcttcaagtcaagatgacaatagtgtgtctgttacctacgaagaagagggcaagcagaccactatcaaagctgattactgcatggtcactgttggtcgtcgtcctaacaccgatgatcttggtttggaatacaccaaggttaagttggacgatcacggcattgtccaaactgatatccaaggcagaaccgattctgagcatatcttcgcaattggtgatattgcttcaggtcctgcattggctcacaaggcattcttccaaggcaaagttgctgccggtgcaatttccggtaagaatactgccaacgattatgttggcgttccagcagtctgcttctcagatccagaaatcgccgttgttggtatgactcaagcccaagccaaggataagaacattgaagtttccacttcgaagttcccattcgcaggtaatgcgcgtgccgtatcacttgatgaagccgacggatttgtccgtttgatcttcaccaaagacgataagacgatcgtgggtggcgaaattgttggaccaggtgccagtgatttggttgctgaattaagtttggcagttaacagtcacatgaatgttgaggatattgccctgaccattcatccacacccaaccttgagcgaaccagttcaagaagctgcagatgttggattaggattcccaactcatatttaaaaagttctgttttaattaatccggttaattccggaataaaggattcaatgatgaatgaagcttgttcatcgttggatccttttgtttatccagaattacgatctgttaagtcctccgagaaatgaaaaactcacataacttcgaccttttctatttcacaaagtcctcaactatcatataataaagtcaacttggtaatgatcggagtgaagaagatggccgaggggtatgagtacccactaattgatggtttggatgttgatgaaattattgacgttgttaatttttttgaggcaattgaacaggcgtatgaggaagctgaaggcattaaacgagcagactttatcaaagcttatcggaagtttcaagaggtggtccctgccaaaatggaacagaaacaattggagaaggaatttgccaatcgttccggatatgattcctacgaagtcataaagctttctaaggatgggcaggcagctaatttgaaggtacgtgaggcataggatggaaattaacgaactcaaacaaattgataaaacggttaaaggttggctgcatgagtcacgggacaacgttctaagaaaaattgacacccgactggaagttgatactaagaccagtcgacgtgatttggtgaccaacattgataaacaaaatgaaaagtttttagtcggtaaaatccgtgaatttgaccccaacgcccagattttgggtgaagagggatttggcgaccaggttcattcaacagaaggtcggatctggattgtggacccaattgacgggactatgaactttgtcaagcagcggaatcattttgctatcatgattgccctttatgaggacggtaaaggcctccttggctatgtaatggacgttattggtaagcatttgttgtctggcggaccggatattggcgtatttgacaacggccacccgctgccgcaagttaaggacacaccgcttcgagaagggttaattggcctaagtgggccgatggttcttcacaacgattacaatatggtagacattgcccaacagtctttgggaatgcgcatttatggcagtgctggaattgatattatttccgttctccgtggtgaattggttggatacatttcttatctcaagccctgggattttggggcaggcagaattctgtgcgaaactgccggacttaagatgacaactattgacggacagcgattagatgtgttatcatcaacaccagtattgttagcaacacgaaatgcacatcaagacattcttacaattgtaagtcaatgatcggactgtgacagttgtcacagtttttttatgcgaataatatgatgtacaatattcggtttgatttaaatgaagggaagcaaacgacttggatactaaattaaaaacacgcgacgacattcgtaacattgctattattgcccacgttgaccacggtaagacgactctggttaacgaaatgttgaagcagtcagatacgcttgatcaacacgtacaaattgaggatcgggctcttgactcgaatgcgatcgaacgtgaacggggaattaccattctgtcaaagaacacggccgttcgatatggcgacaaacaaatcaacatcctggataccccaggacatgcggacttcggtggtgaagttgagcggatcatgcgaatggttgacggctgtttacttgtcgttgatgctttcgaaggcactatgcctcagactcgtttcgttttgaagaaagctcttgaacaacacttaaccccaatcgttgtgattaacaaggttgaccgtgaaggtgcccgtcctcaagaagttgtggatgaagttcttgacttgttcatcgaacttggtgccgacgaggaacagcttgattttccagttgtttatgcgtcagctatgaacggaacttccagttatgatcctgatatcagcaaacaggaacatactatgaagccaatctttgacaccattgttaaagacattccagcaccaattgacaattcagatgaacccctccaattccaagttgcaatgcttgactataatgacttcgttggtcgaatcggtattggccgaatcttccgcggtacaatcaaggttggtgacagtgttactgttatgaagcttgatggttccaagcagaatttccgagttaccaaattaatgggattcttcggtttgaagaaggaagatatccagtccgctaaagccggtgatttgattgccgtttccggaatggaagacatcaacgttggtgaaacggtggttgatcctaaagatccagagccactaccaattcttagaattgatgccccaacactgcaaatgacctttggtaccaacacttcaccatttgccggccaagacggtaaattcgtgaccgcccgtcaattgggtgatcgtttgaagcgtgaacttcacaccgatgtttcattacgtgttgaagataccgaccaacccggttcatggattgtttccggtcgtggtgagctgcatttgtcaattttagttgaaactcttcgtcgtgaaggctttgaattgcaagcttcacgtccagaagttatctaccgagaaattgacggcacaatgtgcgaaccatttgaatccgttcaaatcgatactccggatgaatataccggttcgattattgataccctttcacaacgtaaaggtaccatgcagaacatggaaacaaccgacaatggtcagactcgtttgacattcttggcaccatcacgtgggttgattgggtattcaactgaattcctgtcattaacccgtggatatggtatcttgaaccatactttcgagaaatacatgccagttatcaagggctggaaccctggccgtaccaagggaaccttggtttcaatgaacgccggtaaagcaacgacctatgcaatgatgggtatcgaaagccgtggaacattgttaatcgatccaggtaccgaagtctacgaaggaatgatcgttggtgaaaacaaccgtgagaatgatatcactgttaacatcaccaaaggtaagaacctgaccaacgttcgtgctgccggttcagatgatatggcccggattaagacaccaactcatctttcgctcgaagaatcacttgaattcttgaatgaagatgaattgtgtgaagtaaccccacacttcatccgtttgagaaagaaaattttgaactcaaacacccgtgaaaaagaagctaaaaagaagcgtcataactaaaatcagtaaattatcaggaggggctgggacaaaactaaaaattttgttccagcctctatttgctcttgaatattatctagcaaaactgtgcgccaataagcagcttccggccatataaggggattacccaaacatccaagttctggatgttcgggtaatccccttatattctggaagctaaccgcttattgtcccacgctcttttgtattgaatggagtttgttgtaacttcttaaattcccctaaaccgtttagcaatctctgaatccggttttttaattatgatataataaagctcgatgcacctacatataatttgaaaagtggagttggaccaatggggaaagcacgtttaaaaaatctcgactatgttatttttattccgtatattgtgatgtcgattatcggtgttgtgatggtctattctgccagcgcaaatatttcgctgcagaacgggggaagtccgctgagttacctgatcaagcagttattctttgtcgtccttagtgttattattgttggcgtgatgacggcaatgaacattaagtacttacgcaagcccaaatttttgaaattcttactgtatgctttgattgttgttttgattggtctgctgttagttggcaaaactatcaatggcgcagctgggtggattcatttagggccaattaacatccagccggccgagtttgtgaagttctttttgatcatttggcttgccgacacaattgataaggctcaaccagagatcacgctgtcttttcgggactggtggaatcacatgaaatggccgttgtttttcagcgccgttttgatcgccttgattcttaagcagcctgattcaggtggtgctgccattaatttggcaattgcctttattctgtttaactgcagtggcttttcatggaaacgagctttggcaatcatttatggttgtatggtggccgccgtgctggcatttgaatttattctggtaccaatggccaaatcggattcgttctcccattcctatcaactgcaacgaattgtcgcgtttaccaatccttttggtcatgcgcaggggacaggtcaacaggtggttaactcctattacgctataagtaacggcggccttttcggtgtcggcctcggaaatagtgttcaaaaaaccgggtatctgcctgagcccaacaccgattttattatgtcgattttaaccgaagagctgggggcgattacggctgtcattgtgttggcattattgacagttatcattttgcgaacagtccaaattggtgttcgcagtaacgatacttatcaaagcctggtttgctacggcgttgcaacttatatgagtattcaaacattctttaacatgggtggtgttttgggggtcctgccaattactggtgtgaccttcccgtttatcagttatggcggttcaagtattttgaccctttcgttttgtttgggactggtactgaatatcagtagtcgtcagcggatggaacgaaaagcacttatcgctgccagaaattaaatttgaggagatggcataatggctttaactgttcaacctacgaccgggttaatcgtttatctacattcgattcgtcattccagaaatctgaagtcatatggccgactgtattacgtctccaaacggatgcgctatggtttgatctatgtgaacaaagatgatgaggaagagattactaaaaaattggcttctcaaagttgggttaagcaggtggtcccttcgcatttgaatgaattggtccaagaagttgaaggtaaaaccgagttggacgatgacgattcggttgacgaagattattagagttgaggtaaactatgaggattgtatcaggaaaatacggtggtatccgcttaaacccggtgaagagcgatcaaactcgtccgaccactgataaggtgaaagaatcattgttcagtatgaccgggccctattatcatggtggtcggttcttggatctgtttgcgggttcgggagcagttggcatcgaggctgtttccagagggatggatagtgctgtgcttgttgatcgacagtatcaagcgatcaaaacaatcaaagacaacattgccaaaattcacgctgaagatcagttcaccgtaattaaaggtaacgctgagacagttttaaaacaattagctgccaatggtgataagttcgaccaggtttttctggatccaccctataagcttcaaaagatcgttaacactttggaagaattgaaaagccacgatctgttgaatgaaggggcaacggtaatttgtgagactgataaccacactgaattgccgctcaatctcgatggatttcacgcagtcaagcaaaaaaattatggactcacaaatttgacaatttatgactatcaaatggggaatgtgcaatgacaaaagctttatatgcaggtagttttgacccgatcaccttcggtcacattgatgtcatcaaacgggccagccgaatttttgataaggtgtacgttgctatcagtattaacacccacaaacatgctttgttcaccgatgaggagcgggctgagtttgcccgccaggcattaaatcagttacccaatgtcgacgttgtggtctctgaagagctgaccgtccagcttgcccattccttgggcgcaacggtattagtcagaggcgttcgcggcggcagtgacctggattccgagatgtcaatcgcggggcttaacgagaagttggccgacgatattcaaaccatttttatcccaaccgcggccaactatcgcgacctatcgtcaagcatgatcaaagagatcgctaagttccatggcgatgtatcaaaatttgttcccggacctgttgcacaggcattgaatgacaagtatcaacaataaaatagtttttagagagtggtgaactaatgaaaaagtgggttaaaaaatatttaatttggtttgccattttactttttgtggcgatcggctttttgtggccgcttcccaaatacattgagggacctggtgacgccgctaatctgagtaaaattgtgaacatccaaggtcatcccgaccgacagaaaggtcagtttatgctgatgtctgtcagcatctctcaagcccgaccatttacttatctttatgccaagctcagcccatattattcaattgagccggaagaagacgtgacgggcggccaagacatgaaggaatacagcaaggttcaacagatttacatggacggatcgatcaatagcgccatttacacagcctatcatcaagcccataaagccgttaagattaagtattccggcatttatgtcatgagtttgatgaaaaattccaactttaaaaataagctgaaggtcggcgacgtggtggttgctttggatggccatcacttcaagagttccctgggcttcatcaagtatgttaagcagcaaaaatatggtcagaaactgacggtcacctataaacgtcacggaaaattgcatcaagccacggcgccacttggcatgattgccaaacatcgggcagggattggcatcactttgaccgacgatgttcaagtgaagcccaagattccaattaaggttcaccctggtcaagttggcgggccttccggtggtctcatgtttgccctccagatttatagtcagttgaccaacaagaatctgcgtcacggtcaaaaagttgctggaactggaacggtcgatgggttgggcaacgttggcgaaatcggtggaattgataaaaaagtcatcactgctaaaaagcatggtgcgaaaattttccttgcaccatatgtgaagccaaccaaaacaattttgaagtatgaggaaggccacaagacgaattatcaactggccaaagcaacggcgaaaaaatatgccccatcaatgaaagtgattcccgttaagacgtttgcccaagcggtctcaattttagaaaaaaatcaataagcaaaatcaaaaagggttagataatctaatcctttttttcgtatgtattttttagaagggaggcacagtatggataggatacgtgagtttattgatgaatatctttatcagatactaattggtttagtggcggtcatcgtcatttttatgtttgtaattggtgggctgttgattggtaagggcggtgagactgccagttctgaagagccggttgctgtccaaagttctagcgcaagttcagatacgggatcggccgcgagttcatcgcctggtgatcaacccaagcaagttgctgccggcactaatcaacaaatgtatgttgacgttaaaggggcagtgaagaatcccggtgtttatcaggtcagcagcaatatgcgggtagtcgatgccattgaattggctggtggttacaatcggtctgcggacaagaagaaaatcaatttggcccagaaactgaccgatcaacaagtcatttatgtaccgattcgtggtgagaaggggacaccggtcacgtcaacggttgcggccagcccgacgccatctgagactccagcagattccgggtcggacaactcagcgccatcggcggacggaacttcaggaacgtctcaacagatcaatttgaatacggctgataagtccaagctccaagagctaaccggaattggggacaaaaaagccgatcagatcattgcttatcggcaggcacacggccaattcaaaaacattgaggagcttaaggaagtccctgggtttggtgataagacctttgccaatctgaaggcatcaatttgcgtctagcccaaaaagcgtttttgagatatgatttacaccagagaaggtggaatgataatggataagcgaattaaatgggaccaatattttatgatgcaggcggttttactggcctcacgaagcacgtgcgaaagattgtcagtcggagcggtcattgtcagagacaaacggattatcgccggcggctacaacggatccgtcgcgggagatgatcactgcattgacgtcggctgttacctggaagacggtcattgcgtgagaaccatccatgcggagatgaacgccattctgcagtgcgccaagttcggtgaaagcactgacaatgctgaaatctacgtgacggattttccgtgtcttcagtgcactaagatgctacttcaggctggaatcaccaaaatcaattacctcagaaattaccataataatgattacgcccaaaaactgattaggttgaaaaatattgaattgaacaaaattaagttaactcaagccgatatggatagagtgccattcggatcctatttgtctgactagttatcaataaaaactggctcatttttccggcagccgtcatgcttttgatgagcatggccatgtacgggaaccggctgattgcggcagctttattaagcattctgattatgcggatttattttctgcgggacgttaaagttgttagtacatgtatccttgctggcctgatctttgcctttggtgggcttttgaccaatcgacaggtctctgcaccagtctcacaacaaaattatttggttaaagtctatccggattccgccaaagtgaacggggcaaatttgagctttattgcccgtcctgagggtgcaaaacaaaagatggtgttatatgccagattgaagtccagtagtcaacaacgtcgtttagcagccggtattaacccaatgatgcttaaggtgagtgggaaatcagccccttttttgccggcaaccaacctgaatcaatttgatatggaaaaatattatcatcaccaaaagattcaaagttgctttttggtcgaccatttcgttcttctgccgccaccagctaaactgtcaattgtcgatcgaattcatattattcgttcgaaattcaaccagtattgcagtcagctgcccaaaactctggggatctatgccaccggattgattagtgggtatcggccggtgaacttcttcgatgaaatgacgggggttaagaagctggggttgctgcatgtctttagtatttcagggatgcatgtggcctattttctttcgattgtcgaccagctgctggcttggctggggttgtcgaggtttaaaaaatcaatcatctcaatcacctttttaggcgcctattttgtcttctctggcggatcccccggattgctgagggcagtgatgatggccatcattggtattcttaatcggctgtttaaattcggtctttcccaactggacatttggagtggatcattaatcattaacctgctcattttacccgaggcgatgtttttaatgggggttcaactcagttatggattgtctttggggttgattgcctctgagaagttttcatacattaagcaaacgattttgctcaattttttgaccgtgccgattttgttgtttcatctttacgagtggcactttttaagtgttgccgttaatctgattgtcttaccgctgttcggccgggtcatctttccactggttatcattggcgtcattggcggactggttgcggaaacgttggttctgccgatcgacatgtttttgcgcatctttaatgatgggttaaatgcagtgagtcgtttgccggggatgttgacctttggcaaaccggcattgccgattgtcctaaccatgttggcggtgacaatgctattggccgttgttgatcgtgttcgggcacccaaactgattggcatcttggcagctgtttatctggtgacgtattgttggatccattttccgctcaatggtgaggtgaccatgtttgacattggccaaggggacagcttcttgattcgggagccctttaaccgttctgtgaccctgattgatactggcggcaaggttcaattcaatacccagccatggcaaaagggtgctcaaacctaccaagctaagcgactctcgattaattacctgaaaagtattggcatctcaaagattgacaatctgtgtgtaagccatcaagattcggaccattgtggcgatttgccggcattcattgaagaaatggaaattaagcggatcattattcctttgggaatggaccaaaacccgagttttatgaagagaattgccaaccgcagtcgatctaccaaagtgatttctgtcaatgatgagacgcaagtaccaggtttgccggctcaaatctttcatccctatcttgccggtaagggtgagaatcatgactcaatggtgatcggtactcaaaaaggcggtttgcggtggctgtttacgggggacttggaccgcccaggagaactggacacgcttcaaaggcatcccggcttgtcagcagacgttcttaaagtcggccatcacggaagtaaaacatcctcggaccctcagtttattgcgaccgtcaaaccacggatcgccttaatttctgccggtcgaaacaatcggtatggtcatccaaacgacgaaacacttgtcacattgaaacagcatcacgttaaaatatttaatacccaaaaacacggtatggtaagatatatctatcgaaacaataccggtcatttcgaaacggtgttagccggtcatgaagggaatttataatgaactattctcaattaattcaacagttaaaccaaggaaacctcgcccaggtttatttgatcttaggggatcaggagtatctttccggtcgaattaaggatgcttttgtcaaaatcatcccggacaacgagcgttcgatgaatattggcaattacgatatggaagataccacgatttcagccgcggtggaggatgccatttctgtcccatttttcggtgagcgtcgactggtcatgattaaccgaccgtattttttgactggaatgcgtacgaagtccaaattggatcaaaatatcgacgactttttggaatatttaaaacaccccgaagagtccacggttatggtgatctttgccccgtatgacaaattggattccagaaagaaagtcaccaaagccctgaaaaaggtcgccaccaccattgaaattggaagccttcgtgaaaatgagattaaaaaactggtcacggataagattgctgctgcgggattcaaaattgatcacgacgcattggatcggatggtcgaattaaccggtggtaagctaacggcgatgatgagcgacttgcccaaattgattttgtacaataatgatacgaaagtcattgatcttgcatccgttaatggattggtcagcaagtccatggagcagaacgtttttgacttggttaatagcgtccttgcgaagaatcccaaacagtcaatggacatttatcatcaattaattctggaaaacgatgaaccaattcggattaacgctgttttaattcagcaatttcgattgttgctgcaggtcatgattctgcaaaagcacgggtactcacaaggaaatttagcttcaacactcaaagtgcatccgtatcgggtcaagttggcgatgcagacgatcagaaagttcaattacgatcaattacgagaagcttatattggcctggttgatactgaacgtcagatgaaatcaacccagcgcccacccgaattattatttgaactatttgtgttgaaatttatgaaaagtgtcagttaataaaaaataggagtaagcaaagtcggtcgaccttgtttactcctatttttgtgggacaaaaaaagttgttagtctgactaacaactaagaaagaattattttgctaactttgaagttaaacgtgacttgtcacgagcagccttgttagctttaattaagccctttgattttgcgcgatcaattgcgctgattgcgttaatgtataaatctttaacgtcgtcagaaccggcaacttgtgccttttggaacttcttaacggcagtgcggtatgcacttaattgtgcagcgttgcgacgctgtgctttttcgttagttttaacacgttcgatagcagatttgataattggcatttgactcacctccgagtattattctaagtaaaaattattaaatttcaacaagcatcattatacaaaaaccaacgactgattgcaagccaaactgtcaatgaatatcggcggtaagcttgtatttgtcagagaaatccgttatactattttttgtgtgttgtacaagaccttcaacttagtttgtcgggtaccacttccgcatactcagttgttggcgtcaaaaaataaaaaggtggttatacattatggcaattacacagactaagaagaacgaaattatcaacaaatttgctcgtcacgaaggcgacaccggttcagcagaggttcaaatcgctgtcttaaccgcagatatcaacgaattgaacgatcatatgcgtactcatcgtaaagattaccattcacaacgtggactcatgaagaagattggtcatcgtcgtaacctgttggcatacttgcgtaacaaggatgttacccgttatcgtcaattgatcaaggatcttggtcttcgtcgttaatattaatatcaggagagcggataatatccgttctttttttatacataattattttaagaaagcacaatgttttttgaaaaattcggtttcaacaaaaaatatgttaaactaaaagaagctgaaaacgaacgtaaaaaagaacatattaatttttgaggtgaatcatgaaaaacgaaatcaaagtaatggcgattggtggggcccgcgaaaatggcaaaaacatgtacgcggtcgatatcaatggcggtatttatattttggactgtggtctaaaatacccggaaaatgaattattgggaattgacgttgtcattcctgattttagctggcttgaagagaataaagatcgcattgtcggtgttttcttaacacatggccatgcagattcgattggcgcaatttcttatttcctgagcaaattcgatgttcccgtctttggatctgaaatgacaattgagcttgctaaaattaacgtctccgactctgaagaagttaagcacttcgatgactttcacgttgtcagtgaccgtagtgaaattgattttgaagacattaaggttactttcttcaagacgacacactcgattcccggttcgctggggattgcgttgcatacatcagatggaatcatcgtttataccggtgactttaaatttgaccaaacagcggcgccaatctatcaaacaaattattcagcattgacccagcttggtgatgagggtgttttggcattgcttgatgattcaagcaatgcggagaacccaaatcccagtgcctctgaaaagaagatcgctgaatatgtttatgataccttcaattatcaaaacagccggattattgtcgccggtgtcgcctcaaacattttaagaatgcagcaggtcttcaatgccgccgccaggaccggtcgcagagtctatttaaccggccatgacctggaacggattgttaagactgccatgggattgaatacgctgaaactgccagaggacgatttgttgattggctcactggatgagcttaagaaaatggcccctgataaagttgtcatcattcaaaccggcaaaatgggcgaaccaatcaaagcgattcagcggatggcgaataaagaacaaagtgatattaatattgaacccggcgacctggtatttatcacgacaaccccgtcaactgccatggaaacaacggttgccaagacgcgtgacatggtttaccgtgccgatggcgaagtcaagatgatttctgatgagatgaattcatcgggggatgccagtcaagctgatttacagttgctgatgaatttattacatcctaagtatattatcccagtccaaggggaataccgactactggaagccaatgctcaactggccaaagaaatcggctatactgatgatcaaatcgttattcctgccaagggtgatgtgatctcgatttcagaagatgacattcatttgggcaagggagttgatcttgcggataccatgatcgacggtatcggcattggcgatatcggcaacattgtccttcgcgatcgaaaggtgctctctgaagatggcatttttgtggcagttgtgacgattgaccgcaaaaagaagcggattgtgtccactcctaaattgacatccagaggatttgtttacgtcaaagccaacaaagacttgatgaaggatgccgccgggattatcgaaaagacggttaccaacaaccttgaacacaaagagttcgattggagtaaccttaagcaggacgttcgcgaggatctgagtgattacctgtataaacaaaccaagcggcgaccggttattttaccagttattatggaagttaaccaacatcataaacgttcaaagaaaaagcaaaaagcagctgaaaaaaattagccaactgagcgagtaattcatttttttgaattactcgttttctatctctaaatgttatggaggaaaagatgactgagatgacaaaaaacgatcgcgtcatcctgttgagtgctcaagaggatttgcgggatggccgttataatcaggtcgtaaataaggcggagcatttgttggggaaatatccgcaatccgtggaattgaacgatttgtatgcaaatgcgttgtaccatttgaaaagatatgccgatgccggacaagttgtggccgattttgccgaggatttcatcgctcaaccaaggtatcaaggccatgcgatggaaatccttttggccaacaatctgttcatgtctgctcgagaggtgcttgcccaggtaccgacttcaaagaagggggagtggaagcaaagaatcgtgactgctgaaaacgattatcgtcaacagcattcaaccgagctggcggcgaagtcacgtaaatttgcctatcttggggcactttccgtcactgagcaggttcatgaggttcaagcagcgcttcatctgccactaaatgaatatttgtcggccgctaagacattactgaatgatccgtatgggtggcaggtttcgaaaacgcaggtcttgttacaattaatgaaagctcaagtttctgaaaacgttgatttgatctggttggatgggaagacacatacgataagtttggacgaattaaaaccattggagaaaatcgatgcttttgtgcgtgttcttcaaattgttgagcaacaatttgccgctaaggacccaatcaaattggatttgctggaaagagagttattcactcagagtaattatatttacccctattttgatgatgtgataactgggcccaacttctgggcacaggcaattatcgcccagtcatttggtgagccgttgcccgccaagacacaacagcagcaaagaatgttatcttggatcaaccggatccatgatcaggaaattaaaattggtctcatataactgaattattttcggaaaataaagggaatctgtttacaaacattaccagtatcgatataatacttaaggattcttcgaaaattgactactttgtcttttccagaagatgtagtataataacacttagaaatgcattgatgcgaaattgatgtaattcttgaaaacaacaggaggtttcattaatggcaaaagaacattatgaaagaacaaaaccccatgtaaatattggtactattggccatattgatcatgggaaaactactttgactgctgcaatcactaaggtattggctgcaaagggtctcgctaaggctgaagactatgctgatatcgatgcagctccagaggaacgtgaacgtggtataactatcaacactgctcacgtggaatacgaaactgaaaagcgtcactatgcccatatcgatgccccaggacatgctgattacattaagaacatgatcactggtgccgctcaaatggatggtgctattttggttgttgccgcaactgatggcccaatgccacaaactcgtgaacatatcttacttgctcaccaagttggtgttgattacatcgttgtattcttaaacaagactgatttagttgatgatgacgaattagttgacttggttgagatggaagttcgtgaattactttctgaatacgattatcctggtgatgatattcctgttctccgtggttcagctcttaaagcacttgagggcgacaaggaacaagaacaagttatccttgacttaatggatgttgttgatgagtacattccaactccagaacgtgacgacagcaaaccattcttgatgccagtcgaagatgtcttcactatcaccggtcgtggtactgttgcatctggccgtatcgatcgtggtactgttaaagtcggtgacgaagttgaaatcgttggtttgaacgacgaaccattgaagtcaactgttactggtttggaaatgttccgtaagactcttgatgaaggtcaagccggagataacgttggtgttcttcttcgtggtatcgaccgtgatcaagttgtccgtggacaagttcttgctgctcctggttcaatccagacccacaagaaattcgaaggccaagtttatatcttgactaaagaagaaggtggccgtcatacgccattcttctcaaactatcgtccacaattctacttccataccaccgatgttaccggtgttatcgaattggaaaagggcgtagaaatggttatgcctggtgataacgttacattccaagttgaattaactaagccagttgccattgaaaagggtactaagtttaccatccgtgaaggtggtcatactgttggtgccggtgttgttagtgatgttaacgactagtttttatcattagacacacttaagctgtgaggataattcctcgcagctttttttatgtttttagttcgtttgaaattaattttacattttatgattaatacgttaaaataacaatgttatgcaattatgaaattgtaaaaaattcttttggtctcggaggaaaaaagatgtctgcaaaatgggaaaagaaaggtaccaatgatggcgaattaacattcgaaattggtacagattcaatcaaatcaggattagatcgtgcatttaaaaagaataagaacagcattcgggtacctggcttccgtaaaggaaaggttccacgtcagattttcactaagatgtatggtgaagaagcattgtacgaagatgccctcaacattctcttgcctgacgaatatgaaaaagccgttcaagacgctaagatcgaaccagttgaccaacctaagattaacgttgagtcaatggaaaagggcaagccttgggttattaaagctaacgttaccgttaagccagaagttaagcttggcgattacaaaggcttgagtgtgcctaaacagaatacccgtgtctatcaaaaagacgttgacgctgaattggaaaagaagcgtgaaagccaagctgaattggttcttaaagaagacaaggctgctgagaagggcgatactgttgttatcgacttcgaaggaagcattgacggcaagccatttgaaggtggcagtgctgaaaaccattctcttgaactgggctcaaactcatttatcccaggctttgaagatcagttaattggtcacaaagccggcgatgaagttgaagtaaaggttaccttccctaaagattaccaagctaaagatttagcaaataaggaagccatctttaaaaccaagattcatgaagttaagacaaaagaattgcctaaattagacaatgactttgccaaggatgttgacgaagatgttgacagtcttgatgaattgaaggaaaagatcaaagaagacctcaagtcacaaaagaagtctgaagctcgtgatgccatcgaagacgctgcaatcagtgaagcaactgataatgctgaagttaaagacatcccacaggctatgattgacgaagatattcaacgtcaaatggatcaatatcttgccggcatgcaacaacaagggatcaaccaggacatgtacttccagttaactggaactaagcctgaagaccttaagaagcaatttgctgacggtgctgagaagcgggttaagactaacttggttcttgaagcaattgttgccaaagagaagattgagccatcagaggatgatgttaaggctgaggtgaagaaccttgccaaacaatatggcatgaaggaagacgctgttcgcagtgccttgactgaagacatgttgaaacatgatatcgcaatcaagcaagcaattgatatgattgttgattcatcaaagcaagacgccaaagcaaaatcaactgaaaaggattcaactgaagccagctcagaaaaatagctttttgcttaattaaaagacccgttattttgacgggtctttttttaaggataaagccgattaattgcaatttgtatgtgatatggtaaagttactcttagttgattactactaattgtatttaaagtccatctcggatggaggagtgaataatttgtttgaagataatgaatcaagcgggcctattacttgctcgttttgtggaaaaacacaggatcaagtgaaaaagattgtcgctggtcctggcgtttatatttgtaatgaatgtatcgatttatgtaaagaaatcatcgatgaagaattggcacccgaaaaatcatcagacgatttactcaaagttttgacgccagctcaaattctggataagttaaatgaatttgtgattggtcaggaaaatgccaagcggacactttccgttgccgtatataaccactacaaacgggttaacgaaatgattagcgaacctgatgatgatttggagcttcaaaagagtaacatttgtatcatcggcccgactggctcaggtaagacttacctggctcagacaatggctaaaattttgaatgtcccatttgccattgccgacgcaacaacgttgactgaagctgggtatgttggtgaagatgttgaaaatatcctgctgaaactgctgcagaacgctgattatgacgttgaacgagcagaacatgggattatctacattgatgaaattgataagattgccaaaaagtctgaaaatgtttcgattacccgtgacgtatctggtgagggtgttcaacaagccttattgaagattcttgaaggaacaattgccaacgtgccgcctcagggtggtcggaagcatccacaacaagaatttattcaaattgatacgacgaacatcttgtttatcgttggtggtgcctttgatgggattgaaggaattgtcaagagccgccttggcgataagacaattggtttcggtaccaactcagatgaagctgctaaggtcgatgccaaaaacatcatgcagtcggttattccagaagatttattgaagtttggcttgattcccgaattcattggtcgtctgccaattttgaccgcattggataagcttgatgaacacgatctggttcgtattttaactgagcctaagaacgctttggttaaacaatacaagaagttaattgaacttgatggtgccgaactggaatttgcgcctggcgcattggagaagatggctcaactcgcaattgcccgtgatactggtgcgcgtggtcttcgctcaatcatcgaaggcgtcatgcgtgacattatgtttgacctgccgagtcgaaacgatgtctccaaggtcatcattaccccagagactgtgacggatcataaggaaccggaattaatcttaaaacaagcatcgtaattcctagaaatctgatgtagactttagatagcttactgtcagatttcttttttattcacacattttattcattgaaggagtggtttcatggaagttcacaacgtcgaccttacgattagtgctgtcgcagaaaaacaatatccaaatacacaatttccagaaatagcattggtaggtcggtcaaatgttggtaaatcttccctgaccaatgtgttgatcaatcgcaacaaatttgctcggacgtccagtcagccggggaaaactcaaaccctgaatttctacaacatcgaagataagctgtactttgtggatgtccctggatatggttatgcaaaggcatccaaagccagccgggaaaaatggggccgaatgattgaaacctatttaaccaaacgtgaacagctgcggggggtcattaccctggttgatggtcggcatgcgccaactgctgacgatgtgtcgatgcataattggttgaagtattacaatattccaatgttaacggttgcgaccaaaatggataaaatctccagcgggaaatggaacaagcaggaatcattgatcaaaaagacactgcagttggatgctgatgaaccactcattttgttctccgctttgacaaaaacgggtaaaaacgagatttggcgttggattgaggggagaatgaaacgatgaattttgatgactatcaaaaggcagccaatcggacactgatgggtaacgagcaagttttaacgaactgtgcactggggctcaccggagaatccggtgaagttgctgatttaattcggaaatatacttttcaaagcaagaagctcgatcacgatgaattggttaaggagatgggggacgtcttgtggtacctgtcccaaatctcagagtgggccgacattccatttgatgaggtcgctaccgacaacatcaaacggctcgaaaaacgttatcctgagcaatcaggtggcgttaatcaagtgaatatttaaggatcaatttagaagcagtcattttgagatggctgctttttttgcagcaatttctggcaaaatgacctcttatttgcatattcgacataatattttcacaaataatgaataaaacataaaaacagttgcattaaatgaatattggtgttaatctcaatacattgaatttttcagaagataagagggaatatatatgtcagaaaataataaagtcattttagcttactccggtggccttgatacctccgttgcaattgcctggttgaaagacaaaggttacgatgtcgtcgcttgctgtattaacgttggtgaaggaaaagatctcgatttcatcaagcaaaaggcactgaacgttggtgctgttaaggcttacgtcattgatgccctggatgaatttgccgacaactatgccgctgtggctctgaaggccaacgcgatgtacgaagggtcatacccgttgatttcagctttgtcacgtcctttgatttctaagacgttggttcaaattgcccatcaagagcatgccgttgccgttgcccatggttgtaccggcaaaggaaacgatcaagttcgttttgaagtggccatccacggccttgaccctcagcttgaagtgttgagcccagttcgtgattggcactggtcacgtgagcaagagattgaatacgccaaggatcacaatattccaattcccattgatttggactcaccatactcaattgacgccaatatctggggtcgtgcaaatgaagccggtattttggaagatccatggcaaagtgcaccggaagatgcatttgcaattaccaatcccattgaaaatacgccggatacccccactgaagttgaaattacttttgaaaagggaattccaactgaattaaacggcaagaaaatgaaattcgctgacattatccaagaactcaatgaaactgccggtgaaaatggggttggccgaattgaccatattgaaaaccgtttagtcggaatcaaatctcgtgaagtgtatgaagccccggctgcaacggtgctgttaaaggcccataaagagctggaagacttaacatttgaacgtgacttggcccatttcaagccaactattgaaaaacaactgagtgaacttgtttataatgcactgtggttctcaccactgatggattcaattcaagcattcattgataaatcacaagaggtcgtcaacggcgtcattaaattgcaactgtttaaaggcaacgtgatggttcttggtcgcaaatcagattcttcactttacgacaaggatctggcaacttacacttcttctgattcatttgaccaagaagctgccaagggcttcatcaagctttggggattgccaacccaagtttatcaacaagttgcccttaaaaataagaacgcacagttcgttcaagcagttacaaagtctcagctaaaggacaaagtgacggttcatgaacacaattctgcacatacgggagctaagaaataaatgagtactaagaaactatggggtggtcgatttcaagaacaagcagcgcaatgggttgatcaatttggggcctcaatttcgtttgaccagttaatggccgatgaagatattgaaggctcacttgcccatgtcaaaatgcttgggcacactaaaattttgccaatggctgatgtcgaccagattgtcgccggcctcaacggactccgagaggaccttcatgcaggtaagttgcgttttaccgttgaaaacgaagacattcacatgaatatcgaagctttattaaccgagcgaattggcccggttgccggcaagctgcatactgcccgttcacgaaatgatcaggttgcaaccgactttcatttatacttgaagaaccggttaccacaagtcatcgatgaaatcacgacgttgcagaaaacgttggttgagatggctgaaaaaaatgttgagaccatcatgcccggctatacccatttgcaacacgcccaaccgatttcatatggtcactatctgatggcctattatcagatgctcaaacgtgacaaggaacggtttgctttcaacatgaagcatacggacatcatgcctttgggcgctgccgcgcttgctgggacgacttttccgattgatcgggaatacactgccaaagagttggattttggggaagtttatcccaattcactggatgctgtttccgaccgtgattttgctttggagtttttaagcaacagttcaattttgatgatgcatctgtctcgtttctgtgaagaaatcagcatgtgggtcagccacgagtttaagtatctggaattaagcgatgcttatacgactggcagctcgattatgccccaaaaaaagaatccggacatggcagaattgatccgtggcaaatctggtcgggtatacggccatttaattggtttgttgtctacgatgaagtctttacccttggcctataataaggatcttcaagaggacaaggaggggactttcgatacggtcaaaaccttattgccttccttaaaagtgtttaacgggatgctaaaaaccgccaaacccaacgtcgagcggatgaagcaggccactgagaatgacttttccaatgccacagaactggctgattatttggctgccaaggggatccccttccgtgaagcccacgggatcgttggtaaactggttttaaagggcattgagacccaccagaacctccaagacatgtccttagaggaactacaggcagcttcacctaaaatccaagaggacgtctaccacgaccttaaatcagaggtggcggttgaacgtcgtcattcatttggtggcaccggatttgaccaagtgcggctacagatcaaaaatgccaagaaggaacttggcgaatagttattgcgtaaatgatatatattttctgacaaaaacaaaacgaggcatcgctgaatcagcggcgcctcgtttttcattgtgtatatattggattgagtggtgagaatgctgttggtggatccataagcagttgttcgttgcactttggttgaaatgtgttccgacgggccagatgctaacctctaaaggcacttcaattcaaatcccaaaaccagggatttaaatcaaagcgcctttagaaaccgcatctcccagtcctcgtcacactctgatcgaaacgtgttccgacgcaactggggctaacttctaagggcacttcaattcaaatcccaaaaccagggatttaaatcaaagtgcccttagaaaccgccccaaaccgttgctcgtcacactctgactagaaccatctcttcttcttttccggtttttcttcattcttacgttttttatctttatcttttttgtcgtgttttaagaacttatcacgctttttatcttccggatccatttcggcaaacttgccgaacattgcatccatgtcgttttggcgattgacctttaatgccattgagattcatctccttacccttttcgtcataactatagcaaatctgaccgcaaaagtcacatttgttggccattactcactttttgatgcataaatgtattaattatgtataaatacgacttaattaagatttttcttgcataaaatatattttgggtgtaatgtattggttattataaatttggaagagggaaacttgatgaagaagagtcttaaagcaattattcagacattgattatgattgccgctgtatttactttaaccacagtattttcaaatcctgcgtccgctgcagatacgtcactgcaacgagttaagcagcgtggggaactgattatggttaccagtcccgattatccaccgtatgaatttcaggtgaataaaaatggcaaggataaaatcgtcgggatggatatcgacgttgccaaaaaggtcgccaaagatctccacgtcaaactggtgattaagagcatgaactttgattcattgctggtggcgattcaaaccggcaaggcagatatggcaattgggggtattaacccaactgcagctcgtcgtcaaagtgttgatttttcaaagatctattattcaggcggccaaagcttcttgattaattcaagcgatgtcaacaaatacaagagcgccaaaaatctgaggggggcaacaattggtgcccagaccggtactttgcagtatggtctggccaagaaaaaaattcccaattccaccgttaaagggatggacaagtcaaccgacttggtactggccctcaaaactcataagattgatgctttgggaattgaaaagcccagtgccgaagcttatgtgaaaaatgatcccagcctaaaaatgatttcatccgggtatcatttgaacaaaaatgaaattggcgctgcaattgcctttaaaaaagggtctgggagtttagttgccgccgtcaataagagtattgaccagattaaaaaacagaacctgactgaacagtacctggctgatgccggcaagtatatgaaggttaatacagtaaatacctccatgttccattattggaagtattttgccaaaggggttgagtacacaatcctgatctcggtagtttccacgttctttggggtcttgattggcgttatcctagctttgatgcgtttttccaaacagaaatggcttcgaggcctggcaatcagttacaccgagtttattcgaggcacgccattaatggttcaagttttgttcgtttactttgggattggggttgtcgtcaatattccagctttgatttcagggatgattgccgtgtcactgaatagtggtgcttacgttgctgaaattatccgtggcgggatcaattcggttgccaagggccagaccgaggccgctgccagcttgggcttgtcaaagggtgatctgatgcgttttgttattttaccgcaagcctttaagaacatttggccggctttggggaacgaatttatttccctgatcaaggaaagctccattgtttcgattattggggtgaccgatttgatctatcaattaaacatcgttcgtgcggatacgtatcgtggtgtcatgccgattttcgtcgccatgctgctgtacttcatcatgacatttgcattgaccagagttttgaaccattttgaagggaagatgaaacatgcaggataagaaaattcttgaagtaaatcatttaaataaaaaatttggtgacaatgaaattcttaaagacatcaatgggaccgtcaaatccggcgaagttatctgtgtaatcggtccatccggtgcgggtaaaagtacctttttacgttgcctgaatttattggaaaaaccgacctccggcgaagtgaagtttgaaggaaccgatctgactcacgttgatgaaaaacaattgatcaacttgcgtgagcgaatgggaatggtatttcaaagcttcaatttattccccaatatgacggtgattgagaatctgaagttggcaccaattcgggttaaacacatgaaagatgacgaagcccaaaagatcgccatgcacctcttggatcgggtcggattagctgaaaaggccgacgcctatccaagcagtctttcaggcggtcagcaacaacgggtggcaattgcccgggcactggcgatgaatccggaagtgatgttgtttgatgaaccaaccagtgccttggatcccgaaatggtcggtgaagttcttgaagtcatgaacgagttggctaaagaagggatgacgatggttgttgtgacccacgaaatgggatttgccaaagaggttgccgacgaggtttggtttatggccgacggctacattctggaacgaaataaacccgaggagttgtttgacaatccgcaaaatgagcgggccaaagactttatcggaaagattattcaaaatgtatgacgcaggcttttaactattagaaagatcggtgagatgaacctagatgtggttcattgtcgccgatctttttcttgtttaaattgccctggccgaaactcaggtccaatccctggttcaaagttaaaagaggcagatagatgaaattcattgtcgaatcttgtaaaatctattgataccagatggttatgaaaatcccgcgaatgttggttggatgaaagaatggtttgatccctctaagtcaaacactctctgggacacatcggttgaaccaaacatatattcgatgtataatttttagatgaatattatgaaaggagtgagttttttggcgagtgaatatatcgaacataaattggctttactgcctgacatgcctggctgttacctgatgaaggacattaacggcaagattatttatgttggaaaagccaaaaacttaaagaaccgggttcgttcttattttaagagcagccatgaaggcaaaaccgcccggttggtctccgaaattgccgacttcgaatacattgtggtttcgagtgacaaagaagcttttctgcttgaaattaccttgattcaaaagcatcggccatatttcaacatcaaattaaaacagggaaacggtgggtacccctacattaagattacgaatgaacgggaccctcagattaaaatcgtcaatacgttactcaaagatggcggtttttattttggcccttatccaaacgtctatgctgcagaagagacggttaactttctgcagaaggtctatccattgcgtcgctgcaacggatttcagaatcgaccctgcctgtattatcatatgggacagtgccttggggcttgttttaaagtggttccggaagaaacgtatgccaagcagattaaacggattaagtcgtttctgaatggcaatgtgtctcacgccaagcagatgctaacgactagaatggagaaagcggccgccaagatggagtatgaacgggccgcagaaattcgcgatctgatcaagtacattgaaattaccgttgagaaacagaaaattatttcgaccgataatacgcctcgcgatatttttaattactatatggataaaggctggctctcgattcaggttttcttcatccgtcaatcacgattgatgaaacgtgagaaacgtctctttccgatcattgatgatcctgaagaagaaatggtcagttttatctcgcagttttataagcagaagaatcagattctgcctaaggagattctggtgcccaaatcactgccaacagatgtgattagtcacgtggttgaagatgttcccgttagaaccccccagagagggcagaaacgcgatctcttggagatggcgggtaagaatgcccagatggtcctggaggagaaattccgcctgttagagcttgatgagagcaagacgaccggggccatgaaagaactcactgatgcaatgggaattgcgccggggcacaaaattgaagcatttgaccattctcacattcaaggggccgatctggtctctgcaatggtggtctttgttgatggtcagcccaataagaatttataccgaaagtacaaattaaagaccgtggatcacgcagatgaagccgccagcactaaagaagtcatccgccggcggtatacccgactgctcaaagagcacgctgagatgccggacttaattttaatggatggcggggtcatccagatgaacgccgtcaaggatgtcctggtcaatgaacttggattgaatattccggttggtgggatggttaagaatacgcatcaccaaactgccgatttactgtttggagataatgacacgccactgcaattggatcctaagagtcagggcttttatctgctgcagcgaattcaagatgaggtccatcgatttgcgattacctatcatcataaagttcataccaagaactcattgagttccaggttggattcgattgccggtgttggtcccaagacacggaacaaacttctccggaaattcggatcgctgaggaaaatttcaaatgccccaattgaggaattgcgtcaattagggatttcagagactgttgcgcaaacaatcaagttctcactgagtaagattgatgaagaacgaaaagtgaccaattatcaagataaaaaattgactcattaaaatgattcgaaagggctttcttttcaagattattttgacctgatgtaggaaactcggtatactgctagagtactgaacacgtaactaacgacttgggattaattagaattaattaaatggtgataagatgtttgttgatcaagtaaagattaatgtaaaagctggaaacggcggaaatggcatggttgccttccgacgggaaaaatatgttccaaatggcggccctgccggaggtgacggcggtcgcggcggcaatgtcatctttaaggtggattctggtatgaacaccttgatggattttcgataccaccgaaagtttaaagccaagaacggcgggaacggtgccaacaaatcgatgaccggccgaagtgccgacgatttggtcattcctgttcccgagggaacgacggttaccaataccgatacgggcgaagtcattggtgatctggttaagccggatcaagaattggtggttgccaaagccggccgcggcgggcgtggaaacattcattttgccagcccgaccaatcccgccccggaaattgctgaaaacggtgaaccgggtcaggaagtgtctttgagccttgaattaaaggtgctcgcagatgtcggcctggttggatttccctccgccggtaaatcgaccttgctatcggttatcactagcgccaagccaaagattgccggatatcattttacaaccttggttcctaacctcggtatggtgagattagatgatggccgtgattttgcagttgccgatttacccgggttggttgagggtgcttcgaatggtgttggactggggttccagttcttacgtcatgtcgagcggaccagagtcattcttcatttggtagatatgtcaggtcttgagggccgtgacccatttgaggattatttggcaatcaataaagaactggaacaatatgacgagcgcattttgaaacgaccacaaattattgtcgctacgaagatggacttacccgattctgccgataatcttcaaatcttcaagcagcagttggccgagcattcagatgcagataagacacgagagatctttccgatttcttcagtgacccatacgggattaaccgaactggttcgacgaacggctgacttgcttgatacgaccaagctttcagacatggagcagccagcggaaacgaccaaagagtacgcttaccaaccggctgagaccagcgatttccatattgaatacgataaagaatatgagtcatgggttatctccggtgataaaatcgagaaattattcaagatgactgataccgaacatgatcaaagtatgttacgatttgcgcgacaaatgcatggaatgggaattgacgatgccttgcggaaggcaggggccaaagatggtgacacggttactattttggacttctcattcacatacgttgagtagttatttggggaaatacaaattcatatagggcagggaatatttcgatgcaacaggttcaaacaaaaaaacaaggcaaacggcttaaaaacagccgttatatatccggttttgacgggatcagggcactggcggttgttggtgtcatcatttaccatttgctgccgtataagctgcaaggggggtacttgggtgtaccgaccttttttgtcgtttcagggtatttaattactgatcttttgttacaggagtgggagcaaaacggccggattgatttttgggcgttttacgcccgtcgtctgaagcggctgtatcctgctctggtgtttatgctggtgggaaccggcacatacataacgctgtttcaacgctcactattaaccaatttgcggtcaatcattaccaccaatatgctgtacgtttacaattggtgggaggttggccatggccagagttattttgaccggtttaacggtgaatcaccatttacgcatttgtggtccttatcaattgaaggccagtattacttaatatggccgttaattctaaccgcgatggtcctgattattcgcaaacggcggacaattgccaatattcttcttgtgttggcaattggttccggtgtcttgatgggactgctgtacactggtccggatacgttgaatcgagtctactacggcaccgacacgcgaatgttttcaatcgtttttggtgctttacttgctgttatttggccatctactcatctgaagaaaaacgtgacgacgcgatcgcgttggaccctcaatattattgggctagtgtcaatcgcaatcattgcttacctgtattttgaactctctggtcaaaacacgtttacgtatcgtggcggaatgttcattatggcaattgcttcgactaccttgattgcagcctgtgcccatccgggagccgacgtgaaccgctggttgactaatccggtatttagatggatggggaccagaagctacggaatttatctttaccaattcccggtgatgattttttatgagatcaaagttcaaaatattgccgcccatccactgatgaatgcaagcattgaaattgctttgattatgattattagtgagctgtcttatcgatatattgaagcaccgttaagacattaccgctatagaaacctcggtcggtcaatttacgagtttgttcaaccgaattcggaatacggctggaaacggttgtggctgataccagcagttttgctgattggaatttcggcatatggaagtgcaatttcacctaccaaagatgccaagaatgtactggaagaaaacatctccaagaacgaaaagaccgctaatgcaaataacaaggcagcgttagctaaacaaaagaaggcctccaaacttactgccaatcaaaagcggatgaagaaactgctgaagaagaaactgacggttaagcagtataaaatcgccaagcactatggcctgaacaaacgtcagtatctgacggtttatcaacaaccgttgaccgccattggggactcgattttagctgataacagtcacgatcttcaaaatgtctttcaaaatgcctatgtttccgctgccgttggtcgtcaaatttggcaggctgggcaggttttgacccaaatgaagaataaaaacgagctggcacctaacgttttgattaacttggggaccaactcacccatgacttccgcccagattaattcggttatcaagtcaattggacccaagcatcaaattttctgggtaacgactcatgtgccaaccagaaattgggaaaccgaagttaatcacacaattcgagttgctgctaagcgccataagaatatgcatatcattgactggcacagctatagcttgaatcggcgggattggttctggaacgataacgttcatcccaatccaaaagggaatatttattatacacatctcattgcgacgtcgattagcgatttttatagtaaaaaataaaagtttgaaggccttcattccatgcaagtagctggattgaaggctttcaaacttttttggcttattttaagttaatggtgagtgttgaatccggtgagggggcaactttcttttgagtggtggtgtagatggcaccaaactgaatggtgagtttggttgccggctgagtcgcataattgtgaaggtagccggtcatcgcaaagctgacggctcgattagcaccaattttattgccggcagacgagtcggttaattgattagctgtggtcaacatttgtccttgattggttttaacataattgacaccgtttagtgcaatttcaaagttgtgatgattcgtcactgtgtaattgagaacgaaggtgtagtaggtgtctggaatgctgcgaagattaagcacctgttcggcggcctctttagcttgcggcgtcttggcggtattcttgatgactcttacctggttgaccttataagttaatttgtcggctttgatatcaaccggtttggtggtcacgtcggctaattgctgtcgagtcccaaaacggtcaaaagtaaattgatgtttcgtgctcaagtcgccatttttgacatagtgagcattcttttggactgatttgggaactttgtattgataatcactccacgattggctggaacttgaactggttgatgagctggaaggctcgtttgacatatcagcactcaatgactttttctcagttgcttgattgcttttattaccaccgcaggctgctaatccaaccgacaggatggcaaacatgatgattaagtatccttttgctttcatagttttatcccctagtaaaaaacaattgatttattgacaattctaaacccaaatatcaattggcggtcgtttaaagttcttaaatctgtcttgagggagagccgtttggttctggtcatgaattgatccaacgttattgtagcaaatccaccctgagatgggctcgatttacccaacaataacgaatttttatcaattaacagctgattaaccggcaaaaagtgctgaccttctgaaattaatagggtcaactttgggtttagtgtgctgctggcgcggaaaaactcatctaaattcatggctgccattcccttctaatgattattttaacggatttatgatacaattgaaaagtgattttaagcggttggcaggtgccaatcactctaactcgattttaaaaaataaggaaacgataataatgcagattgaatttttaggcactggggcagggtctccaggcaaatttcgcaacgtgtcaagcttggcgttacggttacttgacgaaatcaactcggtgtggttatttgatgtcggcgaaggcacccaacaccagattcttcgttcaacaattcgtccccgcaagattgaaaaaatttttatcagccatttgcacggcgatcatatttttggcctgccggggttgttaagcagtcgctcgtttcaaggcggcaacacgccattggacatctatgggccaaaagggattaaggaatatgtcaatgtgagcttgaagatttctgagagtcggctctcgtataaaattaatttccatgaattgcccaaggacaccgatagcaaaatttttgaaggcaagaagtttaccgtttatgccgcacctctggaccatcgaattaccagctttggctatcgggttgttgaacacgatcatccaggcgaattgatggtggagaagttgactcagttgcatattccatccgggccggtatatggcaagttgaaaatgggacagaccgttaagctggcggatggtcgggtgattgatggtaaagaaatgatcggtcgtgcccaacccgggcgaattgtcacgattatcggggatacccgcaaaactgacaacgccgtcaaactggcagagcatgctgatgccttggttcatgagagtacctttggcaagggtgaaaacaaacttgccaagaattattatcattcaaccaatatgcaggctgctcaaattgccaaacaagctggtgcaaagatgctgctgttgaatcacatttctgcccgttataccggtaaaatggcccatgaacttgaaaaacaggcacaaacggtatttcccaataccaaagttgtgaaggattttgatgtcattgagatcccgtttaagaagcattaacgaatcatttctggggggataagattgaaaaagcaaattagcacaattatcagcattatattgattatcattattgcaatttttgcattgatgaattttgaatctgtcgaggttaactttggcttcgcatcatttcaggtgccactggtacttttgattttgatttgtctcttaattggcgccctgattatttttctgttctcgtcaactcagaatgtcaaaaagaatcgccaatataagcaattggcatctgaaagccaaaaacgacaagacgatttaaacgccgagatttgcgaactcaataacaatctcaaagaattagaaactcgtttgaaaaattcgacgggtaaacaggaaattggtagtcgagatcaacaaatcagtgatttgcaggatgagattgccaaattaaccgagaaattatcatctcaaaagtaaggtagagtgttttaatgattgattccaagtataagtggcagcttgatcaaccagctgattcgtcagtagttgacaagttggccaaggatgcaaatattgacccatttatggctaaaacgttaattcagcgtggcattaccagtgctgatgctgtcgaggatttcttgaatccttctgtcagtgcctttcatgacccatttttgatgcatgacatgcataagggaattgaacgaattcaacaagccgtcgaaaatggggagcatattactgtctatggcgattatgacgcggatggcattaccagcacaaccgttatgtacgagacattgagtgatctgggtgctgacgttgattattatattcccaaccgatttactgaaggttacggcccgaacgtcgaagcttttcaaaagattattcaaaagggcacatcactgattgtcactgttgataacggggttgccgggaatcaagcgattgtggctgcaaatgagttgcattgcgatgtggtggtaaccgatcatcactcgcttcctgaaaagttgcctgatgcgtatgcgattattcatccgcgggtaaaaaatgaaaatggggatgcttacccatttggcgatctttgtggcgctggcgtggcttttaaagttgctcaagcgttgatggacgaagtaccgtctgatctgattgatattacagcgatcggaacggttgccgatgtcgtatcgttacgtgatgagaatcgcgcaattgttaaattcggtgttcaggcgatttcaaatagtcaacgtccggggctgcttgctttgattaaggaagccggcattgatttggggagatttagcgaagaagatattggctttgggattgctccccgtttgaattcgcttggtcggatcaaagatgccacagtcggggtcgaattattatcgacatttgacgaggatcgcgcaggtgaattagccaaatttgccaatcagcaaaacgacttacgcaagtcacttgtcgaccagttcttcactgaagcggttcagtccgttgaagatagtggcgacatttctcaacggcacacgctggttgtcgtcggccataactggcaccagggggttctcggaatcgttgcaagtcgactggttgacaaatatcagcgcccgacaatcgtcatgaccgacaccgatggtagcgaagaggttaagggatccggccgtagtgtcgacaattttgatttatttaaagcaattgaccccattcgcgatcaaacgatcggctttggcggccaccattctgcagttggattgaccatcaagaaggacaaagtgcctgttttgaaggaccagttggaaaaagctgcggaagagcagcaattggatttatctgttaagcccaagttggccattgccggcgttattccggtctctcaggttacagcagtgttatgtgacaaaattaaaactttggcaccgtttggccaggacaaccctaagcccatttttcaagtccaatttgatcagctcgccaacgtaaaggcaatgggcaagaccagtgatcacctgaagttttcactggttcaaggcaataatcggctcactgcgattgcctttggtcgaggaagtgctgccgttgagcttcaaaattctcaagcagccgttcaagtggttggcgagattggggaaaacacttggaataatcgaacgacgctccaattaatggtcgatgatctgaagcagacattaccgccggtgatcgatgagcggactcacgagctgcaccgaaagatgtttgcgacagtcggcacttacgttttcttccacgaaaaagtcttaaaacagctgcaaggatatgtgggtggccaatcgcaagttgtgatgtatgaccaagtcactgaggcatcggctaatggcaatcgcttgtacattgttgattgtccggacgtgcttgacgatttggttcagctcttagccaaagtccaaccacaaaccacggtcctatatctttacaaaaagcaacttatctccaaaatagggatgccagatcggaattcttatgctaaactgtttaggttcgttaaagaacattcaaacgttaatattgcgatgcagttaaaacaaatttcagagcacttgcacatttctgcacggacaattatttttatggttcaagtctttttggagttggatttcattacgattcaggatcgggtgattaatttgaatccgaattatactgcccgtgatttgaaaacagctccaagttaccatcttcgagttgaacagcttgcagctgaaaagaaattgttggtttcaaatactcatgaattagtcagcttcgtcaaggactgtttgggtgtttgatgaaaggaagaaagaatatgccaatcgatttttcaaaatatattgcatcatatccggactttccggaacccggaatcctatttagagacatttcacctttacttgaaaacggtgaagtctatcgggcagcaaccgacaagatagttgattttgccaaggaacggaacgttcagatgattgtgggtccagaggccagagggttcattgttggctgtccagtcgcctacaagttgggggttggtttctcaccagctcgtaagaagaataaactgcctggtgaaacgattgaagaaagttatggcttggagtatggtaaatcatcactgtacttacgaaccaacgctgttaagccgggtcagcgggtcttagtaacagatgacttattggccactggtgggacaattgatgcaaccattcgtttagtagagaagttgggcggaatcgttgtcggaaccgcatttttgattgagttgtcagatcttaagggccgtgaaaaagtcaaagactatgatttctttactttgctaaaatattaaaccaagttcattactgctggttatccagtggcaatgagcttttttgttacatttgaattcgtacttagttaaacaaaaaagcatctcagcattggtacgctgagatgcttactgtcatataaggtgagtacaggatttgaacctgcgcgccggtattagccggttcgccggatttcgagtccggtgcattaccactctgccaactcaccacaacagttttaattatatcaagagttattctgaaagtaaattactgtctacttggaagaggcaaattttgttttagcatagccaacaactgccggaatgagtgagatagcgacgattccaataatgaccatcgagaagttttctttgacaacggggatgttaccgaagtaatagccggcaccacaacagatggcgacccatgagatacatgcaatcagattatacttaatgaatcgtttgtaagggaaatcactcgtagcggcaacgaaggggattaacgttctgatgattggaatgaatcggccaaagaagatggccattgccccatatttgttaaagaactcccgggccttggttaaatccttttctttaatgaattttcccaggattcgatttcggggaataatttctccaaatttgtttccaaagaagaagttgagtgaatcgccgccaattgaagcggccaaaaagatgattacaaacaagccgatgcttaaaccatagtttacgttggctgataatgccgccgcagcaaatagcagtgagtcaccaggcagaaatgggaaaatgactgcgcctgtttcaataaagatcactccaaagagaatgaggtaggtggagttcccaaatgtattcacgatatttattaggtgatcgtcgatgtgtaagataaaatcaatgagcgtgctcaagtaatcattcctttcgaaaatttataattgattttaccaaattccctgagaagttggcgagttattacctgtcctttaacaaaaaataagttttgttgttaaatcaagggatccacgctacaattattaacagattacagataggatgattattatgagttttaagataggcatgaaggtccatggaacagtcacaggtatccaaccctatggcgtattcctggatattggtgaacatatgcaggggctgattcacatctctgagtgtcaaacaggattcgtggatgacctttataagatctttcgggttggacaaacagtttccgcgctcattattgatattgatgagtattctggcaaaattagtctctccactcgcagcactgatgttaatcttgaaatccttcgccggccaaaaagctttcgtccgaagagaattcactactggactgattaccgattgaatatcggatttaagccacttgccagagctaaaggtggttggatgagggatgcccagaacttttttagttagtttggaagaaagttcttgacccagctttcacaaattggtaaaatattttctgttgtcaattatccatttgatctgctagtgacaattaacatttgaaaaatcaattaaaaatcacttgatttcaaaccggatatctgataatattaaatagttgtcaaaagcgagaaacaagcgcttccgacaactaagtagacctttgaaaactgaacaaaattttcgacaaacaaatgtgcagggcgtttcaattcttcggaattggaaccaaacatttgcgaagtcaattcgtaaaacaaataataaatttaaatcatgagctatcacaggcttatcattttaaacaatttaagatgagagtttgatcctggctcaggacgaacgctggcggcgtgcctaatacatgcaagtcgaacgcgtctccgttaatgattttaggtgcttgcacttgaaagatttaacattgagacgagtggcgaactggtgagtaacacgtgggtaacctgcccttgaagtaggggataacacttggaaacaggtgctaataccgtataacaaccaaaaccacctggttttggtttaaaagacggcttcggctgtcactttaggatggacccgcggcgtattagcttgttggtaaggtaacggcttaccaaggcgatgatacgtagccgacctgagagggtaatcggccacattgggactgagacacggcccaaactcctacgggaggcagcagtagggaatcttccacaatggacgaaagtctgatggagaaacgccgcgtgagtgatgaagggtttcggctcgtaaaactctgttgttggagaagaacaggtgtcagagtaactgttgacatcttgacggtatccaaccagaaagccacggctaactacgtgccagcagccgcggtaatacgtaggtggcaagcgttgtccggatttattgggcgtaaagcgagcgcaggcggttttttaggtctgatgtgaaagccttcggcttaaccggagaagtgcatcggaaaccgggagacttgagtgcagaagaggacagtggaactccatgtgtagcggtgaaatgcgtagatatatggaagaacaccagtggcgaaggcggctgtctggtctgtaactgacgctgaggctcgaaagcatgggtagcgaacaggattagataccctggtagtccatgccgtaaacgatgagtgctaagtgttggagggtttccgcccttcagtgctgcagctaacgcattaagcactccgcctggggagtacgaccgcaaggttgaaactcaaaggaattgacgggggcccgcacaagcggtggagcatgtggtttaattcgatgctacgcgaagaaccttaccaggtcttgacatcttctgccaacctaagagattaggcgttcccttcggggacagaatgacaggtggtgcatggttgtcgtcagctcgtgtcgtgagatgttgggttaagtcccgcaacgagcgcaacccttattgttagttgccagcattcagttgggcactctagcaagactgccggtgacaaaccggaggaaggtggggatgacgtcaaatcatcatgccccttatgacctgggctacacacgtgctacaatggacggtacaacgagtcgcgaaaccgcgaggtcaagctaatctcttaaagccgttctcagttcggattgtaggctgcaactcgcctacatgaagttggaatcgctagtaatcgtggatcagcatgccacggtgaatacgttcccgggccttgtacacaccgcccgtcacaccatgagagtttgtaacacccaaagccggtgaggtaaccttcggggaccagccgtctaaggtgggacagatgattagggtgaagtcgtaacaaggtagccgtaggagaacctgcggctggatcacctcctttctaaggaaaaacggaatcctgcacattgtcgaaagttttgtttagttttgagaggtctactctcaaaagtggttacgctttttgggcctatagctcagctggttagagcgcacgcctgataagcgtgaggtcgatggttcgagtccatttaggcccatccacggcctgatagttagctatcaccggagtaacatggggaattagctcagatgggagagcacctgctttgcaagcagggggtcagcggttcgatcccgctattctccattgacacgagagtgtcagacttggttctttgaaaactagataatattaattttctgtaataatttttttgaaattgtatttatataatttcaaccgagaacaccgcgttattttgagtttgttaactagaaaaaatcgcaaatactcaattaactttgcatcacgtcgtgatgtacaggttaagttaaaaagggcgcatggtggatgccttggcactagaagccgatgaaggacgggactaacaccgatatgcttcggggagctgtacgtaagctttgatccggagatttccgaatggggaaacccagcagttttaatcgactgttactatatagtgaattcatagctgtatagaggtagacgtggggaactgaaacatctcagtacccacaggagcagaaagaaattttcgattccctcagtagcggcgagcgaacggggaacagcccaaaccaatgagcttgctcattggggttgtaggactgaacatttgagttaccaaagttgttgataatcgaacaatctgggaaggttggcgaaacagggtgatagccccgtaggtgaaatcaatgaccctcagttcaggatcctgagtacggcgacacacgtgaaacgtcgtcggaatccgggaggaccatctcccaaggctaaatactctctagtgaccgatagtgaaccagtaccgtgagggaaaggtgaaaagcaccccggaaggggagtgaaatagttcctgaaaccatgtgcctacaagcagttagagcccgttaatgggtgatagcgtgcctcttgtagaatgaaccggcgagttacggtaacatgccaggttaaggtttaaaagccggagccgcagcgaaagcgagtctgaaatgggcgttttagtatgttgctgtagacccgaaaccaggtgatctacccatgtccagggtgaaggtgcggtaaaacgcactggaggcccgaacccgtgtacgttgaaaagtgctgggatgaggtgtgggtagcggtgaaattccaaacgaacttggagatagctggttctctccgaaatagctttagggctagcctcggacgtagaatcatggaggtagagccactgtttggatgaggggcccgtcatgggttactaagttcagataaactccgaataccattgatttttatccgggagtcagacggtgagtgataagatccatcgtcaaaaggggaacagcccagaccaccagttaaggtccctaaatatatgctaagtggaaaaggatgtggagttgcatagacaactaggatgttggctcagaagcagccatcatttaaagagtgcgtaatagctcactagtcgagtgattccgcgccgaaaatttaccggggctaagcatattaccgagactgtggacttgaccttcggtcaagtgataggagagcgttctaagggcaatgaagccagaccgtaaggactggtggagcgcttagaagtgagaatgccggtatgagtagcgaaagatcagtgagaatctgatccaccgaatgactaaggtttcctggggaaggctcgtcctcccagggttagtcgggacctaagccgaggccgcaaggcgtaggcgatggataacaggttgagattcctgtactagttgatgatgtttgagcgatggagggacgcaggaggctaagttgtgcatccagttggaaagggatgttcaagccacgagtcagtcaaagagttaaatgctttttggcgggttgacaagtggtgatgaggaccgaaatttaagtagggaagcaaccgacgtcacactgccgagaaaagcttctagtgagtcatcaactacccgtaccgcaaaccgacacaggtagtcgaggagagaatcctcaggtgagcgagtgaactctcgttaaggaactcggcaaaatgaccccgtaacttcgggagaaggggtgctgtgcgcaagcacagccgcagtgaaaaggcccaggcgactgtttatcaaaaacacaggtttctgcaaaatcgtaagatgacgtataggggctgacgcctgcccggtgctggaaggttaagtggatgagttagcttcggcgaagcccagaaatgaagccccagtaaacggcggccgtaactataacggtcctaaggtagcgaaattccttgtcgggtaagttccgacccgcacgaaaggcgtaacgatctgggcactgtctcaacgagagactcggtgaaattaagatacctgtgaagaagcaggttacccgcgacaggacggaaagaccccatggagctttactgtagcttgatattgggtgttgacacagcttgtacaggataggtaggagccattgaagccggaacgctagtttcggcagaggcgttggtgggatactaccctcgctgtgtgaacactctaacccgcgccactcagcgtggcgggagacagtgtcaggtaggcagtttgactggggcggtcgcctcccaaacagtaacggaggcgcccaaaggttccctcagaatggttggaaatcattcaacgagtgtaaaggcagaagggagcttgactgcgagacagacaggtcgagcagggacgaaagtcgggcttagtgatccggtggtaccgtatggaagggccatcgctcaacggataaaagctaccctggggataacaggcttatctcccccaagagtccacatcgacggggaggtttggcacctcgatgtcggctcatcgcatcctggggctgtagtcggtcccaagggttgggctgttcgcccattaaagcggtacgcgagctgggttcagaacgtcgtgagacagttcggtccctatccgtcgcgggcgtaggaaatttgagaggagctgtccttagtacgagaggaccgggatggacataccgctggtgtaccagttgcgccgccaggcgcaccgctgggtagctacgtatggatgagataaacgctgaaagcatctaagtgtgaaactcacctcaagatgagatttcccattcctatatggaagtaagacccctgagagatgatcaggtagataggttggaagtggaagtgcagtgatgtacggagcggaccaatactaatcggtcgaggacttaaccaagtagaaatggtgttcaagggcagaaaattaatattagctagttttgagagaacgaagttctttcaaggaaaaatagtgtggtggcgatagccagaaggatacacctgttcccatgccgaacacagaagttaagcttctgcacgccaagagtagttgggggatcgccccctgcgagggtaggacgttgccacgcgattattccggcatagctcagttggtagagcacctgactgttaatcaggttgtcgacggttcgagcccgcctgccggagttattatttttaatggagagttgtccgagctggccgaaggagcatcattggaaatgatgtaaacgggtaaaagcctgtttcaagggttcgaatcccttactctccgtaaccgaataataagtttatgacccgttggtcaagtggttaagacaccgccctttcacggcggtaacatgggttcaaatcccgtacgggtcattatggaggattagctcagctgggagagcatctgccttacaagcaggaggtcacaggttcgatccctgtatcctccatttccatagcaacattggttcgttggtctagctggttaggacgcctgcctgtcacgcaggagatcacgagttcgagtctcgtacgaaccgttgttatgtatttgaaaattgaatgcacaacataggtattattatactcaagatggttaatggctcggtagctcagtcggtagagcaatgcattgaagctgcatgtgtcggcagttcgattctgtcccgcgccattcatggaggggtagcgaagtctggctaaacgcggcggactgtaaatccgctccttcgggttcggtggttcgaatccactcccctccatcttatagggatatagtttaatggtagaactacggtctccaaaaccgtcggtgtgggttcaactcctactatccctgttaataatactatggcggtattggtgaagtggttaacacatcggtttgtggatccgacacgcgtgggttcgattcccacataccgccttttgattgggttatagccaagtggtaaggcaacagactttgactctgtcatgcgctggttcgaatccagctaacccagttgggttagccaaagttatggcggtatagccaagtggtaaggcagaggtctgcaaaaccttcatcgtcggttcgaatccgattaccgcctttttccatgtgttggccaatcaaatattattttgccggagtggcggaattggcagacgcgctggactcaaaatccagtgatcgttgagatcgtgtgggttcgaaccccacctccggtatcactaacaaatatcaataaaaaaggaatcattgaatatcaatcaatgatccttttttattgacttgaaattgaatcaagaacaaaaccacaattaccgatacataccacaaccacgctcaacacgaggctgtgattgatgcggcgttgtacaataatgagtgacaccaacggcacccgtacacagcgttaaggcggatgcacatacaattaaaaatttcacggacgttcaccaaccttcataagttaatttaggatagcattctacgtgatcattttaacatagagctcaatgcgagtcattaccaatcaatacaggactgattaacgatagtcggatgtattgggtgagggagggtaggaaaattagtgagcctccattaccattgcctcactaccgttttttagtttaaataggtcatctataaataatcagcgacaatttttaaaagaaaaagattgaagattatcgtcttcaatccaaagttgtcttgattcagctagggtctagcatattgattaccacgcgatgcttgggttgcaccactggcatttgcttgaaaaacactctcgtaatggtaattattgggattcttgacctcagaataatacttgtcactatcagaaacaaacaccattccggatccagcaattgtccaaccgccatttgtagttgtggctgtagcactctgatgtgaattggagctcccagtcgaagtagttgaacgatgatgtgtataagccatcgtcgagctgcgtcggtgatactgtttggcgttgttgctgccgtcttggtaatcaattcggataccttcagcgtcattgataaccacaacttccgtgttcaaagatttatctgatgatcggacatcgacaattgatccacggggcatcgtttcgcttcccttatacaggggagttgtttggtaataaataacgtggtgagtattggggttgtcttcccagtaattttccgccgcttcctctgcggcgcgcattccaccattttgatcggcgcccacattttgcggtcgggtacccgttgtgaaattgtagtttgatgtatatgatttggcccccagcaaactgtcaccaatcgagtggctccggttgtaaaggtagccatggtaggtccgccccgtcagtccataggtaattgacaccatcttgttttccggccatgcaggaggttccagtggatctccttgacgaccgccctgggacagatgatattcagaataagtcagcactgctcgggcagtcgcagatctgccttgggcatcagctgagaaatgatagtcaccagctgccagcccggcaaaatggctaaaatgagcttttccagttgtccaataataatcaccagtcggcccggcggattccttgttggtataactcaccagcttgttcaaaatggcttggtgctgttggcttgccgacgcagttgaactgtggtgtgaatgagtatgaactttttttgctgattgggttgcatgagaactactggttgtagccacctgcgatgcgtgatgatcggcggcctgatgactgccactgccatcgctgcaacccaccaagccgccagttatggcaatcaatatgacggctgttagcaggatatgttgatgtgatttcacgttgtgatccccctcaaaaaatgtttcgttggccaaatcaatcggccgcataagtcgtaatacgataaaatgcgaacaactattcatttttattatacagttgaatctcatctgttaacagacgaactggaagatcgatttggttaaagctagaataaggatcaagaaacttgagcactgatgggggacttgcttctagagacccccatatgaggatccgaaaatgtctgacgatcctttcgtagtgtatgccattgaacgacacactaaaatgtcaactgacgataaaaaagcccgtcacgaaatatttcgtaacgggctgatcaatttaatcatctaatctattagacgttcaaaattttattcaagaaatcctgtaatcgttcattctgcgggtgttcaaaaatttgttctggggtaccttcttcaaggatttgaccgtcatctacaaacacgacccggtcggctacttccttggcaaatcccatttcgtgggtaaccacgaccattgtcattccttgtttggctaagtccttcataactgctagaacatcgccaaccatttcgggatccagtgctgaggttggttcatcaaacaacatgatgtctggattcattgccaatgcccgcgcaatggcgactcgttgctgctgaccaccggacaatgattgaactgtcgcatcgaacttctcctgtaagccaacggttttcagtaactttttagcctgaacagctgcctggtccttggtttcctttttgagttcgacaggagccaacataatgttttcaccaacggataagtttttgaacaaattgaaatgctggaacaccataccaatattttcccgtaccgcgttaatatcaacatcatttctggcaatgtcgacattgtcaataacgatcgatccagaagttggttcctccaacttattcaggttgcggagaagggtactctttccagatcctgaagggccgatgataacgaccacttcattcttttgaaccgttagattgatgcccttgaggacttcattgtcaccaaaggttttgactaaatttgtgacttttactttttcgctcataccttagttctcctttgtacccaatttgataaccaagttaatacagtaataataatcagataaattgcggcaacgattgtccagactttgaatccttccaagtttctcgcaataataattttaccggtctgggtcaattcaagcaaaccaataattgataggattgacgtatccttcaaagtaataatgaattggttaataaacgacggcaccataattcgaatcccttgtggcaggataactttacgcatcgcttttccaaacggcagtcccaaacttctcgaggcttccatttgtccgggatcgacggcttgaatgccgcctttgacaaacgcggcgatatacgcaccttcgttaaaggtcagcgtcacgaccccggcgacaaaggcaggaattttttgcccagtcaaactcggaattccagtataaatgaacagtgccaaaaccagcaggggcattcctctaaacaggtaaatcaacgttgtcgaagttccttgactgaatttgttaggcaccacgcccatcaatccaaccaaaacaccgaagatggttgcaaagaagattgataccactgtcagccaaagggtttcttgcagccctgaccatagggcacctttattttgcttaattaagccgataaacgtccggtcttcggcgctgttgccagatgtcttggcagctgtcttaatctcatcagcacccaaatatttggccttaatgctatcatatgtgccgctggccttcagatctgccagtccttggttaaacgcctgcagaagtgcttggttatgaccttttttaaccgcaaagccatatggtgcgttcaatgcaggcttggtgacaatcttcaacttggttccttgcttgattgcgtattgcataaccggatgatcttcaaaacaggcaactgaattgccggttgagacatcttgatacatattattggaatcatcgaatgtgaccactttaaagccgtatttctttttgatgctattagcataatcggcacccgaggttccggttttaaccgcaacccgtttacctttcaactctgacaatttatgaatcttgctgttcttagcaacagccatgacaactccagaattgaagtacggtttggaaaagtcaaactgggctttccgttcgttggtgattgacattccggcaatcacaccatccgcttgaccggattcaacggcttggacggccgcgttaaatcccagggctttaattttgactttaaagccttgttcgttggcaatagctcggattaaatccatgtcaattccgacgtatttgttattcttgttggcaaattcaaatgggggaaaggtaacatcagttccaataacgaaagttttgccttttactttggaattattggcgtttcccagatacttaccgacaattttgtcgtaagttccattcgcctgaatctttttcaggccggcattgaatttcttaattaatgccttgtgagtgcctttttttaacaccaaacccataccaaccttggttagcgggcttgctggcaatttgaagctttaaaccgtgtttaatgccatactggagaacgggttggtcgtcgaaacaagcaaccgagttgccggtcgtgacgtcttgatacatattatctgaatcatcgaatgtcacggtcttaaacccatacttcttcttcaaactattggcatagtccgcagcggccgttccggttttgagcgccacttttttacccttaagttgtttgaaactggtgatgtcactgccttttttgacggccatgaccgcaccagtcttatagtagggtgttccgaaatcaaacttatcttttcgttccggggtgatcgtcatcccggcaataattccgtcaagctggccggattgaacggattgcaccgccgcgttaaatccaaccggcttaacattgactttaaagccttcctctttagcaattgacttgataatgtcaatatcgattccaacgtatttgttttccttgttggcaaattcaaatgggggataagtaacatccgtcccgatttggtacgtcttagcttgtgctttgctgcctggtagtgccagacagaacaagatcgtggcaaaagctgccagcaatccgaaagccgttaacactttgcgcttcatgaattattcctcctagacatatgtaataaaacataacatataataatgagaacataataccagaaatttgtgaatctgtatagcattaaccaatttgtgcaaacggtgccaagcttgctgcgacattgcaaaacgctgagaattattaattttaaattagaaaatgtgttgacattgatttggcagtttatcataataatcattaaaattcatttagcatttttatgatcatttatacataccacattggaggaaatcagttgaaatttgaagaatcgaacgttttacagcagttgccgaaacaattttttgccggtctggtcaagaaggtcaatgctaaagtggccaccggtgcggatgtcattaacttgggtcaggggaatccggatcagccgactcccgattttattgtcagatccatgcaggagcaaaccgccaatcctgccaatcataagtattcgcaattcagaggtgacccggaactaaaacaggcagcggccaacttttatcaacgtgaatatggggtcactttggatcctgataaggaaatcgccattctcggcggttcaaaaattgggttggtggaactaccgttggcactgctgaacccgggggacacaatgctgctgccagatcccggctatcccgattacctgtccggcgtttcactggcacaagtcaaactggagctgatgacgctgcgtgaacaagacgactttttgcctgattatcggaccattaaacccgaagtcgtggatgcggctaagctgatgtatctcaactatcctaacaatccaaccggagctgtggccacgccggaattctatcagcagacggttaactttgctaagaccaaccatattggtgtggtgcaggattttgcctacggggcgattgggtttgacggccgaaaaccggtcagtttcttacaaactccaggtgccaaagaagtcggaattgaaatgaacactttctctaaatcctataatatggctggttggcggattgggtttgcggccgggaacgccgatatgattgaagccatcaatctgattcaagatcatttatttgtgagtgtcttcccagccatccagaaagctgccattacggctttgaatagcgatcagcagtccgttcatgagttggttgccctctatgaaaaacgccggaatcaatttttcaaggctgctcgagcaattggctgggaaccctatccatccggcggttcgttttatgcctggatgccggttcctgagggctataccagcgaatcattcgccgatctactgctggacaaagcagcggtggctgtcgctcctggtaacggttttggccaaggcggagaaggtttcgtccgggtgggcttattaattgacgagccgcgatttaccgaagcttgtcagcggattgccaagctgcatttatttgattagagtttactagcaacctcgttttgcgcctaaatgttatctagcagaactgtgcgccaataagcagcttccggccgtataaggggattacccaaacatccaagttctggatatttgggtaatccccttatactctggaagctaactgcttatttgcccacgctcgtttgcctaaatcgttaaaatcagccgatcgcgcagctttattttagataatcgtggaactcaaagccaagcatctttggccgcctccatagttaccagtaaccaagaagtttggtcaattttgctcgattcaaatcgcgattggtgatcgtggccatttcggtgccatccaatccattgatggatttttcgaccggcttctgccatgcatatttggcaatcatattgccggcactggtcgctgcatacattaagtctgcctgatagccggtgtggtcaagcccaagggtatggccaagttcatgtgccaggacaccatcccaatattgatcaatcgtaaatttggcagctagactgggtttgatataccccagcggatatttggcatcgtgatagtgggctttatcaatataaatttgcctgccgtcgtaaagaccatcccagccttcttttgtcccactgccaaatgaaatctttaaggtatagtggctttggcttcccatctgaaagacggtttcacccaaggcagtattccatttgttcatggcgttttgaacgtgctggttcaattctggattggccacgtaaatcaacgcttgatgatccttgaacattgaggttggcgaaaaatgaaaaacgttatatgccaagtcaaaaacagcttcatgggtttcatagttcaccggtttcagacttaggatagtttcatccggattcatgtctggggctgcattaatcaatttcatcagcgacttctgagacattgccacttgcgttttggttaaatagccgtgccaaatataccccgttattgttttgcttttattggcaacataatagtagactgccgttttaccattcggctttctgacggtcacccgtttagtagcgtagaagatcgtttccggataatttttagcgttgtgaagtttttgcgttagcgttttatccccatagataatccctttgactgctcgataggctgtgcttttctggggagtgacccggacaacttttgccgctgtggtttttgcatcagccgaggttgcggcaacatcaatcatcaatgcaaacgaaagcagtccgactgccagcaacgttaatttttttacgacccgattcatttgaacgtgcctcctcaaagctgcaagtgtttccattaatataccatatccgattgataatttgctacttatggccttggccgcttctcagaagttgtgaccgtggattttatcagtggtaatctctggcattggttctaccagatgggtcgtatccctgtattcgatgcttagatgactcatgtttttaaggtcggagagaacctgctgatatttgtggggatcgtgaaccaatgctaataactcatgtgagcggaccaacttggtttttaatttccgactataaatgaagaagtaataacggtcgttaaaatggttgtcgacgatcaccaaccagtattggtagttgggaagtcgcttgaagtattggtggtacttgtcaattagttctcttgattctgccagcatggtgaagacctccttgagataaatcgttaagcttgatggccgccaaccaaaccggcacggtcgattgcggtaccgcctttggttttggacgaagctctgattagtgctttgtaaccgtattttttgcggataatgtcgatggtttgctccaatttttccttatccaaggtagtgataggatcctcaaacaggctgaagcgggtttcacgcttttttgaaagccgattgcagcgaaccccgacgttacgaactgcgctgccgtcccatttactttccaataaatagtggacggcattggcaatgcttttggttgagttggtgggttcaacgtgcatttgggctgagaagtgggttcgcccctgcttgtctgtggtggccatcccgatgaaaatactgacgacttcagcgacgacgttgttttttcgcaggcgggtcgcgacttgatcggcaatttcaccgaaaacagtttttagatcacccaattccgtgtagtcgcgcattaatacctgtgaattgccgtaacctttattgtctgaacggggaagataacgcttctcaaggttggagtagtcaatgccccacgcgtggtaataaagctgttcgcccatgacaccaaatttcttctttaacagattaacgtcggcgtgggccagttctttaatggtataaatgcccaactgattgagtttgacggccgtgtggctgccaattccccacatatcggcaagatctggaatctgccaaatagtatcgggaacgtcggcgtagtcccattccgcctgccaaggttcttttttcttggcggcgttatccaaggccagtttggccagcaggggattttgtccgatgccaatcgtcgtgacaatgccggttgctttaaaaactttgtcttgaatcaatttggcaatttgggcattggaaccaaataatttgtggctgtggctgacatcgatgaagctctcatcaatggagtaggggaaccagtgaatatcatcggtaaattgacggtagatgcggttgattcggtagttaagggcaacgtaatcggccatgtgcggttccaccatttcgatatccatctgatcattaacttcaaatcgccgagtccccagtttgacgccaaagtttttcttggtgtagggactggcagctaaaatgagtccaccggaggattcttcgcggctcatgacggcaattttggcggaaaggggatgctccccgcgcttgatggcctcagtggaggcgaaaaacgacttgcagtcaatgcacataatgtcgtggctgggcaaaaggctgggattatcaagaggtgtttgcataaggatcacctgcgattggaaaagttttattgagtatctatataatacgaacatttgtttggtgtgtcaagaaaaacagagcgcggaccaagccggttagcttctgagcatttatgtaatcacgagtgttgatgcgggttaggcatcaatactcgtgattggataaagcggaggaagctggcttggggagcgcattttgaaaacagagcgcgacgagacccgtttagggcccagaacataagtgaggaatgccaatgatgaacggtctgggttcatcgttggcattcctcacttatgtggccgggccctgggtcgtcggagcgcattttcaaggccgaagggagcagtaaatataataagcgcaacaaacttggtggaatctaacccaaaataacatgggaaaaggaaggtgatttatgtataaggaaaattgtatctgggtagaactaaccccaaaaagatcagtaactccacaaaaaagcgcccctcccaagttttccgccttgagaagagccgcttcaatttcatttttatcaattatcatcaatttcatcaatatttcaaaaataatcagacgctaatttgctgcttaaaaaatatctgagttaatcacctgcaactttcaagaacacggcgccaagtcccttatcaaaggttgctttccagtcgccattgctgagtgattcaggtagtaggaaagtaccgcttgaaacgcgttggccagcttgtaggggcattccttgtgattccaacttttcaactaaccagtggagggactttaacggattgcccaatacttctgatgaagcgccgtcctttagcttcttgccgtcatggaatagttcacatttaacgttggctagatcatcgacgttgtcaaataggagattggtatctttttcatcaccgtaaacgacgtagccaccaacggctgcatctgacatgaccatatatttagataggcttgggaaccagtcgctgaagcgtgaatcaggtacttcgacggctggagcaaccttggtctttctcatgagatcttctaaagaatctttgctgctgagatcttctttggcagtaaagagcatttcaacttcagcaagtggttccatgagttcgccacggtgaagggtaactggggattgtaggaaatggctcttaacttgggcgccatatagtggtgagtcggagtcaaacatatcttgagtttgcttactggtaagcgatactttgtagccgccaacgtcttcctgcttgagttgggttagtcgtctttgaacccgataggctgacttttcatccttaacgacaccatcatagtcggactcttttaatggcttgtgtgtctcgtaagcgttaaataatttgtttgctaattcattttccttagttgttaattccatcgttgcttgttcatccataagcgtttcctccataaattgtatttaatctgtggatcctcaactgtatgtacagtgaggaccactcagtgacgtgaaatatatgtgttgttatgtcaatggcactatgtcggttgaaattatgtgtttgcaaaatctgaatctgacctgggttttcattggagctgctaatcaccgattccataagtcctcaccaccttaaataattaattaaattcaaataaaaaggcatccttcaactacccggaaatggatagttaaaaggacgcctattgcgcggtaccaccttaatttgtagtgctattactagcattacctcacacgtacagctttcgcgatacgctgacacaataatgggtgcacccaatgcaatctactaaaactttgatcacatagctcggagatgataatcatctaaggacgtaaattgcttcacaccaaccagcaactctcttattacgaacggaaaatgacgtttctcttcatcgctttttaatttgaatttaatgattgtcattaatttacaccctgttattttgattgtcaacagcaaatttgaaattaattattctttgttgggattttctcgaatcacgcgggcaggattgcctgcaatgatgaggttatctccaaatgatttggtaacggttgaattagcaccaacgatgacattgttgccaagcgtaacgccggggagaatcaccgatccgccgccaacccaaacgtcatcgcccaaagtcaccggtttgcccagtcctacaaagttggctcgttgtttgggatcaaggggatgataagccgcgtaaatttgcacgtgtggagccagcatacagtgattaccaattgttaccggggcaatatccaagatgacgttatcgtagttacaaataaagttatcgccaacgtgaatattgtagccaaagtcacagcggaagttcggttgaacccaggggtcttttccgactgagccaaacagtttgcggaccagggcctctttttccgcaccggcagtgtcgtccagttcattcatcatcttacataagcggcgggctttagtttcgtcgttggttaattcgggatccatcaccaagtatggttcacccgctaaaaatttttccttttcagttgccatgtgattttccatcctttgttgtaaattaatttatattatatcattatttgtaagtataaattgtctttacacataatttattaggataaattagaaattgccgagtgacttaatatcgggtatgataaatgcaattaataatagataaccaaactcacggaatttgaaaggatgcagacaatgaaagcagttattacagtgattggccatgaccaaattggcattgtggcaaaagtttctcaacggttggcaactttgaaagttaacattaccgatatttcccagacgctgatgcatggtgattttaccatgatgctcatgggcgaatgggacgatgatgatgtgcagtttgaagttgtcaaacagggcttacaggatttggcaaatgagactggcctatcgattaatattcagcgtcaagaattattcgacgcgattcaaaagctttaggaggtcgccaaaatggaaaccaaacaaattttagagaccattcagatgatttctgaagaaaaacttgatattcgaaccatcacaatgggaatctcactattcgactgtattgatagcgatggtgttaaggcccggcaaaaaatttatgataaattgacgaccagtgccaaagatttggtgaaggttgctgatcgaattgaatcagagtatggcattcccattgtgaataaacggatttctgtgaccccaatttccatgattgctgccgcgtgtcacgatgataattatgtcgcctatgcgcagacaatggaaaaggcagctgaaaccctgggggttgatttgatcggcggcttctccgcgttggtgcaaaaaggctaccaatcaggtgatcgaaaattgattacttcgatgccggaagccttgagtgagacgcaacgggtttgtggctcggttaatgttggttctacaagagccgggattaacatggatgccgtcaaacaaatgggccaagtggttaaagatttgtctgaaatcgatccggtcagctgtatgagtctggtggtctttgccaacgcggttgaagacaatccgttcatggccggcgcctttcatggcgttggtgaagctgataaagtcattaatgttgggattagtggtccgggcgtggttaagcgggcgcttgaacaggtcaagggggaatcgattgacacggtttccgaaacgatcaaaaaaacggctttcaaggtcacgcgaatgggccagtttgtcggtaatgtggctgctaaagctctgaacgtgccatttggaatcgttgatttgtcgctggcgccaaccccaagtcaaggtgattccgttgccgaaattcttgaagaaatcggtttggaaagcgtgggtgccccgggaacgacggctgctttggcattgttgaatgatgcggtcaagaagggtggcgtgatggcttgtgaacatgttggcgggctgtcaggtgcctttatccccgtgtcagaggacagtgggatgatcaaagctgtcgagcatggtaatttgaatttggaaaaattggaagcaatgactgctgtttgttcggtgggattggacatggtggctgttccgggagatacgccggctgaaacaatcagtgggatgatcgcagatgaagcagctatcggtgtgattaacaataagacaacggcggtgcgggtgatcccggcgaagggcaagcaagtcggagagcaaattgacttcggcgggatattcggctatgcgccggtaatgccggtaaacaccaacagcccagcgaagttcgttcaaaggggaggaagaatcccggcaccgattcattcgtttaaaaactaagagcgcgacgagacccggttgaccccggtatataagctaaagacagcccctgatgaacggtctttgttcatcaggggctgtctttagcttatatgttaggggtcggggtcgtcggagcgtatctcaaaggttgaagggagctgtagatataatgagcgttacaacccctgtaggctaaaggacaaaagacaacccctgatgaacgttttttgttcatcagggctgtctttgacttatatattaggggtcggggtcgtcggagcgtatctcaaaggccgaagggagctgtagatataatgagcgttacaaaccctgtaggctacaaaaccaaagaaaatcgaacacgcatgatgaacgttttctgttcatcgttgcccgtcgttaagactacaaatccttctccaccacaacacaaggcacgccatcctcataaaacacatcggacgtgatctcataacccaggcgttgataaaatttgacggcgtccatttcactatgaatcagtgaatgagtgaaacccatttgtttggccttgtcttcaagggcactgacaacctttctgccaaagccatgtccacgggcttcctttagggttgcgactctgccgactttaagggtgtggtcattgtaagtttcaaaccgacaagtcgccactggcactttgtcatcaaataagaccgcataaaccatgctgtcggaatctttgtcatcgaattcatctcgaaaggcgattccccgctccaatacaaaaacggacattcgaatgtaagcagcagccccacgagctggtttggaactttccacgattaatttcataataggctcctcaaaatagacttcttgaactttaatattgagctggttatcctctgattggcgatactttaggatcggcaggccaatctttgccgacatcaacccaacggtcggcgtttgcatatttgctgagctcatcgacagataatttgactgcactgtgggtgtcacctgccgcagggtagatgaattcaaaccgctgaagggaaacgtccagatagactttaacgccttgattgagagcaaatgggcaaacaccacctggttgatggccaatatattcctcaacttgatctcttgggatcattctggcacgcttgtgaaattcggccttgaactttttgttgtcgactttggcatcaccggccaacacaaccagcagtggatgggaatcaatcaagaacgacattgttttggcaatatgttccggttcacaatttaacgcttcagcagcttccataaccgttgcgctggattcatccaagactttaatgcgatcggctaagccaacctcgtcaaagtactgtttcactttttcaaacgacatatctatcactcccgactgataaagattaagactaatatacaggttcacggaagaatagtaaataagatcttgattattccagaatgaaaaaaatgaatgagcagttaaggatttgtctgggactgaaaagtggctccagttctgacgggaatgggaattccaacagctaccaatgaccttttcaagctgccaatcctgatcgggacttaattaattgtcagattaatggtaacatgaaaccctatgatccaaaattatgagagaaaactgaagatttgtttaagtattgatttggcgagagcttttgctagattgaagtgctaaaacttcgtaaaatatgcttagagacagataaagggggttggcattagtaatgtcacgtaaagagaagttcgctaaaaagcctaagaaaaaaatatggatacggatcctggtgggatttgtgttggttctttttggtggcttcgtgggctctcatttctattttcaaaatcatttcaagttcaccaagattaacgacgttgatgtttccggtttgacggtcgctcaggcaaccaagaagttgaatacctcacatatcgatgaagacggcaattatttagtggttcgggattcaaaaatcaatgtgaattccaaggatgttaagaaattattcaaacaccgtagttcaatgagtgcgatgacttctgccaagctgagtgccaagtctgatgtaaccaacaagcaactcaattaccgcttgaagacgttactgccgaagtttgaaaaccgggttgatcaaatcaataccggtcgcaaacagaccattgattcaaaagttattttgaagaatggcaaaattgttgttcaagctggccagcagggaagcactctggataaggccaagatggtcaaagactttaagaagcaggcaaaatcgagtttattgatttcggttaaaatgactaaagatgcgtacgtcaagccgaatagcactcaaattgccaaacagaagaaacagttagccaacatcttggacaacactgtcacgttgaatacctacaacaagacctataagtttgttgccaaacgctgggttgccaatggttacccaactgctaacgggacctataagtttgattcaaccaagattaagaattgggtggccaaatttgccaataaagtcgatacccttggcaagtcggtttggattaccactcatcaaggcaagagggttcgtgttcatgctggtggaacctatggctggaaagttaatcaatcggctttaaccaaaaatatcatgaagaatcttggtcgttcacattccgtcacaatgaacctgaagcactatgcggttggaaccggttatggtgttaaggggtctggtaagacctatgtcgccatcgacctgcagcgtctccatgaatacgtttataaaaacggtaagctgatggctaatattccaatcatgtctggaacgttgaccggtggtaaccgaacccctcaaggcgccttttacattatgtacaagcagcgtcacgcaactttgagagggaagaacagtgatggttcaaagtatgcatcaccagtcagctactgggaaccattgaccaattcaggggttgggatgcacgattcaccatggcagcccgcctcggtctatggtaatccaagtgctcgtgcacaataccattctcatggctgtttgaataatccaccgtcacgaatgggtgaggtgtggaagaacacgcacactttggaacccgtatttatttattactaagaagtcaaatgactgttggcagggaatcgcctgccaacagtcattttttgatttaatatatgttaaactgatgataaatagcaaaatggggtgaacaatcgtgcatttatataaacacgttgatattagcaataaccgcaatttggtttatggtctaaatgtggtcgccgttattgcctttttaggcttcctgtggctgtttggtgccattgtcggctcaatgactgtcaacttcactgaaagctacttcgtttggctgatcgtggcattattagtgattgtgacgatccacgaggttttgcacgggattctttataaagtctttaagccaaatgggaaaattaaaattggtttcaaaagtggcatgttatccgtttccagccccaagtccctctataccaagcagcaatttatttggattggggcgactccatttgtcgtcatttcacttgtcctgattgcgatatttcttttgggatggctgcctggcgaattattcttaccattggcagccctgcatggggcaggttgtgtcggtgatttttatcttttatggctggtgataagttcaccgaagcactattacattagcgatcaagaaaatggcatcgatatttattcccccaactgaattggtggatttcaacggtgtctccgatacaataaagggattgcaaccaaagtctgagctttggcggcaatccctttattggatggttaacgttaatcttggaccaaaattttaattcctaaatacagattataaatgaacatggccagatccaccaggataactaacgcgattagcgccaggaaaagaaatccggcaaaggcggccttttcggaaatcacaccactgataccgacaaccaggatggtcaggatggtcagcacaagggggattaaatgcaaaataagcgcgtgtctggcagtgctgtgcatatctggattgttatcgctgacgatccaaacaatcagtggaaaaataaacggtgcgaagacaattgaaagataggataaagcattaacaattcgatttgtcgacatgtgagtaactccttagtgattggaataggatttgtagaccggcgaacggaaaagatcgacgaatgcacccccaccggaataatcccggagaacactgatcttttggccctcaacagttcggtgggtcttccgccagccacggtcactctgataggctttggtcgcataggcgttaaacgtgtaccggttcgtaccggaaattttagcaacagctaattttcgatagctcttccaagtggatttataaagggtatgctgcttgccgttgtatttttgggtgacggcgtatttgttaatctgggtcaaacagaacttcccgttgacgtatgaataccaattcccgcgccagctggtcggcgtcgaactgtgaatggcaccaacatgataataggtgtcagcagcttgagcaggctggtggttgacgaaaatggtaaaaatgaaactggcagctgtgataacagcaaccttcaacaatttattcatttaaattctcctaaaagtgtccggatcaaaaacagaattattttgacaaagttggctaattctttagattatactaaaaaatgatagcgtaccaagtgtggctttgtcaaataagcagaaaaaaaggcccgctgactttggtcaacgagcctcaccaatgcaattattgtttatctttacttcttctgattggatgctctttttcttctttatcaacggacttttgatacattttatcgttgacgtatggataggtccatttaaccatggccgacatgataattggcaaggtcaataccaaaatgatcaacccaacaatcacggtcatcgcaacttgaatcaaagtcaaaacgtttgacggaatcaacgcggcaaaagttccacccaagatgatggcagcggaaatgacgaccgttccaataatggttgccgaatttaaaattcgtcgacggacatccggaatggcgccggcatcaccacggtacctcatcatcaagaaaatactgtaatcgactcctaatgccaccaacatgataaaactaaagaacggtgtgttccaagtcagcatgttctggaacagcagatatcccgaaagccatttggtaatctgcagtgatcccatataggtcacgattaaggtgccaataatggtaatggcttgaaccagtgagcgggtaaccaccatcagggctaaaccgattcccaccagcatgatgacaaccgttcggaagaaatcgccattggcaatcttttgaaggtcagaagtttgagaactttgaccgccgatagcgaccttagcatttttcaaactggtgtccttcattttggcattcagatcgcgagtgattgtccgaatccggttagccgacttggtggtacttggatcggaattcagaaccacagtaatcttggtaatcttacggtcttttgacataaatgcgtcaagagaaggggtgaatgacgcactcttgatacttgcggcaggcatatagaaggtgttgcccaagtatgacttttgcatttccttcaagtacttgttaacagtggtggttccactggaaacttgatctaatcctgaattggcagaagtcaaaccagtttgtaattcctgcatctgactctggagctctttcattttcgaattcaatgtttgaacacccgaattaacttgagaactgccactagcgacactttgagccccggaaaccagtgatgaactgtttgaattcagtcgactagcgccacttgtaatctggttcaggccatttgagaacggagcaacttgtgaattcaagcggccaagaccggaagataattgtcttgatccggactgcaatgcggccatccgggcacgaagcgcctttagcttagcggtttggcttctcacttgagaaatccccgtgttcaatcgttgactaccagctgacaatcgaccgacaccggattgaagactggaggtgcctgagctgagttgttgcgaaccgctggccaagttgctgacaccggcagtgtatgaggtgacaccttggctcagttgttgcgcaccggcctctagtttgctggcaccgtcagctaatttctcaacttgtgcgatgctttcagaagtgtttgagttggctaatttttcgttggcactctttaaacctttttgaactttcttgataccttgattggcttggtttaagccgttcgtcagactttccagctgacttcttagataaagtgaatcaatcttggttccacctggacgggtaactgaggcaacactcttgaccccggcctcagaattgaggtagccggttaattggtcgatttcggctaaatgttgttgggtatccagtggtttcttgttttgaatatagacggtcgtcgggccggacatcccagcagggtagtgatcctgaatgatgttataacccgcttttgactgaaccgagttgggcaattcatcggcactgttaaaattgagtttctgactgccaacgaacaacagtggcaaagcagcaatgattaaaatcccaaccataatgaaactgtgtgagagggtgaactttgagaggaaattccacaggaaacttcgatcatgggcagccaggtttttgcttggccaaaagagtcgttctcccaaggtagacatgaagaacatattcagagtcaacagaaccattaatagaatggcaactccgacagcgaccgcaacgcctgaacggtagaaggagaacttggccaatgctaaggccgcaaaaccaattaaaaccgatgaaccactatacagaatggttcgtccggcatgtcgccgcgcacttcttgccgcgtcggttgcgccttgacccttacggatttcctctttaaagcggtcatacaataaaatgttgtaatcagtcccaattccaaacagaactaccaccagaaagacttgggtaaagttggagattgggaaatcccagcgctgggccaaattcatgaccacgtccaatgacagcaggtaggagacaccaactgtcagtaatgaaatgacaggaattaagaaggaacgaaagacgatgatcagcactatgaagatgaagattgccgcaatgatttcggtcttttgaagtccctgctcagtaaccgttgaaaaatcctcatttaagacatcactaccggttacgtaagttctcattcccggggttttaatcttatccaagattttatcagtctggccacgaaccttgtcttttttcggcacggtaatcatgaccatctgggtggtactgtcttttgactgcagctgctgtttggcagcttggttgtcacttggggctgtgacggagataatgtgcaggtccgggtcgttcttgacggcgttggtggcgtcttgaatctgtaaggtctgctcatcactcaacttgccgtgcttgttattgaaaacggcgatgagggttcgggcatttttgccgccctcatattttttctcaatcttattggcaacttcactctgcaccgaagcagggagctgaacagtccctttgtcatggaccagttgggaaatatttggcaacgtaaaaattgccaccaaaattaggccaatccacacaatcagtgataacagatgcttctctttgaatttctgcattaaaattcttcctctcattccctagtgataaaattattctcttgttcaaatttagacacttgtataagcaatattaaaatgataaactcggcgtgaatctgacgcaagggacattttgctgcgttagtttaaatttagacaaaattcgataaatgcaaacagaggctggctcatgaaatatgacttaacaaagaaaccaacgcgtggtgcgcaacgaaccttggaatcattttcgacgacgatgatcgcgcttctctccaaagagccgttcgaaaaaattagtgtcaacgagatttgtgcggtgagtaattttccccgagcgactttttataactactttgacgataaattcgacttggcagcgtattgctggtatgtaattgcccaagaaattgaagtggatcaggcgactgaattgaaagctgatcgaacgttgatcacctattttgatcgactttacgacgtgttcaaaaataaccagacgttactcgataacgtgcttcagtacaatgatttttccggacagctggttaacagttttattaattactttaaaaataagctgcaggaaatcctcaccaaatcaattgattattccaaggcgggcctaccggttgaattgatcgtcgatcattgcagtcagacggttgtgctggttttaaaatggatctttttaaagcatcatgatgccgacaaacagcaggctcatgaatatttggagaagttgttgaatattgaacattttatctgaattgacacatcaaatgaatcattcaatgactatatagtaccatgaacgaccttttcgtgaattgaattttcatgaaaatattgagcgaagcaacctctattatagcaaaagtggccttcatttgtgcgttaagttgagatgtgttagcatgctatttaagtgttcccaaagaatgcttaaatcagttcaatgatgaggaagtgacagaatggtcttaacttcagatgaagcagctgcaactaagcaggaactccaaggcaacttcgagttgtcagggatcactttgcagatggcggccgttgatttgaaaagcacgcctgaacatattcaggacgttttaaacttgaaaaattgccaaaaagaagaaccttggatcctgcgtaattacctaattaagctcattttgcttcaggaaaaagaaccctattcgttctccaaattaataggggatcccaaacgttatcagtttttgaacagtcgcttgattgatcgtggcgaattggcctaaagttttaataaagtgaatgattgtgtcaaatgaaaacaatccaaaattagatccagttaaaactgcttgaatttcagttttaactggatcttttatattactccgaggatgaatgttgggacctggtttaattactactataaatggccaggatcaaaacgcctcgcatcgcactcgcctgaattccacggttatttagcttaaatgtgtgcaagaggacagtaattgaaatttaagcgccgccacccgaaaacctgactcggtttccttgtgtcttactgttatttggattaaacgtgttcaagaggacagcaactaaattttaagcccctccacccaaaaacctgactcggtttccgtctggaggggcttaaaatttagttgctaaacgtcctctttcacactctcatcttgaagtagtcacatcactttgcttaacccagccattgacttgggggtgggcagcgtctgttacatagtagtaagtggcattgccatcgcgattgttttgcttggtgccgaccttggtcacggtcagtggatccttgtaaaagtctgccgttgcgttgagattgcgccccactttatattgggtatagtcaggggcaacgtaggttaacgtggacgcttttggtgtcgtaaagtacattgtggtgttggcaaaataagttgggaccgttgattcctggaaggtcgtcgttgcctttaagccgccggaaacatcactgggattggtcgtcggatcggttgttccggcaaatatccagccccgataggttttatcgaaggaaacaactttcagataccagtcgccatttgaggtctgagccgcccgataacctctgaagtaggtttgcccggcatccgcagttgtgccaagggtctttaaaacggctgccttggtgacaacttttgtactcttatagaccggcacttttgaatagagtggtgctgctccggttgtcaggtaattgcgggagttgccatccgccacgagcgcctggttgctggttacagtcatcgttgatttggcctcagtgtcggttggcgttaaggtaaatgcgccgatcgcaagtgtcaggccaagtcccaatatgagtttgctggtgattgttttcaaattcatccctccaagcacaatctttattcaaaaagtatacacccatttgaaaacgaatcatacaatcgaagtcaattaaattaaaaaatgattagttcgttttcgaatgacagttgacaaaaatacatagttacctgatatatatcactggctccattcattgaacagcttactgattagaatatttttaattttaagtatatttttgaggccgttcgttgtatcctagttgtaaatattatttacaatagtggatattcatacaaggagtgacgacatggaaaaacacgagtggttattttcgcaagttcgctggttgttcattgtgatcgcatttgtcggaatggtgatcggcctgaatacacaattggtggatgcaaaggccagttcgctggaaacagatttccaacgagcggctgccaagtaccaggtgccggtagatctgcttaaagcggtggcttataatgaaagtgcgtttgatagccacaatggtaagcccagtgtggccggcggctatggtgtgatgcatttgactgataccactggcttaacgccaagcggcgcagattccaaagcggttaaagtgccaaatgccgcttctctgcatacgctgcaaaaagcggccaaattgaccggtcacagtgttagtcaactgaagaccaattcagctgccaatattgatggtggggcggctttattagcagcctatcagaaatcctcgggcaaagggctaacgtcaaatattggtagttggtctgcagccgttaagaaatacagccagtcggattttcaggcagctgctgatttcttcgccgccaacgtatataaaattttggcaaaaggcgtcaatcataacggcgccaaaatctcaccccagaaggtgaatgcattgaaagatgaagcaatcgataccaccggtgaatcgggccaaaccgatggacctgccggcctgccaatcgaatggattcccgcattatacaaaacctttgatgatcaaggcgactatgggaactatgacctggctgaccggccgaacgacgaaaagattaattatattgtgattcacaacaccgaaaccagttttcaagaagctctgacactcttctcgacaccgacgtataccacggcgaactacgttgtcagttcggtcgaagggacagtcgctgaaatggttcgaccgcaaaatgttgcttggcacgccggcaactggtacattaattctcattcaattggcattgagcacgagggttatgcggcagttggcggctactggtacaccgaaaacatgtacaagtcctcagccgctttggtgaaatatctggctgataagtaccagattccgctggatcgtcagcacattatcggccatgacaacgtgcccggtttaacaccggcagctcaaaaagggatgcactgggatcctgggacttattggaactggaatcactactttgaattgatgggcgttgatttatcaaaaagtgacggcagcacggatagtcacattatcaccattacgcctaatgacaaaacgaatttgacggccgattcgggacaaaaagtgactgatgacggggtcagccttccgctaaccggatcaaattttgtttacctctacaagcaacctagcttcagtgctgacttgattgctgataaggacttttcttccggtcaagccggcaccactgaaaaggatgactggggcgataaagccgtttacggccaacaatttagtaagatcgatcagcagggggattggacagaaattgattatggcggtcaagatgcctggttctacaatccgggtggtgctaattcaactgatgccactgggaagctcgtagcggctaaaggatcaaaagccgtgccggtgtacggcagtgcctatccaagcgacagtattttgaagaagaataaagttaccggcattaaaccaacaccaatttatcaactgcagccaggtcaaaaatacgtttatggcggcacagtcacctctgattacttcaattcacacttcaattccaactcaccgaagaacgtcattcatggcactgatgattattatcagattcaatttaatcaccgaattgcattcgtgaaggcgtcagataccactctttcagacgattgacagattaatcgatagcaagtgaataacttggaaaggccgaaacagcaaccaatgtttcggccttttttaatcgctattaatgtcaccaaacatcacatcgaccaaaatttgctcattttactgcaaaattctgataatggtgtcaccaagatgtgaggtattggtatacctgtaatttgaggaattttaacgaagactgttgactttctgaaaaatgggtatatattaatagccgtaagtaaatgtcacaaaacattacatgaaacgagggaatagaatgagaattgagagagattgcatcggagaaatgtttgtacctgataacgtcctttatgggattcactcactgcgagcgaaacacaactttccaatcaccaacgaaaaagttgatccggccatcattcaaagctatctgcagatcaagaaggccgctgctttggctaacgagcaggcgggcactttggataaagaaaaaagtgctttgattatggctgcctgcaaccaattgctattctcaaatgactacagtgcctttatcgtgccagccatccagggtggtgccggaacgtcaaccaatatgaacgtgaacgaggtcgtcgcccagcttgccatgcaattaagcgcccagggtggaaaagagcccttggtaatcaagcccaacgatgatgttaaccagtcacagtcgaccaatgatacctatccgacggcaggcaagatggcgatgttaaaacggttggcgccattgacgtcagctgtttccagtttggttgacgccttaaccgataaagccgcagaatattcgtcagcaatcaaagttggtcggactcagctgcaggatgctgtgccaacgacctttggcaggacctttacagcttatgcttcaatgtttaaacgcgatctctcaagattaaagcacgctcaaaaggttctttctcaagtcaacctgggcggaaccgcgattggtaccggaattaacgcgaccgctgaatacgaatcagccattattcccattctcaacaaatattctcatctttcattgcatcaagccgctgatttggtggacgccactcaaaacagtgatgctttcaccacgatttcttcggccatgaagtcattagctgctgatttatccaaattcagcaatgacttgcggctactttccagtggccctcaagccggcctgaacgaactggagctgccaaagaaggctgcagggtcctcaattatgcccgggaaagtcaacccaatcatccccgaagttgttaaccaggtggcatttgaaaccatcggcaacgacgtcacggttacaatggctgctgagagcgggcagttggagttgaatgcatttgaaccaatcatgttcaagagtattttgactagtgagcagcatttgaccaaggcaattgagacgctggttgaaaactgcgtcagcggcatcaaagtcaatgcagcatattgccgaaaggaagtcgaacactcatcgatcgcggcgacggtgctttcaccgctgctgggctatgaaaagacgaccgcgttgattaaggaagcattagccactcaacaatccgtcaaagcactcgtcaaacaaaagcagctgctcccggattcattggtcgacaatctcttcacaccagaagttttgacgaatgttcgcaaagttaagaaagaaaagtctgctgccggttcaaatttaaattaaccacgtttcaccgaaagtcaacctgatgagggctgactttttctttttgaccaaaacagaatcatcaccacgatctccaatcgcgatataattgagttggttaggtcaacaatttgaaaaattggggtgatttgacaatgaaacagaacaaatcgacactgattgacgatgatgccaaggctgatcccactgatttgatgaaccagtttcaaaccagcaacggtggtctctcgcaggcagaagccgagaagcgtttagaaaaatacgggccaaatacgattcgacagggcaaacgaaagtccgaagtgttaatctttttggaaaactttacctctttgatggcgattcttttgtgggtatccggtgtgatcgccatgtttgccggcatgctggaacttggaattgctatttgggcagttaacgtcatcaatggttgcttttcatattggcagcagcacgccgctcaaaaggcaaccgactcattgaagaaaatgctgccatcttatgttaaggttcggcgggatggcaagtctcagcagattaaagttgaacagctggtgcctggcgatatttttgatattcaagcgggggattcaattcctgccgacgccagggtgtttaatgctgccaacctccaagttgacgaatcttctttgactggtgaatcggtgccagttgaaaagcatgacgcttatcagcacggcgatggcgaatttgctcaacagaacatcgtctttgctgggaccatttgtaccagcggcactgcgacagctctctgcttggcaaccggaatggatactgagttcggccgcattgccacgttaactgagtcacagaaaaagaccgtctatccattggaacgggagctcaatcatttaacccggcaactaacgattattgcgattatgattggcgttgcctttttcctgctggcaattttcttcgttaaatatccggtgaccaagtctttcatttttgcattagggatgattgtcgcctttatcccagaagggcttttgccgacggtaactttatcgttggcgcagggaacccaacgaatggcgaaaaaacatgcactactcaaaaacctgagcagtgtcgaaacgttgggacagacgacggttatctgctccgataagactggcacgctgacccaaaatcagatgactatcaaccatctgtggctgccaagtcaagaatatgatgtcactggaaccgggtacgtcactaacgggcagattcagttaaatggccaccaggttgatctagcaggacagcctgacctcgagaagctgttgattaatgcaaccatcaataatgataccgaggttactgaaggtaaagccggtgaaaaatcaaaaattctcggaaccccaaccgaggccggattagtgatcctgtcacgcaaagccgagattgatgccgccgccgaacgccaaaagtttcccagattaaaagaattgccgtttgattccggccgtaaattgatgtcggtcatcactaaaaatgcggacggtaagttggtcatcaataccaaaggggcgttaggcagtgaattaaacgtttgtgaccggattttagataatggtcatattcgacctttaacggctgatgatcaggctaaaattatgcaggtaaatgaaaattacgccaaacaaggcttaagaacgctggcattttcgtatcgggtggtggatgaaaatgatccactaagtcagcagtcacttgaaagctgtacgattgaaagtgcggagaagcagatggtcttcattgggctggccatgatgtcagatccgccacgaccagagatatttgatgctgttcgcaattgtcgacgggccaacatccggatcatcatggttaccggtgatagcccgacgactgccaaaagtattgcgactaagattggcattacttcggacaaggtcagagtcatttccggctccgaactggataagatgtctgatgccgagctgcaggaagccgtcaaaggggaagtcatttttgcccgggttgcaccggaacataaatttaggattgtttccatgtgccagaaaaatggtgacgtggtggcttcaaccggcgatggcgtcaatgacgcgccagcactcaaacgtgcggatatcggcattgcgatgggagtgactggaaccgacgttgcaaaagacgctgcagatatgattttgaccgatgataactttgcctcgattgtcagcgcgatcgaagaaggtcggaccgtttacagcaacttgcaaaagttccttctatatatactcactagtaatgtccccgaagccgctccatcggtcatcttcttgttgacccgtggactggtgccattaccgttgacggttatgcaaattttgacggttgatttgggaactgatttactgccggcattgggactgggaaccgagaaagccgagccaggcatcatggatcagccgccccgtccattgaacagtcacttgttgaaccgatcgattatctggaaagcctttggttggtacggcttgattgcttcggcaatttcgacgtttgcctacttcttcgtcaaccacgtcaatggctggcctcaagttccattggccggatccggtttggtgtacgcggaagcgacgacgattaccttggcggccattgtcttctcccagattgcagcggcgatgaactgccgaacgcagatttcatcagtcttttcaattggcttatttagcaatcaccgcattcttttggggatcgtcgtggaagttgtcttagtcgcactgttgatgtacgttccatttctccagggcgtcttcaataccggaccgctaaacgtcacagaatggggcttcttattctgcattccggtgccgatcttcctgattgaagagctgcggaaatatgtggttcgccagattaaaaagcgacgggcgaagacttcagtctgataataatgttgcatttacaacaaaaatagtttagaatcaattctatcaagaaagggctgattaagtggcagagattttacgacccatcggtgcgattgccagagccttggattcaattgccaacgttgaatttaaacggtttgatcttaccaaaggccaatatttatatttggccaggatttgtgagcaccccgggatttttcaagaccagctggcaggaatgatcaaggtcgaccgaaccacggctgcccgagcaattgataagctggcggcaaaggactttgtagttaaacggcctgatttgaccaaccaaaagattcgacgcttgtttccgacagaaaaaggtcaggcgacctatccgaatattttgcgggaaaatcagtattccaaccaagtggcgctaaagtccatcaccgacgatgaggccgaccaactggaacgccttttgcataaagttagtgccaacattgacgatgactggcattatgttaaaaaaggcaatcttagaaagtattgaggatgaacttgtgacaattgtgattagaaaatgtactttggcagatctttcagaactgcagcagatcagcagagagacttttgctgatacgtttggtccggaaaatagtcctgccaacgtgaatcagtatttggatgaatcgtataatcttgaccggctcaaacaagagctcaccgatccggattccgatttctttttcgccttggcggatggccaagtagccggttatttgaaggtcaacgtcggcaatgcccagacagaagccatgggcaaccatgccttggaagttcaacgcatctatattaagccagctttcaagcgacaaggaatcggatcgaaattgatggctcaagcattggcggtggcaaaagataaacaccgttcgaccgtttggctgggcgtttgggagtacaatcttgtcgctcaacagttatatcaaaaattcggtttcaaacaaaccggcgatcatgtcttcacgctgggcgaaagccgccaacgcgacctcattatgagccgaacaattgaaggagagagccggcattcatgaaaaaattcattttagatcccaaaaccatcgaattatttccagacatccatattgacgtgatgaccttacatggcatcgataatcacgtgaatgaaaaggacgacccgtatttccagaaactcctggatgagggcaccgaggcggccgaacaatttatcaccgttgacccattccgtgataatccggtggttgccgagtggcgggaagcattccggaagtttaagaccaagaagggcgcccgttcaacgattgaggccttattaaaacgggtcagtcacggaaaacgattttcaccgattgcgccgttagtcgatatttataacagccaatcgctgaagtacggcgtctccgttggtggtgaaaacgtcgacgccattgctggggatatgcacctgggagaagccaagggtggcgaatccttcctgccatacggtgagaccgaagatatgccggctttacccggcgagatttgttatatggacgataaaggcgcagtttgtcgttgctttaactggcgcgaaaatcagcggactgaattgaccgaggacaccaccaatccgatcatcgatattgaatcgattaatgaggatcagtcggcccgctcagatgttgccatcagagaaattcaacgtctctgcaaagaatattttggagttgttggtcagcttcaacaattgaatgctgaaaatcctgagattgtcattgctaaataaattcaaaaggcggttgtcacattcccttgcttggggatgtgacaaccgcctttaattttggttccgagcttatttgtgatacttatcggcaatattgtatttgatatcaccactatcaactttcaacaagactttcttcttgttatgcttgtcgatcaccttgaacttggcataggcctggttggcgtaaaccttatggaaagcttttgaacgatcccgcgagcggttaaccaggtagttccatttgtccggattaccggccttgagttctttgactgcttggctattctgactgaccttgatggtgacgcccttgttcttatcggcttcaacggatggtttcttgccgtagggcgtcttatcttgggcattgaacagatactggttcagttcacgagccaccgttttatgacccgggccgtcctgtagggtgaatagactgccgacaaaataaatgacgagcgcggcagcaaccagtgagataaacttgccaaccggtttttggtaccacttcataaattgttcaacatctttattctgaacttcatcttcttcaagccatggctgcttggcgccacagtatggacaaaagtttgagtatgccgggatggttttcccacacatgacacaggacttagtcttttcttcagacatttctcatgctcctccaatatgtacctttgcgaatataccaattaattatagcaaagatttgcttggtgggaacaggtaagtgcaaaattatcgttaattaggcaggtgtttatcgatgaattcttttaccggtagacggaaatcgaggtaatatttctcaagatcctctctagaccaattccaccaggcaatttcttccatatcggttttaatttcgtcaagaaaacgatccttaattggtttggcagggatgccgccgacgatggtgtagggctccacgtctttggtcaccacggcgcctgagccaataacggcaccatcaccaactgttacgccagcttggatgatcacgccgtggccaatccagacatcgttgccgatggttgtccgcaggtgggttcttttttccaagaattcggtgtctggatggtcgaaaccgtaagccccgccgttataggcaaagatgtgttgggcaggccggtcgtagggatgattggtcggtccgattcgaatcatcgctgccatactgatgaactttttcaagtcactgttttgaataaaacaatattggccggtgtaagtataatcaccaattgaactattatcgattaaattgctgcttcctatttccacccattccccgaatgtagtattcttggtttgagtcatttttccaatcgttggtttatcttttgacaactttacaaaatcaatatgcatacgaccaacctctttctcaaaataatttctaaaaactattataatatgttttcacactatttagttaaaaggagcttacaaatgtttgaagtaaagactattgatcggtttgacctgaccgattttgctggagacgtctttcgtacctccaacaccgataccccggatgccattttagtgcggagttccaaggttgatgatagcttgatatccaagcgattgctgctgatcgcccgttccgggactgggacgaacacgattaacgtcgatgcggcaaccgccaacgggactgccgttttcaacacgccgggggttaacgccaacgccgtcaaagagctcattattcaaaaccttttcagatgtctgcgtccactgaatggtgccgttcaaatgatgcagcagctcaaagttgccccgggggaggatttgcaggccgctgccgaagccaaacggggcgattttattggtgaggaactttatggccggacacttggaattcttggcttgggaaccatcggccagcggttggcggacgcctgctaccacatggggatgcagattatcggctataaccgcagcttcaagaatctacgtcacgtccagcaattggataccattgatgaagtgttggagcaggccgattttgtggtgattttactcccgctgactgatcaaaccaaccagctgttgtctaccaagcaatttgaaatgatgaaggatagcgcttatctgctgaattttggtcgcggcgagattgtcgataatcaagcggtggtctcggccttgaatcacaacgagtttgccggttacgtgtgtgactttccgaaaacggaactccaggaccatccaaagattaccctgctgccacatttaggcggcaacacaattgaggcgctgacccattctgcgaacttgattttgcagaacctgctggactttttggaatatggcaccgtcagaagctcggtcaactttccccgggttgatttgccgttcatgagtaaccagcggctgacgtttttcttccacgccagagataccttctgggtggatgttgccggtattatgagtcgctatgacttgccggttcaagaaatgatgggaaacaccatggacggttatggctataccatcgtgaataccgatttggcggaaatcacgcagcaacaaacacagaccttgttaaatgaacttaatcagattgacgggatgattcgggtcaggttgttgaacaacccaacccagggagaatggcagtaaactttagtaagtgtttcacaaccttcgaacttttttgaaattatgagactgaaagtgggagtatgggtctcgtgatttgatgagctcgtttcacaaataaaaagcaaaagaagtattgaaattaattttcagccgcctataataagcattgtaagcggttgttagttgaaaaaagcaaatgattaattcacatattcgcactcatttaagcgctggataatcatttgcttttctgttgtttgcaattgctcactaaataacaaatatagtatttggagatgtgattatgcgaattaaagcagctgttgttaacaaaaaaggcggagacttcgaaatgaaggatgacgtcgaattagcagatatgcaagctgacgatttacaagttcatatggttgccagtgggatctgccattcagacgaagctttacgaaaaggaactgccgaaattggttacccaatcgttcttggccacgaaggatcaggaattgttgaaaaagtgggccctgaagtgaaagacttcaagcccggtgatcacgttgttctgtcattttatggctgtggcaactgtatcaactgtttaaagggaattccaacccaatgcttgaattacgcagcaaacaacttgtcgggggttcgtcctgacggcagtgcccactttactgaaaatggtcaccaagttgccgacatgtttgaccaatcctcattcacgacgaccactgttgtccgtgaacgtaacgcggttaaagttgataaggacttggatttgcgtcaattaggacctcttggctgtggctatgttacaggtagtggcacggtcttcaacactttgaagccggaaccaggttcaaccattgctgtctttggtactggagccgttggcttagctgcaatgatggccggccgaatttccggctgcaccaaagtcattgccgtagatatcgttcctgaccgcttgaagttggccaaggaattaggtgcgactgataccattaacagtaaagacactgatccggttaaagccattcaagatttgactgacggttacggtgttgactatgcggttgacaccactggtgttaaatctgtcatggaagcatcaatcaaggccttggcacaaggcggcacgactgcaacaatcgccgttaccgaccaacacgttgatctggatacttggaacgatctctgtgtcagcgaccgcaaagtcgttggtgtcaacatgggtgactcaattcctcaagtcgatatccctcgtttgatcaagttctacaagatgggattgtttgacttcgacaagactgagaagttctacaagttcgatgatattaaccaagctaacgctgattctgtcagtggcaagacgatcaagccagtactcgttattgacgaagattacaagccaggcaagtaacacgtttccacaaactcacatcaaggcatccaaaagtttcattaataaactaaaaatatttgttcctgccagatggcgttcaattacactgttttcgacaggtatcttgaaagggagcaactattatggcacaaaatgctgttgcattaaaacattatcaaatgtacattaacggaaaattcatggattcaaagtcaggtaacgaaattaccgttttaaacccatcaactggtgaaaagatttcgacagttccagctgcaactcgtgaagaagctaaagaagccatcgatgctgcatacgaagctgaaaaatcatggaagaaagttccagctgctacccgtggccaatatttacacgatgttgccactgaaattcgtaacgagaaggatcacttggttgaaatgctccaagaagagcaaggtaaaatcaagtcattggcaaccactgaaattatgttctcagccgactacttcgattacatgggcagtgctgcgcgaacttatgaaggtgaaattctccaatcagacaacaagaatgaaaatatcatgattgctaagcagccaattggtgttgctgccggcatcttaccatggaacttcccattcttcctgattgcccgtaaaatgggtccagctttggtaactggtaacacgatcgtgatgaagccatcttcagacacgccaaacttgggacttgaatttgccaagattgttgaaaaagttgggattccaaagggtgttgtcaacattatttccggtcgtggttctgtggttggtgacgaactcaccaagaacaagaagattggcatcattagtttgactggttctgttgattctggtaaacgggtcatggcaggtgctgcaacccacatggctaaagtttcattggaattaggtggtaaagcaccagccattgtctgcaaagatgctgacatcgatttggcagttcaatcaatcattgactcacgtgttgataacaatggtgaactctgcaacaactgtgaacgggtatacgttcaagaggatgttgccgatgagttcatcaagaagttatccgacaagatgtcaaagatcactgtcggtaacgttatgaaagatgaaaacgttggtatgggtccattgattaaccaagaagctttggacaaagtttccggaatggtagatcgggctgttcaagctggcggtaaggtcacagccggtggtcacaagttgaacatcgaaaatggcttctactacgaaccaacggttatcaccaacgtcaaacaagattcagaaattgtgcaagacgaaatctttggcccagtactgccagtattgacctttaagactttggacgatgccattgaaatggctaatgattctgacttcggtctgacttcatcaatctacaccgagaacttggacaacgcaatgcgtgctgccaacgaactcgaagacggtgaaacttacatcaaccgatttaactttgaagctatgaatggttcacactcaggctggaaagaatcaggtatcggcggcgatgatggtcgtcatggtatcgaagaattcttgaatactcatgttatttacctgcaagggcatccggagaaggcgcaaggttagagtgcgactaggcccggttaaccgcggcgtataagccgaaaggacggattgatgaacgattcttgttcattgattcgtccttttggtttatacgttaggggttgggccatcggagcacattttatccaaataacagtgaacctatcacttaccaatgaaaaaaggcacccacagcaaacgcacaagaaagtttgtccgtggatgctttttatgtatgactaaaatatctgaaatcccaacgaatattaaccgatgtgataaatagaaaaaatgacacacccacgccatcccggcatataataaagccaacaaactcacaggggggcagacacaatgacaccatccaatatcatcggcgggatactaacatgtggcgttggcctgtttttgatcgtcgcaggcttaatggtgagcaagggaaaatggtcaaggatggttgctgggaatcttttccacgatgatcaaaagtcggttggtcggcataagaaagccatcgggggtttatttatcattctcggcggtttgtgcctggtcttttatttggtgcttttttaaacacctggatgactgacagaagatgtgtcgtttcgtataatgtatcagcatgagattcaatgtgagacgttgtaattgagaagggaggattccatgacaaaatatacggcgacaatttcgaaaaatggacaattagttattccagcgccggtgaggcataaactgaatatttccgctggtacaaagttatccattcaaattgatcaaaataataacgtggttctttcaaaagtaccggaggtgtccgactggaagaaactattggctaatattccagatgagcgggttgagcttgatcaagaaggacattatgatccggacaaatccccagagcttgatgactggatgcggaaaggctaggccagatgactaacgcaattctttcccatatctgtttagctgatatcccttatgatgacggacatcttgtaaaatctcaatgagggttgttaattttgccaggaaaagatacctcaagagtctttaagattacgtggattgtagtcaatacgtgagacaattttcggaatttcatcaatatcccatcaaaatagcggcctgcactggtctcaaccaagtgcaagccgctatattatacatacagtaaagattgaatcattgaaccaggtaaaagacgccactaaccccaatcaacacaaacacgcatttttgaatcatcgagatattcatatggaccgtaatgcggttggcaatcatggttccgatgacgccaccgactattcccaatagaatgagggggacgtcatttaaacctaaaataccgttatagaaacgaatacttgttatatacaattgatcaatcaagaagaaagcttgaatactggcgagatattcctcttttgtatccgccaaggacagaaaataaagtgccgtcaacggcccgccaattccaaacaacccattgaagaagccggaaacgatcataaagataatggcaatataaatgggataatgtttccggccttctgatttaacgaataaaaagtacagtgagagggcaaccaacagaccacccagcatggatttcagcaaatggacattgattgagttgactagttgtaatgccatgaaggccacactggcatagacgacaaacggccagatgattcgtttgaatttgatgctgtgccggtaacgccaagccaacatgatgttggaaacggacataatgagggatgccactccggcactttgggggatgggcaagattgtcggcaaaaagaccatcaagacaattgctgagccaaacccggtaactccctggacaatcccggcaagaacggcgggcaggagcacgaatatgaaattagtcatgaccatcctcctctcaagtcatctccgttacgagacgtgtgataagttactctgagacttccggtgaagttttggtgactgtttggtgtaaagttttctggacataaagagcgcgacgaccaagaaggctaaacacatcgtaaagccggcttgaatgcccatctgttggtaattggcgtggccagcaaaaaagtgactggcaatgttgatggtggccacaataatggccgttccaaacgatgccgcgatttgccgcaaggtgttgaaggcggcaacaccgtcggcaatcaattcattgggcagataggatagtgcttgggtctgaattggaatgagaatcaagaccagcccaagctggcgaattgtctgtcccattgtcagcatcaacaccgaagcgttaacatcaatgaatgcctgcatcatggtaccaaaacaatcgattagaataccggtggtcacaatgatccgtaccggatagcgatcgaacagccggccactgattggtgacataaaaccagttaatagcgctcccggcagtaatgagagaccggagatgatggcacttttacccataatcgtttgaatcaacagcggcaacagaatcgtattgccatacatcgtcgagacaatcagtgagttgaccaaagtggcagtggtgaactgactatttttgaagaccgccaaattaacaaacggatggtcggattttccttgagtgacggcaaacatcgtgattaagacaacgccgaccacgaatggcagccagactgttagagatgtgatagggaactggctcacgtttgaaaaactccatagaagtcccagcaaaccaaagctgatggtcatcaacccctcggtgttaaattgaggttcctggttagtggggatcttgggcagggcaatcgtggccattaccaaatcaatgacgataaacggcagcaccaaaatgaataggtagcgccatgagaaatagttcaaaataaccccggaaagtgttgggccaatgatcggcgaaaagttaaacgctaagccgacgatccccatcacggcaccctttttgccgggcttggcgtagcggattgccagggtatttaccagcggcatcatcattccggcaccgattgcttggatcatgcggccaatgatgagggtgaagaaattaggtgccaaggcaccaaaaatcgttccaactaaaaagacgctgacgaaaaaaataaacagagaacgaaatgtgaacttcttggtcagataagcactgaccggaatcataatcgcgttgaccagggtgtagccgttgctaatccattgaaccgtaccggacgaaatggcgaacaccttcataaaggttggcaaagcgacgttcatgagcgttgaacagagaatgccgaagaaggcaccgaagatcataataatgagagaatagcgattttgctttgacattaacaggacttccaaatatgtattttataagttttgaaaaatagcaactctaaatagtgtaattttaataatggataattgcaataggaatatagttaatcactaatcgcagaataaataaaaacgtggaattgtaatcatgcaattccacgcttttattaagctttcttagatacccgataaaagttcggtgaaaatggcgtttctgccgcaatgttactaccgtcataatacacgtgaacgtatccgtgaccaactcgtttgaacgtgaatcgggcttggtgcagtttgttcagttcgtttctgccgacgatggtgtaggcggttttaccgtctgctttccatttggtatcggtaatgtgccagcctgctgactgcgttaaataggcattcacactacttttacgaactcggacagattcatagctatcaaacttcttcatgccaaagtatttaccaatgttaatcgtcttgtctttccagtgaccacggagtgctgttggcgttcccttgtgccaggttgccgcttgtgttgatgtcgttactgctcccaaaaagccaagtgacgcaatcgccgttacgattaactgcgtgcctttgttcatgactgtcatctccaattaatttgcttggtcaaatttattaaccaattgaatgaccatgcttggctcactaccggggactgcccgatagacgacgtagtctcccggaaccagatcaacggatgccagttgggctttttgggcgacgctaaagccagccacttcgtagtaggcgtgaccgtcgacgtcctcgtcggttaacgtgacgttgacttgttccagtggagcaacatctaaggatgcccggcgtaatgccaagtactggtagttgatcgagtcaaccataatggtgatttcattgttggtgcagggaacgctcatggtctgtttcaaattgatttacttccttctttgagtttcgcgtggcgaatatcattgacattgatggtcaccaacttgtcggtttgaagatagattagatcaccattagtgccaattacaatgccacttatattataaacgtttaagtagccgtcatcatttaattgaagtgtaatttgtttggaattctgccaactgtcctgcaaaacgcggtcgatgacttccggatcctgttccggcaatcgatgagtcgggacctcgtcgacttttttgtcagccatatcctgggtatggtcactcaaaaagtaacccagccacttcaccatgccgcggtcgttgtagagccattggtcacgtggaacgtctcgaatcatgttgaacacccccatacgtttaatatacgaacatatgttctaaacgtcaagggggaacagttcaaacaactgaaacttagggctgaagtaattgccagacttgggattgggaaaatgttacagtttatttggctaattcacaatttattcatatttttagaggacaatgaatttataaaatacattgaataggagtgaagcaattgcgcacggtctatattttcaccatcattattgcgtcgatcgccatgtttttgattgattactatgtgtcattaccacatgtgttgcgggcttgtacctggttgggattcattgtaatcgttggaatttgcagttatcaaataatggctcattggcataataatcaataaaattaaattcgaatttgcttctcatctgtcgagatcgggaaacccttcttaaacgcagtccgcaagaagttaagcaggggcggagtcacctttaattcgtccaaatcccgcaatgagaaggtatagcgaattgccttttcatcaccagcttcaactttttgaacccatttgggctcacggatcaactcacggcccatggcggcaaattggacgccggcgtcaatcaacttggcgacttgggcaggggatgccaaatggccgacaaccatcaatggtaaatcatctgcgaggactgcttggactttttcgaagagcggctgctggtcatcacgatcgacaatcgatccctgccaagcatctgccaatgacatgtggagataatcaattggcttttgattgagttctttcaccaaggccagggtgtcggctattctgataccaggcttttccagttcctcaggcgaaatccggtagcccaagataaactgcgggttatcagaatgtttgataacggctgcgcatgcatctacaaccgccaaagggaagttcatccgtttttccaaggagccgccccagtggtctgttctgcggttggaatggggactgaagaattgctgaatcaaataggtgttggcaccgtggagttcgacgccatcaaaaccggcgtcaatggccaattgagtggcgttggcgaagtcctgaatggtctgctcaacttcttcagcggaaagggcccgggggggttcggcacccaaacgttgtggagcgaccgcgctggcagagacggtttgatggccgcgcagtacccgcgagttactcattcgaccggcgctgaagatttgaagaattgctttggtatgattgattttgatggcgttggcaagccgtgataacccgggcagcatgttgtcatgtgcgacgctgagctcgccttcgaaacctttgcccagatcattgacgttggcacagccggtaataatcatgccgggaccaccggcacgcaatcggaagtagtcgatttcgtctccggtgatcgaaccgtcttcaaaactggacatctcggtcatcggcgacattgcgatgcgatttttgatggtgacaccgtttcttaattgggttggttgtaggaaattatattttgtcatatgagacctcctgatgatgattaatactttgagtgtaccaaacaaacctaaaatttccaggtgaaaatgtttggttcattttcctaaaaaagcgtttacaatagaagtggaaacaaaattggaggagtgatagttgatggaaacattgaaaatgattcagtcacgtaaagcagttcgtgagtattcgggccaagtatccgatgatcagctgcacgaaattttggttgcagccaacgccagtccggttgggatggggcgctatgatgattatcgattgacggtgatccaagatccaactgttttgtcaaaaatgactggcatttatgaagccccaacggtgattgtggtttcagttaaggaagaaagtgcctccgatgagatttcagccggtgcgattgttcacaacatggaattggccgctgaagatcagggattaggtgccaactataatatggccagtttggaatccattccaagcggagtcgttccagatggttttaagccggcatttgccttgacccttggccagaccaacgatacattcacaccacgggaaattccgttggatcggattaagacaaatactgtgaaatgatattcaaaaaaatgggttagctctcaacgatttgttgggtgctaatccatttttgatttgacagttaaaatgtggattctttatctgacgaattgcgggtcgtggaccggttataattccccgcctttttcaaaggttggtaccatcttttcagctcgcagcaacagcaattgatgcagcaaatccttcacgttctcagtaattgcgtgagcgatcttgtcgttaacctgattatgccactcaggtaacttgtccttggcaatgtttttaaattctgcatctgcagtcgccactgcagcccggccgttggcaaagccaaacttgcggctttcagaaactgcagtcattgcttcgagatcgtgttcggcaaagaaggggtcagccaacatggcgaccaacttattcagccaatagaagctttctgtcgtggtccgcagcggcgtgtgcttaaagttatccggggtatccgtgcagttggcaaagaatggcaccggcgcattgaactcgttgaccccttcagccagccaatgaatggcggcgtgttctgctggaaaatcgggacgaatttgcaggatatgcatctcttggttgcggttcattccaattggtcgatagcgcaaccgtgattcttcagtaccggttttcccataaggatcaaaatcagtgccttgatagtggctgctcaagaagaaggcaatgtcttcaactgaaatcaaatgatcggcaactctggtaaatggcattgtccgactttctggatcctggtggatttccgggttaaacattttttggccataccaaacccgcggggtgttgtagtagtgatccgcttgaacgtcctcaccgaaaatatcacggaagttaaagccggaacgggccttgttcaagtgatatttatcggcaaatgctttcagatcgtcgctgtacatgaagtggtcaggatcatcaaagttgatttcttgaatgccggtttgattaggtgcgaccgcataggcatcatccggaattcgttcggcagcccaatggtgcccaccgactgtttcgaagtaccagacctcatctgaatctgaaaaggcgatgccgttgctttcacaagtgccaaatttggtgaccaaatcgcccaagcgttgaacgcctgcacgagcgctgtggatgtaagggaggacacaagtcagcatggcctcttcaccgataccgtcagccaccagcgggtccaatcccagcatggtggtgttggtaaattcggtttcagttgagctcatggcaacgttgtcggagttaatgccggattcgccccagaggccatcactaacgtcagcgttgggtgtttcggtgtagcgcagcggattgtttgggagcttaacccgaaattggttaaaagtcaaaacgtattcgctgggttgatctgtcgggttcaccaccacaaagcgcttggcattcacgcctccgccggcatcttcatttctggcaatcatcgtcgatccgtcagttgtagcattctttccagctaaaaatgcggtacagctggaagtcgtttgaaatttattcaatcaaatcattccttcttaatttaatacatcgattcgattcggaagcggtgcttggtgcagtggaaactttagtaactcaaagccagttggttggtgattgatttaggaagtaccagtgcttggccgtaaatccaatatttttgaactttggtgtgtttggtggccttcttggttgagtatttggtgatccggtaccagttgaactgcaatccctggttggcgtacaaatcaacgtggactttggtgccagcctttaagccgctcttcttccatgaagtggtcttaatgtttttatagctgctgttgggggcgtgattagtgagcttaaatgatttgtagttggtgccgattttggcattaaaattagctttgtgataactcaaggatccgggcatgctggcagcgcttgaaacgggggattgagtgacagatacgaaaccaccaaggcccagggctgttaccgccaacaagatacttttcttaaacatctaaaaaatctcctttcaaaattcaactaattttagtataaaagtctggttaaaaaaattccagccgactagctggaattttagtgattagcctaagaacttacgcaagattgcctgacgactgattaaggtggtcttggtttctttatcagaaatcttaaccagatcagcggctagttgggcatgcttctcttgttcaggtgtctgtgggccggcctgaataccgaatagtcgttcaactgcttcaatatcttcgtcaaccgctttccaggcagggttcttggcttgaagagcatccaaggcgtccttgctgaagtatttggcaacgtgggcataatcgtgtttgatatttggatagtatttcattaaggtgttcaattctttgtcgcttagcttgttcaagatgcggccagttccaagaaattctggcggaaccccaactgagtacagggcaccggtaaaggtgatcgcccgaggcatcttatagccatcgacgtcacgtgagtaaccgatgattccgacgtgttggtgacggtcccgacgctttggaaaggcatcaaataccggctgtaagtcgttaatgagtggatccaaagtttcgtgatattctgcagcggcttttttagcgatttccaagagaatgtcttggtcgtcgtgatcgataatttcaaatttgctcttttgaaggccgtcgcgcagtttgatgatcgctggttcaaccacatccagcgggtaatcgtaacggaatgccgattgaatcgttgccgtcttcaaaccggggaattcttcgaggtaacggtcaatcatcattggtgataggccgccacggaagatggtgcttccggttccggcaattggatagattggcaggccggattcttgttcaaattcggccaaaccggtcaaggctaatttgttaccaatgatactgttcaagaaaccgtttgaaagagcggaatcggatccggccaagaagacccgcatatagcttaattcacggccaaagtggtctttgtacatttcaaggtattttttcaggatttgtggggcgtgtaactgggattcgaatccttcaaacaatggaatcatttgcagagtatctgaatctttgtgcccggtattaaattcagttgacttgtagtgggaaaggctggcgaacttgtcttccatggaaatcagctggtcggctgattgggtcatgggcaagatagcttcgaataacggtcgttccttaaaccccaaatcgtaagcaaagtcttcagcggacaagatggtggtcattgcctgcatcaaactgtagcccttttcttcccaaatgtttggcagacggaaagtgaggtacttatctttgccaaggggatgcttttggaaatattcgtagtgctcggagtacaaacggtcaatgacggatgcatcggcgtgtttgccttcccagtcccacatatactcatcggcatcgagcttggaaaagttttggtaagcttcatcaatttcacgaaatgcggatacaaatgcattatcgttgtgcttgaagaatggaactcctgcgttatctggatgttgagtacccataatattagggatttttctatccataaaagaaagcctcctgagatttgattaagttcatttagaatgattatacagtaaaaaatgtgaacatgaaaataatattagcaaattgtgcaaattcataaaacaattaaatacccgaatattattgaataatttaaacagttaattaattatttcaactaaatattacagcttatttgaaaacattaccagctttttagatgagattgagaacattatcgcaatcaaagaggttgggacattaattgttacgctggctttcattgcaaccttcattaccacttttatatagataaaacttgcaacaaacggctgatcccggccatttaacgaataaacgcagtcattccaaagtccggaataactgcgtttattcgttaaattctgggatcaaatcgcctttcgtcccaatctctttgggttaatcaaagctcgtaactgtttcagcggtgtagttcccgctgttcttaagtaattttgaaactgggcagcggttttcagcttcttgtgcaaattggtcagcggtttcaaagtcaacacctttgaccatgatctgagcgtgaactaagaattggtattcagcccgctcaccaatgtaagccactttgacgtggacctcggcggtgtgggggacaccatgttctctttcaacggcttgaagggtggcttccaaacaggtggccaaagacatgcccaaaagttgttccgggttggtacccggctttgaatttaatgggctgctggtttccactttgatgccgtctgggacataagcatggccgttcagaccttcatcattcacagcttcggtttgatacaacgggttattccatctttcgtcttgcattctggcagtacctcctacgtttctttaaccttgattataagcgctttcaatgaaattaaaaagaaaaaggttggtatcaaaaaaagagtgggactaaaggcgttttgatcccagaatttaagagcacagatcgattattcttggttttggaatgattgatctgtgctcttaaattctgggatcagccgattgccatgtaggctaggcaagcatgctggccgtcgtcgcacgtttttgataaataatatgggatcacaaaaaaagaggccaaggcaaaagcgtatacttttgtcccagcctcttgagccgttattcgttataatccattcgaatgatcacaggatctttagtcaaaaagtcgccaaccccggctaaaaatttttggaaatggggcgtattgttgtggaattcaacagctttttcatcctgccaatgttcaataatttcatactcagtgtcactatggagcttcttgaaatggtcgtagctgacgttgcctgcttcgccacgggagccatcgaccaattcatcaataaatgcttcgtagtccgattgcatccctggtttaactgacaattcaacgttgataactttcatctttgcagcctcctatcaaatgtttgggcatgtacacccttagtatatcgaagttttgaacttattgttcaatttatcatccgtaaatgtgagatcgtacgccgtcccttttttgtcagtgacatagagtaagtatttggctgacatcggtccctggccgataatcgactggccgtttggtgtgcccaacgcattaatcgcagcttgatatgtagttccaagacccaactggttaatttttgatttggcagtgattcgctgcttgcgcttggcagctggcgtataggatttcccgacagctttgtgattgagaaactgtactttgaccttggcaaccgggaaagtcgcagaaacatccttccaggtatactgggttgtcttcttggtgacgccgttgacgttgaccgtatcaacgtgggaaggagtcccgaagagtttgaggacttggtcttctgaggaaccataggcagcatcggtaatgtcgccaatattaatccgattaaaattagccagattgatcccttcagcttctcggtcgtgcttgtattcagcggcggttttttgactgtcaaagtgatgattaacctgttttttggctgaattcgaagtgccgcacgctgatagcaacagcgtgctcattaatgcgagtgtaacagtaattggttttcccataaaattccccctgacaagatggttctaaatgttggctggattgacaacattatatacttatttgggcggcgagtcgtggactttttaaccgtcgcggccagttttcgaatataatgaacatacaaagttctcaatgaaagacaggtgaatcaattggcaaatcaaccgttagtatttgattatcaagctgctcaaggcaagccggagaatattcgccatccggaagggtactgcccgttttgtgatgttgagcatttgaccaacattttggcacgggacgacgatcgcatttggctggtcaataagtttcggactcttgaagatacctttcagactgtggtgatcgaatccagtgaccatcttggcggaccctccacttattcagttgagcagaatcggcaagtgttcgaatttgcatttaaatgttggcaccaaatgattgtgtccaataaatatcaaagcacgattatgtacaagaactatggcccgttatccggcggcagtttacgacatccacattttcaaattgtcggattggataattatgatgtttatcaaaatgttgatatcagtaattttaccggagttgaagtgattcatgatgagcgctgtgaaatcacattatccacgcagccgattattgggtttgtcgaaatcaatattgccatcgaagaggtcggtcatattaacgacttggccgatgctgtccaagtgatcgtcaaatacttgttgaacgattacatgggtggccgactgtcatcgtacaacttatttttctacgaaatggccgataaattttactgcaaaattgtcccacgttatgcgacctcaccatattttgtcggctataaaattgcccaagtccaaaatgagggccgactggaaaaaattgcggcagatatttcagaacgtctgtcggctaatcaataacaataaagggaacggcatcttgccgttccctttattgttattgaaattggttaaaccgcactgactaatggaactgatggatcgtcattaacgacagtcacacgggtatcctgggctaatgcctgcttaatcatctggttgattttagtataaacctttggatccgcagccttgatttcattacgggaagccacgaataggtgacgaatctctctggactttaagagattttcaatattctggaagtcggtgaatagttggtccttaaatatcttggtaatggcttcagctgtgttttcacggttgtacgtgtcaatcgccgtgtttaccaatttggcaatctcagtagtggtgtcattttgaacggattgatccacctcgaagtcggctagttgtaagccattattgactttcttgaataggttaatattttgagataggcccatcaggacgaattgatgttgtgccaattccacgtttcccttcaggaaatccattatgacccggtagtaacgttcctggtcgattttcttttcctgggtggtttcgttatgaccgtgatattgggcattgccgccgcgggcactaaagttcagttcaccgccacgcaattcctcaccgagggcttctttaacattggctggatactctttgacatcaagtgcggtgactcgcttgttggaaagttgatagagtttactgttgtcacggtttaattcgatcaatgtgtaatcctgattaggtgcttcactgagtaataacaggaagtcaattgcatcttcaattcgatagtccggctcatcgacactggttcggatcaaatgataaacatttttgctaaggtgatcggcaatcacggtcatgccttcataaggcagctgctcacgggtcaggtcattgacatcagcaataaatggcgcaatatcgtctacgacttctttttggatttttttcagcatattcttaactcggagttgttcactttggtcaaacgacagcttacgcaagttaagattcaaagtaatcaccggtgcttgtaagtcaggtaacttcgccaaatctgaaacagaaataatagttgccataagtaggacactccttcattttttatattaggtataactatttaattatataacctacttctattataacagatccaggatccaaagtcttattcggcgatttgataaaaaaagcaatcctcatgggttcaaggattgccgtattggagattcgtaataattgagattaagccgccaaaaagagtgaaaagtagacttaatactgccagggcgacgaagagttggcgccatttgaaaggtgccggctggccgcgggcatttttatagatgagataaaaggcaccaacgacgatggtaaacaccgctgtggccagtaaaatccagacaactgctaaaacaatatccatgatagcctccgtcaataatgatacttgtaaagatagcattcacaactggcaatggcaacctggggatgatcattacgtttttctaaaaccgattatgatcgcttaaggtttaagtttcagttaaccacgcctttctagaatgaatttaacaaatgaaatttagtcacgaatttgctcgaagaaaggtgggagacgatgattaaatggttgccatatttattaaatattactggtgtattggtctggttgaagattcaatcaaggaacttgaggcaattgacctggtgccaactgttcacaattgtcacttcaatcatctatattttggttgtgagctatcttaccttggcgccgacatcatacgcgttcgtgggaccccaacaagtctcaccgatgatgatcggttcggcacccattaatttgatcccattttggagtaccactgctgatttttatcaaaatgtggtgatgatgctgccgatgggcgtgtatttgggattgctgctgccaaagttcaatctgcgaaaagtcttattgaccgggttgggtgtcagcttgaccattgaaagcctgcagtttgttttggatctgtcggtcgggctgtccagatgggtcgatattaacgacgtgttgaccaacacgtttggcgtgatcgtcggctggctcattttgaaaggcttgatgcacacgatctttcagcgactcttgagtcattttgcgattacagcattttcacaccaaaagggtaaatgattgccctttcaggagtgaggcactaaaataagcttactttaaattaatgggagatgttatgatggctaaattgaaccaggcaatgaaagacatgattgccggagaattatcgtatatttcaactgttgatgcagatggcaatccagatgttggacccaagatttcgatgcgggttctggatgatgagcatctgatttataacgaaatgaccggcggccaaacccaagcaaacatcaataataacggcaaagcaattgtggccgttgccaacgccaaggcattaaaaggattccggttcggtggaacggcgaaactctacacggacggtgactactttgatcaagctgccaaatgggcagaaggtaagttcccagctccaaagggtgccggtgtgattaccattgaaaagatttggacattggatccaggccctaaggcagggaagatatttgaagaatagtgcgctactttactcttaaataataaataaaaccagcaatgatgattatttcatcgttgctggtttttgtgtttcaaggttacgtgcaaacaaagactattatgcttgttattacgagtcaggcttgataactgatactttctgagaaacttgatccatcagaaactgtatctaaagattttgaatcgtcagactcatctgtaatgatcttaatacttttgggcttcagtgtcgtagtggactcagataataagactaagtcatattccacccgcttggcattgggagccaactcttcttcagaacctgtatcagccatcgcatcgtcatcgaagtttatttgataaccgttggaaaatacaatttgcttgattccgccaaagtcaatcgttgttgtggaatgattggtaacaacatactcaattttcattcgcgtgtagtctttaggcatactatctttgttaaacgaagtcagtgcctgatcaagctgatcttctgtatttgcatgaactttgtcgatctcagcgtgtttaaatttaacagaaagcggcccattttggattgtcgtatccggtttagttcctaatccggtcatggaaatttttcctagaacttcgctatttttccactgaccaacttttgacagatggataagagggtttgaagagacttggtttggatcctttttcttagccttcgctttggtcttagcggtcttcgaactcgctgcaggccgcatgacaaccgttgttttcgcgctgttcaacagggcaatacaagttaccaggccaacccccaatacgataatggcccaaatcatccaattcttgtaccaaagctgcctttttgattcggccacatcagtccgttgctttgaagcgtctgatggcataggtgattgactggctaaaccgacttgtggtttgccacagtatggacaatacgatgcagcaaatggaatctctttgccgcaacttaaacagaactttgtttcttgattcatgataatcccccaaaatatgtattcagctttttgcgtcgtcagttttggacaaaatgactcaggagcatgactggatgctcctgagttttcaagtgcattcagctggtcgttgaaagtgccatttaactatacccaaaccgcaatacccacgtcaactattttttgacgattatttaatggtttgatagccggaaagttatattcttatctcttgggaatccttttataatagccgattaaccgttttcaatcaaaaagtcgttttaattgtattttcgattgcacaaaactaatatgatgttaatcagtaattggttacttattttacagggaggttttaattatggctgaaacaattaattcggggattgctgcattacacacacttgagagctggggtgttgatcacatctacgggatcccaggcggaaccattaacaatttaatgtatgcattagatgctgaaaaagacaaaatcacttatgttcacgttcgtcatgaagaagtgggtgccttggctgccgttgccgattcgaaactaaccggtcacatcggggttgcctttggctcagccggccctggtgctactcacttgtatcaaggggcttatgacgcaatggctgacaaagttccggttctcttgattgttggtcaaaatccacaagctctgatgaaccaggacttcttccaggaattcgatgagaacccatggtttaaggatgccggggtttatgctcgaaccgtcatgaccgctcaaagtctgccccacatcttagacgaagccattcgtcgggcgtttgcgcaacacggtccagccatcgtcacgattccaaatgatttggccaataaggaaattccagcagatggctattatagttccgctgccaattttgccaaaccagaactaggtaccggttcagacgagcaggtccaacaagcattggacttgattgatcaggctaaaaagccagtcctgtacgtcggccagggaacttacggcgctgccgatgaggtaatggaatttgccaagaagttccaaattccagtgatcacgaccgcactgggcaaggaaattatcccttatgactttgaatccttactgggttccgctgcccgggttgcttccaagccagccaacgaggcgttacagcaaactgatttgatgctgtttgtcggctccaactatccgtttgctgaagcgatgttcaaaccggacgttaaattcattcaaattgataacaatccacaagtgcttggcaaacgtcacaagacggacgttgccattcttgcagatgccaagaagacattacagaaattcatcgatatgggtcaaactaaagagccatcagattggtacgcagccaacgttgataacgtcacaaattggcacgaatacaatgaccatatgatgaaccggacggaaggcaagctgcgtttcgaaccagcatttaaagaaatcaatcggatcgctgaaaaagatgccatcttctccattgatgttggtgatgtcacccaaaacgctgttcgtttgttaaagaccaacggccatcagccttggattacttccggattatttgccactatgggcgttggcttaccggggtcaattgctgctaagttgagctacccagatcgtcaagtattcaacctgaccggtgatggtgccgcagctatggtgatgcaggacctgagcacccaagttggctacaagctgccagtgatcaacgtcgtcttttctaacgaagcgctgggcttcattgaagatgagcaagaggatgacagtcatgagtggttcggaattagtttgccgcagaccgatttcgccaaggtcgccgaagctcaagggatgcttggaatcacggtgacatccgttgatcaaatgaagccggcttttgataaggccgttgaagagaccaaggccggcaaaccggtgctgatcgatgtcaagattaccaacgagcgtccgattccagttgaaaaattgactttggatccggataaattcgatcaaaagacgattgacgacttcaagaaacgttactacgcagaagacttggttccgttgagtgccttcttgaaacaacacggagttaaataaatcgttctatagctaagtgagaggctaaagcatcagtgtcaattgatgttttagcctcttttgtgtgtcattttgatactgattaaatatgctggagatgactgttttcattcacaaaagattaaaaggcctcaatcatgcaagccggataccattgaattataattaattgtatataaataaggggagtcaaagattatgggaaaatggaaaagtgcactcttagtgctgactggattcgtaactttgggggcggtttcaacgacagcttcggccaaggcaaagcagaccccggtgacggtgaatgttgtctttaatgttcgcgaccgtaatgcaatgaatacttatgttagccaaacggtagatccaacatcggctaattatcatcaatacttaacaccacaacaggtggctgaccgttttggccgaaccaacgccgaaatttctgattttaacaagtacttcagtcaatatcacctcaaatcggcggcttatcctggcaactttgtgatgaaagtccagggatctcaaaagaatctggtgaaggcctttaaggcgaccccagccaagaccaacaaggactgggacgtgaccggcactaaattgcctggtaagctgtccagtcaagtcgcgtcagtcctgggattgtttgttgacaataaaaagacttcgacgaaaaccgataagaaggcgttaaagtttacccacaacttaattgaagacgacacgccaattgtcgccagcagtcaaaatcagctggcgaagaaatatggtccgactaaatttgccgatcgatatggcgttaacaagctgtacgaccagaatctgcatggggccggccaacgtattggggtaattgtgacttacgacttcaacccaagtgatgttgccgactactggaaacaaatgggggtcaacagcgacgtttccagaattcacaagatctacaccaccgataatactggtgggccaaagccaaagaacaatgatgatgtgacctcccaggaagaagccagtttggatgttgaacaagctggaggagttgctgatcaagcacaaattgacgcttatgtcggggtttccagcaacggagacaccacgccggatgttcaatatttggacgcatttgccactgcgattggtgataaccgtgacaaacaattgacgaccagttcgtcctttggtaatgaattgaatggcttcggtcgtggcgggctaagtgaaacagcttcagaattcaatgatgccatcaacctggtttttgaacaggcagccattcaaggaacgaccatttttaacgctgccggtgacagtggaccgtatgaagtcgcaaataagtccaccaacttgccattcccaacatcggaatatgccgttcaagtgggcggaacgacgttgccttataccaaaattattggcggccaattgattcaagttaaaaaagagcgcgcctggggtgattcctattcacaaggtacggttaccaagccaactgtcttccctggtggcggtggtggtttttcaactctcaatccaacccctgcttatcagcttggtgttccgggcgtcaacacttacaacgcatttaacatgttgaaatataccaagggtggttacttggtcaacccagatcctgaaatgatttctgggactcatcagggacgaaatgtaccggacatttccgggaacgctgatgaaaaaactggttatggcgtatacattacttataaagccgggaatacccaggttcccatctggatgaatgcaggcggaaccagctttgttgccccacaaatggctggcgccagtgctgttatcaacagtggtttaaagacttctgccggattctggaacccacagctgtataagtttgctgttcaatccgacacaccgttccatgttttagatgacgcgacgatggagaataccaatctgtactataccggccagccgggcaaggtttataaccaagcaactggtctgggaaccgtcgacttcagtaaactgtttacgaagtttaatgctcagcaataaagcaaattgaaaaacaggacccccaacacgctatcatctcgcatgttggggatcctgttttttggatatttggctaaaaagtctgtttatttaatgctataggtttgtactccgatgatttggttggtgccggctttcacgccgtggatcttgattggggatttggtatcatacagattccaggccattgagcctttggctgattgatttttcttgatagccaccttgtatttgggagctaaatcttgatccggaagtggggcggcgaccaactgctttttggatttagcaggctggtaggcgcggagcacggaagcggcagacactggtgaaactttatgaatgcctgtgtttttaatggtgtaccaaagggcaaaaatgggtttcttgccaaattcattaccagtctcaccagctggaatcacagcggttttggtaattttcagctggaaattcttaacttgaagaaagttcttccgaaaacttggtgtgtctgaagaacttttattctgaccgctacaccctgagagggagatgacggcgattaaggtcaatgcgagtgcgaatatttttttcatgttctgagctccaatgcttatgtatttatgaaaatgatgatttattaatattttacatgtttttttcaataaagaaactcaaaatgaggaaagttgacgttggataaaatgatggcagataaaaagcaacgccatgaatgacgctgctggatgatttgatgcgattatttgttgattggttttccgaggacaatccctgggtattggtcaacggcttcttgatgatgtttgtcgaaatagaagatgccaattggctatctctccaaaagcttactgatttgaattatctaacgctcgtagttcagacataatctgcatgagcttggcatgatagatgtctgatctcaacgcgtcgttctgctgactgaaccagtactgcttggcaggggcaacgtaggtttccggcacctgatacttgtcagcaatctgctggaaagtcgttgggttgtcggctgcctgctgcaggcgatagagcggttcttcctggatgattttgacaacttgtggacggacctcttccggcagcttgggttccacaaccttcacgaccgtattcttaatgggtttatccaaaattgtattggtttgccgctgagcgtcggttaattcgtgaacctgatgaccaacgtaaagaaaaccgactaggacaatcaccaagacgcttaaccaaacaattaacttggtgtgcttagtttttttctgttcctgtttggattgcttctgctgcaatcgtgatggtgtttgattttgcatgttgaatccccctcaaacaatttacgatacgattataacatttttaatcatgattcaatctgggaaggaaaccaggcatgcgaatttaaaagttccttaaaacaaaaaaatggcaagcagcttcgaccttctgaacgcatacgcgccgatcgttacttacttaccgtggtttggcaccaaaatcgattatagcatggctgacttggcagatgcaagcaaatctatgaacgggggctctgatttcgacaaatgcaactgtttgctcgattgaggtataaccacagtgccagataatgtataatcgtttttgataaatttttttgacgggggggaacacatgaaatcacttaaagtgcaaagcttcattctcatttcaattggatttattctagggatgagcgagtttattattgttggaatcatcaatgatttggccgattcttttgacgtgggcatttccaacgtcggcttcttggtgacgatgtttgcgattgtctatgccattgtgacgccaattttaaccatcttggtgggcgagcatcgactcaagcgggtgatgttgctgttgttgagtgtcttcacaatctccaatgtcatgacggctctggccaactcattctttattctgtccttgtcccgagtgctgaatgcagtggttgccgggataactgtttcaattgcgattacctttgcggcagtcattgccccacgagataaacgggcctggttgatttcttgggtcttttcggggtacagtgtcgcctcggttttcggagtaccgattgggacttggattagtgatcaggtcggctggcgctgggcattttggttaattgtcctcatctcagtcatgattacggtcatgttcatgttgtcgctgcctggagatttgcggcaagggaaagcaaagagtttgggtgaacaattcagccttttcaaagatccccgcattctcttggggatttgtctgccaattcttaacttaggcggggtctacgttgtttatacctaccttcgaccaattgtgacgtctggactgcattttccaaccagttttgtgacgccgtttctgtttgtctttggactggcatcgttgttcagtaatcaatacagcggccggttggcgaatcggaatggcttaaaatcaatggtcacggtgtttgtgattcaagctttgaccatgttggcgatttcgctgttattcgggttgccgtgggctgcactggccgccttaattatcatgggcctgacgatgtacttgctgaactcgccaatgcagattttctacctggctgtggctgaaaaagactatccgcagtcgatggtcttggcctcatccttgatttcgatttttaataacgtaggaatcgcggtaggatctgcaaccggtggggtcttgttcaatcacttgggattaaaatcactgggatacagtggggctgtctatacggttgtggctttggccattctaatcgttttgaaccgggtacgaaagagttttgattaacgattgcaagacgacatttctcgccattttattaatttttctgttgttactttgaatgaccaaatcaatgtaatcataaaaaggtcagccatgacaatgctttgtgcactgtcatggctgaccttttagtatattgatggagtcggcgggagttgaacccgcgtccgagcatattgccacctagatatctacgttcatagatctattatttgaatttcacctactgaaacgccataaatcaaggcacccacagcaggctaacctgattagtctcttcagttcacttcaggtgggagcaaactgcgtgagcccactaaatttaggacccagatctaacccatgggcgagattaggaggatctacgttaagcgcttattaggcagctaaagcgtaagaattgttattattttttgcagttataataaactgggcggtttaacgtggcgctgcacgaaacgcaatccagactcaacctatacccgtcgaatccataacgaccccgatacaatacacatcatatcataaatcacgggaactgagaagaattgtgtcttacaacaggtcaaaatatttgaggccgttaacgataccatgatcggtattcttggtcgtgataaactcggcatactttttcacctgtggcagtccattttccatcacgacggggtgatcaacgaaatccaacatcggaatgtcgttgttgccgtcgccaaacgcataagttgggatgccggagagattggcgttggcaatcaactcctggatgccttttttcttggaactgcctttgtgaacaatatccatgctaaacggggtatttctgaagaatgtcagggtgtcggcgaaccggtcaatgtatctttcgtcaggccccttggtgttaatcaacatcatgatcacttcttgattctcaatgaaatcatctacgcccaagtttggcatccgggagttaatgaagttataattgccgcggacgatgtcattgataaaattaatcttggcaccctggctgttcataaccgtggttgcttcgtggttggatttggcaaacgccacaaaatccttaacaacagatttttccaggacagctttgtaaaccggctggccttcaaaaatgacgtaactgccgtttgcggaaaccacagtgttaatcccagtcttttgcattgtattggggatttcaaataaatttctgccggtcgaaatcactgggagaacctgatttgcttttaattggcgcatcgcatcagccacttcgtcgtcgacacgcgtgtgttcattaaataaagtatggtcaaggtcaaagaacgcaattcctttatacatagataagccatccttttcattatcaattttataatcatatactttactatcataacaatattgcgactttccaagcaagttcttctaattattggtaaaatgggttatatatggggtgagacgattggaaaaaacaaccattgcgaatgaaaagaccagccgtttcttcgttcgactaagaagaattcccggcgaacattggtatttagcaaacggtaacgaaaaaaatgtaaatccaaaaaataaaattaaagttccggacagcatcaaggcacaggattttttgattgatgagattagcttcttcaacaaattagtctggtaccacttcacttgtggagatctggaaggctggctgcccaaacgaaatattcgaaagacatttcgccgattggacgttgaaccgattaagcagcccacgcaatccgatattgataatcagtgtacggcgattttaatgctgcttaacagcgccggcattaatgtcgacgtcagcgatatccgagacaaagttgagaagtggcacgcgcaatcgggaaccctaatggatttgagtgacttgattatttcgttaacccactcaattcgtgatctgaacggcgttgattttcgcaaattagataagcagcttttgcgcagaagaccgattttagtcaaagttgccggcctcgataatttaaagtccagcttgatcttgttgaccggttttaacagaaaactttactactacaacgatccgtggaccggcaaactagagtcgatttctcaaaatcatttaagaaagcattggaaacgcgggaacttggaagcaatcagttattgaaggtggggttttagaatgaaattgttgatgattgaagataacaaatcagtgtcggaaatgatgcagatgttcttccaaaaagaaggctgggatgtcacatttgcttatgacggcattgaggcaatggacaaatttaacgaagatcctgatagttgggacatgattactctggatcttaatttacctaaaaaagacggcatggaagtcgccaaagaaattcgggccaagtcacaaacggtcccgattattatgttgaccgctcgcgattcggacagtgatcaggtcttgggatttgagatgggcgcagacgattacgtcaccaagccgttttccccaattaccttggtggccagaatcaaagccttacagcgacgggcccacactgaaactgaagagaaatctgaggacgagaaggccaaaaatgtctttgacgttcaaactgatcactttaaattgaactccagtactcgggaagtgtatttggatgacaagcggatttctgatctgactcccaaagagttcgaactgttaaagacgttggcccaaaagccacgtcaggtattttcccgtgagcagcttttggaaacggtctggaattatgagtactatggtgatgaacgaactgttgatgcgcacgtcaaaaagttgcgtcaaaagattgagaaggttggcacccaagtgattcaaaccgtttggggcgttggctataaatttgatgatagtgaagtgggcaagaagaaatgaaaatgatttatcagcaattattggcgttctttttggtaattggctgtacaattttattgctgggtttttcatttagccgcatgtcgaaaacgtttgtatatgaccaaacctggcataacttggaaaagtattcggatagtttgattcaacaatcgctgacgattagctccaagaataaggccaaagtgacctttgacgaagagaagttgaagaactctgaagccttgttggagaaccaagcggtccattttaccgtcttcagtccacaagaccaggtgatctatcccaataacggcgttgccccccgaattacccagaaagactgggagcatttgcggcgcaatcagatcgttcggaaggtcaataataagaatttcaagctcagcaatggcaagacccggccggcaatgattgaagttttaaagccatactattataagaaaaaactagtggccgccgtgacggttggtgcctttatttcggatgttaactccaacgtcaagcggattaaccgcgatttgttaaaggcgctgtttgtggcgttgctcatttcgatgttcattagttacttcatcgccagacggctgaatcgacggattagcaaactgcgaagtgccgccaatcaggtttcaaacggcaattacaagattcgcttgaaacccggtgggaaagatgaaattggcgaattgatcgtcgatttcaaccacatgacccaatccttgcagcaggccaacaatgaaattcaacggcaggaagaacgccgccaggaattcttggccaatgcggcacatgagatgcgaactcctctcacaacaatctcgggcattttggaaggaatcaagtacgatgtgattccccaggagtcaagggccaagagcattgacttgatgagtagtgaaactcagcggctgattcggttggtgaatgagaatttggattacgaaaagattcgctccaactctattcagcttgacaagcgtcattttaacgccgctaaggtccttgaaaacgtcatcgaccagttggacagcaaagcagaagaatcgcaggacaagctcgttttgaacgcccctaaagacctgtcaatttatgcagattatgatcggtttgtccagattgtcttcaatattgtgaccaatgcgatccagtttactgatcaagggacgattaccgtgaccggtgaacggggctacaacgagaccatcatcaaggttgccgataccggtattggcatgtccgaggatcagcaaaaaaatatttttgaacgttattataaagccgatgcctcacgaagaaccggtaagtacggtgagtcgggactgggattggcgattgttcaccagttggtgaaatcccatggcggcaagatttcagtttcatccaaactgggtgagggcacgacgtttaccgtgattattccggatgcgacagctgccgaaaaagaacaagaaaatcactaaattaaaagtcatcattttgcatttgcttgagagagtctcaaggatgcaaaatgatgactttttgttagctgtttgattcttgggctgcatgggcttcgtaagccttggtgcccttttctgttaaaccattgatttcgttgtggtcggtcacgatgtagccggctgcgaccagtggcttgggatcgccgccaatgacgttatcacaataatcgacgaagtggttgaccggggtgccggatgatacccggccggtataaattgcctttaaaatttcatagtctgttgccgttaattccatgatgaagcctcctaatcttgatgcatttatgataccaccaggacgggtgcgggcggtgaattttgtttggtgatataagacactgacttcagcctttaaagattcggattattagcacagaccattgcgatgagcaagttgtcaccgcataaatggttaaagtgatacaatattttaaaattagtagcgttttcattaaatgtccacaactggtcaccaaaccgaagttgcgcaaatcaaaatatcaggatagtgagaaggctaattatgaaactagcaaagaaatatttatatagcaccattctcggcctctctttaggagtgggaatgtctaccaacgtggtgaaagccgccccaagttccaatagtgccgtggtttctcccacgagtgacccttcacaagacgagcaggcaaatccagacctatcgggaaaggtcgaagatgtctcctacacggttaaggatgaccagctgactttatatggcggcacgatcaaaaaaattcacgagaacttttcacttccttggcaacaggatggggtccgtgaccgcattaaaaagcttaagattgatggcccgcttgaatttgagcaggatggtgcctatgaattttttgaggcgttggggaatcttgaaagtatatccggcttaagaaacgttgatacgtcaaagaccgaaacgctgaattatatgtttgctcaagatggcaacttaacatccgttgatgtctccagctttcggacacccaatgtcatcacgatgagtggcctgttttttggtgattggaagcttgaacaagtcgatctttctaattttgatttttctcaattaaaaaatacggatcacatgtttgggggggattatgtattaacgaatatcacttttcctcattcgaaagcttctaagattgataatatgctggatatgttttacgggaatcactcattgaaaacattggacctttcagactttgacatgaccaatgtcacggctattggcagtatgttttccgaggatacgttactatcgaatctgaaactggggccaacctttaaaaattcagctttggccactctcccgccgcatcaaaaaggcgatgaaatccccattgatcccttgaaggacgccaccggtccaggatggcaagcagttggtgccaatggaacggtcaacaatccacagggcgagctctatccaacccttgaggactttgtggctaagcggcctgctgaagacgaaacctatgtctggcagcaagacaccacgcccattaatcaatatatgctgaacctgactaatagttcggcttcagtatatgagggccttcaagctaagaattgggatccgaccagtgtgattcaattagcgactcacaatggaaccgatgataagaatgctgttacgattactgatgctaatggtcagccggttacccaggcaactattgcagcactggctcctggaacctactcgctgacttatcagaatggtgatcagaaacaaccatttaccttaacaattaaggccgatcaggccagcttgaagacgacggatattgatctttatttaaaccaggcgttcactgaagatgcgttgaaaagtaaaattttggcggtcaattccgatggccaggctcttccgtacacttacaccatcaaagatgcaactggcaaaactgtttcgcttgatgacgtcaaatcaaaggttggtcaatacacggtcgacattgttaccaatcagctgctaagtggtcacgagcccctggaagggaagctcaccatcaacgtgactgacagcagtaccctcaatctcaagtatggcaagctgacaatccccgtcaatcaggcatggaaaccggcagatgcatttgataatgccaaagatgccagtggaaaagacctagcctttaaagatattttggtgacggcgaaagacagctctggaaagatcatctcagacctgagtaatctgtataaaacgccaggcgtttacacaatccattacagtaatgggtcagcttcaaaggacgttcaattgacggttacccagccgacgccaacaccgtctccattgccaacccctcagcctgtgccaaatccgcaaccatcaccgacgcctaaccccatcaatccagtcacaccaacgcagccaacggttccaactcaaccaactaatccaaagcttcctgattacgcggggacaaagggcgcggcagtcgctgccattaacaatgtctatttgtatcgaacggttaacttcaccaaaggccagcgaattgccaaatatatcaagaaaccgcgcatttaccggccgatgtttgtggtgacggggtatgctcgttccacaagtgggaagatgcgttacaaagtccgtgatgtcaaccacttatcgaagacggcgggcaagaccggctacatcaccggcaattggcgatatgtccgtccaatttattacgctactctgcacaaacacattacggtcatttctccggcaggggttaatgcctataagcacaaagacttgactggtaaggtcagaagttatcaacagggaaccatcctcaaagttaaagggatcgtgaagcacaatctgaccacccgttatatcttgacgaatggcaggtatgtcaccgctaaccgaaagctggttaacatgggtcggcatcggaccgttaagaaagttcgggcgaagacaaccattcatcgttatcaaaacgtgaacttgagcggacggcctcacacgattaagaagggccagatcatcaaagtatccaattatgattattcccgtggccataatctacaaaagcacggtgccttgcgataccgtgtggctggtgggtatatcaccggtaactctaaatatgtcagaattattcgataatttacattagacagtgcgacgagaggcgttttgatcccagaatttaagcaaagaagcgggctattcctattttggagtggctcgctttttggggatcagtcgatcgccaagtaggccaggcaggctttcagccggccgtcgctgcacgttgtatcaatacaaaagtggtaatcaaatccaccgtagcaattaatgtccgaacctcattatttttctgcgaccagaaattgcatcagtgtgaaatttttgttgtggcattttttgttagacaatttattgaaactgtctagcggattttgcaacaaaaaaggtgttagccaaaaaaatggctaacaccttgctgatccttgttaaatcaacgattatcacccgaacggtaatcggattagttaaaagaatagctagtaatcgttgatgtgacagcttataatgttccaatcgttcatctataattacaaaaaaatggcaaagagaaaaactgatacaactataacgtcaattgttaaacccttttcccagcaatttcatagcttctttgtccgacttcccgttctctttttctacaaagtgaatgtaagtattaatcgtggtttgcaactttttatgccgtaaccgatgttgtacataagtcagattagcaccattttggattaagtagctggcatgtgtgtggcgcatggcatgtgtcgtaaccctctttatttcaagtttagcgcaaattcgacttagcgcacggttagcagaatcattggtaatgatcctacgaaatttgctaaaaaagactaaaccacgtggattgagcttggcgtaatctaatttttggtcggaaaagaattcaatggcttcttccttgaactttttaagagctcggcaataattttcaggaatggtaatagttccatccgcctgcccgttgcctttggttttagtgaatgtattggctgctgggtaccattggcggtcaattattacttttccagttttaagatctaagtgatcccaggtcatgccagctgcttcttcaaaccgagttccggtttctagctgaaaaagtaacattgctgaacttatatgttcaaagtcggcatgcttgattagatagtcgcgtaaaattgcataatcatctaaatccagaaatttatcatcgactggtttagggcttgatccagtaattttaactttgaaggtaaaatcacgctgaattagattctcagctagtgcatcttgaatggcagatcgaatttgttgattggtttttcgtgaggtggcaatgccatggctgttgccaaacagattcataaatttctgataatcttccttttgaatatcaattaacttttgagcagggaagtagtgccgaagatgttgagctgtcaattcatacatatcgtgtgtatgcttagcgacaccatcagttttatagattgatacccaacggtcaaagtaatcggcaaacgtgatgttagcgttgcggaaatcggcgccagagttgattttagcccgcatatctgtttcccagtgttcagcttcagtttttcgtttaaagtttttgctacggcgacggtaacgaacaccatctcggtaacttacacgagcttgccacatgccattttctaacctggcaattgccattgattgtcaccccctacattaaggactacgtttatagatgtactctacctgaactaagtagcaaatctacaaaattgataatcaagttatttggttcttttaccagtgaaatatggtgttaaataattaattggagcaagtttggaattaagagttttgaagtgactacttgttttgggcattctttttgcatctggttttaaacatgtatatcgaacaccatttttatcttcaataataaaaatacgattgaaatcaccttttgtgttaataactctagcattttcatgcttaatattaaaaatatctatataattcaaaaaattacttctttcatttttaaatccatgtggaaaagttaaaaacaagtgcaaggttgacgtgattgaatttattcaagaaagcctatttttgggaattattctttttcaaaatatcagcaatttcttgcaggtactgagcttccattgagattggggcagtgggagcttcttttttaggcataactttattgataccttttactaacagaaatacaacaaaagcaataattagaaaattgataatggaattaataaaagccccatacttgaatgttgcactaccaactttaaaggcaagatcagaaaaatcaatttgtcccaagaagataccaattaatggattaattaagttatcaactaatgacttaacgatagatgtaaaggcagctccaataatgacaccaactgctaagtccattacattaccacgtgaaataaactctttaaattcttttaacatacaaatttctcccttaaatttttcagcttttaacgtcatcagtatttggactgtaatccccatgcctgagtcgaacaggtactggttccgagtggggaagtaaattaattattgattgaacgttgatgctataatgatacaaagttattcttttagaaagaggatattttatggacatcagagaaaataaaattaaaaagttttgtaattcgctagattattgggaaactgtaaacttattaaccatgattttaaaggctaataatcctcactggtcagaacctgattgctattcagaagcaactgcaatatttggagatgagaagagaaaaaaatttttaattgaagaaacgcttaaaacgggtatacacactagaaggtagagctatttgcagtattccagccgaggtcttcaagaaccgtatccccaacttcaattggattgttgtcgttaattgaaccgccactaatatccttggggttaacatctaactctggatattcttttcttctaaataaagaagaaaccgcagtaatatcggaaatatggggaattgaggtacaaatagtaaatttcttgtagatagtttctgccattatatgtgctttaataggctgtagcgggccataatcttctttagtatctggatcgacgatgtttgtaacctttttaccaatgattctaaagtgatctccctcttttatgtcattatcgtcaccagcgttgataataatatgggtaccatcaattatctttaggactttgtattctttttgtgtcattctcagttttacctccttcgtttaataaattagtaaagatttgtaatagttgatccgaccgtgctctttcaacaactatgccacgattgtcttctcgtaaatctctttgtaagctttccttatcagcttttaggcgagttcgatcagatatcaaagcatctctatttattttgagtgtgtcatacttcttttttaggtcatccttcgattgatttaagactgtaagtttatttttaagttgttgattatcaatagacatatgagccatggttgtacataaccacaatatgatagaaagacttatcgaaataaaaatagcaaaattaatgcgtatgttgaatttgttttgcgtgatcgcatataccaaaatgccagctaaaactgcagtcgacacggcagaaataaaggctagaaaacgtattaagtttttgattaatatgccccctctattttgtacgtccatgtgtatctctccaatagttagtccactttgacattattaatttttgaagtataattttacaattctcaaaattatttattttcggtgatacgtttctaggatgctcataccatattcaagatgaagggtatcagaaccgccatgccataaaacaatcggattagcgtttgaaaaatggacagtgtaatacgaaccagatttactaacgtacttaacgtgtctccagttcgtatacatttttacgtaacgtgctgtaatcctcatatggcttttattatcataattataccaatgaccacgcatcgaatatggaatggttgacgaggcacgtgtaattgtttgatttgttgtaaacgcaaagccaaaaattaatgcgatggttgcgaaaaaaatcaaaaaatatttcttcaattctaagatctcctctaaattataataagactatttaatatttaattttagtgttctaataccaccgagttgtgattcttcttcggttgaaaccccagcagttttaatagtaaggtgtttgctattaatctttttgtaagcgtcttgaacgtcattgccataacataaaattgcatccattgatttatcctgaacagttttatgaggttgaacagttaaactatttgtttcgtcgttaacttgcaaacttgaatggtcaatctgaaccccattatcggttgtccaatcaaaatttccaccagcgtacccagaaaatccgtcgtaatttaacggtttgctagtattattttgaaaatcactttctagatgcagcagaattattgttttgcccgttaagctctttggaaagtcaccattatttgggaaaacagttttagcatcaggctgcatactgttgtattcgttgtcagatgataaattttccatagctataacagcatactgcgtattaaacaatttcatcccatgaactgtttgattagggatatcttgtaaacttgtaagataagttactctttgtccttctgggcccttcatccaatctccttttttaggataaatagttttactagatatttttttaacatgaaatttatcatgtaatacttgtggcttctttgctgcgactttagaagtcatagtttttgatgagctattttctttgctacttttcgtgtttccacatgcgcttagtgttacccctaacactgctacgcttaacaaagacgctacttttgataatttcatttaactcgctccttaatattttccctacataaatttccaagcaattcttagcccataatctccttaatcaatagatttacatctaaatctgtacacaaacccaactgtatgtgagtaatagatctgaacgcctattttgctgtttttttattagtcgctttaagaagctcattgttttgtttttgcagtgtatcattctgcttgatcatcagccaattttgttccacgatagtttgcagattattgataatcatgttttcggcatcggatccatgtatacgagcacctaaattataagcaagcacgtctattaatccattttggctcataatgtttttaacaagctgataagattttggatttaagtcatccaagccgtgttgtgctaaaaaacgcttaactttttgctctcttttttgttctttttcttcttttgatttaaataaccccattttaagatctcctcaataatcattgtaataaacttgttgcgaatacatatttacctaatatcctaaaatcttggtcaatgttcttaggaaagatcagcggcttataaataggattaaatgattctggttcaaggataactgctttggaggtttccttgaacctctttagtgtggcattttctccatctatcagaacggcgcagatgtcaccattatctatcccacaatccttagcaaacacggcaataaaccctggagcaataaccctactcatcgaatccccattaacttgcaatgcaaataaattgtcacgtccaaacctgcgtatcaaatcatcggggataattgtttgaccaatgatatgttcatcggcaaaggtaggaataccagcggtaattttcccatagacgtctaatggttcatgcgatgtttcccattttgtggttgccgcagcctcgattccatcaaaagttggcgtagttttggcattagtcgcggtaggcaaatatccagcccttatcattaagtcatcgtaacttgcgtgataaacttttgatagctccttaagagtatccggagatgggacaaacgattttccacgtgtatttatacccttttcagcttgtgcaacagcactgtggctaattttattacctgaccgtctagcaacctctctatatgataagttgcctcgaagctttttcagatagttccccaattgattcttatcattagtcattgaagcacctccatctttattgtaattcattgtgtacaaaaaatatataaaaaaatcgtatttaggtgtttacatatcgtaaatcatgaagtacaatatatttgttgattgagaagggagatgatcaaatgcgagcgagaaatatttcaaataatgtccgaaaggcccgattggcagttgatatttcgcaagcagaacttgcaagaaaatcgggtataaataggccgtatataagtaatattgagcgtggtaaacaaactccgtctgtatacattggtaatcgtttggcagaggaattaggaactacaagtgaatacctttttcctgccaaaaatgtacacattgatttacagaaagcccattccgctaaatatatgcaaacaccacccgtgccaccgagaaaggaggtgagcgaatgaataacttagtaatcatgaagaataagcaggctgtcactagcagtttgcaagtcgctgaaacgtttgggaagcgtcatgaccacgttttgcgtgacattgaacactttcgaaaagatctacccaattttggggagatgtttgttgaagtaaacgttcctgattcttatggacgtgatcgaaaagcatactacttgaatcgtgatggcttcacattattggcaatgggatttaccggcaaggaagcattgaacttcaaactgcagtacattcgagcttttaacaaaatggaagcttcacttcaggaactcggcaaggactcttatcagatttctgatccagtcacgcgggcaaccaagtggattgaagaagagaaacgtcgacaggagcttgaaactgagaataaggaacttcgaattccggctttgctaggtaacgcagtcagttcctcaaatgataccgttcgtgttggaacctttgccaaaattcttaagcagaatggctacaacattggtcaaaatcgattctttgagtggctacgagaacacggttacttaattcgctctggtcagcgccggaatactccaacacaatatgcaatggatttgaaagtgatgtcggttcgcgaaaccgtgattagcactaatcatggttccattaataaatttacaccactaattactggcaagggtcaacaatactttataaataagctattaaaacccaaagaggtgattaaatgaccggacgggagccaaacacctaaggaggtgagcgaatgagtcgaaaatcaagcacaaataagagcgtcattaaaatcttatcatcaaaagagagaggtctcatgactggaggcattcttcctaaacacgtaacgattttaattggcactcttgaaattgatttaacgattgatagtgttggcgacagcgttgatgttgaatttgacagtgaaaagaatctaaaaaagaaacctgaatctcacagtcttgaaaactttttagaggcttcaaaattgattgaagagctttttaacgataaagaataactcaccagatccttcatagcagaaaaaagcgtatttgggatatcgcgaatttaaaaacctgacagtttcctttaaatcacgataagaaatatccgaagtttttaatgaatatcgtatagcttttccctcagtaagttccgacgcttttgtcaaaaactgattaactaaatcttgactaatggccattgttaccacctctgatgttgtgagataaatacattatctcactaaagaggcaaagccaccgagaaaggaggcaagggaatgatccatcattacctaaccgaatatcgtaatggaaaaaatgaagttgtctttgagtcctggattcagctcaactttttaggcttagtgtggtgctactccgtaaaaagcttcgttttgaacccggataaagacaactccgatgcgattgataagttcttgagcactatgtcgtatcacgaacgttaatcagttcgtccactggtatgcttccacttattgtgagtatcaggactcacagggggaagacgatgaccagacacacgaattgtagcgtgtctaggattttgaagtttaccaccttgagggccgacttcaagatatttaccagttggaacgttatcagttccgggttcataaagtttcacattatgtcaccacctttaatggaatagcttaattatcccactaaagatgatgttggattcaattttcaaagaacgaaagaaggtgatcccatgactcgtgcagaaatgatagaacaaattctcaatagcccaactgccaaagcacatggcgttgaaatggttaaagaaatgattgaccggcatggtgatgattttctcaaagccatgtatcaatcactttgtgatagtgaggagcaattactgttttcttaactccttaagtccaatttaccaaatcagatggaaaaggacgattaatcttttttcaaaatggagatgatcaaaagtgaaagattcaaaatttgctaaacaattaacacttgatttagacaaattaaaaaagacgtttgaccgaactgaaattgctgaacaggcccatatttctgatagtcagttaagcaatattcgagctggtcgaagaaatgcaccacgagatgttaagaaagcactggtccaaaggctatggtcgttaccactggcattcagtgcttcaagaagtgagtttggtattccatcaatgatgaacaatccagttttacagcaagatttatacgctgatgaggtttctcagaaaaaggaagaacatgagcggcaatcatctgaagatgaagcagattacattattgccatggatccgcgtcagcgaacacctgcacagtcagacttcttgcttaagcattttaaggattcttttgaagagattggatccgaattgaaatacacttacgcaaaaatgatttttgccaagttatcagatggcgagattaaagaattggttgatgaatataatcaaaagtttgggggctagaacatgagtgaaccagttgattcaattattgttaaatatcaggcacccgatggttacaagctggttcatgacaccgactatcaagactttttaacttggaagaatcgaatcagcattgaggaatggacactcaaggaattctcttggaacgtttggcaccaaagaggcgtgaccagagcaaagaactttttgtatagtcaccgtaacgatttggatatagctaatggtggatttatcgattacgagcatactcacaacggttggaggattccatctgaacaaattcagaattatatttctaaaatacgagcaagggagatgtgaacatggttttagtattaccggattggatttggtgggcagtcataggcgttgctggtattactgttggttatcagtaccgtgtttatcaacaggataaagttgcttggatgaataaatggtttgatggtccaatcaacattgtgccctggttcaaaaagtattttgagcaggttaaaatcgacatcaacgaaataaggaaaggatgagcaatatgcaaagcttagataataaaaaaagcaccagacatgtaggattgtctggtgcaaccaaagagagattgtttatactacaaaacattctattcattgagtatagaccgacacgaacatttttgcaacgatttttgggaggtattaagaatgaatgaggatgagtattacgaaaacatggctgatgaatatgaggatccaaagccaacacaagaagagttggcggaggcggaatatgccgaatatgaagaccagcatgaagacgagatggatattggaggagtggaaatatgaataataaactggaatatgggttgagaaaaattaaatatgcgcgcttgagagtcactggattggaacgagcttatgaccaagaaagcaacccgatcgttaaaagagcgttgctgacttgtctcagaaaagaaaaagataaactaaatgattacgaagttaccggaatctacgaggaggattagctatggatgaaattaaagaggcaccggaaaaacaaacatttgttattgatgacgataacaaagcaaactgggcatttcgtaaattagctgaggttaagcaagagctggatatcaaagcgcaacaaaaagccggatttgacgaacaaaccaaggaatggtacgaaagcgaaactaaaccattgaaagaaagccaggattactttgaacagttgattgaacagtatcgccaaacgcaacctgatggcaaggttaaagttccggctggttataccagcctgcgtcatgctaaacaataccaacgtgaacccagcaagcttcttccgtttgtagaaaagaattatccagacttactaaaaaaagacattaaatgggcagacttcaaaaaacaactgaccgattatgacggggtagccattgatcaaaatggcgagaaagtacctggaattactgtgatcgaaaaggaatctgttagttatcaccctaataaattggagagtggtctatatgaagaaaagtgagaatatatctgaaattgcgaaggcactcaatgaggttcgtaagaatatcaagcagccagaaaagaatgcgaacaacccattctttaagtccaaatacgtaatgctggaaggcgttgtagatgccattgataaggcactcccgaaaggcttcgcctacacacaggaagttaccagtgatggaaatcaaatttctgtctccacgtttctcatgcacgaatccggccagtacatccagttcgatccgttgaacgttccagtgggtaagaatgaggcccaggcgtttggatcagctgagacctacgcacgtcgttacaccttatcagcagtgtttggtgttacgtctgacgttgacgacgatggtaatcaagcaactaagagtgctcgaaaagaacagccacataagcgcaagtatggccgtcaggctccagctaagacacctagcaagccaatggctaccgctgaagataaagacaccatcaagggtaaggttgcttctctggccaaagagatggcaatggagcctaaaccattacttgaagcgacgatgaagcacgccaaagtatcaagttggggtcagatgagtaaagaagacttgaatgctttggatcatgaactcagcactgagctgatggaatttcgttctaaaaaatcaaaagacgatgagaaatcatcggatgaattgtttgacagcctaaatgtttaaccactaatcaaatccaatggaggtgaaaaaatgaactatctacttcagatcaaagcgttctatgaccggctcgaactaaatccattgaactcatcagaaattgccttatggcacgccttaatgtccataaacaataaagctgcatggtcaaatacatttacggtagcctcgtcggtgttatgccagcgatctggaataaaggacacatccaaatcctccaacttttacaaagcacgcaacgcactcacccaacaaggtttcattacatgggaatcacgtaagggaaaccagtcagcaaagtacagtattaccaagctttacggcaatttgtctacatatagtgtgggcaacggtgtagacagtggtgtagacaacggtgtagacagtggtgtagacaatagtgtggcattaaataaacacaaacagaaacaaaaaaagacttctcgtcgaaaccgaaaaaaaccggtttacgaccaagcaaatgatttcatgaaattggctgtttatctgcaaaagcaaatcatgctgaacaatccagactttaaacaaccaaacttgcaaacttgggctgacgatatgcgtaagcttgttgaactggaccatcgtgataagcaccaggtagctttggttatcaagtggtgccaacatgattctttttggtcgaccaatatcctttcagccaagaagctaagggatcagtacgatcagctttacctcaaaatgcaagccggtcaaggttcaacccctgaacaacgggtttctaaaaagcaggatgagcataaaaagtggctgagagaccgtgacaaattcgttctctacaagtattccgagaccggaaatgatcttgacgaggcgatgccaattatccaggctgagtacccgcaagtcactaaagccgaggccgagcgaatactgcatccagaactctatttagcagcaggaggtgttgatgatgggcactaacagaaacatgccagagattgagcgtaaggcgatgtggttcctgattaaccaaccgcaagtcctggaatcaaacacggtcgacgagaaatggtttaccaacaatgcttaccggactcttgcaagctatgtcaacttgtggggcacccgctacgagaatgctgaacagatagcggcagcttttggtgataccccgtttggcaagaagctggatgttcaaaggatcttccggtcaattcaaggggtcgatcggccactagacccagaagctaccttcaaacaattacgccaggcttattacattggcatgatgaaaggcgccgctatcaatgtggctaaagatcccagcgaatttaactttgaacatttgcttgatattcgtaagcaggctgagcaaaccgatactcatgctgacattgacgccagcaagcaggttgaagaggctctgcgggatttgaatacgcccaatacttcgtttatcaaaacctatccagggcttgataagtatctgggtggtggcctggtaccgaacgagctaattgtaattggggcacgtccgtcagttgggaaaacagcttttgctttgaacctggcaaccaacgccatcctgggtgatccaagtttgacagttgaattattctccctagagatgagttccaagcagaatatgcggcgcgtgtatgccgccacgtctggaattccgttgaatctttggaaaaatccagctgtgcggatgagtgagagccaaaaggaagtcgctgccaatacgattaagcaaattgctggcattcgcttctggtcaaacgatcgggtggccaccattgacgacatcagcagtgtgattaaacagcacgctcaccgatgcaaaactagccgctacttggcgattgtcgatcacattgggcttgtggagaccagcaatccacgtgaagatacccgtcaagcactggaagaagtttcccggcggttgaaattgttgacccagaacttgcaaattccaattattgcgctcagtcaacttaatcgaggggttgaatctcgccaaagcaacgagccaaatttaagcgacttgcgggaaaccggtgccattgagcaagacgcaaacgtggttggtttcctgtggcggccaagtgatgacctggatgatcctaacttgaacttatcgatcaagaagaatcgtgatggtgaaactggtttgttgaagttctatttccagaaagatttacaaaagattgctgaggtgagcccacatgcagtacatgaataatcaagaattaaaagagttgtttaccaaagaggatctgcacattaccaaagcggtagccattctactcaaacaggctgcattgtataccaagcgcattcacgtgcttcaggattcacagcagttagcggattgtgagaatgaacgagcgaagtacatctacaaagcaattgaggtggctacaatcgaaaagcaacagcattgtcggttgattgaggacaagaaacgttatcttgacgccatgaacgacaagtacggtgatgtggattttatcaatgatttgaaggatttaaaaaaactagtgctgatataccggctggagaatctggatgagcaacagcaagctcatcattcacctgagtatatggcatgattggagagattattatgcgaattatgtcaatcactggcaacgtgggcaaagatccacaagccaggcaggtaggaaacaaccaagtagctgatttcacagtggcggttcggcagaaacgaccagatcgaaatggtaattacggagtagattgggtgcgatgctccgtctttggaaagcgttctgataccatcatgaaatacttccaccaaggtgacaacgtggctttgtccggtcagtggtcaatcaaccaatggacgaatcaacaaggcgaaccacagtttagcctggagttgagcgtgaacgacttcgatttaccacatcgttcaaagccagaacggtcgaacaaccagcgaagcaatgatccatttgcaagcagtaatgattcaattgagattaccgatgaagatatgccattttgactgaggtgattatatgtttggcaagctgcaaggaatcaagggcgatgaagtcacgattaaacttgatgatgaactgaatatgtatcggctaaaccggtttgccagccatcaacagccaaccgtgtacttagacattgatgatggccggaaaatttcaccggatcaacgcaagaagatatttgcgatgttacgtgatatggagcagtggataaagtattactactatgcccaaactggctcagaggctttctcaatggcagattgcagtatggacacagcaaataagttcctgacattcatcttagacttctgttttgccaatgatattccgtttaagacaaaaacgtgggatcagatccccaccgattatcacttggctgtccaatgtttaagataccgaaaatgtgtgatctgtggccagccgcacagcgatattgatcattttacgccggttggccgccgaaatcgtgcattggttgaccaccgaaagctgtattttgaatgtctctgccgtaagcatcacacggaaaggcatcaattaggtgctaagagctttattgagaagtaccacattaaaccggttaggttgtcagaagatgacctaattagccttaacattatgaccagaaaacggatgaatgaaatcgacggggagatgtaattatcaaattaatcggcattaagagtcacaaaacatatgccaaggggccaacaagggcggacttattacgccagcttcagcatgattacccatcttttcagaagcctgccaaggtgactgataaacacggggttgccaatactccggtcttgcctgaagagatgataatcatacgaattgagtctaagaaggttgttaaacacgaaaccgaattgagaacggaactacacaagtatcggagcaattaatggaggaacaaaaaatgaaatttagtgaattgaaaagtaaagttgaagacctgggttatcgggtttatgtagacaataatgcaacgataatagggacaaaagatcatggatggatacttttaatcaaaaattaccagtgcgggcttatgagttattacgatgacgcaacatatttagagcctgatagcttgcttgccttgcaaaaactagcctacaagtattcccggacaccgattgatgagcgcgcggatgagcctaagtttcgggtaaagatgtttcccgaaagtactgggtatttaggttgctatttatatttagatgatgaatcgaatgatataaccatatttggcgatgaggcaggtaccctttttactcaatccgaatacgataaacttcaacagaaatacccagaatggttgccaaagtttgataaaaatgatccacactttgaatttgtggaggatgattaaatgtttgaatacgaagatgaaaacggccaacaagctattttacttagcaaagttagctttgtaactaaaactacaggaaatacttttgctatatattttgctggtgacagtagagataaggttgatgtgccacttgagcaatataccaagtttatgaacatgcttaaagcgtgggcgatgaaacactaaggaggcagacaaatgaaaaccaaaagagacctatttgatgaagtctatcgtcgatatggtattcagacatctgcaagatttcatgtaaatttggatgaaaaaatgagcgatgaagattatcaaaaatcattgaatatgtattcaaaaatgccaaaattgtttgaaaaattagacgaggaggatggcaaagatgagcagagaaattaaatttagagcgtgggataaggaggatcaagttatggattggccaactgaaattagctgggatgatggaggggatattcaaaacgttgatgcttatcataaaaaaatgactaataactttgttcttgaacaattcaccagtttaaaagataagaatggtaaagatatttacgaaaatgatattgttcaaaatgaacaaggacaacagatgctaattaattataagtctggatgttttcttgttggtaactattattttggatctattggagcaggcaaaatacttgaagttataggagacattcacaaaaatccggaattattggaggtagaaaatgataagtaatgtgggttatgtgtttgcaggactaggtttattattctttgttcttcttggtttaagctttgtgattagttcaataaatgaattccgtatcaacaaacagtatttgccagatattaccaagggtggcaacatcaaaattaaaattgatgacggaaattttgagtattatcgagttgacgaagtggttacttatgttggcgatcggggtaaacgatcagttcaaaatgatgttaaacagatttcagtgcataaattaactgatgacgaaatttctgacgagttactggaggtagagaaatgagccagtttgaatatgaagcaatgtcagaaaaagggattattgaaagcacttttggaattcagccaaattcagatggtacctttacctttattatgaatcaaaagtatcctcgtaagaaagataaggctattcaaatgcggtttaccaagaatggtttgagtgccattactggaatgttacgccttcttgaatctcgggaggcagataaatgagcagatgggacttgaaaaggattaagcatcagaaacgattgaaggctaaaaagtataagattgggcaagatgttgaagcacgtttgaaacagcagtctcttgatcggtttgagaaggctaagcgacggcaagagtcaatgactggttggcacaagttaatttggaggtagatgaatgaatttactagagcattacattcaaccaggatggacagtaacacccttatcagataaagaaaagcaagcaatgggtaagtattctaaattggattggatccatgtaaatggcaaagtggattgctacggaagtattaataaattccaagatatttggattagaagcgaatgggaagatgccgttaagcaaggatactatatggggtgatctaaatgttactgcaagaaactaaagattatatagaagatgtcttattaccagaaaatatggatggatatactactgcacgtgaaatagctgacgatactcttattgatattgaagatcttggcgatggtaacgagttgattagaccaacgagattaaatagaaacattgctgctaatcgcaaagagtttactgattacgttgttaaggcatttcaggatgtggaggaaaaataaaatgaaatatcaaaagaaaccagttgtaattgaagcatttaaatggacagcagatcaagaacaattagaagatccagaatggattatcaaggcgcttaagaatggaatagcggctttcatctatgaaggaacgccaaacgttaagttggttatcaaaactctcgaaggggatcatattgctaatcgtggtgattacatcatccaaggtgtacacggtgaaatttatccatccaagccagatatttttgaagaaacttatgacagagtggaggaaaaatgaaatgtacaattatagcgaaactaatagagttcggtggattaaattacagggaataacttttggagatatggaatgggtcaatacggattcaattcaaagagttgtggataatggatcagtaattgctgtctatttcaatggatatagtgagccggtttgttataaatatgattttgacaaggttcctgaattattgattaagcgtaaataaaaaaactcccgtttccgggagccaaggtgatgctaacaaataggcaacttcattataacatcaactaaggcttattagaaggggtgtcgggcttggataaccaaatggatagcttgtttccacaaattgataaagataaaacggttgagaattgtaagcatttcttgggcagtgtatttccaagaatgctaaggataagtgggctaacttcagccaactatgacgcaatgattgcagacttgaaatctccgacgatggatggaatgccaaaatcaccaaccacactgaataatgctgatacaacaattgttcgaagagcatacgctcagcaaattgttaaaagaacggttgaagcaattggtagatgcaacaacgtcggcaaagagcttttgagtatgcgatatttagataattatacggatacaatgtgctacatgtccattggctattctcgttcacactactttgaccacattaagcccggtgcattactccaatttgctgatgcgtatcttttggatgatttacatatttataaatcagactcaaaccagactcaaagtggactatgatcggactatttatacggatttatgaggtatattggtattgtggaatttgttaaaagagtttcactctctttccttagatgtgtgactgtaacgtatacgtacgaagagggcggaaagattaccgtgcagggttcgattccctgccagccacgttgttgattggacttgtatcaaagtaaattcttcctaaaaattaatgagtagtacccgtccagtcaacgaacatgcagctcacgcaaaaacaaaaacttgtatgttgtgttgtctagaacttgaactgtagtgagttacatgatgcctgcggcggaaaacgtgggcttttttgatacataaattggaggtggcaatgtggccacattaatgattttaattctggtcatgttgttgccagcggtgattgctgaatatggccgttataggggctggtggtactgatgagtgatcgtaagcatccatatacgcccatgaagcaaaccagctatggctacacttctaaggaagaaatacagatagacaagcaactggacaaagacttaaagaagcgtcttcgcaaagagggcgcttttaatttgcacaaaaaaacaggcaagcctggttagaagactcgcctgaaattgataaattacttgtccttatctgcttttttcttaatgtcatcaactgtgtccttaacggtttccttggcatcggataatttatccttggctttgccgagaatgccttggcccttaccttcagcttctctagctttgtcaccggtaactttaccttcaacttctttagctttaccgcttaccttatctttagcactgtctgctttatcttttaaactcataaataacatctccttagttattttatggtacacatacattatcttaaagtaattaaataattgcaaacaatttgatgctttgaatggaggatttttactattgagtaaacacaacaagcatacaaagagccataaaaagtccaaaattaaagatcgcaaacgtaagagtttagcagctcgacgattgaatgagttaaaacttaggaataaaaccgataacattgcttaacggcagtgctttttaatacatagaataactaaatggaggtgtggtgatatgtaatgtctaaacgtaaattaacaccaaagcaacgcaaatttgctaacgaatatattaaaactaataatgcttatcaatcagctataaatgcagactactctaaggcttacgctaggaatgcaacaaaatttttattggaaaatattggaattcaacaattcattcacaggaagactggtaaggccgaagcagaaactgagataacaacggatatggtgattgctaacttattaaaaacggctgctggtatatcctcaaagcatcgtttgactacttatgatcatttaaagcagaaactgactagtgacaaaacatatactgggccgccaacggttaaagatcaggtagcagcggcccaactagttttgcagatggccggtaagctcaaagccgatgatggggagttaacgaatgctaagatccgcaaagctaatgctgaggctgaaattgctgaaaccaagttggcagatcttgaagatgataaagacgatcagatggatgcattaaccgacatgatgagcaaacttgctaagaacgtgccaagggggtgacaaagatgacagttgacgatctatttactaagaagcaacagcaggttttaaatcaagaactgaataatcaacactggaaattgatgattaattatggtgctgttcgtgctggtaaaacctttgtcgataattttgtttttctctatgaggttaaacatgccgccgaaattgcacgatctaagaaagttaaatatccaatgtacattctggctggggtttcaagcaagtcaattgccaataacatcttgaccgagatagccaatacatttgggttgactttcaaatttgataagcataattcattcaaaattcgattccctggtttaccggcagtcaaaatagtgcagacgtttacaggctctatatctggattgggtgctattcgtggaatgacttcgtttggagcctacattaatgaagcctcacttgccaataaagaagtattcgaagagatccgatcacgatgttctacaccaggtgcacgagttgtttgtgatactaacactgatgtgcccacacattggctcaaaacggattatatagataatccgaagcattctaacgaaatcattagtaatcactttataatggacgataacacctcattggatccggaatacgtagctggccaaaaatcaacaacaccatctggcatgttctatgaccgtaagatactcggtttgtgggttgccggtgaaggattagtttatcaggactttgacaagtcaaagaatataattacccgtgccgagtttgataaacggactgctgatcagcagctaacatattactgcggtgttgactggggatacgaacacgatacgtcaattgttgtattggctgacgatactgatggtaatacttacttagttgaagagcatactggtcatttggagcagattatgcactgggtcaagattgccaagcaggttcaacaagattatggctacaatataccgttttattgtgatacggcccgagttgaacacattgacaagttcaaagaaaataacattaatgctcagtatgcgtataaatcagttttaaagggcattgaacaagttgcagggcttatcaagcagcataagtttatggccgttcaagaaggcatacagcagttcttagatgaggtttatcagtatgtttggaatgacaaaacgggtgaaccagtcaaagaacatgaccacgtgatggatgctattcgttacgcgattgcaacacgtcaatggaatcatgaatataatcagccacacgataattatgatcagcaagatcaactgctcgctgacaaaggattgatcgattatcccgatgatttattttaggagtgatgaaaatgtcaaagttaatgacaatggaagaatggaaaaaacaagcaacaactaagcaaacggcaccaatggatatgaatgtgtttgagccgatgcttaatggaaagccgcttgaatttaaagatcgtggcataacttattccattccaattggtttggatgtcaaaataatatttgaaagtttagcaaaattagtgaatgacaatattaatgaaaaagacaaaccggtcaatgactccaaaaagttgttggccgttaaatttgctcataaatattgtgaattacacaaaaacgatgaaagtaaggtaaatgacagtggcggaaacaaatgatttatcagcacattatcgttcaatcaatccacagccaaactccattaacttattaaacggccaacgttatggtaatcgatatgcatttcaaactaatcagtcgtacaacattccggcgtcttcatggaagccaattaaagacgatcaaagtaaatttcaaaagttagtgcaatggtacgtcagcgatcactttaataatcaactgccccgaatcttggagctggaacgttattatttagctgataataacattcactattggttgtctaataagcgttctaatcgggctgataatcggatatcaagcgctttagcacgatatattaccaacatccaagttggttatgagtttggaacaccgctgacttttggttatcaaaataaagatgatgaaaacgacactggtgaaaatgttattcaggctgttgatgattttaatcaaactaatgatgaaccatatcatgaaaagattatgggtaaaaatttggcaaatgttgggcgggcatatgaattactgtatgtacctgaaggaactaagcaacctaagattacggcgattgaccctaacagcgcgtttgttgtttggtcgacagatgttgaaccagttgagttatttgctgttcgttattatgccgtgaacgttgctgatgaaacgtattatcaaattgaggtatacaccgacaaccacatctatcactttactgctggtgccaatcctgattctgattggaaattaactagcgatgaaggacactatttccaacaagtcccattaactgaatatcgattgaatgaggaacgggtcggtgcgtgggaaactaaattagatgaaattgatgcctatgatcaagcgctatctgaaatggctaactcacaggaagatttcagtaacgcaatgttgatgattaatgggaaagttgctaatcattctggtaagactgaacaaatgttagatcctaaaggtcagccggtatatcttgataacgttagtggaggttatacaaatcaatcaacgacaaatggcaaacctaatgcgccagttatggttcagaaagttttggatacaaaagctaacgtgctttacctaaagccctacatgcatgataatcctaacggttcgccaaccataagtaatacttcagcatcgtatttaaccaaatcattgaatgctgctgagtggcagatttatattcagcagttgttatctgatattcataaagacactaacacaccagatacaacagatcagaactttgcagccaatgcgtctggcgttgctatggcttataaactgtggggatctgatcaggaaatgtcaatgtcggaaactctttatcagcgaggtttgagaagacggctacgactattggcgatttattggaactatgtttcaagcacaggtatcaaagttacgaatgactgtaatccagctgacaatgtaaccattacgtttacaccaaacttaccgaagaataaccaagaaaccatgacattaattcaaggtctgaatcaaactggcaagttctctgcacaaacattgcgtgaattagccgaacccattactgggatccctgctgttcaggaacaagaaagatctgatgatgagggagctcagcaagatgatcggaccgccacaataatggcgaatgtacaagctaagatgaacaacggatcgggtgatgatgatgacaacgatcaagcaggagcgcaagaagatcaacaaactgattcaacgggacaaccgcaacaatcagacgattgacggtttttatcagcaggccttaagtatcattggtaatcatctccaagagttttataacgaatatgctgatgataatggtttaactcttaatcaagtgtctcaacaggttaattcctgggatattcagagcttttaccaagcaattgatgaaatgctagctaacgctagtcctagtgataaattgtctaaacgcttgcaagcaatctttgcccaagcatctatttctcggcgtgatatgttgggtgcgatgattggcgccggtatgagtattgctacagcaaacagtgaatcatttgccgttaatgaacttaagcagcagtacatcaacggatatgaggactctagccctaataagttaacaacggttccggctaaagtagccaaccaagctgagtattctcaacgaatttgggtgcatggcgacgtcatgacgacacgaatgaaagaaaccctgaacaagggattgagtcgcggcatgaaaaaatcagacatcaataaaatgacccgcagtattcctcaaagtggtgatcgaattaatgacaatctagcaacacctatgaacaaaatgctatccagaattcatactttaacaacttcccaaggaatcgaaaatacaaactctggcaaaaataaggcttatgatgaacaaaatgttaagtatgttatttggttaacaaaagaggattataaagtttgtgaccaatgtaaagacctggataaacaaatctttatccgtgggcaggcaccaattcctcaggatgacacacatctcaattgtcgttgccagttagttaagtgcgatgaagatggaaacgtgttgcccggtgagctcgatcgtgtatttaaagaataaaaaagtccacatagttttaaactatatggaccatgaatatcagtaatttaattcactcataataacttgattgaggtactgacttgttaataaatgtctcaaccaaaacataaaagttaactcttggatttaccgacaaagaaagacactacggcaacaacaactactgccccaatgattgaaggaacgattgccattccggctaattgaggaccccaagatcctagtatagcttctccaatagaagaaccaattaacccagcaataatattagcaatccaccccattgactttcctttactagtaattgctccagcaatggcaccaatgatggcaccaataattaaaacccataaccaatgcataaaacatcatcctttcttattttttgaaggatgctttttagagtcgttatagttttgaatttctttaaaaatggctaatagaagttgagatatagaaatgataattgatatttttgaccaaagtccaaatcttttcatatgaaatcctccattatctaaattgcatccttctaaatctgattatacgcaactgaatatttgtatacaagttattcgattgtgccgttcttttaaaataggaatttttggattgcctttttctcaattacaggcgttaaagaataatcgatctagttattgcacttacaaacaattcagtctatggacttaaaaaaggagttttgacaatgaaaactaatttgcaattctttgctgatccaagtaatgaccctgaaccaactgatccaaagccaacaactaacgatcctgctcaagatcctaaagatcccaagccatctggtaaaacctatacacaggatgatatcggaaaaatgatggctgctaaagctaaagaagttgaaagtaatctgcaggatgattttgaaaaggagcttaagcaaaaggaacaagaatggcttgaaaaaggtgaaaaacgcgccggcatgaatgctagtgagaaggcccaagccgatttagaagagcaacgacaagctctgaaggagcagcaagatcgccttcaagagaaattagatgaagctgatcgtaagaatgctttagctgcaactaaaactgttctaactgacaagcacattccagctgaatttgcggagtttattagtgatgttaaagaagatgttcgtaacaataacttagataagtttacaaacttatttaacaaagcagttcaggaagctgtcgaaaagaaagttacgggtaatcaatcaccacagaatggcggtcaacaatttaacgcttctatgacacgcgaagattttgcacagatgagcttagaagagcagactaacctttatcgtcaaaacccagatttgtacaacaaacttaaataggaggtgtaggtaatgaccgtaattaacggaaaccctaccaattttagtaatttaattgaaccaacagtctttttagactggatctatcgtcaaaatactcaaactaatcgctttgttcaatctggtgttctaaaaaacgatccagtattaggtggccgattgcttcaaccaggacgatcagttgagatccctgcaatgaatgatttaagcggtgatgcagatgaatggaatgatactaacgatattcaaactaatggtgttgattcggctattgaatacggcattaagatgtatcaaagcaagtcattcggtaatactgactggggagatttaatttctggtgcaagtacccaacagcagattgctaatcgctttggcaactggtggactcgccaagatacaaagattttgctggaaactgtgaaagccacttttaacaatactgatatcgcgactgccaagacttatggtgtgggttctgaaaaagaattatccgcctcagatttcgttaaggcgctcgcccgcatgggtgatgtaatggataacaccttatcgacattagttgttaactcagcagcttattcagaaatgcgtgaacaacaattgattgaatatctgcaacctgctggcgcagctactccaattgccacttatcaaggtatgagcatcattcaagatgatagcattccggttgcttctgatggaactacttatgcactcatcttcggccctggagccattgattatgcaactgctactccgactaatggcctagttgttcaacgtgacgaatttcaaaagggcggcatggtagcaattattcaaaaacgagtagttacttgccacgttgccggaacagatgttgacttgactcaaactaaacctgacacttatttagctgacttggcagcaggaactaagccgttattccaagtatcctatgacccacgtaacattcaattagttaaatatggttttaaagtaggaactgattatgttgtcccaactatcaattcacctaaagctaaagcatcaggtagctcatctagctcatcaaccagcggatctggtaaataggaggtaattagcaatggctgaaacacctacaattgctgatgttaaaagcgattataaaatttttcaaaacttcagtgatgaccatattaccgaaagaattgatgatgcaatcgcaaaagctcagcatgatcaagttagtgatgacgcgttagctaggggaattattgcctggacgcgtcatttattatatacagactggtttatgaactatggtggtgtacagtctgctggtacttttggcaatacccaaactatggttaacttcaatggtgttgatccctacttacaagagtatgaccaagtagttgatgattatggtgtttcagacaatctgggagccgtgtggacagaatgacagaagactttaataatttaccagtcggcattgaacagctggaaaagttgcagagtgtcagattatccattggggtgccctggactaacagtcgtttaaacatgatagctttggttaatgaatatggggcggacgatagcatagcagatgcttatcagagtattaagcctaagaataaagcatatctaatcattccaactaaagaagctaaagggcgtaagcctggagagattgctaatctttttcggcccaagccaccacataatcatgttttggcggttccagataaatcgcaaccttatggaatgcgagtgatgttcatattaaaggatgaggtgcatattccaccgcgtccttttttacgttacacgtttgaccactaccttgataattggaccgaactagcggctgatttggcatttaaagtatttgttggagagataaattatcaggacgtttttcctgttttaggcgatgccgttgttgaagatattaagcgaactataaaagagtttagtaaacccaaaaatgcaccgttgacaattgcaaacaaaggatttgatgatccattgattgaaaagggcgagttacgcgactctattcattggattacagaaaggatttgattttatgagtaaagaattagttgttgtagaagctgctaaagacaatagcggagcttatgtaaaaccggaccgtagcacagaaacatcagacaatattgcatttttgcctagcacttctgctccctatgtggttcatattattggttatgatgctggcgatagtgttcccgatggaaaatactatgctgccttttatgatccggatacccaaaaattcttaggccaatttattgctgtaccaggatttaccgttgcaggtgaatcaacccccggtaatgttcaagtaacaccaacttctgtcggtggggacgtaagcttgagtgatcagagcaccgcccaagcctcagatgcaactggtacccaagcaactaccggtaagtaatcatggcgtttcagaactttaacaactttgcttttatgaatgatcagttagctgaagacctaacgattactgttattggaaaagataccggtgaaacagatgatcttgggaaaccaattatgggaccagatgaggtctatcacgtttccgaagttatcactaataccactaatcctaacatgacgtacagtcaagaagatggcggacaattaccggttggtacgttatattggttatctcatatggtagcttgtcctaagggaacgctcgttcaacgagctagcggggctaagtatgaagtagtcaatcatgcggacgatctatctgctggaatgacttactatcagataaaagaggttggtactgatgagtaacgatttttatcatgctttctcggccgccttggttgtcgagattaagcaatatttccctaatgttcccgtacgtccgcaaagtgtcaacaatgcttcgccagcgtatccctatattacttataagatatacgatgactatgatcgggtattgtttaacgatgtggaaaacgaaacgtttgatttgcatgttcaatttaaagctatttcaaatgatgaaatggaagctaaatcattaggacatcagttacgaaaattgttttttctacagcagcctgaatatgatttgcttcaaaaaggcattgtggctaaagactgtgatgctattccaccagttgatcaatatttagatgttgattggcaattcacggcgggagctgattatacgtttggagttcaagacaacttcactgatcagacgcaaacaggaaatattgctagtgttaatccagaatttaatataaaaaaaggagctgaatcatagtgtcagatattgttaaacaaaccactgatgtacatttcattgtcgctattcatgccttaactaatccaaatagcgctccatcagtagcaattgctacaaaaaataccgatgccactaccaagagcaacatttatgatgacttagatagtttatcggcagattatgcagaaaacacaggtgtctatgctcaagcagcagctatgtttgatgttaatggctttaatgggcctgttgaagttattgcgtgtccgaatgtggattccaatacaccttcaggggttcaatctcaaggaacaactaccggtggtacggttacggctaccacaacaccgggaattgttgttggaattgcccagcatctatttgatggttttaaatatttagtacttgacggagcaaccgagactgagatcgaagcgctttctgattttctatatgacaaccaaagaattatgttggtaactcaaccaaactcggttaccgcactgcaaacgttagcaactcatgttgctggctatcaaacagtaaagaaccagttaggcaacactgctgcaattgttgaaacagctacggatcgctaccctgctgctcaggcagtagcgtacgccgctgctaacttaccagttgattttcagcatattggtaatctttcacagtttgaaccagatgctgatttaacaaccgatgattatgatacaattgctggcttgaatgccactttggtcgttaataaggctggcgattatatgctgttaaatggtaaagcactcgctggcaattacattgatcaatttgttcatactcagttagtgattgatacattgcaaactaacttgcagaaatatcttaaccgtaaaaatttcccaatttacaatgatgcaacaatcaaagagatgacacaaactatcaacgccgtcagcacaagcctattacaaatgggtgtgctgtacacggcgattgtcgttaatagtgttcctcgagccaacgtgttaaacagtgacgttgccgcccgtaaatataatgggtttagtttgaacactcaaattgctgatgacattaatacaattaatgccaaacttgatttgactttgtaaagggagggaaataactaatggcaattacattatccaatggtaaagaagttaacctatattcggctcgtttccttcacatttatttgctgtggaagaatcaatctaaagagcttggcggttttcaaaacggtgaaccatttagctcacagagaacaaatgctgatactactatgcaaggcgattttcattcgaatgttatgttctttgatacagaagatgaaactggaacgattaccttaaacacctacccaggaacatctacgacagatattctgttctatatgtatcatgctcagcatgacttaatggaagatggcccaatgaccgctgatgatttgttcgggttgaatattgttaatgcatcaactggagaaaagattaccgcagaaggctgccgactcgccggtttgccagctaaccaaggcaatgaagcagcatattcattggcttggacggtattagttggttactatcaaaacactggtaaccagccagacgattcaatgttttcttaaattaaaatggaacagggggctaccgctgcggtggccctctacataaggagtaaattaaaatggaaaataatgaaaaaaagctcgaagccttgatgggcaatgagattcataaaacggttgaatggacagacgacaaggataaaaaacacacaacaaagatcactttgcaggatccaggtattggagtagctactcaaatcatggatttaatgaatgtcggtggcgataattctgattacggtaaggcatttgagatgttgatgcaaaacgtcttggttagtccgcatttggattatggcgttttgaatcatgaactgccagaaaaattaactaagaaaaccgttattaagcaaaatagcaatggtgacgatgtaaagattaatatggtctttccggattatcgaacagccttacagatcttcatgatgactaaccgcccttctggggcactcaatatgcacgacaccctggtttctcttaacaaggaagttttgcgtactgatgaaaccacaccggaaattgttaagatgaagtattggaatattggtgaacatggttctggcttgggtgctactgctttaagtgaagcacaagcatatcttgggacgctattggcacgaaacggcctgctaaatattttgatggaatcgtttcgctttcttgcaacaacgttacgaccaaagtaattccaaatatgttaatgaatttggtaaaatcgatgatcggttggcagaggatgagatcaataaagattttctggttatgtcaactgaattaggaattagcgaagatcagattaatttgatgacccaagatgagtatatttttaatcgagctaaagctaaattagttcgacaagaaaaggaatcggttattgcccaaggtgtgtattacggcatggctaaaatattaaatgaaatgtttgggaaaaagaaaggaaaataaatggttaaagtcaaaaaaatggagcagccaattcatttggatgggaaagactgttccagcattaatattgtcgataaagttcatggcaatgaacttatcgccagtgtttcattcaacgatgtaattctgaagaaaggctacagcatcgtatttgaagattaaccgagattattgtttgttgttgaatctagttttgacagaggcaagaatttaaggaggcagagtatgatgtgcaaaaaaatgcgattccagaaagtaaagatttccaaaatcacaaacataagtctatttttactgggttaacattcaaaggcagtcccgtttccaagcaagagtatgaacgtcattaccaagaatatgttgcacgatgctctggttagggcccgaagttagtcaacaaggattttgaacgagcttcgtgggagtatgcattagagaattcgacgatagacattgtagctgaaagaaggtgagcaaatgagtgccaaggatgatgtaattatggagcttaaacggactaatcgactgcttaggttattgattctaataaacgtatacggaaacgaaaacagtgttctagatagaaatatcatgaatagtatcaagctcctagacaataactacagtgccaaaactctttttgagagcaaaaaggagcaggattaggtcccactcctttccacaatgactaatcgataattcccttatcgcgcaatagctgatcttgctcttcaaatgataagtcagcatcttcaaaattgccctttggttcttttgcgttatgcacttgagcaattttgacagcttgctcgtagaattctaaagcatcttccagagaaactttatcctttcttgaagcaagaactgcgttagcaaacgaatccggatttacaaaagccatttttatcaccacccttcgttggaataacccaattatcccactaaggagttcaacataagcaaattaattagaaaggaggtaaatagtaatggctgaagcaaaagaagttcgtcatgcgggtattggccttgatctcaacatgaatggcatggatgatttcaaacgagctaacagcatgatggatgatttcctcgagacaatgaaagaagcctcacgaattactgataaattcaaaaataattttagtggctttggtggtaagagtagtgacgaagtcagaaagactcgtgatgcaatccaagacgtttatcacagtatggattctgcaaagaatgaaacaaaccaggtcactgaaaatgttcataaaatgcagcaagaatttaagtatacgagtgatgccgccaaaaaaatcaagctgaattcaggactgaatagcgatattaataagagtgctgaagaagttaaaaaattggcaaaatcggctgaccaatcaggcaataaatttagtgaaatgtttcgaaaattgcgtagtggatcttctgagtcgaacggttcatttagtaagttacatgattcagctaaaaaaacatttgatgaagtccataaggggactcattttttgagagatgttgtgacggccagctttatttctaacgcggcaattaacacttggtattctttgaaatcgggaatagggtctgcacttaaagcgggtgaagagtatgacaaagagcaacaagttatgcatgccacatgggacactttaactgattcatctgttaaaggtaatcgcatggttaaagctattaatagcatgtcagtttcctttggtcaatcagctggattagtgaatgagttgaaccagcagttctatcacgtcctagacaaacaaggcccaactgatcgtctgaccaagtctgttttgacaatggctgatactttaggcatgggtgctgaaaatacaaagcgcttagggctcaacttcacacacatgatggcttcatctaaaatgcagttaggtgacttcaacatgatttcagatcagttgccaatgtttggatcaaagctactagcctatgaacgtaaggcaatggataattcccatcttacaatgagtcaattgcgaaagaatatgactgctggtaagatcagtgccaaagatgccgaaaatgttatgaattcattgggcaaaaaatatgctgaggcttctgaaaacatgatgaaaactcttccagggatggaacgagttatgtctgctcgaggagcagcgttatttggtgcactcgaaaaaccttttatgaaagcgaagaatccaatctttggcgcaatctctaagtgggtttctgacagaaagactgaaaaggaatttactaaagttggaacagatgcttctaaaggattaaatactattacgcaatcttttgctaaagtatttaatcctaaagaaagccctcatttggctaatgatgtgatgaatagtattgctaagggtgttaccaatgtttctgatacaattgctcaccatgctaagtcaattgttgagttctttaaaagtttatactataccgttaagattataaaggatattagtgttggttttgctaagggcctagtttcaggattgagtgccattgtgactccaatagggaaactagctggtaacagcaaaaagattcataacttttcagatgcactaaaaagtattactacccataagaaaggtttagaggatattggtaagttgttagctggaatttgggctacatcgaaagctatgaaaggggtctctgcaacaaaaaactttttagggtttggcgaaaagagcggcttgattcttaaacctagagttaatggaaaaagcggtgaaaaagagttaacgttatttgcaaaagcgattcgaggtactgctagaggaattggcaaaagcctcaagtggactgcaagtattggttggaaagaggccaaagccgctaccagaggattgtgggcagctactaaagcaacaagtagagcaattgacaagagtcttaagtggacagctaagcttgcttataaaggtgtagttaaaggattatcagtcattaagacggctgccattgcaaccggaaaaggattcaagctggcgtttaacttcttaaaagctaatcctttcatcgcaattatcacaggtgctattgccgttggtgcagccttgtatgaattatataagcacaacaagaagtttcgcaaatttgtcaacggtttaatttcatgggctaagaaagcttgggaaggcgtaactaaatggtttggaaagctagccaatggcgttcgtaaatatattaattatttggtcaaagatgtcaataagcgttggggttggctattcaaggatatggccaaaataattaaggacgcttggcgtactatcaagagccttattcaagtaattgttgacgtgtttactggtaaatggggtcgacttggtaaagatattggtaagctaaccaaaaacttttggaacgatgttaaagatttatttaagactgggtttgattgggtgaataaactaaccgggggtaagcttggcgatataattagtttctttaaaaatgcttggaaagatatcggcaagggatggaaagatttctggaatgggattgatgattggtttagtaatctttggaaagggattgttaagcacgttcagaatggtatcaacgacatcataaaagttctaaatgatggcattggtttaattgatggagttatccacatgtttggtggttcaagtacagcaatcggcaagattggctacgttcactttgccaatggtacaggtgtgtttgggaatcaacgccgtgagattactaagccaactttagcaatgctaaatgatggccacgactcacccgaaaccggtaatcgtgaaatgctgattcatcctaatggtatgagtgagttgattaaaggcactgacgttaaacgattgattgaacccggagccgaaattttgaatgcttctgaaacaaagtttgccttatcactgaatggaattcagcattttgctactggtggactatggaatggcgtcaagaaagtcactggtaacctatggagtggtgctaagaacattggttcatcggttgttggtggcgttgaaaaaggaatcggagcgattggtggcttcgctggtggcattcttaaggccactaagaaagtatttgataccgttaagtcaatcgttaaagatccaagtaaatatttaactggactgcttaaaaagccatctggcaagggaactgttttatcagactttgccaatggcttttttggtaaggtgaaatcctcggctactaattggtggaagtctctttggggaatggttaatctggatggaggcagtggcggtgatgctaccggactactggccgccgttgaaaagtatggccgtggtaaaagatatgtttggggcgctgcgggtcctaacacatttgattgttctggacttgttatgtatgctctaaaacatgcctttggcattgattatccccacttttctggtgctcaatacggtaaaacgaagcacattagtcgttcaaacgctaaaccaggtgacttggttttctggggccctggtaaacacgttggagtctttgctggtggaaataaatattggtcagcatttgcacctaatggccatccagatattggtatccattcaatctctggttcagtaccaggatatagcccgctatttggtgaggttaaaggactagcaaggaagactgcttcaaaaggtaaaaaatcagcttctaatagcattcaatcgctcattaagaaacaagttggcagcggattcttcaaatttatgtctaagttagctgataagtttggcgataatggcgatatgggtgccgttggtcttgctggggatgagagtcaacgagctagagaaatagcgaaagcccttaagcaagcttatccctctgctactgatgccggaattgctggtattctaggtaactggatgcaagaatcacgcttaagtcctaaagcaattgatagcgctgatcatggtactggattaggccaatggacatttactcgtgaaactggattacgtaactggttaaagaaacacggttatgcttgggattctgccaaaggtcaactggaatacgcacttcatgaacctggcgaatctggagcctttaaagcagtattaaggatgactaatccagcagaagctgctagaaagttcttcgctggttgggagtcaggcggtaacgaagacgcaaccggaagaactcgtattagcaacgccgaagccgcatataaagcaattaagggacacgctaaaggcggtcgtattaacaaagatgagctttcggttgtaaacgaaaaaggatgggaactatttaaacctgatacgggcggcctgatgatcccacatgaggcttctgaaaaaattattaatggcaagaaaactgcgaccatcgatgcccgcactaatgtcactatccaaggtggcggaaatatgagcgatagtacgatcaacaagctttatgaagtgcttaataaagcgaatgatgaaaaggttgccaaatttcgtcaacaacttggctttaatgatgaaggaggacttccggtatgaccaaaaaatcagcaacgcattctgttaaaggcaagactttaacatacttgcaaaagaaatcaaccgaatggaaatcaactgtcagcaaagatgctgaccaaattgataatgctaaaagtaccattgataaggctaaggataagttagacacttacgatgattatttacaaaagcaaaatgggtataacagtcttaaagatgcctatgacgctaaacaagacgaaattgataagcaaaataaattattgagtaaaaccaagaaatcttctaagaaaaaatcaattgagtcaaccattaaagacctaactaaacagaaaaaagaagtctatcaatcaattactaagcttaccaatactgctgaatatcaaaagcagttaaaagctcgcacaaaagccaatcatgctattaatgttgaaaagaaaaagattaacgatattaatgcaaaaaagacgaaagataagaaggtttatcagacttatcacaatgcttatgttgctaataaaaaggcggaaactaagaagaaacaaactcaaaatcggtctaaaatcaatgatgaaattgctgctgccaagaaaaaatataagatacacaaaggtgtgtatcttaatggactaacaacaattcagcgagcagacgcaatgactagtcgagtttatatcttaggtgaagcagatccaaccgaaactgatgagcaggatgtgccgactaatgctgtagatagctcagaaactcgaactaattacagtgttcgaagctccaagcaactatcaggaacgtattatttatttggcaaagctagtgatttagattcagagtttagcattttacaaggttgggctagaaagggcgttgaggttacagtacgtggcttttctaagtgggcacacgcttacctgtcttctgttggtaaaacagctaacacgacaggtaacaagaactcgttgacactatcaataacctttacgtatgccatgaagtccaaaatcgattatgctaaaaagaaatcaaagaaaaaaactaagtcgtcaagcactaaaaaaagtggcaccaagaaaaccactcataaaacgacaaccgttaaaacagggatgacctattggtcaatttcgcaaaaaacgggagtaaaagtttctgagttagaaaagttaaataagtggccagctaattcgatcccagttggagcgaaagtgaggtatgaataatgccagtacatgattatattccggtatcaccagatgatattccttatcagcaagagattgatttagactcaggaaactatttatttggattccagtggaatgaaattgatcaatcgcttacagtagatatttatcaactagatggcacaccaatctggcttggagaagtggtcactttaaatcaacctttatggcgcggtataaatgctccaggacttccaactgaaacgattattccaatggatgagtcaggaaatgaagatgagattgatcttggaaacttaggcgatactgtgcagttatgtattgatgatattccggatggtgaggattaatggcagaaaaaactacaaacaagggttactattggggatattcaactactttagttattaaccataatggtaacaagctaacactctcagaaaagaagggcgtaccaatcaactatgatattccctctgatgatggtggtagtcctgctacctgcacggtaaccctatttaatttatcaaaagcgcatttggccaagattaatcaaaatgaccacatcattgtttacagtgggccgacttatctctacggaaaattaaccgagggtactatcacacaaattgctccagagactcaaagcggtatggataaggaaactcagataacttttgaagaagggcgcgattattcaaaagataagcgcctttacagtaattttaatggttcgaaaatggtaactcacaccgttaaagccagtgatggaaagtcaatttcatacaagaaacgaaagatcagcaaagttaacattacgttcaaaaagggaactaaagccagccaaattattgatcggattaaacgtgaagcaaggattgaaatttcagaaattaatttaaagaaaaatcatgttttcaaaaaaggatatacattatcggctaagcctttagctgcaattcaagcaattgtaaaagattgtgggagcacggtttattatcgtaaaggtgctttatatatcgatgatggcaataagcctaacccctataatgagcatctatatctcacgatgtaccatggattgacacaagaaccaacctataacagtgatgatgacggtaagccgacatggactttagaatgctttgatgatccacgggtttgtgccggatcagcggtttatgtgaagtcgaccaatcttactggtcttcaaagagtaaaaagtgttgatcatactcatgaccaggattcttataaaatggaagtggtagtttatgcctaagaaaagaaaagtcgcgattgatgccaaaaataagcaatccaattttttgaaaaatgaatttttggaattttttaagtcagaaattaattgtcatacaattggacgggtaatttcatatgataaggctcatcaccgttgtgatgttcaaccgctgccacttcaatcagatggtgataaacgagcggctttaactgaagttgttgttcctgcatcagtttggcaaatggacaccttctttcaaaaaatttgtactaataaaaatgttaatcttaatggttataagccaatggcaattagctcggttgtttgggttggcttttgtgatcgtgagatggacaattggtctggtaaaagcaactacaaaatcgataccaaaagaatgcattcgatacaagatgcggtgattgaggcggtgattaaaccatgattgcatttggattagacagcactggtgatttggattttaacccaaacactggtgcttttaatatggtcgaaaatgatgatgaaattgctcagaaactcagtttactattgaacattaatgttgctgaattgctttggaatgaagatattggtcttgatcacaacgaattacttgctaatgcagatgatcaagggattattcagtcaattttatctgactatctgcaagaacaatggcctgatacttttgactcagttgaaattactaaattcaaagctaatcaacaacagcgaattacttcactggaagcaacggtcacccttacaactggtgaaactgtcacgagtaatgttagcgtcgatgatcaaggagatgaaaatgatgccactaacagctaatggatatgatcgtcctgaactagatgatctacgagacaatatcaatgctatgtttatcaaatattttggcgatggtattgatctagatgatgagcaaacgccaggaatgattgctggaattttatcagaggttgatgacaagttggaaagtctggctcagggagtttataactccttttttgttttaaaaagttccggagcaaatttggatgatttggctgctgaaattagtgtttaccgtaaaccggcaaccaatgcttatgtgtatttgcaaattgatggttatgtagatccagattcaccaactgtcattccagaaggaactcaattttctaccccagatggtcaactgttttcaaccttggcagacattacgattactcaacaagcaacatatgttgatagtggtggaaatacacaaccattgattgatgatgatggtaatcccttgggccggcaaacagttcaggcggtagctatggataccggaacgggctcaaatgttatgccagcaactattgttaatccagttaattcaattgatggcttttatgcagttactaacctgcaagcagctacaggtggcatggatgcagaaactgatgatgcgctacggcaacgaattttagctaaccgtaaaagtgctgagaatagtacgcctaatggcattcaaactgccattaagaatttaactggagtaactgatgttcgtttggtcaataataatacaatgagtacagacagctatggaaatcccccaaaatcagttcatctttatgtaattggcggtgatgatagtcaaatttctcaaaagttctttgatgttttacccccgcagactaatactattggctccgtaattggtatggcaacggacgtaggtggtcgtcaatataccgttttgtttgatcgagctgatacggtaccgatttatattgaattagatttgaatgttaacagtacggtttttgatactgacaatgggccacaagccattaagactaacattttaaattattttgatactctcaatatgggggataaagttctttattcaaaactatttggacccggatattcgcctgctggtgtgactgatgttgctgttaaattaggcacaaatgctgatacattggcagaaacggatattagtgtcagtgattttcaattagcggttatcagttctgataatattacgattaacgtgattgaaaactaaagaggtgtgcaaatgtatcaaactgaaacggatttatccgatagtaccttacgaaactggttagtttcaatgtttccggcgattatgaatcaggaagatgaatcaaataatcaaaacttattaaatttgattgctgatcttcttaatgaacacaaaaatgatttgctcagtatatcagatcaggttttgttaaataatgcaagtgggcaaacattaacagatattgctctggactatggcattaatcggctagatgatgacgatgattttttacgatttcaagttcgtttgcaattgttggaaaaccatatgggcattacaactaatgatttaaaagccttgattgcaacagttttaaacattggcacggatatattcgatattaacggtactgataatccagaagaagtcgaagtgaccaatattccctttgactttaattcgggtgacaaagcagaggtcaaacgtaaaattttaactaatgctattcagtcaatgctaccaccggaatacttattaaaagatttgcagtatgcaacgacggttaacaatcaactttatatgggagttcatgcccaattctatccacaaattactgttaaggagatggcttaattggcaacaccaaatgtaggaattttaactaattccggtaaggccttaattgatcaagttaatgctggtcaaactcaaattacttttagcaaaattgttttttccagtatggataatagtcaattaactgatgatcagataaaagctttaactgcaattacaccacaagaaattgtagttaataacccagaagttactcttgataagaacactggcgaaactcgaattcgagcaactggtaataatgaagcattaactgatggcgtttatgttaaaacttatgctgtgtatgctaaagatgattcaggtaatgagatattatatggacttacgatatctcctaatcctaattacttgccagaatatgatggtgtaactccgcaagcggttacttattcatacaaggtcaatattagcaatacaagtaatatcacttttactaattcaaatgacatttatgtttcagatactgacttagcaggggcattgcaaccttacgccaagacggttgatgttaatcagcagctggataaaaaagtaactgacaatggcgatggatctatcgtagtcaacgggaagacttatactccggctgacgacagtcaagttgtgcatgcggccgacttaccaagcttgattccagccactacggctgataccgctaaaatggccaacttcacaaacggcttacaatcaaatagcagtccagttattactcaagcgcagtgggttattgaggatagtgattccgatgcccagacggcatcaacaaacgatgctagtgggttctattacacggaggaaagctaatggcaatttatcacaatggcaacaaaattattagcttgtatcacaaaggcaagaaaattgaatctgtttatcataatgggataaaaatatactccagtggcctaccaataggaacaattttatggtcaggtagcaaagcatttgctataaatgatccatttggtggtggttatgatgattttaataataattttcttgtaaacaagaaaattactttgtccaatgcaattagtaaatgccaaaatggaatagtagtgaacttctcaaaagcaatatatatttcttctgctggagttggttttgataatagttatagtggaaatattcacttgcctaaaagcttttcaaatgggcaaatatatgcagagtctggcttaacgataagacttattaagagcaatgattcaactgtatatttcaattcaacggatgaagggaacaattcaacctttattggatataaaaattataatgatgcctatctttacattgacagtattaccgcatattaatttacttcacaggttatctgtagtacagaagtaaagtatgttataatatctcacgtggataacagcgcattcactgttgttattcatacccctcgagtgtatgttttcctcagaatatacgccttcagtaatatctatattttcttttcatatatcccccaaaagtatatgaaaatgcatctatctacggataggtgcttttgttttgcccgaaaactttcaaagaatgttataatggctatgttgagggaccgacttatttggtaaagatgattgacaattcaacttacacggtctctcagcaggctttgattcaatacccaggatcaaggcttttttagtttcatatttctattaataaaattatgtatatgcaattagccgtctatgaaaatagatggcttttcttttaccccaaaatagaagggaagtgaggccatgcctttaagcgatcaggatcatcaaatgttattgaaacatggtaaagaactatcggatcacgaacgtcggattactgatcttaacaacaaaatgactgacactttaaagagtgttgatgaaagcaacaaatatttgcgggaacaaaacaaccgtatcttggaagcggtcatccgtggagacgagaaaagtgaaaatcataaagacgagatggaagttatcaatcgtcagaacttgtggaaggtggttaccattgcgattggctcgagttccgtgatttatttgattctacaacagttaatgcactttattcattaggaggaatttaaaaatgttaactaaaaagtatggtacagtttcaattttgtttgctgcaaatgttgccgatggtggccggacgattgatgaagtaccgacaccatttaaagcggatgttcaagtattactcaaaacagatgaattatcaagtgaaccaaccttaccagcagcttcaacagattctggtaatggttttgcaaaaaatgatacccaggaggtggccaaataatgttcgcaattttaactaagacttttaactatttacaatcaactggcgttttggctgcaggaattgcttttattctagccgtttggaaagccgctttgccacttgctcaagcacacgctaagaccgcccaagagaaatcgcttttaaccgcgattgaaggactagttgccctaaatgcccaggtagcagcgttaagtaagcaaggccgttttgatgctgtgcttaacggagcattaacttttgctagtgatcgtggttacacgtgggctaagtcagacttgattaaaggactcattgaaggcatttatcaagagtacaagcgttcaggcaaagatattgcccctgttgctactactcctagttctgacgttgttgaagagaagcctgaagtcgatgctcaaccaacaaccgataacacgaatgccacagtagatacttcaaaatcagatagcaccgatactgtagaaagtgacggtgcaagtgatattgcaaaattggaaggtgaggttgagaaataatggcttattcaattatcgttgacacgtcatcatatcaatccgattccttttcattttttaacggcttaaaatctcatggtgtttctggtgcaatggttaagctaagtgaaggtgttaaatatacttcaccaaaggctgccaatcaaattgccaatgcttataaagcctatggcgttgttggtgtttatcatttttggcattatggtactaatgaagctcaatatttcctggataaagttaaaaaaatgggcttggacaaatcaacgtggctggcacttgatgtggaagccccagatttaccgcaaaaatgtactgctggcatcaataaatttctaggctatctctatgccaatggctaccacaacttaatggtttatggatccacttcatggtttcaggaaggccggattaatcaagcaaagttgtccaagcatgctaagttatgggtagcggcttacggcacttcacaacccggaattaatcatgtggatatctggcaatacactgatcgttttaaaggaatgtcgcttgatgctagttatgatttcaaaggattattaaagtcaaacggtaaatcagacacaccaatcaaaccagaatactatgctactaaaggcctgtatgaagttaaagctgatatggtgcatgcgtataacaagttgccccttaagggagataagaacaagcgctatgtgcgtttcgctaagggtagtcgcttctatggagtcgcagttaaaaatggtgacatctactccctcaaaacgcaagttggctatgtaacagccaacaaggattacgtagacttaatcaaagaaattaaataaagtatgcaaaagggcccactcagattaagttctgggtgggcttttttgttttgtctaaaatattatatttaagttattgcgacaatcataaccgatatgataattttggaatttcaaccattcaagtgtacattcctataacttaaggcatcaattatgtaaaagcatgaaatttgccactaatttgccattcttatgattttaattcagatagtggcaaatcagtggcaagggttttgtatttctatgtttttgagagaaaacaaaatccctttaaatgcctttatatcagcattgaagggattcctgtttttccatatcactcaaataatcacccgcacggggctcgaacccgtaactccgccttgagagggcgacgtcttaaaccagtttgaccagcgggcaatgctatcaaactcactataatagtgtatctaaatcagaaagatttgtcaacaaaggaaactgaaatataaagttgacaaaacgcagaaaaatctttaatatatttagttgtgatattcattgggtattcgccaaatggtaaggcaacggactctgaatccgtaatttactggttcgaccccagtatacccaatcttttgcaaggtctgttatgtttctctctaatcagagacaatgtaacagacctttttatattccataaatcccactatcatcctgtgcagaaggggatctttaaccgttacccgttcttactcgtcccagattggaattgcttacaccacagtgacccaaagtgtgctaatctagaattaaatggttaatgattcacgcatattcatgcagataggagccgatatgtatggatcaatttacgttagtcaaagaaacgctggataagatgggaattccctatgagattgttgaacatcctgctgcccacactactgaggaagccgatgagttcattaagggcaaagagggcgttcggaccaaaacaatgtttatgaccaacaagaagaaaaccgagttttatctgttggtgatggacgatgccaaacgtctagactttcatgaatttcaagacttgaccaacactaaacagatcaagatggcctcagcggaatcacttaaagaacaaatggggttggagccggggatcgtctcgatttttggattgattaacaatcaagagaagaatattcatgtttatttcgatcgggccattttagatgaaaagacaatgaccttccatcccaatgtcaacaccagaacaatttttgttgcttccaaggatgttttaaaattcgtgaaggaaatgggctatgactaccagatccttgacttggaatcctttgattaatcagagaggttacgaatgaaataccaagatgttaccaactatgtgattgaaaaatatcatgttcaccctgaatacctgtggaaaaagtatccgagctttgccgttctgcgtcacaaggagaaccgaaaatggttcggcttagtcatgcaggttgaaaagtcgcaacttggacttgatgggcagggtaaggaagacatcctggatgtcaaattggatcccaaagaagttgagtttcgacaaactagtttggggtttctgccagcttatcatatgaacaaaaccaactggttagccattcggttgaaccaggtggatccaaagcaaattcacgacctaatcgaagctagttatcagttaactcaataatcaaaaatgaggcatccgccaaggtaaattgttccttggagggatgcctcattttagtgagggtttatttaatttcatagtaatcatcggccttagattttaactgattagtctcaagcttgttgagatccagcttccgcagcgtctgtttggtaaccatggttttgacaatggttcgtttccgaccgttgccaacatttcgattgaagataatggtgaattgatcataacggtcatagtcggtctttttaatcgccttcaaaataccaatcgtggttaaccgaaaggactcggttgtatcgcttttatcggtaacggtcactgtgagtgccgtctggctggcatgcagcttgacttgatgatcaaatagaagcgtatgggtggtgttcagttctttcttgacggcagtttcagtattttgagtcgactttctggccggctttttcacggtcttttcggtccgctcagcctgctcggcattgccttttttgatgacttcttttcctttgggcgaattaaaaaacaacgtgccgaacacagccatcagcaccaatgaaatcagcgcatacttgccgtatggatatttaccgtgtttgccggtggtcttaaagtagacaaacatggcgaaaaaaatcaccatcgcataagacgacagcttggtaatgacatcaaacatcgtgctaatcaaagtgaaggtctcctttatttggctggttattcaaatgaaggtcaaccaggtatttgtgttggtctactaaatgcgaggtggtgatccacaattcgtgataattggcgtctttgacctgggtcatctcatgaaaatagtccagcaaatcactgtacattgacagaaaatctgacgacattcgattaacctcgagtttttgttcagggaaataaatctctggatttcctaatttaacggtgtcatcaaggtacatttccacgacgttgtcataggtgtccggcttggtgaatactttatccggatgggccttaatgtatgataagacgtgataaattgtgtctgagttacttgccacttgaacttcctccgatcttaaaaatcctacgttcctattgtaacaaatctgagcagagtggggaaaatgttttcaagcaaccgccggtgcgcttctttatccagttgtggattagcggtacaatgaatgcatctcaatgcgaaaggatgctgtccatggattatccaaacacggtcacaagaattcatcagtttgtggatgccggaattgtccccggcgtgagttacgggattattgatcgggatggccttcaaacagacgtttttggtcaacaggaactgttaccggaaagattgccgcttcacagtggtgaattgtacgatctggcctccttgaccaaagtgattgggaccaccaatttaattttacgactactggcttccgggaaaatctcactagatgattccttgaccaagtattttcctcaatggcagtcgccccaggtcaccatcagacatttgctgacgcatacctcagacattgtcggctatatccctaaccgcaatcaactgcccaagtcggaactgatgccggcgttgttggccctgaaaagcggttcagatatcggcaaagttgttcactatcaagactacaattttatctttttaggctggattgcctcaagggtgatgggcgagcctgttcaacagctgattagtgagtttgtgttaagaccgttggaactaaaccaagcgacattcaccccggatcaggttaataatgttgtcccgaccgaattaattcccagtaaggggttgatccgcggcaccgttcacgaccccaaagcgcgaatccttggtcctgactgtggctctgccggcttgtttgcgccgctcagcgatctgattcatttttcaaagtggttgttgggcgatatcagatatcccaactttctgccggcagactgggttgaccagctcttcgttgaccaaacgccgggacacatgaagaatcgttcgtttggctggatcctgcgtcattataatggtcatccatacattctccacacaggctacacgggcaccctgatcgtggtcgaccgctattcgcataaggcgttggtctttttgtccaaccgagtccacccggatccaagcaaccagttgtttttgccatatcgcagccaactgattcgaacctttgtgaaagaaaacgagattgcacaccaataattttcagacaaaataagcgtgggacaataagcggttagcttccagagtataaggggattacccgaatatccagaacttggatgtttgggtaatccccttatacggccggaagctgcttattggcgcacagttctgctagataacattcaggcgcaaatagaggctggaacaaaatttttagttttgtcccagcctctatttctatattaaaatgttgcgccaactttcagattctcttgtgctgttaaatcggcgtcaggatattttcgcttcagcgcgttcatcaaaacgtgtttagcaatatcattgtttctggcaagaattggaccatggaaataggtgcagtagacgtttttgtaaattgccccttcagtcttatcctggccgttattgccgtgaccctccagaacctttcccagtgggcgttcaccgcgacccaagaaggtaattccctgatgattttcaaagccgtgatacttttcgccggtttcttcattttcaatcacgacgttaccaataaaacggtggtccttttgtttgtcggtatagtgatccaatgcaccgatgcccatcagcttttcaccgttagccccgatatagtagtgacccagcaattggtagccgccacaaattgcgaccacggagccattatcttcaataaagtcggttaaagcctgctttttggtttggatatctttagaaataattgattgttcgaaatcttggccaccgccgaagacgacgatgtcatatttgtcaggatcaaatggttgatccaagctgacaacttcagacgtcaggtcaacgcccattttgttggccagatacttgaggaccaaaatgttccctaggtcaccgtaagtgttcatcagatcgccgtaaaggtgacagacgtttaaagaataggtcattaatccattcctcccttgataaagcctttggctgcaaatactttccttaagtgtagcatagccgtgtaagttgcgaggatataaacctttttggttggtgccttggggatcatttcgacaactttgtccaaatccggttcaaccaaatgtttctttgggtcgactccggcaacttggaggcggtaggtgatatctttgtatcgctcaccgccagtaatgaactgtttgatgttcatcttgggcagccgttcaaaatcgccatcccaaatccagctggtatcaatcccatctgcgtaattggcattgagaagcccaatgaaggtaaacgggtccttgtcagtggaaatcatgtcgatcacctgattgaggccgaccgggtttttaaccagaatcagtgtcaccagtttgccgtcaacgttgatctcttcttggcggccaaagatctgttttcctttttcaaaggctttcttagtctgagcaggggagactcccatgaatcggccaactgaataagctgccagggcattgtagatgttgtaaaccccaccgatcccaattttaatcggctcaccatcgatttcaaaggtagatgatttgggggtcaagtcgttgattttgttcagcgcaaaattcaattcgggccgctcaaaaccacagttggggcagaagtacttgcccagattggaatagctgatgaaatggtagtgcaggacatgctgacattggggacagagaacgccgtccgtgttgggcgtcgccttgatgtcgccatctttttgattgtcgaagccgtagtagacgatcgggttcggcagttgttttgaatggaaaatcggcgcgtcaccattagcgataatggttgcgttgggcgctaaggcgaccccattcaaaattttattataggtcgtatagatttcgccataacgatccatttgatctcggaaaatgttggtgaaaacaaacgcttttggtttgatgtatttggtaaccatgatgacattggcttcatcgacttccaacactgccaatggccgcttgccctttgactttggtgcatgaaggaaagtggtaatgatgccttgctccatgttcgagccggtggggttggtcaaaatgttatcgtacttttctttgagcacttgaaccgtcagagcggtcgtcagcgttttaccgttggtaccggtgatgacgatcacgtcgtagtcacggcccagggttgccagaatttctggatcgagccgtttggtgattttaccgggaagcgaactgccgcccttgaaaaatgtatgcagaaaccagtaagacgacttaccggccgcagtcgcaattgaactttttaatgacataaactttactcccttaaaatgaagtacataatgaacctaatcaaacattaagtgtagcatatgctcaactgtttgaacatatatacgctcgttctttaaggggtcgataataatgagggtgctggcgaattttctcattattatcgattttcaaaactttttctgtataatggaagagaagctcttaaggaaaaaggtggatattttggctcaactattttatcggtacggtgcaatgaatagcggcaaaacaatcgaaattatcaaggttgctcataattatgaagagcaaaataaaagtgttatcattatgaccagtgcgttggacacccgagaaaagcagggcatgattgaatcgcgcatcggtttggaacgaaaagccgaaccgattcgcgaggataccaatgtctttgatttggtacaggaactaaatccccatgccagttgtatcttaattgacgaggcacaattcttaaagaaaaagcacgtcatggaactggcccggatcgtcgatgagctgaacgtgccggtgatggcatttggcttgaagaacgactttcaaaacaacttgtttgagggttccaaataccttctgttatacgcagataaaatagaagaaatgaaaaccatttgctggttctgcggcaagaaggctatcatgaacctgcgttttcacaacggcgagccggtgtatgagggtgaacaaatccaaatgggtgggaacgaatcctattatccggtctgcagaaagcattattacaatccacctattaagtaacaaaagtgaggaatattaaatggacgaaattttcgacaaattacaatcggtcgttgatcgatatgatgagttaaacgagttaatcagtgatccggaagtgattgccgatactcaaaaattcatgaaactatctaaggaagaagccgaccttcgagacactgtggccgcttttaagaagtaccaaaaagtcagcaagcagctcgacgatgacaaagagatgcttcgagaaaagattgatgatgatcttgaagcgatggtcaaagatgagattaccagcctaaccgacgaaaaagacaagctcgaagaccaaatgaaggttatgctgctgccaaaagaccccaatgatgataaaaacatcattatggaaatccacggcgccgccggtggtgatgaaggcagcttatttgctgccgatttattcagcatgtattccaaatatgctgagcgtcagggctggaaagtggaaatcatcgataagaacgaaactgaagttggcggtttcaaagaaatcgttttaatgattaccggtgacaaggtctattcaaagctcaagtatgaaaacggtgcccaccgagttcaacgggtgccggtaaccgaatctgccggccgggtgcacacttccacggcgacggttggtgtgatgcctgaagaagaggatgttgatattgatatcgatcccaaagatatccgggtggatgtttaccgttcatctggtgccggcggtcagcatattaacaagacttcctcagctgtccgaatgacccacttgccaaccggcattgtagttgcgatgcaggatgaacgatcccagcagcagaaccgccagaaggccatgaagattttaaaggcccgggtttatgattactatgcccaacaagaacaggatcaatacaacgctgaacgtaaatcggccattggaaccggtgatcggtccgagcggatcagaacttacaattacccgcaaaatcgggtgaccgatcatcggattggcttgactttaaacaagttagaccggatcatgaacggtgagttggacgaaattattgatgccttgattgtttctgatcaagccaagaaacttgagaatttgaccaatgaataatcaagaaaacgtgacctactttgaagcccgaaagtgggcttcttttcgtattaaggaatctaatgacattgacatgtacgacgtcgattttttgttagagaaactatttaagatgtcggctaccgatctgttgattcattaccacactcagatgccagacaagcagtggcaagtatttcaagacgcgatcggtcaattgctgaaaggggtgccgccacagtacattgttggcgaggcagatttttacggtttatcattgaaggtcacaccagatgtgctgattccccgagttgaaaccgaggagttggttgactggatattggctgaaaactcagattctgagttgaaggtcttggatattggtaccggcagtggggcgattgcgattgccctcaagcattccagaccccactggcaggtatttgccagtgatatttccctgccggcaattgaagtggctcggcaaaatgcgattgctaatcacacggcaattcattttatggcgagtgatgtttttgcagcaattgatgagtcatttgacgtcatcgtgtcaaatccgccatacattgccaaagatgagcagacctatatggatgccagcgtgatcaaaagcgaacctgacttggcactatatgcgaaagaccagggacttgctatttacaaacaaattgctgccgatgcggagagtcacttaacttcaaagggcaggttgtacttggaaatcgggtttcagcaacaatcggctgtgaccgagatcttccaagcagccatgcccaacgctcgagtaattgccaaacacgatgtctccggtcatcaacggatgattcaagtaaagaaatgaaggctatataatatggaaactttaattttaaaacagcagcaactagaccaagcggcggactttatccgtcaaggcgaactggtggcatttcccaccgaaaccgtctatggattgggggctgatgcgaccaatgaaacggcggtcaagaaagtttatgccgctaagggacgtcccagtgataatccgctgatcgttaccgtatctgacatcgcgatggttgaaaaatacacccagccattttccgacgacgccaaagcattgatggccaaattttggccgggttctttgacgatgatttttaagctgaagccaaacgctttatctaaggcggttactggtggtttggacaccgcagcgttcaggttcccgaaaaaccaagccacgctggatttgatttcaaaggccggcgtaccaattgtcggtccatcagccaatacttccggtaagccaagtccaacgactgcacaacacgtttatcatgatttaaatggcaagattgctgcaattgtcgatgatggaccgaccacggttggtgtcgaatcgacgattcttgacatgtctgtggcaaccccgtcgattttgcgcccgggtgctgtgaccaaagaggatattgaagccgttattcatcgaccggtgattgatgaactccatcatgtgggcgccaaacaaacccctaaagcccctggaatgaagtacaagcactatgctcccaatgctcaggtctacattgtcgatcctgacgacgattggcacgatgtggtcgcctggatcaagcagcacccacagccaattggggtgatggcttttgatgacgtcatcaaaacaattaattggccggataatgtcgatgtgatttcacttggcaatgatgcccgcacagcagcgcatgatttgtttgccgaactacgggattttgataaccaccctgcctataaaattatttttacccaaggaattgatccaaagggaattggtgaggcttacatgaatcgtttgaataaatcagctgggcaaatgcatttcaagcagttataatttatttgtaccaaataaattagtgaggtgttgcagttgaactacgattataaacagcaggatccagaactttgggatgccattgccaacgaagagaaccgtcaggagcataatatcgaactgatcgcgtctgaaaatatcgtatcaaacgctgttcgtgccgctcagggttccgtgcttaccaacaagtacgctgaaggatacccgggccggagatattatggcggctgtgagtacattgatgttgttgaacaattggcgattgaccgtgccaaagaattgtttggtgccgaatatgccaacgtgcagcctcactcaggttcacaagcgaaccaagaggtttatgccgcattcctaaagcctggtgatcggattttagggatggggttagacgccggcggccatttgagccacggtgccaaagtcagcttttcaggcaagctctacgactctttctcgtatgggcttgatccaaagacgcaattgatcgattatgatgaagttgccagaattgcccagatcgttcaaccaaaattgatcattgccggagcctccgcatacagtcgaatcattgactggcagaagttccgcgacattgccgattctgttggggcttatctgatggttgacatggcccacattgccggtttggttgcggttggattgcatccaagcccagttccggttgctgacgttgtcaccacgacgacgcataagacactccggggacctcgtggtggattgattttggccaaagaaaagtatgccaagaagctgaactcagctgttttccctggcagccagggtggtcctttggaacacgtaattgccggaaaagcggcggccttctacgaagatttgcagccggcattcaaagaatacggcgagcagatcattaaaaatgccaaagcaatggccgacgtattccagaattccaagtcagtctccgttcttaccggtggaactgacaatcatttaatgacgcttaatttaacgcagacctcattgaatggtaaagagctgcaaaacctgctggatactgttcacatcactactaataaagagtcgattccaaatgatccattgccaccttcgaagaccagcgggttgcggttgggaacgccagccattaccacccgaggcttcaaggaagacgatgccaaagcggttgccaatttgattttacaagtgattgacaaaccaaatgatgaccaaaacttaaaggatgtcgctgccaaagttgaacaattaactgcagctcacccaattaatcaataattttgactggcttgaaactaattgtggtttcaagcctttttgtatactttccgatcgcgtatatgtgatacaattatttcggaatacaaaaaggagttggaaaataatgggtaagtttcaagttatggatcatccgttgattcaacacaagctgtcaatgattagggacaagaattgcgggactaaagagtttcgggaaatcgtcaacgaaattgccactttaatggcttttgaagtttcgcgggatatgcctttggaagatgttgatattgagacaccagagggtattgcgcatgccaagcagatttccggtaaaaaggtcgccatcgtaccaatcttacgggcaggtatcggaatggttgatgggatgcttgatttgattccagcagccaaagttggtcatatcggtatgtatcgtgacgaaaagaccctcgaacctcacgaatattttgtaaagctgccatcagacattggccagcggcagatttttgtcgttgatccaatgcttgcgaccggaggctcatcaatcatggcgattgatgccttgaagaagcgcggcgcatccaacatcaagttcgtttgcttagtagctgctccggaaggggtcaaggcacttcaaaaggctcatcctgatgtggatatctatactgctgcacttgatgaaaaattaaatgataagggctacattgttcctggactcggtgacgctggtgaccgtttgtttggaaccaaataattgattgaagctgagacaaaatgaaaattttgtcgtcagctttttattttatttacaaaaggattctggctttgatagccaacgaattaagtctaatcaaagacccttgggtgacattcgttgtgcatgccgttgaacactactgctcacgcgaagtttccctgtcaagattgttttgaattttgtaataaatggtggtatgatttcaattgtatttgaacacggttctgtgttcagtaccatcgcaatgtttcactttggtattactgtcttctggaccaaaaccagattgatttgcatgcgtgattatgtggaggaaagaggtgagattttgtggaaggagctgcttctacttttgaattcttaggactgacgtttaacgttggtaatttaatttcgatattactggctgcttgtgtggtttttgttctggtgtatgctttatcaaggcacttgacaatcaaaccgggcaaggcacaaaacgttttagaatatgcggtggactttaccaatggtattgtccgaagctcgatttccggtgaaacaagtagaacactaggtttatggggctttactctgtttatgttcatcattattgcgaatttgcagggactcttcttgcatatcgacatttctggtgtaacatatgtcaaaagtccaacttctgatccggttgttactatgactctgtctctgatgactctaacgcttgcacaattccttggaattcggcagttaggttacaagggacattttcagaattatttaaagccattcgtatttttcctgccaattaacttattcgaagagtttactaatttcttaacgttgggattgcgactatttgggaacatcctttcaggtgaaatgcttcttggaataatccttggcatgtcgcatggtggagcagttatgtgggtcgtttcattcattcttgaattggcctggacaggtttctcagtctttatcggatgtatccaagcctatgtttttgtgacattatcatccgtatacatttcacgaaagctcgagcttgaagattagcaaaaatatttttggagactataaggaggatttttaattatgggagcaattgctgcaggtattgcaatggccggtgccgctatcggtggagctgttggtgatggtattttaatttctaagatgttggaaggaatggcacgtcagccagaattatccggacaactgcgtagtaacatgttcatcggtgttggtttggttgaagctatgcctatcatcgccttcgttgttgctttgctggttatgaacaagtaataaccggtttagtcaaatacacaaagaaggaggtgccaattgatgttttcatattcagtagttggagctcagctttatgttggtgatatgctgtttgtcatgatcacatttcttgttttaatgtggttggtcaagatcgttgcatggaagccaattacgaagatgatgcaagaccgttcagacaagattgttaatgatattgattctgccaaggaatcacggactaaagcagctgaacttgctcaaaaacgtcaggctgaattagacaaaacgcgtgatgacgcaaataccattattaacactgccaaacagaatggacaaagacaacaagaacagattgttgaagatgctagaaatgaagcatcgaatcttaagagttctgctgaaaaggacattgaacaagagcgacaagaagctttggctaattctcgaaaagatgtggcaagtctttctgttgaaattgcatccaagattatttcaaaagaattaaacgaagatgatcaaaaaggacttgttgactcttatattgaagggttgggtaagcagaaatgacattagatgatatgagcgcttcaaaaaaatacgcaaaagccatgtttgaagttctgagtgattctaatgaacttgaatctggttacgctgatttgcttgaattacgtaaaatttttgctgctaatccaaggttgattgaaattctcgatgatattcgagtttcagatgacgagaaaaagtctctgctggctcctatcacccaaaatgcatcagactttattaataactttttaaaggttgttgccagctatcgccgtttcccacaggttctgagcattattgatcagttccaaaaggtttacgaagatgacaagaagattgtccgggcgcaggttgtttcggcaacgccgcttgacgatgatcagcttgatcgtttggcaacagcatttgagaagcgggtaggtgcggttaaagccatttttgataccaaagttgataaatcactcatcggcgggatcgtgattcgatcatccgatgtgattatcgacggaagtgttcaaactcgcattaataaggttaaagaattattgttgaattaacgatatctatttaaagaggtgaaacttatgagcattaaagctgaggaaatcagtgctcttattaagcaacaattacaaggctataagaacgagctcgacgttcaagaaacaggtatcgttacatatgttggtgatggtattgctcgtgctcatgggctcgaaaatgcgttgtctggagagttgctcgacttcggccacggcgtttatggaatggtacaaaacctggaaaccaatgatgttggtatcatgattttaggtgatgacacgaatattcgtgaaggtgattctgtaaagagaaccggccgaattatggaagttcctgttggggacgagatgattggacgagttgttaattcactcggtgaaccaatcgatggtaaaggcccaattaaagccgacgatcacaaagcgattgaacataaggccccaggtgttatggaccgtcaatctgttttcgaaccattacaaactggtattaaagcgatcgattcattgattccaattggtagaggtcagcgtgagttgatcattggagaccgtaaaactggtaagacttcaattgccattgatacgattttgaaccaaaagggtcagaatatgaaatgtatttacgttgcaattggacagaaacaatcaactgttcgaactgccgtaagtacccttgaaaagtacggtgccatggattacacaactgttatttcagctgggccatccgaacctgcatcattgctttacattgcaccttatgccggcgcaacgatgggtgagtacttcatgcacaagggtcaacacgttttgattatctacgatgatttatcaaagcaggctgatgcttatcgtgagttgtcacttattcttcgtcgtcctccaggtcgtgaagcttatcctggtgatattttctatacccactcacgtttgttggaacgggctgctaagttaagtgataagttgggtggcggttcaatgaccgcgatgccaattgttgagactcaagcaggggacgtttcagcttatatcccaactaacgttatttccattaccgatggacagatcttcttggatgccgatagtttctattctggtgttcgtccagccgttgacgctggtacttctgtttctcgtgttggtggtgatgcgcaggttaaggctatgaagaaagtttctggtactttgcgtcttgatttggcttcatatcatgaattggaatcatttgcacaatttggttcagatcttgatgaagcaactcaaagcaaattaaatcgtggtgcccgaacggttgaagttttgaagcaaccacttcattcgccaatttccgttgaaaaacaggttgtcattctttactgcttgacccatggattcttggataaaattgcaattgatgatattttgagatatcaaaccgagatcttcgattacttcgatcaaaatcacaaagatttgttggaagatatcgctaagaccggtcaattgcctgatacaagtaaaatggatgctgcaattaaagactttgaacaaactttccaaccaagtaagcacgatgatcaacaatcaaacgatgatcaatcagctgcttcaaatgactagttttaaggagggtgagattacatgggtgcttcgctaaacgatgttaaacatcggattacttctactaagaagacgcgacaaattaccaatgccatggaaatggtttctcaggcaaaactgaaccagatccaaaagcatacggttagttatgcggaatatgcaagccaaatcaaatctgttgtattgcatttagcccaatctcacattttagatgggctaaacaaatcctcaggtcattcagctgatcaagatcaatctaagactaagagaagcgcatatttaattatcacctctgatcgtgggatggttggtagttataatagtaacgttatccgtgaagccaatgagtttattgagaagcattcgggatcgaatgattatcaaattctcgctgttggtggaaccggatccgacttttataagaaacgcggcgacaatgtttcttatgaataccggggcgttagcgatgtgccaacctttaacgaggttcgtcaaatcgtcaagatggtgacatcaatgtacgataaaggtcaattcgatgaattgtacgtttgttacgagcatttcgttaaccgtcttatttcccgtttcagagctgagaagatgctgccaatcgatgatgaagccattgcgtcagctgccagccaggacattgaagttaagccgatgagtgctgaatacgatgttgagccttctgaaaaagaagtcttggatgttgtattaccacagtattctgaaagcttggtttatggtgcaatccttgatgccaagacttcagaacatgcttcaagttcgactgcaatgaagtcggcatctgataatgctgacgatttgatttcctcattggaattgcagtataaccgtgctcgacaggctgccatcaccactgaaattactgaaattactggtggtcaagaggctcttagtcactagaaagatttgaatggaggaattaactaacatgagttctactggtaaagttatacaagttattggaccagttgttgatgttgaattctccttggacgataaattaccagaaattaacactgctttagcaattcacgtcagcgaagacaagaatttgattgtcgaagttgcccttgatttgggtgatggcgttgttcggacaattgctatggatggaaccgatggtcttcgtcgcggtatggacgttgaaaacaccgaatcttcaatcagtgttccggttggtaaagatactcttggtcgagtattcaatgttcttggagatccaatcgatggcggcccagaatttggccctgacgctgagcgttggccaattcaccgcgatgctcctaagtatgatcaattaaacccatcaactgaaatccttgaaacagggattaaggtgattgatttattggaaccatacactcgtggtggtaaagttggattgttcggtggtgccggagttggtaaaaccgtcttgattcaggagttaattcacaacattgcacagggacacaatggtatttctgtgtttaccggtgttggtgaacggactcgtgaaggtaatgatatgtactacgaaatgaaagggtcaggggttctcgagaagacggccatggtttatggtcagatgaatgagcctcctggtgcgcgtatgcgtgttgccctgactggtttgacaattgcggaatacttccgtgatgaagaaggccaagacgttctgttgttcattgataatatcttccgattcactcaggctggttctgaagtttccgccttgctcggccgtattccatcagccgttggttatcagccaacgttggctactgaaatgggtcaactgcaggaacgaattacttcaaccaagaagggtgccattacatcaatccaggctgtttatgtgcctgccgatgattataccgaccctgctcctgcaacgacatttgcccatttggatgccacaaccaacttggaacgttcattgactcaacaaggtatttaccctgccgttgatcctttggcttcaacatcatcagctttggatccagcaattgttggtcaagaacattacgaagttgccactgaagtccaacatgttttgcaacgatatcgtgaactgcaggatatcatttcaattcttggtatggatgaattgtcagacgaagagaagacggttgttaaccgtgctcgtcggatccaattcttcttatctcaaagtttctcagttgctgaacagtttaccggcttacctggtaaatacgtatcagttcaggatactgttaaaggctttaaggaaatccttgaaggtaaatacgatgatattccagaagatgccttccgtaactgtggccctatcgaagatgttgttgaaaaagccaaggctatgaaacaggaatcagacaatgaaaagcagcgtgctgcaaactaaggagggattctaattggctgataattcagttattaccgttagtatcgttactcccgatggaaaagtttacgagcatactgctagtatgatagttgtttcaactcagtcgggacaactaggaattatggctaatcacgttccgattattgcaacacttgacgttgatgaaacgcgagttaaatacgacgacaaggaagatgatattgctgtcaacggtggctttatcgaattctcaaacaacgttgcgacaattgtggctgatagtgccgaaactcaaaatgatattgatattgcccgtgctgaaaaagcaaagaagaacgcgcaacaaagaattgccgaagcccgtcaacgacaggataaggctgctcttgatcgtgctcaagttgctcttcgccgtgcaattaacagaatcaacgttgccgggaaataaccgttatttctgattgcggtttccggaaactgaacacggtacttcaaaagctgcgcccatttgggttgcagcttttttggttggttggagttaatccttgaaattaccggtgaatcaggttagaattcctttatcgtgatttgtgaatgatgtatttatgtttgcgtttttctcccgttttgtcggaatcatatacagtcattgttatccgaatgtgccgattagatagcaattctgcttatatttttgtaaaagaaaccgaaaaggtaagacaagttcgcgtctttatgatatagttgtctgtgaattgggggaagactcaaatgaatacgattggcattcaagcgctgattacattgattacatacattttgtttatcgctatggcgttttggacagttcaagaaatccacatcgagcgttatatcccattgagggcaatgccggggaaattactgatcgtgctcgtttcaattgcgattgggtacgcatgcagttcatttttcctctctgtaatatttaacattcagaatttgatgtatctaattaagtgatgtaggaggcgttcttgtggaaaaaattattgtacatggtggtaagccacttcgagggacagtacatattgatggggccaagaatgccgttttaccaatccaagctgcaactattttagccggtgagggaaagacggttatctcaaatgtgccattgttgtctgatgtgtataccatgaataaagtgttgcggttcttaaatgtaaaggttgattttgatgaagccaataacgaaattacgtttgatgcttcaaaagatatctccagtgaagcaccttttgagtatgtctcaaagatgcgtgcttcaattgttgtcatggggccgcttttggctcgactcgggcacgcaaaggttgctttacccggtgggtgtgcaattgggtcacgaccgattgatctgcatttaaaaggatttgaagctttaggtgctcggatcgaacaacatgacggctacgttgaagcttacgccccggatggacttaccggagctgaaatctatctggattttccaagcgttggtgccactcaaaacattatgatggctgcaacgttagcaaagggcaaaacagtcattcagaatgctgcccgcgagccggaaattgttgatttggccaacgttttaaacaagatgggggccaaagttgtcggcgccggaaccgaacagattcgcgtggaaggggtgcctgaacttcatgggactgatcacgcggtggttcaagatcgaattgaagccggaacgttcatgatcgctgctgcggttactcgtggtaacgtgatgattgatggcgctattcccgagcataacaaaccactaattctcaaaatgcgcgagatgggcgttaccatcaacgaaagcgatgatggcattcaagtcatcggccatgacaatctcaaaccggttgacgttaagacaatgccgcatccaggctttccaaccgacatgcagccgcaaatgaccattttacagttgaccgctaacggcagcagctcaatgactgaaaccgtttttgaaaatcgtttcatgcacatggaagagctgcgtcggatgaatgctcaatatacgatctctggtcgaacagtcattatggatggccctactgattttaatggtgccgaagttgcggccaccgatctgcgggccgccgcatccttggtgattgccggcttggccgctagtggctataccaccgttaccaacttacagtacttggatcgtggttaccacgatttccacaagaagctcgctaatttaggtgctgaaattaaaagagtcaacgttgaagacgactcaatcgtcttgaatcaatcgctcaagaatcgttcataatttttcggggttgggatcgttacttgatctcaaccctttattgtttggagacttattagaaacgcaaactttatgtggtataattattttttgagattaaagtttttcaggaggaacctacacagatggcaaaagacattggaattgatttaggaactgccaacgtactcatttacgttgccgggaagggaattgtattaaacgaaccatcagttgtcgcagtcgatactcggactggtaaagtcttggcagttggctccgaagcctatcggatggttggtcggacgccaagtaacattcgtgcgatccgcccattaaaagacggcgttatctctgattttgatattactgaagaaatgctgacatacttcattaacaaattggacgttaaaggatttatgtccaagccaaaaattatgatctgtgcaccaaccaacgtgacggaaattgagcggaatgcgatcatgcaggctgctgaaaaggctggcggcggacaagtctatctggaagaagaacctaaggtggccgctgttggtgccggaatggatatcttccagcctcgtggtaacatggtcatcgatatgggtggtggaaccagtgatatcgccatcatttcattgggcgatattgttgccagcaagtccattcgagttgccggtgataagatgaacaccgagattgccagctatatcaagcaaaagcacaacctgattattggtgagcatactgccgaaaagattaagattgaaattggaaccgctaagaaagacgattcagacgtcaaaacattggaagttcgtggccgggacgctgtttccgggatgcctcgggcagttacgattgatagcaatgagatcgccgaagcaattaacgataccgttcaattgatcatcagtggtgccaaagaagttctcgaagtgattccacccgaattggcgtcggacattgttgaccgtggaatcatgctgaccggtgggggtgccttattaagaaacatcgatcaagtaattgccgatgcactaacagttcccgtgattatttccgaaaatcctttggataatgttgccaagggtgccggtatccttttggaacactatattaagaaccctaagttgaaggcaaaagatcaaaaataacaggagtcaaagtgaaaaacattctgattagtcttgttcatggttatcagcgctttatttcgcccttattcccgcctacctgccgttattatccaacttgcagcagttatatggtaactgcccttaaaaagcatggtgcgttcaagggggccgttatgggcattgcccggattctgcgttgccatccgtttgttaagggtggctatgatccggttccggatcacttcaccatttttcggaataaggacgcacgcgatgaataccggaaatccatgcacctgaaatgatctttgaacaaggagaatatgatgagtaaagcaaataaaagtatcaacgttgaaattaaagatcgaacggatcaaaatggagaatcgatctccgaattatttatcggcaagaaattgattggctcaattaagcagttgagcgaaactaaatttcaagcagtcaacactcacgacgaagcgtttcatgttaaaaccttcgatgagggtgtgacacaattaatcaaagattttcatcttcaccattaatttggcgatcgaaaacgaggagggtctaatttggatagcagtcgcagaacctctaaagacgaccaatcgcgaattgactggggaattattttctgtgtcttaatgctggcgttgattgggctggcatcgatttacgttgcagccactcatgattcaagctctaccagcgtcatgagacaggtggtttcgcaattggtttggtacgtcatcggaattatcgccgttgtcattattatgcagtttgattccgagcagttatggaaagttgccccgattacttactggctggggattgccctgctggcgagtgtcctggtgttatacagtcggacctattacattaatacgggtgccaaaagttggttctccctatttgggttgacctttcagccgtctgaagtgatgaaaccggcctatattttgatgatggggcgggtgattgttcaacataacgataattacccaatcaggactgttcgaagtgatttcctattaattgggaaaatgttgctgtggacagttccggtagccgtcttgttaaagctgcaaaatgattttggaacgatgttggttttcttcgccatcttaggtggcttgatcatcgtttcaggagtgacatggcggattattctgccagcggtgattaccatctttggatttgccggaaccatcttggctttggttattccggagtccgggcgtcatctgttggagaagtttggttttcaagcctaccagtttgcccgagttgacacttggctcaacccgtcagccgatacttctaatcaggggtatcagttgtggcagagtatgaaggccatcggatctggtgggatttttggaaccggatttaatcagtcacatgtgtatgtgccggtgcgagaatctgatatgattttctcggttattggcgagaactttggatttattggcagctgtattttgattttattgtatttcctgttgatttatcaaatgattaaggttacattcgatacgaggaatgttttttacgcttacatttccactggcgtgattatgatgattctgtttcatgtttttgaaaatgtcgggatgagtattggcctgttgccattgaccggtattccattgcccttcgttagtgccgggggatcggcgttgattgggaacatgattgggattggcttaattatgtcaatgcagtatcataataagagttacatgtttggagaagacaaagaattctcataatttttagaaaaggtggaattaatgatggatacaaaatattattggactgaagaaaataacggggaagtcacagttggcttgaccgaagcaggtaagaacgaactgggtaacatcacttttgtttcccttccaaaggttggtgctcaattaaccaccagcgatactttattaaacgttgaagctgacaaagccgtttcggatatcccaagtccagttgccgggaaagtgactgctgtcaacagtaatgccgttaatgacccttcagtactaaacgggactgacaaggcaacttcatggattgctaagattaaaaaataaaagttcttgacgctaggaccttttttaggtacactaactgatagtttgatgatagaaaaattacaagatgagtagataattagagattgtcaagagagcccggctggtgggaaagggtcaatcatcgttattgaagatggtcttggttaaaaatgtgtcggtgagcaattgcaagccgataatgggtaacgaccattatttcgttgagtatgaagatactcatgaggcgattgttgaaagacaatcgcgaataaaggtggtaccgcgaagcttttcgtcctttcataagtcaattaagacttatggaggatgaaaagctttttttgtctaataaggggtgaaaagattgattcgatttaaagatgtatccaaacagtacagtaccaaggatggcggtctaaccgcggtcaatgatgtcaacattgagattaacgatggtgagatcttcgggattgtcggctattcaggcgccgggaaaagcaccttggtgagaatgctggacggacttgaagcgccatcaaccggtgagattgacatcaacggcacggatgtttccaagctccacggaagccaattaagaaagcaacgccaaaaaattggtatgatctttcagcatttcaacttattgtggtcacgaacggtgctggacaacattgctttaccgcttgagattgccaaagttcccaaagccaaacgaaagcaacgcgcagaggaattaattaagttagttggtttggagggccgtgagcattcctatccttccgagttatccggtggtcaaaagcagcgggttggcatcgcaagagccttggcaaacgagccaacaatcttaatttcagacgaggcaaccagtgccttggatcctgacacaactaatgaagttctcgatttattactgaagattaataaagaaatgaacctcacgattttattaatcacccatgagatgcacgccattgccaaggtttgtgaacgggtggcagttatggacagcggcaaagttgttgaaaccggatcagtgtttgaggttttccgtcatccacaacaagaaatcaccaaaaagtttgtcagtgaagaatttacaccacaacaaagtgacaacacgatgacccttgatgaattagttaagaaatatcctgatgggcaaatcatccgactgattttccatggaccacaggcggaactgccaattgtttcggatgttgtcaaacggttcccggaattaaccatcagcattatttcaggggcgattcatcaaactcaagaaggcgcgttggggtcgctggatctgcaatttgtcggcgatgacaatcaaattaacgatgccttggaatacctgaagaagatgcgggttggaacggaggtgattcatcatggctaattcaactggattcaaatcttacttccagtttcataacgtcgattggggttcgatgatgtcggcaacttgggaaaccgtttggatgaccttgttatcaatggttgcaattgttattttaggaattattttggggttgatcttatacgagactcgcaacaagccgggcattggctatcgaattctcaattggctggtcgggttgttcgttaacatcttccggtcaattccatttatcatcctgatcattttgttactgccaattaccatgaagttggctggaacgatcattgggccgcgggccgcgttaccatccttgattatttcggcggcacctttttacgctcggatggttgagtcctacttccgtgaggttgattccggggtcttggaagctgccgaatctatgggtgccacaacctgggaaattatcaccaaggtcctgttaccagaaagcaagccggcattgatcgccggagctactgttaccaccatttcgttgattggttacaccgctatggcaggtgccattggtgccggtggccttggaaacttggcttatcaagatgggtttcaggcaagcaacaacacagtgaccttagtcgcaacggtcatcatttgtttatttgtatttgtcgtccaatttgtcggagatgtctttgtcaagattaccgacaaacggacattataatatttgggagggtttcaaatgaagaagaaattattgagtttattcgcagttgtctttaccgcctttttgttggtggggtgttcatcatcgtctaattccagcaaaaagaccaccactttaaaaattggtgcttcagccgtgccccatgcacaaattttgcgccacgtggccccagaacttaaaaaagaaggcgtcaatctgaagattaccactttccaagactacacaatgcctaacaaggctttggccaacggcgaactggatgccaattacttccagcatgtcccattcctgaaactttggaacaagcagaaccacgggacattagtcaatgccggtggcgttcacttggaaccgatcgctgttttctcgaagaaagttaagaggcttcaagacctcaagaagggggccacaatcatcgtcagcagcaatgttcccgactatggccgaatccttcagatcttcaaagacgccggcttaattactctgaaaaagggcattgacattacttctgccaacttcagtgacattgcttcaaacccacgtcatctgaaattcaagcacagctatgaaccaaaattactgccaaccatttataagaatggtgaaggagatgcagttgtcatcaacgccaactacgctgttggtgccgggttgaatccaattaagcagtcaattgcgattgaaaaacggaattcaccatacgtgaacatcatcgccacccgtaaaggtgatcagaacaagccagccatcaagaaggtagtcaaggttcttcaatcaaccaagactcaaaaatggatcttgcatcactataaaggtgccgttttacccgagaagaatgttaagtaattaatatcaattaaaagccgtccgctatatacttgaattagtaattgtttacgaatccgagtttatagggggcggcttttttgaaagagaaaaatgtatttcatgttaatggttatgtgggcttaattattgccttgattttgctgggagttggcggttatctgctttggattggcggtgaaggcagctcaattggctcgatcgtttttgggacaatcatcattgttttggatttgttatttgcaagttcattaacgattatccagcctaacgaagccaaagtgttgacattctttggtcgctatattgggacaattcgaacttccggattattcatgaccgtgccattgaccagcaagcagacgatttcactgcgggttcgcaattttaatagttcaattatcaaagtgaacgattccaaaggaaacccagtcgaaattgccgctgtcattgtctacaaagttgttgattctgccaaagcaatttttagtgtggaagattatgaacagtttgttgagattcaaagtgagtccgctattcgacatattgccagccagtatccttatgatagttttgacgacagtaccgacaaattgaccttgcgggggaacgcaaccgaagtttccgtggcgttgcaaaaagaactccaggaccgtttggatgtggccggtctgcagatcattgagacccggttgacgcatttggcatatgcaactgaaattgctaacgccatgctgcagcgacaacaagcaaccgccattttgtcggcccgaaaaattattgttcaaggagccgtggcgatttccgaggatgccgtttcccagctgcaaaaggatttgggatcatcgattacagatgaacagcggatgaaaatgatcaataacgtcttagtctccatcatcactgaacgagggacccagaatgtcattaatactgataatctagattaattaacgcttttagacgattaagaggctgaatgttatctagcagaactgtgggccaataagcagcttccggccgtataaggggattacccaaacatccaaattccggatattcgggtaatccccttatactctggaagctaaccacttattggcccacgcttttttgtttttggttgacatccggattcttagcatatatagttagttacataagtaattaactaacgcacggaggaacacttatgacaactaaaatcgttcaaacagaagatttacacaaaacctacgataaagacagcgcaaaaccatatgaagctctgaaagggatcagcttgtcggttaacgagggcgaatttgtcggaatcatgggcgcgtccggttccggaaagacgactttgctaaatattttggcaactctcgatcaaccaaccagcggttcggtcgaaattgacggccaagatgtaactcatttaactgcgaaccagatggcagattttcgttctaaaaaattgggtttcatcttccaagactttaacttattggaaaccttaaccgcccaagaaaatattgctttgccgttgtcgcttcaaaatgccaaggcggccaccatccaaactgctgtcaaggaagccgccagcaagttgggaattgatgacttgctgagtaagtacccaacgcaattatccggtgggcaaaagcaacgggtcgccgctgccagagccttagtgtcaaatccgtcaattatttttggggatgaaccaaccggagcgcttgactcaaccaacgcccgtgaattactggacaccttaacgaacatcaatcaacagggggtctcaattctcttagtgacccatgacccgttctccgctagtttctgtaaacgaattttatttatcaaagacggaaaaattggcgatgaggtagacgccggcgataagccgagaaatgaattctatcaggaaatcctcgaaaaactcggtacatttgaacagtaatcaatcaaaggagcttagcgatgttatttaaaatttcaatctcaggaatcaaggctcgttggaaagattatctggttctgttttccgggatgatcattaccacagccattttctacatgtttgaagcaatttcaacaaatgataaatttaccaccagcagtgcggtgggacaaaatgccaagatcgttttcatcttcggatccatcttactggcaatcatcacactggtatatgttttttacgcgaataatttcttgatgagtatgcgtgaacatgattatggactcttcatgatgctgggggccaaatcaggggtcatcagtaaattgatcatccttgagaccattgcgatcggtttaatttccacagttgtcgggattgtcattggcattggctttacccaagtgctcagccattttctggccagcctcattcacatgtcattgactaatttctcggcattttatatgccagctgtcattgcaacgattatcctgtttgcgattttgttcctggttgctggtttcttaaatgccaggacattcaccaagacctccgccctgcagcttttgcgttccggacagcaaagtgattggcagcagcctaaggccttgacacttggcgttcaagcaattcttggagttgttctcttggccggtggatattatgcgatgtatgacattcaaaaactgaaagtcatgtccattccaatcgcgctcatcacgattgttctagggacctactttgtcttcaactcattttttgtgatgctgctccaggcatttcaacgttctaatatgagcaccaagggcctgaacagtttcacattggcccagcttaaatttagaattcgtgattataccaaaatcctttcagttgtctcgctgctgtttgcgttgtcactaggggcaattactgtgggaaccggttttcaacacatggtacccaaattagcttccggaaatggctactattcagttgctattaccaaccccaatcaggaaatgcgttcactggttggccagattcaagataaatccactgtcacttaccaacaaaaagttgatccgacgaccaagcgggtttattaccggagtgaccagcttcagcgccaacccttgaagtacgcggcgtttgtgagtcgaaagacactggcatcaaaggcttttaccgccaaaatttcccagttcaaacggagtgattcatcggcataccaagagctgtggggactgcaggtaccaacgattaaagcctaccaaatcaaagtggtcagttctcaggcattcaatcaaattaatgccaagaccaatcaattattgttggttcgcgcaaatgatatggacgctgccgcaacgccactcaccaaaattaccaacattcagtccacgcagtacggctatcgaaacggggaacaggtcggcgtttcgtttacgatgtatcaatccctgaagagtgtctttggcagtcttgagtttatgggaatcttcttaggaattgcctttctggccatgctcgccagctgcctaatgtttaagattttgagtggggcagccagtgacaagatccgctttgatatgctcaataagattggaactcgccgatcggtcttaaatcactcaattgttgttcaaattctgggcttgtttgcactgccgggaattttgggaatcgtcgacgttgccttcggacttcaaatgttcgccaagagtggtctattgatgggtggcgcctaccaaacctttggactgacgacagtcggcttcttggtcctctacttgatttactttgccttgaccgtcctgatttattcccgaattgtggttccaaagacgaaggtggagcgttaaatgaaagaaattatagaatgggttgataaatatgaagtttgagtttaatagttcagagcccatctaccgccaggttgccgaacaaattgaggacgcgattgcttcgggagggtttgctgaaggcgaccagattccgtcgacgacagaaatttccaaggagtttcatattaacccggcaaccgttttaaaagggatgaacatcgttgctgctaagaatttgatcgaaaaacggcgggggctggggatgtttgtccaagcaggcgccaggcagcgaatcttggcagaaaagcggaatggcttttttgacgagtttgtcgaaaatctggttcgggaagcccagaatctggatatttctgaagatgagttattgaatttagtgaaaagaggttaccagcaatgagcgtattggaagtcagtcacgtctcgaaatcatttgggtctaagcacgtcttgtcagacattaatttgtcatttgacggcaacaaaatctacggcttacttgggcgaaatggtgccgggaaaagcacactgctcagtattattaccgaccggatttttgccgacagcggcgaagttaagattgattctgaggatgtcagcgataacgactcaaagctgggtttgatgtatttgatgagcgaggccaatctttacgctgacggctggaagttgacccaaattctcaaggattccgaatccttgtatggcggattcaaccatgaattagcggatcacttgatcaaagaatttggcttggatatcaatcaaaaatttggtaaattatccaccggttacaactcgatttttaaactcattttggccttgtgccttccagtcaaatacgtcttgctggatgagccggttctggggttggacgccaaccatcgagaactcttttacagtgaattgattcaatcctattccgataacccgcggacatttatcgtttccacccaccttatcgaagaggttgccaatattatcagtgacgtgatcgtcttggatcaggggcgggtgattttaaaccagccggttgaagacgtcttggccaagactcattcggtcgtgggaccagaaaaagacgtcgagcaatataccaagggcttaaacgtcattggccacgacatgatgggcaccatccgggctaactacgtctatggtgaccttgacgaccgcatcctgcccgacacagtccagctgtccaactttgacttgcagaaactgtttatttttctaaccaatcaatatgaggggagtgccaagaatgaagacaaataaagtcaccaaattcctgtttcgacgacagattatcggcttagcggaaatgtatctgttcttgtttgccgcctttttggtactgccgtttctgttttccgccatctcagaagctgtttagtatctttgattttgacccaataatttgataaactactgtcaaaaaagttggtgatcatatgcaacattttagtcatcattaccaaagcgatatttctcggcaacaattcgatttgatccgccaggatctggaagcttcaagaaaacgaactcatccaaaacacattgatccttatgatatcttctgtgccatgctctatgtccttaaaaatggttgtacttggcgtgatttgccggctgattttccaaagtggtccactgtttactactattggatgaattggtcgaaagcccccacccctgataaaccagctttattaactcaggttttaaaaaaattgtcgctgatcgacgattaaggcaagggcgatcagcccgaacttcgttcgtcattttagatgcccaaagtatcaagaacaccgctaccgctgaaaataagggttacgatggtggtaagaagatctcgggaattaaacggcatttagccgtcgacatcaatggcttcccgcaagcgatccatattacccgggctaacatcactgatcgtgacggggcgattgcactcgttacccttaatttagagcagtttaaattggttcgaaccatgatggttgatagtggttataccggccaaaattttgctaatgagattagcagtttaacgtcagccaaggtaatcgtcgttaaaagaaatgagttacaccaattttcggttatcccccaacggtggctcattgaacgttcatttagttggttgggaaattatcaccgtttatggcgtaactgtgagcgtaagctcaacactagtctcatgatggtttcgttagcttttatcaggttacttcttaaaagatactaaacagcttctcaggatctctgaatgattattccttgaccaatcagatgcaggggtcctgggtgacggcggcgtttggcctgtatatgtttgttatttcaacgctgtcctatgaaaacttcaagtttttgatccaaaatgggatttcccgagaaacttttttcaatgcgcaagtcattgtcaatggcttgttaatcctgatcggcaatacctttaacttagtgtatcagtacgctgtcttgatgccattggggcatgccagagacaccaacatctacatgtcctcgtacgctggatactttaataatccaattgtcgcatttttgttcaactttatttttagcggattgttgttaatcgttggcgctttgagcgggatggttatcgggaactttctaacgttgttctctaaatttgtccagcggatcattttgatcgccacgccggtcatcggctacatcaccgtgatgtacaccgcgtcccgggtcattttggatcgcaattttcagatgacctgggttgccaattttgccaaatttgtcctcggctggcgggccactggtgcctacgatccatttccgatgattgtgagcatgctgatcgtttctgtgatcttgttgttgatcacccgctacttgttcagtaagaaacaattaaaacgtgaataattgtgatcggtgaattcagcctaaaaatgtgatgagaagcgtttgtaaatgttttcaactgtgaagttccgtgatatacttaagtttctggaaactatacgaatttataaaaggatgagaattcatggaaaaacacaaaaagcaacacattggcctcatttttggcggtaactcttcggaacatgatgtctcaaaacgctctgctcataacatttatgacgcgatggataaagagcgttacgatgtgagtttgtttttgatgaccaagaacggctacttcctggatcatgaagcttcctctcgggttttcgacggagaaccggaagacgaagttgccaagcaggaattagctaaattggatctcaagaatcctttggctcggataatcaacctggctgaagaatccgatattgacgttttcttcccgattattcacggtaatttgggtgaagacggaacgattcagggactattacgcctcctgcacaaaccatatgtggggacggcaatcttagggtcagccatgtcatttgataaagacattaccaagaagattgtcaaactggctggagtaccaaccacccgctatgaagtgattaccccgctgacggccgagcagtacagctacgaatctctcagtgatgaactgggacagactttgttcatcaagccggctaaccagggatcttcggttgggattcacaaagttgaaaatgccgaggaatattccgaagggattcgcgatgctttccgatatgacagcaaagtcttgatcgaagaagcgattgaggggccggaagagctggaaatttctatcctgggtaatgatcatccaatcgcatccaagattggggccattcgcgtacccaaagacgacgccttttatacttacgacaataagtttgttgatgccagtcaggttaaatttgacgttccagtggatatctcggaagaacttgcccaacagatcactgaaatgggcctgacaacttatcgggcattgggactcaaggggatggctcggatcgattatctggtttctaaagacgacaagccatatatgagtgaggttaatacgctgcccggatttaccaacatcagtttgtatccgcagctattcgctgcctctggcatttcatattctgaattaatcgatcgcctgatccaacttgccattgatgagtttgaacgtcagtcaaaaatcttatatgactttaagccattgccaccacgcgatcaaaatattaacaaatagcataatcaaactggcgcagaattctgctgccggtttttttgcatgtagggaagttttttgatggggaataatgaaaccaaactttatgattatttaacgggggcattgatcgtccttattttactgttgagacgttttctggacacttaccaaagcttcgcaacggtggtattttgctcactaacgatgtttttactgttggtcggtctattttattatgggatcgtccaaaccgttcacaagacaattttgagccgaacgtggtcactattggcgctgctgggaagcggtgtttacctgtttgttctgctggtgccattaggcctgtttggcttctcaaatttcattaagttttcggtgccgatttctggggatcagtttacttggctgacagtcaatcgctatccgcttgcgctgactgccatcgtcggctattttggtttattgctggttgggatttatttttctcattttgcgctaaatctgcttgctgcggatggcgattatccgattcaagctttgaaacagactgttaaattaatgacgttgaaaaagtatgcccaaaagctgtgcttattatttttgatgctggttggcatctgcctgttgattgttgggctgggctggttgaacagattgcttcccaattcattcctattctttttgtcacaaggaacgattgatgtggtggctccatttgttgaaatcgttgtgattggtcgcctgctggggattcagtttgcccggctgacaggaaaggggctgattgctggtgtgggcggatgtctgattatcttctcagcgctgtttgccgggatcaatcccgccttttccgtccgaccggttggccatcccacgatcattgttcaccgcggggtcattaatcataacgctcagggaaacacaattactgctttgaagcgtaacagccattatcactttccatttgttgagatggatattcaagaaaccaaagatcatcactttatttgtgcccatgataacgatgtgccaattccaggccacggggatcaggagattaaccgcctcaatctggcagaaattaccaaattccatcatgttgatatgttcggtgattatctgcgaacggcgaaccgattaaagcagccgctgatcattgaattgaaggtaactaacagcagtgacccacagatggggactcgatttgcccaacagtttgcctctcaattgacggttttaccacaccgggttcattcggttggttatccatttctccgacaaattaaacaacggattccacaaatcaatgttggtctggtgactatgcttaattttggtaatattggcaagtacaaggtcgatttttacacgctgcagcatctgaccgccaatccattcttgatttcctcggttggcagaaccggtcggcccgtctattcctggacagatgatagtcagttatcaatgatgcgaatggaaatgctgggcatcaccgggcaggtcaccgatcaagcgctgcgtcttcaaaaattgcgggttaactatcaaaaggaccgttggattctacttttgaactcgttgcagaattatttgtgactttttcgtaggtttatagtaggaggtgtagtgatggttaaaagatgcccttgggcaactaccagccctgaactattggtttatcacgatacaatttgggggcgggtacaaaaggatccgcaaaaactattcaaagccctgtgtcttgagacgatgcaggcaggattatctttttcaacgattttaaaatttgaatcgggaatggatgaagtctttcaccacttttccctggattatttggccaagtgtgaccagtcagatgtcgaacggttttgccaagatcgtcgaattatccgtaatcatgcaaaggtcagtgcgataattgccaacgccaaagtcattcaaccgaatcctaaaatgttggttgaagcaacctggggaccagttaatggggtttcactggatcatttactaaaagcagcgccagacccaaaaatgtatcaaaaatttaccgaaaagtttgtgaaggcctttaaaaatatgggccttcaacggattggcttaattactgtgtacagctatttgcaagcggttggcgttgtgaatgatcatctgatcacttgtgattttcatgaggaattacccgccaaaaatgaggaaaaatcttcttgattgtcgattataaatataatatgatactcaggttgtatgttaagcatgttaactatagggagtcgttgtatgacaatggtgattactggggccttgatcaaaaaggcaagaaaagataaggggatgtcccaagttcagctcgctgaagggatttgtacccaagcaaccatcagttccatcgaaaatcaaaatacgtgcagcagtgttgacattctggtcaacctctgccaaaaactggatttaaaaattaccgatgttgccaagaatacgcgatatggtgataaagtcttctcttacattgaagacgatatgcggaatcatttgtatgccgacgctaatagacaaattggtcggattgactgcaaaaagttgaatacccgatatatgttgggcaagtatcattgctatcggggattcattgaattgtatatcaatgatgatattgatgaggccattttcaacttcaatcttcaattgacgcagtattccgctgatgaattcaccttttaccaagcctggtccaatttgggcattggtctggcttatcaaaagctggggaaattggatcgcgccgaagggttcattgattccagcgccaaaattttggctaaagtcaaaaaggccggcaagcacgatatgatcgtgattgttgacctctatgtggatattattgccgcgtacgccgagttgggtaaatatgatcgggcgctgccgctcattcatgaaattttacacgaattgacggagcaggatttgatttataaggtggacgtgctggcggagttggaatcaaaatgcctgtatgccaaaggacaggtcgtccaggccactatgaagcagtttgcagcgatgtttattgccgaacttcgaggcaacacggaattagctgagaaaattcttaagcgcaaccagtcccatatcgtcgagatggtcaaaaacgagcttgcaaaaagtgaggggcatccgacctttgttaagtgatggctggcatgttagccgcaaaaagcagttaaaacaaaaggatttgacttttgttttaactgcctttttagcttgctttaatcaatttgatgatcgaaattggaagcattaaacgtgcttgcttggattaactgccggcttattgtctaaatcagttctaacgaccaggacatcgcaaaccgcagttctggtaacatattcggtaaccgaaccaattaagagtcgttcgacggcattcaaaccagttgcaccaatcatgatgaggtcgatgttgaggttttgaggaatatctctggcaatcacggtctttggtgcaccatattcaattgagtaatcaacatcgttgagccccgctttttttgcatcttcgatgtatttatccaaagtttcctttgcagtatcggtcacttgttcgaccattgatgtgtcaaaacttgaaatattttgaaatgcacgtgtatcaacaacgtggactaagtgaagagatgcattattacggatcgcaactgctacaccttttttaaaagccaattcagcctcgtaggaaccatcaactgggaccaaaatttgtttatattgttgttgtaacattatgcccaccctcatttctatctgtttaacttaattgtactttactttcggcaaaatacaaaggaataaatctattaccgttgtttatggttaatgacgttgagaattgcgaattcaacaaccaaaccatgtgcagtcatccacaaaagaaccactaaaatgagaatatcattttgaatgattaatgccagaacgcccaaggctgccaaaatgatgaacatgatgccgccgtttttggcagctcctttcaggcggggatcatcttgaactgaaatattaaacatggttttgtgaaggtgggaaagtaagtagtagccaatatatagggcaattaacacagcaagggctactaaaatattaattatcatcattacactccaatactatttatgaccggcagattttctaagcttggcatattgttctttaaacgcggtctcaattcgaccgttttctttcgggtggtaatactgagcattcttaattttatcaggcaggtactgttgtctaacccagtcgttgggaaaatcgtgggggtatttgtaggtcaccccgcggccgagtttcttggcaccttgataatgagcatctttgaggtgcagtgggacatcaccatagttaccggatcgaatgtcacttaaggcaccatcaattgcggccatcgcggaattggacttgggacttaaacaaagctcaatgattgcgttagcaagtggaattcgtgcttcgggaagccccagttgacgcgcagcatcaacagcagccacggttcgctggcaggcactgggattagcgagaccgacgtcttcataggcaatcactaatagacgccgcataatcgaaaccaagtcgcctgattcaatcaatctgcccgcataatgcagggctgcatccgtatccgagccgcgaatcgatttttgaaaagcagaaatgacatcgtaatgggcatcaccatttttatcggaattgagtgcttttcgctgaaggcattcctcgacgattgcctgggtgacggcgatttttccgtgatcatttttgggtgtcgacttcactgcaagttccaaggcatttaacgatgagcgcaaatcaccattagtggcagttgccaaaaagttcaacgcttctttggtaatcgacaccggataattgcccaaacctttttctttgtcgtttagagcgcggttgagggctttttgaatatcggttgccgtgaggggatgtacctcaaaaatttgggttcgcgatcgaatggccggattgatgttaatgtaggggttctcagtggtggccccaatcaaaataattgagccgctttcaagtaatggcaatagaaaatcttgtttcgttttatcgagtcgatgaatttcatcgagcaacaggacgaccgtgccgctcatcttggcttcctcggcgacaacctgtaaatcttttttggtgtcggtagcagcgttgagaactcgaaatgcatatttggttgagccggcaatggcgctggcaatgctggttttcccagttcccggcggcccatataaaatcattgacgacagcatcttggcacgcaccatccggtcgattattttacctgggccaactaaatcctgctggccgacaatttcttcaagcttggtcggtcgcattcgataggcaaggggttgttgcatactcatcctcctctcaaattgtgatggttaaaaatcaaatcctataaattataacatgatcgtgagggcacaaaaaaagcgttttgcataagcaaaacgctcgctgaatgattaacccaacttgttgtagtattcaacaatcagtgattcatcaatatcagcatcaagttcttcacgttgtggaagacgaaccaatgatccttcaagcttgtctgcatcgaagctgacgtattgtggacgacccacaacagcttcaacagcatccttgataacttggaggtctttagacttctcacgaacagagattacttgaccaggttgaacttcatatgatggaatatcaacacgtttgccatcaacagtgatgtggccatggtttactaattgacgagcttgacgacgggtagtagccaaacctaaacgataaaccatgttatccaaacgctcttcaagtaagatcatgaagttaacaccatgcttaccttcacggatcttgccggcacgaacgaacaagttactgaattgacgttcagtcagtccgtacatgtaacgaagcttttgcttttcgtgtaattgcaaaccatattctgaaagttttgaacgacggccttgaccgtgatcaccaggagcataaggacgacgtgagagttctttaccagtacctgataaagagatacccaaacgacgtgaaattctccaacttggacctgtatatcttgacataagtaatcctccaatatttttttggagtaaaataagccgttgcagacttagtattcgtgcatgttgctttgctctttcgctcaagcagccgattgagttacttgcagaaccaattgaatggcaacaacatgttgacgagcttaccgtctactgctgcgttattttacacaaccaccattgtataaagatttctactgtaagtcaacatgtttgacgaagatgtcggcaaactggttaagaacctgctcgtcttcactcgaaaaacgatcgagtgatggcgaatcaatatctaagacaccaagggctttgccgtctttaaacagtgggacgaccaattcagaattggaattggcatcacaagcaatgtggccggcaaattgatgaacgtcggcgactcgtagtgaatgcttttgtttgagagccgttccgcagacaccgtcaccatttttgatatgcatgcaggcaacatttccctggaaggggccgaggattagttcatcgttagcgggcacataacgataaaagccgacccagttgatatcttcgaggctgacttggagcaatgcagtggcgttagccatgttcgaaatcaaatctgtttcattttctaaaagtgaatcaagctgttgattcactaaattagtaacgttttgcataattgttttcctcacttcaaaaataatatggtgaaaaggacctactatgatataattcaacttagagcacattaattgattattcatacatattaaattgttttgggcaattttactaccataatgttcaattatatatctttatttctgaaggatgggatcgaatgcttactttgttgattggaattatcgtgttggttggggcgggttatcttggttttgttttctaccaaagaagaacaatcaagatggcaaccgatgtttacgagaacaaacgggacttaaataaaattccgttggatgatgagtttgcgctggctaagaaaatgaacttaaccggtgaatctcacaagaaatatgatcaattatacaataagtatcagcactacaagaaccaaatgctgcccaatattgatgaggggattgcggcagtcaaagaagacggtaagggcattaactttttaaagaccaagagtgactggcagagtgccaatcaggcaatcgccgacgctgacgccaccttaaaagaaattcaggccggccttgctcaactatatgatttaaacaagcagcacaaattagcgctggaagaactcgaaaagaagtacaaacgcttgcgagaggacatccttaacaagaacgagtcatttggcccgagtatcgacagcttggaaaaaatgctctcggacattgagggaactttcgatgaatttacacaactcacaaagagtggggatcccaacagcgccgaagaagtgttgagtgatctcaacaattcgactgacaaattggaatcctatatggggcgaattcccaaactatatcaactactttcaaaggaatttgttgagcaggttgacgaaatcaccagtggttacaaggaactcaaaggaaaacagtataattttcccaacgataagttcgatgaaacgcttaaggggatttcagatcagataaaagtcaacaccaataagctaaagactttggaagttgattcagtggaaaaagccactcaagatattgccgaccggatcgacaaattgtatgatgcaatcgaaaaagaattccaagcccgccccaaggtcgagaaaaatactaagattatcggccaatatatcgaacatgtccgtaaacagaacagcgacttgcagctgcggcttgaaacgctgaataaaagctatattttgaaccatcaagaaattgagaataatcatcaatttgatcaacaaattgccaccattgaaaagaagtaccaggatgaagtcaacgccatgcaaaatgggacggctgtttattcaacgattgacgccgaccaaactcacatgatcaaagagctgggtcagatcgagtctgaacaaaaggatttgttctccgcaacagttaagttgccagagcaagagcaggcagccagaaatgcattggccaaatttgatttggcaatgcgcaataccaaacggcgaattgacaatcacaatcttcctggactatccaacgattatcaagatgcttttacggcagtcattagagaaatcaatcacctggacgatgccatgaatcagccgcagattgatgtcgatgacatttccaaacagttaacaattattcaatcggatatggacactttggatgaaaagaccaaccagttgattgatgatgccactttggccgaacagacaatgcagtatgccaatcggtttattggcagcaactctgaaattgcggcggccagcaaaacggcccagatgtattttgaccaaaaatatgattatgagcagagtttgaatattatttccaaagcattggaaaaacaatcgtcggggatgtttgccaagatcaaagatgattatttcaatgctaagaaacatttaaagacagaaaaaaccgatgaagatgaatcataatatgacgtatgagacgaagctgaatgtttaccaacagcttcgccttttgttttccatcattgattgcccagcgacaatgcttgtgagactcacagtttgggtgtatcatcgtgggagttatatttgttggagtcgaaccaataaatttagagaagaaggtttcaaatgatttattttgacaatagtgccaccacaaaagtcttaccagaagttcttgacacttataacaaagtgagtgagcagatttggggaaacccgtcgagcttacacaactttggtgaacaggcgtttaatctgttggaacagtctagaaaacagattgctgatttgttaaacgttcacccagatgaaatctactttacgagtggcggaactgagggtgacaattgggtcatcaaagggactgcaattgaaaaacgtgaatttgggaagcatctgatcaccacctcagttgagcatgcagcagtgcgcaactcttttgagcaacttaaacagctcggatatgatgtgacctatttaccggttgatgatgaggggcggatctcgattgctgatttgaaagcggcaattcgtccggatacaacgctggtatcgattatggcggtcaacaatgaaattgggacgattcagccgatcaaagaagcgggagaactgctgaagaactacccgaaaattcattttcacgtcgatgctgttcagggcctcggcaagggaattcaggatcagattttcaatgaccgaactgactttgcagcattttctgggcataaattccatgccccacggggaaccggctttatatatggtcgccgtggccgtcgaattgcaccgttaatgaacggtggcggccaggaaaagaatcaacgttccggtactgaaaatctgccgggaattgctgccatggccaaagcgatccgattggtgcttgaaaaagaacctagtgcaattgatactgagcgccagattaagcagttaattatggatcacatcagtcagtttgataaagtcaccattttttccaagaatgatgatacttttgccccgcatattctttgttttgcaatcaagggggttcgcggagaaaccatcgttcatgcttttgaaaagcaggggatttacatttcaacaaccagcgcctgctcatcaaaggatcatactgaatccggcacgttgaatgccatgcaggttcccgatgatattgctaccagtgccgttcgaatttcacttggagatcacaacacacttgatgaagccaaacaattcgtaaaagtatttgaccagttgtatgaagaatttgacaaattaagttaggagtaactatgcactatacagaaattatggttcgttatggcgaactgtccacaaagggcaaaaataaaaaagactttattaagcagcttggcaagaatgtgcgggctgttctccacccatttcccaagcttgaggtcaagccgcaacgggatcgtcttcatgtggctctaaacggtgaggatgaccagcaggtgatcgaaagcctgaagggtgtttttgggatcgaaaatttctatccttctgttcggcttgaaaaggatatggcaatcatcaagcagaccgctcttgaaatggtgaaagaacagtatcatgacggagcgacgttcaaaatcaacacccgacgtcaggataaacattttgaatacgataccaatcagatcaacaaccagttaggcgattatattctcgaaaatgttcccggaatcacggttgatgtcaaacaccccgatatttccattcgagtagaaattcgaatgaatggtgcctttctctcatcagaaaagattcatggtgccggcgggttgccggttggtaccggtggtcgggccacaatgatgctgtctggtggaattgattcgccggttgccacgtatttggcaatgaaacgtggtgtcaaaattgatatgattcacttttacagtccgccatataccggcgagcaagccctgaataaggccaaacagttaacctcagtgttgggcaagtactcgggtaatattcagttcattcaggtaccgttcaccgagattcaagaaaccatcaaggaaaaggtccctgaaggttatttgatgaccatccagcggagaatgatgctgcggattgctgcccaaattactcaaaatcgtcattgtaccggcgtctttaccggcgaagcactgggacaagttgcctcacagactttagagagtatgatggcaattaacgacgtcaccacgatgccggttcttcggccgctggtctcaatggacaaaacggagattattaagatttccaagcagatcaagacttacgacctgtcaattctgccatttgaggactgttgtacgatttttacaccgccggcaccaaagactcggcctgatttggccaagtcacgtaagtttgaacagtatatcgatgttgaagggttgatgaaaaaagcaatcgacaacattgaaattaccgatattaaacctggcgaagaattcctaaaccaaaaccaggacgtcttcgctgagctgctttaatgatcggggacttgcgtattccgtttgtttaggctacattatgtataaagtcgttagaccaagggagtgcttttatgaaaatcacgatcaatggtaaagaagagagtatgtttggcaatccacccgaagtcggtgaacaactgccaaagtttaaacttgaggatgcagatggcaataaggtgaaaactgctgacattattggcagaattaccctgctgtcaacggttccggatattgataccccggtttgttcagttgaaacccgcaagtttaaccaggaagccgacaagtttcctgatgtccagttcttaacggtttccaacaatacgattgaacagcagaagaattggtgcgctgctcaaggggttgccaatttgcagatgctgtccgacgaaaacctctcgctgggatacgcaatgaaactttatctgccaaactttggtgcgttggcgcgaacaatttttattattgacgccaccggtaagattatttaccgtcagattgttccggaaattgggaatgagcctgattacgatgatgcactaaatgctttgaaaaaagttgctcagcgtattgacgattagcagatatttagttaagattaaaattaaattaaagtgttgagcaagagagtagccaacgtttcggtttcagaaagaaaatcattgctgtgagatttttaccgggcgttgagtgaaggtagcttgtgagctgcttatcttcaattgaagatgagtcggtattatcagaccgttattatgatattaagtggggcttttcagcccaatttaggtggtaccgcgaacacttcgtcctaatttacaggatggggtgtttttttattacataaaaacgatttgaattttggaaggagtgacgttatgtcagacaaattgcacgaaatgtcaacgaagtatgatccaactgccgttgaaaagggcagatatgatgaatggcttgatgaaggggtatttacaccgagtggggataaaaaggccaaaccattttcaattgtgttgccgccgccaaatgttaccggaaagctgcatttgggccatgcctgggatacaacccttcaagacatgattattcgccgcaaacgaatgcagggatacgatactttatggctcccaggaatggaccatgccgggatcgctacccaagctaaagttgaagccaagctgcgtaaacagggtatttcccggtacgatttgggccgagaaaagtttgttgaaaaggtctgggaatggaaagatgattttgcccgaaccatcaaggaacagtgggccaaattaggtctttccctggactacagtcgtgagcgattcaccttggataaaggattgtccaaagctgttcgtaaggtctttgttacgctttacaataaaggcctgatctaccgcggtgaatacattatcaactgggatccgcaagcaagaactgccttgtcagacattgaagtgatccataaggacgataaaggtgccttttaccatgttaaatacccatttaccgacgggacgactttcaacggcaaagattacatcgaaattgcgaccacccgtcccgaaacgatgatgggtgataccgcggttgccgttaatccttctgatgaacgttataaggatatcgttggcaagaaagtccgcgttccattgattaatcgtgaagtgccgattatagccgatcagtacgttgaccctgactttgggacagggatggtaaagatcaccccagcccatgatccaaatgactttaaggttggtaatcgtcacaacttacaacgcattaatacgatgaacgaagatgcttcaatgaacgaaaatgccggtaagtataaaggcatggatcgttttgaagccagaaaagctatggtcaaggatttgcaggatgaaggcttgatgctctcaatcgacccaattgtccattcagttggacattctgaacggactggggttcaagttgaagcccgtttgtcaactcagtggttcgttaagatgaagccgctggctgaacaggccattaagaaccaggataccaacgacaaggtcaactttttcccagaccgttttgaaggaacctttgaacagtggatggaaaacgttcacgactgggttatttcccgtcaactttggtggggtcatcaaattcctgcttggtacaacaagcagaccggtgagacctacgttgggatggaagcgcctaaagacgccgaaaactgggagcaggatccagatgttttggatacctggttctcgtctgccctgtggccattttcaaccatgggctggcccgatgaaacagaagacatgaagcgctatttcccaaccgacaccttggtgaccgggtacgatatcatcttcttctgggtttccagaatgattttccaaagcttggaattcactcatgaacgaccctttaaagatgtcttacttcatggtttaatccgtgattctcagggacgcaagatgtccaaatctcttggaaacggtattgatccgatggatgtcattgataaatacggtgccgatgcccttcgctggttcctgtcaatcggtgggacgcctggccaagatctgaagttcagttatgacaaaatggactctgcctggaatttcattaacaagatttggaatgccagtcgttacgttattatgaaccttgatgggattgacaagccggaattacccgacaagtccgagtggcaattatctgacaaatggattttaagtcgactgaacgctactgtgaaccacgtttcagacttattcgagaagtacaattttggtgaagccgaccgttatttgtatgacttcatctggaatgatttctgtgactggtacatcgaaatgagtaaggaagctctcaacagtgacgatgagaagttgaagaagaacacccaaaacattttggcttacgttttggatcaaaccctgcgcttactgcagccgatcatgccatttgtgaccgaatatatttggcagatgatgccacacgttggcaagtcactggtaaccgccgactacccagtggaccacaaagaatttgacgatccaacttctgagcatcagatgcagtcactgattgatttgattacagcagtgcggaatattcgaaatgaagccaacgcaccgctgtcctcaccaattgatatgttaattcaaactgacaatcagaccctcaaatcaatctttgaatccaaccgcgactacattgaccggttctgccacacccaggaattgcaaattggcaaagatattgaagcgccaaagctgtcaatgtctgcggtgattacggatgcgactgtctttgttccattggctgaattggttgacttgaaggatgagcaggcccgggttcaaaaagatgttgataagtttgaagccgaagtggcccgttcagataagaaactggctaacaaacggtttgtggagaacgcgccggatgcagtggttgctgaagagaaggccaagcaggctgattaccaatcaaaattggatgcagccaaagaccggctccaacaaatttccagtgagatgtaaagtgatttaactgactttaatttttaaaaacgtgggactaaatgctgtttcctggcacatgccaggctataagccgcatttttgcccacgttttttaaggagaaaataatgattaacacatatgatgaagccttggctttcattcatggacggaccaaattcaagaaaattccaaccttaaaacggatgcggcgattcttagacgaattgggtgccccggacaaacatgtcaatgccatccacattgccggcactaatggcaagggatcaaccctggcatttttacggaacttgtttcaagcggaaggcaaaaccgtcggcagcttcacctcaccatttttgattaaatttaatgagcgaatcagtgttgacggtgtcggcatttccgacgatgaaattctaagactcactcaggaaatttatccgacgattgccaaacttgacgccgagttgccggaaggcggcccaaccgaatttgaaattgtgacagctatgatgttcaagtactttgctgaaggacacgctgatattgttttgatcgaagttggccttggtgggctgtatgattcaaccaatgtcattatccccaaagtctcggttattacgtcgattggctgggaccacatgcacattttaggggatactttgcccaaaattgctttccaaaaagcagggattattaagccgggcgttcccgtagtcgtcggcggagttgaccccgaaccgctcaaggtgatcgtaaatcttgctgagcaaaagcaaagcccgattcagattctggggcagaattttaaggtcaatgatcgcggtgagcacaattgggttcaacaatttgactttagttccgccgactttcaattgcatgatttaaaaacagccttaattggtgattatcagactcacaacgctgcgttggcgatccaggcatacattgactaccaccagctcacaaagcgctctgtggatgtcagaaacattcaaaagggaattgcagcaacacggtgggcgggccggtttgaaaaaatttcggccaaaccgaccatcgttttggatggtgcgcataatatctcggcagttagcctgattgtcgataccctgcagaacgattttcctcagggccacatttatattttgatgggcattctggcagacaagcaggctgataaaatggtggacaagatggccaccgttcaaaatgcatcgatcatcttgacccagttcgccggaccaggaaaacggctcgcagccaatccagaaaaattggaaagtcaactgaaaacccaaccggaaaatgtttccgctattgatgattggcaagacgcaatcagggaattgagacggaaactggcgccggatgatatgctcttaattaccggatcgttatattttatttccgatgctcgaaagttcttgttgaatgccgatcacaatttcaaataatctattaaatcgggcgtcgtttcacttgattttatttatttttggacgcgttatgatatacttgtttcgttaaacaataataaatcaatctataaaaatcgaactaaattaagttgatagacaacgaagggatggataacgtgtttggatttggggaaaaaaacataggaattgatcttggaaccgctaatacgatcgtttacgtcgagggcaaaggaattgtccttcgcgaaccttcagtagttgccaagagcactaaaacaggcgaggtaatcgccgttggtgcagaagcgcgagcaatgattgggcgcacaccagcaagtatccaagctgttcgaccaatgaaagacggtgtcattgccgattacgataccactgttgccatgatgaaatacttcattcaaaaagccttgggacactcatcaggtaagccatacgtcatggtttgtgtgccaactggcattactgccgtggaaaaacgggctgtcattgatgccacccgggtagccggtgccagagatgcctatgtcattgaagaaccattcgctgcggcaatcggtgctggacttccagtcatggatccaaccggtagcatggttgttgatattggtggtggaacgactgacgttgcaaccatttcattgggcggcattgtttcaagccgttcagttcgaatggctggcgacaagcttaacgaagcgattgctcaatatgttcgtcaaaagtacaatttgttaattggtgaacggacttccgaacagcttaaaattgatatcggttccgcttctgccaaggaagctaaagaaatcaaagccgttccggttcgtggccgtgatttggtaaccggtttgccaaccacagttgaaattagtggaacggacgtcaacaaagcaattaacgaatcagtgttggccatcattgccacgattaaggaaacccttgaagaaacatcgcctgaaattgcagccgatgttattgatcatggaattgttctgacaggcggcggcgcattactcagaaatattactgatgtgattgcggaagccactcaagttccggtttccattgcatcggatccacttgattgtgttgccatcggtactggagaatcattgaagagcattaatgtaatgaagaaaaaacaataattaatcgtttatatcgattcattattgaataacgaatggaggcaattatgcaaaaatttttctccagtcgaaagcttgtgattgtcgtaatctgtttgatcgtcagttttggtttaatgtcgttgtcggttgccattcgggacaagcggagcacaccgccgttggtacaacaatttggaaatgatattgttggttttgctgatcggattgttgccgccccaatgaacggtattcatcacggatttgtttcaactaagaatcttttgaacacttatcaggaaaaccaacgtctcaagtcaaaagttgatcaattgacccaaacacaggtcaaggatcaggttttgtcgcgagaaaataaacaattgaaacgtcaattaaacgtcggcagcactttgaccggatatgaaaaaatcaacgcagctgtcattacccgaacaccatcatcatgggcaagtcaggtgatcattaataagggtcaagcttctggtattaagaaggatatgcccgtgatcgccggtcctggactgatcgggacagttgctgaagtcaacaaaaccaacagcaaggtggttttaatttccaacaccgccgaaaactccaaccggtttgccatccaagtgcttggtgataattccaaagttgttaatggtattatcacctcgtatgattcggctgccaaccggattatcatggggaatattacctcgaacgccaaattatcagttggcaatcgggtgacaaccagtgggcttgggggcgtcattcccaaggggatttacgtaggtactgtttcaaaagtgacccaagacgattatggccttgccaaaaaagtttatattaaaccggctgccaacttaaacgacattgaagttgtttcagttgcaatcagagattgatgggagggacaattaagtgaaacgaaaagttcccattgcagtttactttgtaattggtcaattcattgcgttctttcttgatggttccatcagccagacaatgtccggtattttgtttaaatatcccaacacgatggtgccatatttaaccgtcctctggttgattttggcagccttctttggtaatggcaaaaaattacatctatacacctggtccgctgtgattggctttatttttgatatgtactacactggattgcttggggtatacgtgtttattttcccattagtcgtttatttatgccaattggtttaccaaattttgccaccaaatttcatgagtggctttttggtgtattttttaggaatcacagttttagttagcctaggatacatggccaatgtctttattggggagacggactcatccgttgctcagttcttagttaacacattggcacctacactggctctcaatctggtgttattgacaattgtttactttccggttgaggcactctataggactcataggcaataagaaggggagtagacaatgcaagatgcagctgtattaaagggcaccaaggatggttatgaaatcattctggatgagaatgccaatctaaaggatattttttcctcacttcgaaaacttctggataatttgaaaacccagacggcctcaactaatccgcaaaccattgcttttgatatttataccggaatgcggttatggccagctgctgaccgttccgaacttgagaaaatcttttcagattattcgacgttttcagtgcataagattacgtcagatgtgatcactaaagaggaatccaatcggattttggaacagtccagcgtccacattgttgatcgggtgattagaaacgggcaggaagttcacatccaaggcgacgtcttatttctcggcacggttcatgagggcggcaaactgtttgtcggcggtaacatttttgttctgggcaacgtccagggaattattcaagccggcgcaccggatcttgaggacaagatgattattggggatgtacataacgcacaacaagtccggatcggcgaacagttcgaaatagttgctgacatgaaacgtgaaatggacagcggcacagtgatttatgtgaacgatctgcatgtactggattatggtaaagttgagaatcttaagcagattaatcccaagttttacaatcagataggaggagtcatcaatgggtaaggcttacgttataacatcaggtaaaggaggagtcggtaagaccacttcttctgctaatattgggactgcactggccatgctcggtaaaaaagtggttcttttggatcttgatattggattgcgtaacttggatgttgtcttgggactcgacaatcggattatgtacgacattgtcgatgtcgcggctggacgagccaagctcagtcaagcactggtcaaagacaagcgttttgatgacttgctttaccttttgccggcagctcaaaatactgataagacggccctaaatgaagaccaggttcgcgaaattgttgatgaattgaagccggactttgatttcatcctaattgattgtcctgccggaattgaacagggtttcatgaacgcaattgctggtgccgatagtgccattattgtgacgactcctgagatttctgcggtccgagatgctgaccgggtggttggtctcttggagcagcatccgcttcaagaacagccgcatctgattattaaccgaattcgtcaacatatgatgaaagacggttcggtgatggatgttgatgaaattacccatcatttaggggttgaactattggggattgtctttgatgatgatgcagttatcaccacttccaataacggcgaacccgttgttcttcaagcggaaaaccctgctggtcagggatatcgagacattgcccgacgactagtcggtgaatctgtgccattgatggaaatcaaagatgaacagcagccttcattctggcaaaaagtgagtcattggttccgtaaaggataaaagtccttgacgggaagcagaattaatattattataaatctaacttaattaaagatttttaaagacgttgatcagaaccgattaatgaatcaaatcacagagagcttatcaaggtgggagttaagcatttgagcattaatcgtcacatctgggagtcatttttctgaagctgagtaggaaaaagcggtaagcacgttattgctgaagtttagtatgttgcatattaaacccattgaggcctttcatgtgagtgagaggtgaatcagaggtggaaccgcgaataatcgtcctcttaagtcatcatggcttaagaggatttttattttaaaacaagactaaacttcacgaggcagcaggtgtgaatctgttgcgaattgaggtggaaccgcgaaaaccatcgtcctcttgagtcaatgtgtactcaaggggatttttttatggagggatgtcaaatgattcaatatatacaagaaattttaccggcgttattatctggaaccaaaatgactttatcaattttcttctggacattgatttgttcaattccattaggggcattagtcggattaggactcatccaaaaatttaaaccgctgacctggctgcttaacttttacgtttggattatgcggggcacaccactgctattgcaattaatttttgtcttttatggcttaccgattgttcacattgtgttccaacgttacgatgctgccatgtttgctttcatcttgaattacaccgcatatttcggtgaaatctttcgaggcggtttccaatcagttcccaagggccaatttgaaagtgccaaggtgctgcgattgagttatggacaaacgattcgaaagatcgtgattccccaggttttcaaaattgttctgccatcaattggcaatgaagtgattaacctggtcaaggattcctcgttggtctacgttatcgggttgggcgatttactgcgagccggaaacgtcgcaacggccagggatgttacgctgttgccgctgatattagtcgggattatctatctggcattaaccgcggtatgtacgattgtgttgaagttaattgagaaacgtgaaaatgtttggcgttaggaggggattacgatgttagagattaagaatttaaccaaacgatttggcagccgaaccattattgatgacttgtcgatgaccgttaaagataatgaaattatggcaattgttggcccttccggtgccggcaaaacgaccctgttacgttgtattaccggtttggagtcggtgaataccggggaattttactggaacggcactcagtttgatccaaccaacacgactcaaaaagacacgatcatcggggtggttttccaagattatcagttattcccaaacttaacggtcctgggaaacattactttggcaccaacgatggtcaaaaaagaaacgatggcagacgtcaaaaaatatgcgcgggaattattgagtcgcttgggcttggaaggcaaagaaaatttatatccttatcagctttccggcggccaaaagcaacgggtggcaatcgttcgggcactggcaatgcgaccgaagatcctatgttacgatgagccaacgtcggcccttgatcccgctttacgagatgaagttgcccaaattatcttggatcttaagaagcaggaaatgacccagatcgtcgtcactcatgatatggattttgctaaaaacgttgcggatgaaattcagcaggtcaaacaaattcagtaggaggggtaaaatgttaaaatctttgaaacgattattactcattaccagtctcctactcgtgaccattgggttatccggttgcggggtacgctatgtcagtcgccaaggctcacaggaaaatccggatacgtggtcgacggtttccaagcaaaaaagaatcgtggttggactggatgacagttttgtcccaatgggctttcagaccaagagcggcaagattgtcggctatgatgtcgatctggcccgtgccgtgtttaagcaatacggcatcaaagtggattttcagccaattgattggtcgatgaacgtcaccgagcttcgaaacggcacgattgatcttatctggaatgggttctctattaatccccagcgagcaaagaagattactttcagcgaaccctatctaattaatgatcaagtattggtttccaaaaagaatcaacatatcaacagtttcgcagatatgaagggaaaagtcgccggcgtccagagtgggtcggcaggggccatggatattgataaccaacctaaattgctgaaagataagatcaagggccacgagccaatcttatacgacacctttacagatgcgttcatcgatttgaatgccaaccgaattcagggattgctgattgacagcatttatgccggttattatttggaacatcaaccaaatcaatccagttttaagtcgattcccagtgaatttcctaaagaagaatatggtgtcggcatgcgaaaaggtgatactgtcttgaagcggaaaattgatcaaggtctcaatcgattagccaaaaacggcgagcttcacaaaatcaacatgaagtggtttggaactgatcgggacagtccgctcattaagaatgctaaataattttgatcattagtagtctgtggcaaatgtgatttgtcaacagactatttttgtattcgaatcctttgccgatcaattctctatttttccttattattggcagattatattgagattttaatgattttattttatgataaaatttgtgactaattgaggaggaaactcagtgaaatacgagattgcaaaagggattagcttgacgacaattcccaccacaaaattcaaaaataataaattggtgatgaatttcacctttccggcccaacatcaaaactacgccaaattggcactgttggctgaactgctggaaaattgctctgcccaatacaacagtgagttgttggtttcccgccaactgtcaaaaatgtacggggccagttttggtgtgactgtcttacggtatggcaatcagcataccctgcaggtgtcgattacgtttcccaatgacaagtacctaccgccaaaaagtgagctaactagtgaaatattggcatttctaaaggaaatgattgaggatccatttattgaaggcgatcagttcaaccaagcatattttcaaattcatcaagggaatatggttcattatctggattcgatccaagataacaaggagtttttctcaaccttggagcttcaacgtttgtattacccaaatgatcctgaccacggtcacttcctgatgggcagtcatcaagaaatgagccaaatttctgctcaagagctgtacacattttatcgatgggtccttaactcagcgaagattaccatcctggctggtggcgatttagttgacgaccaactagtaacgggatttaaagaatttacctcatttactgatcgaatgccggaagactatcaattaagagttgtgccggcaccaatatcgaaggtccaacaaggaaccaaagtgattgccggttctcagtcagttctcagcatggcttacgaactaccaatctattttggggacgacgactactttgctgccgtcatttttaatcagttatttggtgggtcaagcagatcgttgctatttacaaacgttcgtgaaaagaacagtttggcctacgacattcatagtggctataattcattagtcggaatggtaaccgttcaggcggggattgattttaaggatgaagatcgcgttattcagatggtcgccgatcaattgcagcagaccagcgacgggcaatattccgatgaattgctcgacggtgtcaaacaggcattgattaaccaacatcgttcagaagccgatcacctcggatcattaatcgagaagcagtatctccagcagatgatgggctttagtttgagtgataccaaatgggagcaacaggtcgcttctgtgacgcgttcgcagattgcccaagttgccaagcggttgactttacgagccatttatcagttgaacagcaggggggatgcataatggaattgattgactatccaaactacaatgaaaaattatttgttcagaccctctcaaatgggttgaccgtttatctccaacccaaagcagggtttaataagacgaccgctgttttgggggtgaattatggctccattgacagtcagttcatgctcaatggcgaaaaagttgttcaacctgcaggaattgcccattttttggagcataagatgttcgataaaaaggattacgacgtttttgagctgttcaataaaaccggagcgcgttcgaatgccttcacaagttttaccaagacgaattacctcttctcaactgccgaatccgtgaaagaaaatttggatattttgttggattttgtccagattccatattttacccaagctaaagtccaacgtgaaaagggaattattgatcaagaaatcaatatgtatcaaaatgatccggacaatcaggcgtactttaaaacgattgccagtttgtatccaaactcggtgttggcaaacgatattgccggcgacattcagacggttgataagattaccctggaagatgttgagttggcttatcgaaccttttaccggccggaaaatatgagtctgtttatcaccggcaaactcgatcccagcgaagttatgaactggattgaggataatcaacggcgaaaatcgacaccggcacccattagcctgcaacgccgactgacgctccccgaggcatccaaagaaaccgttcttcacacgaaaatggatgtttccaggcctaaaataacgctggggctacggggaagcgaccaagtcccaacaggccgggatggactaaagtacgaaatcgccatctctgtgatgtttgatctgtttttgagtgaaaactccgtggaatatgataaactgtatcatgatgaaatcattgatgacacgttttcatgggaatttgaaaatgaacgcggctttcattttgccgtgattaacggcgatactgataagccattggaactcattaaccggctcaaacaaatcattgcagatattccaaccaagattggtcacctccaaaccgaatttcagttgcaaaaaaacgagttattcggcaactacatcgaaatgatggattctgaagaagcgatcagtggccagtttgacggatttatcggtgaacctgttacaatatatgatgaggttgagattctcaaatcattaaccttggaggatgtttttgaggcggcccacagttttttggaccaagcaacagttcaagaagtgatgattcaaaattccgaccagccaaagggatagttgataaattatagtttatgaattacttaaaataatcaaggctttccttatgatatacttagtggagaatacaaaaaattcaatggagaatgagtatgagcgacgaaaaagataatttaacaattgggaaaaaactacatgacgcacgagtggccaaaggttacacgctggatgatttacaaaagaacactaagattcagaaacgctatctaattgcgatcgaagataatgattttgacgccttgccgggtgatttttatgttcgagcatttgttaagcagtatgccgattcggttggtctggacggaagtgagctgctaagccagtttgatactaaattgcccgataccgaagacccggaatatgtggatcgggtcaatgatgacaaccctgagacgagatctgctcaacgaaaggttgaagaacgcaatgataaactgcggcgctatattccgattatttcggtgtccgtcgtcgttttaatcattttgattgctatttgggtggctgcggctagaagtacccgaaacactgccaaaacgcaaattgagaccagcaaagtttccgtttccggcgacaaatcatccagttccaaggcttccagttcgaagaaagccaagacgactaagaaggccaaggggattacctttaagaaggttactgcttctggcagcaatctgacttaccgagtcaccggaacttccggtacaacgccactgaagatttccgtaaccggttccgggagtgcctggacgtcggtttctgcagatggcacttctttatggcaagcttcattaaccagtggtaattcacatacaatctcgcttccaagctcgaccaataccgttacgattaatactggcaacgctgaagcgacccggattaccgtgggcggcaagaagttgacgttggcggcaccgttaaatggcggttcaactcaggtgagagttgtcacattgcagtttggcaagtcaagttcatctgcttcaaccagctctagttcaagtagtgccacgacgggtgcctcaactaccaatagcacaaccgggacgagtggcaccactggaacgtcctcaacgactggtactgacacaaccggcaacacgaatgcaacaactggcagcactggtacgaataataataccggtaccaccaatggctattagtcagctggaggtttaacatgaatttaccgaataaattaacactatttcgaatcatcctgattccgttctttatcctgatcctcgcggtcccaatcttttccggcagcgttgtttgggcgggaaccacgatcagtatgaccagattgtgggcgacaattatttttgtggtcgcctctctaaccgatttcttagatggtcagattgccagacgaaatcatttggtaaccaactttggaaagttcgccgatcccttggcagataaaatgctggtaatgacggcatttctgtttttggttggcctgggggatgttccggcatgggtcgccgcgattattgtctgccgtgaattggcggtaaccgggctgcggctaatcattgtcgagaacgaaggccaagtcattgctgcggcctggccgggcaagatcaagacaaccactcagatgctggcgatcattttactgttcttgaacaacgtcttatttgatgcagtcaacattccaatgggcttaattctgttatacatttgcctattcttcacgatttactcaggaattgattactttgtaaaaaatcgctcagtattttcagattcattttaatcacagctgccggagggttcatgaaaatgagtcttccggtatttgtgtcttgttagataaaaaccaagtatttaacgtacttatgaactagagggagcaactaagatgacattggaagagacattagtaaatgaactattatcccgacacattacaattacagcggctgaaagtttaactgccggtgaatttcagagcactctcggtaatgtgcccggcgtctcagaagtttttgaggggggatttgtcacatactcaaatcaggttaaagaacaactactgcagataccaagtgaagtaattgatgaaaatggtgtcgtgagtgaaccgactgccatttggatggcaaatcaggcccgaagcatcatgaataaagatctgggcgtatcctttaccggagtggccgggccggacacgttggaaggcgatcctgctggcacggtctggattggcattgcctatgggacccaacatacttatgcgaaacagtttcatttcacgggggatcgaaatcagattcgggctgctgcagtcaaggccggcttggagatggcgttggacatgattcatcgttattaaattaatcgaacttttgttcgcgttttgattgcttttttggataatcattagtatagttagtaagtaaacttttccgttaaggatagtgggaggaatttaatggctgaccaaagaaaagtagctttagataaagccttaaagaatattgaaaaagaatttggtaagggatccatcatgagaatgggcgacaaagccgatactcaaatttccacaattccatctggttcattagcgcttgatgatgcactgggagtggggggatacccacggggcagaatcgttgaaatttatggacctgaaagttcaggtaagaccaccgtggcgcttcatgcggttgccgaagttcaaaagcgcggcggcacggctgcctacattgatgccgaaaacgccctggatccggtttatgcaacccacttgggcgtgaatattgacgatctgttactttcacaaccagatactggtgaacagggtcttcagattactgacgcattggttaccagtggggcaattgatatcgtcgtcattgattcagttgctgcattggtcccccgagctgaaattgaaggagaaatgggggatgcccacgttggtctgcaggctcgactgatgtcgcaggccctccggaaactttctggaacgatcagtaagaccaagacgattgccattttcattaatcagattcgtgaaaaagttggtgtgatgtttggtaatccggagactacccccggtggtcgtgccttgaagttttatgcgacaattcgactcgaaatccgtcgggctgaacagattaaggacggtaccaacatcattggtaaccgtgtccgcatcaaagtcgttaagaataaggttgcaccgccatttaaacgtgctgaagttgatatcatgtatggcaagggtatttctcaatctggcgaattggttgatatggctgttgaaaaagacattattaacaagtccggctcatggtattcatatggtgaagaaagaattggtcaaggccgtgagaatgccaagacttatcttgaagaacatcaagatatgtatgacgaggtgatgaagaaagtcagggctgcctacgacattcctgatgaaactgactcggacacctctgatgacaaagccagttccgataagaagaccgataaaaaagccgacaaaaaggattccaaaaaggaatcggcaaccggttcttcaaaagaaaccaaaactgatagcatcgatcttgatattggcaagtaattggcactaccaaatgcaaatagatttcgttaatgggcactcagaggagctgcccattttttgtgagttaatcaaggcacagcgggcttttgtgaaacattttaaaagaaaatatggtcactcaaaaatcttgttatatacaaataccaaaaaccgcaacgtaaagatgattgacactagtgttaacaaacattaaaataagaattgtgtcaataatcaaataacatctaattggtttacaaataatcattttttgatgatttggaggtgaaaagccatgaccatggctgggataatcctcgcaatcatcgctataattgttgttggttttgttggtattttaagctttgtaatcggcaagtctgcacaaaagaagatccatgagaaagatcttgactctgccaatgggtcggctaagaacattttgaccgaggcccagaagaaggctgagacggttgtgaaagaagcaactctatcagctcaggagaagaaccaccgttaccgttcatcggttgaaaaagaactgaagacgcggcgtgcggagattcaaaaacaagaggatcgtttgctgcagcgagaagaggctcttgatcgtaaagacacggctttcgaacgtcgtgaaagttcgttgaaccgaaaagagcagaagattaatcgtgaacaacagaatttagttacacaacaagaagaagcaaactcacttatcgcaaaacgccaggccgaagttgagaaagttgctgctttaacgcaagaagaagcccgggacctgattttgaaagaaactagcgaaaagttggctgacgaaaaggctcgaatggtaaaagaaagttattaccaagcccaaacagaagctgatgaaaatgccaaaaatctgataattgaagctattcaacagagttcagcggacgttgtctcagagacaaccgtttccgttgttagtcttcctaacgaagacatgaagggacgaattattggccgtgaaggccgtaacattcggactttcgaaacgttgaccggcattgatttaatcattgacgatactccacaagcagttgtgctgagcggctttgatccgattcggagagaagttgccaaaatgacacttgaaaagttaatcaaggacggtcggattcatccggcacgaattgaagaaatggtcgaaaagagccgtaaagagcttgacgagcgtatccaagaaattggggaagagacgctattcgaccttgggattcattcaatgagcccagatatgatcaaattagttggacaactcaactttaagattgatcatgggcagaacttgctgagtcattcaattgaggtcgccaagttggcgggtgcttttgcagcagaattaggtgaggatgttactttagctaaacgcgcaggattattacacgatatcggtaaagctgccaataatggtgttgagggatcacatgtacaggttggtgttgatttcgccaagaagtatcatgagagtcccgttgtcattgatgctatcaaaggttatgaagaaggccacaatccagaaacaattatttctgagttggttgctgttgcggaaaagatcgcgatttcgcgtccaggcgcacacagtgaatcacttgaaagctttgttcatcgacttgatagtcttgagaagatcactgacagctttaacgaagtacaaaagagttacgcaattcaagcaggtcgagagatccgtgtgattgcaaagcccgaagatataacggacacacaggcaattgtgcttgcccgtcagatcaaacaaaagattgaaactgagatgaagtatcctggacacattaaagtaacggtgatcagggaagttcgttcagtcgaatacgcaagataaaagatcagagtctctggtcttttttcttttataaatgttagaattattttatattattcagaaagtatcgaggaaaaatacatgcgaattctttttatcggtgacgtggttggcgacaagggtgtttcaatgattggcaattatctgccaagactcaagcaggatctgaaaccccaggtcacaatagtgaacggcgaaaatgcaacttcaatgggtcgcggcatcactttgagtatctataagcaattgatgagtgatggtgtggatgtggtcacgcttggaaaccatgcttggagcaataatgaaattctcgacttcatcgatgatactaaacggctgattcggccgtacaattttcccaaacgaacaacacccggaaaagggtataccatggtcaatgtcaacggcaaacagctggctgtcctgaattttcaagggcgcgtcttcatggacaaccttgacgatccattcgagctggctgacgaactggttgaagagattcgaaagacgaccaattgcatttttatggattttcatgccgaagccaccagcgaaaaattagcaatcgcccgttatttggacggccgaatttcagcggtggtggggacacatacccatgttcaaaccaatgacgcacggattctccaaggcaagacggcctttttaaccgatgccgggatgaccgggccggctgacggcatgttgggcatgcagccggacagtgtgattcaacgcttcttagatcagcgaccagcccgatttaaagttatggaaaccggtcgcggaatcatttccggctgcttcgtcgatattgacgataagaccggtcacgcgacccatattgaaaccgtgtcgatgactgatgatcaaatttaattgtgttttataatagtttagacgatactgaaatcgaattcagtgagaatttaaggggactttcagttggcaaaaaaagaattaactccaatgatggtgcaatatcaaaaaatcaaggaccagtatccggatgcttttttgttctaccgtctcggtgatttctacgagatgttcaatgaggatgccatcaagggttcacagttattggaattaactttgacgaaccggagccggaatgcggccaatccggttccaatgtgtggtgtgccccacaaagcggtgcaaaattatattgatattctagtcgaccagggatacaaagtcgcaatctgtgaacaaatggaagatccacgattggctaagggaatggtcaaacgagaagtcattcaattggtgacaccggggacgcaggtggatgttggcagtgaaaacgccaagtccaataactatctgactgcggtggtggatgatcaaaagaatcatgagttcgctttctcatacgccgatctttccaccggtgaacttaaagttgccaaattaaccacgcaggctgaatttgttaacgaattggtttctttgcagactaaggaaattgtcgttgatactgatttaccggagtcaattcaagatacgattcaaaaattggggattttgatttcccatcaatcggttctgccggtcaatgcctcagtcagttacttaagccaggacgttgatgacgacttgatgaaacgggtcgtcaaactcctgttggattatatccaagcaacccaaaaaagaagcctgcagcatttaaagcgggcagtgatttatgaaccctcagattttttggaactcgaccacaattctcaatacaatttggaattaatccgcaatattcgcacaggtaaaaaagccggcactttattgtggctgcttgaccaaaccaaaactgcgatgggcggccgaaaactcaaacaatggattgagcggcctttggtgaaccgcaaactgattaatcaacgccatgatgcagttgccgtgttactggatcactatttcgaacgaaatcaactccaagacgagttaatcaaggtttacgatctggaacgattggcaggtcggatttccttcggcagtgtcaatggccgtgatttgattcaactcaaggcttcgctcaagcaggttccgaagattaaatatattttggagcaaatcgccgacaagagttttgaggctatgctcaaaaacctggttcctttggatgatgtcgttgacgaaattgattctgcgatcgtcgaggaaccgccaatttcagttaccgatggtggtgtgattaaggatggctacaatcagcagctggacacttaccgggacgctaccaataacggtcaaaaatggttggctgaattggaagccaaagaacgtaaaattaccggcattaataacttaaaagttggttttaatcacgtttttggttactatattgaagtcaccaaggtcaacttggacaagattccagcaaaccgttatcagcgcaaacaaactttggccaacgccgagcgattctcgacgccggagctgaaggaaaaagaagcgctgattttagaggcccaggaacaaagtaaaactttggaatacaagctattcgttaagatccgtgacgacattaagaaatccatcaaacgaattcaggatttagcagatgccgtagcgtcaatcgatgtcttacagagctttgccgccgtcagcgaggagtaccgatttgttcgaccaacgcttacgacgcatcacgtggttgaagtcaaagatggtcgccacccagttgtcgaaaaggttttgggccaccagcaatacgtcccaaatgacgttaatctgggcgaagataccagcatcctactgataaccggtcccaatatgtctggtaaaagtacctatatgcgtcaaatggcactatgcgtcatcatgaatcagatggggtgttttgtgcccgccaaacaggccaaactgccggtgtttgacaaaattttcaccagaattggggccgctgatgatttgatctccggccaaagtacgttcatggtcgaaatgaaagaagccaacgatgccattgagaatgccactcccaacagtttgattttgttcgatgaaattggtcgggggactgcaacctacgatgggatggcgttggctcaagcaattattgaatatgttcataacaacattggtgctaaaaccctgttttcaactcattaccatgaattaactgttttggatgaatctctcaaacgactgcaaaatgtccatgtcggcgcgaccgaatccaatggcgaactggtttttttgcataagattcagccgggccctgctgataaatcatacggaatccatgtggctaaattggcaggcctgccagaagggttattacatcgcgctaacgacattttaaccaaccttgagcaacaggccgacaaagagcatcaaacagcttcggcaccaaaacaggcccctcagcaggcgcctgagcagcagacgtctttatttccacttgagcaaattgatgataaacaagccgaagttgtgtcacaattaaagaaattagacttgatgggaaagactcccatgcaagtgatgaatcaagtttacaaatggcagcagaagataaacggagactaaggtgattgatttgaatgaaattcataagctaccaacaatcctttccaaccagattgccgccggtgaagttgttgaacgaccggcatcagtggttaaggaattagttgaaaattcaatagatgccaagagttcggaaatcgatgtcaccgttgaaaattcgggcttgaagttgatcaaagttgtcgatgacggcaacggaattgacagctctcaagttcagacggcctttttacgacatgccaccagcaaaatttctgagcaacgggatttgttccgcgttcggacactcgggttccgtggcgaggcactccccagtatcagttccgtcgctaacgttcggatgaaaacgtcaaccggctcgattggaacggaagttgaatacaaaggcggcaagcttgtcactcaaaaggcttctgaatcacggaaagggaccactgttgaagtggcatcactgttctataacacgccggctcgtttgaagtatttaagctcaccgaatacagagctttcaaaaatatcagacattgtcaaccgcttggcattgagtcatcctgagattgcgttttcatttatcagtaacggccgtgaattgttaagaacgtccggacgtggtgatttacgccaggttttgggcgcaatttatggtgtcaagacggtttcaaagatggcggcaattaagggaaatgatttggacatcaaagtcagtgggtatgtgagtttaccggaattgacccgttcaagtcgaaactatatttcactgattttaaacggacgctttattcgcaactttccgttaaccaaagcggtgattgcgggctatggttccaaattaatgatcggacgatttccgattgccgtaatcaaaattgacgccgatcccgctttgatcgatgtcaatgttcatccaaccaagcaggaagttcggattagtgacgaaccgatgattggtaaattaattgccaatgccatttacgacatgctaagagacaagcagctgattccagatgcaaccagggatttcaaacagccggttcaagctgcaccaagacagtttgatgtttcgactgccacccaggctcaaacgaatccaccgctgtttgccgtcgacacaccaacgacgccttcaatttcccaacctgaagtaacgccggtggtggtcaaaaccagagacgaccttgccagctcacaagttgctcaatttgatgactttcttaaaaatgagccgagtggcttgcctgcatttgaaggaacccagccaaaaacgattgacaatcaccagtcaagtaccaagcctgagcagtctgaactggtagttgaaactggttttccgcaccttgactatattggtcaaattcatggcacctatctggtggctgaaacagctgataatatgtatctggtggatcaacacgcagctcaagaacggattaactatgagttttaccgtaagcaaattggcgaagtttccgatgaccaacagaaattattggtgccaattgtgctcgattactcaacctcggatttcttgatgattagcgaccgtttggacctgctggacaaacttggaattcatttggagccgtttggacagaacagtttcatcgtccgtgagcacccaatgtggtttaaagccgggcaggaagaagacaccattaaagaaatgattgactggattttatccgatcataaaatttccgtggccgctttccgcgaaaaaacggctatcatgatgagctgtaagcgagccattaaggcgaaccatcatcttgatgagctccaggcaaaggccttactgaagcggctgccggagtgtgagaatccatataactgcccccatggccggccggttctggtgaaatttactaacgaggacattgaaaaaatgttcaaacggattcaagacccccatcatacagaccaagaaatcatctagattgttgcccagtaccgagtgagatatggtacaatttattggcaaacatacgttttagtgaagaggagaagttgatgtttgaatttttggaagggacggttgttgatatcacacccacccacatcgttttattagtgggcggcgttggttatttgatcaataccgcagacccgtaccgttttaatgttgatgagaaaaaagtcatcagagtctatatttatcagtcagtgagcgatacggctatcttgctgtttggctttgcgaccattgaagacaagcagatctttgaaaagttgatttcggtttccgggattggccccaaaagtgctttggcaattttggccggcaacgaccgggatggattgatcaccgcaattaataatgaagacgtcaagtttttgacgaagttccccggagttggtaagaaaactgcccgccagattattttggacatgcagggaaagctcgacgacattgcaactaatggtgcttcgctggcccaaccgcttggcagtcccgaaaagtctcctgaattggccgatgcgttatcggcattggaggcgctgggttatggtgccaaacagattgccgccatcgagccggatttagttaagcaagctgatttgtcaaccgatgaatacttaagtttaggattgaaactgttaatgcattagggatgaggagatgatccattggccaatgaaaaagatgatcgattggtttcaccagagaatgtggatgccgatgagaacagcattgaaaaatcgcttcgtccccgagttttaagtgagtacattgggcaggatgatgttaaaaacgagttaagagtctatatcaaggctgctaagcaacgtgaggagtcattagaccacgtgctgctttacggacctcctgggcttggaaaaacaactttggcgatggtgattgccaatgaaatgggcgtcaatattagaacgaccagcggtcctgccattgataagcctggggatctgttgtctttactcaatgaacttcagcctggcgatgtcttgttcatcgacgaaattcatcgactgcccaaggtggttgaagaaatgctttattcagccatggaggacttttttgtcgatattatcgttgggcagggttcaggcgcccacccaattcattttccactgccgccattcactctgattggtgccaccacccaagcaggaatgctgtcggcaccactgcgtgatcggtttggaattgtagagcacatgaattattacaatgcgacggatttggaggatattgttcgccgaactgcggatatttttcaaattgatattgaggactccggtgcccatgagattgctttgcggtcccgaggaacacctcgagtcgccaatcgcttgttaaaacgggttcgagattttgctcaggtatccgacaaagaccaagtcgatttggcaattgtcagatacgcgttggcaaagttaaaagtcgacgatttagggttggatgccactgacctgaaactattgacgacaatgatcaagtattatgatggtggaccagttggcttaaacaccctggccgccaatattggcgaagaaaccgacacgattgccgagatgtatgagccttatctgctccagatcggtttaatcaaacggacagccagaggaagaattgtgactcccaagggatacgctcatttgagttatccaatgccacctcaggacgaaaggaattagaatcttgaaaacaaattacacccttgaagactttgattatgatctgccacatgaattgattgcccaaacgccgattaaagatcgcgatgaatcacgactgctggtgttggataaagaaaccggtgagatgcaggaccgtcatttttacaacatcattgattatttgaatcccggggatgccctggtgatgaatgactcaaaggtcatgcccgctcgaatatacggtgtcaaagccgataccggcggccacatggaagtgttgctgcttcataatattgagggcgaccgctgggaaactttgatgaagccagccaaaaaagccaaggtcggcacggttatcaattttggtgatggccaacttaaagctgttgtgaccaaggaattggatcacgggggccgcgaaatcgaatttaaatacgatggcatttttatcgaaattctggagcggctcggtgagacacccttaccgccgtacatcaaagaaaaattagatgatcctgatcgctatcaaacggtttacgccaaagaaatgggctcggctgccgctcccacggctggtttacactggaccaaagatttacttaaaaaagtcgaagataagggcgttcatttagtttatctgacccttcatgtcggcttggggacatttcgaccggttgatgaggaaaatattgaagatcacaaaatgcacagtgaattttaccgtttgtcagaccaggcagcggccacgttgaattctgtccgggataatggcggaaaaattgtggcaaccggaaccacgtcaattcgaacgctggaaacggtcgggaccaagtttgacggtcaaattcgccccgactccggctggacggatatttttatcaaaccgggataccagtggcgggtggttgattcatttatcaccaatttccatttgcctaaatcaactttggtgatgctggtggcatcgtttaccggacgggaaaacatcctgaacgcttatcagcatgcaattgacgagaaatatcgcttctttagttttggcgatgcaatgtacattcactaggaggattattatatgcaaccagcgataagttatcgcttgattaaaaaggagaagcacaccggcgcccgcctgggagaaatcaccacgcttcacggaactttcaaaacgccgatgtttatgccggttgggactcaggcaactgtgaaaactctggctccggaagaattggagcaaatggggtcgacaattattttggcgaacacctatcatttatggctgagacccggagaagacatcgtcaaagaggccggcggtctgcacaaattcatgaattggcacaagggaattttgacagattccggtggttttcaagtcttttcgctggctaagaatcgtgatattaccgaagaaggcgtgaccttcaaaaatgaaattaatggttcaaaaatgtttctgtctcccgaaaaggcgattcagattgaaaatgatttgggtcctgatatcatgatgagccttgatgaatgtccaccattttttgagtcgtatgattacgtcaaaaagtcagttgagcgaaccagtcgatgggcggaacgtggactgaaagctcaccgaaatcctgactggcaggggttgtttgggattgtccaaggggccggttttgaagatcttcgcaaacaatccgcccgcgatttggtcagcctggattttccgggttactcgattggcggattgtcagtaggagaatccaaacaggaaatgaatcgtattctggaatccaccagtccacttttacctgagaataagccgcgttatctgatgggtgttggagcaaccgattcactgattgacggtgtgattcggggcattgacatgttcgattgtgttctgccgactcgaattgcccgtaacggaacggtgatgacgtcccatggccgactggttgttaaaaatgccaagtatgcccgtgacttcacaccgttggatgaccagtgtgactgttacacctgccgtaactacacgcgggcatacatccgtcatctgatgaagaccgacgaatcgtttgggatgcggttgtgcagttaccacaacctttattatttaatccatttaatgaaacgggttcaacaggcgattgttgacgataatctgttggacttgcgggcagaagtttttgaacagtatggatataacaaaccaaatccaaaaaacttttaggtgtagactattcagggcttatttggtaaagtattactatggaaagtgtgggtgaaaaattttgaatcaatcttattactcaattttaatgattgttgtcttgtttgcggtgatgtacttcttaatgatccgtcctcaaagaaagcaacaacaaaagcgtcgggatcaactttcaaagatcaaggaaggcgaccaagtgattacgattggccggctccatggtgtcgttgacgaaatcaacgaagccgaaaaaaccgtgactttggattgtgatggtatctacttggtatttgatctgagcgcaattgcttcggttaagcagcctgctgttgctgcgcctgcagcaaacaacgatacaactactactgcaaatgatgatcacaaagatgacgctgcttcatcaaagagcgatcaggacgctaccgaagattctgataccaaagatgaaacaaagtcggaagacaaatagtttgaccaagtcggttgggaagttgatttctataatcccgaccatttttttacccggcaaagaacatatgtttgattggggtgatctcagtgaaaacatcggctagaaacatcatccatgtggatatggacgccttttatgcgtcgattgaggaacgcaaagaccccactctcaagtctcaacccttgattgttgccaaggatccgcgcaaaaccggcggcaggggagtggttgcaacggctaactataaggcccgtcaatttggggtacattccgcaatgagtgtcatgaaagcgctggaactttgtccgcaggcggtttttcggttctctggatttgatctttaccgctcagtttccaatcaaatccacgagatttttcacgagtacacggaagtgattgagtacgttgccttggatgaggcttatttggatgtcactcataataaaaaacatctcacagacccgattcaagttgcccgaatgatccaaaatgaaatttgggatgccacccacttaacctgttccgtgggagtatcttacaataagtttctcgccaaagaagcctctgattacgccaaaccagtgggcattacagtgattgaacagcgagatgcattagaatttttaagccgtttgccaattgaaaagttccgcggcgtcgggaaaaagaccgttcccaagatgcatgaattaaatatcaataacggtcaggatctgattcagtggtcgcagatggatttgatcaagcactttggtaaatttggttacgttctctatcagcgcgctcgaggcattgacgatcggccagttgagtatcagcgggttcgaaaatcgattggcaaggagcggacatttggcccggcgattgacacacaaaccgaagtcgatgacgaactccagcgaattgctgcgatggtggtcaaggcaatggatgacaaaaagaagcacggtaaaacattggttcttaagatccgttatgccgacttttcaacgtttaccaagcgggtcacgatggataactatcttaaaaatagccccgaagaatactttacacttgccaacgatttactggtcgatatgccggatatttcaaaaggggtgcgcctgttgggaatcaccattaccaacctggatgatttaacttacgagaacattgttcttcacctgtttgattaattcaccaccccagcggtttatcttattcacaaagtaatgtatacttaagtgttcgacaataaagttatggagcaaataaaatgtcaattcaagatcaaatattaagtgaaatcaaaaaatttaaaaccattattattcatcgtcacaaacggccggatccagatgccatcggatcgcagatgggactggctcaactaattaaggggtcatttcctgataagacagtcctgtgtgctggtaaacaatatgatagttttgcctggttgggaaccaccgatgaaattgccgacgagcaatataaagatgctttggtgatcgttgttgatactgccaatcagccgcgtgtggatgacgaacgttatacgacgggaaaagaattgattaagattgatcatcacccaaacgacgatcagtttggtcacattatgtgggttgagcccgattcatcaagtacatctgagctgatttatgatttttatgatgccaatcgtgatcagttaactttgcccgatgaaggtgcccgactgctttatgccgggatcgtcggtgatactggcagattcatgtatccttccacgtcgccacatactttggcagttgcttcaaaacttgctgaatatcagttctcaaccagtgaagtcaacaaaatagaagacgagatcgacattccactggcacggctgtccgcttatgtttatgagaacctgaatattcttgatagcggtgccgcttatctggttttgtccaataaagtattagagcccttcaagttaggggacgaaagtacttctgccgtcgtgccgttacctggcaagatcaaacaagtggtttcttgggcaattttcgtcgaacaaaaagatggctccttccggattcggttgcgctctaaaggaccagaaatcaacgaattggccaagcagtatggcggcggtggccatccactcgcaagtggtgctgttgtcgaagatgaagcccacatcaaggaatttgtgagcgatttgaatgatttagtcgccaaaaacaagtaggagattatatgagtaatttttcagaatttaatttaaagccattcttattggatgctgttaaggagctgaacttcagccacccgacacccgtccaggaaaaggtgatgcccgttatcatgcagggaagagatgtcgtgggccaatccgctactggtagtggtaagacccatgcttttctgctgccgatttttaaccagcttgatcccgcaaaagatgaggttcaagcggtgatcaccacccccagccgggaattagcctatcagatcattgatgccgctaagcagttggctaagcactcaccagaaccaatttctaccggtgcctacattggtggaactgacaaggcccgtcaggaaaaaaagattcaacatgagcagcctcaactggttgtcggcactccgggtcgaatttgggatctgatccaaaacggtggactggatgttcacacggcttctcagttagttatcgacgaggcagatatgaccctggacatgggattcttggatgtggttgataacattgctgccagtttcgggaaacatgttcagatgatggttttctcggcaacgatcccacaaaaaatcaacgtctttttgaagaaatatatggttaatccttttatcgaagagattccagtgtcgacaattatcagtccgacgatcgataattggttgatttcgacgaaggggcaggacaaaaatcaactcatttataaattgctgaccattggggaaccttatttggtcctgatttttgccaatacccgcaaacgagtcgaggagttaaccgaatatttgaagggccagggattgaaagtcgccatgattcatggcggtctcaagcctcgtgaacgtaagcaaatcatgaagcgggtcaaaaacctcgaatttcaattcgttgtcgcaactgatttagctgctcgagggattgatattgaaggggtatcggatgttatcaatgatgatattcccaccgaggatttggaattcttcatccatcgtgttggtagaaccggccgaaacgggatgtccgggacttcgattaccttgtattctcccgatgaggaaaaagaagttgaagaacttgaagatatgggcattcatttccaaccgaaagcccttaagaacggcgaaattgtggattcttatgatcgaaatcgtcgaaagactcatcgaaagaaacacgataagctggatccaacgatgatcggcatgatcaagaagaaaaagaagaagatcaagccgggctacaaacggcgaattaaaaataccattgcccgaaaggacgagatggatcgtcgggttgctaaacgtgaggaagcacgggccaaacggaaacaacgtaagaatagttcttcacggtatcaataggtctgtattgacaccatattcacaaaaaagtatactttgagatgtgttaagaacatgccgtttaattttttgtttcagagacgttttggttggtgagaaaagcgacgaaaattaaacggtgctctcttaaaagttaaattatcaaacgcaactctgcgttatagagatcaagtggttaacgataaacatcgttgcaatcagagtggtaccgcgtcaatgggcgtctctgtgagcaacggtgttttaattttgtcaaaggagaagagaacatgaaacagttaagcagtggtcaaatcagacagatgtacctcgattttttccaggaaaagggtcataccattgaaccaagtgcctcactcattccagtcgacgacccaacattgctttggatcaattcgggtgttgccactatgaaaaagtattttgacggttcagttgtcccgaaaaacccacgaatgaccagttcacaaaagagtattcgaaccaacgatattgaaaacgtcggtaaaacaccccggcaccataccttatttgaaatgttagggaacttttcagttggtgactatttcaaaaaagaagccattacctgggcctatgaactgttaacttcacccaaatggtttggctgggatcccgataagctttatatgacggtttatccgaaagataaagatgccaaaatgtattgggaaaaagtgggcgttgcgcctgatcatatcattgaaattgaggataacttctgggatattggccagggaccatccggccccgattcagaaatcttctatgatcgcggcaaggactttgacaatttagctcctgatgacccggaaaattatccgggtggtgaaaatgaccgctggctggaagtttggaacattgtgttttcacaatttaatcacaccccccaagatacttacgaaccacttcctcgaaaaaacattgataccggaatgggccttgaacgagtggtttcaattttccaacatgcccgaaccaacttcgaaaccgacctctttttgccgatgattcgcaagactgaagaattaagtgacaataagaaatacgataccaacaagaaggataacgaagccttcagaattattgccgatcatgcccgggcaatcacggttgctatcggcgatggcgcattgccttccaacgtcggccgcggctacgttatccgtcgcttgatccgaagagcaatcgttaacggtcagcggcttggaatcaacgaagcgttcttatacaaattggtcccagttgtcggccagactttggaatcatattatcctgatgttcttaagcaaaaggattatattgccaaagttgtccgttcagaagaagatcggtttaacgaaacgctgactgacggcttgaaactgttcaatcaagtggtaaaagacgccaaagcaaatcatcaaacgaccatcgatggcccaactgccttcaaactctacgatacgtatggtttcccagttgagttgacggaagaagaggccaatgatgccggcttatccgttgacaagccaggctttgaggttgaaatgcaaaaacaaaaagatcgtgcccgaaaggccagaagtggtgccaagtcaatgggtgttcaacgtgatctcttaattgaaatcaaggatccaagcgagtacgttggctacgataccttggatgtcgatcacgccgagcttttggaaattgtcgagaacgaaaaactggtcgatcattcaaagggtggctctgttgaagtgatttttgatagaacaccattctacgcagaaatgggcggccaagttgctgaccggggagttgtccttgatgaagagggagacaaggttgccgatgtcgttgacgtccagcatgcacccaatggtcagaatttgcacacattaaaaactcaggaaccactcgaaaagggcaagacctatcacttgattgttgacaaattattccacagtcgcgttgagaagaatcacacagcaacccacttgttggaccaatcattgcgaaatgttttgggtggacacacccaacaagctggttcactcgttgaacctaactatttgcggtttgattttaaccactttggccaggttacggatgaagacttacagaaggttgaagatatggttaaccgtcaaatcttcaatgaaatcgatgtcaacaccgttgtcacggatcctaagactggtaaaaagatgggtgccattgccttatttagtgaaaagtatggcgataaagtacgtgttgtcagcattggcgacttctcagttgaattctgtggcggaactcatgttaacaatacccgcgacattggcttattcaagattgtctctgaatccggagttggggctggtgtccgccgaattgaagcggtcacagccaaagatgctttcaagttgttgaacgatcatgaaaaggaactgaaacaaattgccggcgacttgaaagtcacccaaattaaagacacacccaaacgggttgaccaactactgggcgaaattaaggatcttacccaaaaacaacagtcactggaagccaaattggctgggcaacaggctcaaaatgttttcgccgacaagaaaactgccggtaagtattccattatcaccggaatcatcaaagatgccggaatggatcagctgcgccaattagctgatacttggcgctctaagcatttgtctgacgtcttggttcttggaaccggcagcggcgacaaagcaaacttgattgtcgcagtggcagatgaacagatcaaggcgggcattaaggctggtgatctgatcaaatcgatcgcgggcaatattaaaggtggcggcggcggtcgtccaaacatggctcaggctggtggcaaagatcctgctggccttgataaagcgatgagcgcagcggttgattggttggcaaataaataattattacaccacggttacatgtcggttacattggcttacttgattgtagtttcacttataatcagttaaaattaatacaaatgaccttaagtcatagaggtgaattgtatgagttcgttagataaaaccatgttttttaattttaatgaaggtcagccaaaagacgtccgcgaaacattgttgactgtgtatgcagcactggaagaaaagggttacaatccatataatcagattgttgggtacttgatttctggcgatccagcatacattccacgtaaccttgatgcgcgaaatcttatccgccgacatgaacgtgatgaaataatcgaagagttagttcgtttctatttggataatcatccaaccgaaacgaaaaaaggtgaaaaatgagattaatgggtttagatgttggttcaaagaccgtcggggttgctgttagcgacgagttgggctggacctcacaaggggttgaaataattcgaatcgacgaggacaacaaggaatttggtttagatcgggtttccgagttggttaaaaagtaccaagttgatggatttgtcgtcggccttcccaaaaacatgaacaattctttaggcccccgggctgaagcttcacaacagtatggcaaacgacttgaagataagtttaacttgccggttgattttgaagatgaacgattaacgactgttgaggctcagcggatgttgacagaagaagcagatgtttccagggccaagcgcaaaaaagtgatcgataagctggccgctggcttgatacttcagaattatttggacagcaatggtaaattaactaaaatatagcgaggtaaacaattatggcagaccaagaaccagtacaacaacaaattacattagtcgacgaaaacggcgatgaaactttatacgacgtattattcacttttaaatcagaggactttgatcggtcgtacattctgatttatccagatggcaaaggtgaagatgaagaagtcgaaattcaagcttatgcactgccaaagggtgatgatccaagtgatcctcaaggtggagaacttcaagcaattgaaactgacaaagaatgggatatgatcgaatcagttttgaacaccttcttgggtaaagatggcgacgatcaggatgatgacagcaacgacaatcaataattaaagattgtccctattgcgaaaggattgaggcgaagcatcgttgagtctcagtcctttttaattgaaagaatttaggatgtgatgtaatgtctagtaacgaaaaacgtcgcttcaaaacaaccattgatggcaaggattacgtgcttgtcggtaagggatcggttgatcatatgcaggcggtgtccgatttattaaatgagcagctcaagcaacttcatgaggctatgccaactgccactgatgagcagcgggcaatcctaattgcctttaatgcaatctccaaacaatttgatgttgaggaaagcgcacacagtaaagaggttcattagatgatttttacaattgggatcattctgattttaatatttggctttttccgtggccttcatcgaggtttcgtgaatgaagtcctaagtctgattggctttttggcggcaacaatcgtcagtatcgttggaaccagtccaattgctgactttattaatcaggcaatttttaaaaacggcggcaatcaaactgctgagttgattatcaaatgggtgatctttgccttcctttttgggtttgtttggcggattgttcgtttgctgagtgatctattatctccgatcacccgcctgccattattacatcaattgaacgcactactgggtgcagccgcagatcttctcatcaagtatttgttcattttcatcttgctgaactttctgctgatgttccctgatcagagcattcaagaacagtaccaacaatccgacgtttcccagtggattgtgaaaaaaacaccgattctctcagataaaatgattcagatttggaatcaacattctagtgaggttaatgtatgaacgaaaaagttttagaaacattagagtatggaaaaatcaaggagcagctggccaaatatctgacgaccgaccgtggccgacaaattgtcgatttattgacacccagtccttcctttgaaaccgtttctcaacgcttggcacagacggccgatggggctgacattgtccgcttaaagggagaaattccgattccaaaactcgcagatattgcaccgtatatgaaacgcctgcggattgaaaatgcgtcattaagcggaactgagctgtctcatatcaccaaattactacgcgctgtgcaggtcgtcactgaattttttaggggtttggcggctgaagaagtgactttaaaatccgttccctcaattgtcgatcggctcacattgatgcctgaagtgaccaaacgaatggtggcttcggttgatgaagacggccgcattctggatggcgcttcttcgcaattacgttcaattcgccggaccattgctgccactcaaagtaatattcgttcgaaaatggggaagttcattaagggttcagatgccaaatacctttctgagccgattattaccgtccgtgacggtaggtttgtcctgccaatcaaggccgaatataagcagcgatttggcggcatcattcatgatcaaagtgcctctggccaaacgttgtatgtggaaccaaacaacgttgtcgaaatgaacaatcaattgcgtcgggatcagcttgctgaaagagctgaagttcggcggattttggcagagttaaccaatttaattcgcccgcatcgtgacgagttgttggccaacatggatttggttggccaattggactttgtgaacgccaaagccaaatttgcccatgcgactggtagtgtgatgcccaaagtgtcaccgaaaaatgttattaatctcagaaaggcgcgccatccgttaattcccagagatcaagtcgttgccaacgatattgaacttggcgatcagtacaatacgattattgtgaccgggccgaataccggtggtaaaacaattaccattaaaacagtcggcctcctgcagttaatggggcagtcaggcctgtttatcactgccaatgaagactctcagatcggcgtgtttgataacgtctttgccgatattggtgatgagcagtcaattgaagccaatctgagtaccttttcatcgcacatggacaatatcattagtattctaaaacagaccagtaaagatagtttggtcttgctggatgagcttggtgccggcaccgaccccaaagaaggggccgcactggcaatggcaattattgatgcttttcatcaaattggcggtgaactgattgccacgactcattatcctgaattaaaggcgtttgcttacaaccggcaggggattattaatgcatccatggagtttgatgttgagacactccagccaacttatcgatttttactgggaattcccggtcaaagtaacgccttgaacattgccagcaaacttgggatgccagaggccattattgaccaggcacgggcgtttaccgactccgagaaccaagacatcaataatatgattgaagagctgacagcgcaaactaagcgggctcacgatgaagctgatgaattagatcaacaactgaaagaatcaacccggcttcagcatgacctgcaagacaagtttaccaagtacgaaagtcagaaggaacggctcgtcgaacaggctaagcaacaggctaatcaagtggtcgaagaagctaagaagaaggccgaccgaattattgatgatctgcatcaaaagcaggcccaggtcggcaaagttgccgttaaggaaaacgagctgattgatgccaaaggggcgctcaatcaattggaatctgctccaagtctgacaaagaataaggttttaagaaaagaaaaggccaagcacgatttccatcccggcgacgatgttttggtcaaatcttatggtcaacaggggacgttgctgaggaaggataagaaccatacgtgggacgtccaaatcggcattttgaagatgcagattgaagaatctgatttggaaaaggcaactccagccaaacaagataagaatcagtatcagacccacgtgtcccggaccaggtcgactgggatgtcaccgaccttggatctgcgcggtcaccgatacgaagaagcaatgacagaagtcgatcgctacattgattcggccctacttgccggctacccttcagtgacgattattcacggcaagggaaccggggcgcttcgtaaaggggtcaccgaatatttgaaacgaaacccacgggtaaagagttttggctattctgcaccgaatgctggtggggatggttcaacggttgtgaagttaaaataaaaatgattgtgtgcaatctgtttgctttttgctaaaaaattgttagtattaaactattaaaggattggagtgttttaatatgcttaaagaaactacggatcaaacttttgaaaaagacactgccgaaggtgtcaccttaaccgatgtttgggcaacttggtgtggcccttgtcggatgcagacacctgtcatcgaagagctggcagaagaaatggataatgttaagttcactaaaatggacgccgacaaaaacccggaaactttatccaaattcggtatcatgagtatcccaaccttgttggttaaaaaagacggcaaagttgttgataccatcgttgggtatcatccaaaggcccaagttaaaaaagtgcttgatcaatatgccggctagtctttagaatgacttcggtgtctcaagcggttcacagtcaaaaagcccaccgcaaaaccaaatcaggttttgtggtgggctttttgattccaatgagttaatcatcaggcttggaattgtcatcgggatcgggttgaacgatttcaaatatagcagaagcttcttgaccatcagttggcttgtcagggctcaaataggtgcttaaaagcacaaatcccttattaacattggccttttcgagctcagcttcggcttgttggttaagaatatactgacagctttgagcgatgaatccggattccagataaaaatcaggatcatcaaatgcgttgagacgctgggcgacgatcttgccgcttagcttccagctgatctggttaccagagcgtttaagtagctttagatcaccaaatttaaattgtttgaaaaaggtttccaaatcttcataggttgccagacgatgatttcttgccagatgcttgccggcccaataggaaatttcgtgggcgtctttgcctaaaatctcaggaatcagtgaatcgcgaattaattcctggcccagtaggtctctcattgtatcgtcagtcataaaatgcttgtatacttcgttatccattttttaatctccatcaatgcaaaatgtaataaataaattatacaataaaatcattaatcttgttttgtaagttgaagtaaagattcttttgcaagataataatgttattgagacaaaggaagaaggaattctgttggataatcggccgattggcgttatggactcgggggtcggcgggcttaccgtcttaaaggaaatcaccaaaatcctcccgaatgaatcgtacatctttattggcgatcaggccaatttaccgtacgggcaaaagagttctgaaaccgtcagaaaactcacaaaaagaattgcagactatctggttgaacaaaatatcaaaatgtttgtaattgcctgtaacacagctactgctgcggcatatgaatatttaaagaaagttttaccgattccggttatcggcgtaatcgaaccgggtgcccaaatggccgttaaagcctctaaatccggccagattggtgtgattgccaccaacggcaccgtccgctccggagattatcagcgattgatcaaacaagccaaccgatcagcagttgtgtcatccttaggctgcccggaatttgttacgatggtcgaagaggggcttgccggaaccgttgaagctcaggttgcggtgaacaaccgactggcttggtttatggataaaccgattgataccttggttatgggctgcacccattttccaattttaaaaaatgaaattcaaaatgtgatgggcaacgccgtcacgttgattgacccgggagtcgccactgctcagcaagtcaaggcagatttagcagctcatgatggttttgcccccgatcaaaaacagcgtgttcgaagattttacaccaccgggaacccggcggatttcgccaaagttgccgacaagttactgggaacaccgatcagtgccgttaagttagatatttaaaggagtttgataacgtgaaaagacccgaatcgattgtgattgcctcacaaaacgctcataaaatcattgaatttgaggatgcttttaaaccaaccggtatcacaattaaatcactgaagcattttgaaaatgtgccgacgatcgctgaaaccggcaccacatttgaagaaaatgccaccctcaaggccaccggcatcatgaactttacgcatcaagcggtgatcgctgatgattccggcctggtggttaaagcactcaacggccaacctggtgtccactcagcccgttatgcaggtgatcacgatgatgacgccaacaacgataagcttttgaaggaaatgcaaaacaaaacggatcggacggcttactttgaatctgttctggtctatttaacgcctgagggtgacaaggtggttgccaacggtcgaatcgacggcgaaattttacgtgaacgccgtgggaataacgattttggctatgatccattattctatgtgcccagccagcagcgaacactcgccgagatgagcacccatgataaaaatctgattagccatcggggcaatgccatccgcaacctgatccgtaaattgttggggttgtgggactcatgaaaattgttgttgttagtgatagtcatggagatcgcgccattatccaagaattggtgaacaaatacgccggtcaagtggatgccattttccattgcggcgattctgaattaccggcggacgatccattagtttctcaactgcggattgtccaggggaatatggactttgccgaatttcccgaccacctggttcaagaaattagcggcaaacgaatcctcttgacgcatgggcatcatcaaaacgtgaatggtggcatgcttaatttggaattatatgcccggagcttatccgccgatatcgtcctttttgggcacactcatcaattaggagctgtttttgacgatcagatgctgtttgtgaatcctggaagcattgcctatccacgtgggcaatacgccgggttgggcggtacctatgccattatcagcatggatcaacgcaattacaccgttcaatattacaaccgccaatttgaaccggtggcgaatttggaacttcgttttccgttctaaccaaaaaggagtctaggattacatgatcgataaaccaattgagaccgtgatgcgtgaaagtcaccgggatattttaatccccgctgatttggtcgcaactgtcaatcaagacaatgatctccaacacgtcttcatggttttgacgaaagttaaatacgcaaaaattcccgtgttagataacgataaccatttcatgggactggtttctttacccatgattactgaactcatgatgcaggataccggcattaccagtcgaccgcttgagtcagtgaaagttaagcaaatcatgcaaaaggatgtcccaacgatttacgagcgggataacctggaagccattctcaggtatttggtggatgaaaactttctggtctacgttgattctgaaaatcactttaaaggaatcattacccgtcgggaactatttaaagaaattaattatttggctcacaactttaataaacactacatcgctttgccggtgtataatcacaaatccaaaaacgaaaccaagcacgccaagattcaaggctccaagggtctgattaatcgataatccattgggtgaatatcgttgatggttacaaaaatgaattaagtcaaaaaacgagattactgacaaaatttgccggcaatctcgtttttctaataattggtcactttattcaaacatcagttggcttgtccattcaccattgttgggctcgccggcagttgaatcccggcctcattaattgcagctagatagaaggccaaaaagttatgggcaacttcgtactggctgccgttttttgtggtgatatttacctgaacaaccagtttgccgttggggaggctaatggtgccaagaatcttgggatctccgataatatccggatagtgggggatctgttcttcattgacctggcggataatttgggtgactttatcaactggcgtttgtgggaaaatgccaacttgaatcatcgccgtcatattgtttcgagacatgttggcaatggtggtgatggttcggttggggatgaaattcaacgtgccgtcgtccccgacaacctgcgttgttctcagtccgactgcagttacagttcctctaattgttccaatttggacgtattcgccaacttcaatttccttttcaagaagaatgaaaaagccactgacaatgtcagtcacaaatccttgggcaccaaggccaattgccaagctgaagatcccagctgaggcgaccagggttccaactggcaccccaaccgttgagagaatggagtaaatccagaagaaccataggcagtagttcaaaatgttcagcgtcagggtgtgaaaggtcttgatccgtttttctgctacggtattttgatatttgcgccgatagcgtttgaaaaaatgattaatcagtcctttaccaatccgacgaaagagtaaaaataacagactgaataaaattaataatccgactttttccagaatcgtcatggccagctgatcccagtcaaccatgttgagatatttttgccaattaatggctaaaactgtgaattttaaggtatttatcattgggattcctcgctttgtgtataatatcatcttagcaaattggttctacaaaagaaaccactcttcgttcattttcattgtcaaaccattgctggaatgctattcttaagtaaatgttgcacaaggaggaagatcaatgactgctggacaaatagccggccttatcgccgcaactgcatttttgcttttggtaatcttcattggcttattcttaatgaaggtaagcagaactatttcagaagtgaaccgcacaattaagacaatgactagtaatgtggacgtcattgccaaacaaactgataatattatggcaacatccaacgatttactgaaggatgttgatgacaaattgaacattgtcacaccggtctttcaagccgccgctgatttgggtgagagtgtgtcaagtttaaataccgctactcaaaacctcactaaacgggtcaaagataccggtaaaaagggtgtttcagcagggctcgccggtaagtttggcaagagtgcctggaacatgtaccgcaatcgacacggttcaaaggatacaactaaataaacaatcgaagggatgattagaatgggtaaaaaattagcatttggcttattcgctggtgcattgggtgccggtctatatgcagcctaccaaaaattggacgaagcaaagaaggcccaactcaaacgagacgcccgtcaaaaggctgatgagttgcgggatcgggcagttgactacgcgttttacgccaacgatgccgttagcgacttaaaagatgtgattcatgatgaaatgcaaaataccaaagggactgtcaatgatgccaaaacgcaattcgctgacaaagcaaaatcgtttggtaccgaccaagcagctgatgatgacgatgctgacgacaatcaggatgatattgttgttgatgctaaagatgccttccaagataccggaattcccaaggctgctgatgatttggattcacaatccgaccaggatgacggcgataatgagattccaatcactgacgactccgataacaacgatcacaaataaaaaacaacctcaatgtgcaatttatccaaacagtcaaagtcaaacttcagctgttgagataaggcacaaatgaggttgtttttttgatgctgttaattattgttcaatgtagcgtaattccttggtggtttgcgtaaatggttcgcagccatcttcagtaatgtgaacacaatcttcaattctgacaccagcaacgtttggaatgtaaatgccaggctcaattgagaagcacatccccggttgaagttccatcttgttgccagccatgatagatgggaattcgtgctcactcatgcccatcccatgacccaaccgatgaatgaagtattccccgtagccggctttggtgatgacatcgcgagcaatcttatccagttcttcagcggttattcccggtttagcggcttcttgggcagccagctgtgcttccagacaaacttggtagatgtccattgacttttcatcgggtttaccgactgcgatagttctcgaagcatcactaatgtagccgtcccagacagttccgagatcaaataagaccagctggttattttggactttattttcactggttgccccatggggttctgcggcgtgggggccggcttggacaagggaagggaaactgagttccatgatcccgtttttcatcagtgcatattggagatcagcggcaatttggtcttctgttttaccaacctggacggcttcaaacccggtttgtaatgcaaaatcgtcccacttgccggcaatcttcaatttttcaatttcgtcagccgatttaattaaccgcatttgttcgatcagtggggtcaggttcgctgagaaatccgcgttgggaagaacttgttggagagcttccaatcgttctacctggagctgggatttttcaattgcaaaatgactgtcgtcagtatttctggcatgaatttgatcggcaatcatcacccaagggtcttcgtggtcgaggtagccatagactggggatgaaaagccggtgtctttaatggcttctgattccagtgccgggccaaagataaatggttcctgatctttaaaaatggccatcagtaagactctttcaaccggatcactataaaatccggtgaggtattggattgttttagggtcggtaatcagtgcgatgtcttggccgttatcagccagccaccgttgaatttgttctatcttgttcataggatcactccttcgttattttatccacagtatatcatacaaaattcttttcaattatcgccgtaaagttccgttttcacttgaattttcagcaatcttagtttatgatttgactgaaaacgttttcaatttgctgaaaacctttttatttggtatattagatgatgttttgaaaatcgatgaaaacatattctaacgagaaagaaagggctatctttatggataaacaaacaattacaatttatgacgttgccagagaagcaagcgtgtcgatggcaaccgtttctcgagtagtcaatggaaatgccaatgtaaagccggcaacccggaaaaaagtgctcgacgtaatcgaaaaattggattacaggcccaacgccgttgccagaggtttagcaagtaagaaaaccacgactgtcggcgtcattgtcccagatgtgactaatatgtactttgcctcattggcccgtgggattgatgatgttgcgaccatgtataaatacaatattatcctgaccaattcagattccaacaatgaaaaagaagttaaggtgttaaataccttgctctccaaacaagttgacggcattattttcatgggtaacgaaattaacgataagctccgtgaagaattcaagcgaaccaagacgccaatcgtgtttgccggatcagtagatgaagaagatctctacgcgagagtcaacatcgactacgttgccgctgtccaagaagaggttaagaacctgattgatcgtggtaatcggcgggttgctttcgtttgtggccccttggagcaggcgattaacggcaaattccgtctgaaaggctacaaacaggccctaaagagcgctggaatcccttacgacgagaagctggtctttgaaactgatgatacatacaagaccggaaccttgcttcaaccagcattaatggcagttaacgccaccgctgcgatggttaccgacgacgagttggctgccgggattatgaacggtatgtcagatgccgatgttaaagttcctgatgactttgaaattatcaccagtaacgataccaagttaaccgaaatggttcgaccaaaaatgtcttcaattacccagccattgtacgacattggtgccgttgccatgcgtctgttgactaaattgatgcacaacgaaccggttgacgaaaaaaatgtgttgctcccatacggtttgatgaagcgtgaatctaccaaataatcaggtatcaaatcaaaggagtggaccgtggcgattcgctctttttgttctggaaactggtttgaaaagccgccacatatttggccgcgctttcttgaaagaggggggcgtatctggtagaatattgacgtatgtttgtaaccagctaataaattttagaaaagaggagttattatgtcaggacattcaaaatggcataacattcaggggcgtaaaaacgctcaggatgctaaacgtggaaaaattttccaaaaaatatcacgtgacttgtatcaagccgctaaaaaaggtgatcctgatccagaaaacaatcctcagttgcgtctagtgatggaaaaagcacgggctgccaatatgccaaaggataacgttcaacgtgcgatcgataaggcttccggtattggtggagctaagttcgaagaaattacttacgagggttatggtcccggtggtacagccatcatggtttctgctttgactgataacaagaaccgaactgctgccgcaattcgttctgcattcactcatcatggcggaacccttggaacaagtggatcagtttcatacatgtttgatcgaaagggttatattgtgattctgcgtgatggtcttgacaccgacgaagacacaatgttgatggacgcgcttgatgccggtgccgatgatatgaagaccagtgatgatgaattcgaaatcttcactgatcccaaatcaatggacgacgtccgcgacgctttgcaggaaaaaggctacgacttggatactgccgaagttcgtcttttccctgaaaacacgacagaagttccagaggacaagatttctcaatacactggtttaattgacgaactcgcagaaaacgacgacgtccaagacgtttacgaagccgctactttaccagaagaataatttaatatgatttcaatgtctcaatggccgatcatttgatcggccatttttttgtgctttgataaataaaattcaacttttcattcgtatgtattacatgtgaggtgaatgaaatggaaattagtcagcaagttaatggtcttttgaatgaagccattaaaacacaagccagtgatctttattttttgcctgaaggagacgaatacttggtcaaaattcgtaatgcaaacgaagtcgttgtttgggataaaatcggctatctacaggcgagacggatgatgaactattgcaagtacatcgcagatatggcattaagtgaacaacggcggccacaaattgggtcgatggattggcattttggtgataaccaatattttttacgattatcctcggtcggcaatttcacggggttggagtcactggtcatccggattatctatcagcttgatgatgtgcacgcggcattttttgatgaaaaacaagttcaactaatttccgaaatgagtcgaaaacgcggactcattgtcttttccgggccaaccggctctgggaaaacaaccaccatttataatttggtgaaccagatggtttccgaccaatttgtgatgacgatcgaagacccgattgaaattagggaaccacgttttttacaacttcaggttaaccacgatgcagggatggactacaccgacttgattaaggtgggcctgcgtcatcggcctgacgtctttatcgtcggcgaaatccgtgatgcaatgacagccgaagcagcaattaaagcggctctgagtggccatttggtctacaccaccgttcacgctcaggatccggttggagtcattgatcggctcaaacagctcggaatcagcgacgaatttattgcccaagcattaaccggcgtcgcttatcagcggctgattccaaccaccgacggcaaacagcgggcaatgttgatgggacatgattattcagagttggtcaatatgaatacatacgattggggtgaatggcaggatggactcaaaacagctgttaaagcaaaactggttacgccggagactgcacaacgattcgagttcggttaagaaatggccggtggttttccaagctaatttttttgactctttggcgaatcttttgtcaattggattctcactgactcaagcgttgaaatttatcgccgacactgacaaacaattgtcccgaggcgttaatgtggtgattggatcgttaaagtccggccgggaattttcggaaagtgttcgacccctgattgaaactcaagcttatcaccagctgttaatcgcggagaagcacggtcaactcagtgacattttaaacgaactggccaactttgatcgattgcggctcaaacaactcaaaaagatcaaagcgatgttggtgtacccattatttttgtgcctgatcttaggaacgttgatcttgatgattcgagtctacgttttgccacagattcaggatttaatgcccacagccaatcatcagcaaccggttacgtactggcagcagctgattcgactttcgccaatcccaattttgatcggcatcattggcagcacagttcactggagtcgacaggatgccataacccaggcccaaatgattgtcaaaattcccgtcgtcggcaaattgtttcgaaaatatatcgcttattatctggccagcaatttggccactcttctgaaaaacggtttgagtgttaaagaaatttatgccacgttatccgagttcaaggagggatcactgattcatctcttaggtgaaaggcttcatgccactttactttcgggagggtccttaagaaaattggtagaccggcacaattttattcccaatgagattatcaaatttatgagctccggcaacacgattccggaaatggccaattcgatgacggcctattcacggttgatgtttgacgaaatgatcctgaccaccgataaactgatcgggtttattcagccggctatgtttgtggtgatcggtgtgacgattgtttcgacatattttcaactgctaattccaatttataactcagtgaaaggaatgtattgaaatgaaaaagcgcgttaagaaaatgagagaaggctttacgttaattgaaatgaccatcgtcttgtttattatttcattattaattttaatcattattccaaatctatccaatcaaagaaaacacgcccagtctgttcattcatcggcaatgaccgaagttgttcaggcacaaattgacgcctatttcagccagcacccaaccgccaaatcagttagttttccagacctgacaaaaggtggctatctcaccgccaagcaggttaaacaagccaaggatgaaggcctgaagattactcataatgaagtgcaaaaatagggagggctttaccgttattgagctggtggtatatttaggcgtggtgttaggtgtcttgatgattaatttgatgctgatcaaggtcgtccagtctggaaatccaagtgaggcgttgttttggcggtcatttcagagtgcctggacccgcatgacattaaacgcaaaggccgagaacatttcttatcgaatctccattcgggataaagatgttattttctttccgatgaaggtgaagaaaactcactatgacgaggtaaatgaggagcgaatttcggttccgccttccattcacgtgagatcacaacgaagcatgattgcccatgacgatgggtttgcatcaccaactaagattatttggcttgattcggatggtaacgtcaaatacaatcaaaaaattcaaatgggatggagtggctatcatgtggaaaggaacaaataagcgggcttttacggtgatcgattcattaatcgggctgaccatcatctgcaccttcagtttgttctacatccaaaccacccatcaaatgaatgagacaattaccaacgcagaaaaagtgatgacaattgagaggcaaaaatatgaagcagaaattgtccgtgagtaaggttgatactcggccgggctacttattaattgagggcctgatcaccttggtgattggtgtattcgccatttggacgatcatgacgatgatcgtatatgcgggaaacgaaaaaaagcaaaacgtgatcaattttcattcttatctcagtataatcgaatctgaccgttatcggtttgaaatcaagcagtgtcaaccctctaagtgcgtgatgtacagtccggtcacgaaaaaaacttatcgaattgaacggtatgaaaacatggttcgattggccggtgcctacaagggtcacgtaccgtcgttgacaaatgttcaatgggtacgctggacaaagagcagggggtgtctaagaactgatgttactttcgataatggccaaaagtgttcagcttattcaaaattaccgttcaaggattgataaatataagcgtggatccctaacggtggtggctgtgatttttgtcggtattttgatgtcatgcttgatgtttcaactggctgcttataagcaggagttgggatcaattaatcgtatcaccgagcatgaacggcaaatgagacggcaattccttgaaaagccactcaaaaaagatgttcacccaaaacgcacaagtggtcacgaatagtggcctttttgtggttgtgaaataacaatctaacttgaattattgacagcttatctggtagtatttaatagtgttcaactattgaataaaggggttgagagttctggctcaagggaaaattgagcagctttttgatatcttgaatcgttcgacagaattgattcaaaaagccaaggatcaatcgtatcttgattctttcatcgaaacactgggatttatccagagtgacgatgaagaagatgacgaactgactgaagccgataccaaaaagctgactaatatttatgcagactttaatccggacgatttcactgccgaaactttccggaaagcaattcaaatggctgtgctcaaggcgattcgagttgacacgattcaggctaactaccaactgacgcctgataccattgccaacgtcattggctatattattgctggaattttccatgaccgcaaagaattaagtattcttgatccggcgatgggaactgccaatctactaacagcaatttatcatcagcttcaaactagtattggcgttacaccgaccatttctggaattgaaaatgacgatgcaatgtttgaattggctgcagactcagtcgagctgcaaaagattcacgctgagcttttccacgaggatacgatccaaaatgttttagctcccgtggtcgatgtagttgttagtgatttgccgattggctactatccaatcgatgctaatgccaagggatttgctacccattcagacacgggtcattcatacgtgcaccatttgctgattgaatttggcatgaagcatgttttgccgggtgggtttggtttcttcctggtgccaagtcagcttttccaaaccagcgaagccaagcagcttcttaaatggatgcaagggaaggtttacctgcagggattacttaatttaccaaaagaactctttgcaaacgccgcggctcaaaaggcaattttaattcttcaaaatgccggcgacggtgccaaacaggtggatccggtaatgttgggggaatttccatcatttaaggaccaacaagcctttaccaagttcttgaccgagattgatgattgggaacaaactgatttattataaaattgtttatcaagctttttaaaaaatacagaggagcattatttattatgggaaaatcaattgcaattaacgctggtagttcaaccttaaagtacaagttgttccaaatgcctgaggaaaccgttctttcaagcggtgctattgaccgaattggattgggcgcatcagatatctcaatcaagtacggtgacggcaagaagttcaaagatacccaagatattgataatcatgaacaggctattcaactcgtccttgataaactgttgagtttggacatcatcaaagactatagtgaaattaccggtgttggccatcgaattgttgctggtggggaactcttcccggattcagttgtgattgacgacgaggtcatcaaaaagatcgagtcattaacagagtttgcaccacttcatgagccggctgcgttgcttggcatcaaagcctttaagaagattctcccagatatcattagtgttgccgtctttgatacttcattccatacaacactcccagaagtcaactacatgtatagcttgccttacgagtattatcaaaagtatcaagttcgtaagtatggtgcccacggaaccagctatcgttatgtctctgccagagcagctgcccttttaggtaagcctctgaaagacctgaaattaatcgtccttcacttaggtgccggagcttcaatcgacgcaatcaaagacggcaagtcatttgatacctcaatgggcttctcacctgttgccggcattacgatggcaactcgttcgggggacgttgatccttctgcattacaatatgtgatgcaaaaagccggtattaaaaacatggatgatatggttgatattttgaaccacaaatcaggcctcgtcggtttatcaggtgtttccgcagatatgcgtgaaattgaaggggttatgaagactaatcaccgggcaatgctcgctcgcgaaatctttaagaatcgtatcatccgctacattggcagttacattgctgaaatgggtgggattgatgccttggtcttcactgccggaattggtgaaaacgacattatgattcgccaggaagttaccgataagttgggctacttcggtatcaaagttgatcctgaaaaaaataacattcgtggcgaagaacgtgacctgtcagccgctggttcaacagttaagacattgttgatcccaaccgatgaagagttaatgattgttcgcgatatcgaaagattacgcaaaacacagaagtaatttttggacggtcgtcattaatacccaatcattacgggcgaagatcgttgctttttcaagcatagaatccgttgagccccatttgaattcggacgtcgcgggttacaaacgaggctgagacaaaagggttttgcacttttgtcccagccttattgtttaataaaccaaattgtcattttttagaaacggaggcacattgtggaaaatcaagaagacgacaaccaactatcccggggcctcaagaatcgacatgttcaattgattgcccttggtggaacgattggaaccgggctgtttcttggtgccggtcagtccatccatttagcaggaccatcaatcatcctggcctatgggattgccggcctggcttgtttcctattaatgcgggccctgggggaactgttggtatctgatgttgaaagcaattcgtttgttttcttcatcaaaaaatatttaggcgaaaaaatgggcttcgtgatcggctggacctattggatgtgttggatcgccattgcgatggccgaagtgacagcctctggattatacgtccagttttggtttccggacattccaatttggttgacaggtctggtcctcttattgatcctatttatcatcaatatcgtcgctgtgtcggcattcggtgaaaccgagttttggctggcaattgtaaaaatcgtcgcaattgttgcactgattgtcattggaatcgtcctggtggcaatccattttaaaacaccatacggacacgcatcattgatgaatgtggtggatggcggtttctttgccaacggtgcgaaaggatttgttttgtcctttcaaatggtgctctttagtttcgccggaatcgaaatgattgggatgacggcttctgaaactcaggatcctttggtgacaattccaaagagtatcaacgaagtgccaacccgggttctcttgttttatattgggtcgctgttggcactcatgagcattttcccatggcagcacgtttcgccaacttccagtccttttgtccaggtttttgccggtgtaggcatccagtccgcagctttgattattaactttgtcgtcttaactgcggcaatttcggcttgtaacagttcgttatttaccactggtcgaatgctgttttcattgacttataatggtaaatcaaaattcagtcgaaaagtcggtcgtctttctgcccgtcaaattccgtttaacgcaattcttttttcgaccttggtgatcgcggttatcgtgctcttgagtattatgatgcccggtgatgtgttctctttcatttccagtgttgccacaacttgtttcctatttgtctggggaatgattgtgttggctcatatcaagtatcgaaagcaggttaaaaaaaccggcagtcagaaatcgctcaaatttaagatgccgctttttccaatcagcgattacttcgtactgattttcatggcttttgtggcagttgttttgaccatgaagacggatacgttgattgctttaatcggctcggtggtttggctaattggactgtttattttcaaaagtctgacagataaggttaaagaagttgaaaaatgatgattggccaaggcatcggcgccttggcttttttcattggtgttatcagctttgtttgaatactttttcattactaaacggctgctgggtggtatcattaatggtataacttatgtacgaaagaggacctgttcatgcaattttttactgctgatacgcatttctttcatgaacgtttacttggcgttagcgagttcgcaccacgaccatttctgactgtcgaggatatgaatgaaaccatcattaacaattggaatcgtcgggtgggcaaaaacgatgtggtttatcatcttggtgacattgcgattttgcatacccgacctgagaaagtggcactggaaaaaatttttgaagtgctggatcaattgaatggccgcttggttttgatcaagggaaatcacgattcccgtgctttattcaaatatctgcagcagcataatcatcccgtgggcaatcatcaaaagtttgaatttcacgatgttggtgttctcatcaagatgaatcatcgtcagtattatatgactcactatccgatgatgatgggcatcgttaaacaaattattaatttacatggacacattcatcattatgcagttccgattaaagaaaatatcaatgtcggtgtggatacgcccgagactgattatttgaaaaagaagccaccgtttggaacgccattttcccaagctgaaattgaagaaatggtcgccggaaaagctgaagactttgccaagcggcactaatttagaaaagattggatggtttgatgactgagaagctaacaattttacacacaaacgatctgcactcccatttcgaaaattggccacgcattcgtcaatttatcaccacgcgccgagcagaacttcagcgagccgattcttccgttatcactgtcgacttgggggatgcggttgatcgcgtccacccactcactgaagtaaccaacggcaaggccaatgtggagttgctcaaccaaattcattatgatgccgtcacaattggcaataacgagggcttgaccaatagtcatgaacaattggacgagttgtacaatgatgccaatttcgacgtcattttgggaaaccttttggatcagcagaccaaatcaattccaaaatgggctcatcccagcaaaattattaccaccccgcaacatacacgcgtgcttctgattgggctgacagcgccttatttactgacatatccgatcttggggtgggagcctctcaaaccggaaacggttctgcctaaaattctcgccgataacgccggcaaatatgatatctgtgtgttactatcacatttggggctgccaaccgaccgtctattggcacgtcagtttcctcaattggacgtgatcatcggctcgcatacgcatcacttactcgttcacggtgaaaaagtgaatcattcactactggcagctgccgaaaaatggggtcattatattggtgagattacactgaccatcgatgattcccatcggattgtgtccagtcaagccaaagtgattaaaaccgctgatttgcccagcaagcctgaagatgatgcagaaattcaggaatatcaacaacatggtgaaaaactgctggcacgcaacaaacttgccagaatcaaagccccaatgacaactaatctcattggccattcgcgcttggtaaacgaaggtttgcatgcgataatggaaaaagccgatactcgcgctgccattttaagttcgggcctatttttaaccgacctgcctcaagggattgttgatcgaaatcaattgcatcagatgttgccccacgcgatgcatgtcatgcgggtcactttggacggttataatctctggcgcctcatcaaagaaatggaaaagaacaagaactttttgaccaaattcccacaaaaagggatgggttttcgtggcaagtattttggtcagctacattatggcggattgcggtatgatcaagatgccggccagctctttttccatgaagagttggtttcaccggcgaaaacataccagattgccatgccggaccactatttgtttattccgttcttcccgacattggagattatcggccacaacgaaattttatacgatgaaaatttaagggatgtgtttggggattatctcgccaaacattatccacttaatcagtgaaaggagggttactttggacagaaaaaccttagatgaactcgttgcaaaacaagacgagaatcgaaagccattggcacgaatcaaccgagtcagtgaaacagaattcttaatcaatgatcataagtatgaattggataccaatcacacggatggctttgattttaacgaatttgttcgtcggtacaatccggcttttagtcagtatgattacattgttggcgactggggatacggcaaattacgtttacgaggattttttaatgatgaccgaactgaaacttccggcccgtttatttccgcactcaatgactggattttggaagatgtcaacttcggtgccgcttattttgtcgttcataatcttgaggcccgaccggtgatcagaaaatcccggaataatcatggtaaccatcgatcaaaccggtctcataattcccgcaaccggagtaatcatcgcaatcatcggaaccacgcctttgaagaaaagaaggttaccgcccataagccaattgaaaagcgccataatatggtcgtgaagactgaagaaaaatcaaaaaagcaccactttattattcgtgagagtaaaaattaattagaaggattgacttgatgacaaactataagggctattttattgatcttgatgggactgtgtatgccggtaaaaaacgcattccggctgccaaacgatttattgagcgcctgcagaaggccaatattccatttttatttgtgacgaataattccactcagctccccagagacgtggtgaagaacctggctgataaccatgatattcacgtcaaaccggaaaatgtctatacatcagggatggcgacggttgattacatgaatgagcatcgtagtggggatgcttcatccgtttacatcgttggtgaaatgggcttgaaacaagttatcttagccaacgattatcgtttggaagccgatcatcctgattacgtggtcgtggggcttgattcagacctaacctatgaaaagctttcagaggccgtcttagctattcgaagcggttcgacgttcattggtaccaaccccgatacaaacattcccaaagagcgcggaatgatgcctggagccggttctgttgtgaagtttgtcgagtatgccacccaagtcgaaccgatcatgattggcaagcccaaagccagaattattgaaagtgccattaaaaaaattggccttgaacagtctgacgtcgtgatggtcggggataattacaacactgatattaaggctgggattaatgccggagtcgatacgctcctggtttacaccgggctttcgacaaagcaacaggttgccaaagaatcggttcagccgactcaccagattgactcacttgatgattggcggttataaatgtgaaaatgcttggaaaacaaattggttatggcactttaatcatattggggtgccttgccctcgccatctttttgactgtcaatagtgtttggctgtttgacctcaatattaatccgctcaaattagctgcggccactggtcgcactgctagccagatgcatcatgattatgtcaggattattgcctacttacaggtgccgtggattccttctttaaagctggattacttcttcagttctgcaaagggacttcagcactttcgggacgttaaaggtttgatcctgttcaacaattttgttgggctgattttagtgccgactggtgcctacctactgcatcggctcaacaaaaaatcactaacttggctgttgatgacgccaattaaggtcgtcaccacagtttcgttagtgattgtcgcgttgatgtttgttaattttgaccaggtatttgtggcatttcatgaagtattattcagaaaccaggactggatttttgacccgaacaccgatccggtgattaacatgctgccagatacgttcttcttggaatgctttctactgttctttgtcctattttttggtgggttggcagtcatctactggcttggccgcagatcactgaagcagcactaattattctggtgctttcatcaaaatccaaagcagtaggtatgcgatgattcccgggaagaatggggtaaatgccagaatgacaaatacgacccgtgccaaagtgggattccattgaaagtgctcagccaagccaccaatgacgccggcaagcaccttgttcgttgcggaacgatggatattaattttcataatcatcatctccatattttaatttaagtataagcttactataaccaattcgcatttgcattgcaattatgctatattattatgttgtataaaggaaataactaggagaattttaatgttaactattaatgtcaatggaaatctaggaaaccaacaagttgttctttctgataattcggttgggacgttgactggtgccagagttttcggctcagccttgagtggtaatcaagttgttcaatggacctttatctcaaccggccatcagcatgaaggcttcgtctatgcgggtccattactggaaggcttagtgattcagtcgatgaacggcaatgacacctaccaaattcattttacgaataaataatcattaacaatcagcggcatacataatgagactggatattgcacctaaaatattcggtctcattctttcttaaaggagattattatgacaattggaatcgacaaaatgggcttctttacttctgattactatttggatatggcagatttggcaaatgcccgcggtgaagatcctaataaatatttgattgggattggacagaaggaccaggcggtaatcccgccaacacaagacgtggtcacaatggctgccaatgctgccgccaagattttaagcgatgacgataaacaagcaattgatatggtgatctttggaactgaaaccggtgttgacaactccaagtcagcggccatctatgttcagtcgttgcttggaatatccaactccgccagatcgtttgaaattaagcaagcctgttatggtggtacggccggcgttcagatggctttcgatcatattgcaatgcatcctgaaagtaaagtgttggtcttggcagcagacattgcccgatatgggattggaacagctggtgaggtcacccaaggcggcggggcagttgccatgctgatgagtcaggatccacaaattttagctttggacaatcaaagtgcatttcactcagaaaatattatggatttttggcgaccgttttaccgtcgggatgcaattgtcgacgggcattactcaacggatatttatatcgatttcttcaaccaaacatttaaagattactctgcgaaatatcaacggacgctgagtgatttttccgcggtggcttttcatctgccattcaccaagatgggcctaaaggcgcttcggacggttatcgatgatggtgctcactcacaaaaactcctcaaagaatttgatcattccaaaaagtataatgccctcgtcggtaatctctataccgggtcactctacctaagcttgttatcactactggccaactccaaaacgcttcagccaggtgatcgaattggtttgtttagttatggatcgggagctcaaggggaattttacagtggtacaattgcccctgaaatccaaccgcagagccttgccggccaggttgaacaagtgattgccaaccgaacgaggctgtctgttcctgagtatgaagcgatgtatgcaaatggattgtcaaacgccggtggagatgttacatttgatgctgctgatgatgacagtcgattcgtgttgcttggcagacaggccgaccagctggtttatcgagatcaacaggcataatattgatggtagaagggctcgttgggcattgccgaaaagtcctggaccagaactcagggtaaaagaaaaggactgttagcagaacagtccttagctagaaataattatgaaatatcgctgcggtacaaactgaccacttttcccaaaatgctgaccttggtcaaaataatgggcgccatggtatcgttttctggctgcagtcggtagtgatcgctttctttgaagaaccgtttgcaggttgcttcattttcatcggtcatcgcaatgacaatgtcaccgttatcggcgctttcctgtttgcggacaaccacatagtccccatcgagaatgccggcgttaatcatactttcgccccgaatttgcagcataaataatggttgatcactgtgtgccagagcaggcgggagcgggaagtagtcggtggcctcctgaacagctaagatcggttcaccggcagtcacagttcctaaaaccggaatctgtttttgttgtggctgcatacccaggacatccaagccactactggtgacttccagcgcgcggggtttggccgggtctttaacgatatagcctttccgctcaagtcgagcaatatggccatgtaccgtggaggttgatgatagatgaacggcttcaccaatttctctgaccgttggcggatagccctgctcattaacccgttcccagatgaagtgaaggatctggtattgtttactttggggatcattggtcgtttttgacattttagacacctcataagtctttgtttaatacctaaatcatatcataaccgcggtcacatttcaaaacacacgttcgcgtatctatcaataattgtgttattatagtcgatatggaggaattttaatgaacgaacaagagaaaaaagaattgcaatcaaaaatcggtgacgatgttttcaaagaactcatcccaagaattaatgaactggcccacaaagcaaaaaatgagggcttatctgaagttgaaaagttggaacaggctgatttgcgtaaaaaatacgttgctcacttccgtgaaaacttcaaaaaacagattgaaatgatgaaagtttatgataagaatggcaaggaagtgacgcccggaaaagtcagggaagtccaacgtcacaaaggtcttcgggacgattagggggcagttttcccctaagaatcgggattttgttgattagccctttaattctatggcataattgtgtagaattacttagtgatatgataaaggaggccttgtcttggcaacttggatttggatattaatcgttgtgttagccttgatcttgggcttggttggtggcttttacggtgcacggaagtatatggaaaagtacctcaaagaaaacccaccattcagcgaagatcaattgcgccaactgatgatacaaatgggtcaaaaaccttcccaaaagaaattaaatcaaatgatgcattcgatgcaaaaccaaactggtaaaaattagaatgtttcaatgacaaaaagtccccaccaacttggtgagggctttttgtcatttcacttactcttctttttttgatacatcaacgtatttaaaattcggattaacagcataatccaaggcgtcgaacgcgctttgcatctccgtttcaatttgtttttgaaaatcgtccgtcaatttttgtttacggtcaattgtaatgggttctccaaaggcaatcgtgacccgttttcgagtaaaaagctgtttgaatgtcagtggtccttgataaacggccgggaccagcggaacacctgacagctgggcaataaaggcagcaccgctttttaattggctggaatgccgggtgcctgatgggaataagatcaaagacaaatctgattttctgagaattcggactggtttcttgatggcagaaggaccggggttatcacggtcaaccgaaaaagcattggcatgaaccaaaatccaacgcaaaattggatttttgaatagttcttttttcgccatgaaactaaactttttcggactgccggcaagtgcaaagtaaattggatcaaaccaggtgcgatgggggccaaccaaaatatagttgccttttggcagtcgctccttgtgctcataacgggcattgccattgataataaacaccaggattcggacaaggactctcatgaatgaataaaacaattcatttccttctttcatatctgatagaattatattaacttaaaatagaagcgtttggcaaactaatttgtgaaggaacataacgatatgcaagtaaacttacatgaagacgaacgaattgaccaattatacagcaaaggcatccaaattattcaaagcaaagacgttttttcgttttcattggacgcggttttgctggccgactttgttcggaccacgcaacacagaaccaaacaaattgtcgacatgtgcgctggcaatggggcagtcggactgtttttaagtgaaaaaacggctgctcacatcaccatgatcgagattcagacaaggctggcagatatggcacagcggagtgttgaactcaatgacttggctcagcagatatcagtggtcaacgacgacctcaaaaatgccgaccaatatattccaaaagattctgttgacgttgttgcctgcaatccgccgtatttcgtcaactacaagaccagcgaaaagaatccgaatcgatacttggccatcgcgcggcatgaaatcaccactaatttaaatgaaattgtcagctcagcggccggactgttgaaaatgaacgccaaacttttcatggtgtaccggcccgatcggctgacggatttgatcgtggcgttacgaagtcaccgactggagccaaaacggcttcaatttgtcagaccccgaatcaaagaggacgccaacatggtcttggttgaggcgattaaagacggcaagtcaaacggtctcaaagtcaaccgcgatattattacttatgacggcgatgactatactgatgaagtaaagaagatgctttatggaacaaacagataagtattatatgtacgtgcttttatgtgccgatgatactttgtacaccggtttttccacgaatgttgaaagaagatttcaacagcatgtgaaaggcttgggtgccaagtacacccgctctcaccgaccaatcaaaattttgttcaagcaacaatttgacagcaaacacgctgctttgagcgctgaatacgcctttaaacaattgagtcgggctcaaaaaattgcccatttagctcaagcggggataaaattagagtgaattattgaacaaactacgaaaagtagtgaaaattattatcaaaaagtgttatactttaagtattctgttaggaggtaatattcgtgaaaattattgcatatggcattcgtgacgatgagaaaccttatttagacaagtggagtgaagaaaatcccgacgttgaagttgcttcaaccggtgaattacttgacgactcaactgttgaccaagcaaaaggtgctgatggtgtggttacataccaacaaaagccttacactgcatctgtattagataagctgggcagctttggtatcaagtacctttcacttcgtaacgtaggtgttgataatattgatgccgacgctgccaagcgtaacggtattcaagttaccaatgttcctgcatattctccagaagcaattgccgaatttactgtaactcagttaatgagattacttcgtcggaccaacacattcgaccgtaaacaagcaaatggtgaccttcgttgggcaccagatattgctgacgaattgaaccaaatgactgttggtgtctttgcaactggtcggattggccgagctgcaatgcgcatttacaagggctttggtgccaaagtaattgcttatgatatttatcataatccagagcttgaaaaagaaggggtttatgttgatactcctgaagaactttatgctcaatcagatgtcctttcattgcatgcgcctgcaactaaggaaaacgaacatatgattaacgataagacaatcgctcaaatgaaagacggtgtcttcatccttaacccagctcgtggtgcccttgttgacactgatgctttaattcgcggccttgattcaggtaaaattggcggtgctgcccttgatacttatgaaaacgaagttggtattttcaatactgactttggcagctttgacaagatccctgacgaacgactcaagaacttgatgaaacgtgaaaatgttttggtaagtccacatattgccttctacacaaaacgggccgctcgtaacatggtctacttcgccatggacgcaaacaaatcattaattaatactggtaaatcagacaagttggttgaactttaatttgaccggcttgatatacaaaaaaggtttcagtcagacaatctctgattgaaacctttttattttaaataggctagtccatttgagcagccaaatccatgagtaagtcttttaattcttccggtgttttgactgtctggtcgggaatgatttgaggatctgcgattggactttgatggctgttataccacacggtttcccagccggccttttttgcgggcacgatgtcttcaaaataggagctgccgatgtacatcatctcattgccccgtaaattgaattttcggttcatcaaggtaaaaataagcgggtccggttttttagccttcgcatcttctgaggtaatgatttgttcgcggctaaaccaatgatgaagtttgagcttcatgattttggcgagttgaacatcgttgcttccgttggtgatgatgcctaacttgaatttggtagtcagggtattaaagacagtggtcaatccatcaaatagatgaatggagctgctggccgtttcaaaggcctccgaaaaggcttttgcggactcttgtgtcagtccgggcagatcatactttttaaatgtatggtgtaatgaatgatagttgatttcttcgtcagataatttcaaatcggagtctgagttggattctgcaattgccaactgttcttgctcgttatagttggcaaagatctgattcatctgttcttctggtaaatttagattgaatgtttcttcgaaagcctgtacaaatgcgggctttgtatcatacaaagtatcgtcgatatcgaaaacgatggctttaatcatgtataaattcctcctcgccacgaaatatcattctaacatgattcatcgaaatttaacaattttgacaaaaaaataatctgttccgggtatttgtgcttgcgcttccgcggcttttcttatatacttttaaaggtgttttaaatacacacctgacgtaatgggttgagagttgccagggatggttcttaattcaaatgatcgttggggaggaaaaaaacaatatggaggctacatcatggctgttatttctatgaaacaattactggaagccggagtacatttcggtcaccaaactcgtcgttggaatccaaagatgaaggactatatctttactgaacgtaatggtatttacatcattgacttacagaagactgttaagttaatcgatgttgcttacaacttcatgaaggacgaagctgccaagggcgccgttgtcttgtttgttggtactaagaagcaggctcaggattcaattgctgaagaagcaacccgtgccggtcaatactacgtcaacaatcgttggcttggtggtactttaaccaattgggaaaccattcaatcacgtgttaagcgtttgaaggacttgaagaagatgtcaactgacggtacttttgacattcttcctaagaaggaagtttctcttttaatcaagcaggaacagaaattggaacgattcttgggcggtattgaagacatgcctaagatcccagacgttatgtttatcgttgatcctcgtaaagagcaaattgctgttcacgaagcaatgaaattgaacattccgatcgttgcaatggttgataccaacactgacccagatcaaatcgacgttgttatcccatcaaacgatgatgctattcgtgccgttcgtttgatcacttcaaagatggctgacgcaatcattgaaggtcgccaaggcgaagatgacgttaacgaaaagacctttgaaggtaaagatggcgccaaagcagacaaaaaagaagattcaattgaagacattgcagacgccgtagaaggcagcaacgattctaacaaataaatattagcactcgggctgactctaccgctttggaccaatttggccttggtgtggagtcagtttttagtcacaattaaagggaggccactaagatggcaaaaatttcagcatctcaagtaatggatttacgtaagaagaccggtgtcggtatgatggacgctaagaaggccttggttgcaactgaaggcgatttcgacaaagcaattgaagttttgcgcgaaaaaggagttgccaaagctgagaagaagagtgatcgcgttgccgccaatggtttggcaaccatcgcagttaagggtaataccgctgcaatcgttgaaatcaactccgaaaccgactttgttgcgtcaagtgatccattcaaagaattagttaaacgtgttagtgacgcaatcgttaccaataagcctgcagacgttgatgcagcgatggcattgcagaccgacaaagggactgttaaagacgatttaattgaaacgactcaggtgactggtgaaaaggttactttacgtcgttttgaagttgtcgaaaaaaatgatgacgaagtctttggttcatacctgcacaatggtggactcattggtgctttggttcaattaaaaggcgctgatgaagaaactgccaaggatgttgccatgcacgttgctgcaactaatccggaatatttgaatcaagcagaagttcctgctgaccgtttagctcatgagaaggaagttttgactcaagaagctttaaatgaaggcaagcctgaaaagatcgttgaaaaaatggttgaaggccgtttacacaaattcttggccgaaatttgcctggaagatcaagacttcgtcaaagacccagacgtcacggtttccaaatacgttgcttccaagggcggttcaattgttaaattcgttcgttacgaagtcggtgaaggcatcgaaaagaagacccaaagcttcgaagatgaagttcgcgatcaattgaagtaagctgacagaatttagtttacaaatcgtttttccaaagataacgacgtaaccaaataataggggttaggacagagcattccgcttttcctaactctttttatttaccatcatgaatgactcaaccctgttttctgaaacatctctgtgaactggctgagaatatttgataagaattcttgaatatccctgttttcttgttgattgcaacgttaatatgctaaaattggtagtaacgattaactatgggaggcacttggatgtctgaagtaaaatacaaccgaattattttaaaattaagtggagaagcattggccggagaccgcggctttggtattaatccacctgttatcaaaaacgtcgcccaagaaatcaaagatatctttaacctgggtgtccagatcggaatcgttgttggcggcggcaatatgtggcgtggtgaagccggtgccgagatgggcatggaacgtgctcaagcagactatattggcatgcttggaacaacgatgaacgggctggcccttcaagacaaccttgaacatttgggagttccgaccagggttcaaacttcaattgaaatgcggcaaattgccgagccttatattcgtcggaaggctgttcgccatctggaaaagggccgggtcgtgatttttgctgccggcaccggtaatccgtatttttcaacggataccactgcagcgttgcgagctgccgaaattggtgctgacgccatcttgatggctaaaaacggtgtggatggcatttattcatccgatccccgaactcacaaagatgcagttaaatttgataccctttcatatatggatattttggaaaaaggccttaaagtgatggactctacggctagttctctgtcgatggataatcacattccattggtggtcttcaatttgaacaagcccggcaatatccgtaaggtcgtgactggtgataatatcggaacaactgtgaaggagaaataatttatggcagatgcacaatcagtattaactgaagcgaaagaaaaaatgaagaatacccgtgaggtgttggaacatgatatgggcagtatccgtgccggtcatgccaacgccagcttgttgagtggcgtcatggtggattactatggtgcgccaacgcccttaaaccaaatcgcttcgattaccattccagaagcacgggtgattttgattaccccttacgataaaagtgccttggaaggcatcgaaaaaggcatttatgaagcagacttgggcatcagtccggctaatgatggaacggcaattcgattggcggttcccgcattaactgaagaccggcgcaaggaaattgccaagcaagtcaaggcaaccggtgaaaaaagtaaggttgccatcagaaatgtccgtcgagaggccatggacacactcaagcgtagcaataagagtgaagatatcactgacgacgaactgcatcgctatgaagatcaagttcagaaattgactgatgatgcaattaaaggtgtcgacggaattgtcgccgacaaagaacaagaagtcatgaacggctagaaagaggtcaatacgatggcagataatcataataacaataataattcagataacgatgaaattgcggttgtacctggaaccgatgaatttggcaagatgctttttaaactgaatacgcctgttactgaggacaatttgggcgtcttggattataacggcggccacttgcagccggtccaagatggcttatatgcaatgcctgcatatgtaaacgacggctttaacttattcttcatcgtttcgcaactggttgaaaacgactgggtaattgccttttctacagcaactattgaaaacgaccatgaaatcacggacctttcagaaccctatacaaccggcaaaggcttaaacctgctgggccaaaagagtccggaagatgccaataagctgttgaagtatttcaacacattggctgaggcaaaccgcggtgaatggcgaatggttgaacgtccagacggcgaatccgactaatacgaatagcattttatggctgggaaaaaactttggttttgttccagccatttggtgtttaacgatatgtcgcgaggatcccatgctgtttttgaatctgacagccaagccaacattcagtttttaaggagcgtaaaatgtttaacaacacacaagacaatcaacaagcaaccccgcaactcaaaacagacaacattccggcacacgttgccattattatggacggtaacggtcgatgggcacagaaacgccatttgccaagaattgccggtcataaacgcgggatggaaaccgttaaaacgattaccaaagtcgctagtgatcttggtgttaaggttctgacgttatacgcgttttcgaccgaaaattggaaacggccacacgacgaggtcagttatttaatgggcttgccggttaagttcttcaacgatttcgtgccggacttggttaaaaataatgttcaagttcgtgtgatgggtatcaaggatcaattgcccgttcaaacacaaaaggcagttaatgacgctattaaagacaccgctgactgcacagggatgatcctgaactttgccctgaattatggcagccgtctggatatcagaatggcagttcagcaaatcggccgtcaggtcgccagcggtcaactggatccagagcagatcacggatcaaaccatcgatgcaaatttaatgaccggatttctcggcaatttagccgatcccgatctgctgatccgcaccagcggagaagaacgcatatccaatttcttgctgtggcagattgcatacagtgaacttgtttttactgatgttttgtggcctgattttgatcgaacggtttttgaacaaatgatcatggaatatcagcagcgtgaccgtcggtttggcggaattaaaactagtaaatagaggagaaacaaattgagacaacgtgtgataacagccgtagtagctttattaatctttattccaatcatcgtaatgggtggaatctgggtggatattgccgctttggcacttgggattgtagccatctctgaaatattagtgatgaagaagaaattattgatttcacctgaatcaattattgcttatttgggagtctgttcactcattctgccagatgcatggacgagctttttacccggacacatcagtcaaaactttgtcttctttttgtttgttttgatgctgcttctccaaacggttctgagtcgaaacctgttctcgtttgacgatgccggggtaattgtcctgggcatgctgtatatcggtatgggatttcactacttcgttgccgcccggggagttggactgacagtattgctgtatgctttgtttatcgtttgggtaactgacagcggcgcgtacatttttggtagaatgtttggcaaacacaagttggcaccaagaattagccccaataaaacttgggagggttcgatcggcggttcacttgcagccaccattttatgtaccgcatttatcgcattttacccaattgccggacactccctcttgcaaatgttcatcttcacgattattctctctatagctggtcaatttggcgacctcattgaatctgcattgaagcgttattatggcgtcaaagactcggggaagattctgccaggacatggtggaatcttggaccgctttgatagcttactttttgttttaccaatgcttcatttgttagctgttatttagtttttaggaggaaagtgtcacttgataactacaattattgttttcattatcgtctttggtattcttgtgatctttcatgagtttggccattatattactgctaaacgctcgggcattcttgtccgggagttttctgtcgggatggggccaaaagtattttattatcggaaaaatagtacaacttttaccctaagattattgccgctgggtggttatgttcggatggccggtgaggccgatgacggtgaggacgaattaaagcccgggacgccggtgactcttcaattgaatgacagtggtgtggtaacatcaattaacaccagcaataagcattcacttttccagggcattcccttaaccatcacagatactaatcttgacgataatttgtatgtcaagggatatgaaaatggtgatgagtcccaagttaagtcgtatccggtggatcatgacgcaactatcatcgaaaaagacgggaccgaattacaaattgctcctcgagatgttcaatttcaatcggcatcgttgcctaatcgaatgctgacaaacgttgctggtgtgtttaataacttattacttgccatcttggtatatacaattttaggctttgttcaaggtggtgttgcatccaataccaataaagtcaatgtcatgcccaccgattctgtcgcccggactgccggtgtcaaatccggtgaccgaatcgttgaggtcgatggacacaagaccactgattggcaggatcttactgttcagatccgatcaaaagctgataagcaaatttctgtgaaggttcagcgggatggtcaggataaagtcttaaccatgaaacccaaagcccagacttccggcggtcaaaagacagggttcattggcattactcaaacaatggataccagttttaaagccaaaattctttcaggtttcaccaccacttggacagttgccaagcagctgtttggcgccctgtggagcatggttagcggccactttagtctcaacgatttgggtgggccggtggcaatttttgcgacaacttcccaagcagccaagatgggactttcaggagtcttgaacttcctcgcatttctctcactcaacctggcaattatcaacctcattccaattcctggtttggacggtggtaaactgattttaaacattttggaagctatcagaagaaagccggtttctcaaacaacggaaactgttatcacattgatcggcttcgcgttcttgatgctgttgatgattctggttacttggaatgatattgagagatactttttacattaaacaagttaattttgaaggagaaccttataaatgaaacaatcacagatgctgatcccaacgttaaaagaaacccccaaaggcgccgaagctttaagtcatcaaatgttagttcgtggtggctatatccgccagatttctgcaggtatgtacgcatatttgccattggcctatcgcgttttaaacaaaattgaaaccatcattcgccaggaaatggaaaaaacatcagctcatgaaatgctgatgcccgacattttgccggctgatctttggaaagagtcagggcgctatgatacatatggcccagaactattcaaatttaaaaatcgccatgaaaccgattttattttgggaccaactcacgaagagacgtttacggcgttaattcgcgattccattaaatcatacaaacagctgccactggttctttatcaaattcaaaacaagtatcgggatgaaaatcgtccgcggtatggattactgcgaagccgtgaatttattatgaaggatgcctactcatttgccactaacgatgaggatctggataaaacgtacaatgcaatggagcaggcttatcgtaatatttttgatcgaattggtttgaagtacaaagtgatcatcggcgatggcggtgcaatggggggatctgattccaaagaattctccgctatggctgctgtcggcgaagatacaattgtttattccgatgaaagtgactattttgccaacttggaaatggccaaatcaaaagtcgacgaccagccttcaactgaacctgaagaagaccttaagaaggttgaaacgcccaacgcgaaaaccattgccgaggtggctgctttcctaaaagtctcagataagcaaaccatcaaatcgatgctgtacattgccgatgagaagccggtgatggtccttgtccgcggtgactacgatgtcaatgacgttaaattaaagaactatctgggtgctgactttctggatttggccactgacgaacaagccaagacctatttgggggcagactttggttctttagggcccgttggcgttggtgaggatgttcgaatcgtcgctgatcaacgggttgccaacatgaagaatgccgttgttggtgccgatgaagatggttatcattatgtcaatgccaattctgatcgtgatttccgaattgatgacgtggacgattttgtggttgtcaaagaaggcgagaaaacacctgatggtaagggaacactgaaatttacccgtggcattgaaattggccatatcttcaagctgggtacgcgctattcgaagagtctcaaagccaacgtcttggatgaaaatgggcgcgctgtgccggtcatcatgggatcgtatggaattggtgtcagccgcctactttcagcaatttctgaacaaaatgccgatgaaaatgggttggtatggcccaaagcggttgccccatttgatgttcacatcatccccattaatgccaaaaaagccgttcaaatggatttagctcatcaaattgaagcccaattaacagctgatcaattacaggttctggtcgatgaccgcaaagaacgggccggggttaaatttgccgattctgacttgatgggaattccactgagagtaacaatcggaaaaaaggctgaagaggggattgttgaaatcaaaatccgaaaaactggcgaaaccgttgaggttaacgtcaccgaattgagtgacacaatcaaaaaaatgttgaagaatcttgactaatgatgtcgtaactaattaatatagacgtatgttttcgtcacttctaaactggttggaccaaaacttgggttttgtgtccagccagttgttgttaaaccgttatttttagaagaggtattgtgatgagtttggatcgaaatcaattatttgaaaagttgcttgaacagcttcaatggacacaggcaaatgaattgccttattttgaggatgctaaaattgatcgcctggaagttcataaacaaagccagcggtggcaatttgacatttcacttccacgaatcctgccatttgaggtttttaacgattttaatgccagactacagtctgcgtttaaagaaattgctgatgtttcactgaatatttctgcaaaaaatgatacctttactgaacaactgcttcggcaatactggcaatgggtcgttccacatagtggggttacctcaccgttaatgaaggaattatgtgcagacaagtttccctccattgtcgattcgcgggtggagtttgtcgctgaaaatgacatcgtcaaggactttatgaccaacactgccttggggccaattgaagatgcctttcaacgggcaggttttcccgactttacaattcacacgatcgtcgatgaaagttcttctcagcaaaacattcaagccctcaagaagaaaaacgatgctgccaatgcggaattagttaagaaggctaaccaagcgatcaaggagaatgctcaagctcatcccaagagtggtaacggtgggggcaagtcaaccattggtcggcgaatcaaagatgatttacccgtcatgaagatggaagaaattgtagaagaggaacgctctgtggttgtctctggctacattttcgataaagaaatccgggcattgcgttccggccgccagcttttgatgctgaagattactgactatacatcatccattcaagtaaagaaattttccaataaaggtgaagaagcgctctttgaaggcgttaacgaaggcgattgggtgaaggttcgtggtagtgtccaagaggataactactctcatgaactaactttgaatgcctatgatattaaccccattaagacggttagccgtcaagatactgcagatgatgataagaaacgggttgaactgcacctgcacaccacaatgagccaaatggatgccactaataacattgccgactttgccaagcaggccaagcactttggccaaaaagcgctggcaatcaccgatcatgcgggtgtccaaggatttccagacgcctttcatgccggccaaaaaaatgacatcaagatgctctatggtgttgaaattaacctggtggatgacggcgttccgattacttacaatgataagcacgttccgttaaaggatgcgacttacgttgtttttgatactgaaacaaccggcttatcagccatttatgaccgtgttatcgagctttcagccgttaaaatgcagaacagtaacgtgattgatcaatttgaagaatttattgacccgggttttcatttgtcggaacgaacgacgaatctgacgtcaattaccgatgagatggttcacggctccaagtctgaggaagaagtcttcaaacttttccgggaattttgtggcgatgcgattgtcgtcggccataacgtgacgtttgatatggggttcatgaacaccggctacgttcgtcatggcatgcatgagatgcaaaatccaatcatcgatactttgactttggccagatttttgtatcctaatttacgtggttatcgactcaataccttggctaagaaatttgatgtcagtttggaacaccatcatcgagcaatttatgatgctgaaaccactggccacttaaactatctatttttaaaggatgctgaagatcgatacggcattgtctatcacgatcagcttaatgatcacatgactgataacgatgcgtaccgccatgctcggccgtctcacgccattttattggccaaaacccaggccggcctcaaaaacatgtttaaaatcgtttccttgtcaaacgtcaagtacttctaccgggttccacgggtcccccggacgcaactggagaagtaccgcgatggcctgattgtcggttctgcctgctcatcgggtgaggtctttacagccatgatgcaaaagggattggatgaggcccgccaaaaagctggcttttatgattatcttgaagttcagcccaaacgtgcttacgcaccactgattgaatccggtttgattgccgatgatgaaaatcttgagcaaatcttaaccaatatggtcaaacttggcgatgaactgaataagccggtcgtggcaaccggggacgttcactatctcaatccgcaagattacatttatcgaaaaatcttgattaattcccaaggtggcgccaatcccctgaaccgtcaagaattaccagaccttcatttcctcacaactgatgaaatgttgagtgacttcaacttcctgggcccagaaaaggccgaagaaattgttgtggacaacaccaatcaaattgctgatgaaattgaagatgtccatccattgaaggataagttgtacaccccaagaatggaaggggccgaagacgagattaagtcacggacgatggacaccgcccacgcttggtatggtgatccactgcctaagattgtttctgatcgtttggataaagaattaaagagtatcatcggaaacgggttctcggtgatttacttgattgcgcaacgactggttgccaaaagtaacaaggacggatacttggtaggttcccgtgggtcggttggttccagtttggttgcgaccctcaccggaattactgaggtcaatccactgccgccacattatcgttgtccgaactgtcaacacactgaattctttaccaagggtgaatacagctccgggtatgatttgccacacaaaaagtgtcctgaatgtggcaccatgatgattggcgacggtcacaacattccgttcgaaaccttcttaggcttcaccggaaataaggttcctgatattgatttgaacttttcgggtgattatcagccaattgcccataactacaccaaagttttgtttggcgaaaagaatgtttttcgtgccggaacgattggtaccgtggccgataagaccgcctatgggtacgttaaggcttacgaacgcgataagggtgaagtctaccgacaagccgaggaagatcgactggcaaagggcgcaaccggcgtcaaacggaccactggccaacatccggctggaatcatcgttgtcccggattacatggacatctatgatttcacgccgatccagtatccagccgacgatcaggatgccgcttggcaaacaacccacttcgatttccactcgattcatgataatattttaaaaattgatatcttgggtcatgatgatccaacgatgatccggatgctccaagatttgtcaggcatcgatccaaaaacgattccaatggatgatcccggcgtgatgtcgatcttctccagcccaaaaatcttgggagttacggaagatcagattcaatcaaagactggaacactgggagttccggaatttggaactcgatttgtccgtggaatgctcgaacagacacatccaagtaactattccgagttgcttcagatttccggtttgtcccatgggactgatgtttggatgggtaacgccgatgagctgattaagaatggaacggcaaccattgccaatgtgattggatgtcgggataacatcatgaccgacttaatcaattggggactggactctgaattgtctttccagattatggaaagtgttcgtcatggtcgtggaattcctgacgactggcaagccgaaatgaagaaagccaagatacctgattggtatattcaatcgtgtctgaagattaagtatatgttcccccgcgcccatgcggctgcttacattttgatggcccttcggattgcctatttcaaagtctacttcccaatggtttactatgcttcatacttctccgttcgtgccgatgattttgatattgtctcgatgtgcagaggtaaagaagcggtcaaaaacgccatgcggatgattaatgataagggaatggaagcttcgaccaaagagaagaacctgctgacagttttggaactggccaatgagatgctcgaacgcgggtatcactttcaaatggtggatttggacaagtctgatgcgagtcaatggctgatcgatggtgatacgttaattgccccatttaattcagttccaggattggggttgaacgtggctaagcaaattgttgctgccagagaggacaagccgtttatttccaaagaagacttagccaaacgcggcaaagtttccaaaactttgattgacttcatgactgagaacaatgtgctggcgggattgccggatgaaaatcagttgaacttgtttgatttgatgtaaggcgagcataattgatttgcacattggcgttaaaacgcgccagccttgtaatgaatcatcggatatgttatagttaatttactaaataacttgtaagggagtgagcagagatgctcgctctttttaatggataatttttaggaggcctatttttgagcaatgttgttgaaacggtcaaacaagttgttgaaccaattctggaaaaacactcattttacttattcgatgttgagtttgtaaaagagaacaaaagctggtatttacgggtttatattgataaaaaaggcggcattaccattgatgactgcgtcttggtcagcgatgaattaagcgaaaagctggatgcaatggatcccgacccgatcccccaggcctatttcctggaagtttcgtctccgggtgctgaacgaccacttagaaacgacgccgaactcaaacaggcaattggcgagtatattcacgtttccctctatcaaaatcttaacggcaataaaacatttgaaggcaccctgaagtcgttggatgacgacaaactggtgcttcaaaatgataagtggggtaagcaggatacgttggaagtaccgcggaacttaattgccaaagcacggcttgcaattcaattttagttaaaggagacacaataatgagtaaagaacttttaggagcgctgtctgctctggaagaagaaaagggcatcaaaaaagaggttgtcattgaagccttggaagccgcgttggtttcggcatacaaacgaaactacggtcaggcccaaaacgttgaagtgtcattcgacgacaaaaaaggcgagatgcacgtttacgccgttaaaacggtggtcgacgatgttgttgacgaccagcttcaggtatctcttgatgaggcccttgaaattaacaaaggttatgaactgggagacgaaatcaaattcgaagtgacccccaagaactttggccgaattgctgctcaaaccgctaagcaggtaatcatgcagcgggttcgggaagctgaacgggaaaacgtttttgatgaatattccaagtatgaagatgaattggtgactggaactgtcgagcgtcaagacacccgatttgtttacgttaatctggggaaagttgaagccgtgatgggttcaaaagaccagatgcccaacgaagtctatcgtccacaggatcgtatcaaggtctatgtcaccaaagttgagaatgcgaccaagggtcctcaggtgtttgtcagccgaacggctacagggatgctcaaacgtttatttgaacaagaagttcccgagatttatgatggaactgtggaaattgtctcaattgccagagaggccggcgaccgggccaaagttgccgttcgctcaaacaactccgacattgacccggttggaaccgccgttggcccaagaggtcagcgggttcaaaccattgttaacgaactccacggcgaaaatatggatatcgttgagtgggatgaagacgatgcatcttatatcgccaactccttgaatcccgctgaggtcattgatgttatctttgatgatgacaacgagcgggcctgcacggtcattgtgcctgactaccagttgtcattagcaattggtaagaaggggcaaaatgctcggttggcagctaagctaacgggcttcaagattgacatcaaatcagaaactgaagccaaggaaattcttgccaataaagccgctgccgctagcgatgatacagaagctgatgaggcttccgaccaaggcgatcaaacggaggattcaactgaggatgccccgacagacggtgcggatgttaataccaatcccgatgagtcgaatgaggacactcaagactaatttttaggaggcgattttttgaaaaaacgaaaaattccaatgcgtaaagatatcgttactggtgaaatggcgccgaaaaaggaattagtcagaattgtccgtgactcagacggccacgtttcaatcgatgagactggaaagaagtccggccgtggtgcctatatctcaattaacgttgagattgcccgcaaagctaaagcggaacacacttttgaaaaagtcttttcaacaactttggatgacaacttttatgacgatctaattgcctatgttgaccataagcaagcccgaaaagagttgtttgaagatggacaatgatcaggcaattttgaattttttaggtctggcacggcgggcaagcaaaattgtctccggtcaagatatgcttttgtctcaaatccgcagcggcaagatttttttcttgtttatcgcagaagacaccggcaaggcaactcaaaagaagtttaatgataagtcaaattactatcatatacccgtgaataacagttacactaaagcagtgcttagtgaagcaattggaatgaaacgaaccattattggcatttccgatcggggtatggcaaaaaaattggttgaattaaccgataacaataaaggagagtgattatatggggaaaaagcgaatttacgaattagctaaagaactgaatgtctccagtaagcaaatcgttgaccgtggtaataaacagggcttcgatatcaaaaatcacatgtcaaccgttgacgctaaccaagagcgtcaaattcgggcgatgtttagtaaaggcggcaaacaatcgactggaaatagtcaatcaagccataagagcagcaccaacaatgttcattcggcaaactcaaagccaaaagaacatgccaatgctcatgcacagagtcgaccggctgctcaccatgacagcaacgggtcccatccggtaagccgaaacacacagcaggctaaccgaaatgcagagagcaaccgtaataacaacggccactcgagtgttgctcgcaacacaaataatactgctcaaagaaatcattccaacaataataaccattcgaataatcaaaatcattccaacaattcgaaccagtccaataatcaccggaccaaccagaataatgatcgacgcaatcatcaagcttcaaacaattcatccaatacgtcgacccgtaatacaaacagtcattcaactggcagcagtacaactgcaagcaatcataccagttcgaataataacagtaatacaaaccgtagttccaacaatttctcaaatcacaataccggcagtggtcgttttggcggcagcttgaaccggaataataatcgtggcggctcccgtaaagccaacaagaagcgcaacaagaaacaacgtaagcaaaagaatcaacgattgcgtgaagttgaacaccatggtgcaccggaacgaaagaatcgtccattaccaaaggtgcttgaatatcaagatggtatgaacgcccaggaattgggtaaattgctgcatcgtgagccagcagaaattgttaagaagttatttatgctcggcgtcatggtgaaccaaaaccaatcacttgataaggatacgattgagattttggcagccgactatggtattgaagcaaaagaaaaagtccacgaagatttgtccgatttggataagatctttgaaaaagaaatggagaatactgagcacttggtatcccgaccaccagttgtgacgatcatgggacacgttgaccatggtaaaaccactttgctggatcacttgcggcattcacacattactgctggtgaagcagggggaattactcaagcaatcggtgcttatcaagttcgtcacggtgacaacctgatcactttcttggatactcctggacatgccgcttttactgaaatgcgtgctcgtggtgccaatattaccgatatcacgattttggtggttgctgccgacgatggcgtaatgcctcaaactattgaggctatcaaccatgccaaagctgccaagacgccaatcattgtggctatcaacaagattgataaaccggatgccaatccacagcatgttactgatcaattgatgcagtatggtctggttcctgaaaaacttggtggtgataccatcttcgttgatatttcagccaaatttggtaagaatattgacgaattgcttgatatgatcatcttggaagcagaagtgatggaattgaaggctgatccggatcaacccgctgccggatcggtaattgaagctcgtttggatcaaggtaaggggccggttgccactttactggttcaacaaggcactttacacgtcggtgacccaatcgttgttggtcatacattcggccgagtgcggaccatgaccaatgaacgtggccgcgatgttaagaaagcaacgccatcaagcccagtgtcaatcactggtttgaatgaagtaccagaagctggcgatcgttacgttgtctttgatgatgaaaagaccgctcgtgccgttggtgaagaacgtgccaaggaagctcaagttgaggaacgacgaaagaccacccgggttaccttggacagcttgtttgattcgcttaaagaaggcgaaatgaaggaagttgacatcgtaatcaaagctgacgtgcaaggctcagttgaggctttggctaacagtctgcaaaagattgaagttgaaggcgtcaaggtcaacatcattcattccggggttggtgcgattaatgaaagtgatgttgccttggccgaagccagcaacgccattatcattggttttaacgttcgaccaacaccacaagccaagtcacaggctgacagcgaccacgttgacattcgtcttcaccaagttatttacaacgccattgatgaagttgaatcagcaatgaaggggatgcttgctccgacctacactgaacaagttactggtgaggttgaagtgcgcgacatcttcaaggcttctaaagtcggaacgattgccggtggtatggtggttgacggtgtcgttcagaagaatagtaaagttcgtttgattcgtgacggagtcgttgtctataccggcgaattaaacagtttgaagcgcttcaaagatgacgtcaatgaagttaaacaaggctttgaattaggtttaactatcaaagattataacgatatcaaagtcggcgatgtgattgaggcatatgtcatgaaacaagtgcctgtcaagtaatttggaggtgttttgatggctcattatcgggttggccgattagaacaggaaattcaaaaagaagttaacgacattctgttaaagcgggtccgcgatcctcgagttcagggcgtcactttaactggtgtcgaagtcacaggtgatctccagcaggcgaccatttattacagtattttgtccgataaaaaagaggacgaagaaacaactgcaaagggattggaaaaagccagcggactaatccgcggcgaacttggtcatcggttaagtatttataaaacaccggaaatcaagttcgagctggacacatcagttcagtatggtgacaagattgaccgattaattaataaattaaatcaagatggtgaataatcatctcaactgtccacgcctgaatggctgggcagtttttttgtgatataattttcttacatgaaaaaattaggagaattcgaatggatggcgtaattgcactatataaagaacgtggcatgacaagtcacgactgcatcagcaagttaagaaaaattttgcacaccaaaaaagttggccataccggcaccttggatccaaatgtcgatggggtgctgccaatttgtatcggccaggcgaccaagatcagtgaactgttaatgcagtccggaaaagtatatcgcggtgcgattaccctgggagtcgcttatgatagtgaggatctggacggtcacttgattgaacaggtgccggttaaaacgccgttgacggatgaacagattaacgccgctctggctcaattgaccggtgacattctgcagacgccgccgatgtattcggccgtcaaagtcaatggccacaagctctatgaatatgcgcgcaaggggatcaccattgaccgggatccacgccggattcgtattgattattttaagcaaattaaaccagcaacgtatgatgacgctgcccacacgcagacaatctattttgaagtcggctgttcaaaggggacttacgttagaacgctggcagtagattttggaaaacgggttggcttgccgtctgtcatgtctgatctgaccagaattaaaagcggtggttttgatatttcacagacatccactttggctcaagtcaaagaagccgttgctgcggaagacctgagtatcgtccttcatccgttatctgaagcactggcggaatatcccggttatcaattggatgacagccgctggtcaatcgtttctcatggcggtttcttggaccaatcaatcagtcctacccacgcgccggtagttcgattagattatcaacaacaggtgaaggcattataccggttggacgaacaaatcggtcaatacagaccgtttagaatgtttttagcttaatgaaggtggtttttaacaatgcaaatttcaagattacactatccgttgtctgatgactttaaggtcgatggtccgacagtcgttgcaatgggattttttgatggctttcataaaggtcaccaagcagttttacaacgggcaaaaaccgaggctgaaaagcgcggtgccaagttggcggtgttgacatacgatcatcatccggcaattgtttaccgaaaaatgtcgccccatgaacagcgatatttgacgctgaatgattataaaatgcagctgctaagagattttggtgttgaccaagtctttctggtgaattattcgtatgattttcaaagtcaaactccggaagaattcatcaacaactttctaaagcggttcaatgcagtggcagtcgtggctggttttgatcacacctatggtgataaaaaagtggccacgatggccaatttccccaaatttgttaaaggggcttttgacgtcatcacagtgccgtctgtcgacattaatgataaaaaggtcagttcgactcggatccggattgaattggattcaggcgacgttgatagtgttactaaattgttggggcgcccatttcaaacccgtggcgtcattgtccacggcgaggagcgggggcgactgttgggctatccaactgccaacgttgaacactcagaatatcaatggctgccaacgattggaatctacgtggtcaccgtcgaaattgccggcaaaaagtacttgggaatggcttcaatcggcaagaatgtgaccttctcggatgttcatccgatgacggtggaaatcaatttgatggattttgaccgcaacatctatggtgaagtcgtcaacgtgaactggctttcatacttaagagctgagatcaaatttcagactcccgaagatttaattgatcagttggataaagacaaagttgcgacccgtgagtacttagagcagcatcctgagatcttgaattagcactattagcactctacacaaaataatgctaaaataaggctatattcccttgacttataatagacggtttgttaaattataaatgtgccttagcactcggttatattgagtgctaaaaagaggtgatttgggtgctaacggataggcaaaaagatattcttcaaataatcattcgtgattacacaagaacgggaatgccagttggttccaaggcattggctgaggagtttccgacccacgttagttccgcgacggtcagaaatgatatggctgcacttgaatcaaagggcttaattacgaagactcacttttcttccggacgggttccatcgatcgaaggttatcgttactatgttgataatcttgttcagccggacccgctggacgaaggtgcggaagacttaatcaaaacttcttttaacagtgagttcaatcggattgacgagattgtccaggagtcagccaaagtattgtcagatttgacaaattacatggcgctgacttttaatccagagtctggcgataacctgaaacttggcggtttccggttggtcaagttggatgatcgtcaggtaatggccatcatcgttaccaatactggtcacgtcattgataagattttcaggctggccaacgtctcgtccgagcaacttgaaaccattgtgaatatcattaacagcgaactggtcggcaagccgctcaaggatgtcatggacaagttaaagtttgatattccaatgttgatgaccaaatatattcagaccccggaaggcttcttgaagatcttcggggacatgctggacgaagcgggccgagacaaagttcacgttgatggtgaactgaatctattgaagtttgcagaacggcaaaatgttgatcggcttaagccactctacaatttactgggcaccgaggattcggtttcaaagattattgatcccaactctaaagatgttcaggtcagaattggcggcgagctgcgcaacgacctgttaaaagattatagtattatcacaggaacttatgatttgaaagagtatggtcatggcgtgattgcagtcattggaccaaccagaatgccttactcaaaggtcatcggaattgttggtgctttgcgggaagaattgaccaagaagttacttggctactacgatgacgataatcaataatttaaggaggcgattgtttggcagaaaacaaagatgattcggttaagaagaatccaagtgggccaacacaggaccaatcaactcaaccagccaaggcagccaaaaaggcagctaagccggaaaaaaaggctgatcaggcccaaagcccagacgcaaatgatattaaaaagttgaaacaaacggtagtcgatttacaaaagaaacttgatacaatggaagataagttccttcgtgcggaagccgatatgcgaaatattgaaacccatgccaagaaggaacaggctgatttaatcaagtatgacggccagcagctggcccatgatatcctgcccattgttgataacctgcagcgagcgcttaaagttgatgtcaccgacgaaagcggcaagcaacttaagcagggggtttcaatggtttacgagcattttaccaaggctttgtctgataatggcgttgaggtgattgatgcgttgaacaaaccatttgatcccaagttcgatcaggctgttcaaacggcgccggcagatgatgatcatccagctgacacggttgttcaggtcctccaagacggatatcgtttgaaggaccgagtgcttcgaccagcaatggttgttgtagcaaaataaaactttaaaagaaaaagaggattatttatggcaagtaataaaattattggtattgatttaggaactactaactctgccgttgctgttcttgaaggcagcgcgcctaaaattattccaaacccggaaggtgcccgtacgacaccatctgttgttgcatttaaagatggtcagccacaagttggtgaagttgccaagcgacaagaaatcaccaaccctaacacggttcgttcaatcaagagtcacatgggtgaacaaggttacactgttgacattgaaggcaagaaatacacccctcaacaaatttctgcaatgattttacagtacatcaaggactttgctgaagattatttaggtgacaaggttgaaaatgccgttatcactgttcctgcctacttcaatgatgcacagcgtcaagcgactaaagatgctggtaaaattgccggtttaaacgttaagcgaatcatcaacgaaccaactgccgctgcgttggcatatggtttggacaaacaggagaaagatgaaaagattctggtttacgatttaggtggtgggacgtttgatgtttccatccttgaattgggtgacggtgtcttccaagttctctcaaccaatggtgatacacatcttggtggtgatgactttgaccaacgaattattgactggttggttgacggtttcaagaaggataatggcgttgacttatccaaagataagatggctttgcaacgtttgaaggatgccgctgaaaaggctaagaaggatctctctggtgttactgaatcagaaatcagtttgccatttatttctgccggtgacaacggtccattgcatctgcaaacaaccttgactcgtgccaagtttaacgaattgactgccgacttggttgccaagaccaaggtgccatttgataatgccttgaaagatgccaaattaagtacttcagacattgatcaagtgatcttaaatggtggttcaactcgaattcctgccgtccaagaagccgtcaaatcatggactggcaaagattcaaaccactcaatcaaccctgatgaagccgttgctttgggtgccgctgttcaaggtggtgtgatcaccggtgatgttaaagacgttgttttgcttgatgttaccccattgtcattgggtattgaaaccatgggtggtgtcttcaccaagctgatcgatcgcaacacgaccattcctaccagcaagtcacaagtcttctcaacagctgctgataaccaacctgccgtagacattcacgttcttcaaggtgaacgtccaatggctgctgacgacaagacgttgggtcaattccagttgactgacattccggctgctcctcgtggggttcctcaaatcgaagttaagtttgatattgacaaaaacggcattgtgaacgtttctgccaaggataagggaaccggtaaagagcagaagatcaccatcaaagattcatcaggcctttccgatgaagagattcaaaagatgatgaaggaagctaaagaaaacgaagaggctgataagcaacgtaaggaatcagctgatttgaacaacgaagtcgaccagttgatcttccagactgacaagactctcaaagacgtcaagggtaaggtttccgatgacgaaatcaagaaggctgaagatgcacgtgatgccctcaagaaagctaaggaagacaacaacgttgacgaaatgaagtctaagaaggacgatttgaacaagattgttcaagatttggctgtcaagttgtatcaacaacaagctcctaaagacggcggtgctgctgccggcgaaggtgccaagggtggttcaactgatgacaaatccgacggcaagggtgacgatggcaccgttgacggcgacttccacgaagttcacgatgatgataaaaagtaatttataatcagatattgtaatgagaagtcaaggccggctggctttggctttttgttaaaatatggtatattatcatggttaatgaattgaatgaggatgggagtttctaatggcagaaaaagattattatgacattcttggagtttccaaggacgccagcgatgacgaaatcaaacacgcctatcgtaagctttctaaaaagtggcatccagatatcaataaagcgccggatgctgaagcaaaatttaaggaaatcaatgaagcatatgagacgttaagcgacccacaaaagcgcgccaactatgaccaatatggttcggccgatggtgccggtgccggctttggcggcggtggccaaggcgggggctttggtaactttggcggcagcgctggtggatttggttttgatgacattttcagtcagttctttggtggcggccaacagcgggcagatccgtccgcaccccaacagggccgtgatcttcaataccagatgaccctggaatttgaagaggccattttcggtaagaagactgtgatcaagtacaaccgtgaagcccagtgtaagacttgtggcggaacgggtgccaagcctggtacttcaccagtcacctgttcgaactgtggcggccgtggttacgttaccactgagaccaacaccccacttggcagaatgcaatcccgtcaagtttgcccggtttgtcatgggactggtaaagagatcaaggaaaagtgcccaacctgtggtggtagtggtaaaaccgacgagcgtcacgaacttgaagtcaacgtaccagccggaattgatgacgggcagcaaatgcgtcttcaaggccaaggtgaagccggggacaatggtggtccttacggtgacttatacattgtcttccgagtcaaacccagcaaagactttacgcgtgatgggtcaacaatctacgttgaccagcccatcacttttgccagagcagcacttggcggcaaaatcaaagtcaaaacggttcatggtgatgttgagttaaaggtaccagccggaacccagaccgggacaactttccgtctcaaaggtaagggtgcgccccgccttcgtggtaacggtaatggtgacgagcgggtgacggttaatgtggtcacaccgaagtcacttaataagaatcaaaagattgccttggaagcattcgccaaggccagtggtgacaacattgctggcaagggcggtagtaatttttttgacaagatgaaagatgcttttgataaataacatgatcatgtggaggggtcagccggctgttttgccgttgcttgacctctttttatgtcaaggcaaccctgctggttcggtttaactttggataaactggaatggctggtataattattatcagtaaacaaatgaaagtgagaatacaacatggatttagataaaatgaagaatcaccaaaaatatattcgaaacttttccatcgttgctcacatcgaccatgggaaatcgaccttagccgatcgaattctggaaatgacggataccgttgccaagcgggatatgaaagatcaattactggataacatggacctcgaacgtgagcggggcattacgatcaaattgaacgccgtggaattgacgtatcatgccaaagacggccacgactatgagttccatttgattgataccccaggacacgttgacttctcctatgaagtttctcgaagtctggctgcctgtgagggtgccgtcctggttgtcgatgcagcacagggagtcgaagctcagacactggcgaatgtttatctggcaattgatgacaatttggaaattgtgccagtcattaataagattgatttgccctcggctgaaccggaaaaggtccgaaaagaaatcgaaaacgtgattggcttggatgcctctgatgccgttctggccagcgcaaaaaagggaattggtgtcccagaattgttggaacaaattgtccacaaaattcccgcgccggacggagacgttgaaggacccctaaaggccctggtctttgactcggtttacgatgattaccgtggggtcgttttgagtgtccgtttatttgaaggaactgttaaacccggcgacaagattaaaatgatgaacagcggcagtgaatatgaagtcactgaagtgggggttaactcgcctaaacctgttaaacgcgactatctgatgtctggagacgttggttacatcaccgccagcatcaaagatattacccaaacccgagttggtgataccgtcaccaatgcccttgatcctgcagatgaagcgctcccgggttatcgggaaatgcatccgatggtttatgccggactttatccaactgacaatgccaagtttgacgatttacgagaggcattggaaaaattgaagttgaatgatgcagcactggagtttgaaccggaaatttccaaggcgctgggatttggttttcgttgcggattcttgggcctgctgcatatggacgtggttcaggaacgtttggaacgggaatttaatctggaactgatcaccacggcaccatcagtaacctatgaggtcaagctaaccgatggcgagtccaaagaagttgaaaatccatctgaaatgccggatgtttctgctatcaagcaaatttctgagccatacgtcaaagcgacaattatggtacccaatgattatgtcggcccagtcatggaactttgtcaaagacgacggggtgaatttgacacaatggaataccttgatgagtatcgggtcaacgtgatttatcacatgcctttatccgaaattatctttgatttctttgacaaattaaaatccagcactaaaggctatgcatcccttgactacgagttggaagactacaaacccagcgacctggtcaaaattgatattttgctgaatggtgaaaaggtggatgctttaagcttcatttctcaccgtcaatttgccgcaccaagagctcgagacatcgttggtaaactcaagaacattattccccgacagaactttgaaattcccgtccaagcagccattggcgccaaaattattgccagaaccaatattaaggcctatcgcaaggatgtgaccgccaagttatatggtggtgatcgaaccaggcggatgaaactcttggagaagcaaaaggttggtaaaaagcggatgaaggctgttggaaaagtggatatcccccaagaggcctttatggctgttttgcagactgatgaggaagaaaaaggcgacaaataggtacttttactgggccattgggcttaacgaaataatttattcagatcaataattcttgcacatgcccgctacctgaagaaccgtagtccagccagaaatttcataaaaaagcaagcaacagccagtgatattgaggaaatcaaatcactgattcgtttcaggcaggcaatgcttgttagcaacgacacttcggttgagtaaacgggagcgttggttaatggttgcgacgctaaattaaggtaattttggtatttaaaagacgtcttactaggcgccttttctattgaaacggcctttatgacgtcaaaaaagaccgcagcgaaataactcgttgcgatcagatgtcttcaaactattttgttggactcgttaattgctcactatcagaaaacgcgcggctgtaaatagtctctaagtgttccagctccagtttgttggcgataacatcgttgaataactgttcaatggccactgtcatagctttttcgtccggcagggcatttgtggcctcagccttggcctgttgcatttggtataactcctgcaggagattaatgagtcgatgacgaaaatgggataactgtaccgaatgaggcaggtcatcgttttcatgtttgacatggtaatcaaaataccgttccagtttttcaaccgtccccagtgataagttatccaccagtcgcgtgtgatttctgagtcggatgataattgatgagttcaccccggtcaacttctggatctgataggcactgtcttcactgtcgaggacagcttgaaccttttgtcttgcatccatattcattcccccggaaatttagaatttgatgataaaaaggttgcttcggcatatgtatttcttgtcacatttaccatatgacaagtgacatataattgtcaaatttttcgctatctcactagcggtgtgtctgctaaccaatccgcaattcggtgactaatttggtatcgataaccggcttgccgtcctctccttggtggtgaacgacgcgatccaacatgccgttatcgatgatgtattgatcaaagaactgcttggttggaacctgcaggaggcttcggtcatgcgactgttcaaaagctacttgatccaagaccaagtcttttggagtggcagaaaaaatattataaattgctttaagggcgacttcacctgatttcaaaatggtggtatccaaataacttcttaggaataactgatggccctcaaaaaccgtatcacttgaatgtgattccaacactgcccggtagcgaatctcaatcgtgtcgggtcgaatcttattgataaatcgaatgcggaataattccattattctcagctcctttcctacatcatatgctaaacttgttaaggagtgcaactttgattcattatgagaaaatgtttgcgtttcttctcacattcaattattatatatattaattgttttttattcgattcgaaaaattaaaatttaataagctgggaggtgttaatgattctaagtcgaacaaaacaatatttaagaaaaaacggttacttctataaaaaagaatatattcggcccttactgacaccggataatatttatattttcagatttggccgcgaccgcttggataaccggcttattattcgctacagtcataagtggactggcagacagcgaatcaacgaaattgatttacggctgcataagcaaaagcatccccggattttcgagaacgaatccgaactattgaactacttggaaggacacctattgaagcacgaggcaaaggtccgtgcgcgtgagaaagaaaaacaacatgaaatatcagatggtgcatctaagtgatatggattcgaaatcaaagctggtttttgcctcattgtggggtgaagccagctttcattttagaatcaaccgacaaaggagaattccatggactggacagaattatcaattatgacgacaagtgaagcggttgaggccgttgccaacattttgatggcatacggggcgaccggggtttcaatcgaagatgccaaagattttgagaaattaaaacccggccgctacggagatcatggtgaaattgtcgatcctaaagatctcacccacattaggcaaggggcgattgtatcagcttattatcccaacaatcagcatattgatgaccaagcagaccaaattgccaccagggtccgaggtttggcgaagtttgatttgaatcccggaccagcagaggttcacctgacgccagtcgtgaatcaagattggcaaactgcctgggagaagtattaccatccagtatcaatttcgcgattcatcaccattgttcccagttgggaagactatcagccaaaatccactcaggaaaaaattgtccgcttggatcctggaatggcctttggaaccggaacccatccaactacccgactatcacttcaggctttggaaatggtcatgcagggcggcgaatcaattctggatgtcggcactggttccggtgttttaagcatcgccgccaagttgatgggcgcgggggaaatccacgcgtacgatgttgacgacatcgctgttgaatctgcagaaaagaacattcaactcaatccaggtgctaaaggaatccgcgttgcggcaaacgatctgctggccggaatccatactcaagctgatatcgtggttgccaacattttggccgaaattatcgtgccgctggttccccaagcatgggataatctcgttcctggtggctttttcctcacatccgggattatcaaggacaaatttgaaaccgttgaaaatgcgatgacctcacaaggatttcagatcattgaaaccttgagaatgaaagattggtatggggtcatcgcccaaaagccaaaggacgaggacaaataatgcaacactattttgtaagtcaacatttaactgtgggacagtcgattgaacttcccaaaactatttctcatcatttgggccgggttttgcgtgccgaagttggtgaccggtttgaactggttggcgatgaccaccaggtgttcgaagctgaaattagtcgactggagggaaaccaagttgccgccaatattatcaagccacttgatcacaacgttgaattgccggtcgctgtcacgattgtcagtggtctgtccaagggcaacaagcccgaatggattgttcaaaaggctactgaacttggtgtggctcacgtgattttcctgccgatggactggtcgattgttaaatgggatcaaaaagcaactaaaaaaattacccggctgaatgaagttgcgttgagcgctgctgagcagtctcatcgaaacgtcgtgccaacagtggcttatttaagcggattagatgctttattccaattagattttgatacccaattggtcgcttatgaggagtccgccaagcaaggcgaggaaaccaatttggtcaaggccgtcaagcagactccttcaggcggcaccatggcggctgtcttcggtccggaaggcggcgttagtccggctgaagttacccaattagtcgatcacgactttgtgttagctggtcttgggccacggattatgcggactgaaacagcaccactgtactttctcagtgccgtttcaacgctgaccgaactgatttagtttgctgaataactttgacaacaatgatattattatgataaagatgatttgatgatgcctttgggcaaatgagagaagagttgatacaatggcaactaaaatttggacaccggacgatgtcattaataaggtttctgagtatatgaacaaggaacatgttgatgagattcgaaaagcttaccaatttgcaaaaattgctcaccagtaccaaaaacggcagtctggtgagccctatattacccatccgactcaggtggctggtattttagctgacctgcatatggatcctgagaccgtctcagccggttttcttcatgatgtagtcgaagataccggggctaccttaggcgacatccaagagctgtttggccacgatatcgccttgattgtcgatggggttaccaaactgtccaagattaaatataaatccagcgaagaacgattggctgagaaccaccgtaagcttttgctggcaatgtgtaaagacatcagagtgatgattgtcaagctggctgaccgcctgcataacatgcggacattaaaatcactgcggcctgacaagcagcggcggattgccagtgaaactttggagatttacgcaccaattgccgatcgtttaggtattggaaccatcaaatgggaactggaagacatttcacttcggtatctcaatccccagcaatactaccgcattgtgcacttgatgaactcacgtcgtgatcaacgggtggattatattgaaaaagccatcaaagaggtcaaaaaggcgatttctgcattgggcgtcaaggcggagatttatggccgacccaagcacatctattccgtttaccggaaaatggttgaaaagcacaaacagtttagtcaaatttatgacctgttggccattcgggtaattgtcgattcaattaaagactgttacgccgtattaggcgccatccattcagagtggaaacccatgcctggccggtttaaagactatattgcaatgcccaaagccaacatgtatcaatcgctgcatacgaccgttattggcccggaaggcaagcccttggaagtccagattcgaaccgaagagatgcaccgcgtggctgaatttggtattgctgctcactgggcctacaaagagggaatcacaaacggggtcaaaacctcgcaggataacaataaactcaactggtttaagcaaattatcgagctccaggaagatactgacgatgccgccgatttcatggatagtgtcaaaggtgaattgtttggcgaccacgtctatgtctttacccctaagggcgacgtttatgagctgccaaaaggagccggtccacttgatatggcctacatgattcataccgaggttggtaatcacaccactggtgcccgggtcaacggcaagattgtccctctggatcaccaagttaaaaatggtgacattgtcgatattattactgccactggttcagccggcccgagtcgtgattggctgaagctggttcacaccaggcgggcacgaaataagattaaacagtacttcagacaagaagaccgtgagaaaaacattgaggacggtaagaacctgatttccagaagactacgggaagccgggtttgagcccaaccggatcatggtaccggataaattgaccaaggcagccgttaacatgcattaccaacacgctgatgatttgttggctgcggtcggctttggggatttgcagccgactggggtggttaaccgattgacagaggatgcccgggcccaactcaaaaaagagcgtcaggatcaagctgaacgagaagttttggaaggccaccagaccatttctgaagattctgacagcgctaagaagcagaaaaaacgcaagtcctcaaatggtatcgtgatcgaaggcgtcgataatctcctagtgcgattgagtcactgctgtaccccggttcccggcgatgaaattgtcggctacatcaccaagggccgcggcgtgtcaatccaccgggttgactgcccgaacattaaaactgcggaagaaaacggtgagcggctgattgaggtcgcctgggctgacaatcctgaggaacggacgatttatgatgccagtttggccgtccaaggatataatcgggccggcctgctgacgaatgtcttgactgccgttaatagtgtcaccaagaacgtttcgtcagttaatggtcaggtcgataataataagatggccaccatctccctttcagttggcgtccgcaatttggagcagctggagcggttgattggggcaattaagaacgttcacgatgtttatttagttgaacgaaaattcagataggagttttgctggatgaaagtggttttgcaacgagtcaaggaagcgtcggtcagtattgacggtcagattcacggcaaaattggcaggggattcgttctgctggttggtgtcagcgatgccgacggtgaggcagaagttgactatttaacccataagattagtaaactgcgggtatttgaagatgatgccggtaaactcaatttggacatcaatgccgtgaatggcgcaattttgtcgatttcgcagttcaccttatatgcagataccaaaaagggaaatcgccccagctttaccaaggcaggcgaaccgcaacacgctgatcgggtgtatgagcaactcaatgaacgtctgcggcagaccggtttggaagttcaaacgggcgtttttggagccgatatgctggtgaatattcaaaatgatggtccagtgacgattatctttgatacggataacaaataaaaaatgatcagataaaaataaagtcgaatcgtgtggttcggcttttttaaggagtaacgaaatgattaatcaattattttgggattttgacggcacgttgttcgatacctacccgaaaatggtttccgcgtttgttcaagcattgggtgatttagggattgacgatgttgaaatcgatcaagaccagatttatgttaccatgcgccaacacgacgttgggacagccattcgaaagttctcagccttttacgggattgatgaaaaacagcttcgaaaattgaatcgcacccaccaaaccaaattggttgaagatgccctgccgtttcccggtgttaaagaggttttggaattggctaaatcaatgaagggacgcaactttttgctgacacacagggatgaccaggctaaaagcatgctgagaaagtttgatctgctggacgatttcagcggctttgtcacatctgatcagaattttccgcggaaaccacagcctgattcaattaactggttaattgagaccaaccaggtagacagaaaaaaagcgatcatgattggtgaccgcaagttggatgttgctgcgggtcacaatgcaaatatcgcttcgtgtctgtttgatcccgatggcacaatcgttgattccggcaatcccgagattcgggtcaccgaaatcaatgaactcgtcccatggttgaccaacaaataattaatgattgtttttaaaatagtttgcgatgccgtcgacaacgtctttcgcaagctttttttgataggccggcttttgaatttggttaaaatcttttttggtattgatgtagccaccctcaatcaaaatagcgggaaccgaattgtctcggattaccaggaagttaccgaattccaccccccgcgaacttaacggcagatttttcatctgctggttgactgattctgccaaatgtttggagtcgccgctatggtagaagtaacaggtgtagccagacgcaacgttgttctcatccgaagagtcaaagtggaaactgacgaagaggttggccgatgatgaattggcaatttccggcctggcggctaatgggacggttttatcggaactgcgcgtcatgacgacccgggcacctctcgcctggagcagtcgttcgactcgtttggcaacttccaaagtgtaccgtttttcgggttgcccggtcattgacagtgcccccgtatccgatccgccgtggcccggatccaaaacaattgtcgcttccgataagctgctgacattttgaacgttgctgttttgaaccagccaggacgctacccagccaatcgtgcgatgcttatagatgaccttgatccagttactttttcgactaatcacctgcaatcgctgtccatgctgaactttggcttttaccgagtaggtaacgtctggcccgcttcgaatatttaattgattgaccttaacagtcactgaattggattccagcgagacgatcaacaccaaaaatgtgatgatgatcgtcagggtggcaacaatccagcttttgttttcccaaatttttttcacagttcaatcgttccctcactcaaataatcatattatagttgaaataagcctgagaggccagtctgaatggaaataacgccgatgttcccttgacattttctggctggtacactagtcttatagacagttaaatatccaaccgataaaaagaactatcgaaataagcggcatacagagagcattcatttggtggaaggatgcgtcgattattttgaagtgacactttttgcttatgatggttaatagcgaaatgctattcgtgcgagcgttatccttgagaattaattaaggtggtaccgtgcgaatgcacccttgtctatggacaggggtcttttttttcggaatttaagtgggaggaaacaattatgcgatatcaacgaccaaaaggaacggccgatattttgccaggtgaagctcaaaaatggaactatgtcgaagagacggcccggatgctgtttgacgattatcgttatcaggagattcggacaccaatgtttgaaaattttgatgtcttttccagaacgtctggtgatacttccgacgttgtcacaaaagaaatgtatgatttcaatgataagggcgaccgtcacatgagtttacgccctgaagggactgctggtgttgtccgggcctttgtcgaaaacaagctttacggacctgaacatccccgcccagtcaaagtcttttatatggggtcgatgtttcgctatgaacggccacagtccggccgccagcgtgaatttcaccaaattggggtagaagcttttggtagtaatgagcccgaattggacgtcgaagtgattgccatggggatggatttgctgaaacactttggcttgtctggcctccggttggaaattaatagtctgggtgataaagcctcccgtgacgcatatcgtcaagcgttgattgactatcttgacccgcactttgatgagttgagtgatgattccaaggttcgtctgcacaagaacccgttgcgggtattggacagcaaagacaaacgcgaccaggaaatcgtcaaaggtgcgccatcaattttggactacttaaatgaagattcccaaaaacactttgataaggtcaaacaccttttggaatcactcaacattccgtatgtcgttgacccagatatggttcggggcctggattactacaaccacacgatttttgaaatcatggttgattccaaggccctgggcgaaggctacacaaccatttgtgccggcggtcgatacaatggcttggttgagcagcttggcggccctgaaatgcccggaatcggttttggccttgggatggaacggctgatgcttttgatggaagcccaaggggttaaattcccggttcttgatcaattggatgcttacgtagtcgggattggcgaacagaccagcgtcttgacgttacaaatcgtccaagcattgcgggcagacggtttcgcagctgaccgtgattaccttgaccgcaaaccaaaagcgcagtttaaaactgccaataagctgaatgctcagtacacaattaccattggtgaaagtgaactggaaaaaaagactgccaacgtcaaacagatgcggaccgggaccgaggtttcagtaccgctggctgagattttcaaagattttgatgagatcattaccaaatattttacagatgatgaggagattgattagacatgaagagaactacttatgctggccttgttgatgaacagctcatcggccaagaagttgtcttaaaaggctgggtccaaaaacgtcgtgaccttggcggcttgatttttattgaactgcgtgatcgtgaaggaattgttcagttagtattcagtgaggaatttggccaagatgctttagcggttgccgataaactgcgcagtgagtacgttgtggaagccaagggtaaagttgttgcccgggatcctaaagaaatcaaccctaagatgaaaaccggtaagattgaagttgacatcaccgatgccaagattttagccaccgctaagacaccgccattttatatccaagacggcattaacgtttccgaggacctgaagctcaagtaccgttacttggatcttcgccgccctgagatgcaaaaaaacattttgttgcgaaaccggattattcagtcgattcacagttactttgaccaaaatgatttcattgatatcgaaaccccaacactgacgaagtcaacgcctgaaggggctcgagattatttggttccttcacgggtttatcctgggtccttctacgcattgccacagtcacctcaacaatttaagcagttattgatgggtgccggttttgataaatactatcaaattgcgcgttgttatcgtgatgaggacttgcgtggtgatcgtcagccagaatttacccaaattgatatggaaatgtcatttgccgatcaagaagaaatcgaagatgtcactgaaggattcattgccaaggtcatgaaagacgccatgggcatcgacgttcagctgccattcaaacgaatggattgggacgagtcaatggctcgttatggaactgaccaacccgatgttcgctttggcatggaattaaaagatctttcagacattatgaaggatgttgatttcaaggtcttctccggtgctgtcaaagatggcggccaagtcaaggcaattgccgttcccggcggagctgagaagtattcccgaaaagatttggacaaatttgccgattacgttgaacgtttcggagccaagggcttggcctggttgaaggtgaccgatgatggctttaacggcccgatcgccaaattcttcaaggatgccgatctgcgtgaaaagattttggccaaggctgaagcaaagcctggcgatctattgctgtttgctgcagataacagccgggttgttgccaacacgctggcctatcttcgagttgagattgccaaagaacagaacatgattgacgaatccaaatttgccttcttgtggattgttaactggccattattcgactgggatgtcgacttgaaacgttacgtggctgcccatcatccatttacgatgcccaatgaagacgatgttcattacttaatgaatgaaggcgaagacccacacaaagcctacgctcaaagttatgacattattttgaacggccttgaattaggcggtggatcaatccgtatccatacccgggcacttcaagaaaaaatgtttgaagcacttggatttaccaaagagagcgccgaagcccaatttggttacttcctgaacgctttggattacggtttcccgcctcatggtggtctcgccattggcctggatcgctttgtccgcttacttgctgatcgcgataacatccgtgatgtgattgccttccctaagaactccaaagcagttgagccactgaccagtgcaccacaacctgttgctaccaaacagcttgaagatcttggcttgtttgttgccaaacctgatggtgaaaagtagtttcgagtttcaaattaactgatttcaataaaatcctgtaatctagtcactgattacaggatttttaatgtaatttttgtcatttacgtttatcattaggcaagacgttcaaaaagttttcgaaggggatttattttatggatgacgtttcaaaattaatgcgtaggcacacctacgtcaccaaaatttcaacttcatttatttacgcaattttagtgtcgattgcggttaattttttctggacacctggacatatttattcatcggggattaccgggttcgctcagctgttgaacaccatcagtacgcgggcgtttccgtttgaaatttcaactgggctggctttattcctgctgaacttgccattatttgtcttgtcgtggcgggcaattggccacgaatttaccattttcacaattattaccgtctttttatccagttttatgattcaattactcaaaccaattccgctcacccatgatccgattatctgtgcaatctttggtggggcggtcaatggatttgggaccgggttggcgcttcgaaacgggatttccactggtgggctggacattctgggcattgttattcgtcaccgaaccggtaactcgattgggacgattaacattgcctttaactcgttaatcatcgtttcagctgccgtcatgtatggctggccatacgccttttactctgtcctcagtctaatcgttaatgcgcgcatcatggacatgacctataccaggcagcagcgaatgcaggtgatgattattaccacccgccccaacaccgtgatcgatagtgttcaaaaccatcttcgtcggggaatcacgatcgttcataatgccgaaggggcttatcaacacgatgccaaaacaatcttgttcacggtcatttcacgatatgaaatgggggagttggaggaagccttattggagtccgatcccaacgcgtttgccagcatttcagattcggtcaagattttggggaggttttacgagccgaaaccctgagggcatttttaaagatttcctaagaaacaagttctccaagtggattatgttataatattttttgtgtgtgatcacaaaatattgaaatacggtgaaaattttgaaagttgtttacttatggttaatcaaattattctcagtcctgaatatttggcggccaaagaacaaagttgtttatgtgatgagctttgatgataatgttgacttcattaagcaattggcacaacgactgcctcagaagtacgttttatatgttctttatcgagccaataccgaagcggctgcgacggatttagcagcctttggtatcaaaacgcggcagtttcgcgatggcattaaattcgtgatggacgatgtttcgcttttgatgtcagcaaagctgattatttgcgataactactacgcttttttgggtggcctggttaagctgccgttcgtcaaaattgtccagatatggcatgctgacggggcgattaagaagtttggctgggaagatccgaccaccgacaaacgcagtcgttctgataagcgccgttttcagaaagtttatgatcactttgatgaatacattgtcgcatcaaaagcaatgggacaggtgtttgtgcacagttatcatgaaaattttgacaagatgcagctgctgggataccccagatccgaccagtatctcagtcaagattggcagcacaaggcccgtgagcgaatttatcgatcagttcctgaactgaaaaatcatcgggtcattttgtatgccccaacttatcgggagcatcaggactttaagctgcccaagggccttggcagtgctttagcagcagatccaactgccttggtggttgtcaaactacacccggttttgcgggataaagaagtgccgatgcgccgcattggtaatcccaagattaagttttatcacgaattggagaccagtgatttattagctgtggctgacacactggtcaccgattattcgtcggtggcatttgattttagcttattgccaaatgccaaatcgatcatcttcttcatgtttgatcttgatcgataccgaagcgatccaggaattcaggatgattttctcgactggctaccggtagagccggtttataaggtcgagcagctcagaaacgaaatcctggcagggacaagcgttaacttcgacaaatttaacgcccattggaacacctataacgacggtcaggcgactgacagagtcattgcgcgttatgtcaaattcttagggtctaattaaggagtgcctcaaattgaaagaagtcagtactttaattaaagaacaatttcaaaatatcggcattatcttccgaatctcaaagtatgaagataaagccgagtatcaaagccattatctgggcctcatttgggaatacttatatccattgattcaaattggtatttattggctggttttcggtatcggcctgaaacacggtaattccactcatggtgtcgattatctggtttggatggttatcggaattacaccttggttctttatgaaccgggccagcctggatgcttccaagagcatctaccaacgggttgggatggtttctaaaatgaaatttcccgtcagtattttgccaaccattaagattgtcagcaacttaagtgccttttggaccatgctggtcttttcaattgtgattggcttcttatatggggtgacgccgtcaatttactggattcagtggatttattacttcatttgtatgattgcctggctgattgcttttggtatttttaattcaacaatttccgtcctggttcgcgattatcggatcttgttgcagtcactcatgcggatgctgttttatatgtcgggcgttctcttcaatttccagacggatgcctttccagcaccgtttgttcatattctgcagttgaatccattcttctacgtcgtttccggtttccgtgacgggatgctgggcagtgcctggttctggcagaaaccaactttgacgattgtcttttggggcatgattctcttcttcttattggttggttctcatctgcattacaaattccgttctcgatttgttgatttaatctagttttgagggtgagcttttgaaacgttcaatgatcaatcttattaaactcatagcccgcattgtactcatcgtgatgaacgatgggtttatttgtatgcccgtcaaaaaggggacggtgttatttgaaagttttaacggcaaagatgtcagtgacaatccatttgctatctacaatcaattaacccaagatgacccgactgcccgaaagcggtgctatttcagtgtcaaacccagtgagtacggcaggctggttaaacagtatccaaatattcaatttgtcaaacggttcacgccgggatgggtgaaatacattgccagggctgattattgggtgatgaattcacggatgccaaagtggtggcgcaaaaataagcgaaccactttcattcaaacctggcatggaacaccgttaaagaagctcggaatcgatattgaaaacgttgagattcccggcagtcagacagctgaataccatcaggaatttattgatgaggctgcccggtgggattatttaattgcgccaaatcaatattcacacgatatttttaaatccgcttttggctattcaggtaaattcttagatattggctatcccagaaacgatattttatatactgaaaataacgctgatgacattcgaaaaatcaagcaaaccctagttggctatcagcctaaacaggtgatgatgtacgcacccacctggcgggatgacgatttttccgagaaagggaaataccaattcacgctgccgtttgatctggcacaattttttgaaaatgtcgatcctcaaacgctactggtcattcggccacattacttggttaaagacaatattgatattagcgggtttgaagaccgggtcaaaattctcgctgatgtcgacattaaccaactatacttaataacagatctactcattactgattattcatcagtgatgtttgattttgccaacctcaagcggccaatgctgttttatccttatgatctggctcattatcgtgatcagctgcggggcttttactttcagtacgatcaagctaatctgccgggaccaatggttgaaaatcaaactgacttttatcaaaagttaagtgaataccgtcaaactggcgcttttactgatttcagtgacaatttgacccgttttaaccaaaaattctgtgcctgggaagatggtcaggcttccaaaaaagtcagtcaattaattttacaagggggatatacaaatgagtgaaacaccatttttaatcggttctcatgtcagtatgaacggcaaggacatgttcctcgggtctgccaaagaggcggcttcctacggtgaaaccgtctttatggtttatactggagcgccgcaaaatacggttcgtaaacccattgagaagttgaatgccgatgccggcaagcagtatatgtccgatcatggcctcaaagcggttgtggtccatgcgccttatatcatcaacctggggaacactttcaaaccggaaaacttcagttttggtgttgattttttgcggcaggaaattcaacgtgcacaagccattggggctaaagaaattgtgctgcatcccggcgctcacgttggtgccggtccgcaaaaagcgatcgatcaaattgccaagggcttaaatgaagtgattgaggagaatcaacacgtccaaattgctttggaaaccatggctggcaaaggtaccgaagttgggacgtcatttgagcagttggctgaaattatcgataaggtcagcgataatgacaaactctccgtgaccttcgacacctgtcataccagcgatgccggttatgatattaaaaatgactttgatggagtcttgaatcaatttgaccacatcatcggccttgaccggctcaaagttattcacctgaacgattccaaaaatccacagggcagccataaagaccgccatcaaattcttgggttggggacaattggctttgataccctgaactatattgcccatcacgcacaattaaaaagcgttcccaaaattatggaaacgccaattttgaaggatcctgacaataaaaacgttaagtggaatcctcatggttatgaagttgcaatgctgaaaaaacagcagtttaatcccaacattattgaagatatgaaagccagaaaaccttactaggcaggccaaatcaatcttcgaattcggtggtatttaaattgaggctttccaagataatggtggccgtttcctcaatggacttgttggccacgttgattgttaaacagccaatttgacgatataattttttcgcgtacgccaattcagttttgatatgggccggatccgagtagggtgtatcagcgtccaggccgtaagaaatcatccgttgtttacggattttgctcagtttctcaggggtgttcagcaggccaaacattttatccttatcgatgtcgttgacttcttcagggagttgcaggtccggcccgattggcagattggcaacccgttgattttggttggccaaataaagcgacagcggcgtctttgacgtcctggaaaccccaagcaacacaatgtcagcttccagcaatcccttgggatttttgccgtcgtcattttctacagcaaattcaatcgcagagatccgttcaaagtaattttgatttaaatcatgaatcaacccaggcacgtgagccggttgttggccagtaacctgactgagcattgccattggcgtttggacgcagtcaaagtcataaatgccattttggcggcagaaatcttgaaccatctggctgagctccgtacttaccagcgtgtgaaaaatcatcgcctgtttgttgagggcaatttttaagatacctttgagaattgagtcggtttgaataaatgggaaccggcgaatttcggctttcacatctggaaattgtgacaaagccgtctgggcaattgtctgggcggtggcgccgcttgaatccgatataataaaaatgttttgagttttcatgataaataactcctaaaattatatttgttaagtaaatattaacatgacacatcaattttatcttaaatcattgacgatgtattgattaatatgtataatttacttcgaaccgttttagaaggcacttaaagtgttgattaaacagttacatttaagctcggagggagggaatttcatatggcaaagacagtcgttcgtaaaaacgagtctcttgatgatgctcttcgacgcttcaaacgtacagtttctaaaagcggtacattacaggaatatcgtaaacgagagttttatgaaaaaccaagtgttaagcgtaaattaaagtctgaagcagcacgtaagcgtaacaacaagaagaaacgtcgtttttaataaatgatgactaaaggtcggagctaatgtttattagtctctgatcttttttaatgttaaaatttaagtattaagcgaaaagaggttactttgatgagtgtatatgataaattgctttctgacatgaaggacgccatgaaggctcgtgataaggtccgcttgggtgtcattcggggcattaaggctcaggtgatgaatgccaaagttgccgatggcaatcatgatttaactgaagatcaaattaacgatatcattatgaaagaaattaagcagcaaaaggaatccttggaagaattccaaaaagctgaccgaaaagatttggcagaagaacaggaagccaaattaaagattgccgaggagtatgcaccaaaacagctttccgaagctgaagttgaaaaaatcgttcaagaaactatttcacaggttggtgctgaatcaatggccgactttggtaaagtgatgggtgccatcatgccaaaggttaaaggtcaagctgacggcagtgttatcaacaaattggttaagcagcagctgcaaagctagtatactttagataaccacaactttgtggtaatatctgaaccaatatgactaataaaaaaggagctcacttacttggctgatactcaacaagttacaagagagtttattgtatccgaccccaacgaattattacaaattgtcgggactcaagacgagttcattacaattatcgaagagggaatggatgtctccatcaatgtctttggtaattcacttcgagtgactggtcaggatgaacccgttagcattaccttacacattttggagaatattctctctttaattcaaaagggaattaatattaacagcagcgacttcatcagtgcgatgaatatggctcaaaacggcacgctggagtactttaaagatttatacaatgaagtgctcatcaaagacgcaaagggcaaggcggtccgcgttaagacctttggacagcggcagtatattcaagcaatcaagcatcatgatgtcgcttttggcattggcccagccggtaccgggaaaacttacttggctgtcgtcatggcaatcgcggctttgaagaagggcactgttgacaaaattgtccttacccgaccagcggttgaagctggtgaaagtttgggctttttgcctggtgacctgaaagaaaaggttgatccttatctgcgtccaatttacgatgccctgcacgccattttgggtgccgagcacactgaacgattgatggaccgggggacgattgaaatcgcgccgctggcttacatgcgtggtcggactttggacaatgcctttgtgatcttggatgaggcgcaaaacaccaccaacatgcagatgaagatgttcttaacccgattgggatttggctcgaagatgatcgttaacggtgatatttcacaaattgatttgccaaagcattcgaccagcggattgattaccgctcaaaagatcttgaaggatattgatcaaattgaatttgtgaccttcacggctaaggatgtcgtccgtcacccagttgttgctaaaatcattaccgcttacgaaaaaagcggcaattaatctcgaatagacttgaggaactaaattaatggatttagaaatttacgataaaactgaaaaaggggtttcggaaaaggatcaaaaattgattcgggatgttttggaatttgccggatcttacattcatttggccgacaataccgaaatgtccgtgaccctggtcaataacgatgagattcaccaaatcaacaagaagtatcggggggttgatcgggcaaccgacgtcattagtttcgccattgaagatgacgatgatgacgatgatttccccattgtgatggatgaagaattgaaagagtcaattcctgaaaatattggtgacatcttcgtttccgttgataaagttgccgaacaggccgattatcttggccactcgtttgaacgggaattggggttcctgtgtgttcacgggttcttacacctgaatggttacgatcatatgaagaaagctgatgcggatgtcatgtttccgcttcaaaaagagattttaaatgcttatggactcaaaagataaccgcaagccacaattggataagaataagtcgtttcttcaatcagtcggccacgctcttgaaggcattaaacgactgctgttggaagagcgaaattttcggattgacttggttgtggcaatcattgtgttaactttcgccattgtcatgaagattagcatcaacgaatggctctggctgttcgcggcttttttctcagtgattgggtcggaagttttaaacaccgttgttgaaaacgttgttgacctcattgttggtcaccactttgacgctttggccaaaagagccaaggatgtagcagctggtggtgtgttactatcagcactgtttgctgtgatcatcgggatgctgatctttgttccgagattcattgcattattaaattaagaggagtaagaaatggataatccagattttcattcaggctttattgccattgttggtcgaccaaacgttggtaaatcaacctttttaaaccgggtcattggtcaaaagattgcgattatgagcgacaagccgcaaacgaccagaaataagattcaaggggtttacacgacgaaagaagctcaaattgtctttattgacacccccggtattcataagccacagaacaaactcggtgatttcatgatggaatcagctttgtctgctttaaaagaggttgacgctgtgctgtttatggtcaacgccactgaacatcgcggtgccggggataatttcattatcgaccagctgaaaaatgttgataagccaatttatctactgatcaacaagattgatgagatttctcccgatgacattatgccgatcattgagcaatacaagaacgctttggaattcaaggatgtttatccaatttcggcgctccagggcaataatgtgcccgaattgatcgacaccttaatcaaagaattgcccaacggacctcaatattatccagctgatgaggtaaccgatcatccggaacgatttgtgatttcagagttgatccgagaaaaagtgctggaactaacccgtcaggaaattcctcattcaactgcggtagtgattgaaagtatcaagacagaggacagccttttgagaattcgggccacaattatcgtcgaacgtgatggccaaaagggaattgtcattggtaaaggcggctcgatgttaaagaaaattgggacgcttgccagaaaagacatcgaaaatatgatgggcaacaaagtctttctcgaactgtgggtcaaagttgaacctcactggcgcgataaggccaacctgctcaattcttacggttaccgcaaagataattattagaggtgaatcagtttgtcaaaaggtcagcgaacggattttaatggcattttgctttatacaaaagcctatcgggaacacgacctgctgataaaatttctcaccagagaattcggcaaaaaaatgttcctggttagaggcgccaaacgcccacggttcaagatgcgttcagcaatcctgccgtttacctacgggctatatggcggtgacattaaggaatcaggattgtcatatatcctcaatgataagcatctcgtccactttcaaaacatcagtgaagacattactaagaatgcttatgccacttatatcatgtcactgattgatttggcctatcccgacggtgagccgattgccacttggtacgacaagctgttgaccggcctgcaactgattgaccagggctttgatgagcaaatcatcacaaatatttttgaggtccaactgctgaatgcttacggcgtcgcaccaaattgggtggattgcacgatctgtcaccggacggatctgccttttgattactctgaggcctacggtgggctgttgtgtcagaatcattggaacaaagatccataccggatgcatttggatgcccgcacaatttactatcttcgactgttttcggtagttgacttatccaaactaacccatatcaaggttaacgatcggaccaaaaaagctttgcgggaagttctcgaccagatttattcaagaagtgtcggtgtcgttccaaaaagtaaacattttattgatcagttgggaaaattcaagttataactgataacggcgttgacaatattttgattgtcaactatgattatttttgaaataaataattcaatgatgacaaaagaaatgacaggatggaccctggtagcgaaatcaggatagtgggagctgattatcgtcggtactgtcaatggcgcttttcgagttgaacaattaagtgctggtagtaataccagaagtagggtggaaccgcgatttcatcgtccctatgttgagtggcttagtctataagtcgttgaacatagggactttttttatgcgtttgaataattaggaggaaaatttatgactgaaaaattatcagttcaagaaattatcctgcggctgcagcaatactggtcagcccagggatgtatgttaatgcaagcttacgataccgaaaagggtgccggaaccatgagcccctatacgttcttacgggcaatcggtccggaaccgtggaatgccgcttatgtggaaccttctcgtcggccggctgacggtcgttatggtgaaaaccccaaccgtttgtatcaacatcatcaattccaggtgatcatgaagccgtctccggaaaacatccaagagttatatctgaacagtttaaaagaattgggaatcaatcccttagagcatgatattcgatttgttgaagacaactgggaaaacccatccatgggttgtgccggtgttggttgggaagtttggctggacggaatggaaatcactcagttcacctatttccaaatcgttggtggtctggaaatggatccggtcgcttcagaaattacttacggattggaacgcctttcttcatacgttcaagacgttaattcggtctttgatctgaactggtctgacgatgttaaatacggtgatattttcaaagagcctgaatatgagcattccaaatacagttttgaagtttccgaccaagagatgttgttgaccctgtttaatgattatgaacgcgaggccaaacgcctgttggaccaagatttggttcacccggcctatgattacatcctcaagtgcagccatacctttaatctactggacgccagaggggctgtttcagttaccgaacgagccggctatctgtccagaattcgcaacttagcccgttcggttgccaaagagtttgtggaagcacgcaaacgactcggcttcccactcattaaagacgaaaagaaacgccaagcactattaaaagacgacaaggaggagaaataatggctaataatttcttattagaaatcggattggaagaaattccggcgcacgtggtcaccccaagcatccagcaactaaagaagcgtgccggtgatttcttgaaggatcaacggatttcatttgctgagattaaaacgttcagtactccccgtcgtttggcactttacattactgatttagctgacaaacagcccgatattgacaaatctgttaagggcccggccaaaaaaattgcccaggatagtgacggtaattggaccaaagcggcgattggcttctcacgcgggcagggtgcaactcctgatgacatcacctttaaggatgttaagggcgttgagtacgtcttcgttgaaaaacacattgccggtaaatcacttaaagaaattttgccggggatgaaggatgtcattaccgccatgactttcccaaccatgatgaaatgggggacgtattcgtttgaatatgtccgcccaatcaaatggctggtggccttgttgaacgataaggtgattcccttcaagattttggatgtcgacacggatcggatgacatctggtcaccgtttcttaggcaaggatattgaacttgccaatgccgacgaatacgaagaaaaactgactgaacagtatgtcgtcaccgacgccgccaaacgcaaggaattaattaccaagcagattatcaagattgctgctgacaacaattggcagatcaatctggatcccgatttattggaagaggttaataacttggttgaatggccaaccgcgttctttggcaactttgatgaaaaataccttgccatccctgatgaagtcctaatcacttccatgaaggatcatcaacgcttcttctacgtgactgatcaagacggcaaacttttgccgcattttatctcagttcgtaacggtaatgattatgatattcaaaatgtggttgccggaaacgaaaaagtcttgactgccagactcgatgatgcaatgttcttctaccaagaagatcaaaagaagtcgattgccgattacgttgagcggttgaagaaagtcagcttccacgataagatttcaacaatgtatgagaagatgcaacgagtccaagtgatttcaaaataccttgggaaccttgctggcctatccgagcaggagctcaaggaccttgagcgggctgcttcgatttacaaatttgatttggttaccggaatggttggtgaatttgcggaactccaaggggtgatgggcgacaaatatgccttgttaaagggtgaagatcaagctgttgccaccgcgatttctgaacattacatgccaatttcggcaaatggtgagctgccaaagaccaacgtcggttcaattttggcgattgctgacaaactggacagtattttgacgttctttgctgccgggatgatcccaagtggctcaaacgatccgtatgctctccgccgccaagcaaccggcgtcgttcgaattgtcgctgacaagcagttaaactttgatttggagcagactttgaatctgttaattgatcgtgaagatcaagcgtcagttgcaccaaaactggatatgaaagcccaagttcctgccgtcagtgacttcgtcaaagaccggatcaaacagtacttggacgacctgggagttcgttacgacattgccgatgcggtgacctctggttcccacaccaatatcctgttcaacattgccagtgccaaaacactccaggatcataaagacgataccgacttcaaggacattatcgaatcgctgacccgagttcagcggattgccaagaagggcgccttcaaggctgatgacttaacggttgatccggcattgtttgaaaatgattccgagaaggctttgaatcaggctgtggcagctgccgccaaggattacactcatcaaagtgccgaagaagactttggtcgtttagctcagctcaaagataaaattaatgattatttcgatgccacgatggtcatggccaaagatgaaaagctgaagaataatcacttgcgccaactcaccatgattgccaacatgattatgtatctcggcgacctcgataaattggttgtcaaaggctaattttgagggctaatatttgtactaattaatgttttatgataatatttaaatacgtatcgccagtaaaacaagtcgcacttttgggtgcggctttttacaggcattgattcagttttgaagatgggaggcgaagtaatggcgaagatcccagaagatgtgattgaagaaatcaggtcacaggttaacattgttgacgttgtctcccagtttgttcaattgaaacagtccggaaagaatttatttggtctttgtccgtttcacgaggagcggaccccatctttttccgtctcggaagataaacagatttttcattgttttagctgtggcaggggcggtaacgtctttaagttcattatggagctgcagaatgtttcctttcctgaggcagttaaaaaggtcgctgagatggaaaatatttctgttgatgagaagtatttccgtgaaagcggcaattcccaatcaagtcccgaaaacacacaacaaaaagcattaattgatctgcacgagcaaagcgtcaagctgtatcatcatattttgaccaataccaagatggggcagccagcgctcgattatctgcataaacgtggtgtgaccgaccagacgattgccacttaccagttgggatatgctccggcacagcggttgctgaagccatttttcgacgagcgcaaagttgattttcaactgctgcgaaaatctggcctgttttctgaagaccaggatggcaatttgcgagaccgtttcgtcgaccgggtgatgtatccgattcgaaatggatccggtcaaacgattgctttttctgggcgattgttaaccactgattccgacatgccgaagtacctgaacagtcctgagactgacattttcaacaaacgaaaagtgttattcaatctagatttggccaggtcaaatattcgtaccggtgagccggcaatcttatttgaaggattcatggatgtcattactgcctttcaagcagggatcaagtccggaatcgcttcgatgggaaccagcttaaccgagcagcagatttatgacatcaaacggattacgcgcgaagttgtgatttcctatgatggtgatacgcctggacaaaaggcgatcaaacgcgccattgattcattcaatgaacagaagagcaatttggtgatgaaaatcatctcgatacctgatggaatggatcctgatgagttcattcgcaaaaaaggtgccgacgattttaaacagttgattgaccatgctcaggctccagttgagtttgaattgaattatctcaaaaaacaatacaatttggattctgagattgaccaaactaattacattgctgaagctttaaagctgattagcagagtggattccggcatttcacgggatctttaccttaaccggttggcggatgaattttcagtggccaagcaattgctgcaacagcagttagcaccattgatcagacaacccgccccggcggctgaaccgcatccataccacaagcaggttcaggtcgttaaacagcaaaagcatttctcgttagttgagaaagccgaaatgcagctgatgaaccgtatgctgcactaccatgatatttggttaaaggtaagtaatgtttcggggttctcatttgttgatgaacagtaccaaatgttgtaccttttagccgaggggtattttaccaaattcgatgattataatgttgccacgttcagcaatctgatttcggaagactcactgcaaagtctattagttgatattgacatgctcgagcttccggataatccgaccaatgctgaaattgatagctatttaaacattttaatgcatcgagccccggtggaagaaaagttaaagaaaaagcgggcagaactcaagcaagccgttaagattggtgatgttgacaagcaacgtgcgttaacgattgagattgttaagcttgaacaacagaagagaatgaagcaacaagtataacttcaggaggcgttttgatggctactaaaaaaaccgacgataaagtaacagaaacaaagactgccacagctaagaaggcaactgcagctaagaaaacgactgcatcaaagaccagtaccaaggccaagtcaaccaaagcgaagacaactaaggccaagacgaccaaaaaagctgacaagccatacaagaaggaatttgacgccattgttaaggctaataagccaattggccatattacctatgacgaattggaaaagaagattgaaaagccttattctctgagtgaaaaggatatggaaggcctcttggagagtatcgaggactccgggatcagtgtcgttgatgaaaacggcgatccggatccgcgagccatcggtgctgccaagaaagtgaccaagaaggaactttctgatgtttccgcgcctactggtgtgaaaatcaacgatcctgtccgaatgtacctgaaagaaattggtcgagtttcacttctgagtgctgaccaggaaatttcattggccaagcgaattgaagccggtgacgaagaagccaagcaggaacttgccgaagccaacttacggttggtggtttcaattgccaagcggtatgttggtcgagggatgcaattccttgatctgattcaggaaggtaacatgggcttgatgaaggccgttgaaaagtttgattaccgtaaaggattcaagttctcgacttacgcaacttggtggattagacaggccatcacccgtgcgattgccgatcaagctcggacaattcgaattccggttcatatggttgaaacgattaacaagttgattcgaattcaacgacaattactccaggatcttggccgtgagccattacctgaagaaattggtgccgagatggacatgccaactgaaaaggttcgagaaattctaaagattgctcaagaaccggtttcccttgaaacaccaattggtgaagaggacgacagtcaccttggtgatttcattgaagatcaggatgcaacttctcctgctgaccatgcggcttatgaattactcaaagaacagctcgagagcgtccttgatacgttaaccgatcgtgaggaaaatgtgttacggttgcgatttggtcttgacgacggtcgtacccgcacgcttgaagaagtgggtaaagtctttggtgtgactcgcgaacgaattcgtcagattgaagccaaggcattaagaaagctgcgtcacccatcacgaagcaagcagcttaaagatttcttagattaatttaatatgatcattcattgagttggggcatttcggtgttccgactttttttgtccgctaaaatggcccttccaagtaaaatgcttctcggaatctgtcattttccattaggataatttataatgaatttatacacaaaatgaggagcaaaatatgaatagcacgcatttatcgaaacgactacaaactgtcagtgaccacgttgaacctggcagccgactggcagatattggctcagatcatgcctacctgccgattcacttggctcaaaatcatgttatcgactatggcgttgtcggcgaggttgccaaagggccgcttgccaacgcgacatcagaaattaccaaggaccatttattggatatccttcatccccgacttgccgatggcttggcagccattgaacccggcgacgacattgatgccatcaccatcgccggcatggggggcaacctgattacccacattttggaagctggtaaagctaaactgaccggaaaagaaaaattgattctccagccaaacgtcggcgaaccggtcgtcagaaactggctgatggccaatcaatatcgaatctttgctgagcagattctaaaagaagacggccatatctatgaaattattacggctaaaaaagctgacaaacccgtcgcttattcaaaattggcccttcagttcggtccatttttgctacaagaaaaatcgccggtgttcgttgaaaaatggcaggaagaaattggcctgctaaagcgggtgattaagaatatgcgtcaggccaccactcccgatacggcaaaaatgacggccattcagtcagaaattaatctaatcaatgaggtgatcaaggttgaaagctaagcagttaattgaaagatttgagcaatttgcccccaaaaaattggcaatggaaaaagatccggtcggcttacaaatcggttcactcaatcaggaaattcacaaagtcatgaccactttggatgttcgcccggaagtcgtcgatgaggcgattgccaaccacgttgactttatttttgctcatcacccggtgatgtttcatccagctcataatcttgatctcgatgacccgcaaaatgcgatgtacgctaaaataattgccaaccacatcacggtttacgctgcccacactaatttggacgctgctgacggtgggatgaacgattggctcgcagaagcacttcagttaaccaatctaagtgggatggtcccagcctatgatgaatcggtctttcgattaaccgtgcaggtgcctaaagtctatgcgacggctgttcgaatgtcacttgtcgatgccggtgcgcaggccagtgctgctcagtacagtggatatacctacgaaattgacgggacagtctactatgttcccaaggccggcgccgatccaactatggggactgccggtgaaccaaatgaaatcgaagactcgcgcttggaatttgaagttcccgaaagaaatcttcatcaggttctgaagactttgtcagatgttcatccgctggaaaagccactttacaatttgattcgcctggaagacaaaaagcatcactttacgatgggtcgaatcggtgatttgccgcacagcatgtctgtccgtgaactggctgaagactgtaagcagacctttggtgtttccggccttcgggtaatcgctcacgacatggctcagccgatcaaacgagttgccattcttggtggcgatggcggcaagttcttccacttagctcagcagaagggcgccgacgcatatgtcaccggggatgtttattatcataccggccacgacatgctggctgccgatttcccggtggtcgaccctggccaccacattgaaagtatttgtattcccaaattggccgagctgttcaaacagtggtccgaccagtatcactggcagctggctatttatcagtcaactatcaataccgatccattcacatttatgtagataaaaggagataactgtcatggcaaaatacgccgaattaattcccaactttttaacgtttgtaaagattaatacccgttctgatcctcaatcaacgagcattccgtcctctgatagagagacacggtttttgaatcaactgaaggatcgtctgactaaaatgggcttaaaagacgttcacaccaacgagcaaagtgcctatgtctttgccacgcttcctggaaacgtcgacaaatccgttccaaccgttggcttcatttcacatattgatacggctgattttaatgctgaaaatattcaaccacaaattgttgagaattatgatggccattctgtcattaaacttgatgagaagggtgaatatacgctggaccccaaagtctttcccagtttgaagaagtatgcaggccaaaccctgattactacggatgggtcaacgttgttgggagctgacgacaaagccggcgtagcagagatcattgctgcaatcacctatttacaagcccatcccgaagtcaaacatggtgacattaagattgcttttggtccggatgaagaaattggtaccggcgccgaccattttgacgttaaagatttcggcgcggatgttgcttacaccgtcgatggcggcccacttggggatttgaattacgaaacctttaatgctgccgatgcaaaagtcgtgatcaaaggaaccgatgttcatccagctgaggccaagggtattatggtcaatgccatccaagttggaatggatttccacgccgccttacctgactttgaccgtcctgaaaagacccaggatcgggagggattcttccatctgtatgatttccagggaaccgtcgaccacaccgaaatgggctacatcatccgtgaccatgaccgagatcgctttgaagctcgaaaacgactcttcaaggggattgccaaccaaatgaacagtgactttggtgaagaccgggttaaggtgaccatcaaggaccagtattacaacatgggagaaattatcaaaaaggatccgacaccggtaaaaattgctgaacaggcgatgaaaaacgttgacgttacaccgcatgttttcccggttcgtggcggaacggacgggtctaagatttcttacatgggactgccgacgccgaacattttcgctggcggtgagaatatgcatggccgttttgaatatgtttctgagcaaaccatggaaaaagcggttgacgtggtactggaaatcgccaaattatacgctgaaaagtaataggtcaaaaaaggtcaaattattgttcagggcattcaaaatttgatagtatagcgttagtggtttggaatgaaaagaatgatttttgtttcgaacctttttattagaacgaattcttgaaaaaatcgtcaactaaaatacattaataaggtgataatttaatgaatcctgataatttaacggaagccgtcacgcaggcaatttctcaggcccaacagattgcggctactcgaaagcagcaaaacattaccgtggcccatttattcaaattcttggttcaacccggcgagttggcccgagagatttattctcaactcggattgaatttgggggatctgaatgatgaactggatgctgaaattgatgccatcgcgacggttgaaggcagcaacattaattatggtcagtcactctcttccaatttgtacgaactgttgcagaatgctgaacagattaaaaatgaatttggcgatacctacatcgctgttgacactttaacgattgctgtgatgcagttacacggtgacaaatttgccgattatctttctcaacagggtattaccgagcaaaaggtgcgcaacgttgtggaaaaaattcgtggcggccaaaaggtgacgaccaagaatcaagaggacagttatcaatcacttgaaaaatatgggaccgatttagttcaggctgcccgggacaataagctcggtccaattatcggccgggacgaggaaattctcgatgtgattcggattctttctcgaaagactaagaataacccggtcctgatcggcgctcccggtgtcggcaaaacggcggtcgttgaaggcttggcaatgcgaattgcctctaatgacgtgccggaaaacctgaaaaacaaaaccatttttcaattggatatgggatcattaatcgccggcgccaagtaccggggcgagtttgaagagcgattgcaggcggtgttaaaagaggtcaaaaaagccgagggccaaatcatcatgttcatcgatgagattcataacatcgtcggtgctggtaaagctgaggggagcatggatgccggcaatatcctaaagccgatgttagctcgtggcgaattgcatttaattggggccaccacgattgacgaataccggaagtacatggaaaaagacaaggctcttgagcgtcgtttccaacgggtcatggtccacgaaccctccgttgaagatacggtgacaattctgcgtggcttgtccgaaagtttggaaattcaccacggcgtcagaatccatgacaacgcgttggtggctgctgccaaactatccgaccgttatattaccgatcgctatttgccggataaagctattgatttggttgacgaagcctcggctgaaattcgggtcgaaatgaattccagtccaactgaacttgaccaatccaagcgccagatgatgcgcctggaagtcgaagaagctgctctcaagcaggaaaccgatgaagcatccaagaagcggcttaaagaagtcgaagaagaactggccaatattaaggaaaaagtcaaccagttaaatgcccgttggtcgcaggaaaaagaagctattaagaaaatttccgacaaaaagaaacaactcgatcaggccaagaatgaattgaaacaggcggaaaacacctatgatttgaatcaggctgccgtgttgcagcacggaacgattccccagttggaagccgatttgaagaagcttgaagataacgatcagcattccgattggctggtcagtgaatcggttacagccaatgaaattgcggcggtagtgagccgagagaccggcattccggtcaccaaattagttgagggtgaacgaaagaaattgctgcacttggcagacaatctgcacaaacgggtaattggccaagatgcggcggtcacagctgtctcagatgccgttattcgctcacgtgccggccttcaagacccaagcaagccactgggttcattcttgttcctggggcctactggagtcgggaagaccgagttagccaaggctttagccgaagacttgtttgattcggaaaatcacatggttcgaatcgatatgtctgagtacatggaaaaagaatcggtttcccgactggtcggcgctgctccggggtacgtcggctatgaagaaggcggtcagttaactgaagccgtgcggcgcaatccatacacgattgtcttatttgacgaaattgaaaaggcacatccggatgtctttaatattttgctgcaggtcttggatgacggccgtttgacggatagtcagggacggacgatcgattttaaaaacaccattttaatcatgacttctaacttaggttcagacattttgcttgaaggcaccgatgagaacggggttatttcacaaaaagcccaacagcaggttaaccaattattaaaagcttcgttcaaaccggaatttctgaatcgaatcgatgatgtgatcacctttacaccgttgacgaaggccgatattgaacagattgtccagaagctgattaatcagttatctggccgtaccaaggctcaagacatcaaattgtcaatttctgacgaggctaaacgctggattgccaataacggctatgaaccgcaatatggggctcgaccgcttcagcgttatgtgaccaacgtcgtggaaactccgctggcacgaatgatcgtggctgatcagatcaagcctcacagcgttgttcacattaaccttgataacgatcagttaagctttgttcctgaacaattacctgctgacgaacagatttaaaccaagctacctggggaggaattcggtgtgccgattaattaccagcttccaactgaaaatcaaactcaattagcggtggcgtattttcccgctgatcatccaaagggaattgtccaacttattcatggcgccttggagcataaggaacggtattatgaattttgccggtttttgagtgaccatggctatgttgcggtgatctcagataatcgcggccacggccaatcagtttccgacgatgacccttgggggatgatgcgcagtctgccgcaattgatccatgatcagctgttggttacccaatccatcaaagcccggtatcccaatttgccagtcagtctgtttggtcattcttttggatctatcttggcgagattgtatttacagcaccacgaccaggaagtcaatgcggttgcgttaaccgggaccaccaactatattccggtggtgccgcttggcttattcattggttgggtctttttgaaatgccattctgaagatgctaaatggtccttgctatctaaaatttccggtctaactccgggggatcattcctggttgagctataatcaggcaaacattcaccgggtcagtacagatccgttaatgatggatgaatatccggttaaaagtttggtaacactgtggcagggcgattattccctgaaacgccttcaaaaatttgactgtcacaatccacaactgccaattctgagtttggtcggcagtgaagataagttcagtggtggtcagaagggcttggcagacacggttgcaacgctgcatgagatcggctatcgaaatgtagtcagtcttcaagagccgcatatgaagcatgaggttcttcaagaaacgcatcgggaagttgtttttgaacgtctgctgcagttctttgacacacaccagtaaagttgattgagacaacaaaaaggctatggcaaaatctgccatagccttttaacgtttcgaaaaactattcttttgatttacttgatgttgcagaatccttgctgatcagatagataccgtttacggcaataaatgcagtaattgcggcagcaattccgatttgggaaggatcccatgttcgaacttcgagggcggaacctatgtaaccaatgatttctccaaagatgtatgcccacaaaacagctacaatatttgaactaataagtttcatgtctaatgccacctcacaatcaatagcattttagcatatattttgtgaaaaatcatcatttatttaatttgccaatttgaatgtgggcttgatatatttggtataattttaattaagaaagaagggcaatcctgtgagttatgttccgttgcaagtcataagttcatacagtttactgcagagtccgattcgcattgcggacttgattgctgaagccaaggatcgcggttatcaggcgttagcgttaactgacctcaacgtgatgtacggggccgtggaattctacgacgcttgtttaaaggctggcgttaagccgctgatcggtctgactttgcagctgaccggcttgattttgaccgataaagaatatgggtgggtgctgattgccaaaaaccagcaaggatatgccaatcttctcaaattatcaacattgaagatgaccatacccgaattgacagcttctcagttaggtgactatttaagtgatttagttctgattttgccgccggcagcagaaatgaatgacctgcttctacaagggcgggctgatgacgctgctgatttgattgatcaggtcaaatcccttggcgtcgatcctaatgcccttaaaatcggtgtcgactaccattcctctgacagcttaaatgacatgttaagtaagctggcggctgacaagcaagttgctttggtggcggattcgccagttgaatacttaaacgccaccgactatttttccatgcaggttctaaaaaatatcggcgcgggagaaaaaatcgccaacgtggcccaactcagtaagcaagtggggccctattggctgcgtccggccacacaaattgaggctcaataccgtcagattcacctcgctgacgcactgacgcaagtcgaccaaattgtcgctgattgcaatgtcgagattaagaaacagcagcccaaattgccgcaattcgacacaccaaacggtatcgattccggaacttacctgcgccagctttgcgaaacgggattggcggatcgattaaagaaaaatcagattaaagatgcgaccccttatcatcgccggctggatcaggagttatcagtgattcattcgatgggctttgataattactttttgattgtttgggatgtgattaatttcgctcaccagactcacatcattaccggcccggggcgtgggtcggccgctggatcattagtagcgtataccttaacgattaccgacgtcgatccaattaaatatgatttgctgtttgaacgtttcttgaatcctgaacgggttcagatgccggatattgatttggatattccagacgacaaacgcgatgaagtcatccaatatgtccatcaaaaatacggtcacaaacgggttgcccaaatcatcacatttggcactttggcagcgaagcaatcgatcagagatgtcggccgggtgtttggcttgaatactgcccagcaagatcagtggagtaaggccattcccaacgcatttcacgtgaccctcaaggatgctttggccaattcccagcgactgaagaatctggtggctgacagtccgcttaatgaagcactctaccaaaccgcccagacgctggaaggcttgccaagacactattcgacccacgcagccggactggtattaagcgacgatcccctggtgaatttagtgccgcttcaaaatggcaacgaagggctgttgatgactcaatattccaaagattatgttgaatcggttggtttgttgaaaatggattttctgggactccggaatctgtcaattttggctgatgcactacaacaggttcaactaaccaccggaaaggttctggacatttctgctgtgcccttggatgacgccaagacgattcagttattcgccaacggtgacacgactggcattttccaatttgagtccaacggcattcgaaatgtccttaggcgcctgcatcccgaacggttcgaagacattgccctggtcaacgcgctttatcgaccgggacccatgcagaacattgatgaggtggttaagcgaaaaaccaatcatgaagcgttaacctaccccgacgactcgctcaaagatattctccagccgacttatggcgtaattgtctatcaggagcaagtgatgctggtagcttccaaaatggccggtttttctctgggtcaagcagatattttacggcgggcgatgagtaagaaaaagcttggcgtgatggaacaaatgaaggctcagttcatcaccggcgccaaacagcggggatattcagattcagtcgccaataaggtctttgactatatcgagcggtttgccaattacggcttcaacaaatcccatgcggtcgcctatagcaagatggcttatgaattagcctacttgaaagtttattacccgggcgaatttcacgttgcgctgttaaattcggtcaacaataattcggttaaggtcaaagaatacctccaagctgccaaatcaatgggggtcaaggttgttggcccaaatattaatcatagtgaagcccggtttacctttcaagatcaacaaattgtgtttggccttgattcaatcaaaggcgtgcgtcacgacatggtagtggatttattggctgagcgacaacaaaacgggccatttaagtcgtttccggactttttaagccgcctgcccggcaagtaccgcaaagttgaattgatcaatgccttgatttatgccggcgcattggatgtttttccatttaaccgttccgaattaatcgctgccgcccctgaatttatcagctccgttgaattaagtggcaattcgatgagcttgttcaaagcgttggaacccaaaatgccaaagatgcctgagatgcctctgatggacaagctggaaaaagaaaatgcttatttaggggcctatttgtctggtcatccgacagaacgatttgcccccttggaacagcgattaaatgctgagacaaccgctacgttgagtgccggtatgaaaaatatttacttgattctctacattaccaaggttaagattatccggaccaaaaccggcaaacaaatggcctttttagacggtaatgatcaggtggggcagacttcggtgactgtctttcccaacttatttgccaagacccagtcatggcttcataaagacttggtgattttgatcaaaggcaacgtcgagaaagtcaacgatcttcaggtggtcgccaatgacatccagccggcggctaacgccctgatgaacctcaagcgatcaaaacagcaatctaaatggtatttgcgaattgatcgcgatcatgacaaaaatacaatgtttcacaaactggccgacctgagcagccaatatcacggccaggtcccggtcatcgtttttgaaacagaaaccaaaaaaacttggcagctcgaggacaagctgtggctaaatccaagttctgaaaccaaagagcaattaatcacaatctttggcaggaataatgtggtttataagtaaatttttggaataatttttcagaagtcaggttcattacgtaaaggctttcatttgcggtagacctaacttttgccattccaagtcggtgctggaaagcccgcttacccccaaaaggtgggcgacaacccgcttaaaaagtgataaaatacgattgaaatctaaaaggataccgatgcgttatttaaattgttttgcgacattttaataaggtgttgcgtgcccaaaaaccgaaggagagattttacttatgaagaaaactaagatcgtaagtacattaggcccagcaagtactgatgtagacacaattactaagctgattgaagctggagctaatgttttccgatttaacttttcacatggtgaccaccctgaacatcttgatcgtatgaacaaggttcacgaagctgaaaagaagactggcaagactgttggaattatgcttgataccaaaggtgctgaaattcggacaactgttcaaaaagacggcaagatcgaattccacactggcgatgttttccgtatttcaatggacgcaagtcttgagggtactaaagacaagatcgcggttacttaccctggactctttgacgatgttcacgaaggcggccatgttcttttcgatgatggtttgttggacactgttgtcactaaaaaagacgatgctaacaaagaattagttgtcactgttcaaaacgacagcacccttggttcccgtaaaggtgttaacgcacccggcgtttcaatcaacctgcctggtatcactgaaaaagattcagatgatattcgttttggtttggacaatgacattgacttcatttctgcttcattcgttcgtaaagcccaagatgttttggacatccgtgaactgcttgaagaaaaacacatggaacatgttcaaatcttccctaagattgaatcgcaagaaggtatcaacaactttgacgatatcatcaaggtatctgatggtttaatggttgcccgtggtgatatgggtgttgaaattccagcagaaaacgttccgttggttcaaaagactttgatcaagaaatgtaaccaacttggcaagccggttattaccgctactcaaatgcttgattcaatgcaggaaaacccacgtcctactcgtgccgaagcttccgatgttgccaacgccgtctttgatggtactgatgcaaccatgctttctggtgaaagtgctaatggtgattaccctgttgaatcagttcaaacgatggctcgtatcgacgttaaggctgaaaatgctttcagcgaatttggtaccccacgtccagaatttgactcaagcgatgttactgaatcaattggtgactcagttgcccgtgttgccaaagaattaggcgttcactgcatcgttgcagctacccgttctggttacactgcacgaatgatctccaagtatcatccagatgctgacatcctggccattacttttgacgaacgtactcgtcgcggtttgatggttaactggggtgttcacccaatcttggttgacgaagttaagagcactgatgaaatctttgaactagcttcaaagaaggctctcgaaactggtttagctaaggaaggcgatttgattatcgtcactgccggagttcctgttggtgagagtggtaccaccaacttgatgagaatccaactgatcggttcaaagctggttcaaggtcaaggagttggtgacaagactgttattggtaaagcggttgttgctaaaaacgctgctgatgccaagagcaaagtaactgaaggcagtatcttggttactaagtcaactgacaaagaatacttaccagctattgaaaaggcaagtgccgtagttgttgaaaccggcggcttgacttcacacgcagctgttgttggtatttcaatgggaatccccgttgttgttggtgcagctgatgctaccagcaagatttctgacggtgaattgattaccgttgattcacatcgtggcgttatttaccatggtgcttcatcatcaatctaaatttaacttgtgagtaatcacaattaatcatgacaggtccgggcggttaatccgttcggacctgtttcctgttatgataagggcggtcgaattttcactgaaaaacgtgtaaaataagattaagctcgattagatcggagataagcatgaataatattattgcgcaagttgtaaccggtaaggtcatcgatgaaaatgacaaggactattacgttcagattgaaggagaaacatttctccttgataagactgagctcaagaaacccttgcgaatcggtgcatctttcactggttttacgtatgaaaatgaacagcataaaatgcaaataaccagaaacattccggatatccgtcgtgatcattacggttttgcgaccgttgtgaaggaaaaatttggtttaggggtctttgtcgacattggcttacccaataaagacgtcgttgtctcaattgatgaactgccgacggtccggtcattgtggccgcaagacggtgatcaactgctgattgatttgacggtggataacaaaaaccgaatttggggtcacttagccgacgaagaaatttttgcggcaattgccaagccggccaaggatgatctgcagaacaaaaatcttaaggctcgggcttatcgtcttaagatttctggaacccggttgttgaccgaggattacaatttggcttttctgcatcctgacgaacgactcatggagccacgtttgggacaggaagttgaagccagagtgattggcatgcttcgggatggcagtgtcaatatttccaccaagccacgggcttaccaagaaattggtgaagacgctcagatgattttggcggccattgaacataccgacgacaaacaactggcgttcagtgataaaagtacgccggattccatcaaagattactttggtatcagtaaaggcgcattcaaacgggcgttgggacatctgctgaaggaaaacctgatcgaacaagctgatggccacatttccttgaaaaagtaggcttttatgatgcacgaacaaattgaggactatcttcattatttacgggtcgaacgcggcctttcagataatacgattaaaagttatcggcaggatctgcaggaggccggtgctttttttgacaaacacgccaaatcaattgccgacattgaccaatttgtcatcttggattatttagaaactcttcaacggcagcataaagcccggaacacggttatcagggtggtctcgacattacggcggttcttccagtacttggttcaattccacgtgattgttgacgatccgatgctcaaggttgattcgcctaaaaaggcccagacactgccggacgttttaactgtggcccaagttaatcagttactatcgatgccggatactcataaaaaattaggtctgcgcgatcgcgcaatcctagagacgctgtatgccaccggcctgcgggtcagtgaactggttaacttgaagttgggtgacctgcatttgccgatgaacttgctgcagacaattgggaagggcgacaaagagcggatcattcccatcagcgacgtggcaatcgactggttgaatcaatacatccaatcgacgcgagtccaactactttcgggaaggcccaactccgagttcctatttttaaatgcccacggtcaccaactgacccgccaggcaatctggcagatgattaaaaaatatgtcaaccaggccggcatcaaacgccatgtcacaccacatacactgcggcattcatttgcgacccacctgcttgaaaacggggccgacttaagaatcgttcaggaactgttggggcattccgatatttcgacgactcaaatctacacccacgtttctcataagcatttaacggaagtttataataaatatcatccgcgagcataacgaaagaggttgaataaatgttatatcaataccgaaaagattatgaaaagatcacgatgggcctcttttcgttggtttccgagctgcagaatatggacttggttgcccaagaaatgagctggtacgccgccaaagacgaccgattgatttatttgtggcgggacccatccaataattggtcgggtttagtcggcattgaacttcaaggaaatcagctgttggttcatcaattggtgttaaccccgcaaagcgtcagtcaggggaactataaccggatttttgacgacctccaggatttatatccaaaatatcaaattgtggtcggctttgaaaatcgagccgcctgggaaaaatgggagaatgcgattaatcatgcctgaagtcaagcagccggaattacatttgaatgattttgacgggccactggaagtcctccttcatttgattcaggaatccaagatggatatttatgatattcagatttcaagaattaccgagcaatacatgcagtatatctatgatgcccagcaattaaatttggaaattgtcggcgaatactttgtgatggctgccaaactgatggtcatcaagtcaaagatgctgctgccgacgattactgacgatcaaccggatgaacagcaggccgacccccgtgaggaattagtgtcccagttgctgaattataagcggtacaaactggtggctgccagtatgaaaaagcgggaaatgaaacggcgggagagttttacccgctccgagttgagcgtggcgccaaccaaggccgaactgattcagccatctccgttcaacagcggcgacatcatggccagctacgtggatgctttgaaacacttcaagtataatcaacccatgtcgacggtaattcacgagtggtcctttacgattgaaggccagagtcaacgggtgcgcgagctgttaaaccaaactgataaccggatttccttcgataaattggttgccaattcaactcaaaccgaagaggtcgttaccgattttctagcaattttggaaatggccaagtataacgaagtccggctcaaccaagcaaccgtacagtcgaccattgaaattcgaaaggggcctggatacgttgatcagtaatctggcaaaaattgaagcactgctttacgcctctggtgaccaaggcatcacgttgcggcaaatgtcccagcggacggcgttaacggtggccgcctgccggcaattgttggaaaaaattgtccaaaaatatagccaagatcaagatagcggcttaaaggtgtttgtcagcgacaacgtctatcggctgggaaccaaggaagaattgtctgaattagtgggcgattatgtcaacgatgccaaaccgcgggttctgtcggaagcggcattggaaaccatttcaattatcatgtataaccaaccgattaccagaattgaaattgatcagatcagaggggtcaatagttcggcgattctccaccggctggtcaaccaggatttgatcgaagtgactggggtcaaagaagaggtcggcaaccccaagcaatacgggatcaccaattttggcctggattattttgggttgaagtcgttgaaagacttgccgccattgccaaaggatgaagtcttggatgatgacaccagtgattcactattaacccgttttaacaaagaaattgataaagaaaattaggaggtggatgtatgaatgaagaacgtttacaaaaagtgattgcacacgcgggagttgcgtcccgacggaaggctgaagaattgattgccaaaggacacgttaaggtcaatggcgaggtagttaaagaactgggaaccaaagtcaccccaaacgatgaggtgaaagtcgacgaagtgccgatttcaaaagaagccccagtctattacctgctttacaagcccagaggggtcatcaccgcggtgaccgatgacaagcaccgaaagaccgtggttgatattttagaagaggtccccgaacgaatttatccggtcggccgcttggactatgacacgtctggcctgttattattgaccaacgatggcgacctggacaacaaattaacccacccaaagtacgaggttgaaaaaacctatgtcgccaaggtcaagggaattgtgaccaatgacgacctcaaacacttgcggactggcgtcgtaattgagcatcgaaaaacggccaaggccaagaccaagctgattcgcaccaacaaggactcgtcgattgtccaattgacgattcatgagggtcggaatcaccaagtcaaaaacatgtttgaaaaaattggtcacccagttgaaaaattaagccgggaaacctatggctttttgacattgaaaggcttgcagccgggggattatcggccgttgaaaccacatgaagtcgaagaattaaaggaattgacgggcaagacaaatcgttgacatttgccttggttctgctatatttgaattaaataaattggtttatcttcagggcagggtgtgattcccgaccggcggtgatagtccgcgactcacgagtgatcgtgctgagctggtgaaattccagtgccgacagtaaagtctggtatgtagaagattaaattttacattttttgtaatgccctgacaaattctttttgtcagggcattattttgaagattgaccattggaggagaggttttttcaatggaaaatagtggtaagcatacgcagtttgcaacaacgcgtctggttgagatgtccgtgtttgccggactctcatatgttttgatgtttttgtcggtgccgattattccaatcgtgccttacatgcgcttggatttggcagacatgccgattttactgggaaccgtcttatttggaccggttggcggcatgacgattgctggtttgaaggccttgctttactgggtaacgactggcgccgatgtgattaacttcattggcgtgggttcatccctggtttcatctttggtgctcatatgggcatactacttggctgaccggcttttctcattcaccaaggggtggaagaaagcaggactggtaattttgaccatggcgattgccttgacaattatcatgtcattgaccaactggctgggagttattccgctatacatgaacctgattggcatgaaattaggctttccactggcaaccgtcattttgtctggggttgtaccgtttaacttcatcaagggaattgtcgtcggtggtgttttctacctaatcaagaacagtttcctgccacgcttaaaactccggtaaatgtggatagatccattcaaaatttgtttgatatagtataattgaacagtgagtaatcttagaggctgggacaaacttgcgggtttggactggctttttgtttcggaggtagttcatggacttaggcattctcatgttaatttttggtagtgatcggcagtttcggcgggtgaaggcgattaaaaacaccttacgggggcgccgcactgtttccaatttatactgggcactggaatatgggatgcttgattttatcgacgttctccacggtgccgactttggtgaggaccagccagtcttgacccagttgtctgccaacgggttggctcaagccgatgatgacttcagaatccaactgactgcaaagggggtcgaacagcagcgagcttatttgaatcagctgctgcctctcaaacacctggcagtttcgtcgcgctatgatgtggccaagttcatgcggcggttcagttttgccacccagattgtttcagaattcagctacggtaacaatcaatactatccccagtcaattaattattttgaagatcagctgttaaaacgctggtttattgatcataagcaggaccatctaccggaacatttccgccaattgttaaacagctttttgagtgacctccaccaggatgaactggctgatctcttcgttcaaagcctggttggacatgacttctcaggattgacagctgagcaggtggcagtcaaacgccacgtgccgaccacaattatcgaactgcagtggctgcagttgtatgggatgctcctggaaaaagtcatgcgcgcaggaaagacgagtttatttgcaccattgactgccggattggccaaaccaattatctccaacagtgctcaaaccacctttaagatgtttgtccggcaagcggatcgaaatccccacgccatcgcaactcagcgtcacatcaagctgacaacggtttatgaacatctcttggaggcagctatcctgaccccggtggcgaagtttccatataggaccctgatttcagaagatttgatgaatcaactagcagctcatcagccaacaaacgtgggcgagtggtctttccaagatgccagtcaggtggttaatcaattggcatttttccaatttcgactttttcagatatacaggagtaaaacgacagatggtcattgatctcaaacgtgaattaaaaaaatattttggctttgacaccttccggccgggccaagaaaaaatcttacagaatctgttggcccatcaggacaccttggcgattctgccgacaggcggcggcaaaactttactttatcagatgtatggggcaatcacccgccaacgggtcatgattgtgtcaccgctgatttctctgatgcaggatcaggtcagtcgactgcaatttctgggatccaaacgggtggttgcgttgacttccgcgttagattttcaagagaaaatggcgattttaaatcatttgaatcgttaccagtttatttatgtttctccggaaatgctggcaaatgaccaggttcaacaacggttgaagcggctgagcatcggcctgtttgttgttgacgaagcccactgcatttctgaatgggggcccgattttcgcccggattacctcaaattagggacggtgcgggagatgctggggcggccactgacgttaatgatgacagccactgctacccaaccggttcggcgagatattattcggcatatgaattttcgattcgaggacgttcaccaaattgtcttgccggtcaatcgggccaatatatttttaagtgcaaaaatttttgccaatcaacatgataaagacgctgctctgattgaactggtcaagcagctcaatggacctggaatcatttatttttccagtaagagtaaagccgagcaggctgccaacacgttgacgaatgaaaccaatcgccgggtgatggcctaccatggggggatggacagtcagccgcggtttcacattcaacagcagtttttggcagggaatttggacattgtctgtgccaccagtgcctttggaatgggcattgacaaggataacatccgctttgtcattcattaccacctgccggcgaacattcaaagttatgtccaagaaattggtcgttgcgggagagatcagcagccggggttggcgattttgatgtatgaacccaatgaccgcggcttacaaatgggtctgatcgatcatacgatcccggatgaaagcctattgcgttatttgtatcagcatcctaaggcattagccaccgatgatcagtttcgggtggtcaaatattaccacgacagcggcgactcgtttgagcaggccaaatcgatctttgatcctgctcgtactcggcgggtgaaggaactgggggcgatggtccaatacgtctacacggaaaaatgccgtcgtgatgaactgctgaagtattttgatgaaacagtcccggatggcgaacgaaacccggcattttgctgcgatcacgatgtcgatttttggaatcgctggcaggattttaaccggcaatatttgattcaaccggaaaaatcaggtcaaaacgaaaccaaaggctggcagcaagtcatcgaccagctgtttttatcaaaaaattaaggtaaatttaagtgaattaatgataaaataagtttgtctatatcctgatcaagaggggggtcaatatgaattcgaatgatgaacataaaaaaactgatgaagatcagccctggaatcaaacattttctgaggatcgtgatgaaaacggtaatctctcgcgagtcaagcttcgaaagcagagccaaaaccaccatctgattacgatggttttagcggcgttaatcattatcgtggcggtggttgcgctggtttacggcctggttcgccaaagtgcgatgggcaatgattcaaagagtgccgcgtcttcgtctgtcagggtcgtccgacaggataacgcaaaaaaaaatcttcttcagcggccaaagccaaatcgaattcaactaaagccaagccagctgtaaagaaagagcagccaaagtcggccagtaaagccgcttcaacccaaccgaaagcctcgagctcgacatcgtctgcttccactgtgcaatctagtaacgcccagtcagcatccagcagttcaacgactaacaagacgactgctgccagcggccatcaatacgccactgtcaaggccggccaggggatgtttcgggttgcttataataacggtttgaccactgaacagctgatgcggatgaacgggctgaatgccaattccaagctgtatccggggcaacggcttcgggtgcggtagctttaaagaatcactcaaaaataatgtcaggtaaggaatgttagaatgcgaaaaaatggattacaagtagcaattgatggaccggcctctgctggtaaaagtactgtcgccaagcgggtagcaaagcaatttcactatatctactgcgataccggtgccatgtatcgggcaattacactgcaggcaattcgtcagggcgtctcctttgacgacgttgacgagatcggcaaaattgtccatgcctcaaaaattacttttgagcccagtgatgacggacaaaaggtcttcattgacggcaaagaaatcaccgaggcgattcggcaagaagatgtcactaattcagtttcggcagtcgctgccattggcgaagttcgaaagcaactcagtgctcaacagcaggaaattgctaaagacggtggcatcgtcatggacggaagagatattgggacggccgttttacctgacgccgaagttaaaatcttcctgattgccagtgttgcggaacgagcgcagcgccgatacaaagaaaacattcaaaaaggcattaatacacctttggatgaactacaattggaaattgaggccagagattataaagattctcatagaaagatttcaccactaaccaaagcaaaagatgctgtagaaattgatacaacgtcactttctatcgatcaggtggtttcaaagattgcagatgtgataaataaaacactgaaataacaactaattagtcaattgactggtaatattgttcaatttaagataaaattatgattagagttgtttcaaggaggaattgtttgatgagtgaaaatgcaaataatgataaaaatgatttattaaacgctttaaacagcgttaatgaagtaaaggttggcgatgttgtcaccggtgaagtattggccaaagatgacagtcaacaattaatcgtgggtattgaaggctccggtgttgaaggcgttgttcccccacgtgaactttcgtctgaccaaaatgttgacgatatcaagcagggtgacaagctcaaattggttgttacttctcgaatcggcagcgacaaggaaggcggcagtttcctgctttcttcaaagcgtttggaaacccgcaaagtttgggatgaattggctgaaaagtcaaagaatgatgaaacgattactgccaaagtcagccaagctgttaaaggcggcttggttgttgatgccggtgtccgtggattcgtgccagcttcaatgatttctgaccattacgttgatgatttaaaccaattcaagggtcaagaacttgaattgaagattattgaaattgatccagttgaaaatcgcctgatcttgtctcacaaggctattgttcaagctgaaaaagctgaagaacgtgaaaagttaatgcaaactcttcacgaaggtgacgttgttgaaggaaccgttgctcgtcttaccaacttcggtgctttcgtagatctcggcggcatggacggattggttcatgtttctcaaattgcttacgaacgtgttgacaagccttcagatgtattaaaggttggccaaacagttaaagttaaggtattatccgttgacttcgaccgtaaccgaatctcactttcaatcaaacaaactcttccagaaccttgggacggaatcgaagaaaaagctccagttggcagtgttcttgaaggaacagttaagcgcctggttgatttcggtgcctttgttgaagtgttcccaggtgttgagggattagttcacatttcccaaattgcccatgagcacattgatacacctgctgatgttttgaaggttggcgagaagattaaggttaaggttcttgatgttgacactgaccgaaagcgtttggcattatcaatcaaagctttgaccgatgctcctgaagaagaagccaagccaaagaagtcaaacaaccgaccatcacgctcacggaagtctaacgaccgttccatcagtaatgcaccggaagaagaaaccggctttactttgggcgatatcattggagacgaattgaagaagtccggcaacaatgatgacgatgataacaaataatcaattattttaatcatgaaaaggggctggaaacaaaacgcaagttttgtcccagctcctttctttctgaattaaccaagcaaaggagggatttacatggcattgccaacagtggcttttattggccgcccaaacgtggggaaatcgactatctttaaccgcattgccggtgatcgaatttcaatcgttgaagataccccaggtgttacccgggaccgtatttattctcatggtgaatggctggcaactaaatttgcaatgatcgatactggtggaattcaaatcagtgatgcaccatttgcaacccagattaagagtcaggccgaaattgccatcgacgaagcggacgtgattgtctttatcgtcagcggtaaggaaggggttaccgcagaagatgaacaagtcgccaaaattctttatcgaagtgataaaccggttgttttagcggttaacaaggtcgataatcctgagagccgtgaagatatctatgagttttattcactgggatttggcgatccaatgccgatttccggagtgcatggcctgggattgggagatctactagacaaggttgttgaaaaatttcctaagaccgatgaaaagacggataacgatgatattcggttcagtattattggccggcccaatgtgggcaagtcgtcactggttaacgccattttgggtgaagaccgggtcattgtttcagatattgccggaaccactcgagacgcaatcgatacccgctttgaggcggatggtatcaagttcacgatggtcgatacggctggaatcagaaaacgcgggaaggtttacgaaaacactgaacgatatagtgtcatgcgggcgatgaaagccattgaccaaagtgatgtgatcttattcgtcatgaacgccgaagagggcattcgtgagcaggataagaaagttgccggatacgctcatgaagctggaaaagcaatcatcacggtggtgaataagtgggatacgctcaaaaagaccaaccacacgcaacaggactttgaaaccctgatcagaaatgaattccagtacatgtcatattcgcccatcattttcgtttcagccgttactaagcaaagaatcgaaaaactaccggcattaatcaaacaggtttatgacaatcatgagaagcgggttcaatcctcagcactcaacgatgtcattatgggggcggtcgctgttcatccaaccccaacggttaatggcaaacgactgcgaatttattacgcgacccaagtcgtaaccgggccaccaacatttgtggtgtttgtgaataatccggacttgatgcatttttcttatgtccggttccttgaaaaccaaattcgtgataattttgacttcaccggaacaccaatcagaatcatcaaacgcagccgaaaatagcccaaaaatcagcaattcttaacaaaatcttgatttttcggcgtttatcgacactaaattgggcaaaaccattgcaatgacggcattcttatgctatctttgaaaaagaaatgatgttggcaaacggcgttatttcagcattccggatttgtgagaattcgacttgcaatggtttacatacctatctttgagggaggtgaatacactcatggcaaataaagcagaattagtaaccaatgttgcagcagcaactggtttgactaagaaagacgctacatcagctgtggatgcagtatttgaatcaatccaagctagtttagcaaaaggtgacaaggttcaattaatcggtttcggtaactttgaagtacgtcaacgtgccgctcgtaagggccgtaacccacaaacaggtcaagaaattcaaattcctgcaagcaaggtaccagctttcaaacctggtaaggcgctcaaggatgctgttaaatagtattcatctgttaagccagaacggcatttgtcgggctggctttttttatacactttggaggacaaatatgagctattcaaaaactgctttagaccaacttgaaggcggccaaattgatgattttaagaaatcatttcagcaagctttggatcacgattcggatgatttgctgtactcattggccgaagagctgtattcactcggcttttcaaattactcaaatactatttacgaaaaattatttaaaaaatatcccaacgatgacggtctaaaaatcaatctcgccgaacttgccattgatgatgatcaagacgacaaagctctcaattatctgtcacaggtttcgccgcagtcggacgaatacgtccgttccttgatggttgcggccgatctgtaccaaacccagggaatgttcgagattagtgaacaaaagctcttagaagcccaaaaattggctcctgatgaggatgtgatcaagtttgctctggcagaattttatttcacgactagaaactaccgcaaggcgattaatttatatttagcgctgatcacctctggtacgttggaaatgtcctcagtcaacctggttgaacgtctgggtgtttcctacgccgaaattggtaagtttgaacaagcgatgggctatctggaacaaatcaagccgattaatatgaacgccgacgttaaatttgaactggcattcacctactttaatttgaaagagtatcaaaaggcaattaaagccttcgaggatttgcgtgattcagatccccagtacagctccctatacccgtacttggcggatgcctatgttaacctcaaacgggttgatgaagcgttaaaggcgatccaagaaggaatttccattgaccaatttaacgaaaaaatctggcagaaggccggccaaattgcggaaatggcgaacgaagacgatttagccttgacctatttccaaaagggccatgagatcgcccctgacgacatggaaatcttgaccttactatcagactggtacgttgctcacgaacgctacagcgataatctgaagcttttagaaggggtttttgaagaccacgtcgtcgatgcccatcttgcttataatttggcactgtcttatcaaaataccggtgatatcaaaaaagccgccaacaattacgaattggccgccgatgaactttccgataatcccgattttcttaaacacgccacgctgttttaccgcgaaatcggcaaaccggatctcgaaaaacagtccttgaaaaaatacttggatttggttcccgatgacatggaaatggaagaattgtgggatgaaatgtgattcacaatccgcaactaaacatcagaaaaaggtcaccagttagggatctcgctaaagttaaagtaaaccatggcgggatagcccaaatgggtgaccttttatcatacatatagccttctggttctatagcagtttaaatcgctttggccgcttataagtgaagccttcaccgatcgcctcgttaacttcaataattgaaataaaggcttcttcatcgatcgattcgaccagcttttttaaagtgtgcagttcgcttggggagaccacacagtagacaatctgtttggaacggtgggaatagcctccctcggcattcaaaaaagtgacgccacgattgagctcgtcttggatggcattggaaattttttctgactcgttactaatgatcaaaatcccccgagccgtgtaagcgccgcgttgggtaaagttgacgatcattgaaaaaatccagacgtagatcaacgtatatgccatctggcggacatttaaataaatgagtgatgacagtaaaaccaagacatcaattgtgagcagcgtttggcccatttgaacgcccttaaaccgctcgaataagcgggcgacaatatcaacaccaccggttgtcccaccaaagcggtaaacaattccacagccaaagccgccaaataagccggcaccaattgccgacaacaacaggtcgtgatcgatattaatcacgattgggacccgctgccaaatccataaaaagatcgccagggcaattgttccgtataaggtataaaacatatctttctttcctaagtagcgataaccgatcgcgaacaggggcacgttgaccaggatggtcgaataggccgggtcaatgtgaaacagggcccggagaatcagtgtgataccggtcacgccaccatcggctaaatgattgtaaatgttaaagaagacgattccaaatgaataaatggcggttccagccgcgattaccagtaaatcaattaacgaaatatctaatttgaagcgactttgcttttgtgccatcgtttttcctccctgaatgatctgacaactcatcatagcaattctaattgacaattggcaatcatttcaccgaactttttgtttcaagcggaaattctgttaaaattacaacaggataaatattaaatggatggcgattattgtgcggatggtagaaattccaaaagaattccacgaagcattaccaattttacaaaagattgaatcagcgggctatgaagcctattttgtcggcggttcggttcgagatacgattttaaagcggccgattcacgatgtcgacattgcgaccagcgcttatcccagtgaggtcaaggcgttgtttaaacggacggttgacacaggaattgagcacggcaccgtcatgattcttgatcacgggactgggtatgaagtcaccacttttcggactgagtccggctaccaagattaccggagaccggatcacgtgacgtttgtgcgctccctgaaagaggatctcaagcggcgggatttcacgattaacgctttggcattggctgagaacggacaggtcactgatttgtttggcggccttagcgacatgcgaaaacacattattcgcgcggttggcgatcccaatgagcgattcaatgaagatgccttgcgaatgatgcgggcggtccggtttgccagccaattggacttcaagattgaggatgccacactagctggcattgccctccatagccagttattggcaaaaattgccgtggaacgctcccacaccgagtttgtcaaaatgatgctgggatcagatgccaaccacggcctcaagatcatgattcagactaatttgtatcaacacgtcccaatactgggtgagcatttagatcaactcagacaaattgccgacactgatttcacccttactaatgaagttcaggtttgggcccttctggcttttaaattcggattcaacagccaacaaattacccgctttttaaaaaggtggaagactgccaataaaataattaatgatgttatacttacggttgaattacttttcgcaattcaacgtggtcaagtgactaatttaaccctttatcatgccggaagtgaaaacgtcgacaacgcaatcgcagtatttgcggaccagtcgaaaactactggactatctgaacgttacaaccgacttgccattaaaaataagcaccagttgaagataaccggtggcgaattaattaaaagaggggtcttaaaacccagtccacagcttggccaggttttgaattatcttgaacaaaatgtggttgccgataagatcaacaatgaacctgaagatcttgttcaggcagctatcaactttttaaatgaggactgataattgaatggaaacaatgcgcgttgagaacttagcaaaaacatacggtgaaaagacgctttttgataagctgaattttattattaatgaacacgaccgaattggcttaattgggactaatgggactggaaagacgtcgttattgaatgccattgccggcattgaccatgactcgacaggtgacattattacctcgaaatcttacaccatcggttatttaaagcaggatccagaactggacgagagtctgtcaattatggatgccgttttttccggatcgcaaactgtctatcggacaattcgccattacgaagctgctttgaaagattattcaacgcatccagaggacccagaagcagccaaacgatataccaaggctgaagcccgaatgaatgaagaagacgcctggaacgcgcaaagtgacgttaaaacgattttgacccagttgaagattaccgattataaccagaagatttccgagttgtccggtggtcaaagacgacgagtggggttggcacaagttctgattcaagcgcccaacttactgttgttggatgagccgaccaaccacttggattttgattccattgattggctggagaattatctggctgcctacaagggctcgttgatcgttgtcactcatgaccggtattttctcgatcacgttgccaacaaaatctgggaactgtcatttggcaaactgtaccagtatgacggcaattatcaggactatgtccagcaaaaagcgacccgagttcaaggtgaaattcaagccgagcataagactcaacagctctacaaacaggaattggcgtggatgaagaccggtgcgaaggcccgttcaaccaagcagcaggcccgcattaatcggtttaatgacttaaaggaaaacgtcggtaccttacagcttgatcaggatgtcaacatttcccttggccagacccgattgggcaaggaagttcttaagatgaaagacgccaatttaaccattgacggcaaaacaattctcaaggatttcaatattctcgtccagccgaatgaacggatcggaatcagtggcgagaacggtgccggtaagaccagcctgctcaacgtcattgccggtcgactgaaattggattctggaattatcaaagtcggcgaaactgtcaaaatcgcctactatacgcaactgaccgagccgattcctgaagataagcgggtcattagttatttgagtgagattggccaacaggtcaccgataataccggcaacaagattagtgttgccgaattgcttgaagaatttctgtttccccgtttcatgcacggcacgttaatccgtaaactttccggtggtgaaaaacgacgcctgtatctgttgaaattattgatgcagcaaccaaatgttttactcttggatgagccgaccaacgacttggatattgcgaccttgaccgttttggaagattacatttccaaattccaagggaccgtcattaccgtttcccatgaccgttacttcttggacaaagttgccgatcgattgctgatctttaaaggcaacggtgtgattgaagaacaccgcggtcggttcaccgattacctggcctcattgaagaaggcgccgaaatcgtctgccaagtcagacagcgggcagtcaacttctcaatcggattcggcaagctcaagtcaagacgcacccgcttcaaatgctaaaaccaagaaaaaattgacatattctgaaaagatcgaatatgatcacatcgaagatgacattgaaaagctcgaatcacaagttgaagacattgataagcagatgcaaaacaatggctcagattatgataagctggcggatcttcaagcacaaaaggaccagttgtctgccgaggccgacaaaaaaatgaaacgctgggaatatttaagcgaatacgctgaataattaaaaacagtcacgttctgataaaaaggagaattgccatgttagaagacgcctatttagatcttgcacgttatgttttggaaaatggccacaaaaaagctgatcgaacccataccggaaccatcagtacgtttggctatcagatgcgattcgatttatccaagggatttcctttattaaccactaagaaagtgccgtttggattaatcaaaagtgaactcttatggttcttgaagggtgacaccaacatccaatttttattgaagcataagaatcacatctgggacgagtgggcttttgaaaagtttgtcgcttcaaatgactataccggcccggatatgactgacttttctcatcgggcacaaaaagatcccgaattcaacaaagtttatcaggagcaaaagaagcaattctgtgatcgaattgtcaacgacgatgatttcgccaaaaagtatggcgacttaggtctggtttacggcagccaatggcgggcctggaagacttccactggtggaacgatcgaccaaattcaaaatgtgattgatttaattaaaactcaccctgattcaagacggatgatcgtttccgcatggaatccagaggatgtgccaacaatggccttgccgccttgccacaccttattccaattctatgtcaacgatggcaagttaagctgccaattgtatcaacgttcaggagatattttcctcggcgtgccttataatatcgccagttacgccttattgacctccatgatcgccagagagtgtggcttggaagttggcgatttcgtgcacacctttggggatgcccacatttacctgaaccatattgaccaagtcgaggaactcctttcccgtaaacctcgtcaggcacccgaattgtggctgaatcctgaaaagaaacatttggatgaattcgaaatggctgatatcaaggtcaaaaattacgacccatacccagtcattaaagcgccggttgcagtttaggaggaagtcgatgctagcttttatctgggctgaagacgccaacggcttaattggtgccaatggccaacttccttggcatctgccggacgatatgcattacttcaaagaaaccacgatgggcaatacgattatttccggatcgaaaaccttccgcagttataatcggccactgccgggtcgtgagaatattgtggtttcacaccaaactgattttccaacgggcgtcaaagttatcccttcgattgaacaactgtgtgacttgattgctcaaaatcccgataaacaatatattgtgaccggaggtgccaatctatttgcccaattacgttcaaaagtcgaccggctttatcgcacgaagattgaagctgaattttccggtgacacctatatgccagccattgactattctttatttgaattgagcaaatcggtcgttggtgttgttgacggcaaaaataagtacccccacacttttgaagttttcgatagaaaataacgccggcataaatgcttatgaatctttggcagaactttgatataattgtcgttggactatcaattaattattaattttgtaaagaaacgagtggcgtaaatggcaaaagtaaaaattgtgacggactcatctgcccagttgacagatgaagaactcaaacaatacggcattacaattgttccattaacagtgatgattgatgatacggtctacgttgatcgtgatacgatcaccaatgaaacctttgttcctcaaatgttggcggctcatgatctgccaaagaccagtcaaccaccagttggtaaatttgttgaagcatttgaccggttgggtgaagacggcagccaaattctctgtttgaatatgttggctgccatcagcggcacggttcacgcagccgaacaagcagccacaatcagcaaatccgatgtgaccgtggttgacagtcaaagtaccgaccgcggcctgggctttcaagtgcttgaagcggctaagctggctcagcaaggtgccgacatggacaccattttagccagagtcaatcaggttcgtattaacaccaagctttatttatgtgtcatgactctggataatattgtcaagggcggtcgattgcatccgattgccggggcaatcaccaactttttaaacattaagttggggcttcaagtcactgacggcaaacttaaaattatttctaaaggtcgcggcgataaatcgcttaaaaagtttttcaatggtattattgatgaaatgaaaaacaccgccgctgttaagtcgattggcgtttcatacgtcactgaaactgaagtattaaaggacactgttcaaaagcttaaggctgactttcccgatgcatcatttcttgaacgggtgacgtcaccgaccatttccacgcataccggtaaaggggcttttgcgttgatttattacagtgatcccgagtaattgcagatctgaaatattgcttaaaggggcgaggcaaagcggctgttttgttgtcaccccttttagatttgatcaccatttgagaggttgtttttgtgagtcaaaataaacatgttaaacagacacagcatcattttcgttggattatcggattgatcggcctgatcgtgattggggcagtcgcatttttcggctaccattatttcaactcggccaaagaaaccctgccaagagaagttaaattgacggctgttggggattcactgactcaaggggttggcgatccgaccaacaaaggtggctatacccacttgattcgccaaaaagtgattcaaaaaaatcccaatgttcacctgtccactgccaactatggcatttcaggggaaaccaccaaccaaattaatcatcgggtggtttattcaaaacggctgcagcacagcatacgagaagccgatgtgatcacgattaccactggtggaaacgatttactgaagtttttgaaggcgaacgttgttggcttgaacaaacatcagttgaaccagaaattgaccggttattgtcaaacatatcaaaccagggttacccggctattccgaaatatccgccacttaaaccgtcgggcgccgattttcgtttttggcatttacaatcctgtctacgtttacttcccccaggtcaactatatcaacgacaccgtggcccataccaaccagattaccaataaagtgatccaccaacagcacaggatgtactttgtttcgattaacaaaccacttacagacggtcagtttaccactgccaaatccagaaaaactttggaagaaaaggccgctgccagcattatcgccgagaatcatgattcgcctgccgatattgaacagttattgagtggccaacctgcccaagcaaataaatatctctcaaatgatgaccatttccacccgaatttgaaggggtatcaaattatgaccaatcgcttgtattcccaaatggtcaagcacatatcctggttaaaggagtgatccaaaatgagaaaagcctccaagcagacgaaatcccgcaatccttggaaaatcgctttcatatcgttaatcggcctcctggttgttttagttgccggcatgtttttggcggtttctttatcgtcatctacgacgaaattggtgaatcaaaagtcgaccaaccaatcggagccaatttccgccactatcaataaagctcaactcaatcaactatccaattattatttagataagctgcagaagggccgaccttcgcaatatcactttgaagtcgccaacgaagggattgtctatggctcgctgactttattaggttccaacgtcgattattcactgaccttcgacccgaaagtgatgcccaatggtaatattgaacttcacgctaataagctggcactggggaagtttccggtgccaatcagttttgttttaatgtatgtcaaacaaaactataaactgccaaagtgggtccaactgattcctaaagataaaaccatcaaacttgatataattcacatgaacggtaagaatgggattaattatcgggcccggaccatcgatttgaaaggccaaggaaaatttgcctttgagattcttttgccgaccactgacaaggaggactaatatgcacaaaacgttctaccaatatttaatgaccaaacgcaaccccggaagtactgatccagaggctgaatttgccaacaacgcattttatgatcagtcatttcccaaacaagaagatgagtttgacgcgttatccaagtatttagaagaaaatgcttcataccttccgaccatggaaatttttgattccgtgtggaaggaatatcaagaaagcttttaggaagtgaaacaatggcagtaacaattcaatggtttccaggacacatggccaaggcaattcgtcagtttgaagaaaatctttctttagttgacgtggtatttgaagtgattgacgccagaattccgctgacttctcaaaaccctgaaattcgacgaatcagtgccgataagccgcatctttatatcatgacaaagcgtgatttggctgatcctcaattaaccaatgcctggctgcagtattttgctgaacacaaccaaccggcaatcgccattgatgccaaaaccaaatttggcattaataatgtgatttcggtgatttcacccattttgcgtgacaaattgcagcgggaacaggataaaggcatgaagaaacgaccgatccgagccattagcgttggggtaccgaatgtcgggaaatcaactgttttgaaccgattggtcaaccgtcgagccgctcaggttggcaaccgtcccggcttaaccaaggggcaacagtggcttaaatctaatgataagttggaattactggatacgccgggaattctgtggccaaaattttccagtcaagaggttgcggataagctggcattgaccggtgcaatcaaagagagtgtttatgccagtgacgacattgccttgtttggcttaaagcagatcagacagcttcacccggaaggcctcaaagaccgttatcatttaactgacgacgatttggatttgtccgacgttgacctgctgttacaaattactaagaaagtcggcatgcgcgatgattatgaacgtggctccaatcggattattcaagatttccgtgccggcaaaattggtcgttttactttggatgatcctgaaacggtgagtgacgatgaccaagctaacaattaaagacgttaaacaggttttatcccagatgtctgatctcgctgatccgcggttgattgagttaaaggctgacccgcgaaaaggggttcaattggcaattcagtcaacagaaaaccgcctgcaaaagcaggccagagccctcgctgaatttgaacagcggtttaaatatgaacggtctttttggcatcaggggctgcaatatgttgccggtgtggatgaagtcggcagaggtcctctggcggggccagtggtggctgctgcagtgattctgccgcacgactttgatctggtttccgtcaatgattccaagcagctgacaccggcccaacgcgcagagttggccccgctgatttcagctgaagccctgagcgtggggattggatcggtggataatcatgggatcgatgagttaaacatttaccaagccactcgtgttgccatgaaacaagctgtggaatctttaaccccacagccggatgaaatcattgttgatgccatgcagattcccgttccgattcggcaaaccagactgatcaaaggtgatgccaagagcatcagtgtttctgcagccagcattgtcgccaaagtctatcgggaccatttgatggacgagtacgccaagcagtacccggaatacgattttccacacaacgccggctatggaacggccaagcatttagcagctctcaaggaactgggaccaacgccgattcatcgaatgagttttgccccagtgaaaaagtttagcaaaaaataaatatgttttacgtagataactcttaaaaggatgatgacaatgcttttaagagattttttgttaagaatacatttatgtaaaggaatcggcataattggtaagtcaaaaatttatacttgggtaaatcaggtcgactggcgggatgatcaactgccgacctcaggattcttggctgccgtcgctcaactaaacgttaagaacacggctaacttcaaaaccagttatcaacagttaatgcgaaacgaagaccgggtggaccagctggtcgatggtgaacagtggctgagcattgcagatgctgaatatccacttcaactgcgagaatcgtttgcgccgccgttagtgctgttttatcgcggagatttgtcgcttttatcccagccgcttttaggaatcgttggggcgcgggactgcacctcatattcagtcgaaatcctaaaaaatttgattcctggaagagtttccaatacaatggctattgtgtcggggctggctaaaggggttgatacgttggcccaccaatgtgtcatcgccaaccacggtaaaaccattgccgtgattgggacagggttggacgtgtgttatccatataccaatcaggaactacaagcaacgattgccgccgaccatctgttaatcagtgaatatcccaatcataccaagggctatcgaaatcactttccggaacgtaaccgcatcattgccggattggttcaaagtgttctggtcactgaagccaaaaaacattccggtagtttgatcacggccaatttagccctgcaaaataatcgcaatgtcttagcagtcccggggtcaattatgatgccgctgtccgttggtaccaatgaattaatcgctgccggcgcaaaaccggttttacgtgaattagacatcttggaggactactttcagacgcggatttaagggcagtgagttgacactttaaaattcctgcaatatgatgtggtagatttgtaataaaaattcctacaataatataactaaaaataagcagttttgaggggagaaaatatggcaacttctacaaaaacgaaaccaaaagccaaagcaaaatcaaaaactaagcgaaaatcgcctaaaaaaaatctggtcattgtggagtcacctgccaaagccaagaccatagaaaaatatcttggccgttcatataaggtggtcgccagtaaaggacacgtgcgggatttgcccaagagtaagatgggcgttgatatcgaccatgattatgaaccacactacatttccattcggggtaagggtgacacgattaaagaattacggtcagccgctaaaaaggccaaaaaagtgtatctggcagccgatccggatcgtgaaggggaatcgattgcctggcatcttcagcacattttggatttagatcccaacgaagataaccgagtggtatttaatgaaatcaccaaggatgccgtcaaagaatcattcaaacatccccgaaatatcgatatgaatctcgttgatgctcaacaggctcggcggattttagaccggttggtgggatattcaatttcaccgcttctctggcaaaaggttaagaaagggctcagtgccgggcgggttcaatcgatcgccctctggctgattattcaacgcgaaaaggccatcaaagactttaccccagaagagtactggtcaattgattctgaatttaagaagggccgcagtaagttcaaagctgccttttatggcttaaacggtaagaaaaaggaactgccaaataacgaggcggttcaaaaggttctgcagcagttggatcccaaaggtgactttgatattaccaaggtgacccgtcgcgaacggaagcgccaaccgcagccgccatttaccaccagtacaatgcagcaggaagccaaccgaaagctcaacttcagaacgcgaaagacgatgatggctgcccaacagctgtatgaaggaatcaatattggtaaagagggtagtcaaggtctgattacctatatgcggaccgattcaacccgaatttcagtcattgccaaacacgaagcgtcccaatttctacatgagaaatacggcgccgaatatgcggcaacgaaaccgattaaaggtaaattgcctgagggtgctcaagatgcccatgaggccattcgtccgacttccgttttcagaacgcctgccagtttgaaacaatatctgacccgcgaccaatttagactctatcaaatggtttggtcaagatttgtggccagccaaatgactccggcaatcatggataccatggcagtgacaattgaacaaaataacgtgatttttaaagccaatggttccaagatgaagtttgatgggttcttgaaggtttatggtgacagtaaagaaaaggacaacttgttacccgatttggagagtggcgatgttgttaagttggttaagaataatccggaccagcattttactcagccaccggcacgatacagtgaagcaacgctgattaaagcccttgaagaaaagggtgttggccggccatcaacgtactcaccaaccattgatacgattcagcgccggtattacgttaaggaagttggccgtcgatttgagccgactgaattaggggaaattgtcaataagattattgttgaatacttcccagacgtggtaaacattgacttcactgcaaatttagaaggcaaactggatcaggttgaagaaggtaaagagaactggatcaaattagtcgatacgttctataaaccattttccgatgaggttgatgccgcaaccaaaaatatggaaaaggtccaaattaaagatgaaccggcaggcattaactgtgaaatttgtggcgccccaatggtgatcaaaatgggccgttacggtaaattctatgcctgttcaagattcccggattgtcgcaataccaaggcaattgttaaggagatcggtgtgatttgtcctaagtgtcacaaagggcaggtcattgagcgaaaatcaagaaagaaccggattttctatggttgctcaagatacccggattgtgatttcgtttcttgggacaagccaatcggcagagattgtccaaaggatggtcacttcttagttgaaaaacgggtcaagggcggcacgcaagtggtttgtccaaacggcgactatgaggaaccggcacaaaaataaaaagcatgcgacgagccctgggttgaccccggagcacaagcagaaacaaccagtgatgaacgttttttgttcatcgctggttgtttttgtttgtgcagtaggggtcaggggcgtcggagctgaactcaaaggccgaagggagcacgaagtaaactaactgctgtatccctgtaaaagcaatcctgaataaattccggggtacgaattttgttcattgttggtgctcctcacttatgcagtaggggtcaggggcgtcggagctgaactcaaaggccgaagggagcacgaagtaaactgatcgctctagccctgtaaaagcaatcctgaatgaatctcggggtacgaattttgttcatcgttggtgctcctcacttatgtggtaggggtcaggggcgtcggagctgaactcaaaggccgaaggaagcacggaataaaccaactgctgtatccctgtaaaagcaatcttgaatgagtcctgatgaacgtcttttgttcatcgctggttgtttttgtttgtgcagtagggtcctggggcgtcggagctgaactcaaaggcccaagggagcacggaataaactgatcgctctaaccctgtaaaagcaatcctgaatgaattccgaatcacgaattttgttcatcgttggtgcccctcatttgtatagcagaacgggaagcctaatcgttaaaaagcatccaactgccaccagaatcaattccatggaattgattcctttgacaaaaagccaccaccccgcaatccccatttttgcattcaacggtcttttgttccacaatgcacaaaagggtgtaaaatcaaggtgatagaaagacaaggggaggcttcaaaatgttttcatcaaaacacagtagttgtacaactattctagtcggcaagaaggccagctatgacgggtcaaccatcatcgccagaaatgaggatgccggagatgccgttaatccaaagaagtttgtggttgttgaaccagaagaccaaccacgcaattatcagtcaaaattaaccaagtttagtgttaaactgccagacaatccattgagatatacctcagtgcccgatgctgtccctgacaagggtgtttggggcgaggcgggcatcaatgcccataatgtggcaatgagtgccacagagacgattaccaccaattctcgggtgatcggtgccgacccatttgaaaaagacggccttggcgaagaagatctgttaacaattaccctgccatatatcaattctgcccgagaaggggttcaacgagtgggtaaactgcttgagaaatatggcacatacgagtccaacggaatcctgttttcagatgtcaacgaaatttggtacatggaaactgccggtggccatcactgggtagcccaacggattccagatgatgcctatgtcatcgcgcccaaccagacaggcatccaagagatcgatttcgatgatcctgacagctttatgttctcaaaagacttgcgtaaatttgcccaggaacaccatctcaacccaaccagtcactttaacttcaggaaggtctttggctcagatacccagctggaccgtcactacaacacaccacgtgcttggtatggtcaacgatatttcgatccggaatcagtgaaggataagacgccaatgagcaatgatttgccgtttatctgccacgccaaccgcaagattacgattgaagatatcaaattcgttctgagctcccattatcaagacacgccttacgatccgtttgcgccgggagctgattataagaccgttccatatcgaccaattggcatcaaccgcaaccaagagctgtcaatcttgcagttacgtccaggaattccttcagcttattcagcaattcagtggctgacattcgcctccaatccgttcaacacgttgacaccattctttaccaacgtcgtcaatacaccggactgctaccgtgataccaccgagacgctggacagccacaacgcctattgggcaaatcgcctgatttcattgattgctgctgatcattatcaggccttgatgcaagacattgaagactatcagcttaaagaaatgggttatgcccacgaacgaattgcccaagttgatcagcagatggccgaaaaagaggcttccggctcacacgttgttcgagcccttggccaagccaatgcccggaccgctgatcacgtcatgaaagcgaccgaggatctgctgacaaaattggttgtcaaggccagccaggatctgccaggctcatttacccgagaacattactaaactaaatcagtcatcataaccaaacgaagccggctcacaaaattgaatttgtggccggcttcgttttgttattcaatttttaagacagattatcttaatgttggagacgagtcattataggttcgtgtcctgggtaaaattgattggtgagaggtctgttgaattggtgatgatgtcactaatcaattggttgtaagcatccaggcccatcttggcattggcaaagttgactttggtcagataattggcgagttcgacattggacaaaccttggaatgaagcatcagcttgtttgactgcttgttggaaattcactcgcagtttggccttggtgtcatttaatttgggcccgaatttgacgtaatgcgggtcaactaagacaccggcaagcttgtaagtccaataggcttgattgggggcatagctgcctgaagcattctgataggattttggcgtggtgtttgcgccggcataaaacggcacaaaagaactttgagcagcgacgcccattgccaaccattgaatccctgcagcaggagtgggcatatttggccgaatttggaggatgtgggcctcttgcgtcttggcgagactaattggtcgatagaggtgcttatcgtgctcagagccctcgccaatggggtcaaacggtgtgccttgataatgggagcttaagaaatcttcaacgtcaaacaagcttagtttgcggttggcctgattgataaacggcatttcctggctggttggctcaaaattcaattctggtgagaacattttcaagccgtaccatacgcggggggtgttataaactgtgtctgacaagtcagcggtaccaaagattttacggaagttgaaggttttcccggacgggtccgggttcaagtgattttcggagacaaaccggcgaatcttgggtgaccacatgaagttgtcggggtcgttaaaatcaacgtcttgaatggcgctttgattggcaatcaccgcgtaaccgtcgtctggaatgcgttgggcaacccagttgtggccgccgccggtttccatataccaagcctcattcttatcggcaaacaaaatgccgttggattccgatgttccgaagtattccacaatttggcccaatcgagcaattccttcacgcgcggttttaacgtaggggaggacaaccgtaatcattgcttcttctccaatgccatcttcgttgagcggatcggcccccaaagccagctgattggtataggtgctttcggtagcactcatggcaaccccgaactcattaaagccattttcttcaaacaggccgaacttgtcagtccattcaggggtggcagaatattgaaagcgcactttcggcagggttaacttgaagccgttgtctttggatgagaaaaccggggtttcactaaattcttgatgctcgtggatgacataattctttggccaagaggatttactatcctcgtttcgggcaatcataattgacccgtcaatgctggctttcttgccaacaatcatactggtacaggcggaaaagtttttgtatggtatcattttaaaatctcctattcgcagttaaatgttactccaattattgtatcatctttgctccataaacggtcctgacacgtccaaagtgccatcaagatattgcaggcaaaaataatttaaggtatacttttgccattcgaaacaaatggaggaatcaaaatatgccaattgtagatattcatttaattgccggccgttctcaagatcaactgaagggcttggtggaagacgttaccgcagccgttgttaaaaataccggtgctcccgcagaacatgttcacgtgattttaagtgaaatggaaaagaaccgttacagtgttggcggtgtgctcaagagtgacgaaaaatagtcgcaaataatttggaagtccgccagacaattgttgcgggctttttgtttgcgtttaattcggggatgaatcatcaaattcttttactttgataaagtttatctcaaggttggtttgccagtcgatattattgtatacttaacaaagaaaaagcgtttaaacgcacgaataataggaatggagacctttacatgaatgatcagcaatacataatgtccattgatgaggggacaacaagtacccgggcaatattgtttaataatgatggtgatatcgttggtaaagcacaacgggagttccaccagtattttccaaaatccggttgggttgaacacgatgccaatgagatttggaatgccgttcaatcagtgatctcagaagccttgattaatgcggatgtccaaccatacaaggttcggggaattggtgtgaccaaccagcgggaaaccacggtcatttgggataaaaataccggcgagccgatttatcatgccattgtttggcagtccaaacaaaccgctgccttagccgatcagctcaagcacgacggttatgatgatatgatccatgaaaaaaccggcttgatcattgattcctacttttccgcaactaagattcaatggattttggatcatgtagacggcgctcgccaaaaggccgaaaatggcgatttattgtttggaaccattgatacctgggtcctttggaagctgaccggcggcaaggttcatgcgaccgattataccaatgccagtcggacgatgctgtttaacattcacacgttgacttgggacaaagatattttggacctgctgcacattcctgaaagcatgctgccggaagtccgttcctcgtcagaaatttatggttatacagctggttattccttctcgggtgttcaggttccgattgctggaattgccggtgaccaacaagcagctttgtttggtcaaatggctctgcagcgcgggatgatcaaaaacacttacggaaccggtgcctttatcgtcatgaatactggtgaggagccgacactttccaaacgggggctgttgacgaccattgcttatggaatcaatggcaaagttaattatgccttggaaggaagtattttcgtcgctggttctgccattcaatggcttcgagacggaatggaaatggttaagtcatcccctgactcggaacaaatggcgattgatgctaaaagtaccgatggcgtctacgtcgtaccagcctttaccgggttgggtgcgccctactgggatcaggatgccagaggggcggtctttggcctgactcgtggcacgaccaaaaatcagtttgttcgagctacgcttgagtcattagcttatcaaaccagggatgttgttgacaccatggcagctgaaaccggaatcgatttgaagtcgctggcagttgacggaggggcagctaataacaattatctcatgcaattccaagctgatattttgggaacgccaattcagcgggcctcaatttcagaaaccaccgcgctgggtgcagcctacctagcaggcttggcagtcggcttttgggattctatcgaagaaattcgccggaccgttaaatcacgggatgcttttgaaccgcaaatggacgagcagacacgcacaaaactgtataccggttggcaaaaggccgtccaggcaacgattcagtatcatcccgacgaaaactaatcatttatcattttttcgttgtgagttcaatgaccacttttgattgctcaaacttacgacaactggcattacttgtgtggcaaactggccattaacaaagaaacgcagtcacttcaacatttggaatgactgcgtttctgcattaaactatgggattaaatcgctgttcgtcccgagggttagtttttgctatcggttaagcaccaacagcaatgtccagtcgatcttgaagataatgggcaacaccatcttcatcattggtgaattccgtgacctcgtcggcctggcccttgattttatcaatggcgtttttcatcgcgacaccggtgcctgcgtattgcatcatggtcaaatcgttgccttcatcaccaaaggcaataatgtctttttgcaggatgccatagtaatcggccaaaaatttaaggccggtggatttatggacacctttcgtggcgatttccacaatcggatttgggccgccccaaggggagacttcaacctcgtcgccaaattgatgttcgacgaagtcaatcaacccctgcttgagttcgggttccacttgaacagtaatgctgatcgggttttcttttaggcttttgcgactcagtacctgattggtggccaaggtgctggggaagaagccgaaaccactgcttaatccctggttggccaaaaacatattccggccttcaacggcaatcaatgacaagccgagcggtttgctttttgccagtaattcagtcacaatttctttatcaattgtgtactggtattcacgattccactgttgatgtggtaaaatgccaaggttgccattgaaattaatcattggcgtcgttagctttaaatcgtcataaaaagtttcagagagtctattgggacggccggttacgatactgactatgtatccttgcttcgcagctgcccgaattgtttgggcagttttggcgctgattagactatcgttatttagggttgtgccgtccaagtcgagggcgattaatttctttgtaattgtgatcactccttactaacatatccatttataatatccaaaaacacctatcacgtcaattattagtaccaaaaagggagattagaatgaacttaccaactgattttgtgaataagtatcagcaattaatgggcaaatcagaagccgaccagttcattgccagctttgacgaaccgacaaccccgggttttcggcttaatccattgaaagccagtcaaccaactgatttggacctgagtgagcccacggaacactgccgatttggctatcatggtcaggtcagcggcaaaaccatcgatcatcaaagtggggcggtttacagtcaggaacccagtgcgatgtatgtgggtgaagttgcccaccccaacctgggagaaagggtattggatttgtgtgcggcgcctggtggtaaaaccacccatcttggcagctatctgcaaaacaccggcctgctaatcgccaacgagattgacagcaagcgtgccaaagcgttggttgaaaacgttgagcgatttggcatgaccaatacgattgtcaccaacacggatccggaccatttagcagcccaattaccggaattcttcgatcggattttggtggatgcaccgtgttcgggagaagggatgtttcgaaaagacccggacgccgtccaatactggtctgtcgattacccaattgaatgtgcggcccgtcagcggacaattttggcccaggcggttaagaatctaaagcctggcggggaattgatttactccacctgtacctttgcccctgaagaggatgagcagatcattgcctggctggtcgacacctatggatttgacattcaaccgattaaaaaatttgccggaatggatgacggtcaaccagattgggctgatggcaatcaggatttaaccaactgtgtgcgtatctttccacatcattttaacggagaaggccattttattgccaaattgaaaaagccggcagacccggaagttagcaaaggaccgcgtcgcttccgcggcatcagtcgaaatattgaaatgccctccaaatatcagaatcaattgttcaaccagtttgccaaagcaaccttaaagaacgttcactttgacaaattggtggttttcaaagatcatctttactcagtaccggaaaatacgccgaacttgtctggcattaaaattgtccgacttggtttggagatggggactttcaaaaagaaccgctttgaacctagttatggcttagccttggcactgcatcccgatcaagtcagtcaaaaaatcactatagacttggcggattggcaaaagtacgtgcatggcgatacattccaagtctcaccagatctgaaaaaggggtggtacctcctggtttgccagcagcagccagttggctttgccaaagttgtgaatggtacggccaagaatttcttccccaaggggctgagatttgcgatgtaaaaagagttaaatcaccatcagaagattgtggcttctgatttttgatttaactcttttttaataggctaatttcctttgttttaaatagctcaacaattgtggatcaaggatcaaccgttgccgttgtaagtcagcaatggttcggcagttcaacattaacatgattgcttttagtccgtactgccattctttgacatcgttaataatttcattatcgcttttatggatgatctcatgaagccagtaacctgccacgccaactgctgaggcacccagtgtgaggcatttagccacgtccagcggtgatttgacaccaccggcagcaatgatgcccaaccgatcagaaaaggcgcgggcttcgaatagcgactcaacggtgctcagtccccaatccgtcaaataagccatgtcttttgaggagcggcggaagttctcgatggcagcgaaattggtcccgccatgcccgccgacgttgacatacttcactcccaggtcaaccagttgtgaaatagttgcttggctcatgccaaagccaacttctttcacaatgaccgggacaccgacattggcaacaattgcttgaatattgtcaataaagtgaaactcccgatctccttcaggcatgacgagctcttgggcgacgttgatgtgcaactccaaagcatcggcggcgatcatctcgacggctttttgggcatcctcaacgctgtggttggcaccgatatttgccaagacaattccgtttggattggtttgacggacaatactgaaggaatcgcgcacctcaggatcacttaacccaacgctttgagagccgaccgccatcgccaatccacaggcttttgccaccacagcaagtcgccggttgatctctttggtgcgggggctgccaccagacatcgcttcaatatagaaaggggtcgtcagcgacagggggccaagctgggtggttaaatcaatatcatctaaccgatatttgggcagactggcattcacaaatcgaacgccggcaaacgagctgtcgacaggttggtagaacttttcagccagggacacatgttcatctttacgatgggaatgttgtgaagtcataagctactccttgtcaagatcgatgacgggatggactttaagggccagctgctggatgccattttcctgccaatgggcgatcatcgaatcaacatcggtatctttgtcggcaaccacgatcccgcagtcaccgccaccagctccggaagatttggcagctgcagcatggtcgacggcaatgtcgcacatcttcttgagaattggggtttcaatcggcactttggtaaaagcagccaaatgttgaaggatttcccggttacgggcgattccctctttgatgaccgacaggctgccatttttgaaaccgtcaatcaattcgtccaggcaggctttgctttcggccagaaaatgggtgtaagtctcatgctgattgctcttttgaacggcaaccttgtcaaccaaatgcgaagttgaggccggagaaccggtccagccgataatcagcttcaacccgtcaggtggcgttaattgcgtaatttttaaatgcggccaaggcttgttgactaaggaaatcaggtcttcctgcattcgagcagccatgagccagctgcggtcaaatgaacggtaagcgatccagccgccgtatacactggcagcgatatctcccaaagaaccgtttccttggacgtccaaatgggcaattgccgacagtttgaacagtttactcttggtcagcggtaagttgtagaactgacagagagctttgacggtggccaccgtcacggcagctgaagaacccaatccatacttttttccgttggggctatccaaatcactattgatccgcagatcatagagctccatctgccggccgagggactgcgcatattcctcagtgagctgaatggctgaaattatgtagttaaaagtattgtcacggttatccagaatcatttgatcaccgcgacgacgccaatagaccgaatcttctcggtattgttttgaaacgatactgccataggacttgcttcgagaaatttcgacagttacgaattggtccaaagccacaataatagaagggtagccagtttcgactaccgcgtattcaccggcgatatataattttcccggagctttaaccttaatcaacggatcatttcctttctagtttataaatatttgacacccgggccaggcttggcaacggtcactttggttgggccaaacaggtttgagaaggtatcggtgatggtttgaacattggcttgttgacaaatgactttaatattggggccggcatcgattgtatagtaacattcaatcccggaatgcctgagccgtttaacttcgttcatggcggtcaaggtgtcgccgttgaagtagagaaaatccggatcggcactcagtgttagggcgtgcatccgcatggcatttaactcactaattgtgccaaaacgcgtgaagtcatcatcttggatggcggctttgatattctccagatcggcttcgacgaccttaacccacgttggatagtatggggaggtggtgactgaaagggccatgccttcccgactggaaatgggcttttgatgcttttcaatggttaatgcaacgatgcggatgtcgttcaaatgagtcgtttcgactggaatggcgtacgaattggtatcgtctgatccttttcgccattccacaaagccgccaaagattgaccggcaggctgaaccggatccccggcgggccaatcgggacaagtccgttaaactcagattcatgccggcggctttgctggcagcggcggccaacgcagcaaacgccgaggcagaggatgccaggccagctgccgttggcacatgattagtcgatttgacttgggcgtttaaatcaattccagattcttggcggacaatgcttaagaagttgtgaacccgttgaccgctttttccggttaccggctggccatcaattgtaatctggtctttatccaggttggcgttaaatgtcacgctggtttgagtataaaattgatccagcgtcaaagagagactgccagtgtaggggatgatgagttcaggattttgtttgccccaatatttaattaaggcaatattcgtgtgagcaactgctgtaacggtcttatctgacgaggttgtcatgagcttctcctgttgaaaattgataattcttaaatgattgaatccaagtctgagtggcaccggcttttcgaagggcagtcgaaatttgttgagcatcccgttggttcttggctagggcgatgacacagccgcccaaaccactgccggttagtttggcacctaaagcgtgattgtcacaagcaacttgacagaatgtgtccagagtgtggttgctgacgccgagttgggccaggtcacgttgggattgtgtcattagtttgcccagtagcacatcgtcggtggttgccaaagcattgcgagccgtttcggcaatcttgccaagctcgtcaattaatggttgagaactttccggttcgtcgaccaggttatcatgaaccaacgaaacggcctcactggtttttcctttaatcccactatcggcaatgaccaatgatgaggttggcagattaaagtcaatctgctcgttgattttgtttcggataaaccaaatcggcatgttggagctggcggtcgcagagtccaggccgctgggattgccgtgggtaatcttttcttcaatatccgctaacttcagcaattggcttctggtcaaattgacctcaaaaaaatcaaaaaaagcccgcacaattgcgattgccgttgccgctgaggatcccattccgcgttcggcaggcagtttgctttggatgtcgagatcaaaagcaagcctttgagcgccaaacaaactaacgagatgagtgattaatgttttaacaccccgcagattctccgccatttcactaattgggccgtcaaagtaacgacagtgaatttgttggccggttggaattctttgaatggtcgcaaccacatcaacggagtagattgggatggcgatggcgggcttttcgtaaacgacactatgctcaccaaaccaaataatttttgcgtaactttttccagttgctttatctttcaactttatccgctcactttcaaacattccaattttatcatagttcactgattcgagaacgttttaaagatatttttagagattcataaataattctacttctttccatggtagattatcacatcttgcttgtagtatgattaaagttagtgaatatttaagaaaagtcagctcataaacagattggtgaatgacaatgaattcaaaaaccacctttgccgtggttgatattgaaacgaccggaacagatatttctgcggataatcggacaattcagttcagctgctgcttggtttccaacaacaaaattattaaaaccttcgtgaccgatatcaatccacaacgagaagtccctaaccgaattgtgcagttaaccggaatcaccaacgaacggctgcaaaaggccaaaacttttgaccaggttgccgctcagctgtattccttgctcaataatacggtttttgtggcccacaatgtgaattttgattttccgtttctgaactctgaatttcaacgcgtcggctaccccgaattacaaattgaagcaattgacactgtcactttaagccaaatcctgctgccaacgttatccagttatcggctgcaggatctcagcagttatttcaatatcgaacatgaccatccccatacagccgatagtgatgctttggcaaccgccaagctcctgcttattttactacgacaaattaagatgctgccgaaaatgaccttggaacagatcatcagcgttaatccgtctctgcctcaagacacgatgcaggtttttttggatgccgatgaaaccaacaaaaggcaggtgcacgctgccaaattgcctgatcagctgagaatctcatcaggactggttttgcgaaaacaggacccaatcgtcgtgactgatgagtctgataaacagcgtcttcgctatccaaaaacaaaaaaggccaagcaaaaactgcttccggacaacctggagtcgcgacttgagcagaataaaatgatgaacttgatctataacaattatgccgaccaacagcatcacgcagccaagaccctcttaattgaggccccaaccgggattggtaagagcttggggtattgtctgccattgagttatttggtgtcggcccacaagcctgcagtcatcagtacttcgacaacttatctgcagtttcagctgcaaaatcagacgttgccaatgctcaatgaagggctgcctttcaaagtcaatagtgtcattttaaaaggggccagtcactacatcgatctctacaagttccgcaacttattaaacgttcctgacaactcaacccaaaccgcgtttattaaagcgcagatcttagtctggctgacggttaccactacgggtgatttggacgaactgcacttaaacgtcgatcaaacaccatttgtctggaaaattcagcataccggcgtgaaatggctggatccaaacgaaccgttttatgacgacgattttttgcgttacaacttgaaaaaggcacaaaatgctgattttttgattgtcaatcacagttatctaattaaaaattggcagtatttcaaggatctgccgaccaaaccctacttactgattgacgaaacccagcagtttgctgaaactgccattcgtaacaatcaggagcggattaatccgttatcactgacaacggcgattaacaaaatcttggcagatattaatgggactcacgaagataatatcaaagaaattgtggaagacgacgccatcttggaccacgctatcgaagcccttgacggcaaactccgacaggccaagaccctggtctcgaccgtcacgacgaccctctttgaaatggtcgtcaagggcaaacggctccaccggaatgccgagttcttcgagcgcttaattccgattaatgagatgaaggcagccaccgctgccaatcaagaaccgatcaaccgtctccgcgcgctccacgacagcttggacggactgctggccactttaaatgcccaaattgaccataatgccggtgcatacaccaaccacgatttcttaagtatttattctttttttgaaaactataatgagtttaatcatcaattacgcttgctgttagcaatcgttgatgttgacgaccagtcaattgagcagcatgtgacgtgggtcaccgtcaataatgtcaaagacgtcaatagcctgacacttaaccgggggattttgaaaacggaagattatctccgtgaccatgtctattctgcctttgaaccggcaacttttaccggggcgacaattttctcttcacgacgttcacagttcatttacaacttattggggattagtcgcgacgattcttcgattaaacgactcaaaagcgacttcaatcccaaagatcaagcccgactctatttggtcaccgatcaagacgaccggcaattcgcaaccaattccgataattatcttcaaaaggttgccgacaatatcgaagtcatttataagaatgaaccgcggcagaccttggtactgtttaactcactcaatgcgattgaacggacgtatcggctgcttcaggaaagtggcttcacagcgacccattttgttttggctcaaggcgttcacggaacagccgccaaaatcagcaagcagttcatccatcatgaacccgctatcctgcttggggccaatactttctggcagggagtcgatttcccgagaaatctactggaaaacctgattgttgcccagctgccgtttgatacgccctcagacccttataatcacgcgctgtactcgattgagcgcagtaagggtaagaacccattttatagtattacgctccccaaagcgactctcaggctgcgtcagggcatgggacgcctgttgagaaccaaagatgacttcggaaccatttttattttggatcccaggttattatctaagcggtatggcagcaccattctagccaatttgcgcaacgatattcctgtcgtgcacggttcaattgatgaatgtgtattagacatggttaagttttttgaaagcagaaattaatctgcggttgagcagtcggatatttgctataattaggaataacgaaatttgagaggaagttaccatgcaacggcatcgaagagttaaaaaacaatcatacgttaaaatttcctggatcgttatctcgatcattttgattctctgcttttcgttcttcattatcctgcacacggcggagcggccgatgacaattgcccgcggccagaccgaaacgattgctaaaaagtacgccgggttaacgaaagtcgactcgttttacacctctaatttggggaagacttattattccgtttccggtgttgataacaagaacaaaaatgtttacgtcatcgtcgctaaaaaaggcggcacggtcaacgttatcaatagcagcagcggtattagcgagcagcaggccaaaaatgtgattcaacggcaaaaacacccatcaaaattaaacgggattgggctgacgatgattaagaaccagccatattgggtggtcagctatatgaacgccaagaatcatttgtgctttacgacaatcagcttcaaaaacggcaccatttacaaatcgattgaaaacatctagaaatgaaaggacacttcaatgaaattttcaaaacgggcgatgcaggtcacgccttcagcaaccgtcaaagtttccaatactgccaaggcgatgatcagaaagggcatcgatgtcattaatttgggcatcggtgagcccgattttccaaccccaaaaatcattgccgatgcagcaattgacgctattcgatcgggcaaaaccagtttttacaccccggccagtggtttaccccagttaaaagaagccatcgccgagcgcattaagcaggactacggcgttgtctacccagctgatcaaattagtgtgaccaacggtgccaagatggcgctgtacgtgttaatgcaggtattggtcgatgacggcacggaagtcttgctgccccggccaagctgggtcagttaccgccagcaggtcaatcttgcaggcggcaagccggtaattgttgagacagggacggacttcaagattaccacccaaagcctggatacagctgtgactaaaaatgctaaggtattggtgatcaattcaccgcaaaaccccactggaaccgtgtattccagggatgaactggcggcaattggtcaatgggcagtcttgcataatgtgaccttaatcgctgacgatatttatggcaaattggtttataatcaaaaccagtttgtttcgttggttcaaatcagtgacgaggttgctgcttcaacggttttggtcaacggcgtttccaaagcctattccatgacggggtggcgaattggctatttagccggggcgccggaattaatcggcaaggtaaattcgattctatctcattcgaccggaaatccagccacggtaagtcaatatgctgcgattgctgcccttcagtcggaccaatcagccgttgagacaatgcgagaggcctttgaacaacggttaaatcaaatttatccgctggtgcaacaaattccggggtttaagttggcagccaaaccgcaaggggcgttttatttattcccaaatgttgaagcggctgttgacctggcaggtcttaatgactcaggggaattggtcgatcagctgctggccaaagcccacgttgcggtggttgacggagctgcttttggcatgcccggctacctcaggttgagttatgccactagtttggaagacctggtaaccgccgttgagcggatcactgaatttatgaatcagtttttagaaaaacaagtatctggaggaatcggaattgaaacaaattaacatggttgacgcacctaagtacgttaacgaaaaagttaaaattggtgtttggttaaccaacaaacgttcaagtggtaagatcgcctttctgcaattacgtgacggaacggcatttttccaaggcgtcgtcgtgaagagtaatgttaccccggaagttttcgagttggcgaaggaagtcaagcaggaaaccagcatgtgggtaaccgggatcattcatgaagatgctcgttccaaatttggctacgagatcgaaattgaaaccatcgaggtcctttctgaaacccatgactatccaattacgcccaaggaacatggggttgacttcttaatggatcatcgtcatctttggctgagatccagccggccccacgctgttatgcggattcgtaatgaggtcattaaggcgacttatgatttctttaacgatgaaggtttcatcaaaattgatgcccccatcctgactggaagtgcgcctgaagggacaacgacgcttttccatacggaatacttcgatcgcgacgcttatttgtctcaaagtggtcagttgtatgaagaagccggtgcccaagcgtttggcaaagtgttctcatttggccctacctttagagctgaaaaatcaaagacccgtcgtcatttgatcgagttttggatgattgaaccggaaatggcattcatgcaccaagaagaaagcctcgaaattcaagaacgctatattgcttacttggtgactcgagtgcttgaaaattgccaaatggaactgaagacattgggtcgcgacccggaagttctcaaaaagtacaccgttttaccttatccacgaatcagttatgatgaagccattacgatgctcaaaaagggtggctttgatttggagtggggagtcgactttggttctcctgaagaaacctaccttgccgatcaatttaaccaaccggtttttgtgatcaactaccctaaagcaattaaaccgttctatatgaagccacatccaactcgtgatgacgtggtaatttgtgctgatctcttggcacccgaaggatacggagaaattatcggtggttcggaaagagcaacagattacgactatctctatgatcaaattgtcaaggctggtttggatcctaaagaatactcatggtacttggatttacgtaaatacggcagtgtgccgcattccggctttggtttgggacttgaacgggctctgacctggttaacaggtgaagaccacgttcgtgaggcaattccattcccaagactgcttaaccgaatttacccataaattgaaattaaacactggtttggtggattcgaggtgaattgaatggacgattatgcacgcaatctactaaatgaggggcaaactactgtcagcaactatctgttaaaacattatcatcagattggggttaccaatcaggagcttttcatttacctattgattaaggggaatcatgacctggtagttccaatgccggaaatggcagatctgcaagcacagacgaattattctgaacagcagctgttcaatttatttcatcaaatgattgaaaagaagctgaccaaaattacgcaagtagtgattgagggtcagcaggtggatgcttacgatttcacgccgatgtatgaaaaattggcattggtcaagcccacgggaacctctcctgaggcgtcagtaaacgaaaagcccaagactgttagcagcagcgaccgccaagctgtctttcaaagtattgaacaagaatttggtcgaactttgtcgccgattgagatggagtctatcagtcagtggttggatattgatcattattcaccggaattgattcaactggcgttgaaggaagccgttttaagtcaggtttataatttaaattatatggaccgaatcattagtacttggtacaagaaaaatttaaagaccccacaacaggttgaagccgccaaaaagaatcggaatagttcacattcggatgatatttcaactggttacgacggtccggaaattccgtttatcaacttgtcaggtaattcagataaataaacaattaggaaatcggctaaacttttagccgattttttcgtacatagtcaaagggacaatcagttcttcaatctggcattcagaaaaccgtaataaggaagcccgcagaaaatattggtaaacgaaaagaggccctcgacaaatgatgtgtttgtcgaaagtctctgatggactgtgctgattttattgggtttcgtcagtaccaccgttattgtcattgctattggtattgccgccaccattgtctggcgtcgtaccgccattgtcagtggaactcgatgatgcggaactactgtttgaatcatcgttaccaccatcgccactcggtttttgctcagatggcgtggatgcggatgactcgttggaactttctgtactgctggaactctcattttcccgtggttgcgtgacaactgccgagctggaacttgaaccaccttcagttgtgtagccactggtcgtttgatttgaactattatcggtgactgtcccaggataaccggcgacgtaatactcagtggtgccgccacggttggttgcgacaacgtcacttggctgggtccaatcggtgttgggtttatcttcagaaatatagcccatcacgtttttatagatttcctgggcgattgatgtttgtgccgaagtgacataggaattggctttgaattgatggtcgtatccagtccagatggctaatgaatagttcttggtataaccggagaaccaggaatccatcgtcgacatcgccggcactttgttcaaataatcgtcgggatactgtgtcgtaccagttttaccggcttcataaagaccagacactttggctgcagtcccggaacctgcagaatctgtcatcacgcccttgagcatattagtgatcataaatgcggtcgccggcgacatggcgcgtttgccttgctggtgatacttgtgggtcacaccgttaacttgaacaatcttgttgattaagtacggtttgtaataggttccgccattggcaaaggctgcgtaagatgcggccagctgttcagaggaaatgtagagcccaatcccattttgaatctcgagtggtttgctaaacgacatccccaggtttttcaaaaagccggttgctttaggaaccccaacattttcaagtgttcgaattgccgggatatttcgcgactcaaccagtgcttttcgcatcgtgatcgtgccttggtatttgttatcaaagtcatagaccgatttatcggttccaggataaacgtacggcgtatctttgaccggctggtaggtcgggtatttaagatattgaatggctggaccataatccataatgggtttagctgttgatccagaagacctgccggtttggacagccctgttcaaaccgaacgccactttggttttgcggccgccctgcatggcaacgactttaccgttattgacatcgacaatggttgcaccgacttggaaacggttgttggggtaggcaatggtcggatcgttattacttacctgataaagtttcttttgtgcactcatgtccaaattcgtataaactttcaggccgctgtttggtttgtagcctttatcctcgagttcctcaatggtctgctttaaataagaatcaatgtatttagaagtcttttcagaggttcgcgccttcgcgtgggtcgctgaaagatgggctttgacactggtatttttggcagcttgggcttgcgattcagtaatgtctttggtcttgaccatcgcatcaaggacttcatttcgccgcttggtcgcatactgaggatacttataagggttgtagagcgttggtgattgtggcatacctgccaataaagcgaactcaggtaacgttaagtgattaagcgttttatcgtaataatattctgccgccgtctgcatgccgtagacgccgttgcccatatagactttgttgatgtaaaattccaaaatttgactcttactgtaacgattttcaactttgattgccagccaagcttcctgagcctttcgcttaaaggttcgatcactggcagccgttgaaaagaccgacagtttgactaactgctgagtgagggtacttccaccctgaagacctaaagaagatccggtcaaattcgagatcgctgctccggcgattcggatggggtcaacgccatggtgtttatagaatcgtcgatcttcaatggaaacaacggcccgtttgagggttcttggaatatttttagatttaacgtagtcccgattctggcttcccagacgtgaaatcactgtgccgttggcatcatagaatttagtggagttatcactggtcagcgcagaccgggtaattcgtggtgcactggaagcgtagtacgtgaataggccggcgccaaacagaaataggacaccaaccaggattaaagcccatttgaagattcgccgaaaggggccttttttatgggtattgctaaactgtcgtccgcgccgaacttcagcgcgtgaatttttcggattgttctgtgacatagccttctccttcgtaacttattcgatgaaagaatcaaccgcgcgaagatagggtagtaatgggttaattctgtattgaatcaaaaagccttccttttcaatgacttttctgggaatggatttgcggccgccacttttttgggcgtcccaataggtaatcaagtcggtggctttcaaaacatacacggcctgatccgaaatgaatttgataatcgcaaagcagattccttgctgttgtaggcattgtcgcatatgttcaacttgatgttcatgaaaatttttgagtgggaaagactgtttattcttggtctctttggcatcaaagtcaatgtattttccgcgatatacgccattataatcagtagtggaagcacgacgaaaataagcttccttaattctggcggcacttctcttgggatagtcaacagaaacgatctgaattggagtcggcttcttatgaataactgcaattcctgcacgaagataatactgattgctcttgttgatttcgtcctctaaggtcattcctcgatttgagaagttaatcgaatcattgtgggtaccggaagaagtcggctgctcatgaaactggtttccattcgggtatctgatagtcattgaacgttagcttcctttttgtgaatagttatattgtacttcatttaacttaataataaccacaataatgttattataccaagtagagtcttcatttaaaatatttaatcgttagggtgatatcatgagccgcttgtgggtaaccggctatcgaagctatgaattaggaatttttaaagatgatgatccaaaacgaaaagtcattgatatggtcttaaaaaatgaaattgaccaggcaattgttgacggcatggattggttaatttccggcggacagttgggaattgagcagtggtcgttggaaatggccctgaatttgaaaaagacctatccaggcgaatttcagacgtcaatgatgctgccgttcgctgacttcggcagtaattggaacgaaaacaatcaaaccaagctgcagaccctaaaggcacgggtcgatttttcggcgtcagtttctcaaaagccgtatcagtcgccccaacagttaagaaattaccaagaattcatgctgagtcataccgatcaggcattattgatatatgatttagataatccagggaaatcgcaatatgattatgatcaaataaaaaggtttgccgacaaccatccatatccgtataagctaattactttcgacgatttacagagtgctgcggatgaatatcaggaaaacttgaataatagtgttcaagatgactaatttatgatattattttagttggtttgttgcaaatagtgaggtgtaacccatacatggaaaacattaattatactccgaaggatattcttcaaaaggaattcaagcaaaagatgcgtggctatgatcccaacgatgttgacggctttttagacgacatcatcaaggattatgaaactttcaacaaagaactccagtccctcagtgatgagaatgagcgattaaaagttcaagtcgatgaattgaataagcagattgcggtatccggttcgcagccaatgccatcagctggtggcactgctccaaccagaagtgttccgagtcagccaatgtcaagtgcgactaatatggacattttaaagcgcctttccaaccttgaaagacgagtattcggatcacaacttgataataataccaatgattcacacaggctttaaagcttgcatataactaatatggtgtaaatcctgagtaattgcggtcgtatcattacggctgaggaaagtccattctcgcacgggctgcgatgcccgtagtgttcgtgctcggtgaaaaaataagccgggggactctttgtgagttacggcggatattaaagctaaggcttgctatgctttaattccctaaggtgccacagtgacgaacagtattggaaacggtactgatggaacgcggtaaacccctcgagcgggaaacccaaacttttggtaggggagcttcacacacggtaaatgaaccaagtgtgggggagaagtatttcgatatttctcagatagatgattactacttgttatgtcgtcctgggatataataagcacaaaacatggcttatagggatttacaccaaacaggttgagtgggagcttgctcccacttttttgttacccagaaaatgcaggagatagataaaatgaaatttaatttaatggctacttgtgccgccggtatcgaagccttagttggcaaagaaatgcgtgacttgggatatgacgtccaggtcgaaaatggtcgggtccgattcaccggtaatgaagaagatattattaaaaccaatctgtggttgagaacggcagatcggatcaaaattgttgttgatgaatttgacgcccaaacgtttgatgaattgtttgaacaaacgactgcaattgcctgggacaagttgttgccaatggatgccgcctttccagttgagggccgttcgcgaaactcaaaattgcacagcgttcctgattctcaagcgattgtcaaaaaagcgattgtcaatgaattgagcactgcctatcatcgccacacccggttaccagaaaccggtgccgaatttccactggaagtggcaattaataaggatcatgtgatgctgaccatggacaccaccggttcaagcctcttcaaacgtggctatcgaatcgaaaaagggtctgctccccttaaggaaaacatggctgccgccctggtgatgttaaccagctggtatcccgacatgccatttctggatccgttttgtggttcggggacgattccaattgaagcagccatgatcggtcgtaacattgctccaggtttcaatcgtgacttcatttgtgaacaatggccttggattgatcatgatatggcccaaaaagttcgcgatgaggccgacgccaaagctgactatgacattgaacttgatatttctgccagcgatattgacggcaatatgatcgaaatttccaaacgaaatgccgaagaggccggcctgctggctgatattcagtttaaacaattggcggttgccgatttcaaaactgataaggtcaacggcgtgattgtcggcaatccaccctatggacaacgaatgagtgatgaagaacatgcccatgagttatacaaacaaatggggaaagtcttcaatccgctcacgagttggtcaaaatactttttaacctcggaccttgactttgaaaagtactatggggaaaaagcaaccaaacgacgaaagctctacaatggatcaataaggacggactattttcagttctggggaaagaaagttcgagatttgcgtaaattagaccaaattaagagcaaataagtcggaatatatgctaaaataagaacaacttggtgaaaagaagtgggtaaatggttaaacaagtcgcgataatcggcggcggaattattggtgcaacagacgcattttatttgagtttcctacaaggcaatgacaatattcaagtgacactatttgacgacgacacggggcaagccactaaggcagcctccggtatcatctcgccatggctctcaaagcgcagaaataagcgctggtacgcgttggcaaaacgaggggcagaattgtacccatccctcgtttccgacgctcagttgagcaaccaagcctatcagcagacaggtacgattgtgactcgcaagaaccacgatgacctattggcgctttatcaggaggccaagatcaaggagcagcatacaactgcgatgggccgggtcgaattgctggacgccaaagaggtaaaacgccggatgccattgctcacggatgctccggaaggtgtttttgtcagtggtggcgcacggattgacggcggccactttgtttccgagctgctggaacgggcggctgccaataatttggatgtcaaaaatgaacgggtttccttgacggcgaatggcgccattaacacgacagcggggcccaaacattttgatatcgtgattattgccaccggtgctaggatgcacgaatcacttcagccattggggttgaacgtgaaggtccggccgcagaaaggacaattaatcgatttaactgtcaagatgccgcataaatggcgaaatatgccagttatgatgccagagggcagtagtgacgttatcccgttcaatggcggtaaattggtgattggtgcgactcacgagaatgatgagggattcgatttaacgcctcagccagctgctcgccgacagttactcaacaatgccaaagtatttatcaaaacgctaacggacgcccaagtgagtgacatgcgggtcggcaccagagcctacaccgaagattttgcgccattctttggagcagtcccgacattgcccaacttcttgattggtggcggtctggggtcctcaggtttaactaccggaccgatgattggctatcttcttgctcaggcagtgtttgaacgggaaatcgatcactggcaggattacacaaagccggtcagccagtatattgactagattgaatgcagtgcttgaagtgccagggtatgcgcgcccatgttttgtttgtctggaatccaggtgttgaccaccgttgcgaattgattttgcagtcccagtagtttgtcgagatgtttttcgaaatgtttggcatattgtttattgagactgtcaatgacgattttgctgtcagtatagaaaaaaatcaattcactgggatcaatttgtaagtcgatcaatttttggaatccggcaattgctgcgctaaactctgcatcatgattgtccgttggcgtaatcacttgattaagttgaatttgtttgccattgttgacaatgagaatgccgatggcggtgtgtccagtatgctgattgacggctgcgtctgtatatagtttaatcatgttatctacactttctttaaggagtttatttatgataagccaaaagcgtcacttcttttatcaaccaagcccattgagcagtattatttgttggagttggacttttgtcgtctttttcattggcgtgattatctggctggaaattactcattttcagtggattacgttatttttctttgtgttgtttgcggtgatcgtctgggcggaaattcattttcgcagtattcacgtctacgatcacaaatttgtcgtcagtcgcatcacgaatcctcactggttaaccgttgatctggaccagatttcacatgttcagacctcgaaataccaactggcctttgtcgccaacaccaagatctacagcttcattttacccgccaactccgttattgagatcaaagaattgatttccaacaagtaattgctgccccgttgtcagtcgatagttatttaggagggtcataatcattatgaagagcgatgttgaaatttctcaagaaactgttatggaaccaattaccaagatagctgaaaaaattgggattgctgaagatcaaattgaacaatatggtcagtataaagcaaaaatcaattttgacccaaccactgaaaaggcaaatggcaagcttattttagttacttcgatcaatccaactgctgccggcgagggtaaaaccaccgtgacggttggattgggagatgctttcaacgaattacataaaaaggtggttctggcattgcgggaaccatcactgggaccggtcatgggtatgaaaggcggcgcaactggcggcggctacgctcaagttgtcccaatggatgatatcaatctgcatttcaccggggactttgatgctttgactgaggccaataacacattagccgccttaatcgacaaccatattcagcacggcaatcaattaaacattgatccgcgccaaattacttggaaacgggtgatggacgtcaacgatcgggaattgcgccaggtcgtcatcggtcttggtgggagaacctccggtgtgccgcgtcaagacggttttgatattactgttgccagtgagttgatggccattttatgcctggcaaccagtctgcctgacctgaagcaacggatcagtcggatgttgattggctatacttacgaccggcaaccagtgaccgtggctgatttgcacgttcaaggggcactcactttattgcttaaagacgcgattaaacccaacctggtccaaaccatcgaacatacaccagcatttatccacggcggtccatttgccaatattgcgcatggttgtaacagtatcttggcgacccaagcggctttgcattttggtgattatgcgatcactgaggctggtttcgggtctgatttgggcgcagagaagttcatggatattgtcacaccccggctgaagcagagtcctgattgcgtcgtagtcgttgccacagttcgtgcgttgaagctgaacggcggtgctgataagcatgaattgaacacagaaaatcttgaggctcttaaaaaaggcgttgtcaatttgaaacgtcacgttgaagggatgcagcagtacggcaaaccagtggttgtcgcaattaataagtttgccactgataccgaagacgaattaacttatttacaaaactatgtcaccaatgatttgaaggttactgggacgatcatcaacagctgggctgaaggtggcaaaggggcagtcgaccttgccaaggatgtcattgaagcttgtgaacggccagccgaattccacgaattatataacgatgatgattcaatagaggacaaaatggccaaaatcgtcacccaaatttatgggggtgatgggattgaattttcaaataaagccaaaactgctttaaagcgaattaaaaagttgggttacgatcaattacctgtctgcatggcgaaaacccagtattcatttactgatgacgccaagcagcttggggcacctgagaatttcaaaatccatgtttcagatctgcaactaaaactgggggccggcttcatcgtcgccttaaccggaaaaattttaaccatgccagggctgccgactcatcctgcagcactcgacatggatattgatgaacagggtcggattaccgggctgttctaaagggagcgtttattttgccagtactttatgttatcggaatcattgccttaattgcgattgatcagattgttaaacacttggtggttgccagtttggcattaggtgattcattttctgtgatcaacggtgttttgtcgattaccagaattaacaataccggggctgcttggagcattttatccggccaccaatttattttcgtgatcatcgcgattttagcggcaatcttagtgacttactttattgtgaggtactggtcaaatatgccgtatcgaattggtctggggcttttgctagccggtacgctgggaaacgtcattgatcgcatcatgaacaatcacgtggtcgacatgtttcaactcgactttatcaattttccgatttttaactgtgctgacatgtacttgacgtttggaattttgattttggccattgcaatcatccgtgaaagttgattaaggggaacaattattttgaaagagtatattattaccaaccagactggacgtttggataaagtcatctcggaacttgattcttcaatcagccggtcacgggcaaaaaatttaattgacgatcaacatctcaaggtcaatggtgagccagtcaaaccaaagtatcaagttaagtcgggggataaaattcaggtcgattcggtgcaaccgactccgatcagtcttgaaccggagaatattccgcttgatattgtttatgaagatgatgatgtgattgttgtcaataaaccacaggggatggtggttcatccttccccaggccatccggaccacacgttggtaaacgctctgttgtaccatagcccactgtcaacgattaatggcgagtttcggccgggcatcgttcaccgaatcgataaggatacttcaggattgttgatggttgccaaaaatgacaaagcacatcagtttttgtcacagcagttgaaagcccaaaaaaatttgcgaaaatatgttgctctcgtccatggacgcattaaggaagattcaggagtcgtcaacgcgcccattggccggtcaccaaaggatcgaaaaaagcaggcagttgtttcggacggcagaagtgccgtgacgcattttgaggtgttggagcgatttgctgactacactttggttgcctgccggctggaaaccggtagaacccaccagattcgagttcatatgaaatacatcgggcatccgatcgttggggatcctttatatgggccaagaaaaaccattcgtggcaatggacagtttctgcacgcccaggagttgggatttgaacacccccggacgcatcaattgatgatcttttcggcgcccctgccaccaatatttgaacaaacacttaataatttacgattaaacaacgctctaggatcttgacaatccggcgctgttttcatattctgaagtggtatagcatttttatgcaatcatcaggtacaaacgttactcaattaaggagcttttactaatgggaaagataatactagataaaatggctatgcagcgggccttaacgagaattacgtatgaaatcgttgaaaaaaacaagggtgttgaagatttagtcttaattggtatcaagacccgaggaatctttttggcaaaccgaattgccgatcggctccaacaattggaaaatgtttcgattcctgtcggtgaattggatattaccaactaccgtgatgatatcgaacacgatgccatgagcagtgatgtcaaaatgtccaataacaagattaacttttctatcgaaggtaaacgggttattttggtagatgatgttttatacacgggccgaactgttcgggctgccctttccgcggtcatggacttgggtcgtcccaagagtatcaatctggcagttttggttgaccgtggacaccgcgaattaccaattcgggccgattttgtcggcaagaatatcccaagttctcaaaaggaaaagattaaggtttatgtttcagaaattgatgacaaggatgctgttgaactcatcaaataattctcattgcgaggagtcagcatgacggaaagatatttaattttagaagatggatccgcgtatgctggaaaggcattcggatcactggcaacaacgacgggtgaaattgttgccaattcaacaatgaacggttatcaagagattatttcaaatcagatttaccataatcagattatcgtttttacccaatcatctatagggaataccggactcgaccagaatgcgtacgagtccattttgccgtccgcaaaaggtgtcattgtcagggagtacgaaaatctggcgactgaccactttaagcggatttctttggataaatatttaaaacaacacaaaatccccggaatttatgacgtcgacacccgagaaatcagacatcatctacagaagcgcggcaatatgaaagcaagcattgtcgacgtcgcggatgatcatgcttttgatcagctgcacgcgacggttttgacaaatcaacaagttgctcaagtggcaactcccaagccgtttcccaaccctgatgaaggcgccaacgtggtcgtagtcgattttggcttaaaaagcggcattttaagggagttatcccatcgtgactgtaacgtgacggtggtcccttggaacttttccgccgcccaaattttggatttggatccggatggcattgttttatcgaccggtccaggttcgccggagaatttaccaaaatctgtattagacatgattacagaggttcagtcgcaggcgccattgtttgcgatgggcttaggccatgaactgtttgcacttgccaatggcgctaaagtttcccaactaaccgttgagcatcacggcagtaatcatcccattcgggaaattatcaccaatgagatctttttctcaggtcaagaacaggggtatgcagttgatccaaaatcaattgaccatgccaaactgtttatcacccacatcgatttggtgaatggcactgttcagggattacggcacagagattaccccgcattttcggttcaattttctccagatggggcaccagggcccaaagacagtgttggcttgttcgacgactttatggaaatcatggcaagaagaagggacagcaatgacgatagatattaacaaggtcctcctgcttggcggtggcccaaccaacattggccatgaaaatgaacttgatgcagccgcttttgaacgcttgatggcgctcaaaaagaccggtgcgaagattatttacgtggataacaatccattttcggtaaccaccgaagaaattcaaccagccaatgtgtatgttcaagaggtcaattttcaaaatatcgtcaacattattgataaagaaaatccggacgccattatggcgaccactggcgggcttaatggcatgcaaattgcttggcagctggctgaaagtggcattttggcctctaacaatatttcactcttgggcatcaagccggctgatttgcggaaggtcatggacaatcagaaacttcgtgatactttaaccgaaattaacgaaaaagtcattgcctcgaaaattgtggccgatgacgacgaagccatggactttgtccgtgaggttggtttcccagtgattgtcaaaccgatgtcatcaagtcatgataccagtcggtttatttgtaataatactgacgaattagaagatgctttggacgtgagtttcaagcgagcctacatcaagcgctgctcgattgaacagagtattgtgggttacaaagaaattgaaatggtcggtattcgcgatgaaagcggcaataagctgctggtttcgggaatggaagatatggatccaattgggattcattctggggattcaatcatttttgctccaacgcagactttgattaatgaagaatatcaagcgctcaggtcagcaacttttcgcattatggatgctctgaatgtgacgggaacttgtcatgttcaattcgcgcagtccagaaccgatgccaactattttgtgaccaaggtgagtccgttctttaccagaaacaccatcttggctgccaaagcaacggggtaccccttaacgtacgtctcaagctttcttgaaatggggtacaatctgactgaaatcaagttaccgagtaaatataacaagtttctgccgttcatggagccaaccatggatcatgtggtcgttaagattccattatggccgtttagagacattacggacgttgaccagcatttgaacaccttaatgaaatcggttggatctaccattggaattggccggacagtagaagaagcaattattaaatccatgcatagttcccagttttcaccacgggatattttgcccagcgtgtcgacggttaatgatgacgaggtcattaatcaactcattcatccattggccagtcgaatattaattttaatggaagcattgcggcgaggcttttcaattgatgagctatctgaactgactcaaattgatcgtttctatttctacaagttgaatcaattattgagagctcaggattttgttgtcaataacccaatgtcaccgcaatccattgaaattggacacaaatacggttttggtgacggcatgctggctgaattatggcaagtcaacatttcaaagattcagcagttgaacgaaaactaccagaatcacgtcacttacaaggcagttgagccgagcgccggtgagatgctggaatcaaccaatattttttacagcagttatgaattggaaaatgaaagccggccatttgaagaaaagagtgctttggtgattggtcggggtgggaaccaactcggccccaattcggcagcggattattacacctcacagattctcagggcgcttcacaagtcaggctataaaacaattatcatgaacacaaatccgaatgccgtctcactaacgccacagttaagtgacaaacaatacattgagccgatccaactcggaaatattctcaacattattaatttggagaaaccagatgtcgtcattctcccagggaaccgacactacttgtctaaacagttaaaacaatttcaaaatcttaatatcatcgttttgccgccggatcaaaaagttgccacatacaatcaaaagtatgcaacaacagctgtcgatctgttcatcgaaggcgatgaaattttacccgtgacgaccatttcttttgtggggaaagatcaacggactgacctgcggtttattaacgactataaagagccgatggataactggaagtctgacgaagcaaaattgattgctgatgccactaacaaggtagatccaaaagaatggcaggggctggttcaagtcttgtataatacaactggtgattctaaatatgagatgactggcattcggcctgtacgaattactgagaccgccttcctcaccaaaacgaccgggattaattggattaacgttttggtccgtaaatacctgcacacattggatatggaagccttgcgggaagacttgaagccaacggagcacaaacgtgcatcgattatgactgctcatttccctttcagagaactccaatccagtcgcattgagggaaccactaagcaagaagtcggttcatcactatcatttaagaattttgaataagattacgacaaaagggtcggggcaaaatagtaacttttgccccgaccctttgtgtattctaaatattagcaagctaaatagtgtgataaacagctgccactgacaatgttaagaagacgctccttatatatggtgcgcattctttgtatgccggaaattgaaagcagattactcacccgcttattttcgcatctgatcaattagactttcatcaggggtgacgaacaatgtcgtttgattatcgtaaatgacataccccggtttagtaccattgggtttgcgaatatttttgactttcgtataatcgacttgtactttggcggatccgcgcgctttcgagaaataggcagctagattggcagcttccgccagggttttctcagacgggtcaaagctgcggataatgacgtgtgatccaggaatatttttggtatgcagccaggtatcacgtttgtcggcggtatgcatagttaatttttcattctgtagattattcttaccgactaaaatttctgtcccatcacttgcgacaaacttttctggtttgttaatcttttgtcgcttatttttcttctttttgttctgctcatgatcacggagataatgaccttgttccaattcgtacttgatgtcgaccaggtcttggggatcagccagttcaatttgggattgaatattttcgaagtaatcaacctcctgcttggtcagttgaatttgttcgccaacaaatttaacagcgttcttcaatttttggtatttcttgaaatatcgttgggcgttttgggaaggggattgttgatcggaaagctgaatggtaatcaatttattttcatcatagtagttgggcagttcaatgctggtcattccacgttgaactttgttgagataggttgttaaaatctcgcccttgacccgataatcatccgcattttcggtgtctttcatatcccgctggagtttcttaagcttcgtgcgattctttttaagctgttttttaacgacttgaatcagcaccgcgccttgttctctgacccggtctctttgggctttgctggcgtaaaaggcatccagcaattcgctcaatgttgagaaagtttgatttttagttgtacccggatagggaaatgcggtaaaattaatcttgttacctgcaacatggctaaaggttggctctggtgagtcgaatttttggaagaaatccttgaaattagtctcaactttctcgtccttatgcaaactagttgctaatgccaaagatgtgtcgttgcccaatccttgaattgttttccgtagattttcagctaaaacgtccacgtttggaaaatctttgatcaattggcggacccggtcaaagtcagtcatcgtaaatgggttttccaagtcctgcttcggcggtttgatataagttgctccaggcagcaacaggcgatatcggttaacgtcagaaccgacgtgtttaatagcgtcaataatcttccccgtggcttgttcgaccaggatgatgttactatgacgggccataatttcgacaaccagatctaattttgtctggtcacccagttcgttgcgcgccgtgaaggtaaacgtcaacacgcgatcattttcctgttgggaaatctcactgagaattccaccgctgagatgcttacggacaatcattgtaaagtttgtcggcacactgggattgacatatggaaccctggtaatctgcacccgggcatacgtcgggttggcagacagcagcagctgttgattctttccgtgagctcggattgttaatatgagttcattcggatagggttgattaattttgctgatccgacccgtttgcagcagatcggttaattcatttttcatagaatgggtaaaagaaccatcaaatgacatcttatcactcactttcgtataagtagcatgtactagtatagcgcactttcttgactgatgctaaggaaggcacatgttatttgtatgtcattatcaaatagcgtatactaatttttcggaggtcttttcatcatgaaagatattcttgtggcacttaattctgctgccaaaaatcatcgatctcaaatattcaatattactaaggcaatgaacctgacaatttctgaatggaagttgttaaatcaagtcattgccggcaataccacccaggaattattgtccgaaagtaccaaattggatatttcaaccttgtcgcggcagttgaagcgactattagaaaaagatatgatcgaaaagaccgcggttggtcgggacaagcgacaattgatttataaggtgactgacaagggaactcaggccagtcaatatgttgccgccgaaattcaaaagctgactgaccgggtatttaatcattggactgatgaagagaaaaatcttttaaagatattgatcaatcgtcttgaaaagagtttggatagaatttaattacgagcaggtgaatttaatgaaaattgcgatcgtgactgatagcacggcgtatttaaccaaggaagaacaagcgaaatacaacattatcgaagtgccaatccctgtcattatcgatggccgtgagtacaaggaaggtgtcgatttgacgacggcagaattctacgataagttaaagaattctcaggcctttcccagtacatctcagccgccaatcggtgagatgattgatctctacaattctttggctaaacaaggctatgacaccgtgattagtattcatcttgccagcacgatttctggcttctatagttccctgactcaaattgcaccaacgatcgaagggatcaaagtcatcccatatgattccaaaatcaccgttaagttaatgggctatatggccatccaagccagtaaaatggcccgacttgggcgcacgcccgatcagatccttacatatcttgatgggcttcggcagacaattgacgaactgtttgtcgttgatgatctgcaaaacctggttcgcggtggccgactttcaaatgcctcggcattcattggcggaattcttaaaattaaaccgttattgacatttgatgataaaagtaatgaaattgtcgcctttgaaaagatccggtcgcgtaaaaaagccctcaaacgagtggaggaactctttgctgctgccaaacaaaaagctgattatcctttgcgggcattggtcattaacggcaatgatcctaaagccggaaatgaatgggcaaataaaattcacgaactttatcctgatatgacaatcgaacaaagttattttggtccaaccattggcacccatttaggcgacaaagcattagctcttgcgtggcttcgagactttgatcaggataacatttaaaatgaactattttaacatgcaatcgcttattgttcagtaaaacacgaactaagcgattgcattttttagtgcatgtgataaactttaatagttacataaaataaatatggggtaggattcaatgcgttaagtgtcggaggaacggaatgtgaacttcgaacgaaaaatgatcggcttcgacttgtcgaccatttgcggtgttgtttccgcattcgctatgttatttagttctctaaataatggtgagctcctttataaggagatgctgcatcatgaagtcattgtcattgggttttcgtaagctgcgggttgtggatattgttgtcttgggaattttcatgtcgttattgttaattctcggtcgatttacggtcggtgttcagtcctggcggttaagtttcggcttcgttgtcactgcgattgccagcatgctgtatgggccactgtggtcatccacaatcgctgcattaacggatatcatcggcacattgatgtctgggagtgtttattttcctgggtttacaatctctgcgattttaggcgctgccatttatggctattttttctatggcaaagagatcacatggaaacgcgtgatcattgcccaattaatcattgcggttgtcgtcaacgcaattttgaatacctattggttgacaattttatataagacgccattttgggcatttttaccggttagagcgttaaaagaattggtcatgactccgattcaaatggcaattctttactatatgctgaattcccagacgatgagtaatattcagagcaggttgtttaaataaaatgagaagcgacgcaccgcaccaacatattggtcggcgggccgctttttgtcgtatacaaaggagtgaatcatgatgtattacatttcattacacaacatgcggttccacagtcatattggtgttttgcccgaggaaaaagtcgttggtcaaaatattcaaattgatttaaaagtgaaagtcgatgccgatccgactgatgatgatttgaagtcgacggtgtcatacgcggatttctatccaaccatcgccaaggtgatcgacaataatcaggttgacttagttgagaccttggcccagacagtgattgccgctattaaaaatattgattcgcggattatgactgtcaatgtccggatccgcaaacaaggaacgccgattgatggtgttttggacgacgtcgaaatagaaatggagcattagtatggaagatgtatatttaagtttaggcagtaatattgggaaccgcgaggcatttttggaacaggccatcgaggcattgggtagtgacccacggattatgattgaaaagcaggccagtctgtacgaaacatctccggttggtggtgtcaagcaacgggcatttgtcaatacagctgtcaagattgggaccacctatgaacccctgacactcttaaaggtgattcatgaaatcgaaagtggcctccatcgaactcgccaggttcactggggtccaaggaccgtggatattgatattatcttctttggcaatgaacaaattgatcaaccagggctgtcggttccacatcccgaagcgtttaatcgattatttgtgttgattccgattcaagaattaattgatgaacaatttccagacgctgaaaagattgctacggccattaagtctctccagcaagatgatcaatcaatcaagaaaatcagtccggctaataacttctacaccgaaatcaccagtaacgtcactaacgtattggcagcaattggtgacgacccgactagaaagggccttattgaaaccccggatcgggttgccagaatgtatgccaacatctttgattctatcggactggaagattttcaagactataaattgtttgactcaccggagtcagatgactcaaagacggttatggtgaaaggcattccattttattcgatgtgtgagcatcacatgatgccattttggggcaaagtcagtgttgcctatgttcctgataacggtaaaattattggtctaagtaaaatcccgcgactggttgattttgtatcacacaagttaagtctgcaggaaaaaattacggatgatgttctcagccaaatggaaaaaattctccatcccaaaggcgtggcggtaattgtcgatgcccgccatatgtgtatcgaaatgcggggcgtcaaaaaaaccggcaccgtgacccgaaccactaaatttaccggtgtcttccagcaaaacgatgagctgagaagtgagtttttgaattcaatccaggtgggacaaatatgaacgatgatttaaccagtcactttgccgaatttttatataatcaaggtgatcgcattggtttgttaaagcaagttctgcgccaattgggcaacccggatgctgactatccaatcatccatatctgcggtaccaacggcaaggggtcaacggcaacgatgattgccgcaatactccagcagatgggaaaacgagttggtttatttaccagcccgtttatcggtgatattaccaatagtattcagattaatcgccaggcaatcccaactgatcaatttgataagtatctgaatcgcctcaagcagctgatgacttcatttggtgatggacagcaggaactctctgaatttgaggccatgtttgttgccgccatgcagtacttttctgatcaacaagttgactatgtggttttggaatgcggtctgggtggggagctcgacgcaaccaatgcagtgaaaacaaccatatattcaatctttactaaaattggcatggatcatattggcattctgggaaataccattgaagaaattgcgacaaccaagtcaaaaattattcgacaagggaacacaaccattgcggcccccaaccaacggccggaagtcctggcagtcttgaaagatgaagcgagccacaaagctgccactttccttgatgccgacgcagttcaaattgatcggcaattaactaaagcaactaatgtcgtttatcaagtcggtcatcaatctggtcattttcaatttggactgccgggcgattaccaattggaaaatgtccgaaccgtgttgttgtggttggatgattttcaaaaaaagcagcacttatcactggatgtcagtcaattattaacccaagcgctgggaaagctggatgtccctggtcggtttgaaaccattcacgctcaaccgacgatcatcatcgatggtgctcataatgttgatgcgatcacagctttcgttggatccgtgaaacattcattttccagccaatccaaattgattattaccgggtttctgaaggataaagattatgtcgataatgtgcgcttactggcacagattcccaatgcaaccttcaaattaacgcaacctgctaatccagagcgcaagctggacgaacgtcgtcttcaaacggtcttccaaaacattactggcaagatttacccggttttttccgacccgatagctgcccttaaggcaagcctcaaggaatcaagcaatcaccccgatcagctgattttggtggtgggttcattttatctcatcaacccaattcgagattatttaataaagacaaggagcaattcaaatgactaattctaatgaagtccatttcaaagggaagaattttgatttcaatctgactgaaacgccgattatctattccattctcaatttaaccccggattcattttacgatggtggggtcaataccagtattgatcaagttttggaccgcatcgaaactgaaatgggctatggtgccaaaaccttcgaactgggtggcaaatcgtccaagccccattttgatgatattagtcccgatgaagagtggcagcgggtagaaccctatcttaaagcgattcaaaagcggtttccaaatattgtattggcaatcgattcgaataccaactcagtgattgaacgggcgttgcaatctggaattcagatcattaatgatattgatggctttaattctcaagccaaactggatttggttcaacaatatcaaccctcagtcgtcacgatgtttaatggtcgcaattttgacgaacaaccaacgacacttgaagacacgatgcattcatttttcacaggctcgattaaccgtttagaacaagctggtcttcaaagggagaacattgttattgatcccggggttggcttctctgatcgcaatacactggaatttgatttgattaaaatgcgttacacaaaacagatgcgccagtttggagcgccgatcatgatcgcaatttctcagaaaagttttgccaaacggctgtttgatgcaggctcagatgagcggctgatcccaacattactgtttgaagcttacatgacccaacttggtgggcgaattatccgagtccataacgtcaaagaaacccaagaattaattaaaacgtatcagatcttcaaggacattttaagtgattaaggaagtgatcaaccatcttagttgaacaattaatcgcccaaatcgtaacgctaaaaagtcagccgtatccctggatgaatacccaaaaagtgcaaacggcgatcgaattgctgagggcaaactctcaaggacttcgcgaccggaaatcgccatttcatctatccgcaagtgcgatggtctttgaaggaggcaaggggatctttatccggcatccttacctgcatacaatcctattgcctgccggtcacgttgagccacacgaaatgccgattgattgtgccatcagagaatttaccgaggagaccggtttggttttaaaaactagtccaaattcgttaatcgatgtcaacatcattgatattccagctaatccgcaaaaagacgagggtgctcatcaacacctggattttcgctactggttctcctcgattgaaccacataccaaatatcggcctgagctgccagtatttcagctgaaaaggcgggaggccccggcggagtttcaaccatattttgcactaatttgatcgttaaaatgagagattatgattgttgctatatacaaatagatgattcaaattaagaaaagactcaggcaaaaccggttattggcatatacaatcatttaaaaagaaggttcaacacaatggacaatcaaattatcaccagaaaaatgcaggcagaagattatccaaatgcttatgcattgtggcaacaagttcccggcatgaatctgcgggaatttgacgatagttttgaagaaatcagccgattattgcgattcaatcccaatttctgttttgtagcggagaccaagactgacaaacagatcatcggcagcattctgggtgcaactgatggtcggcgcgggacgatttatcatttggcagttgctccgggttatcagaatcaaggtttgggaactcaactggtcaataaagtgattgaacagctccaagctgtcggtattcataaaatctttgtcaatgtcatgaaagataatcttgcaggccaatcattttggcagcagctaaaatttgttaaacgaagtgacgtgattcgttttaataaaattatttagatacgtatcagagaagcggggtgcagactcaattttcttgatacagattctactttacataatatatattatacgaagtagacaaaaagtaaaaagaaccagctaccaaagccaacactctcggcaatggtaactggttctttactttaatttcgtgaacaattaactaacggcttcttccagagaatttccggattcaacttgagtgttcgtttggtaattatccactcgtacttttaaaacgtgacgctgaatgcgtttatttaacggtggcaatttcatatagtcaccgtacaatcgcgttaagtatgcatcataatctgctaggactggcacctgtaaattttcaaaggccattgggattaaatgatggatctctgtcggcttgattaattcttttccgtactgatacggtgatgacatgttaatcaacggtaattccgagtgaccgttatattgggtcattgtgctgagtcgaatatcgtatagctcactcaaattataatcggcatacttggactgtgtgatactttgctgatacaggtcaggataaaatcgctttcgaatctcttctaacagcattgccaactttgcttgctgtttttcctgttgcggccgtttatttggcattcgatcgaacggaaacacatcaataaaaatgccattcttagcttttgtcaactcacggccatgttccaagatccgcgtgccatcagccatcactttagcgaaatcgtattcgtactgtggatcgaggcggttctcttcaacgaagtatcctcgatgtgacaactctgccggtgcgacttgcagaaacttttcaaaatcagtgcgcggcaaaccgatgtcaatatcatcgtcccatggaataaagccgtgatgacgcacggcaccgattgctgaaccaccggttagaaaatattccagatgatatttagaattgattgctgccacatttgccagaatacccagttgaacttgatgaattaattttaaatcaaccatatttagaacctccttaatcaaaaatccgatctcatatctaaacctctttcaaattggattgttcacttattaatattaatcgattccaacattgggtcaattaatatgctcatttatgatatacttaacttaataaaatacagattttattaagttatacgcaaaaaaataaacggccccaccaaatttactgcgatttgctgggatatgattaactgaattaaggagcttaaaaatgcaatcatctcaatatattcaacaaaatcaacagctggttcaaaccctgccaacttatattaatgaatattatctcgacaaatcaacggttccattatcccccgccacgctatatcagtatctaaacgagtttcaccgtttcttcacttggatgatcgatgttgggattactgacgtgaaaactgtcaaagaaattccactctccgcgctggaacacttcaaaaaacaggatatggaactgtataagtcttacctgctgaaccgtggcaagcaaacggcttcccatccgcaagcaccaatttctcatcggacagtcaatcgttcgctaaacgcgctctcagccttcttccgatacttatcggaagaaaccgaaactgccgatggtgagccttatttttaccgaaatgtgatgaagaaaattgccttggttcccgacagcgaaacctaccaaacccgtgccaacaacatcaaggatcaacttatgttgggtgacgcggatgtgaaatacgttgaattcatccagaatgactatcccaagacactgaccaataaacggacgctatcattatatcaacgcgatcgtgaacgtgacgtggcaatcaatgcgctgatgcttggtactggcattcgggtgtccgagctgaccaatgcaaatgtctctgatttaaatttgagcaaagcggcaattgtcgtccggcgaaaaggcggcaagtacgattccgtgcccattgccagttgggtgcttccctatctggcaacctatttaaacgtccgtaagcaacggtatttggccaccaagactacccctgccctctttttgacgaaaggggcaagccaacccagaagaatttccaccgcgactgttgaactattggtggcgaaatactcccaatctttcaaccacgtacggattacaccccataagttacggcatacattggcttcgaagctctatttggaaaccaacaatgagcacttggtggccactcagcttggccagagttcaaccaatgcgactggcttatacacgcacatcattgacaccaagcaacgccaagcccttgatgaacttcatcgtgacaagcagcgtcactaaaagaattcgtgggtagattgccacagcattcctcatcgatttgttttctgatccacagctgactcatcaattgattgagttgattttaaagttttctgataggcagaccacatttttgattgaactttcgaaaatgtcatctgatcaaattcactggagtggatccatttacccggaaaatagcttaaatcaatattttccgctatttggccttccaataacttaattttccattgctgatgggtaaaggtgtgaacaaccgttggcgtagatactggatgcaacgcgacacttagttggtaatcggtctgcagtcgggtttcgattatatcaattaacgttgattctgtcaccggttggtcatcagttaaatttttgcggtcaaataaaggaaacatccaaaaattggccaggatgccatgactcgggcgtttttcaaataagtaccccgccttggaatggatgaccactccaaagtaatcgtggcgaaccggtcgcttctttttggtcttcactgggtaatggtcttcgatcccatccaaatatgactggttgaaatctttgaccggtgattggctggtatcataattggtggctgtcatgtagctggcacccaaatccataattgcttgattaaagtcgcctggtcgattctttggaacgattgggttgattattttttcaaatacctgacgagtgtgtggtttagcaacatcgtcgtcgatttctaacagcctggcaaaaacgcgaaaagcatttccatccactgccgccactggttggccaaaagcaatactggcaatggcaccggccgtataaggcccgataccgctcaattcctgaagctcttttgcagtcgttggccattggccctgataatcgaaaacaatctgttgagccgccttttgaaggtttctggcccgagaatagtagcccagtccttcccaagctttcatcagcttgtcctccggggctgcagccagatcttcaatcgttggaaattcgttcataaaccgtaaataatacggaatgactgtttccacctgagtttgctgaagcataatttctgacacccacacatggtaaggatcctgatcctgccgccatggcaaatcccgcttattttggtcataccaggctagtagcgtctcctgaaatgctttgattgtcttatttgaccatttgatcatctgacgatttctccttacagtttaattcaaaataataaagggctgttggcaaaatttgcgttttgtcacagccctttaggtgaatggtcattaatagctgaaatatccttggctaactaatttttctgccagttcttcttgataaagttttcgcgtccgcccatttcttccatttgataacggagcggatttttcttgtagaattcttgatgttcttcttctgccggatagaatggtttggcatcctcaatttgggtcacgattggactgtcaaattgttcactctcggcgagggccttctttgaagcttcggcaatttttctttgctgctcatccttcacgtaaattaccggacgataattatcaccgcgatcttgaaattggcccatggcatcggttgggtcagtttgatgccaatagatttccaccaacttatcatatgagattacctcaggatcaaagaaaattttgaccgcttcagtatggccagtggtgtggctggcaacttgttcataagttgggttgggaacatggccgccagtatagccggaaacgaccttgttaataccgggaatagtgtcaaatggcttgaccatgcaccagaaacatccacctgcaaaaattgctgtatcttccatgcattgcacctcaatttcatttattcaaataattgtttgtatttactgtatccctttgcgtccaattcggcaaccggaataaattttaaggctgctgaattaatgcaaaatcggtgaccaccagcatctttgggaccgtctgggaacacgtgcccaagatgtgaacccgcctgcttacttttgacttcttcgcgaatcatgccaaaagaagtgtccaagtgcttatcaatattggctgggtcaatcggtttggtaaatgatggccaaccacagccggcatcatatttatcggtcgatgagaacagcggttctccgctcacgacatccacgtaaataccggcttggtaaaagtcatcatactgaccgctaaacggcgcctcagtccctttgttttgggtaacatcgtattgttccggggttagtttgtttttgagttcctgcttgtccatgataaccctccattaaattaggttgtgtacaactaaactaaattcattatagtggccaaccaacccaaagtaaacaaaaacggccaaactaaccattcagattagccggaccgtttgaaagagttgatgaattagcttaatgcatctgttaatggcggaacaacttgcttcttacgtgaaacaacacctggtaatgacattgtgtcgtcactgagtttgctgttaaatgctttttcaactgcagatgctggttcgccgacaacaatcatctttgaatcgctgttcaaaacgttagtaatcagaactaagaacaagtcgtagcccttatcagcagcttcagccttcatggcattctcaatgtcatttttacgcttgtcaatttcgctgaattcaacgacgttgatttggtcaatccgaacactcttaccgcccattgtaaatgacttggcatcagaatcaatgagttcttggtccgtctttgctgaaacgttggtcccagctttaagcatctcaatgccgtacttttcgtaatcgatgtcagcaatttcagctaaagtcttgacagcaattttatcttcttcagtggtcgttggtgacttcagtaacaacgtatctgaaataattgctgaaagcattaagccggctaattgagcagggatttcaactttgttttcgtcaaacatcttaacgataatcgtgctgcagcagccaactggttcggcgcggtagtatagtggctgatcagtctggaaattagaaattcggtggtgatcaaccacgtgagtgatggttaaatctttgatgtcactgacactttgttgaaattcattgtggtcaaccaacatgacggagtcaacttcatttttagcagttttgatgattcgtggagttggttcgtcaaaataattcaacacaaatgcagtttctgaattaggttcacccaaagcaacggcttcagtatcataccctaatttgttctgcagatatgaataggcttttgcagcaacgattgcatctgtatcaggactttgatgaccaaaaactaattctttactcatttacataatctcctttgataatcaaaatttatttccctaaacgggctaaataatcttctttagcaaggaactcatcgaacttctgtaagaaacgttcaatccgcgggatttcgttcttgcggttccggtagacgaaattcagatcaaacttgactttaggatccaattcagtgacccaaatgtcatcgtcagtcaacttcttaaggtcgatattgagcatatatgactttggtaatgccgtgttggtgtgggaattaatggcaaacttcaaaatctgctcgggcatggtatatcgtgccgctacctttggccagtcaaccatttggttcttaaaggattcccgcaaagtttggttgagataataatcttgtggatacatcacccatggcctgtcgttgacatctttcaagtggacccgtttacgtttggccaaacttgggttgtggtggataaacaataagtcatccgagataatcttcttggagctgtatggcttccagttcttaatcgattcatccggcaggtacatgattgccaaatcgattcggttgttctccaagctttcccaaatctcttttctggtcagcatgtggaaattgacttccaaatccggattttcctggtaaagtgccagggcaaaatcttcaaagactttggtttcaacggaagcgaggattcccagattaatttgaccagtcgttgagctggtagcttgttgaatctggtcgttggcatcatttaacagatcgtatatttgccgggttgtcttcaacatgatcacacctgcatcggtcagccttaatttcttgccaaccgagtagaataattcagttcccattgtcttttcaagcttcttgatttgttgggtcagcgctggttgcgtaattcccaagatctgggcagcttgtgtgtagttcatcgtttctgacaactggagaaaatacgataaagtctttgatgcaaaaatattttcctgagtggttttcattcagactctccttatcggtccgtgcgaccattatataattaacaggatactgctattatgataattcttattgttaatacaatcaattaatatggtaaaaatttaatcaattgataagccgacaaactttggtctgattgaaaccggggtgccttcactgtcaacatcaattacaaatgagccgttggaatagcgcccacccaatgaataatctgccggtaaaatatcgtgaacccggcgatgatcggtccgcacttcaagcggctggtcttcgctttcaattcgacaaaagtccacaattctgtgcggattatttttaagttcccgcaggatcataacgccctttcgagcccttgaagtggcaggaatttctttaacagctaatttcttgaaagatccacgttgggtcacaattgccaagacatcgtcttcagagaccagttggaggttggtgactttatcaacacctcgaagccccatggattttacgccggtagttctggcgccattaaccggtacctcatcgatcccgtagcgtaacgccaagccattattagagataagaagcatttgcccagcagttgcgggcgtcttcaaataatgaatggccactacccgctcatcagcagttttgagcttctcataagtgtaggcatggctcttgtaggtccgtcccggcttcatatccgcaaaaccagtttgtttgacatgcccttggtcagttgcaatcaagaaggttcctggttgcttgagtgaatcaaaagcataggtgccaatgatttcctcgtcagcatccaacccgatggtctgagaaatatgctcaccggtatccttccacttcacatctgccaattcaaagactggccgatagatcagattacctttattggtgaacataaacagatgatcgcgggcatttaattcggccataaagattggataatcttcatcttttaaaccagtgtcggttgtcgaagctttgtatgaccgaatgctgcttcgcttgatgtagccgtcatggctgaccatcacgatcacatcctcgtcagggatcaagacatctgtattaatcttgatatctgaaacctcagcttgaatctcggttctccgagcgctgcgataagttttcgccaatgcgcgtaactcgttggccaaaacccgattgagttcttttggactattcaaaattttgttgtctttggtaatttcgtcggccaggtgctggtgttcgttctccaactctgtcacgtcggtattggtcaaacgatacagttgcaaggcaacgatggcatcagcctgtttttctgaaaaatcgtaggttttgaccagattgtcacgggcatctttacggttcttacttgctcggatggttttgatgaccttgtccaaaattgataaggcatgaatcagtccctcaacgatatgctgacggtcctgagccttcttcaaattgtatttggtccgcttctcaatgacttcttgctggaattcgagataggccaccaagatctttttcagtgacaaacgttccggccgcatatgggaaatggcaaccatattgaaattgtaggaaacctgcaggtcggtattcttgaacaggtagttcaaaattccttttgagtcgacatcacgctttaattcgacgacaatgctgagtccgttacgatcactttgatcacgaacctccgaaatgccttcgatcttcttgttcaagcgaatttcatcaatccgtttgactagttgagccttattaacctcgtaaggaatttctgtgatgacaatttgtgatttgttgcctttcagtggctcaatggaagtcttcgagcggacgataatcttgccgtgaccggtttcgtatgcttttttgatgccgtcaattccttgaacaattgcaccagttgggaaatcgggccccttcacaaactgcatcaaatcatccagagttgcatccgggtgcttctgcaggtaaagaatcgcgtcaatcacttctcccaggttgtgcggtggaatatcggtcgcatagccggcagaaattccagtagaaccgttcacgagcaggttgggaaatcgggatggcaaaacagttggttcgtactcggtgtcatcaaaattgaggacccagtcgaccgtgtccttttcaatatcccgtagcatttcgctggcgattttgctcaaacgggcttcggtataccgcattgcggcaggcggatcaccgtccattgaaccattgttgccgtgcatttcaatcagcggctcgcgaaccttccagtcctggctcattcgattcaatgcttcataaatcgaactgtccccatggggatgaaaattacccatgacatttcccacggattttgctgacttacgaaacggcttgtcgtacgtattgccgtctttgttcatggcataaaggattcgtcgttgaaccggctttaaaccatcccgaatgtcaggcaaggcccgttcctgaatgattgatttggaatatctgctgaaccgttcgcccatgacatcttcgagggtcaaactttcaattttactcattttttaaacgcgccccctaatcacttgtattatccaagatgctgccatcttcttctaaattaaatttgacgttatgttcaatccactttcttcggggttcaactttatcgcccatcaaagtcgtcacccgtttttcagcgagggcggcatcatcgattcgaacccggatcaaagttctggtatcaggattcatggtggtttcccacagttggtcagcgttcatctcacccaaacctttgaaccgctggaggctgtagcccttgccaaagtcctttgataccttatttaattcttcattggtccaagcatattggactttcaacttcttgccggcacccttctgcagcttgtaaaggggtggtaaggcaatgaagactctgccattatcaatcattggccgcatgtatttgtagaagaaggtcaataagagaatctgaatatgagcaccgtcatcatcggcatcagtcataataataatcttatcgtagttggcatcatcaatgttaaaatcggcgccaacgccggcaccaattgtataaatcatggtattgatttcttcgtttttcataatttccgggagttttgcccgttcggtgttcaagaccttccctcgaaggggcaaaattgcctgatatcttcggtctcggccctgtttggcagaaccgccggcggaatccccttcgaccagaaacagctcatttcggctgtaatcctttgattgagccggggttaattttcctgacagcaggcgttcttgttttttatgccgtttaccggttcgggtctcatcccgggcttttcttgccgcctgtcgagcttgtctggcacgcaacgctttatgaaccaaagtctgggcaaattcaccgttttccatcaaatagtagcccagcttctcactgacaacgttatcaacgattgagcgggcttcaggggtgcctagtttttctttggtctgaccttcaaactgaagaatctcttctggaattcgtaacgataatacgacggacagcccctcgcggacatcgctgccttcaaggttcttatccttttccttgagcatccccacttttcgggcatagtcattaaaggctttcgtccaagcgtttctcagacccgcctcgtgcgtgccgccgtccttggttcgaacgttgttgacaaatgacagcatagtttcagaataaccgtcgttatactgcgcagccacttcgacttccacgccgtcttttttgccgtcgaaatacatcacgtcgcccagggtatgcttatcttcattcaaatattgaacgaattccttaataccctcttcgtaatggaaaacgtcttcctgctcctgatcggttcgttcgtcagtcagggtaattttggttcctttaagtagaaaggcggattcccgtaatcgctcggaaagaactgagaaattgtaaaccgtgctggtgaaaatagttggatccggtttaaaggttaccgttgtcccactatgagcgcgggttttgcctaattttttcagtgtgcccaccggatggccgccgtttttgaaatcttcttcgtaacggtaaccgtcacggacaatcacaactttcagccaagtagaaagtgcgttgacaacgctggcgccgacgccgtgcagtccaccggatgttttgtagccgccctgaccgaatttaccgccggcatgaagcatcgttaaaatcacttcaggagttggtttccctgaagcgtgcataccagttggcatcccccggccgtgatcgaccaccgtgatactgttgtccttatgaattgagacgtcaatttcgtccccataaccggccaaaacttcgtccacggcattatcaacaatttcgtagaccaaatgatgcaggccacgtgaatcagtggaaccgatgtacattccaggacgctttctaaccgcgtcgagtccctcaagaatttgaatcgaggaatcatcatatttttgcttttgctttaccattcgttatgactcctttttttgcaatctacttcataataacctaaatttacgccgatggaaacgaaattttattggctgaacccaaattacatgctaaaatgagaaacgctattaagtttattaattgcgactattgtgaggtttaagatgaattctaatattgaacaaattataatgctgttagtgctagcttatttgctgggatcaattcccagcggtgtctggattggtaaaattttctttcacattgatattcgccgacacggctccggcaatatcgggaccaccaatacctaccgggttttagggccgattgccggctcaattgtcatggcgctggatatttctaaaggagcggtggcgacattactgccgacattttttcatatcaccgcgatcagtccgttgatctttggactcatggcgattttggggcacaccttttcaatctttgataaattcaaaggcggcaaggcggtggcaaccagtgcagggatgctgctggcatacaagccggctttcttctttttggcagccgggatttggattctggtgattttgttaaccagcatggtcagtcttgccagcatgatcggttttaccttaacgaccatcgcaattttctttacccacgacattttattgagtgtcatggcggtgatcctgacctttttcattttttaccggcatcgggccaatatcaaccgaattaaaaacggcaccgaaagtatggtgccatttggccttggcaatcggctgcgaaaacgtaaagatccgaatgaataacccaatcaaaaacgagtgatttctgaaataaggaatcactcgtttttagtttgaattttaatcggccgggcaattgatgcgacagctactatcagttagaagaaactaattgaatatcgaccggcaaaggcgtggcggccagccaactgattaatcgcaaatttatcttccagcttgccgtcggcattgactgtatcagccagtccccaccacggttcaatgcaggcaaacggggcttttttcgggtacggtgaccagataccgacatatggtgcattctcaaccgtgagtgaaacaccatgatcattttgggcattggccagcatcacagtcgtttcctggcgatcaaggctcaaaacgatggcatcgctgttaaacagctcgtggttcaacggcagcggcttggtcaggtcaattgcctggggatcgtttggatcgctatacggcggttttaatgggatttgaacgtatgacttctttggtgctacccgaataaaggaatcctcgaagttaccttctcctttgaccaaaggaatgttaaagccgggatgagctccaattgaaaacaacagtgtgtcttgacttggattgatgacgtttagactcacattcaattgatgatcaaccagttcgtaaatgattcgcagttcgaatttaaacggatatttggccaacgtttcctcagtgggccgtaaaaccagtgagactttggttggtaattgggattcaacttcaaactgattgtcgcgggcaaacccgtgttgggtcatttcataagtctggccagcataggtgtattggttgtccttaagtcgaccgacaattggaaacagaattggcgcatgccgcttccaaaatgctggatccgcctgccaaatatattctaatccgtcagtatctttcacggaggtgagttcggcaccctgctcgttgatgagcacggtcaaatactgatttttcaaggtaatcatttaatctcttcctcccaattttacagaatgtaacgtgaaagatctttattttgagccagtttgccaactttatcatcgacgtatttttcagtgatcgtaatatcgcccatctgcatatccggtccttcgtaaaggatatcttcaagcaatttctcaagaatcgtgtgcagacgacgggcaccgatattatcagtattgtggttgacatcagtggcgatttcggcaatccgattaatcgcctcgatggtgaaagttactttgatattatccgtcccgatcaaagcaatgtattgcttggtcagtgagttggttggttccgtcaaaatgcggacaaagtcttctttggttaaatcatttaactcaactctgattgggaaacgtccttggagttcgggaattaaatcagaaggcttgttttcggcaaaggcacccgaaccaatgaacagcatgtgatcggtattgacggtcccgtatttggtattcacctgagagccttcaacgattggtaaaatgtcgcgttgaaccccttcacgggaaacttcgccactattttgagactttcccggggcaattttatcaatttcatcaataaatatgatcccggtattttcggcgcgaacgatcgcattatggtaaagatcggccttgttgatcagttcttcagaagcctggcgggttagaatttctcgcgcttcacttacaggaacggtgcgtttgattttctttttgggcatcagtccggccaaggtatcattcaaatcgatccccatttggttcatcatcgtgctttgaccagcgggttgttgggatggatcatccatttcaatttcaacctggtcgttctccagcaagccagccttgagtttttctgcgatcgacatccgtttttcacggatatcatccgtaacttcttcttgatcgtcctgattttcagacggcatctggccattttgcatctgagtaaacatattcatcaggttctgcatctcattttggcggttctcttttttctttgccggtgccaaaagtttaaccaagcgattgttggcctgcttttctgcttcgacgtggacctgtttgtactgatcagcccgttccaattggatggcattttcgaccaggtcacgaaccattgattcaacatcgccacccacgtaaccgacttcggtaaatttggtagcctcaactttcacaaacggtgcgttgacgattttggccaaacggcgagcaatttcagttttcccaactccggtcggtccgatcatcaaaaggttttttggtgaaatttcatcctgcatgtcttttgacagctgcattctgcggtatcggttccgcaaggccacagcaaccgcttttttggcctcgttttggccaacaatatattggtcaagcacggaaacaatttcttttggtgtttgagtagactcagtcaatttaagttcctcctataattcttcagaaatcacgttttggttcgtgaaaatatcaatgttgccggcaatgtgaatggcggcttcggcaatttctctggcgctcatgtcctgagcgtgatgtttcatggcagttgccgcagctaaggcaaagttaccgccggaaccaatcgctaaaatatcatcgtctggttcgatcacttcaccttggccggatactagcaataaatctttatcgttcatcacgattagcaaagcttcgagcttttgtaactgttggtcgccacgccactcctgggccaattcaacggcggaacgtttcaggtcaccgtcaaactggtttaatttcttctcaaatcgttcttcgaggttaaaggcgtcagcgacacttccggcaaagccgacaacgacttggttgtcataaatccgacgaaccttgtgggcggttcccttcataatgactttttcacccatggtaacctgaccgtctccagccattgcgagatggccattgtggcgaacagcgacgatagtagttgcttcaaatttgattggcataatatacccctttattagtttgattttaatgaatcattatttcgaggaaaatactttttataatcattcattaaatgtgatttggtaacgtgtgtgtagatttgagttgtcgacaggctgctgtgtcccagcaactcttgaactgaccgcatatcggcaccattattgagcatctctgtcgcaaacgtgtgtcgcagcatgtggggatgaatcttcgtcgtcagactactttgtttgacgatttgatccatcagatattcgataccccgacttgtcagcggtcggccgtaatgattcacaaataaaaatggatggtcttgatggtacttggccatgattgggcttctggcgtcgctgagataagtttcaatcgcctcttgagcatattccccaaagggcacgtatctttgcttgttgcccttcccagtgactaagatggttcggttgtccaaatcgatgtcattgagctgaattccggcgcactcgctgacccgaatcccagtcgcatataaggtttccagaacagccgtatcgcgcaatcccagttggtgattgggattttgtccggctccctgaaaaagcgcccgcatctcattttgatacaaaaatctgggcaaacgccgatgattggtcttcaagtggacatattcgaatggattgttggcgatcacagtattcttcaccaggaaagcatagaacgacttcaatgccgataccttttgggcgatggaatttctggcatattttcgctcataaagatcgctcaaaaatgcttcaacatcaaacgagtccacctgggtcaatggtttgcgttcactgggaatttcggccagaaagcgggtgaattcggcaatggcctgctgataagcctggatggtatcagtagaatagtgacggtcactttgtaaatacttcagaaaccattgaatatttttttgatcttcatctgattcagccataactatcaccttcaacgatgtaatcgtgttcatgtcctaatatctatgatagcaaataaacgccgtttgtgcccgatttgctatgaaattaaccaaaactaaatccgatcataatcatcgaataagcgtcattttaccgacctgattagcagtcatcaatggattgtgctagtcttaaccagaacttaagcattgaggtaggctgaatcctgaaaatgagaatacaaaaaaactgaatcgaataattcgatccagtctaattgattcattatccacgtgaacgaagggaagctcgaatacgagcagccttaccttgtaagtcacgcaggtagtaaagcttggcacgacgaacgtgaccttgtcttactacttcgattttatcaactcgtggtgaatgaagtgggaaaattcgttcaaccccaacaccgttacttactttacgaacggtataagtggcttgaatgcctgaacccttgcgtttgataacaacaccttcgaacaactgaatacgttctctggtaccttcaacaaccttaacgtaaactcttacagaatctccggcacggaaatcaggaatgtcattacgtagttgcttcgcgttgatcttgtcaatcaattgattttgtcgcataaacaaatcttcctttcactaacattcattatcttgtctgacagcggaatgttgttttgcggcttgcgccaaaaattagtgtaacacaattattcatcgtctgtaaaggtgtttttcttgtcagtatcttttgcggcttgcttttcttcttcctcaatccgaacgtcagccaacaatttcttttgggtgctggttaaattgtgatggtcgatcagatcgggtcgccggaggtaagttcgtctcaatgcctctttttgattccataaggcaatttttttgtggtcgccgttcatgagaacttcagggaccttcatcccccggaactctgccggccgggtatactggggttcttccaagagacccgttgaaaaggattcctcaacactggattgatgattgcccaaaacgccgggaattaaccgggtaatggcatcgatcatgaccatcgaaggcaattccccgccagtcagaacaaagtcccccaatgaatactcatcggtcacgatggaacgaatgcgttcatcatacccttcataatgaccacagataaaggttaaatggtcatcatgtgacaactcttcagcatcatgctgtttgaatggctttccggccggatccatgagaatcactttgcccttaggatagccggcagcttcagcagtttgtttggtgtggtcgtacgcatccaaaatgggttgcgcctgcagcagcatgcccgcaccaccgccaaagggataatcatccacgtgacggtgcttgtcggtggtaaattcacgaaaattggtgacatctaaatcaataatgtggttctcaattgcttttccaataattgaatcgtgcatcgggaccgcaaacatttctggaaataaactcagtacgtcgattctcattcgtccaagccctccggaacatctgcggttatcttaccggcatcaaggtcaacattcgtaatgacagaatcgatctttggcagcagtaaatctttgtgctgatcgcgttcaaccacccaaacatcattggcgcccggtgagaggatctccttcacttggccaattgggttaccatttggatcaacaacgtctaggccgatgatttggtggtagtaatactcaccaggcttaagatcatcacttgagaggcttccctcatcaattttaagttctgatggctttaagtactcgacgtcattgatcgagggatgattcttaaagtgcaataggataaatcctttgtgtttgcggacaccgtcaattgtcagcgccacttgttcgtgcttgttaggcaatttagcaaaaaccgtgttgccgactttgaaccgtttttccggaaaatcagtaatcgaaatcactctgacttcgcctttcaagccttgggtattgacaattttgccaatattataataattcattcactcactcctccagctctaatgaatctcattttgaataaagaaaaaagggcctaaacaaaaccttcgtttcgcttaagaaccctattgtttcccatcgtcgacaatcagacgagctttcttttgaccctcaaccggaacactgtaaacaatggtccggatagtctgaatcacatggccatgctttccaatgattctgccaatatcttcttcgttcaacttcagatgatattccataaatcgatcggattcattatgcgaaatctcgatatccttaggatagtctaccaacggtgagataatcttattaattaaaccatcaatacttgtcatgatgataatcactcacttacttttttgagtatttagcttcgtgatatttcttcataataccggcatctgataagatgttacgaacagtatcagatggttgggcaccattgttcagccagttcatgattgactcttcttcaagagtaatcttggcaggctgagttaatggactgtaagtaccaacgttttcgatgaaacgaccatcacgaggactacgtgaatcggcaacaacgatacggtaatatgggcgcttctttgaacccatgcgctttaaacgaatcttaactgacatgcttttacctcctgtaatgttttaacgattaataatataccagtaattcgaatgcttgtaaaggtttttttctttacaccatcaaaagaactgatggattgacttgttttggccaaactgaccaaattaatggcgtgtcaatgctgataacttgtcagaattaacggcgcttcttgttctttttcttcaaacggcgtttcttattctttttcattttacggctgaactgtttcattgccagtttggacattttaccgcccatgccagtactgttcatcatattttccatgccagacatgttgcctttggaaaccttgttcatcatggttttcatttggccgaattgtttaatcattcgattgacttcttggattggtctaccggagccgcgggcaattcgccggcgtcttgatgggtttaatacatcagggtcagtccgttcctgatcggtcattgaatagacaatcgccttcaagtggtccatgtctttagggtccatgttggcgttttttaattggggattatttgccatccccggaatcattttcatgatttcatccaagggtcccatcttttgaatttgatttaactggtcaacaaaatcgttgaaatcaaaggtattctcttggattttctcggataattcctgagcctgtttttcatcatactctttttgggtcttctcaatgagtgaaagcatatcacccattccaagaattcgcgaagccattcgatcaggatagaagacgtccaaatcagacattttctcaccctgaccaacgaatttgattggcttttgagtgacggcacgaattgaaagtgcggcaccaccacgggtgtcaccatccaacttggttaagacaactccggttacgtccaaggtcttattaaatccttcggcggtcgccacggcgttttgaccagtcatggcatcaatgaccaacagaatttcgttgggttcaacggcatccttgatatgacttaattcgtccatcaacttttcgtcgatttgcagacgaccggccgtatcaatgatcacgtagtcattatggtcttgcttggcctgttcgacaccccgtttggcgatttcgaccgggtcaacatccgttcccagtgaaaacacggggacgtcgatttgctgaccaacagtctgcagctgatcaatggcagccggccggtagatatcatcggcaattaataacggtcgggcgttctgctcattctttaattttaaagccaacttcccggcagttgtggttttaccggcaccttggagaccagacatcatgataatggtggggattttttctgctttattcaggggaacggcttcttcccccatcgttttagttaactcttcgtcaacaattttgacaatttgttgagagggatttaacccttccaacaccttggcaccgttggcacgctcctcaacggttttgacaaagtcacggacgacttggaaattaacatcggcttccagtaaagccagtctgatttcccgcatggttgcccgcagatcggactgggaaacttttcccttgccacgtaaagttttcatggcgttttgtaaacgctcggttaatccttcaaaagccaattaattcaccccttattgttcttcggttgtttccaaatttttgatcattgaattcagtttgtcatcgtgtggatattttttttgaatataagcttgaatgtggtctagtttgtcgttccggtcaacaaagctgtgatacaaattcagcttgtcttcatattgctgaagaatcttctcggaacggcgaatattatcataaacggcctgccgactgacgttatattcaccggcaatttcccccagcgagtagtcgtcagcataatacagttcaatatagttggcctgctttttggtgagcagtggctcgtaaaattcaaacaaagaattgatgtagttatttttttccagttccatattgaaactcctttgacggccaatatgtcatctagcgtacagatttatataacgtcagtcaacgttaaaatacctgactattcggaaataaggcctttgaataagccgtaaacaaagtcgtttggatcaaacggcttcaaatcgccgacctgctcacctaaaccaacatacttgaccggcaggtgtaattcactgcgaatggcgaggacaatcccgccacgagctgtgccgtcaagcttggtcaaaacaattccggaaacatcagtggtttccttaaacattttggcttgggtcatcgcattttggccagtggtggcgtcaagtaccagcaagacttcgtgtggggcttcgggaatctcacgagtcagaattttcttcattttacttaattcgttcatgaggttgaccttattctgcagccggccggcagtatcaaccattaagatgtcatagtcttcttttctggctttaacaaccgcatcgtagaccacagatgccggatcacttttcgctttgcctttgacgatatccacaccatctcgttctgcccaaacattgagttgttcaattgcgccggctctaaaagtatcggccgcggctaaaacgacctttttgccttggtctttatacatcttagccattttaccaatcgtggttgtcttaccaaccccgttgacaccgacaaacatgataactgtcggaccggattttgccatgttaatggccgaattttcaccattgccggcttgatcgtacatgtcaatcaattttttaacgattacgttttgaacatctttgggcttcttggcattttgcagcttgacttcatcgcgcaactcatcggcaattcgcatcgaggtttcaaaaccgacgtcggattcaatcagcatgtcttccaagtcgtcaaaaaatgattcatcaacgtgacggaagtttgctaaaagggcattcagtttttgaccaaacgaggaccgcgacttttccaatcctttttcgtattgctgagtatttgaatctgtggctgattctgccggttctggactttcaactgatttttcaggctcagctggcatatccgactcttctgtcgaagattcctgctcagccgatgaatttggttcactaacagttggtgttggtttttgagcatcgtccggctgctttgtggtttgttggccatttgattcttcaggctgttctgtcggttgtttttcggtcttttcagctggttcatcagccggactcttagtggctttggcggactcttcaacatctgtggttgtttgatttgaagtggcggcgctttggtcgtctttggcaggtgcttctggtttgggttcggtttgttcagttgattcagtcggctttttttcgtcgtcttttttggaacgacgtttaaatatatcaaaaagtcccaatcaactcacctccgtttttaaattatctaaattaacagtaacaacttttgaaacgcctgattcctgcatcgttactccatacagttgatcggcgtaaatcatggtttcttttcggtgagtgatgaccacaaactgggtctcatcaccgaaacgctttaagtattttgcgaagcggtctgcgttaaacggatcaagggcggcttcggcctcatccaagatacaaaatggcaccggtcgaaccttaatgatcgcaaacagcaatgtgatcgctgttaaggctttctcgccaccggacaagagatttaagttgcgatagttctttccaggcggcttaaccataatctcaattccagtatccaacatatcattgggatcggtcaagaccagtttggcttcaccgccgccaaacatgtcaacgaagactttcgaaaacgcttggctgacttgtttgaacgccatggcgaacttagtcgtgatggtgtcatccatgtcgcgcatggtggcagttaaatgatccttagcatccaagaggtcttgtttttgactggtcaaaaattcgaagcgcttggaaacttccttgaattcctggatggcgccgatattcacaggcccaatttcgtcaatcccggttcgaagcattttaatttggctggcaacctgcttttcatcccaattccagtcgggattcgctaaatcatgttgatcgatctgataagtcgtttccagagtcgcaaagttggtatccagatcctggtggtttttagcagcagctgtctgggcactggtaagttcatatttggcgttattcaagttaatctgctcatcttgaatcttttgatttaactgatccaaatgatcctgtgcttcaccaacggtggctttcaacttgttttgcgtcaggttaagtgcgtgttggttggcttcggcggtcttaatttgctcattcaacgtcccggcgtcgacttgacgactgagttcagcctttaagtggtctcgctgttggatcaggcggtcccgattctgccgatgagtcgcaatctgctttttgattcctgtttgatcaacttcaagctgattcaacttttgctgctcaacgacaatcgcctctcggacttgttgcttttccgtggtaaatttttgagccgattgtttaacgtttgccagttgaacccgtttgttgtccaagtcatcattgactgcccgcaattgtttgtcgatggcatcctgacggttgaccaactggtcggtgtcagttgttccatcagactgggcagcgttcttcaaagcgagctggagggtcttaaattcacgctgcttttcctgaacagcctcttcaagtgaatggcattgatcctccaaggttgcggtctgttggcgaatttcgaacgcttttcgttgaccacgctcatgtgacgcattgattttagccagctcatccttggcatgctgaagctgacgttcattttccgtcagcttttggtccatctgagcggtcgattgattgagagcggccaactcggatttttgaaccaacaccccttggttatcatgacgactggcaccaccggttagagagccgccggcattgacgacttggccatccaaagtgacaatgcgcgtgcgctggttaatttgcttggaaatgttaattgcgtggtcaagcgtgtcggcgataatcgtggtccccaaaaggaagcctttaatctggttgagattatccggcatggataccaaatcggctgctacaccaatgaatccaagaacttcttgtgactcatgaacgatcgtcgaacttagccggcgacttttaatggttgaaattggtaacagcgttacccgccccaaacgctctttggtcagcaaacgaatggcggaggaagctgcccgattatcttcgacaatgacatgttgggcttgagatcctaatgcggtctcgatcgctttcacatatcgttgatcaatcgttaaatagtcactgactggccccaaaatcccggttaattggtttttccgtttgagaagattcgccacgccccggtaaaagccacgataagaatcatgaagatttttcaaagactcagcttttgctttggcctgctcggcaattttgagtgctgccagccaattggcctgggaactgtcgacagcctgctggtgagtattcattagttgagttaaatcgcccagctgcttggaaacatccgtcaattcagcttggctggaagccagagcagcttgtttgttagctaattctgcctgggtttgaccaaggtcctcacgcactttattaatccgctgtcgctgtgaccccagttgctgctcaagttgggcttcatcatgagttttcatggtaatttgatttttaatgtcggttttttgctgcagtaagtcgacatattggttacgcaattggtcgatttcagattcaattaccgaaacgctattcgctttttgggcttctgccagtttgtcgaagtcggcttgtttggcagcaattttttccgatagccgtttgccggcatccaccgattgggtgagtttgacctgaaaatcgtcaatttgcttgtcagtcagtttgatttgttccgaaatccggtttaaatcggcgtccttaaaagacttctcttgagcggacaactgatgcttgctcttcagcgactgaatttgttcagttgctgtcagaatttgctcgttgatttggtcgattttggcccggttttgagttaaattggctttcagtttgtcgcggtcattttcatcccggcgaacttgagcgtaaattttattaaccaagtcagacttttcactaacggtgtgtttgagctgctggctggctgcgatcaatttctgagttgccaaaattaactgctgcttttcaaactgatctaaacgctttttttgatccagataatccgttgccagactactttgctcttcaagcggtgccattcggctttgaagttcagaaatgatgtcttccactcgattgagattatcggaagtctcatcgatttctttttgggcagtattcttgtgctgcttgtatttgtagacgccggcgacattttcaataattgatcgtcgctcctcaggtttactgttgaagatttgttccacattaccctgagaaatgatcgacaaggacccttgaccgatgccggtatccatgaacaaatcggtaatgtccttaagacgacactgtttttcgtttaaataataggaactatcgccgttccgaaagagtttgcgggaaagcttgagctcatcgaagggggacttaatgaaatggtcggagttgtccaaggttaaagttaccgaggccatgcctaaagaccgtcgatcggcggagcctgaaaaaataacatcaggcatccgcgacccacggagatttttggcagattgttcccccatcacccaacggattgattcggcaatattactcttaccgcttccattgggaccaacaattccagtcattccacccggaaatttgatgagagttttgtctgcaaatgatttaaaaccgataatttcaatggatttaagttgcacactcattctccagtctaaactagattgtcgccctcggtatcaaactgttccagggcttgttgggcggccttttgctcggcgcctttcttggaatggccaattccaacaccataaagtttgccgtcaattgagacgttgaccttaaacgaacggtcgttgtcgggtccgtactcgtccactaattcataatcgatggccaccggaccgtccgcttgggcgagttcctgtaactcagtcttatgatcaaagaattccgcaaacatgccttcatcaagctttggaaaaatcactttggtcacaaatcgtgtcacttcggcctgcccttggtccaaataaaggcagccgacgaatgattcaaaaatatcacataacagcgagtcccgatcacgagcccccgccttttcttcgcccttaccgagacggatatactgattaaaatgacattctctggcaaaggtgctgaaactttgctcattaaccattgctgctcgaagtcgcgtgagccgtccttgaggcatctttggataacgtttgaaaatgtagtcggagacgatcagctgtaaaacagcatcccccaaaaattccagacgctcataaaattttaagccttcaccgcgatgctcattgacgtaagaagcctgtgtgaatgcttcatcaagcaaatcctgatcatcgatatggatgccaaaatcttgctttagcatctcatttaaaccctttatcaatcttttacctccacataaaatccagataacagtaaaaaattgaaattatatcaaacttgagataattccaatttaagattacttttattatttttgatgagccatgacaaaatcaacggcctcgttaatggtattcagcttttcagcatcctcatcggaaatttctgcgttaaaagtatcttccatatccaatacgaattcaacaaaatcaattgaatcagcatcaagatcgtttttaaaatttaagtcaccggtaattttacttcggtcgacatcaaactggtcagccaccaaatcggcaattttgttaaacacttcatctttgtccattttgataaacacctatttcataaaattaatttgctaatgattattatatcaactatttactgcttttgatactatcttttatctgctgcagttcatcattatggtcgacgacgtattgattcagatcaggaatcatatttgaggcaataatctggcggatttggccgatcgtattcttcaccgtgtctgctttgctgctgccatgtgtcttgacgaccggtgccttaacgcccagtaaaactgcgccgccatattgtgaatagtccattgaaccgccaattttgtggaaggcgtcttttaacatcaaagccccaaactttgctttagtgccgctatccatgatggtcgtcttaattaagctgagcatcgacaaagcagttccctcaatactctttaatacggcgtttccggtaaagccgtcggtcacaaccacgtcggcggccccgttgagtaattcacgggattcaacgttgccgacaaaattaatatctttgtccgctgccaacagatcatgcactttccggtgattcatatcacctttatccgcttcggtcccattgttcaagagaccgattcgtggattttcgacttggttgacgttttgggcgtaatattttcccatcaaggcatactggtaaatatttaaaaccttggtgtctgcattggcccccacgtcaatcatcacaaatttatcttgattcttaacgccgatgaccggcaaagtggtggtcaatccgggacgatcgattcctttgatgcggccaacgataaacaaaccggcggctaaaatagcaccagtgttccctgccgagaagaacgcatccgcagttccttctttaacagcggttgctgccagaacgatgctggattgttttttggtacgaacggctttaaccggttcatcacccatttcgatgacttcatcggcttggacaatctgaattcgatcatcatttttaagatattttttaatttggtcggtttgaccaaatagttggaattcaacatcggcataagcatcccgtgccaattcaattccttcaacaacttctttaggggcgtaatcgccgcccatggcgtcaactgcaattttcatatttaactcctatttaatccgtagtaatagtttcgttatattttagatactgtgataattgtacattttctggctgcttttgccagtcttgatgaaccgtaatactctgggcctcctgattggcaacttgtaaaatgttcaaatcaccaaccggatcggccactttaaaatcaggcatccctgattgtttactgccggtgatgtcaccttggccacgcaattccaaatccttttgggagaggaaaaagccgtcggtgctgctggcaaccgccgtcatccgctttttacccaactcgttttttgggtcggcaatcaaaatgcagtaggactgcgtgtcgccacggccaacgcgaccgcgaagttggtggagttgtgccaaaccgaagtgatcggcatcaaatatcagcatggtattggcattcgtcacgtcaacgccaacttcaatcaccgttgtcgccaccagaacttggaattgattgttcttaaaatcggccatggccgtatccttttcttcatccgacattcgcccatgtaggagaccaactgaatactgcggttcaaaaatcgctttgaaacggtcgaaaatcgccatggcgttcttcatatcgacagcttccgattcctcgatcaacggtgtgacgacgtacacttgatttccggcatccaattgtttcttaacaaatcgaatggcactatccgttttagcggaggtaatccaagttgtcttaattggcttgcggccctttggcaattcgtcgatcacagagacgtccatatcaccgtacatcgtaatcgccagtgtccgcggaatcggcgtggcagtcattgccagcatgttggtactatttcccttcagtcgtaaggcctggcgctggttgaccccgaagcgatgctgttcgtcaatgaccgccaagtcaagatcgtgatagtcgacttgatcctggaataaggcgtgggtgccgacaatcagattgacttcaccgtcagcgatccgcggcagcatcgccttacgagctaggccagtggtcgccccggtcaacagggcgatgttgacatcaaatttttcaaacaacttggcaaacgtgttggcatgctgctcggctagaatttcagttggggccataattgcggcttgtttgccggcactaatcgctgccaaaattgcaattgcagcaaccacagttttgccactaccaacatccccttggagcaagcgattcatttccaatggtttgcccaagtcggacaagatttcattgacaactttgttttgggaatcggtcagtttgaattttagttgactggtgaactgcttaactagatctggatcataggcaactttggctgccggatccggttttctgtggcgctgttttaaaatttgaattttcatggcaaataagaaaaattccatgaacttggcagttcgaaaagctttttgggcagcgaccggtgatgttggaaaatggatattttgaatggtatcacggaaggattccaatcgatacttggtgcgaattgactctggaatgacgtcaactagctgatcctggtattcatcaaatccaagcttgatcaattgtttaatggtattttgtttgacttctttgttacttggatagattgaatcataggtgtcgcttttttcgccgtttaaaattttcatcccttgaatctggttacgattgcggtcaaaggtaccaaaaataatcacttgggcttccaactcaagctgctttttcagccacggctgattaaaaaaagtgacgttatagatttcatcattaatttttaaatgaaaaccaagccgacttttgcgccgaccaaaaaaacgaacagttggctcgctaatcacgatccctttgacggtgactttttggccatcgacggcagttcttaaatcttttagcgataaatcatcatatcggcggggataataagtcagtaagtcgttgatggtattgattccgagcttattaagagcagtcaggcgcttttcgccgactcctttgagaaccctaaccgaatcacttaagctggccaatgttatccctcctttgtcattgatataaataaaagcttggccagtgttgaccaaacttttaggaattgtttattcaaccgaaattaagaatgggtagactggttgatcaccttcgtgaatctcaacttccagttcgtcatccaatttcaaaatgccggcctggactttttcggcagccgcctgatcagcgccttcaccgtaaatgatcgtaatggcttcactatcgtcatccagcatcttcttaaccatctgaatggccgtgtcaatcagtttatcaccaacggtggcaatatcgccgtcaacgatgcccataaattgatcttttttaatatccaaatcatcaatcttagtctcacgaatggcggtcgtcacttggccggacttaaccgttggcaaattatcttccattgccttttggttatcttcgagcgaattttccggattaaagccaagcatggcggtaatcccttgtgagatcgtctttgaatgaacaatgaccgtcggaatatcaaccaccttggcagcttgttcagccgccaggaaaatgtttttgttattcggcaagacgattgcctgtttggcttttgtattttgaattgcgttgacaatgtcttcggtactaggattcatcgtctgtccgccgctgacaatgtagttgacgcccaaactttcaaacagttggttcagccccttgcctgaagaaacggaaataatggcagtatctgaagttggctgctgggtgctgatactttcagctttttgaattggtgaagcgtcctcttggctgtcctcatcttcttcaatgatggtttcttgttgaagtcgcatgttatcgactttaacagttgccaaatctccaaactcctgaccccaggcaagcactttgccgggatgttcagtgtgaacatggactttgacaatatcatcatcgttgatcaccagcaatgaatcgccaagcttggcgagataatcataaaaggtctgatagtcaaattgatgatcaacttcgcggcctttgccgattcggaccataatttgcgtacagtagccatacacgatatcttctggatttaatttactttgaacactttgatcggccactttaatcatctgattcatttccgcatcgttaggttgatattcaccggattcagcttcgtttctgccattcaagacatcatcgaaagcttccaaaacgaataccaatccttgtccacccgagtcgacaacaccaacctgcttcagcaccggcaataaatccggtgttttctccaaagcggattgtgaggcctggtagatggcatccatgacagcgacaacatcattggtcgtagcggctgctttcttaccagcagtagcggccattcgcacaacggtcaaaatggttccctcggttggcttcataacggacttataggcgatttccgtcccggcaacgaaggcatcagaaatatcttgggcactcaaagtttctttaccctccgtggacttcgaaaagccccggaaaatctgcgataaaataacccctgagttgcctcgggctcccattagaagtcccttagccaaagcagcggttaaatcgccaacgtttgtcttgacatctttattcacatatttataacccgaagccatggataggctcatattggttccggtatctccatccggaaccgggaatacgttcagtgaattgataaaatcagaatttttatttagtttagttgcggctgcttgaaccattgccgtaaattcggtgttggtaatttctgtaactttcaacaacttgtcctccttggtcacttgcataatcagtcattcattacctgaacgccttgaatgatgacattgaccgaatttgcagataccccaagcatactttgtaggttatacttaacctttgcttgaacgtttttagatacttctgaaattttgttgccataagcaacgataatataaacgttaacttcaatttcattatcgtgttgtttaaccacaacacccttgaaataattctcgcggtttaaaatcgtgttgacattgtctctgagctgattgcgacttgccatacccacgactccgtaattatcggtggcagccccaccaacaacatttgcgatgacgttgttgtcgatgtcaactgttccaaatctggttttgattttgacggccatgtgcagcagcctccttaattttctattaacctattaacgatagttaatattaccacaataacgctaaaaaccaaagtaatcttgatgcccccaagaagactgtcaagtataattacttgaaagaaaagtattgcaatatcaatgtatgtatgataaattattctagtgtaatgaaacagactttaacactaaaatcaaagagaagggagatttgttacccatggcaaaggattttattaacggtaagcgtacccactttggtaacaaacgttcacacgctttaaactcaagccgtcgcagctggaagccaaatttgcaaaaagttcgcattcttgttgatggcaagcctaagaaggtttggatttctgcccgaacacttaaatcaggtaaagtaacccgtgtatagtaataacttggatcgatgttaatcggtcttttttattaccttcaaaaatagaggcaactctcagcagccgttttcggtgagctgagggttgccccttttttagttataacgattaatatctttgctttgaataacacacatcaccccactgccaaatttaaacctggcagtttcaccaacaaattcattgctggcaagcgacattgggtgtttaacctgatagtcattcagctggtatttttcatcaaacaaagttaaatgatccatcggtgttaacgccacgaatgccaaatattttttatcaggttccttttcaatctgataagttcctggcaaaaagaaagtaatcgtattttgcttgtcaatcattcgaattttcggtgcgtagggcttgaaccggggttccaaaaccatccacagattggctagaaaatgatccagtcggccacccgtcgcaccgtagatatcaagtcgatcggcgtgatgttcctgcaaagcgaccttcaaccccaattgggtatcagtatcgtctttttcaggaattgactggcggatatccttaatgtggtcacgaactagttgaagttctgccggttttaaggaatcgaagtcaccaatcgcgacaagtgggtcgatcccccgctcgatcaaatggagattgcctctatcgatgccgatccaatcacctttaatctgtccatttttcaattcgtctggccagaggtcaatggggccgccaaccaatagatttaagatcttcatttatttggtcgcatcctttattgctttgattcggctaacaggatcatcggcgtcaaaaacgtatgatccggcaactgccaccgttgcaccggcttgataggcacccacaaccgtgtggtcattaacgccaccatcaatttcgatgtcaaagttcaagccttcagtttttttcaactcatcgagttctgcgatctttttaaccgtttcaggcaggaacttctgaccgccaaatccaggattaaccgtcattaccaagacctggtcaaccatgtatagtactggcttgatggctgataccggcgtacccgggttgatgacaacttcagccttgacccctttgttcttgatcatctgcaaagcccggtgaatatgaggggttgcctcaacgtgaactccgataatatcggcaccggcatcggcgaattggtcaatgaaacgttccggttgttcaaccatcatatggacatccaagatcatcttggtgatcggacgaatggctttgacccacccaggtccataggataaagctgggacaaactgaccgtccatgatgtcgatgtggaggacttccgccccaccctggtcgactttttcaatatctttttgtaaattgacataatccgcgctcaaaattgaaggtgcaactttaatcataactaacttcctcactttttataatttggtttccggtttttaatgtcggtgtacaactgcagataattctcataccgactctgcatgatgtcaccgctggccacttcttttttcacttcacagtccggctcattgacatgcacacatccccgaaagcggcacttcacagatgcccgcttgaactctgggaaataactggcaagctggcggtaatcgatctccaaggtatcatacgaggaaaatccgggagtgtctgcgatatacccatcgttgacccgcaataaagcaacttttcgggtggtgtgttttccacgatttaatgccgcagaaatctcaccggtagcgagctgcaaatccggtgccaagtgattgagaagtgtcgatttgccggcacccgtctgtcccattatcacattttcttttcctgaaaacaattgccgtaaatggttcaacgaattttcatcaaacgcggcttccggcagaataacgtcataaggaatgttagcgtaggcaactgctaaatctttaaaataattcagttgtttttcagataacagatccgtcttggtgaaataaatgatcggcttgatattggcaatttccaatgcaatcaactgacggtccaataagttactggaaaactccggctgagtggttgccgtcgccacaatcgcctgatcaatattggcaatcggtggccgaaccagagaattctttcgtggcagcatcttcaatatgtatcctttgtcgccatcttcaacttggaactcaacgtcatcgccgaccaacggtgtaatttgacgctttcgaaaattccccctggcgcgtgttcgataaaccttgccttctgagtgaacatcataaaagccactcaaagactgaaaaatctttccttgtttcaattgatcacctcgataaaaaatcacttcccttacattataagagaagtgactttgttttgcagtaattattaatgtgaatcgtaggtcacgttgttatcacgcatgatcgtccgaccatcgcggaccactttgtattgaccgacttcattgccggataatttaaatggcaaggtgacttgcgtatcctttgtgatcaccatctgcttgtaaaccgtcgacaaactatgatcatggtctttgagataaatcaagaccacgttctcgttggaaccactggaactatctgtggaagcagcatcactggagatgccactttcattcaatgtggagtcagatgatgccgccgaactgttgtcgaggtacgggatggtaattttgacattgaagctcttcaattcatccgaactgtctttcttaggcccacgagaaatccaaaccgcgacgttactgccctgttgaattgattcgttggcatttggtgattggcggacaactcggcccttgggctggtcgtcagaataaacataatcaaaagttgggttaatttccaccttgttagaatatgagaccacttgagccttggtcatgccggttaagtctttcagcgtaatccgtttaacaccggttgaaaccacaaaggtcagtgtcttggtagccggattgaaccgtttgccggactcaaagtcctgttggagaattctgcctgagccaaatgaacttgaaggagcgttacgccgatgaaccgtaaacccttcgtcttccaatttctgtttgacaacgtcatattcttgaccgacatagttgccgacccgaacgcgacggggcccggaactcacgaccaaattgaccttggtgccctttttgactttggtttcttccttgggactggaactgatgacgcgatgacgatcaattttatcactactttgatatttgacactgccaacggtcaaattagccgctttaatcttggcttccgcctcggtttccaacgtcccggagacaattggcaccgtggttttcccgttggctgaaacaatcatgatgaaggccagaattattaacagcaggccgacaatcccaccgataatccaccaccttcgtcgccgctttttcttcggcggctttggtttgtcgttcgaggtaccggcaggcttttcctcacgtttggccggattggcatccgctgaggcagtcgtatcatccaatggtgaaaatggcatcacccgggttgcttcatcaaccgggttttgtggtggctgaaccgtaaatttaggttcattagcccgtgacttgtccaatgacgtattcaaatcagcagccatttcattaactgtttgataacgatcatcgggattcttagcggtagctttcaagacaacattttccattgcctggggaatgcgcggatcaaaatccctgactgaaggcattggtgtttgtgaatgtttaatggcaattgaaacggcggtatcaccgttaaatggcactttgccggtcaaaatttcatagagaataatccctaatgagtaaatatccgatcgggcagtcgccatctgacccttaatttgttcaggggacaaatagtgaatcgagccaataatcgaacgggtctgagtcatcgtatcttctgtgccggcccgggaaattccaaagtcggtaatcttaatataaccgttcttatcgaccaaaatgttttgaggctttaaatcacggtgaataatattatgccggtgggcttcactgacagctgagcaaatttgctccataatattgacaacttcggcataaggaatgggaaagttatccttgatgtatttctttaaatcttcaccgtcaacaaattccatgactaaatactgcatcccctcaacctcgtcaacatcataaatgccaacaatgtgaggattatccagttgggtcgccgccattgcttcatgctgaaagcgcttcttggctttggggttgtctcggaaatcaagtcgcaacagtttaacggcaacttttcgcttcaagatgaggtcttcggccaggtatacgtcagccattccaccctcgcccaagcgaccgataatttcataacgaccgtttaatacatagcccttattcatcggcggtcacctccgaatcgtattgggcgatcaagacagtaatgttgtccaagccgccgttttgattggccaaggacaccaacatgtcacacttagtctgtaattcttcatccattgacaaaattttttcgatgtcggcatcgtcgaccatattggtcaaaccgtcggtacagagtaaaatttgatctccaggttgggcggtatacggtttgaagtcggcggccgaatcgttgttgattcccagactcttggtaataatatttttgtatgggttggttttggcctggtctggagtgatatcaccgtgtttgaccaattcattcacataggaatggtcttccgtgatctgagtgaattgcccgttggaatagacataaccccgactatcaccaatgttggcgatcagactctgtttgccatcaataagtgtcgccacgatggtcgtccccataccatggagtcgtgtgtccgtgttggattcatcgataatcgcggtattttcttttgccaactggttttcaaaccaagtttcaattttatccagactagaaatactggtcgtttcaaaagcggctcccatgtgggtgacaaccatttgagaagcgacttcgccagcattgttgccgccgattccgtcggtaattaatgccaaaatgagcccggtttgatttttaaacgcgccgaccgcatcttcatttttgtcgcgaacttttccagttgaggattgatatgcaatttgcaaattgatcaactccgttatgatttccgaatgagggagcaaacaaagaagccgtctgaatcatagtcatcggggtagatttgaaccatcttgctatccggattcaaatgattggcagtctttgtcttcgtgatgtcaaaattagggttctcgctgataaacttggcgatcacgtcttgattttcctgtttaacaatcgtacaggtactatatgtaatagtaccaccagttttaactttagcggaaaccgcgttcaaaatttgtaactgaatctcacttagacgattgatatcagcaattgttttgtcataacgaatctccggctttcttctgaggagtcccaagccagaacacggcgcatcaactaaaattgaatcaaacaagccgtcttcaaatttggtatcgactttgcgggcatccaattcaaaagtttcgacttgcttgtagactcccaggcgagtggcatttcgctggacggttttcagtttgtttttatgaatatccagtgcaaagactttgccggctttcaaacggctggcaatttgggtagttttgccgcccggggcactgcaggcatccaaaacgttgtcatcaggggaaatctgcattgattcaactggcagcatggcactttcatcctgaatggttaacaggccgtcagtgaaaaagtcactgtgaatgatttgaccatcgttaataataatcccttcactggaaacttggctgggttcggcatcatagccgtccttggccaaatctgccagcaaatctttttgagagattttggctaagttggcacgaaccgattgctttggcgctttattcagggatgctaagattgaagccgtttttggcttgccaagttgttcgtcaagcatttctaccaaccaggttggcacactatattcaatcgatagtcgggtcttttcatcctgaatgtcatccaagtttggcatcccctgccgatccatctgatgcaaaataccggtcacaaatcggcgggtaccgtcatgtcccatctgcttggcaattttaattgtttcatcaaagattgcccgcttgggaacccgatccagatactccaactggtacatcgcggtatagagcagctctttgacccaggtttcagtcttttccggttcacgcaaaaatggccggagttgatattccagcgttaatcgatgctgaatgaccccgtacacaatgttggtgaacagtcccttatcagctggacccattgaagtagattgaatcacggcattaatctgcagatttgaatatgaaccattactggtgcgaaccaacgtcatgactgcaagttggcgtggattatttgttgtatatttcatttatttaatcacctgttggccaactttaagtgactgaccaatcccatttaagtaatctgttatttgttgttttggcttgccggcgggctgaagctcctgaatggataaaacagtgccttttcctgctgacaataataattggtgcttggttttctcaaccactgatcctggcgccatttcagtggtttgatcgacaacttgtgccccccaaattttggttcgtttaccgttgataaccgtataagcgaccggatccggccgcagggcacgaactttggcgttaaccataaacgcggtttgattgaagtccagttgctcttcttccggtttgatgttgggcgaaaagacgacttgatcctcatcttgaggcactggggagatatcgccggcgatcacttttggcagagtggctaacagcaggtcgcggcccacgatgctgagtttgtcaaacatcgtttcggtatcatcatctggctgaattggaaccgctttttgtgccaaaatgtcgccggcatccatctttttaaccatgtagatgagactgatgccggtttctgaatcaccattcataatcgcgtactgaacaggcgcgccaccacgatacttaggcaaaagtgagccatgaacattgacggccgcaattttgacggcgtttaacatcttcgtcggtaaaaattgaccgtaggctgccgtgacaatcaagtctggatgaaagtcaatgacccgctgcatctccgggcttccactgagtttttcaggttgaaacactggcagatgattggcaacggcggcttgtttaaccgggctttgtgaaatccggtgtttccggccgactggtcgatccggttgggtgacaacacataaaatatcgtatttttgatcaagtaatccttgtagaattgggaccgcgaactgtggcgttcccatgaacacaactgtcgtcaaatttatcgtttcctttcgtgattcaaattacataaagtccagcggctcattatcaattgcaatttggaggccttgacgctgctttttttgtgactggactaaaatctcgtctaaagtggcctttaactgaggttcctttcgatacttgataatgatttggtaatagtaacggttgtcaattcgggtaatcgtttttggcgttgggccgagaatgattgcctgtggggatagctgtttttttaaaaagttcataatcccaaacatctctgaagccgtttgattctcactgggagaattgccggttaacttaaccgtatagtagtacggtggatatttgccatcgtgacggacacgcatttcggtggcgtaaaacttctcgtaatcctgcgttttggccaattgaatcgcataatgatcagggttaaaggtctggatgatgacctccccggttttgtcggctctccccgagcggcctgagacctgcgtaaggagttcaaaagtccgttcgcttgatcgaaaatctggaaactgcaacgctgaatctgcgtttaagacgccgaccaaagtgacctcaggaaaatccaatcctttggcaatcatttgcgttcccagcaaaatatccgccttgtgagcgccaaattgatcaataatcgcctcatgggacccctttttacgggtggtatcaacatccattcgcagaactctggcggttggaaacatgtctttgacctgttcttcaagctgctcactgcccatgccataaaagcgaatccgtttactgtggcattgtgggcagacagttggcaccggttctttgtggccgcaataatgacaattaagagtatgtgtatttttgtgcatcgtcagcgaaatatcgcagttggggcaccgaggaacgtacccgcagtcccgacacatcaaaaaggcagaataaccgcggcgattcagcaataaaatcacttgctcatgtttgtcgaggcgaacctggatcgcatcggccaattttgtcgatagtgcactgtggtgttttgccagttcagtcttcatatcaataatcgaaacatgcggtaaagcatgctgattgatgcgatgcggcagctttaacagtgtatagacacccttcattgcccgtgcacgggattccagcgatggagtggcacttcccagtaccacggggcaattattgtaggcagcccgccatttggcgacatctcgggtttggtagcgggggttgtcggcttgtttgtagctgctgtcatgctcctcgtccataatgattaagccaatattgctgagcggggcaaatacggctgagcgaaccccaacgaccactttggctttcccttggttaatccgctgccattcatcgtagcgttcgccggaagacatcgcactatgaagcatcgccacttgatcaccaaaccggctgcgaatgcggccaacaatttgaggggtcaaggtaatttcgggcaccagcatcaacgccgtccgccccagttccagcgcgtgggcaattgactgcaggtaaacttcggtttttccagaaccggtgacgccttccaataaaaagacctgatcttttttgtggacgaccgcctgttcaatcgaatcgactgctgcttgttgatcaggctgtaacttaaacggctgactgggggcgacatctctgagaaatgggttgcgaacatggcgcttcaatgttgaagtcacccaccccttcttttcggcagctttcaaagtggcgctggtcactccaagggacgcccatttggaaactagcagtgtatcgttttgatgggtcttgagcaggtttaacaattgaatttgtccacgagcatttttccgtacggttttgagggcgtcagcaatctgggcgtcatttaattggcctcgataagcttttcgcataattggccgggcgtggttggtgagatcatactcaacttgaatatcgccggctttctgcagatttaaaatctctgctaaaacctgattattatatttctggcggtcatattcgacttctggctgtccttggaagatttccggatactgctggcaaacttgttcatttttggcaattagtttcttttggttcttagtccgcattccacctgggagcatggtttgtaaacagctgattttaaaggaataggtttgatcagccagccactcagccaagttaagtaactcagaattaacgactgggtataaatcaatcaggtcggcaatcggtttgagcttgccgttgaagctggaactgtcggaaaggccaaccacaaacccagtaattttgcggttgccaaaagggacctggacgcgcatgccaggttgaatttgatccgctaaatgatctggaatcgaatagctgaacggactgttggtttggcgtgctgggacgtcaacaataacttgagcaacctgcaaggcagattctcctttcactgattttgcatttgtgtagcaataatattgattaactgatcggcaacctttgccttactctcgacattcgtcttaatttgcttgccggcagcaaataaaaatgtcacttggttgttatcggcgttaaagccaatcccgctttgggaaacatcgttagccacaatcatgtccaaattctttgattgaatttttttggtggcgttgctgattaaatcattggtttcggcagcgaagccgatcactaactggccagggtgtttgatagtggcaatttcttttaagatatcgggattcctaaccagttccaaggtcatggtttgattgtcagctgtttttttgatttttttattggctaccttggccggtcgataatcggcaacagcggcggccattaccaaaatatcagcgtgaacaaaggcttgtttgacctctgctaacaattcagccgccgtttcaactcgaatgaaattgacgccggatggcggggtaatcaacggattagccgcgatcaacgtgacattggcaccggcatttttgaaagcgttggccactgcgaaacccatttttccagatgaatggttggttaaatagcgaaccgggtcaagtggttcacgggtccctccggcagtgacgacgacagattttccggctaaggatccacccttcagctttaagctttcatcaacccacgttaaaatttcgccgggttccggcatccggccctttccagaatagccctcggcaaggaagccttcagccggctccatgatttgaataccggcttgttttaagttggcgatattttgttgggtggcaaaattggcgagcatatgagtattcatggcaggcacaacaaataccggcactgccatcgttaataatgtggaagtgacaatattatccgcaatgccattcgccaatttggcaatcgtattcgcggatgccggggcaacaattgccaaatcagcatcatcagcagtcttgacgtggggaatgattgtcggatctttactgtcaaaatcgctggtcaggaccgtattcttactgacagtttgaaatgccagtggtgtcacaaatttttgggctgcttcactcataatgacgtgaacatcgttgtggttcttcactaataggcgtaccagtgacagtgatttgtagacggcaatgctgcccgtcacaaatacggcaacgtttttgttttgaaacatttttccaccccgtttcagatttcattctttattgtaccaaatctaagacggataaaaacagtcggcgtcttaaaagttggctgcaccccagtggaaaaggcgattaactccaaaatgatccccccggattgctaacgccgagtttcggccgggatcacaagataagctgataacaggattggctggtatcagcttgtccaacaaagacaaagggactgccagcaaaacagtcgttttgccgcagtcccttaacgatcaatcttattcaaaatcttttgctttaggatcgattttcaatacaccagcagcaatttcttccaaagctttgccgactgatttttgtgatttgtagtgatccaataatggcttggcaccggcatccaattcatgggcccgcttactggaaagcgcaattaatgaataacgggaatcaattttatctaacaatttatcaacagatgggtaaagtaacataattatttatctcctaacattgactcataatcgggcatcacccgagcaacttttaatcgttcacttctaataattgacttgattcggtcaacagccaaaggaacctggtcgtttaagacggcgtaatcatagttacgcatcatgctgatttcgccgacggcctttttgatgcgcttattaatgacatccatcttgtcagttccacgaccaaccagacggtgttttaattccattagatctggcggagtcaaaaagacgaagaccgcatcaggaacattggcgcgaacctgcatggcaccattgacttcaatttccaagaaaacatccttgccggattccaaggtctcgttaacatattttaatggcgtcccatagtagttgtcaacatacttggcgtactcgagcatttcaccattctgaatattctcttcgaactgctctttggaaacaaaataataatcgacaccgttcttttcaccgggacgcggctttctggttgtcattgaagttgaatattcaaaatcaacatcaggctcctcaaacaacgccttacgcaccgttcccttaccaactccggacggtcctgataaaacaatcaacattcctcttttagccatcgaaaaaatcccttcaattatttgtaatacctgctattatcgccctttttgccccatttgacaagtcctagggcactgattaagaaatttgcatttgggggttgcgttttagaacgaacgttcgtataatgaaactacaaacaaatgttcggggtgaacaaaatgcaaaacaaacaatcatatctctcagaaattaccaagacctttcgaaccaactatgatcgcttcttcgaaattgtccgtaacactcaccaaatcaaacaaatgccgactttccagctgaattatttcattcaacagacactcgaaaacaacttccccatcacgatcgaatttaacgatcaggataatgaacagaccggctacttaaccaaactttccgcagaccgttacctattgacttcagatgataatcatttcactcgaattgtgaagttgtcagaaattaaagcgattcgtaaatactaagattatatcagattatattttagggcttgagacaaaacattcagttttgtctcaagcccttttgcatttttatgatttatctgggtaaacagtgcgtccaacagcagtttccaagtggatagcggaaactaatcatttatttttcgacagcacttaagatgctttaatcttttgtttttcctcatccgccaatttcaacagctcactggcatgttccttggttaacttggtaattgccgttccggaaagcattcgcgagatttcagcgacactttgggcggttgtcagttccgtaatcgtcgtggttgtccgattgtcagcaatctttttttcaataaagtcgtgatgatcactcatcgcagccacttgtggtaaatgggtaatacataaaacttgagatttttgtgaaatcgtataaatcttattgccaatcgcctgggcaacccgtccagaaacgccggtatcgacttcatcgaaaataattgatgtgacaccagcagccttggcaaacatggtctttaaagccaacataatccgggacaattcgcctccagaagctgacttgaccaatggcagcattttctcaccaggattggtctgaatataaaattcaactcgatctgcacccagccggtttaaagcacgattttgctggatattgacctcaaagaccgttttatccatgtaaaggtcggataactgctggtgaacggctttttcaagctttttagcccaccggtggcgaatgtcggagatcttagttgcctgctgaattaaatcggatttgagcgtggctaattgcttatccaaatcgtcgctggcttcggcatcccccgacatttgtttcagttcctgtttgattttggcaagatagtccaaaatttgactgaccgaatcaccatatttgtgcttgagttgatagatggtgttgaggcgctgctcaacttgatccaaacggtcctgatcaaattctaaattactcaattgatcggaaatctgactggcaacatcttgaagcgcgaagaaagctccggatagattatccgaaatttgtttatattcaggatccaaatcttcaatgtcctgcatcgaactcattgccgatccgattgaatcaattgacccgctggcctcctcgtcgccgttaatgccttcataactggctaggagggcatcatgaatcttttgaaaattgttcaaccggtctctttcagcgactaaatctgtgtcctcattctcatggagatcggcagcttcgatttctttaatttgaaatttgagcatatcaacccgttgtgcccactgcttctcattttgatgtttcttttgatttagatcgcgcagcttaataaattgatcgtattggtcttgataggattgcaacacatcggccaattcatcttcggcatagtcatctaataattgaatgtgccgttccggccgcattaactcctgatgatcattttgaccctgaatatcgacgatcgtttcgccgattcgtttgagggtggcaatattgaccatgattccgtttacccgacagctgttgcgaccattggcaaaaatgacccgctcgataatcacgttaccgtcactgtgatcaattccaaggtcatcaaggacgttgtaggtggggttatcatcatgaaggatgaagtttccctgaataacggctttggaagccccggtccgaatgagatcatgggatcccctgccgccaaccaagaggccgacagcatcaatgatgatcgactttccagccccggtttcaccggttaacacggtcattcctgcctgaaaatcaatatctaagtgttcaatgattgcaaaatcggtaattgatagttcgagtaacatgttttcaacctctcaataattctattcagttcccaacatactattgatctgattgcgcatattaatcgcatcggcttcggttttgccgataatcaagaccgtgttgtcatcgccgagggtgccgaaaatcccgctatagttcatctggtacatcaaactagaaatgaccggtccactaccaggtaagactttcataaagaccaacttgtcttgagagtcaaccgacacaaacgaatctcgaatcgattgaaccagtttcttttcagtatcaatatttttttgcgtcggcaaactgtatcgatacccaccggtaactgaaggtactttgacgagctgcatatctttaatgtctctggaaacagtggcctgagtgacttttatcccctgcttatccagtagcgagacaaaatcttcctgtctttgaatattattacttgtcagtaattgtttgattagcctttggcgttctttcttacgcatcattacacccccaacaataaaattgaataaaaatacaggtttacgaaccctttaattcagaataagcgttctcgataactttttcaatcgaaacatttggtgacatgactggttgatcatcagattctaactcaactaaaaattcaatattgccagcgccacccttgatcggtgagaaatcaaggttttgaactgaataaccgttggccacagcaaagttcaaaatcttttccaagaccattttatgcacagcgggatccttaatgataccatgcttgccgacgttggccttaccagcttcaaattgaggcttaatcaaagccaccacatggccatttttagtgatgatctgtttcagcggtggcaggattaactctaaagaaatgaatgaaacgtcaattgaggcaaactcaggctgtccatgggtgaaatcggccaacttactgtacctgaaattggtgtgttccatgaccacaacccggggatcctcccgcagtttccagaccaattgattactgccaacatccagcgcatagctcaatttagcaccgttttgcagcatcacatccgtaaacccgccggttgaggagccaatatccaacacggtcagccctttaacattcagatgaaatactttgagggctttttcgagttttaacccgccacgactgacgtacggcattggcttgcctttaaggtgcaggtcggtatccaccggaattttggttcccggtttgtccaaccgttcttcgttatcaccaagaatctcacccgccatgacggcacgtttggccttttccctggtgtcgaacagcccttgggttactagtagtacatcgactcgttgcttttccatattacttttcgtccttatttttaaaatagcttgtgaaatcatttaacagactggtatcaattgataacgcttctctggcggttacgagggcttgctgggcatcggcgaccgtctgattcagcatttcatatgattttgccaaaccaaccaaattgggatacgtatttttattagcgtcctggtgaaccggtttgccgatttctgcttctgtcccaacaacgtctaagatgtcatcgtaaatttggtaagcttcaccaaacttctcagcaaaggttaacagtgacttgcgtttttccggaataacccggcccataatcaggccagcttcaacggcatagcgaatcaaggcaccggttttgttgcggtcaagtttttgaagccctgacaacgataaccgggtgccttcaaattcgatatcgtcggcctgacctgaaaccatcccatgggggccggcagctttggcaagtgccaaagtcagttcagcttgggtttgactgtccaaatcattatccaccagccactgaaacgccagtggttggaggccatcaccagcaagagttgccatcccagcaccaaatttgacgtgattggtaggctttccccgtctgaggtcatcattgtccatagccggcaaatcatcatgaattaaagaataagaatgcatcagttccagcgcacagctggtttttaagacggtctgatcgattgggtcgcccaaactcgccaataccgcaagcgtcaacaatggccgtaagcgtttccctccagcgttgactgaataactcatcgctgcttccagagtggtctgatccgtatccggtttgatgtcattttccaaaatctgattgatttttggaacccacaaccgttcaaaatcagttagcttggttgccatcgctatcatccttttcatctttaggtgcttcaaattccacttcattgccatctttgtccatcattttggccatggtgtgttcggccttggttaaggtgtcttgaagctgttcactcagttgaattccggctttaaatttggccatcgactcttccaaggaaacgtttccctgttccaattgattgacgatggtttccagttggtccattttttcctcaaaggtttgattgtcttgtttatcaggcatattatttctccttctttgcatttatctgattgacagaagcgttgacgataccgtcactaaaatggacatcaattgttttgctgctcaagtcggcaacccgtttaataaaatgtccctgttcgtctgtggtgtacgtataacctcgactgagaatcttcaacgggctcaagtggtcaagtgagccgaccaacatctgataatgttgggaaacatttttcaggttctgagttgttgcccggttgagtcgacctttgagtgttgccagtttttgctgctcttctctaatcgtatatgttggcgcgaccaaacgcaggcgcaatttaagatcagaaaaacgatcctttcgtttaccggtaatcttgtcagattgattatagagtcgctgcgtcagtagatccaaacgttgagcaaaagtttcgtaaatccgttgaggtgtcgtgaaaacagtggactgccggagtcgcttcaatcgctgcttgtcttgctgaacaacctggtaagtcgcattaatgatgcggttttgggtcgtcctgaggtcaactaacacttgatccaacctgggaactgccagttcggcagctgccgttggtgtcgcggcccgaacatcggcaactaaatcagcaattgtggtgtcggtttcatgaccaactgaggaaatgactggaattttactggcaacaatcgctctggcgacgttttcttcattaaatggccacaaatcttcgatcgatccaccaccacgcccgacaatgagggtatcaaaattaccaatttgattgacccgctcaatttgtcggacaatgtctgcactggcctcggttccttgaaccagggcaggaaacaggacaatttgggcaatcggatatcgacggcggacagtggtaataatatcacggataaccgcgccgcttggcgaagtgacgaccgcaattcgtttgggaaattttgccagctgctgcttgggcaaattgaataacccttcggtggacagtttttgtttgagctgttcgtaagcttggtatagctgaccaacgccgtcaggttccatctgttccacatagatttgataacttccactgggttcatagaccgaaatatggcccacaactaaaactttcatgccttcttcagggatgaattttagccggttgaaagccgatttaaacatgatcgcactaattttcgcgtgatcatccttcaagctaaagtattggtgggcattggggcgcaatcgaaagttggagatttccccagtgaggtataccttagttaaatacggatcaacatcaaattttcttttaatatattttgttaaggcgctaacggttaaataatcattcgccacgttcaaggctccattctgctaaatcaacagtttgctgcatcaaagttgcaattgtcattggaccaacaccaccgggaacgggtgtgatgtaagaaactttgtcaaataaatcatcatagtcggtgtcccccactaggtgcccttcttcgttaatattttgaccgacatcaataatgacggctcccggtttaacatcgtttttagtaacggtatgaagactcccggttgctgaaacaatcacatcagcgttcttagtatattcagtaatatcttttgttaaaagatggagaattgaaaccgaagcaccagcatttaacattaaagcagccattggtttaccgacaatggcacttcggccgatcatcaccgcgtttttccccttcaagtcaatgtgatattcatcaaacattgtcatcacacccttgggcgtacatgcaactggatacttggttgaatcatttaagtataattttccaacgttaattggatgaaaaccatcgacatctttttcaggcaaaatggaacgggtgatttgtttttcattgatttgctttggcagtgggtcctgcactaaaatccctgtaatcttgggatcctgattgtactcctgaaccactttcagcaactcatcttgggtaatggtatccggtaattccctgacaattgaatagattcccaatctaacggccgtccgatgcttatttctgacatatcgctggctggcaggatctgtgccgacaatgatcacaactaacccgggagtgattccgtgttggttttggagttgttttacccgttcgctcgtctgtgcgtttaacttctttgccaatgcttttccatcaataatcgttgccatctagaaaccgctcctttatattttcatcgtgagaaatcatatgtacaaaaaaatagatttacacatgtgtaaatctattttaccagttcttctaaggcatgtgacaaaatcccgttaacaaattttcgtgaacggtcgtcactaaatttttttgcaagttcgattgcttcattgattgataccttggcaggcatgtcatccacataaaccatctcgtagatagcaatctccaagatgattaaatcggttcgggcaattcgctcaagtgaccaactggaagctaaatacttttcaattgtatgatcgatttcagacttgtgttccaaaacgccagaaataagttggtgcaggtattctgggtagtcgtcgccatatttaccgctcgtcaaaacttggaagaaatccttccaatcagtttgatcgttggtatttaaggcaaacagtgtttgaaacgcaatttctctgatctggtgtcgtgttaattccactattcctcaccattttcttcattgtcagcgaacggattattcggatcaaccgtactggtggttttttccggaatcacgccttgaacatgcacgttaacttcggtgactttcaagccggtcataaacaacagctgctgttcgacttgactttgaatttccaatgcaacttttggaactgaaacgccatagttcaagtatacatagacgtcgatcgttaattcctcatctgtgtatgtcaaattaacgcccttaccgtgttcttttcttcttccaagtaattcattgacactcgttgaaaatgagccacgcatccggttaacgccgtcaatttgcgatgcggctaccccagcaataatttccaggacattgggtgcaatctcaattttgccaagttcgggatcatttgaatgaagaatgatattcgtgtcttcagccattataaagcctccgtttcagatcaatcggctactatgcccgtgaaatgtaagttccatcggtggtattgatagtcaacttgtcaccctggttaacaaagaatggaacttgtaatgttaatccagtcgtcatagttgcgggttttgaaccacccgaagcagtatcacctttgataccaggttcagtggaagctacttcaagaacaacggtattaggtaattcaattcctaaggtttcgttgccgtattgaataacttgaacttccatgttttcttgtaaataattcagttcgcttttaatttgttcagcaggaattgaaatttgatcgtaagtatccatatccatgaagacatgttgatcaccatcagcatacagatattgcattttgcgcgtatcgatttgagcctgttccatcttagcgcctgaacggaaagttttttcttgaacagcaccggtccgcaagttcttcagctttgaacggacgaatgcgccacccttaccaggcttaacgtgttggaagcttaaaatccgccaaattgcgttatcgacctcgatggttaaaccatttttaaaatcagcagttgaaattgccattgttgttcctcctaaatgtaatgtaacataaatagattatataatactttcggtcaaaatagccaatgaaaatggcattctgatcctgagcaattaaaaagccgggatgcaaaacacgcgttttgtcccagcctctttaattaaactattgtgcttactttgcagcttcagcaactggataaactgaaacctgacgcttgtcgcgtccttttctttcgaaacgaacaactccatcaacgactgcaaacaatgtatcatcgttaccacgcttaacattgttccctgggtaaatatgagttccacgttgacgatagatgattgatccactgtgaactgatgagccatcagcagcctttgtacctaaacgacgaccagctgagttacgaccgttggcagttgatccaccacctttatggtgagagaagaattgtaaattcattgctaacataggtttacacctccagattaattgatttatttcgctgtgtttaacttaatatacttactataactttcggctatatcagccattccgttcgcaaaagtattcaaaactgcatcagcttgaatgcgcttctttgaatcgctaacaactggtacattgactgataaatagccaccattgtcatcgtcactgtcgacatcgacatccagtccaataacctcttgaagaccgttaaccgttgtgatgcttaacacagaaacagcagaacagacaatgtcttgcccatattcacccgcatcggcatggccggtgatggtgaacccacttacatgaccgcgataacgtttaatggtcgccttaatcatatcagtcacctcaaagtaaattatgccttgattgaatcaataacaaccttggtatatggttgacgatggcccttctttgaacgtgagcccttctttggtttgtaacggaagatgataatcttcttttgacgaccctgtttttcaacagttccagttactgatgcgccatcaactaatggtgtaccaactttaactgaatcgccaccaaccataacaacttgatcaaaagtaacctttgcgccttcttctgcgtctaatttttcaacgtagattgcatcgccttcggaaaccttgtattgcttaccgcctgtagtaataactgcgtacatatcttgtgcacctccttataagtttgcttagactcgccgagaacaagcgctccgatcactatcgaagacttatcagcttgaatcgagcggttgtagctgtggaagccacaattacaacgttactagtatacataattggcaggtgttcgtcaatagaaacctgatcccataaaaaaacaaccgctacccacggctgttttatttacgttgagctaaatgtctgccattggctcgcgtggtggttgaagaattggtaaaatactgaataatgccactaacgatgaaaatgaagacaataaagattacaaatcccacaacgtccacctcctaattgttgtgacagcagattgctgcacaactacattatccagttttgtcagcgaacgttcaaatttttgaattcaaccaactcaaattttaataaaaatgcaactttcttaaggaattcataatcatattgacatctttgccctaaaagactgattaaacattgactaccctgttaatatttcatataattgttattgttgatttgtcgcaatagctcagctggatagagcaacggtcttctaaaccgtaggtcgagagttcgaatctctcttgcgacattctgacatcacatcagacatttagagatgtttgctgaataccttcaattcctattttaacgggattgaaggtattttttatttacaccactatttacgccgcactctaggaaatgtcaaaataccagtccgcttacttagtgttatcaaaacggccgaaccgaagctgaatctcttcgtttcgaccgtttcttattatcttcaattaataatcctgatcctgccgatcttcattaatcttgtttttatctttgaaggcctgttcaatctcctgctcagtataaccgaaatcaaccaagccaaatttaagaaacagtcgccaggaatggctaaagctgtcaccgctgtgatcaaagtaagcgtcaaacaacatgcgttttaaggctaaatattgcttatccaggttatcttcttttttgaactgtttgattttgtccagatcatcctgcgagtttaaaatcacgtgattccaatttttgaggttggaaatcaataggtagaaatccattgcgtcaacgtactcgtatagcaacgtttcccgcggcgttttgttgggatcgtgcttaccacgatgcgtcttccagaccttgaaccactcggaagtgttggccatttcagccagttccacgtccagggccacaaaggcatttttcactctgccgtcatttgaccagtgaagttgcttctttgattcgatctggcgattcaaatacaccgatgaagcaatcaatgattgtaaatccatttcaaactcctatccaaaaataaacttgttcgataaaatttcgagctgctttttgttatccaaataccagtctttgatgaacgggtaatccaataatagattcagccagctttctttttgatcctgatcgtggatggttgctccccacttgggccgatcttcatcaccggcgttataaacgttcagctgggtatcgttatccaaggtcaaggaggccccaccattttcaccagacatcaaaatatattggttatcagccgacttaacaaatagctcgtccaaaatcggctctggaattgcgccggcagcgaattcatagaactcaccgttaacgccgtccaagacgttaaagtcaatcttaaagccgaagctttctttgagcacttcagcagcccgcataatcacgttcatcgcatctttaagagccgaaacgtccaagccctccaaatcaacgacaaagtaatcgattaaggccgacccatgaaacatcatttccttactcttcagattcaagtagaatagcggtcggttatgggccgtggggccaaagaagaatccggcagcattcttggtcgatttggtaaaggtaaaggtattatcaccaagtgatgaaaatttagccagcagcttttgaacgtgttcagagttgctaattgaaagtccatcggcgtggtcagacaacttcaataaccgttcaaagaataccagctgaacatcttcatcagaaaattggtgtggaaattccacaaaatctgaattgagttgataattggtcaacgaaacagctgcagtcaacaattcatcgaggtcctgggtctgatttaggctggtaaatgcattgacatacttggacccattgtccaatccggcttgaattgactgagtatagtgattcaaaagttcagtcgtcgttaaaacattcttttctgtttcagtattttcattactcaccgtcagtcacctgcgattctttgctcaagctttgcaagtatttggcgtataagttgttattgttctcaataaatgcttcaaaactgccaaatgaagctcgaatattttgtttttccaaattgtaaatggtctcttctttggacagcgccaaaatttggttttcattctttttgatttcggaccgggcgcctgaagcttgttcatcaatattcgttaactcaagcagagcgttttgtaattgctgatgctcttccttaaccttgccagcttcccaaggcattggcgacttctcttcattttccttgatctgtttgcgaatctcttccttacgctgatcgcgtttggtttgatcttcaatcaattgagtcagtttttcattcttttgtcccagttcgcgcatttgatcgtcgtttacccgtttgttttgagcttcaagttcaaatgatttggccaaggtattatattcatcttcagcaaaattgaatcgaacgttaattgtatccaactccccaaacatccgatggtcccaccagttaccaaagtaaatgttgaatttccccaaatcatattcgtggtaatagaagaatggataggtggttcctaaataatcaatgagtttgtcactcaaatgatgacttaactgagccttcagatcagtggccaggccaaagaaattagtctccggctgatcaggctgttcacccttgacttctgttgcaaagcggttgggatccatcaattcgtatacttttaaatcattgccatttttgatcgagtcattcaaatccgacagatattttaccttttcgcttaacgcggaagctaaaatcgagtcgttttggctgaatggatcgttttcaattttgttatccataatattgcctcgtattccccttatttatacatttaatgttatctgaaaaacgtacataaataaagggctaatcgcatttatttatgaaagatttgtcaaaatgatgagaaaacaatccattcttttgaaaattcggtgaaatcacaaaaacgaccagaccatcataatgggttaatgatgacctggccgcccctgtattcgattgttttcagttgaaagtttgactttctttttccatttgcctatatggagttgtcaaaccgtcccgtgtcgctgcatgataacttatttgacaatgtagacatttttatagttgtacgttgctccggccgtattgtaaataatgcctttcaccttactgctcaacaggtttttacttgctgattgatatagcggtgtaatgccctggttgtccagtaagatattttgtgccttggtcatgtcctcaaatcgcttgtcagcgttcccagcatcggtggttgaagatgccttaatcaacttgtcatactgcttgttcgaccactgtgggacgttgcttgggttgccagacgttaggatgtttaagaaggtaatcggatcggcaaaatctgcgtaccaatcacccatcgtgacttggtaattatgtgatttctgtcgtgacagcaacgtttggaaaggaatatttcttaggttcaccttgagcccaggcagattcttttctagttgcgactgtagatactcactgacttgtttttgcgcgaattcgtcagaactgagcagtgtaaagctcattttggtgatccccagttctttgaggccggctttccaaagtgcctttgccttggttgaattataggttaaagaatccggtttggcagtggtggctgtaaaatctttgccggtcttaggattaattgacagtcctttggaaacaaaactttgtgaattaaaggaaccgtctcctaaaatcttcttggttaactggccgcgatcgatggccatcgaaattgcttctctaatttttaaatttttgaacagtttcttcttttggttgaatgccaggtagtaacaactcgaagtttctctggtcaccaaattcttattgttcttcagatttttggccaaaacaccagataagccaacgtattgcagcttgtcggtcttaaattggttatagccggtcgaagggtccttagtcacttgatagtggagtttgtccagtttgacagctttcttgtcccaataattttgattcttggcaagcgtccaagtcatcccggttccgttccagctggttagcttgaacggtccattgtagaccatatccgcactcttcgtcccgtaattgtcgccaaacttctcaacgaccttttggttctgcgggaagaacaacgggaagcccatcagcagtttgaagtacggaattttcttttccagggttacgactagtttataattgccgtcagctttgattcccagtgtattgggtgactttttgttagcttggatggcatcagcattttgaatccctgaaaaaagataaccgtactgagaggccgttttgggattaacagttcttcgccaggaatacacgaaatcttttgccgtaacgggatccccattgctccatttagtgcctttacgcaaattgaaagtatattttaacccatcatttgaaattttagttttggtggccagtgcattttcaattttgctgtccttacccagacgataaaggccttcatcaatgttgtttaacacttcaaatgtttgaaccgacgtcgttttggaaaggtcaacagttgagagttccgaatcaacggcagtggtaaattcctgtttggccgccagtttccccgaaccgctcttttgcgatgaacaaccagtgagaattaaggctgcggagatcactaaccccacttttaagccaagttgaatatttgacataacagacaccccttcatgatctatatgagactgaaatacattcaattataaacacattatattttaatgagagataatcggtataaaaagggctcacagcagtacaccatcgtgcaccaccatgagctctttgaataatcgatcacgctcttacaagtgcggcaaagttattttaacacactaatacttttcaagatactggtcacgttcccaaccggaaacttgcgtgcggtatgaatcatattcaaggttcttagcttcaataaagctactgtagagatgttcgccgagggcctttttcatcgtttcatcagctgaaagatccttcaatgcgttatgcaaggtatcaggcaggttagtgatatggctcttctgacgttcttcagcatccattcgataaatgtttcgatcaatgctgtgttcgggttcgatcttgttgcgtaggccatccaagccggcttccaagacacaagcgattgccaagtatgggtttgcagttggatcaactgagcgaagttccaaacgagtggaattaccacgagcacttggaattcgaatgagcggcgaacggtttgaaccggaccaggcaacgtagacaggggcttcgtaaccgggaaccaaacgtttgtaagagttaacgattgggttacatacagcagtaaaggaacgggcatgcttcaagaggccgcctaagaagtaataggcttcttgagaaatttccaactcgccatccttgtcgtagaaagtattgcctttatcgttgaataatgacatattcaaatgcatccctgaaccattaataccactcaaaggttttggcatgaaggttgcgtacaagccgtacttgcgggcaacggtcttaacaaccaacttgaatgtttgaatattgtcagcagcagccaaggcatcagcgtacttgaaatcaatttcgtgttgaccaggagcaacttcatgatgggcagcttcaacatcaaagcccatttcttcaagggtcaagacaatttcacgacggcaattttcacccaaatccattggggccatatcgaagtaacttcccttatcgttcagatgaagggttggttccccattttcatccatcttgaacaagaagaattccggttcaggtccaatgttaaatgaagtaaagccggctttcttcatgtcgccaagaacacgaatcaggttattacgaggatcggctgcgtatggctcgccgtttggacggtagacctggcagattactcgagcgattttaccacgatcagtactccatgggaaaatcatccaagttgataaatcaggatacaaatacatatcactttcttcaattcggacaaagccttcgattgaagaaccgtcaaacatcaatttgttatcgagtagtttctccaactgagtgattggaacttcaacgttcttaattgtcccaaataaatctgtgaacatcagacgtaaaaacttgacgtcctcgtcttttaccatcttgcgaatatcatcttttgaataatcatgctttgtggccatctatccatcgctcctatcaatgatttagtttgtttaaattgttcaaattattcggatcatcaaatgacgaagaaggcggcttcaatccaccaatgttaagaaactcgtcttgaagaatctttctaacatcactgtcagtcaaacctttctcgagattacgcttccgctcgtcttccaattgattctgcttcttgtacacctctttgataccagagatattcagaccgtcgtcaagataatctttgatttccaaaagccgatcgacatcattcaatgaatacatccgtcgattgccttcattacgaagcggcttaatcaattcctgctgttcataatatctgatttgtcgtgctgtcaagtcagttagcttcatcacagttccaatcggcagaactgacattgaacgccgtaattccttctctcgcattgttcacctcctaaatcttgtacccataataccattcccataatcaaagtcaagactaaatgtcacattttataacatgaatttattgattgttgtcatccagccatttttcaacgtcgctttcaatctcagttaactgatttggtcgctgaaccaggttataccaatttggttgcggttcagttttgttcctaaaccaagttaattggcgcttggcgtaatggcgtgaatccttcttgatcagctcaattgcttcttccaaggtcgattggccctgaaaatacgggaataattcacgatagccgatccctttgccggcttgaaattgctgtccgtcatggtcgaacaaccagcgaccctcggacagcagtccctgcgccatcatttgatcgacccgctgattgattcgctggtataacaacgcccgatccgtcgttaatccaatgacgaaggcatcgtattttgatccgacattatgctgatcagaaaatcggtgaccggtgtttatgtagacttccaaagcccggacaacccgcctgacgttgtgaaccggaatggcccttgctgcagcaggatccactttggcgagtcgttggtgcagtgccaaatcccctttttctttggcttcagccagcaattgtcttctcaagtcatcattttgatactggtcgccaccaagctccagcccagataaaagtgcctgaaggtaaaaaccggttccaccgacgattatcggcagcttgccggcctcgtgaatggcttcaatcagttccgaggcatcatgaacgaaatcggcgacagaaaaacgttcgtcaatatttctgacatcaattaagtggtgtttgacgcccgccatttcttcctgggtaattttagctgtcccaatatccaagtgtcgatatacctgcattgaatctccggaaataatctcagcgttaaatttttgagcgagtttgatcgacaaatccgttttcccaacggcagtcggtccgacgattgctaaaagtttgatcattccactccctcccgcatctctgacctgatctgaacagctctggcgggatagtcggtgatgatagcggccagattgcgttcaaaacagtactgcatatcctcagtggaattgacggtccaaggacgcaaattttgagcaggggcaaaaaatggatgtcgtttaagccaacgaatgtcgggatggaaatcggcaattaaatggtccttcttgagggttttggcctgcttagcggcagttttgaacaatttggcaccggctaatttaggatccagccggttgagaatttcaagtgaccgggcattaaagctggagtaaatcagctgaaacgggtagtcgattgaggcaaaatagtcaaaaaccgctttttcaatccctggatactgaatcttgttggtcttcaactctaagttaaaaatccccgtgaagttgtctttaattaataattccaccacctcttggagcgtggggaccgtggttcccttaaattcactgctgaatcgaacacctgcgtccaaatgtttaatctcagccagatttttgtcaacaattctgccagaaccgttggtggttcgatcaactgtttcatcatgcataataattaactgatggtcttttgagaaatgaacgtcggtttccaggccgtctgccccatcgtcaatggcggtttgaaaagaaatcagtgtattttccggtcgggttcctttactgccgcgatgggcaataattttggtattgattttcacaataaactcctttttgaacgattaattaatcaattaactagatatctatgaaaaaataaagcataatgaaagtataaacgagtattggagggtttagatatgaaacagtttactaatgggctcattgttggtgttctcggaaccgttgctgctggggttggtgctttgctgacatttaaaaagtcagtggtggatccaatcgaagatgaagagcaaaaattcgaggataaccgaaaaaaggcaatgcgtaagagccgagctgcccaccacggataaaacattatccaatccattacactaataacgattataaaaataggactatgaacaaaacgaatgctttgttcatagtcctattttatcaataattactctttttttccttaccattccaaccttgataaccactttttaagatataaagatctttataaccctttttgcttaaaaagagtgcggctcgtttgctgatcgttttgccttgatcatacatataaaccggcaagtctggacgaagctgactgtaaaagtttttgatggttgagtaaggcatgttgcgagcacctaaaacatggccgtctttaaaacttttttgttctcgcaagtcaatgacctgagcttttctcatgcctttttgaaactcatcatttttcaaatacgttgcaacctgtttaacacgcatattttgaaaaatggtatagccaccccatgcaagtaaaataacgatcaaaatgatggttgtcaccagattggcggtgattgcaccgattatcaacaaaaacatccctctttctctcaaataatttgattatttggttccaaatggttgattatttctaaattgcaaggctaatgatgcggcaccaataattccggcgtcattaccgagttgagccaacttcaaccgtgttgagtcacgaacagaaggaaaggcgttctcttggaaataacgagtcgttggctgaagcaaggtgttaccggcgttggaaacaccgcctccaataatgatgttctccgggttcaacgtgttaccaatgtgtgaaagtgccaatcccaagtatgagcagacccgatcaacaatttggttcgccaagatatcaccgttatcagctaggaagaagaccatcttcgatgacaaatcttcgtcgccatcaatcaattctttaatccgtgaatggccggtaaacttcttggccatatctttagcaatatggacaaccccggttgctgaagcgtactgttccaaacagccgcgctttccacaggtacattgatatccattagggacaaccgtgatatgaccgacttctccggcaccaccgttaataccatgaaccagcttgccattggcgataacaccaccgccaacgccagttcctaaagtaatgaagacgacatcttttgctttgtcgccggcacctttccaatattcaccaagagcggcgctattcgcatcgttgtcgatcagaattggtaaattgagattggctgaaatggttgctccaaccggttgcacgatgtcccagttcaagttatatgctccaacaactgttcccttttcgcggttcacagcaccgggagttcccatgccgataccataaaaatcacttgcgttatagtcgtcttttctcatttgatcactaattgatttgatcatgtcaggcacaatgtgactgccgtgttcactaatgttggttgggattcgccacttcgtcaggacgtttccttttgtatcaatgaatgcaaatttaactgtcgttccacccaaatcaattccgattaatttcttagccaatgtattttcccctactttcttgtttttcttcaattcgatgttcccgcgttaaaatcagtttggcatgaataaactcatcatgactgatcagcttggcatcatggagatggtccaactccaacgccatgacttcaatgtcccaaagtcgtttgccgacatatacataaatatcgaattttttcagcagctgctgaacatcatacagcgttttcattatctcacatcctcatgtaaatttctttcattttcacaaaatttaaaattttgcccgcatacctattgtaaacaaaacgagagcgattacaaccagcataattgccgaaataattcgtttggtttggctggtcttggaaaaaccgacgcccgtcacatacgccacaaggaatccaccaaccagtccccccagatgcccagcaatatcaatgccggaaacaaaaatatcggttccgatatttaggacaataaacaacaggaatgttttggccatcgaaacaattgccgggtttttggaaaaactttctcccagcatcataaaagcaccaaacagtccaaagatcgcagtactggcaccggcagacaagctgtctgtaaaagcaaaactgcccaggttgcccatgattccggaaacaaagaagataaccgcaaatcgccagtgtccaaacaattgctcaacgtactgaccgataaagtataaggtgatgccgttcattaagatatgagtgaagccaatgtgaataaacattggcgtgatcaatcgccaatactcgccagcacggatgagtgggttgtatttagcgccaaattcgaccaaggtgacggggttttcagttccgcccattactgacatgatcgcaaaaaccaccaccatgatgattaatagtccatatgtgatataaggctgatttcgtaaattactcatgaacccctcctgttatccgtttagtaaatgagtttgtcgactttaacatcaaaatcttccacatcccagacgggttcgtcaaatagttgaaccggtgtcaccaaagcgatacttgtgccggtaaagcccttcaaaaagcgatcgtaaaagccgccgccaaacccaactcgaaagtgatttttagaaaacgccaatcccggtaccagtaaaacatccagctggctttttgccagcacttgaccgccaacgggctcaatcgtaccaaatttggtctcactgagtaccgtatcaggttccagcagcacaaaggtcatctggcggtgcggaagtgttcggggaactgctacttgtttatcatgggttaacgcccagtgaataattggctgggtatcaagctcatcatccatactgagggtgatccccagcgtctcactattcgcaaagtgtggctcggcgaataactgctgatacaagcgttgaatttccggcttttgttgtggatcttgtaaaaagtcatgaagccgagcgatctgctgatctcgcagggcggcttttaattggttacttttggccatttacctcacccgattcttcagtcaaatctaattgacagactctgttgtatataaaaaaggtttgggtatttacccaagccttatttggtttctcgatgtaatgtaactttacgctcgcgtgggcaatactttttaagctccaaacggtcgggattgtttcgacggttcttgctggacaagtaagtacgttcgtggcattcagtacattccattgtaatgtgtactcgcatggaatacgacctccaaacttttatagagtagctagtctaatagcctcaacttaaaatattttatcatcaatcctgataaattactaggacaaaatcgataaatgttaagtgtttttacttaacagtcgaagttgattggaccgtcttccaataagccgagtagatttgtttggccagcgccatgttattactttcagcgttaacccccaagttaggcattgccaaagcaaccaccacctgtggatgagtcgatggcgcatatgaagctaaactcagggtaactgtttcgttgccattataaaatgtctgagcagttccagttttggcagaaatttccggtttgatggaatccaacatcccaccggtcttgtaggtgttggttccatgaaccacccgatacaagccggttgtgaccacgtttcgttgcgcttgagtcatatcaatatgattgagtacctttggcatcactgtcgctttaaccgttcctaatttaccatctgggctggtgccgcgaattgcttgaacgacatgcggttcaattcgattaccaccgttggcaatggtagacatgtactgagcaacctgcatcgttgtgtaggcatcgtagttaccaaatgaaagatccaaggcacttccaatgtgcttatagccgctggcaccctgtaacccggtagattcaccagggatatcaatcccagtcttgacacccaggccaaattggttgaagtaaccgcgcatcgtgttgaagacgttgggactcatggttaatgcgccaccttcaacatagttgaagtgaccttctttcatcgctaactgcatcatataagagttggaagaaacttgcagcgcatcactggcatcaacggcaatatttgcatgaccgttgtggttgaaccaagacgactttttaacaccaccggtcgtaattggctgatcggttaaggtactgttcgttggtgtaatgacatgatccatcaatgcaccggaaaccatggcacccttgacaacagaacccataacaattgagctgttaatggttcctaaaatattatcagtgatcttggaagtcttcggattgcggtcaacccctgccattccgatgatggccccgttattcggattcatgacgaccgcataagttccggttgaattaccaccggcaccggactcggcagaacggactaaggattggagctgcttttggaatttggcattgattgtcaattgaaggttgtcacctttttgaccgccatatttcttaatttcctttttgatctgattatcgctattcaaaatgatttgggtctgggatttggttccccgaagaaccggttcatattggcgctccagataactttgaccgacactgtcgtttcgtgagtaaccttgtgccaataattcattgacccgatcacttggcagaccactcttttcattcgagacagttccggtgattccctgaattgaacggccatttggatagttgcgactccaactggttccaacattaacccctggcatatcggccagatgttcccccaccatggcaacttctttagtagaaacgttgtcatccttaatattaacggtggataattggtaggcaccactcatcttggcaaatatggttgcagcatttttgagtgctgatgaaaaagtggcatttggataactctcaaccttattgacagccttgtcgtatttggcatcctcagaataaccggaaatcccagggatcgacttttcgactttggctagattatctgtatttgccaaataataatcagccagctggcgcttggttaaactgccggttggaacagtcacatattgggctaatcggttggcggttttgtacatgtccgaggacaacacattcacgcccttggtataaataattgcttggtgcgcggaattgccgactaaaacgtgtccggttgaatcaaaaatcattccccgctgaacattcccgttaactactgaggtgtctgatcggttcacttcggctttaaatttagaaccgtacatcacctgtaaatacgccaactgggtcagtaatgcaacaaataaaattccgacgataataaaaataatgttgattcgaaaaggcagtgaaacagcctttgctttgttcgttttcttggtgcgctttttaaaaattttcacgatattaactccttgccatgaaacttattctatcaaattttccaactaaaaactacaaccggtagtcaatctttaacttattatgatattctatatgttgttaatcacttttaaaaaggatgtagattatgaattcaaagaagacaacgaaaatttccatattagtgctgtgctttttggtaccggtgctaatttccaccagttactttattttccgccactttgctccgtttggcggctcgtcagttatgaccgttgacttgggtcaacagtatattgacttttataccaatttccatgacaccctcctacatagtccaagcggctttttcttttcattttcaaaggctcttggaggcgacatgatgggaacttgggcttactacttaatgagcccactgaacttgattatgttgcttttcccactttctaaattacccagtgtcttgggcatcatcacgattatcaagtatggtctggctggtttaagttttggctatttcttgatgaaagttaccaaacacgttggctggtcaatcattggtttctctgcttcgtatgcgatgatgggctggatggttgccaaccaattcaacatgctttggacagacgtgttgttcgttttgccaatgattttctatgggctcttcaagatcttgaaaaatcagtcgagtgccatctacatcatcagtttaacggccatgttgattatgaattactacatgagttacatgatcgccatctttttaaccctcttcatgttcatttactgggctgccaaggcattgccggtggaaaaccaaacatcgaccaaaaccgttctcaaatggcttaaggcgtcaattctgagcggtattttagctgcctggctgctgctgccgacctttttctcgcttctgggaagcaaaacccaatattcaaagggccaatacaaaatcaagtttgaatataacccactggacatgttgggcaagttctttaatggatcagttaatttcaatgaactgcctgccggaacagccaacgtctttgtcgccagtgtcgttttgatcctatttgtttactacttctttattccaaccatcaaacgaaacgtcaaaattgccaatatttcgttgacagcatttatgattctatcaatgtgtttccaaccactggatctgttctggcacggtatgcagctgccggtttggtacactttccgtttctcctacctcttctcgttttggatgattctgaccgcctttcaagcctttctgcatatcttggatgaaggcatcaactggaaaggttatctggtcactgccggtatcatggctttgggcgttctttacgtcgaactccgctggaagcatctcgaatacatgcgccacttcgactttctctggggctgtgtttatttggtcgtttcccttgggatcgttgtcttcttaggcatttatcgcagaaacattgttctggcgatgaccttggccgtgctgatgagtggtgaaatggcccttaacatggtcacctcactgaatcatcttgattatttgaaggccagcaattacacccagtttgagcgggtgatgcgcaaacatgtcaataaaattaagcaaaaagataagggattctatcgattgggaaccactttctcgcggaccaagaacgatgccttcactggtaattacaatggcggctcaatcttctcgtcaaccctagaatccgatacgtctcagttcttcaaaaatatcggtcagccaaatggggattcatttgtcctttactcaaacggaaccatgtttactgattcattgttgaacatgaagtattacatgagtcaccaaattccggaagctaatccgaacaaaaaaccaaagaagcagctgttgactactttgacaagaaagcctgattataacaattacaccttgttgtcacaggacgccttgattggtacctaccggaatccgtatgcggtcccgattggtttcctggcgcctaaatccggaatggaacataattcaattgccaagagtccgattacttaccaaaaccaaattgcccatcgtctggatccaaacatcaagaacttgtttgaaccagcaacttacactgacatgcggtataacaacattcaaccgatttctcaattagataatgctgtcttgaagaaaaagaacctcttggaaatgtcctacatcattttctctgtcccaattgagaagaacacgtcttactacatgacgttgggaaccgaaatcaataaaggcaacatttcaatttcggttgatggtcaagcgcagactcaatttacaccatctgaaaaaaccatcattgctaacattgccacaggtaccagcatcaataccactgcaaatgttcaaatctttgtcaacaagaataacgccctcttacaagacgtgaaattgtacaaagttcataattcaaagattgctcagttctctaaggacttaaacgccaagccgtataaagttacgaagtggaaccaccatcagttaaccggaacagtggacgtcaagtccaacaatcaagcattaaccacgaccattccatttgagaatggctggactgctaaggttgatggtaaatcagttaaaccaaaacgctgggcaaagatgttcctgtatatcccaatcaacaagggtcaccataaggttgtctttacttactggcctgaagggctgagagtcggcctactaatcactgcttttggcttagcatttatcggcaccgaggcaacgttgaaacatcgtaagaaacaaaaagccaagcacactgagacaccaacaaataccaaataaattgcatgattaaagggatgaaaaccattttggcttccatccctttttgattggttacgtttatttatcaagatccccattaggtgtgtatgtgtacacaacattttcaggatctttttctggattaaaatcgactttcaaatcaaagccgacaaagaaccagcggtcatcttcgtcaacgaaataagtaattccgtccttttcagttttggtataagtctcacctggatgatcatcgcgggttaacgctaacgagaagccttcatggacgggagttttcccataaacctttccatagaagcgcacaccattgccttggcttaaccccatttcagattggaaccatttgcttgcggaatcagttacatcaattttcattattatgccacactcctaaaatctgtgtttgtattcgcttacaatcgattataacatcattaaggtatttcacaaacgatatgcaagccgattagacgctaacattgttcatcaaggggctgttcacctttcaaaacgtgacgattgcgggcttaatttaacttatcaaaaaagaactaaccgttgagcaaagatgctcacagttagctcttttcacatactaggttatttgtaatatgcaagtagctctattcaaccttagtgattttaactttcatggttccggccggaatgggaatattaacttcttcattgagacggtgaccaatgagccccttggcaattggtgaatcattggaaattttacctgacattggatcagcttcggccgccccgacaatttgatacgtttcgggatcttcatcaggcaattcttggaaggtcactttcttgccaaccgttacctcatccttgtcactatcatttgaatcaatgatttgggcatattgaagcatgtgctcaatcgttgtaattcgactttcaagcatactttgttcatctttagcagactcatactctgagttctcagataagtccccataacttcttgcaattttgatacgttcaaccacttttggtcgttggtttactttcaagtcttctaattctgccttgagtttatcgcgaccatcggcagtcattggatatgtgtcttcagccatttggtaatttcccctttttatctttatattgttgaatcaaggttattcttaatttctttgttgccacgccgcatcaaaatggaacgcattttggtcgtcagcaaatcaatcgcgacttggttctccccaccttcggggacgatcaaatctgcgtaacgtttggttggctcgacaaactggtgatacattggcttaacagtcatcaaatactgatgaataatgttatccagtgaacgaccacgttcttttgtatcccgttcaattcgccgaattaaccgaatgtcatcatctgtgtcaacaaatactttaatatccattaaatcacgtaatcgcttatcgtcaaggattaaaattccttccaagatgataacttcgcgcggttcttgatgaatggtctgctgactgcgggtaaattgaccatagtcatagaccggtttttcaatcggttcatattgcagcagttgcttaagctgcttaatcaacagatcaaaatcaaatgccatcgggtgatcataattcacctttttgcgatcggccatcttcatgtcagcttggtcattataatatgaatcctgttgaatgatcgtgatcgaataattggataattggtcaaaaatcttgcgtgcaaccgtggtcttgccactaccggatcctccggtaatgccaataacgactggccgtgttttgtgatttaccatgtaaatagatgccctctcaattagttgttatcggaagtatgcgctgcaatttgctgctgatgttcagcatacgtctttgagtaatatacttttttcgttttggtattggcaacgaagtacagatagttctttgaacgatccaaaggatgcaggacagcgctcattgaactaatgcttgggctgtcaaatggtcccggaccaaatccggtatacttataaagattgtatggcgaatcactctgcagatccttgttcgtcaacactttgttattccggtgaatggcatacaaaaccgcgacgtctgattgtaatggcatgttgatatcgatccgattcaacaatactccagccatcttccgtcgatcggtctggttgacaccctcccgttcaatcaatgacgacaaggtcatgaactgctgcatgttcatcccggattttttaatggcagcaaagtgcggcgaaaccatctgattggtcttggcaaccatttggttaaccagtgacttcaacgatgtattcttttccacttcataagttgcaggatacaaatagccttcaagtcggtatcgaacgtttttggctttcatcgccggattaagcagcttcggataacgactggccagttgttcaaggtatgtctgattcttcattaatttcaagaaatctccacgatcgaagtcagttgtcactgaaatctgggtcgcaatttggtcaatgttggcgccttctcgaatcaaaactttccccttggtgctttggatcggttgatcagtcccgccgcgttgaagccgtttggcaattgttttgaggctcatcgagggtttcaattgataatatccagccctaaagttggccatgttattggatttgacataataatcaaagaccatgccacttttaacaatttttttattttgcaggatcgaaccaatttgcttgttcgaagcgccaagcggaatgtgaacctgagtgacgttagtgttctgtgggttcagtggctttaaggcatcttgaaaataccggtagcccatcagcccgattgttgcagctaaaataaccagtaaggtaatgacagaaataataattcttcgcccgaggcttttattgggtttggggtttcgtcgacttgagtcatcggtcatgagaagctcctcctatctgttcaatttaattatagtttccaaattacctgatttctgcatttaaatcagctgttaaccgttttttaatcttttcaaaggcggtgttgaccacttcgtccttcagggtttcgcggggatccacataagtcagggagtaagccatcgatttcttgccgtcgggaacattgtcaccttcatagacatcgaataaacgcacatcgttcaagaaggcaccaccacgtttattcataaccgccaaaatttgactgttggtaacatcctgatccacaactaatgaaatatcccgtttgattgatggatatttggagatagcttggtactggttgtcatcttttggcaaatcaatcaactcctgcatattgagttcaaatccataagtttccttgattttgaactgcttggcaattcgtggatggatttggcccaggaaaccgacgtaatggccgtggatcgaaatgttggctgtccttcccggatgcatttcaggatattgatcagtggcagtgtactcaatgtcacctttgacgcccaaattaaccaagaactggttaacaatgccttttaactggaaaaagtcgaccggcttgacatggttattccacagcggatcagtgaaattgcccgtgacaactccggcaatgtgttcaacttcttcaggccgaatttggtccgcactatgtttgtaaaagacccgtccagactcgtaaagggccacatcgtcaactttgtgggcatggttataggcaacatcatcaagtaatcctgacaacatgttcattctcagcaccgcatgatcctgggtcattggccacagcagcttcgtttcttgactatcacgcatcaaaaacatttttgctttttcagcagtagtcaaagaataagagatcgcctgagtcaggcccaagccttccaaggcagttctggaagcgcgctgcagtttttgaatcggcgtcaaaacaccaatactttgtcgtccggtcggcagcgttgccgggagattatcataaccgtaaattctggcaacttcttcatacaagtcagcatcgcggaaaatatcccagcgacgggccgggatggtcacatttaaaccgtcatcgtgggcttcgcttgaaaagccaagccgatcaaaaatacttttaatttctgcggtggttaatgaagttccaagaacatgattggttcgttcagcggtaatataaatcgttggcagtttaggatgatattcactggcagtcaccgtgcctttggcgatcttgcctccagcaagctgcttaatcatgctgacagcttcgtcaacagcatcttggacaccgtctggattaattccccgttcgaagcgttgggaggcctcagagtgcaaattatgccgttgggcagtcttacgaatcttgaaggaatcaaaaatcgcggattcaatcaccacgttgctggtattgtcatcgatttgggtgttgaagccccccatgacaccagctaaggcaatcggtttgtcgtcatcggcaatcacaatatcgtctgcggaaagctcgtgttcatcctcatcaagcgtggttaatttttcacccttttgcgccaggcgaacattgacgttaccgttaattttatctttatcaaatgaatgcagtggctgaccgtacttgagcaaaatatagttggtaacgtcgacgacattgttgatcggtcggatgccggcgttccaaagaacaatctgcagccaagaaggactcggcgcaattttgactccttcaacaacccgcagcttgtaggttttggcaagttgatcgtcagcttttgcctgaatttcttgattggcatccaatgaactgtcttcatcaaccactggttttttaatttctggttgctggttatagattgcagccaggtcgtgaacagtgcccaaaatgcttaacatatcaccacgattgggagtgacatcaaggtcaataatgggatcatccattcccaagtacttgtaaattggttcaccaacaggcacatcgtcatcaaaaacgtaaataccgtctgcccattccttagggatgacgtctttgctgaagccaatttcatccaaagcacagatcatgccggatgattcaattccgcgcatcttggaacgcttgattttaacgttgccgccaattcgtgagttgggcagcgccacgataactttttggtcaacgtcaacatttggggccccacacacaatttgtaagggttcgtcttctccgacatccacttggcaaacgtggaggtggtccgattccggatgtttggtcattgataaaatgtggccgacaacgagctttttcaggccgtcttcggcaacggtgacagaatccacctcaaccgctgttcgttcgatcttttcagccagatctttagcgggcatattcagatctaaatattgtttgagccatttatatgaaactttcattctctaattacccctcttactgaattgatttaagaagcgaacgtcatccaaatagaaatcacggatatcgtcaacaccatatttaagcattgcgaaacgatccggaccgactccgaaggcaaaaccaccgtacttcttggagtcgacaccagccatgtccaaaacatttggatgaaccattccggcacctaaaacctcaatccaaccagtgtgtttgcagacatcacaacccttacccatgcagttaaagcaagtgacgtcaacctccacagacggttccgtaaatgggaaataacttggacgaagacgaatatcgaatttatcaccaaaaatattttgggccatcgtgatcaaagtacctttcaaatcggccatagtgacgtgttcatcgataaacagcccttcaacttggtggaattgatgagaatgcgttggatcatcagtatcccgacggtaaacgattccaggtgagatcatcttcagcggtccctttgaaaaatcatgtttctccagtgcccgtgcttgcattggtgaagtttgggttcgcattaggatttccttacttatgtagaatgtatcctgcatatcccgggctggatgattcttcggtagattcatcatttcaaagttgtacttatcttcttcaacttctggaccggaaaggacttcatagcccatccccaaaaacaaatcgacaatttggtcaatgatctgttgaatcacgtgcggttggccttgagcaaccggctttcccggcatcgtcacatcaatcttttcagctgccagttgcgcattgagggcagcatcttccaatttttcacgatgatcagaaacggcttcggtgatggcatcccgaatcttattggcataactgccgacttccggccgttcttcaggggttaattctttgattccccgcaatgcagcggtaatcgggccttttttcccgagcaaatgcactcgaatttcatttaatgcttttaaatcattggtctgctgaatatcagcaagccctttttctttgatctctgtcaattgatctcgcagtgacatagtatccctccagttcaaattttaaacacaaaaaaactccgcccgataagggacgaagcaacgcggtaccaccctaatttgctgtcaaaagacaacacacttaagacatcgctaacggtgattaaccggaaattttttgttaaataacgcccaatttcagctcgaaaaatgaattcgtgaagatttcctacttcgttttcaccaaccacgaagtctctcagataggttatcaacctactacttttttctcaaacgctttacattagtgaataataagctaaaacaaaaaaatggtcaagctacttttcaacgcttggataccatttttctgaccatgtatgaatttcatgcatgattggagctaattctttgccttgttcagtcaatgaatactcgattaaagatgaatcatcgtgttcggttctgacaacgacaccatcgtcttccagttcgcgcaggcgctctaccagcacacgatcgctgcacttggggatttgtcgggcaatctccctgaatctcaaaacaccttcctgaaggaggacgtcaatgattaagccattccattttttaccaaggaatgaaaatgtcttctcgaacttaggacacaaataataattaatggcatcttgcagaccaactacttgtcgcatataaattcccccctctcatcggacaaccgttatttaacagcagttgttcgcttaacttgcttctttaacgtttcgaactttgatttaagtggactcacgaattcgtgaacagcttcgtagtcatcgaccaaggagacgatgacactttcttcgtacttgggccgtgccaaagttaatccccacatgtgcttaagaataatatctttttccattggggataacttggtgatccgttcggcattccgcagggcaacccgtgggtgaataaatgcgtgagaacccaaatcaaacttggtggttctccagtcgtagaaaaacagatcatgaagcagaccagcacgcgcaacggcacgataatctaagccccttcttttggcaatcttataactgtcaaaagaaacagcaattgaatgttcaagtcgagttgagtgatggtgctgagtatagttagccaatttcttaaccatgtcagtcgccatcaggtcagaaactatttcacgatactcggaatcgtttttccattcatccttttgcatgtaatacccctttgtctttatttacaaacatgatacatggtatcgccccaaatatcaatgaaaacgaccgttatttaacaaacttgaaaagtaatatgccggtcgctacggcaacatttagcgattccgcctcaccattcatcggaatgtaaaggttttgatcggtcttctccaaaatctttgggtcaaccccattgccttcatttcccataatcagtgcaaattgcttggtaggtgttatatcatagtaggaaatggcctgatcatttaattcggtgccataagtcttaacgccagcttctttaaaggctgccatccattccaagatatctccggtaaacagcttcatgtgaaattggctgccctgcattgaccggacaactttcgggttataaagatcagccgatcccttgccaaagacaatgccgtttaatcccgccgcatccgctgttcggaccatggtgccaatattgcccgggtcttgaatgttatccaataacagccaggcaccctttaagtcatcgggaatctgttcatggtagtcctcggtattgagcacggcaaacacaccctggggcgtctctgtggacgagatatgtttggcaatttctggcgtgattaagaaaatttcggtatcatcgtcaaccggcagatcgcccaaatagctctcgtcgacaaccatcagttgtttgatggtctggcgatggcgaattgcttcatcaacaatgtgccagccttcaataacgtattcgccggacttaacccgtcccttcttggactgcatcttggtccattcttttacccggttattctgattcgatgtaattctttcaatatccataaaatatctctctttcattattaattgtaggtggtgatcatttgaacgacaaaattcaaacagtcaaaatgaacgcttccggccgagtccaaggcgttggctttagatggtcaaccatccagctggcagaaagcctcaacatttccggctgggtcaaaaatgaaatcgacggcagcgtttcaattcttgcaagcggcgaaagtgaaaatctggcgcaatttatccaaaaaatcaagaattcacccaccccatttgccaaagtcaaaagtctccaagtcaattatatcgcgaaaagggtaaataaagggtttaatgtgaaatattaaattgaaaagcaggcaataatctagtaagattgttttgtttacgtactaacttaagaaaggtcttactcatgaaaaaatttaaacacctcaccacgctgggattgctttccggcatggcccttcttttgagtggctgtgtccgaacaaccaagtccggtaagccttacggagccgtctatgattatctggcccgccctgctcaggcaattatggaatggattgcccaatttgtcggtagttacggctgggccatcatcgtcctgaccgtggttgttcgcctattcctcttgccaatcatggttcgccagatgaaggcttcaactattcaacaggaaaaaatgcagttgattagaccacaaatggctgaattacagaagcgtcaaaaagcagccagtacccctgaagaacagacagctgccagccaagcaatgatggcattgtacaaacaaaacggcatttcgatgaccggtgggatcggttgcttaccattattgattcagatgccgatctttactgctttgtacgccgcaatccgttactcgccagagctgtctcatacagttttcatgggcattcgactcggccaatcgagttggctgttagccgttttgtcatttgcttcctatctattacagggctacattgccatgctgggcacccctgcagcgcaaaagaagcaaatgggcgccatgatgctgctcagtccaatcatgatcttggtgttcacgctgagtgccccagccggtctgggaatttacttcttcattggcggcctattcgcatgtttgcagacgttgatcatcaatatgtatcgaccaagaattcgaaagcggatcgccaaagaaaatgaaggcaaaaaagctgtgacggttgaggatctgatgccagatccaacgccgactgccagtgggacaaaatcgaccggttccgatattcaccaaagaaatcgtcaacgaaataccggcaagcagcaatccgggcatcagcctcaggctcgtccagctgctcagccaaccaaaacgacggtggataagcaagctgaaaaaccagcggctaagcgtcctcgaaacgctggtaaacaacaacgacatcataaataatcacactcaatcacatcttttggtgtgatttttttatttctgcaagattttgagtgatatgacacccaaactcaggataagaatggtaggatattcatgtatatttttcaggaaaagagttgttttcgtttatgaatcaaatttcgctattgatcattctcctggcggcccttgtcatcccattggcaatggcccgttttaaaatcacttttctaccaacagcggttgttgaaattattgttggtatcctgctgggaccgtcactgttcaactggatcaccaactcggaaaccttggagattctccaaaatgtcggggtcatcttcctgttgttcttaagcgggatggagattgatttcagcctctttaaaaagaagcccaccactctttcaccgctcgagaagaaaagccagcatgatcagccgaagtactcagtattacaagtggctacaatcgcttacgcctcaattgtcggcatgtcgtttgtgatcgcttatctgcttcaactcagcggcttgttcaccgatatttggctggccgcgattctgttcatgacgatttcactcggcattgtcattgccgggttaaaagaaaaggagctgcttagcaagccgttcggccaggcaatcctcttaatcgccgccctgggagaagttgtcccgatggttgggttgactttttacgcttcagcctacagtccccattccaaatccttatggctgatcttgttgattctggttgcagctgcgctcttgttctggcggttcaaagcctttttccgcttctttgatcggatcaacaagtcgaccacccagctggatattcggctttcattttttatcatcgtggccctggtaaccgtcgctgaatcggttggcgctgagggaatccttggtgcatttcttgccggaatcgtcatcaaattacttgaaccgcatgaagaaaccaaagttcgtttggactcaattgggtatggcttcttcatcccaattttcttcatcatgagtggcgttaatttgaacttaaaagaattaattacgaatccacaaacgctggtgttgattcccgtgatttttgtcggctacgttttggcaaagagcttggtattcagtgccttaaaattgcgtttcaagaacctaaacgcagttgcaggaactgcgatgactgccaccaccattaccgttgttttggcagtgctgcaggttgccaaccacttacacagaattaccagccaacagtcaggtgcattcttgctgtcagccgtcatcacctgtgtctttggtccactgatttttaataagctgtattcatcagaagccgaggatctcaaaaagacgagcgtgcactttatcggcaccaatttgacgactgtccctgtggcgcaacaattagccaagggctggtatgatgtgaccatgtataccaacaaccagcacaattatcgggccttcaacagtgaaacgaccatccatctgctggacagtttggaaccggaagtcatgattaaaaacggtgtttttgatgctgatgtcgtggtgtttggtcagattaattccgaaaagaattatgaattggcgaaaattgccaagcaatatggtgtccgccgggtgatcgtccgattcgaagaccgcaatattttagacgatcgcagagacgagttggatcgactgggagtggagctttataataccccggatgttaatatcagcatgttaagagcgttgatcgaagcgccgtcaacaatgcgcttaatgacgtccacagattccagtgtctacgaagttgccctgagaaaccggctgtatgctgacattcaggtccgcaacattccatttatcgacaaagttaccattacccaaatttaccgtgacaaacggtttatccggccaaccggcggcacatcgttaaaactaaatgatcggattatttttaccagcagcaaagccgaggcaccagaagttcgtagggaacttggaaaacttaattagtcacaatgactcttacccattaaaaagacgtcacattcattgcagtttgcaacggatgtgacgcctttttaaacttatttttcatgatgttcatcgtcatttaatggacgatcatcatgtttggaagtatccaagattccttctgggagtcctgaatcttccgattgttctttggaggttgatgaagtctttttctccatttcttcttcgcttggcagatgctgcaagattggcagattgatttggaaaatcgacccggaaccaagtgaactttcaatcgaaatgttaccatggtaagcttcgatcagcctgtgggcaattgaaagtcccagtccgttaccgcctttgtcacgactgcgggctttatcgacccgatagaagcggttgaagaccttttgcttatcctcttcagaaatcccctcaccaaagtcctggacagcaatgttaaccatcgccatcgatgtagacagtgacaggtggacttcttttcgcttggttgaatatttaatggcattatccagaagaatgaccaatacttgttcaagatgattccgataaatcttaacgtaaacgtcatgatcggtgtcatcatcaaacgtaaaggtgaaatctggatgaatcattttgaaatcattataaacttgttcaaacacttgattgacgtcggtaatttcttcgccgtaattaatttcaatctgttcggcacgcgaaagatccaacatttcagaaaccaggctcttcattcgattggtttcctgcagtgaagctttcaaagattcttccaagacttcgggatcatctttcccccaccgcagcagcatatcaatatgaccctgaatgacggcaaccggtgtccgtaattcatgggaaacatcctccacgaattgctgttgctggtcaatatagcgctgagtttgatccaacatgccgttcaacaactgagccaagtcggttaattcatcgttggatcgaaaggccggtacccgtgcatctgagtcgggatcgctcttaacttcattaatcgttttttgaatatcattaattggccgcaataattcctgagctagaatataggcaaaaatcatcgtcaaaagaacagaaatcagcaccagaataattaagataaccagcagcttgttagccgtcgctcggtaattgtccaattgatcagtgacttgtgcgtacccaatcaatgagccattcttctttgaaagcagcggttctgagccaaccagaatttggtggccattatgcctggtggtaaaaattttccgcttgctggcagaataaaacttggccgtactcttccgcgattcaaataattccttgccattgacactgtagacattgactaaaatgttatcgcgggaaaaattaacgatcaacgaattggaatacaaatcgttgccatcagcttgtgttacctgatcgttactgtcggtgatctttggcttcaaatagtgtcccacatcgcttttggtcaatggtgaggcataattggtcaaccttgaagaaacggtactcaaggtattgtcaatgtgcgaacgttcctgttgaaataagacgttggtaaatcgattaaaaattaagcatgagaaaataacaacaatcgctaaaacaccaatggacgtaaaaaacgcccacttccattttagcgatgtctttcttctctttggttttgtgttgggttggttcatgaccgcatcacgtaccccgtacctctaaccgtttgaatgtaactgttctcacctggacgatcaatcttgtttcggagatatctgatgtaaacatcgaccacgttggtctcaacttcggaatcgtacccccatactttggtaagcagaacatcccgggccaggacaacgtcaacgttttccatcaaagtcagcaacaattcatattcacgctttgtgaggttaatcacttcatcgccacgacgaacaattcgactttccttttcaatggtcaagtccttgaatgtgactgatttcttgttgttcttttgttgatcattttcgatttgaattcggcgaagcaaggcccggattcgagctaagagttcctcaatcgcaaagggtttgacaatgtaatcatcagcaccatgatcaaagcctgaaactcggtcaataacagagtcccgcgcggtcatcatgataatcggtgtgttcttcttttcacgtaatcggcgggcaacttccattccgttcaattcaggcaacatcaaatcaagcaaaatgacatcaaagttctcatccaatgcagcctgcaaaccagttcggccgtttagctcaacttgggtatcgtagccttcgtgctttaactccagttcgacgaaacgtgctaaattcttttcgtcttcaataatcaaaattcgactcataaatgatcagctctcccataaaatatcttaatttgtttattagtaacgtagaaaccttttaacataactctcattttaccataattatgagagttttagtcttttactttaataaaacttagaaaaacggctaaaattgcttggaaatatttttcatttaaactaattttgtgtagaaattcacttgataatgcccaaggggacgtttataatgaacttgtttgaaaatatattacaaaaaggatgattaaccctatgaaagctgctgttgtaagagatcccgttgatggatatgttgatattaaagatgttactttacgccccattcaccaaggtgaagccttagttcaagttgaatattgtggattatgtcacacagatttacacgtcgctgaaggcgactttggtaaggttcccggccgaatcattggtcacgaaggcgtcggaaaagtcattcaagttgccgacgatgtcactaacttaaagattggcgaccgtgtttcaatcgcttggttctacagaggctgtggtcactgtgagtactgtatcactggccgtgagacactctgccgtaacgttcaaaattctggctacacagttgatggtgctatggctgaacaagtcattgtccctgcagactacgccgttaaagtaccagaaggacttgatccaattgaagcgacttcattaacctgtgccggcgttacgatgtataaggcactcaaagttggcgacactcgtcccggccaatgggttgaagtcgttggttgtggtggcttgggtaacctcgctgttcaatatgcccataacgtctttggtgcccatgtggtagccgttgatggtaatgagcaaaaacttcaagcagctaaggacaacggtgcagatatcaccatcaaccgtcatgatccagatgttgccgatcaaattcaaaagaaggttggcggcgtgcataatgctcaaattactgccgttacaactgaggccttcactacatctgttaacgctttgcgtccagatggcaagttggttgctgttgcccttcctaagggtgatatggcacttaacatcgataagacggttctcgatggcattcaagttgccggttcactggttggtaccagacaggacctcgctgaaacattccaattcggcgctgaaggcaaagtaaagccaatcgtacaaactcgtcgacttgatgaggtcaatgacattatcgatgaaatgaaagccaataagattgttggccgaatggttgttgattttactaaataaatataatattgatccaaatgaattaagggccaccagcgaaacgcatctcgctggcggccctatttttatgtatataaaaaccaatttagaatccatggcgttctaaattggttattaattacttgttatctttgataactttacggcctttgtaaaagcctgatggtgatacgtgatgtggcatggtgtattcaccggtctttgggtcgaggctcaaattaggagtcgtcaacttgatgtgaccgcgacgcatgcgctttctagctttagaagttctacgtgctggtgtagccattctttttccctcctcgtcaaaataaaatatccactagtgaaattttaagtccagctatttcgaatctcgattcttaaaaaagtccttcaattcggccagacgtggatcaacagttttcaattctgccttctgcttgctgtagtcatcgacggacataacatcccaatcgtcaccacttggcatctctttgcctgcaagttcttcaggagacaggacgtgcataggaatatgcaaaatcacattatcaacaactgctctttgcatatcaaccatatcatcttcatctaaaacaaagacaacgtcatcttttccataccgtgattcagcagccttggaaggaacatagaactcctcaactgtaaaatcaagcggtaggtcaacgggtgtcaatgaacgggatgacgggacgaccaacttcccaacaatatgggagtcaataatcacatcaccgcgatcggcaaaagcagtcccttcaacgtgaaagtcggatgcatcgatcacttcatcagcatatcgatcaagcaaatcggctttgatttgaaggttctcgttgaatgtgaaaggatcagtatccgagtacttttgcaagtctctaaagtaccatttcaatataattcctccaatgcaacaaaacttattataccggcaacaaataggcttgtcaaggcaatttccttgataggagtttacggattattccatgatgattggatgtcgataataatcttgagacaagccattaatcatctgggttaacatcccgccccgaaaatccatttggattgtgtcggcaacaacgtcgtcagtaattttggtaatcaatggaacgtcaaggtctcctttgatttgattcaagtatctttgacctaccgcgttaaagcccaacagccggacatatccggccgcctgaagcatatcacttggaactgcatgtaacaagacataggtacacagccgctggattcttgtatacgtataacgcttggttttgaccaaatgtaggaactcggtgaagctttctgccttgattgcggcccgttttaaacggtactcaattccctcggtcatctgataaatctgatgaagcttttcaatcggactctcaaccaattcaaacctgagaaacggccaaaaatcttgccaggtgagcattcggtcatgctcaagcatccccattgtccccttgggaaccactcgatcagcagccttcaagtcatgtttaacgaccgcttggcgaatcgctgtcgcactggcaataggactgacatcgtcaatttgagtcgcatcatgttggctgccctttcgcttaattggtaccagcgaaagcggcctgcctgcttcaacattggcttttgcgtatccaaatcctaagacatcattgggttgattcaaccgaatgccggttttctcaaatagataatcctggaagacggaggcgtatggacgatcaaatcgtttaaaatcggcaggattttttggctgatggtcaatcagcttttgataatccatttctggatgttctgcaccaaaggccaaccaccgacactttattttggcagccaaatcaaccgccccttttgagaataggtgggaaggctgaaccgccgaaaataatggcagttcaatgaccaggtcaactccacccagcagggcagcgtgagcccgttgccatttgtcatacgccgccggttcaccccgctgcagccaattgccgctcataatggcgacagtaacatctgcgccggttgcctgctttgcctgttcgagcatatataaatgtccattatgaaagggattgtattctgaaacaatcccaacagcttgaagcatattctccgacttccttagtcttttcccgtactaaagaaccagcgcttggtttcccgtacgaaggggttgtccccaaaatcggtgcttgccagagttaccaagaaaccagtctgtgacagcagatctttaatcaccgtgtcatcgtaagcgcgctcacgatggatttcattatacgcatcataagcatccttctcctcattgtattggaagaagttcaactcgtgttcaacagccattggcgcgaagtcaccttcgtagctggtccacataaaagcggcatcttcactccgatagttgtacatataaccaggataaacctcggttgcctgataaggtgaaatcacatcaaagagaaactgaccgtccgaattgagatgatcatacactgctttgaaagttgtctccaaatcattttgatcaatcaaataattcaaggaatcatcaaaacagcagatcaaatcatactgatcaaggccgtccagattgcgcatatcagtttgaataaagggcacgtcaacacttgcttcgcgtgctctttgctcggcaattgtcagcatgtcctctgatagatccgccccagtcacctgaaaccctttttgggctaatttaatcgccaagcgaccagttccgcaggccagatccaaaattttaatttctgaaggcggtttttggatcccttttgtcttgttcacaacaaaatgggcccaacgatcatagagagttgcgtcaaataaatcatcataaaatttggcgaattctgtatagatcattatgcctccacccacgaatcggtattaacgattggggcatccgaccataatttttccaaattgtaaaaatcacggacatctttctggaaaatgtgaacgaccacgtcaccgaggtcaattaaaatccagcgggcagaatctttaccagaaacactgtagacattaacgtcatcggcttcaacctgatcgacaatttcatcggcaatcgccttgacctgtcgactggaagctgcgtcagcgatgacaaaatagtcagccatcagactaaccttttgcatatcgagaaccacaatatcgttggcacgtttactgtctgccgcacgaacaacgacttctgaaatttctttactgttcatatttactccttaatctattcctgaacttggtacccaactattataagtcacgattgtctgtggaaaaactggcttattgtgggcaaccaagtatcccaacgtttgtttggtttggtaggcaacgccatcttgcagattattcttggtaatcttgcgtgcctcatcgacacctggaaaatcccgacctggttcaatataatcggccatatagacaatttgttccaatggcgtcatatactggtgcccaactgtatggtacctgacggcgtttaaaatatcaatatcggtgatttgtaactcatttttgacaaacaaccaaccaacaacaccgtgccaaattgcgttgccataattcagcagttcaggctctaattgatagtccttgattgcttgaataaaatcgtcatccggacgttgcttggcatagtcgtggaccaacccaccaatcgccgccttttcaatatcaaccccgttttgttctgcgaggtccatggcagtctgctcaacacgcagacaatgctgaaaacggtgatcactgagagcggcgcgtagtttgccaaccagctcgtcacgagtgtatggaacaaaatggccttgatagattagttgatcatttttcatataaatggttctcctttatataatgttcaacagcggccggaaccaagtacttaattgactggtgctgtcgcattttcgagcgaatcagcgatgatgaaatatcgatgaacggcacgtcaacccaaattaccgggtatttggaagctggtgtgtagccgtcacgtttgacaccgacaaacgaaaccaatttgaccagatcatcgattcgataccattttggcaggtaatcgaccatatcaccaccgataataaagtaatattgattctcggggtgctgttgggtcaactgtttcattgtgtcgtaggaataactgacgccaccacgcataatctcagtcatttcaatggcaaacttgggattgtcccgaatagcgcagttaatcatggccacccgatctttggcatcaatcgcaaatttccggtcaacgtgcggtggattggcatcaggcataaagtaaactttgtcgagccccagttgatccaagacctgttcggcaataattaaatgcccgttatgaattggattgaaggtcccccctaagatcccgatgcgtttaccgttttgttttgtaattgttttcgtctgggttaatgtttcgacatgattcatgacgttgctcatccttcattacctctaaatcgccaaaacttcgttggataatttttgcttatttggatcttttgacggcttgaagaggaccaaagtcttcccgatcgtctgaaccaccgtcacatcacttttggtttcaatatagtccttgatgtcatcaacggtcgctgcggaattttgtaagacattgattttaatcagttcacgcgtatcaagtgctttttgaatctcttcaagccaaactggtgaaagaccgtttttaccaacttcaaagattggccgcatgcggttggcattggctcttaaaaatcgtttttgttttcctgttaatttcataagtccctctttagttaaatcattgctgggcgcatcaaaacggatacgcctttaggagcccatccagtgacggaaacgccctctggaacagttacccaacccaagccctcgatcactaaatcacttttttcagtggacttaaattcatgaggttccaaagctggaaaatcagccttttgatcttcggttggcggtgttagaaatgaacccacatgggtagcgtaaaactcatcggcattttctaatttcgttcgatgaatgaataaattattctcagcatacactgtgaatccatgacgcttgtcaccagagttgtaatcaaaccgggcaacgccggcaaagaagagcgtttgacccgggtttaactggtaacctttcggcttgattgttttttgtggcgtcaccaaattcaattctttacccgacagatggtgggccatttgctcaggctggatgatccctggggtatccactaagttatgaccgtcattgagcggaatatcaatccgatccaaggtcgttcccggaaaacgggaagtcgtgattaactccttgatgccagttgactgacggacaattgagttgatcagagttgatttaccaacattggtaaccccaacgacataaacatcttttccctgacggtacttttcaatttgatccaacaaacgatcaatatcaaaatttgtcttagcagaaatcagctcaacatcaattggccgaataccggccgcgttagcctgttgtcgcaaccaatccttcaccttgttatgcttcaaggctttgggcaaaatatcgagtttattcccaaccaacaggaccggattgctgccgacaaaccgatggagaccgggaatgaggcttccgttcacatcaaaaatatcaaccacgtacacgatcaaagagtcagtatcagaaatactggttaacagctttaagaagtcatcatccgataaactgacgggagcaatttcattatagtggcgaagtctaaaacaacgctgacaatagacctccccattttcaagccccttctttaaagcagattcaggggtgtatccgagtgcgttcttgtcagtcgtctggacagctgccccacaacccacacaatgaacgacttcaccgtcaacaacaacttcactatttgccataattcctcctatttccaatgtaaatcaggatattttttcgataatttattccagacaatcttttcaaagtaacgattgatcgtggtattccaagcatcgtcacgcaccagtggcttcaccaaaatgctgcgaacaccgcaactgttggcagccaccacatcagtcatcaattggtcgccaatcataacagtgttgcgcttttgtaaattaaattccttgagagcgtgccggataccgatagtgagcggcttcattgccctgggaacaaacggcagctcgtaatcttgaaccgcgcgttgaattcgcttgtgactgttattggacacaacaatcaccttaatgccaaattttttattttctgacaaccagttgcgtaacgcttgagaacccttcttggagttccaaggtaccaaggtattgtctaaatcggttagaacacagttgatattatgatcccgcaggaattggggagaaatcgtgtaaatatccccaatcatccatgttggtttaaatcgagacaacatatgtcgctccttaaattatagtaaatttatttaaaaaaacttccaccaaactatcggtgaaagtcattttagcacatcaaaattacttaagtgcttttttagcttcgtcagttaaagctttgaaagcttcagtatcactaactgctaaatcagcaagcattttacggttcatgtcgatgttggcaagcttcaaaccgtgcataaattggctgtagctgaggtcattaagacgagcagcagcgttaattcgtgcaatccaaagtttacggaagttacctttgttgttacgacggtcacggaatgcatatacctgtgacttcataacttggtctttggcagtcttgaataaacgagactttccaccgcgataacccttagctaattttaaaacacgcttacgacgtgcatgtgtgactgttccaccttttactcgtggcattttgaattcctcctatattttgaaaagtaataattgaatgtatagttgattttatagatgtggcaataacttcttgtaagtcttgatattagtcttgtccatcatactagtaccacgaagttggcggcgttgcttctttgtcttaccgtggaaacggtgactggtataagcatttgcactcttaaatccaccgttggcagttctcttaaaacgttttgctgcagcacggtttgttttttgtttaggcattggtaaaaatcctcctcaagtatttaacaactattatttttgatcttggtcttttggtgaaagcattaagaacatgcttcttccgtccatcttaggtcgttgggtaacggtggcaacgtccgccgtttcagcagccattcggtcaagaactttccggccgatatccttatgcgtaatggcacggcccttaaatcgaattgagacccgaaccttttcgccctttgccaaaaacttcttagcattcttcaatttggtgttaaaatcgttcacatcaattgttgggcttaatcgaacttccttgacactgatgactttttgtttcttacgggattcacgttccttcttctgcaactcgaaacgatacttcccataatcaagaatctttgcaaccggtggcttggctttcggtgcaaccaggacaagatccaagtcggcatcttcagctaactgaagagcttctgacttagtcttaacaccaagttgatcaccattagcaccaatcaaacgaacctcacgagcacggattccatcattaaccatcatatcttttgctatggtacttcacctccgaataatttgaaaaagcagaaagagagcgggcacacatttgcgcccgctctcaattaaagaacttggctgaccaagctcttactcgatatcatgcccagcaaattcagaaatttactcaggcgagaagcgggtagctcctgctttcatttgaacaactattacagaatatcatctaatcacttatgtgtcaactatgaaccgttaagcgcattaataagtgacttggtaatccgttaatcttcttcacgtgaatatgaagcaatgtctttagatacttcatcaatgaagtccggaactgactctgattgggtatcctgctcaccatacttacgaactgaaacactgttgccactcacttcttcatcaccgacaactaaggtatatggaatcttgtgagtctgtgcatcgcggatcaagtaacccatcttttcggcacgggtatcaactgacgaacgaatcttcaatgctcgaagctggtcattaatcttcttagcgtaatccaggtgcttgtcttggctgacaggaataatcttaacttgatgtggtgctaaccaggttgggaaggcacccttatagatttcagtcaggtaagcgacgaatcgttccatggtagaaaccaagccacggtgaatcatgactggacgatgttgtttgccatcttcgccgatgtagtgaagatcgaagcgttcaggaagcataaagtctaattgaatcgttgacaaagtttcttcatttcccagagcggtcttggtctgaacatccagctttggaccatagaaggcagcttctccttcagcttcaacataatccaagcccatttcatccatggcacctttcaacatggtctgagcacgggtccacatttcatcgtcatcgaagtacttttcggtgttcttggggtcacggtagctcaaacggaaggtataatcgttaatatcaaaatcgtgataaacctcaaccatcaagttcaagatattcttgaattcttcttgaatctggtccaaggcgacaaatgtatgaccatcgttcaaagtcatttcacgaactcgttgaagtccggacaaagcacctgatttttcgtaacggtgcatcattccgagttcagcgatccgaagtggcagttcacgatatgaacggatatggtggttataaatttgaatatggcttgggcagttcattggccgcagttcaagctcttcaccgtctcccatgtccattggcgggaacatgtcctcacggtagtgatcccaatgtcctgattgtttatacagatcaaggttggctaaaaccggtgtgtaaacgtgttggtatccgttggcaacttccttgtcaacaatgtagcgttcaatggttcttctgatcgttgcaccgtttggcatccagtaaggcaagccggcaccgacttttggatcaacaaagaacagatccagttcgtttccgatgactcggtgatcacgttcatgggcttccttgcgcttctcaaggtcggcatccaaatctttttgcttgttaaaagcagttgcataaatccgttgaagcattgggttggatgacttgccctgccagtaagctccggcaactgagagcagcttgaagatcttaactttgccggttgatggtaaaacagctccttcggcgattgattggaagtcaccgatttggaagaatttaacttggccgttaacttcgtttgctttgaccaattctttttgataaggatcatcgccggcaacctttgcagcatcagcagcgcttaagaagaccaccttgattggcagatcctgtttgataatcttatgcattgagtcttcaagtgaactcaattgatcaacactgatttgagtgtctggtttgtcagtatcaacgaagaagccgtctttatcggcatcgctttcaccaaagtggatattatcaaaatcattggcaattgccattttcaaaatctgggcggcagttgcgcgtaatacactgaggccttcgtcactatctgacgtaacaatttcaatcttgccgcctttatgtaggggctcgtcattgttgacccattttccgtcaaccttggcggcaacggcttttttacctaaacttacggcaattgatttggcaatggcttctgaggtaacgccgtcatcaaattgtttaacactaccatctggaaattcaaatgaaagttgtgacatatttcttactccctttatattttattggagccacaaaaaaagcccctgacatacttatacaagtacatcagggacgcaattagcgcggttccacccaaattggatttttggatacaattatccaaaaagctctcaagtggctgctaacggtaccaaccgggaaagcattatccgcaatccattctcaaagagtggtaacaaacaatttctcaacaaacggtcttccaggctggaaccattctccctgtgatgagtcatcactgtcatgtctctttgattcattgacatttagtatagagttgccgttcaaaaatgtcaattcaatttgtaaattaaactggtcgccgatttttaccggtcatctcgacctcacgagacaagaatcgaattcgctgcatgagtcgtttggctttcaatggttcatcgtcgcctttttgattgatacgcaaatgttcctgttcgagttgggccattgaaaaattagacgtaaaaaacgtcggtagctgctgttgcatccggtattccaaaatgactcccaatacttcatcacgaacccacgaggacattgagtcagccccaatatcatcaatcatcagcaccggcgactttttgatcacatcaattttttcggtgaccgagttatcggtgatcgccgatttcatttcgacagcaaaacttggaaaatgcaccatagtggtttgaatcccgttatcggcaagttcgttggcaattgcacctgtcagatatgttttaccgacaccaaacggcccatatatgtacagacccggatggaaagtctttttgtcggccttcatttgggcaataaaatccaatgccattgaaagggctgtataacgattggggtctggattatcgggatcagccccgtcgaattcggcgatcctggcatccttgatatctttaggcattgaaaccgtcttaattcgacgtgccaaggactgactgcgctgtttttcgatcacctctggagaggctgaatacgcaatatcaatcaaatgatcgttaatgaccaattggggcaaatacccaggtgcaaatgattgtttcttggccttaatctgatttttgacattcacatactcatacaatttggcagcagaacggtcaaccgcatcaggagccagttcaccttgatgatcctgaagaaatttggcgatctcagggtcatttttgatctgttcaataattttttggaaacctgatgcgacattgccacccttaaattgacggtcttccattagtttcttgacgaaatcacttactttttccattcaatctcacctactccccggcttttttaacttatcaagctgtgctttgagctgcttcttttgggcctcagtcaactgtgaggtcggctggctggcagaggaaggctgatcatccttcgcccaatccggcagggtctctttgacattaacccgccgctgtttgtacttggcagcccactgatcagcctttttctgtttgtcgattgttcgattcttaatggcatcgattgcatgctcggcatcaaaaatcccgtgttgtgaccaatcatcggcaatcgttgacatcaagtttttattgagagtcgaacgattttcatcaactaataaatagtaaatcaaaatattgatgacttcattcggcaacacgcgcaggttgacaagctcgcgcaaggttcgctgctcaccgctggtcacaataccgtgcttttgtttcttgatttgttccaaaaacacgactggagccgtctttttactaattgaaatcagttgattggttgccgtgtcgaattttgcggaagaaggcgtgatctcagcagtagatgctgctttctccacgttctctgcttgatgccggctgaaattatcagtaataattgccttcaactgtgattgattcaattcattggtgctgagattagtcgccttttgaatgagtttagccatttggatctcatcaattccatagagcaaattctctgacaaaatcaaatcacgagcggccttaacagaattaagatcgacgtatgaattttccaacatgcttaataagagcttgaagttaaattggcgactatccggttcgaaactgttctcactgacatttgcagcggatcgaacaatggtctgcttggcgtcattgactgcgcctggaatgtttttaatcaggttctggggtacagcaaataaatccagcagtgaagccgaaatattggtcgtctccccgagatccggaagtggcagcaccagtcggtcgacaatctgcttgtaggttgtttcgcccactttgcccaataaaataatcgacaaaatatcggttcgtaaaaactgttcagcagttagcggcagattcaacgagtagatcaagacatccggtttgttttgggaaaccaaagtattgatcagtttaacgccttccaattgctttcgaatcgccaccagctgatcaattttgcaatttaacatgctctgaatttcgtaatgcttatgcaaaaccaactgattgtgatcatttaagctcatcgaccacaacaaattgtataatcccaatgctttttcaccaatgattggtagatacaagttggttaaaacactgtgatcgaggctccgattaatgtgggcattggtcgtgagatattttgtatcgggtgttaatttatcgaacgactctgccattatttgtcccccgagtgatcctgaccctttttcttatccttttccataatttccttaagctctttataaaagaccgacatatccttgaactgacggtaaacactggcaaaccggatataggcaatttcatccaaattggccaaatcttccatgacgtattcaccaatttgttggctggaaacttcattctcgcccagtgaccgcaatttattttcaacccggtccaccaaattggtaatggcatccatggaaactggccgtttttcagcggacctgacgatcccctttaacagtttttcacgattaaattcttcgcggttaccatttttcttcaccactaataaaggggttacttcgacccgctcaaatgtggtaaatcgaaaaccgcagtgttcacattctcttcttcgtctgatcacccgaccgtcatcagttggccgactgtcgacaaccttggaaccattgtatccgcaatgaggacattgcatggtgttcacctcgtctatttcgtttccttcgccaaccatctgtcgacttgtgtcagcgtcgttgtcattgttcctgagttataaataattgtatcagccaaatcgcattttgtctgcaatggccattgatttctgattcttttagtcgcacttacaatactcagtttattgcgtttcatcaatctctgcaactgagtgaccggatcacagtaaaccaccaccacctcgtcgaccagatggacatagccattttcaaataaagttggtgcgtccaagacggtcaattcagcatcccgataacgtttcaactgagaaaaaatctcttcgcgaatgaatgggtcaatgattcgaaccagttgtttgagatcagctggattgttaaacacaatccggccgattgcctggcggtcaagtgcgccgtcagccagcaaaatccgctgtccaaatgcgtccaccagtgcttggagcccaggagtcccggtttgttcaacttgatgggtcacgatgtcagcgtcaatcacaggaatctcctgctgatgaaggtaatcgctgaccactgattttccggtggcaatcccgccggttaagccaattaatttagtcattttttacaccacgcaaaggttggcattttgggcaaaagtgggtgccccgctgagccaacttgattttaacaatctttgtgccgcatctcgggcagggttcgccttcacgaccataaacattcaattgattttgaaaactgccagcttccccatatgcagttgaatatgagtggacggtcgttccatgaccggcgatcgccttggctaattcggcaataatattttttcgcaactctttaatttgtctcaacgtcaacgtgttggcaggctgttgaggattaattttgcttagccataagacctcatcggcgtaaatattacccaacccggcaatattactctggtctagtaaaaatggtttgatcactttacggctcttgctaaaaattttctgcatgtaatcgacggtcaaattatcttcggtgggctccggtccaatcgttttcaaaccggcaacctgcatttcagtgccggtatcaaccaaattcattcggccaaattttcgcgtatcattgtaacgcaactgacgcccatcggtcagatgaaaaatgatatgggtatgcttaccgaccggtgcatcttcgggctccacatcgtacttgccttccattcttaaatgagaaacaatcgttaggttgtcactcaatcgaatcagcaggtatttaccacgtcgatcaattttttcaatcgttttgccacggagggcttttttgaaatcgtttggtggtaaattaatcattttggcatacaacacatcaaccgattggatggtgcttcctttaaccaattgggtcaggccgcgtctaacggtctcaacttcaggtaattcaggcattgagatcccccatttgcttcaacttattttgcatcataccaggtcttaccccagtggctttcaacttttaatggcacattcaagtggatcgctgaatccatgacgcttggaatcagttgtttgacggtgtccaattcctcgtcaggaacttcaaaaattaattcatcgtgaacctgcagcagcatgcgggttttcatatccttgattgcatcggccatattaatcatcgcaattttgatgatatcggccgcactgccttggattggtgtgttcatggcagtccgttcagcgaatgaacgcagattaaagctcttggaattaatatccggcaaataacggcgtcgatgggcaatcgtctcaacgtagcggtggttacgggcaaattcaacgatgtcttcggtatattttttaactccgggatattcttcaaaataacgttcaataaactgatgcgcctgttttctggtaatgccggtattggacgctaaaccaaaatcgctaatcccataaacaatcccaaagttaactgccttggcctgacgccgaagttccggggtgacttcttcatttgacggcagcccaaaaattctccgtgccgtggtggcatgaatatcctcgccgtttttaaaggcgtcctgcatattttggtcgtcggtaattgacgccaacacccgcagttcaatttgagaataatcagaggagaaaatctgccaaccgggatgtgatggaatgaacgcctggcgaataagtcggccttcctcggagcgaaccgggatattctgcagattgggatcgactgaagacaatcgaccagtctgagttaacgtctgcagatatctggtgtgaactttggaatcatctggatgaatgacctttaatagcccatcaacatatgtcgactgtagtttggaaatctggcggtagtccaacacgttttgaacaattggcgcatccggagccaatttctccaacacgtcaactgaggtcgaataaccggttttggtcttctttagaatcggcaggcggagcttttcaaacagaatctttcccagttgtttgggagaaccaatgttaaattcttcaccagcttcttggaaaatggtctgttcaatttcagccagccgctctttaaatttactgcccatgccctccaaagtggctgcatcaactttgatgccattgatttccatgtgggcaaggacaaaggcaatcttgatttcgatatcccagtacagtttggattgattatgggcatccagatccttaaacatcccgtcgtgaagagcatcaatcgctttgaccttatgaaccaaatgggccaaaaaggcaggtgattgcgggtcaatgtgtcgcttggcaccctttccatagacttcttcatcggttttaacattatagaatccgtgtaaatgggcaacggtgccgacgtcgttgctattattagttgtattaagcaaatatgataccagcagcatatcgaagtccacgttggcaagctcaatcccttgtcgataaagaccgacataggttcgtttggcatcaaagacattctttttgatagtcttgctggtcaaaaggtcaatgacatgctgattgtgaagcaattcaggatcgttggtcacataccatttgtcaccctgtccaatcgcaaagccaaccaacggcgatgtgtggtagttttcttctgacatttccaggtgaaaagtcacttcatctgtgaactgatccagctcagccgcattcttggcggacaagacagtgtattgaatatctgcctgatcatcggcatgatcctgatcatcaactgataacttggccagaaacgatttgaagcccattcgctcgtaaaaatcggtcagtttatcgatattgtctccctgatacttcaactgatccaaagagactgttaccggcgcgtcgcggttgattgttgccaacgtgtgggcgcgctcggcctgggcttggtcatgaatcaaatgttcctttaattttttaccggaaacctggtcgatattttgatagagattgtcaatcgtgccaaattgttgaaccagcctgacagctgtcttgtcaccgactttttcaacgccgggatagttgtcggagttgtcacctttcagacccttaatttcaataatctggctcggtttaacacccaacttttcttcgacgtgtttgggggtatatgtttccagttcggtgacgccctttttagaaacctgaaccgtggtcttatctgaagttaactgggtcaaatctcgatcgccagtgacaatcacaacttggtagtcaccagcttcttcagcctttttggcgagcgttccaataatatcatcggcctcataatccggtaattcataggtggagatgccacgggcattaattaattcttttaagaagggaaattgctcggaaagttcagttggtgtctttgcccgaccacccttataatcagcgtacattttcgttcgaaaagtggttttgccggcgtcaaatgcgaccagcacatcggtgggcttctcgtctgctaatactttgtccagcatccggttaaagccatagatggcgctggtatgtaggccagatggattggtaaatttgtccatggccgtgtataaagcataaaacgctttgaaggcaatactattaccatcaattaataataattttttagtcattaacttctcctctggtgaaaactgttactttaattttaccacgacagataacaaaaaacgatcaaccaaatcaatggccaatcgttgtgacgaaatctgaattaacggtcgttgttaccaaaaatcgagagtaattggagaaacaggttcacaaagtccaagtacaattgtaaggcaccaaagactgccaaaccggtcatggaaacttcaccattaccagaatattggttatacatctgcttcatcttttgggtgtcataggcggttaagaccgtgaagattaacactgcgatgatcgagaaaacaaatgaaatcactgaactacgcaagaagatgttaataatcatggcaatgattaacgcaattaaagcagcagttgcttgggcaccccaacgatcaaggttcttgtgggtaaccaatccaacggttgtcattgtgataaaaattgccgaagcggaaacaaaagctgccgcaattgaggcacctgtatacgcccacgcaatcgtggcgaaaacaaaaccacttagaattgaatacaacatcagtactgtaaacgcgagggtcggccgtttcaatgcttgaagtgagatgacaaatggcaaaacaaaccataaaatcattgatccccacatcacaccttggtgacctgcaatgtaagccgccattccaccagcaacagacccactaactaaaaatgctgttgcagcagaaactaaaacggccaaactcatccagccatacattttagttaaaaaagcattcaacccggctgcgttgttaacgactcgtcgagcttcctgttgttcgtttggataattgttcattaaatccgctcccttttgtttgtaagttcaaatattgcctcaaacaatttgcagtatttatacttatactgttaagtaattctaccaaataaaagccattaatcaagtatttaggactcaactaacggcttttataagatatcttaattaatttttttgcttaaatggcttagcagatcttcgtaagatttttcatacttttgaatgtcgccggcacccataaagatgaccacgtcgttatcgtagtccaatagtggcgacatattgtcaacggacaagatgcgcccacccttggtgatcttctttgacaggtcctcactggaaacttttccgtgactttctcgcggcgaactgtaaatcgaggtcaggaaaacttcatcggccaagttcaagctcttggcaaaatcatccatcaaagcgatcgttcggctgaaagtatgcggctgaaataccacggcaatctttttgcttggatattcctgacgggcagcatcgatggttgccttaatttcagttggatgatgggcataatcgtcaatgatcgtcatcccggcaatcttacgttcggcgaaccgacgcttaacgccttggaaagtcttcaattctttgcgaatttcatccaaatcaacatcttcaaagtaagccacagcaatcacagccaatgagttgaaaatgttatgctcaccaaacaacggtactgaaaagtttcccagatttttacctttataagtgacatcaaagctcgaaccactggtcgtccgtttaacatcaaccgcctggaaatcatcagtatccttgaggccataataataaattggtaccttggcttttagttgacggagacgtttatcatcaccccaagcaaagatgcccttcttcgtctggttcgcaaacgtttgaaatgcatcggcaacatcatcgatactcttgtagtaatccggatgatcaaagtcaatgttggtcataatggcataatcaggttcagttgccaaaaagtgacgacggtattcgtcagcttcgtagacaaagaaccgggcattgggaacacctttcccagaaccatcaccgattaaataatcggttggtgcaattcctgaaagcacgtgggctaacaggccagtcgtactggtcttcccatgggcaccggaaaccccgatgctggtcttacccttgatgattttgccaagaaactcgtgataacggtaaaccgtcaatcccatgtctctggctttttttatttctggatgatcatcagtaaaggagttaccggcaattaccgtcaatccttcgtgaatgttgttttcatcgaaaggtaaaattttaataccagccttttcaagcccacgttgtgtaaacgtgtactggtcaatgtctgacccctgcactttctcaccacggtcatgcaagattaaggccatggcggccatcccggttcctttaattcctacaaaatgatataccgtatctgaattcattagacatcctacctatccattatgttatttttgatgattttgcggtgattcccgagcggattcatctgctgccggcttgtaatacactgtccgcggcttggacccctgctgctctgaaaccaagttcttttcctgcaaatgatcaataatgtttgcagctctattatacccgattgaaaatacccgttgaagctttgaagtggaaattgtctcttcattgccaatatattttaaaacctggggcatcaaacgatcctcggagctggtttcagtactagctcgtttcaagctatcaggagtaaataagtatttaggttctccctgttggcggacataatcaacaatgccgtcaagctcctgattggtgacaaaagcaccttggagtcggaccggctgatttgcaccactccctagatatagcatatctccgcggccaagtaaacgttctgctccggccgaatccaaaatcgttctggaatcgacttggctggataccatgaaagcaatccgagtcggaatgttattcttgatggtcccggtcacaatatcaacacttggacgctgcgtggcaacaatcaaatggatgccggctgcgcgggctttttgagtgatgcggacaatgtaatcttcgacttcactggaagcgaccatcatcaggtcagccaattcatcaatgatcaccagaatataaggcattttcagcccatactcgtgagcctcacttgcctgtcgattgaactgttcaatatttttagcaccagcagctgcgagcttttcataacgctgatccatttcctcagtgacccatttaagggaagctgcggccgtcttaggatcggaaataacaggtgataacaagtgaggaatcccgtcataaggtgccagttcaactgcctttggatcgattaacagtaatcgtaaatccgccggggtcgctttgtacagcaaagaaaccaacaaactgttgatgaaaacacttttgccggatccagttgccccagcaatcaacccatgaggcatctttttaatgtctgtcgttctgggaactcctgacaaatcaacacccaaggcagtggtgagtggcgattgactatcttgaaaatgcttggttgaaatcacttctgaaaggaccaccggtctcggattgggattaggaatttcaattccgactgtcgttttaccaggaattggcgcttcaattcgaatatccttggctgccaaggccagctttaagtcatcggttaagttggtaatccggctgactttgacgcccagtgccaatttgacttgaaattgcgtgaccgttgggccatttgtccagtcaaccacttgggcattgaccttgaaggctgagaaagtttgattcaggatttcagattggtgaataatccagtcatcaatcgattctgattcggcttgctgaggcttggctaataaagacagcggcggaaattggtaacccctgtcttcagtcggcttctctgagacgtttggttcagccaatgaatgttgaacacccttcgtgggttgattaacgtgattcacttttttaacctgggcattgtgactcagttgttgagcgttaaacaaagaaaggtcagattcgctggccctttggttatgcataattgaattgaatgactgtcccaacccatggtgattcaaagccttccgtggttgacgatttaaatgccgtaccccttctcctgagctgatctttggttgatctgtcaaagatgatttttgaggtgatgtctgaggttggccttcagtcggcttggcgggttttggtgattgaacgggttgctttggatgctgctcacgaggctgatcaattgttggttgcttatcggcaatcacaatgagatcatcatatgtaatcctcagccggcgtgtcaattcatcgtacagacggtgacgacgatgcgcctggctgagaaaataattcgtttgaatttgctgtttccgtttatcggattttgaccgcttttgcggtttgaaatttttaatttctttcaaaaaagccggggtctcatcccgacgatcaaacttggaatcagggaccttgcttgatcgtgtatcttggattttcggtgccaccggctgattattctgttttatttcccgctcttgatgaggctttcgggtaatgcccttccgccgaaaaaatgcgggtccatcataatgcttcattactcatccacccaaagtcctttaatcaaataaatgctgtgccttgtcaaaatcaaaggcatcccctacctgataatcatcaggtaaaatcagtgccccggggacttgcggtgcgttgggcaaccccaactcgcggccggaacaaatcatgccatcgctttcaacaccacgcaatttaccgggccaaataatctggccgtcaggcatcatagccccacttaacgcaacaaccactttaatgtcttcgcgcatgttcggcgagccgctgacaatttggacgtccttaccggtgccaatatcagttttggtaatctgtaaatgatttgccttggggtggtcttccactgatttgacatagccgacaacaaacttgggctgattatcataacggatatctgccggaaaaccgtgatcgcccaaatattggttcaagcgagtaacctggtcttcggttaaatgaacttggccattttcatggacaatttctggaaggactttacttgcttctaaaaagttgtaccccaacgtctgattgctatcagcggcaaaaatccgggcaaccttatcatgaattgtcacactttgttcacccacatccgggttcataatgaggaccattgtgtcacctgtgctgtttgggttataactggttattaacatttcaaaattccttccaacaattaattattttgctacggtacttgctaacgagttaataaagttttcaacttcggctttagtcttgcggtcgccattattgaagcggccgatttcttgaccgtctgaataggcaacaaaacttggaatgcccataatgcccatttcaccggcaagatcgatattttcatcacgatcaacctgtaagaatgtgtactctggatattcggcttcaattgcaggcattgccggcttgatgaagcggcagtccgggcaccagtcagcggtgaagaacagcatatacttgccgttctcaagttgtttggttaaatcttttaaattggttttaggtaaattttgcaaaattatcatcctttcacttactaatgtaaagtacatcatagcacaaatttccgcccagccaaatcagtttgctcatccgctgctaatagtctaaagtatacatatcatatacaaaaaaggtgaaatgatgaaaaaacaaaccgtcttctatggcctggcactcgcagcgcttgccggcagtgcctatatcgtggccaagtccgatcgcaaacacgaaaagtttttagcagctatcgtcaaggataccaaacaatcagccgcattaaaaggcttcaaatatattggcagttggagcattctaccgaccactgactccacgccgctttttcactttggcttcaattatttgaaccctgaaggtgatcgcaaaacagaagaattctgggtcgaccaaacctcacagcaagtggttaagcatcaagtcatgacgctgtaaaatgcgcaatcagcttataaatgggtcccttgggactgaacttttgctcatattccgtttcaatattcgattcattttcaggagaatggtgtaaatccaacgaaacataatcgaacttcatcgggaaattattcatggtgaccaaggtgtattcgaataagccgcgattatcagttttgaattcgatatccccatcctggtccagcacgtgattataagtcttcaaaaatagtggtgatgtcaaacgacgtttggcatgccgcttttttggccaaggatcggagaagttcaagaaaatctttttaatttcattttcataaaacaattcatcaagattggcgccatcagtcagaacaaactgcacgtttggcaatggatccgccataaacgaccgcagtgctgtggcaatgaccgaagtctgcagttcaatgccaatatagttgatgtcggggttggctcgagcggtctcgataataaaccggcccttaccaatcccgacctcaacgtttaagggttggactttggcaaaccggtcctgccatttacccaaccaattctttggatcggtcacaatatagtcgccgtggtttttgatatatttatcagcccacggcttttttcttacgcgcatatcattctcctattattcaacaatttatctggttcgctcgcttcgagccaaacgtctgggtaaatacagatagacaaatgcccagatttcgagtgcttcgccgacaatcacgccgatgatcgtgaccggcgtggccaaattaacagcgagaactgccacggcaaaaacaacgccaaccgtactcaacaagtacagcagaaccctttgaaaactcttcaattggtactgattggtaattggataaatgtgcacgaaggcgttatccgagaaatgaaaataaaacggaatcatttggaacccaattaggtagacaaacagcaggctcaaaaagatgggtaacagctcgcccttgacgaataccagaaataaggttccgatcaccagcagacgaacgtatagcccactcatctcattgtcacggacaattccgtgagcgtagagatataagtaggtgttttttggaatcagcttgattcggctcaagatcccgtccacgtaacggcgccgtttgacagaaccttgcagagttggcacatccgtaaataaattaaagaattgatagacggtgtgcatccgactgttttcatcggtaatcatcgtcgtccagtcaagtgatcggctgacccaattccggcgggaaaaataactgacgaaaagcgcagccacagcaatgcccaacccaagccaatagttgatgtagatagacgaccccaatgcaatcactgggagcagcaatcgaaagatgagccgactggccaaccaggattgctgcaaatggtatttacgggcaaagtcggtatttagccacgttattttcaagattaaaatggttgccaaaagcagatacaactccgtcgatgtggcgcgcatggtaacttgaacaaacggcatcaacaagatccaaaacaggacttgtattgcgacagcaatcgaaagactataccgaaagccgcttcgaagatagttataaagttcagattctttgggcaacaaaaaaacatagtctggggcttcaatcaaggtcgcaaacctgcccagctgaacgctaaccaacaaaataccgataatcacaattggtgcccaccacagaccggtgtgcagctgcttaagcgcattggaataatagtatcccaagccaccaatgacaaacaacaaagccaagacaaagtagtcgttaaaaaccaatctgagatagcgcatcatttcctttagatgcgtcgttaaacgctgcctgaataactgcttcatgaggcatcgccttcccttgccagagtcaggtaaatatcattgagagaatcgccggcatctgggaataatttccgcagctcttcaatcgttccttcggtgcgaacttgaccgtcatgaagtaaaacgaaccgatcacaataacgttgcgcggtatccagcacgtgagtcgacatcaaaatgctggctccctgttgctttctttcagagatcaggttcaataagtcgtttacggccagtggatccaagccaagaaacggctcgtcaataataaagagtttggcgttagtcaaaaaggcacagacaatcatcaccttttggcgcatcccttttgaaaagttgtccgggaaccagtctaatttattatccagccggaaaagtttgagcaggtcatgtgcccgtttccaggattcgtcttgatcaagtccataggccagcatggtcatttccaaatgctcctttagcgtcaattccttgtagacaattggctgctcgggaatataagcaatctgctctttatattgtttcacgtcatcgtttaagccgacgccgttgattttgattgagcctttaaatggcgttaataaaccgataatatgattgatggtcgttgacttgccggcaccgtttaagccgatcaacccaaccaactcgccatccttaacgtcaaaattgacgtcctttaacactggtacttgggaatagcccccaaccagattcgaaacttgtaaggtcattgtttacctccgtatcatgataaatgtacaaacaagattataccatacaaaattagcctttgagctgggccaaaaacgcaataatggtataatatcattagtattcacagaaagaaggtagaaattttgaaagattgtattttttgtaaaatcgtaagaaatgagatccccagctacaccgtgtatgaggacgacattgtcaaagcattcctggatatttctcaagggactcctggacatacgctggtgattccaaagaagcacatcgccaatatctttgaatatgatgaagaattagccagtgaagtttttgccagaatcccaaagattgctcgggcagtcaaagcttcaaatcccgacatcaaaggcatgaacattttaaataataacggccaagtcgcttatcagtccgtctttcattcacacttccacctggtcccccgatataccagtaacgacgactttaagatgatcttcaaggataactccaacaaatattcaccggaacagttaaaggcgattcaagaatccattgaacaacatatgggtgattaatcatgaaaaccgtttttaaaattgttggtgcaactgccgttgtcgccggagtttatttatacagccgaaaagaaactccccaagagttcgttgagcgggccaagtcgacctttgatgatcgaaagcaaaaggccgctgactggaaaagcgcttatgatgactttaagaagtcgatgaatgctttcacagcgcagatgccggtccttgagaagaccattaacgacatctcacgggatgtggatgaagcgatgttcaaaattcagccacggcttgacgaaatcaacaagtataccgacaaattaaagtaagtaaaatatgaatatttgtttaaattcttgaggtcattatataaacgacgcagattatgttattattatcgggaacgtttgctttgcagacgaatacttttaggaatggatgtgtttttgtatgaaaaaatggctaatcgttttagccggcattatgatgagttttacccttgcagcttgtggcagcaaaactgttgcaacaaccaacggtggtaagattactgaaagtgcttattacagcagtttgaagagtacttcaagcggtaaacaagtattgcagcaaatgatcttgaacaaggtcttggaaaagcaatacggtaaagatgttaaggactctcaagttaatagtgaattcgctaaatacaagaagcaatacggttcatcattcaactcagttctccaacaaaacggtatgactgcttcacaattgaaagattcaattcgttccaatctcttattgaagcaagccgttaaggacaacgtcaagattaccgacgcacaacttgaaactcaattcaagtcttaccaaccaaaagtaactgttaaccaaatcttggtttcaaagaaatcaactgctgaaaaagttatcagtgaacttaaagacggtaagagcttctcaagcttagctaaaaagtattcaactgatacagcaactaagaacaagggcggccgaatcgcagcattcgacaacaccaacacgtcacttgatgccaacttcaagaaagctgccttcaagctgaagaacggtgaatataccaagacccctgttaagactcagtatggttaccaagtaatccaaatggtcaaccatccatcaaagggaacttggaagcaacacgaatctgaattaaaggatcaaatcgttaccagcaagatgtctgatagcaataccttacattcagttgtttctaaggttcttaagaagggtaaagttaccatccaagataaagacctgcaaaacgtcttatcagactacctttcaaccagctcatcagctaagaagtaatttttaaatcattcatacaaaaaaggattggacaattaattgtccaatcctttttgtatcccgtcaattataacaattccccttgggtcggtttttgtttggggtcaactgatttctcaggtttgtagaatcgtcgattatccaatccaaagacccgatcactgaattggccgggttcgacattcttagtggcgctttgaatcatcataatcgtcgcatctaactcatccaaatgatgcagaatttctgcctccaatatcttcggccgttccggtgaaccatactccagtaatccgtggtgcgacagaatcatatgccgcagtaaaatcagatcctgggatttgggatcaattcccaacttgtcagccgcttcaacgatctcggcatccataatgctgagatgtcctaacagattccctgctaaggtgtactctgtggcaattggaccggacagctcaatggttttacccagatcatgtaaaatggcccctgcgtacaataatggggcattaatgccctcatactgattcacgatcgaatgggccagtttgagaattgaaatggtgtgaaaagctagccccccggcaaaatcatggtgattggattttgcggctggaaaggtataaaacgcgttggcgtgcttggaaatcaaactgcggacgattcgattataggttgcgttggtaatctcaaagatggtttggtcaatgtattcttccatctgatcgcgagacatccccgcccgtttgacaaaattaaccggatcgtggggctcactttggttggccagccgcattgccagaatcttgatttggggagaattcatatagttctcccgcttacctttcagcagaacgactttgcctgaaacaaactgctccacatctgttggcgaggcatcccagtatttgcctgagatttggccggactgatcttgaaagaccaacgacagaaatggcttaccatttttagccacccgcttggaggcgtcttttagtaagacatacatctcaaattcttcatccaacttgatatccatcaattgttttgccataaaatcgcctcctaaagcgttttaagatctaagacgagcttggaatcagtatttgcatcgagattggcggtgaagtaaagcacttgagtcttctcactcacctgttgcagcattgccagagctgccgcttttcgacgctggtcaaagttcacaaagccatcgtcaatgataattggcattggatattgactgctgaagccaaccgccatcgaaaagatcagtgctaaataaagctgttccaacgtcccggttgacaattcgttgattggaaaggagacatcatcttttcgaacgacagaaatttcttttttaaaaataatctccttgtaggcatcattcgtcaaagtggcgaaatattgctttgctaatgccagtgtcttgggcagtcgacccttgctggcaatgtccaacaccgcctggatccactgggaactgagcttcaaagccaggtacttctgaacattctcaacaatttcagtttgttgattggccagctcctgccgcaaatcgtagtattggccattcttgattaaaccggcaatttcagtctgaacccgggtcatttcccggctcaaatcattcagttgatcttgtaaggactgcactttttcggtagcttcacgaacgtcggtgttcaaggcatcttggtcaatattttcaggaattgaaattttggcggccttaatttgactttcaagcgtggccttttgatccagttgcttggccagttcggcctgaaaggcaacacctttttgaaatgcttcgtcgttttcaacatgtcgatccttcaagaaggtttgtttttgctgggtcagttcgaccagcttggcttttgcggcagccagtgtcttcttctcctgagtgagtactgcttgttggtgctgataatcggtagacaactgctgccaatgagcaacggtcttgccgatggtttcaatggcggtcgaatactttgtttgatcaaacttcagccaatcactggcaaattgccattggtcaaggtaatcctggtacttagcctgctgttcattgagtgctgttttttgctgttgataactctgttgcaggcgctgaatttctcgaagcgaactttgcatcggcagccatttggcttcatcaattccctggagcccaaattgcttttgaacagccgtcaactctgttcggatttgctcaagtttctgatcgatctcaactgggtcttcatgacttgggcttgaggttggctgggactttgaactccctttggcactgtaccatccccaaagggccgcgaccaccgccagaatatatccaatccatccaaacgaactagagcctaataagaaccctaataccaccagagcggctgccacaccataccagattagcccaccattaccatgaggctgttcggcagactgggttttctttcgagttacctccgcccgtttctcttggagattctgttgctcccgcagcagttcgttcacccgagaaaaggtctgatcgtcaaatgcttgtggtagatttccctgttcatttttcgcaattgaggcagactgggtctggatttgtcgttgaacgtcctgcagctgagaatcgcccaattcgattgccaaagcaacctttctggcggctggcagctcttggtataaccgttcgatcgtgtcgctatgagcctcatagaaggtttgaaccggttttctggatgactggcgggccacttcagcgacggccgtttcagccttttgaacatccgcgctttcagctgtcagtgccatgtttaatttattaaactcgttgagatcagcatcaccgaattgtggcttcaactgagatgaatcgaccgtgttgagatcgtttagcctgttaaccagcggcatgaccgtctgcagtcggcgtttgttatccaactggtgattagcagtttttaaatcagcttggaggtcctttgatttcgcctggtcctgctttaattgaacctgcagatcctggtagtgtgggaagtgggccttggcagcgctaacctgatcttcgagttttttatattccgcaatctgaatattaatcttttttgtacgaccgcggggcgcatacatttttgccgactgcttatccaaattggtctggaggtccatccaatcgcctgccccggcgacaccaagtgattggattcgcagtcgtaattcgtctcgacctattttgtagaaggccgtctgatcaacgctgccaaagtaaaacagttggtcataagcggttcggtcaattggcgcaatgagctgctggtagtcatcagcggtaagctcagtatcgttatccaaatcgtagaattttaccgtcccgccgtattttaaaccagttcggacaaccttatagttatgttgatcagctgaaaaaataatttcaccaccatatggggcactgcccttgggctggtactgaccgtggatggaatgctttttatcagtgaatccaaacaggatccctttgataaacgcgatgatggtactcttgccggcttcgttaggaccataaatcatctgaagtggatttttgatatcaattttttgatcaatccagcggccaaaaccataaatgttgagttgtttgattatcacttggatttatcctcctcagtatcttcatgaacgacattttcctgaagaatcgccccggcttgatcaaagatctcctgtttggattcttcagatccgacttcgtccttgatgaaagttggctgcttattaaagtccttgagaatttgatcaaaaacttcgtcattcaaggttgccgccttggcttgattaaaataatcctgatcaatactgctatagaccagactttttacttgtggggcttcaattgaagtaatccagcagttgagctgctgccacttgtcggcattaatgtcctgcaggtcatccaagagatcaccattattaattttggccagtaagtcggcatcaatcgccgtttggctggccaactggatccgaatgaaatgtaatttgtcgtagtgcagattagcaattttttctaaaattgattcaacgatctggtctgcagacattttatcaagagaaatggcgacccggtcccaaacgatcggtgcggttggcacaaatttggtttgaaggtgctgatcgtcactttgaaccagcaaatatcctttctcacccgattcattaatatggcggccttgggtgttcccggaataattgatggtttgctgctcatttaacgactggcgcttatgaatgtgtcctaatgcccaatagtcataacctttttcctcaagttcagacagtgtgaatggtgcgtaattggcctccggagaattgagtgaacttaagcttccgtgtaacatgccaatgttccaattaacatcactaacggccgttgggtagtcttgaatcatgggttgggtaatccactgcttatcaaagctaaagccgctgacggccacaacttccccatcatttaaggtatactgcttggtttcaacctggttgccaaaaaccagtgtattcgccgggtagccaaatgaagccggatctgccgtagagtaatcatggttgccaaagctgataaaggcttcaattccatgttcgttcaatcgattaagctgagcaactaggaacgcgtcggcggccacacttcgttcttctcggtcaaataagtcaccggccagcaaaacaaagtccacttgctgctcaattgcgtcatcgataattctttgaaaggaatcaaaagttgattgatgaactttctcccagagctcattgggtaaaacatgacttttgagtcccaagaacgggctgtccagatgtaaatctgctgtgtgaataaatttcatgataggtcccttcttcaacttatgtataaaggaaaggccgaggcaaaagtgcacacactttttgtctcggccccttttgtcacgtgcttgatctgcttatgatttgtacaagtcgctgattggttttgtcacggtctcattaatatctgataataactggctcagtgccttttctttggtcattaatgcggaaattaattgactctcgcgcattttcccagcaatcgcctggatattttgaatctcatcttgggttggttgaacgccctgcatttgcttttgctgaagattctgttgagcatcttgaaagtcattgaataatttgtagtcatccaaactcttcttgagtgcgtcataggcagctttgatctctgtaaattcatcggatgcaatcaattcggcttgaagctggttggttgttgcggtcattttttcattcattaaatagggtcccctaacaattttatttacttaattctaacacattactgaaatggcttcctgccaaagttagtgtttgaaccagcttttggcatcatcaatcaaatctttggctttttgttcgatttgattaccatattgattcgttttcttttgaatggtatcccaaagattgtcattgctgctttcaccttgaacgatggattgggcatccttggtgttaaagctggaattcttggtatatggtaacattgtctgcatttcgtttttgaacagtggcccgacaccagtcccactcaagttttccaaatggtgggcctgactggtattatcaaatccttcccaagtcgccaccaccaaatctggcgtatagccgatgatccatttatcttttgtggcgtcagcagagccggtattatcggcttcggtacttccggtcttacccgcaacctgatacccatacggcttggcgtcagcaccggttccattgttaaataccccaagcatcatgctggtcatctgtttggcaaccgaactggacataatttgacggccttcctgcttggccgtgttatcgaccaccactttacccgtagaatcaacaatcttacgaatataaaatggtttaacaatcttaccgccgttggcaaaggccgtataagctccggccatttgttgaggcgaaacgccgccggacattccgcccaaagcgagcgccagattcttgtccttcttagtgaccggaatgttaaagtctttgactgattgataaccgcgattgacgccgatctgattcagcagccaaaccgccggcgcgttcatactttgcgctaaggcttcgtacatcggcacttttccttgataaacattgttatagttttttggtgtgtaatgattggtgccataagatttcttcttatcaaccagttccgagtcgaacttatagccggcttcaagggccggcgtgtagacagccaacggtttcattgtcgatccaggttgacgggtaatctgagtggcccggttgtaaccccgaaagacgtgcttaccacgcccaccgacaacggcagtcacgccacctgtggtcggtgaaaccccaattgatgccgcttgaacttcggtgccatcagccgcattggccggaaacatggcattgttattaaagttgttctgcatcgcctgctgctgagcctgattcaaattggtgtaaatccgataaccccggttcatgatctcagattccgtcatcccatacttgctgatggcttcatcaatgacggcatcaaagtaatatggatacttgtaaccgtcttttcgaacataggtatcccgcagtgtgattggcgttttcttgtagtaatttgcttgcgcctgggtcagcttattattttcaaccatcagctgtaaaacaacgtttcgtcgccacttggcggcctttggatgatcaatcgggttaaaggcacttggcgatgtcagcatccccgccaaaacggcagagtcaggtacagataaattgacagcattttcaccaaaatattttctggcagcatcctgaaccccccaaacgccgttaccaaagtaggcattgttcaggtacatggtcaggatttcgttcttcgagtatacattttcgacttgaattgagaggaataattctttcagttttcgagtcatcgtctgctcttgagacaggtaagcattcttgaccagttgttgggttaaagtacttccaccaccactaatatagttgcgatgaagcagcttgttcttaaccagtaaaaacatggcccgggcgattcccttgaacgagaaaccgtattcatgataaaagttacggtcttcggtggatagcacggcctttggaatgtttgccgagacttgatttaaatgaacataagtccccttttgagcgtataattcgccggcttttttattattaacgtcaaaaatttcagttgtctttgagagcgaggattccaagttctggacgtgggcggttttggcaaggaacaccaagtaggtgctggtcacaagtgaaatactcagaaaaatgaccacaagccacttaaccaagtggaatcttcgacaaaatcggttgaaacgtttcaaaaaggtcccgaccgattttctaaatgagttggtagaattcttattcatgcgatactccttttgtgaatacctcaatattgtatcatatctgaaaagtggcgaaattcagggtggaaaaatttaacgaggatttaaaaaagagcgcccgccacaagctattgatcaatctgaaatttttcgaaacaaaaagaccctctacctggttggtagagagccttggtttcaaatacaattagattacattgcgtccggtgctttgacgcccaataagttcaatgattctttgagaacaattgaaaccgccttgaccagtgacaaacgagctgccaattgatcatcttccaccaaaatctttgagtgcgcataatacttgttaaaggatttagcaagtctcaaggcatacttggcaatttctgatggctcaaagtccttgcaggcactcttaacaacgtctgggaagtccttcaatgcagtgaccgtttcccaagctgctggatcatcaagctgcttgttggcaccatgaagatcaatgtccccggcttttctcaaaatactttcggcacgggcgtgtgaatattgaacgtaaggaccggtttcgccttcaaatcgaagttggtcttcaagcacaaagtcaatgttgttagttcgctcattcttcaaatcaccgaagataattgcgccaacaccgacttctttggcaacttcatccttgttaggcaaatcagggttcttcgcttcgatttgcttcttggctaagtcaattgcatcatccagcacttcatccaacaagatgatccggccggaacgagttgacagtttcttaccattaaccgtaatcagaccaaatggaatatgatgcaggttttcggcagatggtaagcccatttcaagtaaaacggccttcaactgctggaagtaataagtctgttcggcacccacaacgtataagttcatggctggtttgtaagttcgatcacggtaaatggcagtggcgatatcacgggtaatatacaatgtggcgccatcactcttcaagataagggctggattcaaattatatttatcgagcttaacgacttgagcaccttgggattctacgagcaggcccttgtctttgagaatttgaattccttcgtccatcttatcgttatagaaggcttcaccgttgtaggtatcaaaagtcacgcctaatttttcgtagatcttgttaaatgattccagggaaactttacggaaccacttccagagaaagacttcttcttcattgccgtcttccagcttcttgaaagtttcacgggcttcatcatccaattcaggatgttctttatcttccttatggaacttaacgtaatacttcaccaggttgttgatgggatctttcttgacgtcttcttcgttaccccacttcttgtaggcaacgatcagcttaccaaattgggttccccagtcacctaaatggttatctttgattggatgatagccgtttttaaccaataacttggcaattgagttcccgatcacagttgaacgcaggtgtcccattgaaattggcttggcaatgttaggtgatgacatgtcgattgggacattgccacccttaccactgtcgttttgaccataggctgagccttcttccaaaacctcattcaaaatttcattactgaagtttcctttatccaagaagaagttcagataggcgccctttgcttcaaccttctcataagaggattgatcgattttctcaactaagtcttgcgcaatggcatttggtgctttatggaaaactttagccaatgagaaggctggaaatgccaaatcacccattgctaaggtcttaggcttttcgagcttctcataaacctcggctgatgacaattcgtcatttaaaacacttaaaattgagttcgtaacctgtgctttgtagtccattaatgttccctccatctataaatatacaaaaaaactcttacaagaataattgtaagagacgagtaaacccgcggtaccactctatttgataaaaatatccgctcaaagtattaaattcatattctaaaaagcgcgcttcgctgactcaatttttcggctcccaccatcccgaaatcgctgacaattcagtgaccagctactgttcttttattgttgaatatttataacgttcaatgtgtataataacttgttgacccggtatatgtcaacatttatcaccacaccccagtgctgagacaaccaacactaagcgggtaacgggaatcggacccgcgacgcaagcttgggaagcttgtgttttaccactaaactatacccgcataacaaaaacaattatatcattttaaattatctttgtcataaagatttgaaatctctaaagaattttggaaaagattgcttttttgtcccaaaatacagatacttaacttaagaggtgatttgaatgtggatcatattgaactacagctgttgggcaattctattcgtcaattttatctgggggttaacccgatccatgaaaaagcacgtcatcgattcgatgatgatcgcccgcgtcttctactggctcatcatgattagccaagtcgtcatttcacttcgttcatttcaccgtcatccactgctggttatcattggcacagtggtgacgctggcagtgattgcattaaccgaaaccgcttatggccgaaagcaagacgtcaactacagccccaaactgctgtggttattgatgctcgccacgccaatcgccgtatgcttacaaactttggtcaactattaagttagttggctatttattttgcccgatttgcttcggccaattcaatacacttatcagccaaaaccgtctgggcgtcgatcactggataatcgtgattacccgcccgctgctgggcaactgacagttcagtacagcctaaaataacgatgtcacattttaacgattcaaccatttgagaaagaatcaggtgatacaatccctcatcgacctcgtttttggccttgatatcatcatagattaaggtcatcgtctgatcggcaatcttgtcggttggcttaactaattcatagccggcattaataatttcatgatcataaatttgatcatgtaaggtaccttctgtcgcgattaaaccgacccgtttggcatttggcgcataatccttaatggctgcaacggtttcctttggcatatgcaagatcggcacatccgtgagtttctggagctcatcatagaagtaatgagcagtattgcaaggaatcgcaaaaaaatcgggatgtagggcactctgctgcttgacgtcttctgccagcgggatcaatgggttgggctttgagtgatccaaaatgtagtctgtccgatcgggaacggtcgaatgattgaccaaaatatagttcagatagtcctgatccttcgtcgcctgagtccgatcatttaaaatatgaatgaaggtttcagttgcttcggtgcccataccaccaataattgtaaagaaatttttcaactaaatcagtcccttatttttcgacaaagtatgtcttaaagctcttggcataattgtgcatcatccacttatataatgcaaaacgtttgatatttttatccttggcgtaccagaaagtgtcgccatatcggccttcgttgatcatttccatggcttgctttttggcagcattgtctttggcatacttttcaaagatctttggcgtgacaccaagccacaagaaatattggcgtgggtccttgttggcatacaaggtcgactggtccttcagtgaatcgaagacgtaatcttgaatcacccaatcagctaaatgatggccgttcaaggttacaaagaaactgctccggccggtccgcaaattgatttcaaacagtttgtaagaattgtctcggtggtcaaatttcaaatcaaaattggcatagccgtggaaattaattttttcaaggaacgcctgaactttgttgtagatttcctgattaaattcaggaatgattgcgacataattgccaatcgctgccggcgctggatcttccagtagtggatgacccagacacatcaatttaacttgatgattcttatcgacatagacgtttaaagtgcgcatattactgtcgtcaccggggatgaagtcttggagaataaagtcggatgtatagccgttatcataactcttggcaacaatctcccgaaattctgcttcactcttaatgataaacgcctttttgcgtccttcaaagtgaatatcaagccactcaacactgttggccggcttcagcgcaaccggatagccaaatggctgttcaatcggctcgcccgaagcatacatggctttggaaatgatcctcgttttcgggtatggtaagtcgtattgatcacacatcttgtagaagttttccttgtcgttgagcttcttaagtaaatcatagtcaatgtatgggcaaatgaaaacatcttctagttcggccttgtgtttggcaatgagttccgcatagccatccccacaaccaatcaaaatcaccggttcttgatgattggcataacgtttcttaagctgcttcatcgtatcaatccagactggatcctcactaaagcctgggatcagctccaaatcaacaattttggtgaagcgcgtcggtgccaattgggtttgggcaaatgctttgaccggcttgccataaatttcgtataaacttctggccattccataggcgttaaagtcactgcctaacagaacgggtgtaaaatcaagctgcttatttttcattactagagtcctttcacgagatttttaacaattgccgcatcaccttcatacggaacgtttttgccattaatcttttgatactgatcatgacctttaccggcaaccactaccaagtcacccttctggctttcggaaacggccttggtgatggcctgcttgcggtcggggatgtaggttgtagccacttttgaggtatcgatatgagcggcaatttctttggcgatttgttgcggatcctcggttgccgggtcatcagtcgttaaataagcctgatcggcagcctcgttgattgctttgccaaggccctcgcgacgatcaattcccttatcacccgtgctgcctgtaataaccgtcactttaccgttaggagcctgttttttcaagaaatcgagaacggaatgtaaactgccatagttgtgggcatagtcaacgtaaattgttccatgatcatgggtctgatatatttccattcgcccgggaaccgttgtattggccagaccataagcgatctcagtcggtttggcccccatcaaggcgctggtaatcgcagcggcaactgcattgccttcgttataatctccaggaattccaatccggtatacaccgtcaatgttcaattgcttcgccttggcggttcgggcagtcacttggatttgattttccgtcagcgaatcctttaacgaccgatactcgacatctactggaaattcagtttcctgattctgcccagcccgtccataaataaagatattttcaggttgggtggttgctttagccgtgtaaaagatgtcggttaaatgtgtcccgtcagcgttaagcacacaaacgtcggaattaaccaacaactgttctttgcagtgcaaatagtcggcaaaagttgggtgctcgttgcgaccaatatggtcaggtgaaatgttgagaaaaaccccaacatcgtaatgcagaccataaacccgattcttcttgtaggcttgcgatgaaacttccatcactaaatgactcattccattatcagcggcttttcgcatcatggtaaacaaatccaacgattcaggagtcgttaaatttgatttaacaacatcttcgggctttaatccgacaaccgtattgatggttgaggataaagcaacctttcgctgataagtttgatccagaattgctttggtaaagtaagcagatgtcgttttcccctttgtcccagtgtaggcaatcgttggcaattgatcttgtggaaacccaaaaaatgccgcacttacgagcgacattgctttttggatattcttaacaataatgcctggaatgccggcattttggtatgtcttttcggacatgtacgcggtggcgccattctgtctggcatcatccagatacgcagatttgaagttccccttacagaagaacaaacagttgtcagtgaccaatttagagttatatgcaatctggtcaaagggatgacttgagctgctcaattgactttcaagcaataaattatgttctttgagtaaaactaaaacctcagcaacagtaatttgtgccaatatgtgcaccttccattctttgcatatttctaaatctgggtacgatgaaccaagctgaccgtgttctcagttgtatcttctgggaagtaaacttgataccagaggataaaggtatagatggtgaaaattttctgcatgttggacttaccttcagcatgctccttcaacagacgatccaattcgttggtattgaagaactttttccctgtatcagaatggaaagcattcacaattcgttcgtgatacttgggatcgttaatccagctggcaattggagatgggaatccgagcttctctttaagggcagtcttcttaggcatttcccgttctgctgaggttctcaacgcaattttggtctcatccggtgtaattcgtgtcttgaccggcatggtttcggcaaatttggcaacttccttatcaacgaatggtacccgaacttcaagtgagttacacatactcattcgatcagccttatgaagaatgtcgaacggcagccaagtgttaatatcaaagtactccatttgggtcatttcgtctttgcccttcacatcatcaaagatgtgcttggtgtaggcgcctgaatctgtgttaattgaaggatcttttaacacgcgattgcggtcgtcgtaattaaagacgtagttcacacgatagtaccgttcactcaacggctgggcaccacgaaccaagaaacgtttaccgtggaaacgaggcagccgtttggcaactgcagccagccccttacgaaccggctttggtacatacttctgataacgatcgaatgggatagcttccagataggtgttgtagccaccaaagaattcgtcggccccttcaccggacaaagcaaccttgacgtgcttggaagtgtcctttgataaataatacagctgaatggccgctggattggaaagcggctcatccatgtagtacatcatagttggcaggaaattgaagtaatcatcgccattcatgtagattggcgtattcttttggttaatggtcttggcaaactcagtcgaccaagccaactcactatatttggagtgatgaaaaccaatcgagaaggactggatcggctttaatttggcagcttcgtttaatacgtagcttgaatcaattccactagacaggaaactaccaacttcgacatcggcaatcatgtgggccttaacagaatcatcaatcaacttaccaattttgtcggcgtctccttcaatggtttggctattgtcaatatgatcgtagttgaatttgtagtaacgatgggtttcggttttgccgttcttatgaaggaaatattgacctggcaaaagtttgtagacgtgcttgaacatggtttctctggacggaataaactcaaagctcaagtgaattggcagcaggcgcaaattcagttccttattgaaattgggatgctccagaaatgctttgatttcagatccccaaaggaacgtatcaccgtcatcgtaatagtacagtggcttaattccgaagtgatcccgggcaccgaagacctcattgttctttttatcataaatcacaaatgcaaacatgccgcgaagcttgtctaacaaggctgggccccattcttcgtagccgtataccaagacttctgaatcaacatcagtcttgaaaacatatcccaaatcgcgaagttcttcacgaatttctttataattgtaaatttcaccattaaaagtcagtactttagtttggtcagcgttgaacatcggctgacggccatgtgctaaatcaatgattgaaagtcgacgaaatcccattgaaacattgtcgtcggagaaataagcttcgtcgtcggggccacgatgcttgatccgatcagccatgctattaatggtaccttctggaacatctttttggttaacgtaaccaacaaatccgcacatattttatacccctttatcaaatcttcttggttagtctgaaattaataacgttttatattttatcagattacatagattgctaccagtagtataaacctttcttaaagaacggcttgactaaaggaaattaaaacactttcgaatttcattttaccattcttttaagttatactttagatagagtatcaaattgtttttgaagggagagatacaaatggacgagatcgtatttttcaacccgggagattctatcggcaacttccatgatcacaatgaagctgtcaaaaccgctcaaatttacaaggaaaaagaacacaacaaaaaggttttggttgttcatggtgtcgacaacaagaacttcgatatttttatggccgacgacatcattagtcatgacaatgaaagaaatgcgattcaaaaaccttataagatttctgatcggatttagtgatatataaatttcatcaggaaaagggattcaaaattgttgggagcaattttgaatcccttttagtttatagataaatttatctttagcctttagtattaacaaccaaaacttttgttgtcgcgtttcgaacaacaaaggcggtggtggatccaattaacagtcggttaatcgcatcgacacctgacttaccaatcacaatcaaatctacgtcgtgctcatccgggtaaacgtgcgcgataatgttctttgggttgccaatatcaatggctgtttcatatttaacaccttgtgaatcagcatacttcttggcttcgtcaataatgttctcagcgatcttgtgctgatcgtcatacatgcttggcggcatgccggctgcccctgcaccatagtagaagttggtgttgttaataaccgttaccaactggagctttgagtcaaattgtttggccaacttgcaagcttcctccagtgcctgttgagaatttttacttccatcaagtggtaccaaaatgttgtcatacataaatatcacccttctttcttgtaagcggacacattactgtctacaccactataatgctacgtttatatccgaaaagcaattaataagtctgaagatatatttttaatcacaagcaggtacaattttccggtatgacggctttccaattcagtcaatggactaattaatgttataatttaaatgttatcaaattatggaggaagtggttttcatgaggggcaaaagattagttattggcatattgagcgggatttttgtgattgctggcagcgtgtcgaccagtgcaaaatccaacacgtacacgatgccaaaagtttcaccatcgaaaacagttgtggcaaatattgctttaaaaccgcaaagttcatcccaactgacagattatgtctatgccaccgtcgatccaagttcaccaaattatcatcaatacttaacgccgggccaatttgccagtcaattcggccgcccgacgacagacatcaacgattttaaaagctacttagggaaatatcatctcaaggcatccgtctatccgggaaacttggccatcaaagtcgttggcactcggaagaatttgattcgggcatttaacgccaaacaagtgaaggtcagcaaaaacgattatcgaaccaaagttaaattaccggcaaagctttcggcccaaacagtcagtgtcatcggtgtgtacgcaacgaaacccaaaagtaagaagacaagtcttgcagtaacaccctcactcccacaaaacccgaccccgccaaatactgatttgagtaaaaccagttttgccaaaaaatatggtgccttaaaattcgctgatcattatcaggttagtgatttatataaacaaggtttaaccggtcaaggacagcgaattggcattattgccatggacgactttaatgcaaaagacgtgctcaaatattggcagcaaaccggtgtcaacgccgaccccagccggatcaataaaatttattcaattgacggtgccaagaccggccacttgatcctgtcgatgggattaaacccggctcaaattgaatcaacgctggatgttaaccagtctggagccgtcgcacccgatgccaaaattgatgcttatatcggcctatcattaaaaaacgtcacttcaacgacatcatcttattacaccgcctttatgcaggccgtttcggatgatcgtgataaacaaatttcaaccagcttttcacccaacacggagcttgccagtcaatgggaacaaggtgccagtgcctctttgggtgagtacaacgacgcctttaatctgctgttggaacaagcagctgttcagggcatctccgtctttcgggcaagtggcgactatggtccgcgtgaattggcacttaaacaattcaaccacgttttctcaacttcgccatatcaagtcattaccggcggcaccacattaccctatactaaaattaccgatggccgcttaatcaccattgataaggaacgggcttggggcgacacatacagcaatccacaaaccaaaccggctaattatggcggcagcggcggcggattttcaattttgaatccgacgccccgctaccagcaaggattttccggcgttaacaccttccaggcaatcgatctgctgaaatataagagcggtgggttcttagtgaataaagatccacaaattatcattggcaagggatctggtcgaaacgttcccgatgtttcagccaatgccgacagttacaccggttacgcgacctacgtctccggacaagacctcgcctatgccaaggatggcaaaacggtcatcagcgttccagtcaaacaatggacagtgaacggcggcaccagctttgtatcgccacaaatggctggtgccaacgcggtgatgaacagcgggacaaattcgccaatcggcttttggaacccacaaatctatcaatttgcggtgcaacctgattcaccctttactgtgcttgacgatgctgataacaataataacctgtattacaccggccaacctggtaaactttacaatcaagccactggactaggaaccgtcaacttcgccaaattgtataccaagttctcgtcagaggggcccattaagacaatcgttgttttaactcgagattcgccaacgaaacactcaaggtttaacatgttgataacttaaaattagtcggccaatcctgcttatggataatcggccgactaattttttaaaaaaacggatcaaaaaagaggttgagatcgctatcgtgcaatagtgatctcaacctcttaactttatatgatgccctcggcaggattcgaacctgtacttgattgctcaaacagcgacctgaacgctgcgcgtctgccagttccgccacgagggcaacaacatgttttattttacactaaaagtagtaacttgaaaagaagttttgtcgttttgttttgaaaaccagatatcggctggaacttggatcatgtttcatcatcaggtaaccaatcaaagccatgaggaaagcccctgccaaatcggcgatcaggtcagtcatcgtgtccatcaaggctgctcggccgagcaacaacttgccagcttcttcataccgttgcaggttcaaaccacccagtccatcagcggtaaactcatacatttcccagaaaacaccacaagtcgttccaaacgtaaaggcaaacagactcatcaagaatggcttgttggttgcattatctctggcactcatcaatccttgaaaaattgaaaatcccagtccagccaacatcattgcggaaaaaacgtgttcatacttatcccaaaacggtacactgtaaaattgcaatccggatcctaggaaaatggacatgtataagaaaatataaaagaaaaccaattcaatctgtggaaaataaaaccggcccaacttctcgattaaaaatggcaagctggcaatgaggatcccaataaagacctccaccaagagcaacgtctgcccgtgaaattttggttgtcctttcattaaccaataaccatagtaaccaagataagcagccattgagaccaccgtaatccaaaataaccaggtactaaatctaagtttaccaattttcatatgtaacaatccccttttatgtcaaattaattgtccgcaattaatttgactccctgtgttaagtcttgcttttaaatataaatacattacaataataacataaagtatttaaattgattcgactagtgctgtccgtgtttcacggcagtatgtgcaaaaataataggagttgaaattatgcctcaaacccaaccaattcgcttggacggccaattgtgtttccaagtctactcagcgaacaaaaaatttaatcatttttatcagcaggcactgaagccttttgatttaacttacccacagtatattgcgatgctgactctgtggcaatatgcaccactctcagttaagcaattgggcgaatatctccacctggacagcggcacgttaaccccattactcaagcggctggaaaatcatggctggatcacccgctcccgttgcgaagcagacgagcgaaccgttgtcatccagttaaccgacaaagccaaagagcaacaggacaatgtcttcagtcgtgtgaacagctgctttgatgttttgggattaaccccagctgaaaaagaagcttgttctcagacgatggcgaccattgaacaaaagcttgatttgtacaatcaaacacagatctaaacgctctgaccaaaatgttaagattttggtgcagagtataatctaatcataaatccaatttaaaatcgaggctgggacaaaatgaaagattttgttccagcctcgatttgtgtttgaatgttatctgatataattgtgggccaataagcagcttccgaccgtataagggggattatccaaatatccaactggaattcaggtaatccctttatactgtggagcctaattgcttattggccgacgcttgcttttttattcatgccagccaatcaaccactgactggccaacttgattaaatttttggatcgtttccattcggttcaaggatccagcagtcaacatggcaatgtcaacagaatggttgttatatacaatttgagcgacatcatggtcaatcaaattgccctcaccagtcttattgtatacagcaacattctcgcctgattcatcaaaattacccggtagtttgtatcggaactgctgattgacgaaccagctctggacttcggaaccattatgaagtgcttgctgaagcagccgcaaactttcagtggcactggtatagttatttttgccactggcaagtgcccgaccgtccatcagataacgttccagcctggtctcgtggaaatcatgggtttgaagataatgctgaatatggttcattcccatcaaggagatcaccacattagtagccgaattatcggacacactaatcatcaacgccaacaagtcccgaagcttccatgaccgaacagacatcaattgtaagattccggcaccgcctaccaactcatccgtcgaaacatcaacggattgatccagatcaacgttgctgtccaaaacatcgtttaagatggccaatttgatcaaagaagccgatgggaaagcctcgtggctatcatggtccaccaaggtctgaccgttgctttgaattaacaagccatacttaaacgaactgtcagccatcacccgttcaattgtttcagaaagctcactcatcgccaatatctcctaaagccggcaaactcggccgcaaattttggttcagtcagttcggcaatatcgactttggcgcctggcgttcttgattcaatcatctttccattaccaatgtacatgccaacgtgatgcacgtagcccttgccgtgatcatacgcgaaaaataccaagtcacccggtaggatttcttccggtgctaaaggtaagccgttttcttgttgatcgtcagcgtcccggggaatatcaaatccaagtacccgatgaagcgtgtacgcaaatccagagcagtcaaaaccataggaactggttccaccccaaagataacgctcgcctaaaaattggcgtcccatctcaaccatcgtttcaccagcattgctcccaacgaatggcagtactgctgctgatttgtcaatgaagccctttccaagcggggtcacaacggcaatgtagtcaccactggtgcctgtttgtggcagcacagttcccaagctgatttcgaggaccggctttttgttttcatcatacaaattggctgtccgaacagcaattctcacaattgaggtaaccggtggataactaatctgctgatcgcttaataatttacttggcacccaaccaggatagccccttgaatcagaatcatctcgttgactgggaatatagactttggcccagtcaccgtcgaaatgatcaataatgacttcatcgttaaacaaagcctgcgtttctaataagtcatcatcggaaagcgcaactgattgctcatcactcatttgttcaacccattttttaccatcgccgtctaaggctggttgatcaacttttcttggtgattctttagacttccaaatagttgccactggaactttgactcgtcttgtttccatctgggcacctccattcgttaaattttagtatacatatattatacctcattagccaccaactacctgctagatagcataaaaagcattgccggcttgttcaccctactcaaaaaggccggaacatgaggaatccttatgtccgagcctcttaggttacttaaatcctaatcccggtaaatctggaaaagagatttcgtttttttgattgatgatcccaccgacaattgggttgctggagaacatcatcgatgcgtccaaatctacatactgaatatttcgtttggcggcggccaagtgagccgcagcagtaacggaaaccgacgattcaatcatactacccaccatgcagggaattccggcagcctcggcaagggtattgattttaaccgcattatcaatcccgcccgccttcatcaacttaaggttgataatatcacaaccacgcatactaatgatgcgagcggcatcttcaattgaaaagatgctctcatcagccataatcatcgtcgtggtgttggcggtcacgtaagccagaccatcaaagtcagtggctttaaccggctgttcaaccagttgaatgttcagattcaaatcctgcatccgattaataacggcgacagcctgttttggatgccagccctggttggcatccaaacgaatttgaatggctggcccaactgcttttctgatggccacaattttatcgaggtcggcttcttcagaatcatcccccaccttgattttcaaagtggtaaaccctttggtaatcaagtcttgtgcttgggtgatcatatcctcaatcgtcccaacactgacagtataatcggtcgtgatgtgatccgagtgcccacccaacagttgatatagtggcaccccatacgattgagccagcaaatcgttaacggcaatattcaaagcagccttcggactcgaattatggaccattgactgatcgatagtcgccttaatatccgctgagtcaaacaatggtttgccaatcaatttcgggccaatcacatcgttaatggcactttcaatgcttggaagggtatctccggtaatcaccggcgttggtgctgcctcgccataaccgactttaccatcactggtagtcattttaacgatcagcgtctgggcagtggtgacagttcttaatgcagttttgaacggccgtttgagtggcacagcagcttcctggacatcaatctttttaatcacgggttccaataagtgtcactcctcattaattatttaacgtaagcctctttgaaattgtagttggcaccagcagtgttgtaaacaattcccttaacttttgaattaaccatccatttttcacctgattggtaaagtggaatgattgcttgatctttcaaggccaaattctgagccttaaccatgtcatcccaacgagcgttggcattgctgccatcgtcagcgttgctggctttgattaacgaatcatactctgaattcttccaaccggaaatgttgcttgggttattggaagtcaaaatgttcaagaatgtgattggatcggagaagtcggcaaaccagttggcaacggtcacagtaaactgaccatcagcttgtcgagataaaattgaacgaccaggaatgttgttcaaagtgaccgttaagccaggtaacttttgcaaggcactttgcagatactcactcaattgcttttggtcactgccatcagagttcaacaaagtaaagtgtaatgacgaacgaccaacttcttgaaggccttccttaaagagctgtttagccttggttgggttataagtcattgatgcgggagcggttgtgtctttcgtaaagtcagttccgttcttcggtgaaacggccaatccctctgaaacaaagctattgttatcgattgcgccgccacccatgactttgttggctaatgtctttcgattaatgatcattgacattgcctggcgaattttcaggtttttgaagaccttgttcttttggttaacagcaatgtagtagttggaagactgctttcgtgaaatcatatctttcttgttacccatttgtttggcctgggtagctgaaagttgcgacatatcaagtttgccttgattgtaaaggttcaatgacgttgaaggatccggttggacactgaacttgatgtcatcaagcttaacagctttcttgtcccaataatcggtgttcttcttcaaagtccacttgttattggttccagtccatccagtcagcgtaaacggtccgttataaacttgggtcttggcagaagtgccgtaatcgttgccatatttattaaccgccttggcatcttgtgggaagaagacaggaaagcccatcagcaaattaaagtatgggattcgctgttccaaggtcacagtcagtttataattaccatctgctttaattcccaatgaagaaactttggcttttttgttttgaatcttgtcagcgttcttaattcctgagaacaggtaaccatactgtgaagccgtcttaggatttaaggttcgctgccatgaataaacgaagtctttggcagtcaccggatcgccattactccatttggcacctttacgcaagttgtaagtgtaagtcttaccatcctttgaaaccgtccatgatttggcgattcccggttcaactttactattcttgcctagacgaaccaacccttcatcgacgttgtttaaaacgttgaaagttccaacagccgtggtcttcgatggatcaacagtcgtcagttcagaatcggttgaagtcttaatcgtcttgttggcttgaccagacttttgaccacaacctgccagaattaatgcaatgcttgctacacctgcgagtgcagccactcctcgagataaatgcatgatataatcctcctctaatatgtaagacgcgtaacaaactcatcttggttctaatttagcataaaagtgtcaaaaaaacaggccttttctaatattgagttcagaaagcctgttagaatatgcgattttgctgtgaattttacttagtaattgcgattgccatcttacgagacagataaatcggctcaaatttggtttttggcagccagtattgaccgtcaatcggatcactcacgtggacctggtcgccatcgatcccgtccaacaaaaccgcgtgattattagccggaacctgaccaaatggatacgaatcccactcaggttgttcaaaacggacggtcacaaaggttaacaccggctccccttttgccacaaagtcatacaaccactggggatctgccccactcagttcttgcagattaccataacgatttccccaccacatcaagggtcgggtaaagattgcctcaaacttgccgggccgattggtgaaaggtgaaccaccaaagccgtggtaaggattgctatctggtgaaattggcatctgaaggagaaattggccataattcaggtctaaagctcggccctgataatggagcccctccagcaagctggctgcttcacagccgttgacggcaccccaggcaagttggcgaatgttttcagcacctaataaaatcttcgcactcatttgaccaccccaagctgtgaaaagacctgctcaaccatatcggtataatccggctgctgagaaatcaacttcttgcatgcatcaactaaatttaaccggagccgtccctttcgatcaacgactgattcagcgtgcaccattgaacttaaaatcgcctcatcgacgaccgctgccgtagctctgaagaataaatcaatttggttatcgttaaaccgggtaacagtatcaaactcgctggtttcaaaatggtccaccagattggcagttgaaaatgctaaaacgatttctccgctgccgttgccaatgtagccaccggaacgattaatcccaaccgttgcccgcttagccattcgcttgagttggcgggcattcaatggcgcatcggttgccaggatcgtgataatggaccccttttcttctttttgcttatccttggccaacattttggccaagggggctccaataggcatcccattgacaataaagtcggttaaataaccatagttggtcatgacgagtgcgccaacagtgtattggtgcttcttatcaacggtcacaatccgcgaggaagagccaatgccgcccttgagatcatagcacatcatcccgcggccactaccgactgcaccttcttcaaagtcatcgttaacagcagccaaagcatcggacacattctgttcagtaatcgccattttgcggatattggacacgtcgccatcgttacactcagcaacaatcagattaactgtactggtggtatccccaatttcaggattgtcagccagcatttgtttggtgagggcatttagggccgtgcccacgccaaaggtattcgtcatcacaatcggggtttcaatggttcccaattcatcaatttggacgaggccgacgcttttaccgaagccgttaagcacacaagaggcagctggtaccttgtgccggaaaaggttgccggtatggggcagaattgcggtcacaccgctatgaacatcaccatcatcaatagtcacctgcccgaccttgacgccgccaacatctgtaatcagatttcgccgacccttgaggccatccgaaagatcattcatcaatttaaccgataatcccatgattaacacctctcacaattaattacacagcaaaaatcatcgcaatcattccgccgactgcgattaaattattcaaaaaatggaggccaattgataccttcaaatttttagttgttacatacaaataggccaaaatacaacctaggatcgcatacgtcaaaaaactgatgatattaaaatgggaaagatcaggatccatatgcggcagggcaaaagccatcccactgacaataattggtgcccatttttcagtcgaccgaaagaacgcagtcatcaaatatccccgaaaaatggtttcctcaagaatcggcgaacagaagattgccgtaaatcccatcaaaatcagggtaagatgattgctggacaacaatgattgaatttcctgattgttgtccgtttgagtgacgtgatagaccagtttattaaggtttcccaataagaactcaatcaccaaaaaagcaatccaagcaatgacaattgttttgacatttggccaggtcatttttttgacttcgtagcggccatacttccggtaggcatactgtgccagccaaatggcgattagaaagcccaacaaatacaaagctccaacagcgtaattggcaactgctgacagcttgccttgggcaatgaacatcagtggcagctgaactgagccgaccaaaataatcagcccaaaaaagatcattaatcgttcaaagtagtcaccaaaagttaactttctttgctcttccatgcagcgtctccttaactattaaaagctttgttcaaagctgtaaaatcaatggttccaagtccggtcgcctggttataaatcttccccggctgtccggtatagtacaaattggtgttatttgtccgactgtccaacggtttgaacggcgaagttgatcgtttggcaaatcgatagatctgtggattccaaaagcccaagcggccattggtagtgaaatcagacatcaaaacactggctgcggccatttgaggggcgacgacactggtcccaccggtaatcagccattgccccttggaatttcgattattcttcggggtaatgaacatgctgtaacccgtattggggtcggcattcgctgaaatgtcgggaaggtttctgccgctggatttaccgctaagattaatcggctttttcaacaattccggccggccatatttaaatttccaaagattagtcgcatcatacgtcccgacaccactgatccctttttgataggcgggtctggcattatatttactaaaaccgccgccacctccggcaaagaagctttgaagcatgtccaaagttccgaaaaatcgttggtgtttatagttggggtataaaaagtcagccccccaggcgcgttcctggtgaatggtgacttttttcttattgacagtataggttttcggcagtgtcgtgccgccgactgcggtcacatatggagaattagacggcgtgtcaacggacaatcctgacgttaaaccggtggtaatcccatcataggcgccattatcaccagtcgcggtgaagacactcattccttgggcagctgcctgctcaaataataagttcatgatttgattatattttttcggggtaatcccctgtttcatttcataagccacttgggcttcactttggccccaactaagtgacaaactgtcggccacgttttgaccaactgcggcagcaattgaattcaccatccccaaaatatttgggcgggcaatgtaggtccgaatgttgctgtccggtgcgattgcgccggcctgttcaacgtcgatggtcgtttcatcatagccatcccaggtacccttgaagccgttagtccgataaacgcttagccgattggatttcacattgatgccctcatcatcccagtagcggtacacatcattaggatggaagttggcaaatgaaatgataccaatggttttactgcggccagtcgacccattatcgtatagggactgtagattgtagcgacggacaaaccgcgtcggtgaatacttcttggtggttgtcgtcccgctggcagctctggtatgcagtgaagagggctgaaatttggttttatatgaagaaaacggtgagtaatttgataacccaaagacggtatagacaaccttggaaagtttcttgggtagttgaggatttcggctggccttttgatatttgacctcaccgttattgacgttcaccaggttaaccttaaacgccttctcaacgtttttggttgatcccttgaccaccataatcaaattacctttgtaagtctgcgcctttaaatgatggtgtctgagataggtctgcaaagctttaatctgctttgggctctgactgaatcgtttggcaaaagtacttggggacacaaatttgcgataagtcggtgaactcggcgtcactgtgttgtagacaaattggtgaagtgccgactgactttttggccgcagcacaatatcaaccaactgctgtttggagtcagcaacgttggtcgtcttggcagctgcctgcccgctggttgccgcagagccaccaatggcaagcaagatcaatcctgcggttatgaaaatcctgtggagccaatccttgttcatacaatccccttcaaacaatcttatttgtcacgactattgtcgtctgcttctcgttgggcttttctttcatcgcgttggcgaacaatcatcaccaccagcggcgtcaaaatcaggcgaatggcaataattgcaatcagccaaatcagtgcgaacgacaggactgataaatgccaagactttgtgatgaaaaacgccactgctaacactaatacgacggcgccgacgattaagaataatttagactttttcaaatgaattctcctgtaaaatttcttatttcatactatcatactttgccaatggagttcacgtttgaattgggaaagttagagtttgtcttggggtatttaaagtcgatataataaatacatcatgaaaataagctagttgaaaggagaaaaatcatgctcaaagaatttaaggcttttattgccaggggaaacgtcatcgacctggctgtcggggtgattattggtggcgcctttactggaattgtcacctccctcacaaataatttgatcaacccgttaattgggatcttcttaggaaaaattgacttgtcaaacctgattttcaaagtcggtgatgcaacttttcgttacggggcctttatcaattcactgatcaattttctaattgttgcctttgtcgtttttatcttaatcaaactcattaacaaggtcctcaagcgtcagccgacaaagcctgcaatcgataacaaagaagtactactttccgagatccgggatctgttaaaaaataaacaatgagccgtcaatgacgcaccgcagaccattccaaaacggtaattgattgcgattgcatgatgtctgggctagaattaaaagtgtgaaggtttaatttatttcccaaaaattgagaagaggttttgttatgagaacgtttgctattagggcccgcgatggggtcatggaattaaattattcagaagattccaacaaaccgccgtttcgaaagtttatgatcacatataaccccaaattttcaattggcgataatcttgaaaatatcaaagcagcgctgaccggcctgccgatcgacgccgccattatcgaaaattcgttaaactatgagttttcagatacgattattggcattaatcaccaaaagattgatatcggattggcaattgccaacatgatgaatattccggttgttaatctgcaaaagatcaaagaagttgggctgaaaaaagccgttgccgataaggaagaataccttaagtggcatctggattactatggtgaatatgccggtaaacggaactacggccaagaagccatgctgacaatcgggaacggttactttggtctccggggggcctacgttgagtcccacgctgataaggataattacccgggtatgtacgttgccggtgtttacaaccaattgacgactaagattaatgaccgcgacgttgtgaacgaggatttggtaaacttaccgaatgcccaatacattagtttcggtgttgaccatcaactgccatttaccattaagaaagccgatattcaagatatttaccgaagcttggatctgaagaccggtactttgacaaccacgctgcacgttcagctttcaaccggccatatcatccaagtccgggctacgaaagtcgccaacatggatcagtggcaccgttacgcaatcaaatatgaattaaagcccatcaatttctccggcagtttacaaatctatgccggcattgatggcaacgttattaacggcaacgtggaacgttatcaagactttgatcagcaccacattgatgtcatcggcatgtcagctcatgacaatcaagtctcgatgaccggtcaaaccaagacctcacacgttcaatttgtgattaactccaaactcagcagtccagatttcgataccaaaaaattaatcgataccacgactgaggaaggtaaagtccaacaggctttgagcattaacgttgagcccggcaaggaatacgaattcaaaaagaatgtcaccgtctttacttcccaagacgaaaatgatcatttggaagccgatgcacaaaaagaacttgatgactcctcatttgaagatacgctaagcgatagtgaaaaattctggagcaatgtttggcaacactccgacattattatcgataatgatcttaccagccaaaagttgaccagggtcaatattttccacatgttagttaccagtgctgctttgtcctccggtaaattggatgcatccgttggtgctcgtgggctgcatggtgaagcttaccgtggacacattttttgggatgtcacgtttgacttgccattctatgcaattcattaccctgcgattgccaaacagtgcctactttaccgttacaaccggttagctgaggcgcgaaagtatgctgcctcagaggacaaacaaggtgcaatgtatccttggcagtcagggatgtatggcgatgagcaatcacaatttgttcacttgaatccggttagcggcaaatgggatcccgataacagccgcctacaacggcacgtttccatttcagttgcctatgacattatcaattatgtccacatcacgggcgataaagaattcatggatcaatacggattggaaatgctgctgtcgatttccaagttctgggtcagcatgaccgactacgatcaatcagccgaccgttatgacatccatcatgtcatggggcctgacgaatttcacgaagagtaccctaactccaacgatcatggcttaaccaataatgcctatacgaatatcatggtttcctggctgtttgacaaggtcaataccctggtatcgcaggaagacagcgccgttttaaagcaagccagtgaaaaagccggctttgacgacgcacttctcgccaagatgaacgatattgcccataaactgcgattggacatcaacgaagaaggtattatcggccagttctcagggtacttcaacctatccaaactgaatttcgattcataccggaagaagtatggtgatatttccagaattgatcgactgctcaagggcgaaggcaagtcaccggacgcctaccaagttgccaagcaggctgatacattgatggcctactatgaactgccgtttgacgaagtgcaagaagtcatcaaccgtctggggtacaagctgcccgccaacttctttaccagcaacttacggttctatcttgaccggacgactcatggatcaacgctttccagaattgtttattcggttctggacgaaattgacggcaacatggaccagtcatggcagctgttttcaactgccctgttctcagattactacgacattcaaggcgggacgactgccgaaggaatccatctaggtgtaatgggtgcgacccttcaaattgaaacgaaatgctatggcggtgtccggtttgataccgacgaggtcacgattaatcctcacctgccaagcacttggtctaaaatttcatttaaagaaacttaccaaggaatcaattaccacttcgtcatcggtcatcatcggatcgatgtgaccgcagatgccgatactcacgtcagtgttgcgaaaaaggcttattcactgactaagaacaagatggcaacaattacctacaaataataaggagtgaatgataatggcaaaattttccgatattaaaggcttcgtgttcgatttagatggtgtgattacagatacctcggtttttcacagccaggcatggcatcaagttgccgataaagtcggcgctccatggtccaaagaacttgaagacggtctgaaaggcatcagtcgaatggactcattggaaatgattttgaaagctggaaatcttcaagataaatacactgatgagcaaaaggttgatttagcaactgaaaaaaataccaactacttgaagttggttgatcaaatgacccctgacaatatcttaccggggattaaagcattcttggacgaaatcaaaaatggcggttatttattgtcattggcttcagcatctaaaaacgcgcccaaagtcttgcaaaagctgaatttaaccgattatttcccaaagattgttgatccaaaaacattgagtaaaggcaagcccgacccagaaatttatgtaaagggtgctgaattgattgatctcaagccggaacagtgcatcggcgttgaagacgcggcagctggtgttgaatcaattaacgcagctggcgaaacctcgattggcatcggcgacaaaaatatcttaaaggatgccgacattaattttgccgatacttcagaaatgacgttggctaatattgaaaagcaaatgaattaagggttcgtttcatccctaattctgatgattaacgacgaaaggcaactacctctgtttcggggtagttgcctttcgtcgttaaatggtcgagaacaacctttggcgagatattaatcaatcagcccataatgtttaaggccgttcacaatcccaccgttaatatttgatttagtgacaaaagacgccttttccttaacttctgggacaccattacccatggcaattggaaatttaacttcggaaaacatttgcaaatcattcatttgatccccaaatgcatatgatggaacgtcaccgaggttcagttttttcatcaaagcctgaattcccgtttgtttggaaacgccccacttcatggtatccaaacaacgcgggttgttacggaccaaagacaacttccctttgaacttgtcttggtaaagcttatccttgtcgtaattaaagacgtttaagaaattaacttcgtgatgcttgtaaaattctgggtcaacatgtggtgttaatcgcaacagacgatagttcactttcgtcatgtcattttcaaaagtcaacgcaaattccttattgttgtaaaaggaaatgacatccccctgctgttttgcaaaggcaaggatttcctcaatcacatcatcactaatttgttctgctttgagttttttgccttcatactgaacataactcccattagcgctgactaacgagttaatcccagtggcatcaatcacatactgaatttcaaaaatatttcgaccagtggagatcactggtaaaatattattggcacgtaattcattgattgccgctacattttcgtcggacacgtttttttcattatcaaaaagtgtcccgtctaagtcaaagaacacaaccgctttatacattaaattccctccatttaacttattaactatattgtactacttaatatgtgcggcattcccaattttaacttccgaatcgggaaattatatatattgtgttaccacattttgtggtacactatatattgtcattttattataaagaggggctaccatggtgataataactgcaggaatgattggggtcggaaagaccactttaaccggaaaaattgcggaacatctcgggacaaaagcgttttttgaacccgttggcgacaatcccgttttaccgctttactactccaatccaaaacaatacggatttctacttcaaatttactttttaaacaagcgtttctcaatgatcaaacaagcattgagtgatgataataacgtcttggatcgctcaatctatgaagatgcactgttcacccgggaaaataatgctcagggaaacatcaccgacactgaattggcggtttacctcaagttattgaataacatgatggcagaactcgacgagttgccaaaaaaggctcctgatttgctggtgtatgctgatagtgactttgacaccatcaagcaccggatcaaaaaacgcggtcgcgactatgaacagtttgacgacaacccgggccttcaggaatactacttcaagatgtgggctgcatataagaaatggttccaagaatacgatgtcagtcccaagatcaaaatcgacttgcaaaagtatgacttgtccgatcccaagaatgtcacaatcgttctcggacagattgatgatgctttggctaaaattcgccaaccacaaagtgagacactctaacagacagtcataagtttcaggtctaccagatacgatgaaaaggccacggagttaaaaggagatgttcagctgatcatttcacagctaaacagcccttttttattttgccaatttaattttcccaacgattgcgtccggatccgccttataatcgacgcttccctttgacaccaagtaatcaatccggtggcggtaccaccagtcagccgtgaacggataatcgcccaaagtctcaccaattacccgcagaatatttctaaaccgtctttgactgagattggcaaggacaaaacgatcgtaaaagtcaatcgattgactgacaacggtgccgttaatcaccgttctgatcggattattttcactccttaagtcatgccaatagtaactgaaggctctccgggaattagcagacaggtccctttgtagtgatgccaattgaagttcatcaatggcgtcttcactgatttcacctaatttggaaataatcatcaaactgtcttctcggaccaaggtcattggaaccttgacactcgtcgtttgaactgaaaaatcctttaaataatcgcaaatccacaaaaagccgcagtagtcgtcagcggtctcactccaccaaatgcgaaacgattcgccggcctgagccatttgactcagttgatcaagcccctgccgtaaagcatttaccgcttcgacagttaattgttcagaggcttgataatgagcgtattcgattttataaatagtttgtcgactttccataaacgagcgttgactgatgtcccccaagctcaggtacattggcaatgccaaaacctgcccgtcaagatgtcttttctgatagtaatacttcaatgttgatgcaaaactatcactgaatacgatgtcaatcatgaccaaacctcacccttcgaaattgtcatttctcaatgacgtgcttcgaaaagtataacttttttggtggcctggatgcaacttttatttgactgaatcaggccactcttggtaggcttgatataaacaatattgggggagatgtagatttgcaaaatacaaaacaacataaattatctgccgctcaaatttgcggctggatcgtctggtgggtgatcaccattgtcgttttggcgctggcaatctttatgctgaccagaacgacggatgctgcaggcgttcataactcatggaattatcacatgatcgccatttttcttttgctggtgtatggaatccagcaaatcattgcgttctttggtattaaacgacttcactacaatgaaagttatgtgtggccgattgttttaatcgtgctgggcgtcttgggcagtttcttgtacgtgatttccggaatctggggattaattgttaacaatccgcagaaaaatcagccaaccaaaattgaataatggaccacaaaagaggcgaaccaggtattctcgaaataccggctcacctctttttttatttcagttgttctaaccgacttgaaaccggctagtcgcgatggaccacaaacacatcacagggagcttgggcaataacaaaagcagctgtagaccccattgtcatccggtcaacaaaatttgccccggtggccccgacaacgattgcatccacatgttcgtcatccaccaactcgtgggccaatttatttttgggatcgcctgatgtcacaaaggcactgacagcaagtcctcggtcttttgccatcaattcgtatttatgaacgagccgttgaaatctggatttgacctcatcgatcgttgattgattgacgttgccaaaaccgatcaaggcggcttttgacacccccagaatttcacggtcgttgataattgccacaattgtcagtttggcatggttgtgctcggcaatcgtgattgcctgtctaacggccttggcggcagtctttgaaccatcaatcccaaccagaatattcgaataattaaagtccaacatactaaccacctcaatgtttttacttggctgtcaactcataaattgattgcccataaattgccattgccttgattaaatcggcaaccggctgaaactcatttgcctgatgcatggtatcttgggcgttcgggaacaatgcgccaaacgccaccccgcgtttcatcaaacgggcataagtaccgccgccgacgacttccggtttggaatccatatcgcccgtctgttcctggtaaacgtgcatcaaggtactgacaatcggatcacttggatcaacgtagtgggtgtccatattgttgatttccttcacggttccatggcgtttctcggcagcctgttgcaagtgagctaaaatctcttgatcgtcagttcctttcgggtaacggaagttggtgttgacgctgccgccgtgctgcgtgtcaaatttcataatcccaacgttcatggttaactctcccatgatgtcgtcgacgtgcgcagcgccgatcttggttgcccgggaatcgtcatgcaggtcttcagccaggtaggaaataaattccttagcggccccgtcaaatggataggcattcaaaaacttggcaagatacgtgccggcattgacgccgttcttgggttccatcgcgtgggcagctttaccggtaatgtgcaaagcaacgccctgaccggttgatttgacatcaccggcaatcgggttttgatccaaaaattcagtaaagccgtcgacaaatttttcgttatcaccgacttcgaccagcgcatccgcagatccgggaaccatgttcaagcgcaatccggaatcaaatcgcttcaaagtgaattcggaaccatttgtatggccaaaggtcgtgacataagtggcattgcccttctcaccattaatcagaggaaattcagcatctggggaaaaaccaaaggtcggttgcggttcaacttggaaataatgcttcatcccggtccagtcactttcctcgtcagttccaataatcaaacgaatcttcattttgggcataatcccattgtccttcagcattctcaacccataataagcggctaacgcaggtcccttatcatctgaggttccacggccatagacgttgccatttttttccaccatttcaaatggattggtttcccagccgtctccagcaggcataacgtccgcatgggcctgcatcgccattgtctgatcgccggaaccatactcaatatagccaacaatgttgtcgatattttgcgtcttaaagccgtcgcgctccccaaatgataaaaatttgagcatcgcttgggttggcccctcgcccagtggaaattcatcggtcttgtgctcatcgtcacgaacactgttaatactgatcaattcctttaaatcgttcaaatactcgtcttgataactttgtgcgcgctttttccaatcaactgtcatttttctcgctcctgtccatttcttatagttcaattttatcacactattcaattggcgttggcaatctgtccactccagaaatgctataattagggtgaaaaacagattcggatgggagatctgatgatgataaatgtcaaaaaaatcacaagtcaaattttaacagatgtcattcgcaagcgaccggcagatagttttaaaggcacttacggcaaaatcgctttgattggcggcagccaaaactttggcggtgcgattatcatggcctcactggcagcagtttattccggagccggcttggtcaccacgattacggaccccagtaatcaaaccagtctgcatgactggctgcccgaagcaatgtttgtggattggaacaattttgatcaggcagaaccaatcattaaaagtgccgacgtggtggtcattgggcctggtctgggaaccgatcccagtgcgttgaccctgttgacaaaagtctttcggattgccggcagcgaacaaaagttagtcattgatggttcggcactgacattgcttgctgctaacaacttgccgctgcccaaagattcgaccaacattttgacgccgcatcaaatggaatggcagcgagtatccggcattaagattgccgaccagacgccagagaaaaaccaggcagccgccaaacagctccacgcaatcgtggtggttaaatcacatcgaacgcaagtttatgcggacaaccacgtctacgaaaacactggcggcactcctgcccaggcaacgggcggaatgggtgacaccttggccggaatggtcgggggctttgccgcccagttcaaaaatccgcaaaaagctgtgttagcggcggtttattctcatagtgccattgcagataaattagctgaaaagcaatatgttgttctgccccaccaaatcagtgaggccctgccgaaatttatgtataagcatcaagctaaataactaaattgaatcacaaaagtctccatcagctgaattgtcagtgatggagacttgtttattttatcctggctaaatatgaatgaaaacggctggttattcgattttaagcaaccgtcgcaacttgtcacttcgcgggcccagaatcatatcagcaattcgactcttcaaggctaagtagagataaattaccccaccaaccaaaacggccaccaaggtcacgatcagactgacaacccgtccaaatggattaccaatcaactgaacaacaaaattcaacccataaaccgtcaacagtgcagcagcatacataaacaatgaatatttcgaaatcttccgaaaagcaatgtccaacatccgtttttcaaaaccgaaatggcggttcaaatatctaagaatcagccagttggcaacggtcaagccaatcccggtggaaagcagtggcccaaatgaacccaaaaaataggtacaaggccactgaagcacaaacttaaccactgttccaacagcaaagaacttaactgcccgtctgttttgagacaatccctgcatcacggcagaaataacaacaaacaatcccatcggaatggagataatggatgaaaacgttagaatattagcgccgagtgcctgatgagtggtgccatagaagacccggttaagcggtccggcaattgcggcattaccaaggcggcaggaatcatgacaaacatgaataatgccatgacattggagttttgtttgcgaatttcgacgttgtccccgctggtcagcgcttctgagagcatcggcacggcggtaatcgccaaagcagaggaaagcgacacagtaatcataatcaatttatttgagttcacagcaaacattgcatatagatcggacagggtcgcgtagttgtaatcagtcgccatccgcataatcttgaagaaagtgaactggtcaatcagcataaaaatcgtgattccggcacccaatataataaagggcactgcctgcgcaataatttcctgatataattgttttgcttcaacgtggatctcattattgctggacaaaaccagctgtcgaaaatcttcgcggcggcggaagtaataaacgccaagggtcgccaggccggcaaccgccccaatgaaggcagcgaaagttgattgagaaacagcattgacccaactgccatgcagcacccgcatcataatgaaggctgttaaaagcatgtaggcaactcgagccagctgttcgacaaattgggaaatcgctgatggcgccatttgttggtaaccttggaaataaccacgggtgaggctcatcgtcggaataatcaaaattgcccatgccagtgaatgcaaaaccggaatgacgttgggattgccgccgtcaattaagggcgcaccaaaatacaggatcaccgcacagataactcctgtcgcaatggccaacaccaagccccgtttataaagccgaacgccgacaccatactcatttaaggcattgtaatgagccacttgtttggcgatcgctgagggaatccctgcgatggccgcgatcaagaagaaactgtaaatgttatacccgagtccgtacagcgcattggcttggaagaaataattgccaaaccaaatcccccagggaataatatagactgcaccgagaaatcgactcaaaatactaccggccgtcatccacgctgacccggataacatctggtcacgcgacttttccgtcaggttttgatgattatcaatcatgattgttcctactttcgtatactttgacactcgcttcattttaatcaagttgctaatgaatagcaataacggggtgatatattaaaaattacttaagcatcaattgttttatagagatgtaatgaaaaagtattgtcatgaacaccctaaatgcactagaatatttttatatgtggtcttaataattttcgaggtgaaacacttgtgagtaaaaaaagaatcgagtggattgacgttgccaaagcggtcggaattgtcgccgttgttttcggtcacgccatgacacgacacggcaccatgttccattttctttattggtggcacatgccgatcttcttcatcatggggggctttttcttaaagccaatcgtcaataacaattggatcggttttttcaagaaacggattttaccactgctaatttcatatttaatctgtggtggctttttgattttactgtcacacttcatcagaggcgaaagttggtcgtatacgattttctactttgcccgattactgtacggtggacggacactgaaccactacctcagtgttttttggtacattaatgtttacctgttggccctggttttcacatcgattgtcattacatacgtcaaaagccgggaagcacagattattgtggcctttgcttcattaatcatttccaccagttacaagcacatttacttcctaagttataaatacgtgccttgggacttcgatgttgcttttatcgccatgttcttcatgttatttggctatctttatttccataaaattcagcaattcgttaaggacctgtgggtgattattccagcagccatgctgactgtctggttgttttggatgcagcacatggaccggttcaacttcgcgttcttcctgaagtccaaaatcattcacgcttcctatcaccacattccgatttctcgggtttcctacattacttttatcccgattattgtttgtctagtcgttttcagcgccagttactatttctgcaaattcatgccccagtttctcattaagccggttcaattattgggccaacagacattgggaattatgtatctgcacaaggctgtcatcgacattattgatgaagctggctacaatggtgccattatggaaacaattctggcggttttaatttcgtttatcctgtcactgggctacggctatgtcaaacaaaaaataaagaattcacgtataaggcggtcaattagttgataaattatcggcgctcaagaaacttgcgaatactttactttgtaatcggcgggctcatcatcttgggcttcggttttaacatttggcaggatcagcgtgcttcggatcagctcaaggccaactatattgactccagtacgccgactatctttgtccacggctggggtgccacccttcgttccgaaaaagatatgatctcagcagccgaggttagtggggccgcttcaaggcgaatgattgtccgcgtgagagccaacggaaaattgtcagtcactggaacggttaagtcatggatggttaatccaatcattatggtccgaatggacaataaccgcgccggcgaggttcagtatgcccgctggctgaccaaggtctgcaagttactcaagcagaaataccatgtcaatcaattaaactttgtcggccattccatgggggcttacgccgtcgtctactataaccttttgaacggcaaccgatctgatttgccacgaaccaataagttatgtgtgatcgccgggccttatgatgggatcatggataatcacaagtccaatcagccgacatccggcccactgatgcagttatgggatgatgcgcccaataaaaatcgcattttgccgactggtaaacccaagatcatccatcctgaatacaagttactctatcggctgagaaaaaatttccctcgtcaagccagggttttgaatatttatggtaacttgggcgatggttcaaattcagatggcgttgtcaccaacgcttctgccctatcattaggctatattttgcgagatcacgtcagcttttatcaaacatttcaagcttttggtcccaaggcgcaacacagtgccctgcacaataacaacattgccgtcaataaaattctaacggaattcctgtggaataaaaattaccaagatagttctgcgagtgaattaatgcaatagcaactcaaaaacagccaaaatccattgtggattttggctgtttttcattcctgtggctgattatttaaaagcactcactaatttacgattagccgtgatatatgaaccgtcggctaagacaaaacgcgttgttaaatgataatgaaccatgcgtttgacattgacagtctggccctttttgtatgtggcaactctaccagtcaaattcttaccttgatagccatgaatgccagtcgggttgatcactttgatttttgggtgacgactggcataataaactggtctcacataggtccagtttgctgttagatagcctgccttgccatgggaaggactttgatgattgacatcccgtacccggtaccgcaactggccagtggctgaacgagcatagccggtcaccacaaacatgggtcgggcatagcgcttttgagctggatatcggaaaagtcgattgccggacttaaaattgggggaattgtatagcccgaccgttttgatggcgtagacggccaccccttttacggcgacttttttgtttggagtcggttgggttattgtagtttggcctgcgttcattgggttgtttaagatcgcgaccccaattgctcccaggtgggaatcagtcgctggccgggatgacgtgcggacactctctgttggccgactaacagagatttgactttttcccgccacattaaccctcgtcgaattcgttggttttgacgggaccactggcgattgttgtgcaacctgagacaaatctgacggaagacttgcagctttcgtctcaacaggcttaaccgcctggaacaccggttctttagttactaaagttggttgagtaaccgtgggccgttgttgcttaacttcaacttggggagcacttttttgcgcctgatcagttgagttgactggtaataccggcgctacattcgaactggctggctttgtgtcgccactgtcttgtgtcaccggtttggcagcttccacaagttttgaatcggtgcctgagtgagaactcgtagacacaccagcgtggttcggctttgcctgggcttctttgacctgctcaggctgatctggctgagaagcattcactggccgataccagaattttaccaagcaagtcagatcccttaattctctaaaccagaagttcaccgattgatcgttatttttagtgaaatacgggctttcgaaggttgcctcaaccggctgatagccctgaatcttctttggcttaatggttacttggtcagcgtaatgcagcgttttggtggcggtgtccagcgtgtgactatcttgacgattcatatagttaatattcaccgttgcggtatagaggccagtactttcctggcgatatttgagcaacagcgggtgctgcaagtctgcacgagaatctggaactgtatgagaaatcgttgcggttggaacaaagttctgataaaccggtacttgaaatgactcccctatattgccgaccatcttaattggcttgactccgggaatcacctgccagtcaccagcggaatccgatttggacaccggctgaacataaaatgtcacccgctgccccaactcagtcgtgcgcacgttgtctgctgggaaatccgcgtgagccaacggtgcctgcagcatgattaacccactggcagccatgagcgctaaactgctccaaaatttaaaaccattagctttccccaaagtcactttatcaaatttatccatcatctttctccttcaacatttttcaagacgactcaactcgtcccgttcgtaatatatatacggagaaaatggcggaattttttattttttgaaaataattcaactgttcaaataaaaacagctgaggacaattccccagctgtttgcttgatcacgttaaccgacaacaatattaacgatcttgtttggaatgacaatcactttacgaacagtcttgccttccagatatcgttcaacattctcatcacttttggcagtctgttcaactttttctttatcaagatcacgggcaaccttaatgtgtgaacgaactttcccgttgacttgaacgaccatctgaacggtgttctcaactaacttggaagcatcataggttggccacttttcataggtaatcgtgccgtcatgacccaataaactccacaattcttcggcgatatgtggggcaaccggtgacaggagtttgacgaagccttccatgtaatcaattggcagtgaatctgccttgtaggcgtcgttaacaaagaccatcatttgagaaatgccgacgttaaaccgcatatgttcaaagtcatctgaaacgattttgaccgtctggttataaatcttgtccagcttgccgtcattgatcgtggtaacgcggtcacgcaaatgattgttatcatcgatcagtaagcgccatacccggtcaagccaatggtaggccccgtgaataccttccgtgctccaaggcttggcagcatcgattgggcccatgaacatttcatatacccggagtgtatctgcaccgtattcatcaacaatatcatccgggttgatcacgttaccctttgacttcgacatcttttcgtggttggttccaagaatcatcccctggttaaccagtttctggaacggttccttagttggcacaacccccaaatcgtaaaggaacttgtgccagaatcttgcatatagcaaatgtagaacggcatgttcagccccgccgacatataaatcaactggtgaccaatacttcaacttttcaggagaagcgatggcttggtcgttatgcggatccatgtaacgcagccagtaccatgaacttccggcccactgtggcatcgtgttggtttcacgtttgcctttgcggccgtttttatcaaccacgttgacccagtcatccaagttagcgagtgggctttccttgccaccagaggtctgaatatctttggcctttggcaatcgaagcggcagctcatcttcaggaaccagcgtcgtttcgccatcttcccaatgaatcactggaattggttcaccccagtatcgttgacggctgaagatccagtcacgcagccggtagttgaccttttcatgaccggctttatggtcagttaaccaatcaatggctgccttaatggcgtcatctttgcccatgccatccatgaagccggagttgaagtgaggaccgtcacccgtataggcagcttcgtcggtattaccaccttcaatgacgggaacaattggcagtccaaatttcttggcaaaatcataatcacgatcatcatgcgctggaacggccatgatggcaccggttccgtacgattcaagaacgtaatcaccaatccagattggcacttcttttccagtcattggattaatcccgtaggcaccagtgaagaccccactcttatctttgttcaaatcggttcgttcaagatcggatttgcgggaaacttcttcttgataagctttgacttcagcggcttgttcaggggtggtaatctttgaaaccagctggtgttccggcgcgagcaccatgtatgttgccccaaatagggtgtcaggacgggtggtgaacacttcaaccttgtcatcaggatgacctttgacctcaaagaacacgctggcaccacgcgaacggccgatccagttgcgttgttgttccttaatactttcaggccaatccagatcgtccaagtcatcaatcaatcgatcagcgtaagccgtgatcttgaggacccattggcgcatcggcacccgataaaccggatagccgccacgttcagtcttaccgtcaacgacttcctcattggcaacaacggtcccacccataaaatcaggggcccagttaacttcaatattgtcttcataagccaatccgcgtttgtataattcttcaaaaatccattgggtccatttgtaatagcttgggtcggtggtgttaatttcacgatcccaatcatatgagaatccaagcgaacgaatttggcgtttgaaagttttgatgttcttagccgtaaagtctcgcgggttatgccccgtcttcagtgcatactgttctgcaggtaatccaaaagcatcccatcccattgggtgaagaacatttttcccctgcatccgcttcattctagccataatatccgtagctgtgtagccttcaggatgcccaacgtgcaggccctgacccgatggataagggaacatatccaagacatagtatttgtctttgtcagcaacttcttcggtcttaaatgtcttgtgttctttccagtaatgctgccatttgcgctcaattacctcatgattgtatgccattttgcaacttccacctttcatatttctcaatcaatgaaaaaagtcccataagaaaccagactgggcttcttataggacgatttatcgcggtaccacctatattctcaattacttgagctctcgaatcaataacggcgacaaaccggcttgatttacttcgttcgaccaagcattcgacgatgagttcgccacgacctgttctgagttcacagcagccactcagtttctggaaaacaggcagttggttactaattcgtctctgcattttcacaaattgaaattattgcttattatcataccaaaacaggtcttaaaaaacaactgctcagcgtgctataattttattattggagttgaaaacatgaaaaaacaatcacaaaaaatttcaagcaccgttagtttggtttcactggtcatctttttgattctgacttacggcgtggttttacataaagaatggatcaatacctttgacacctacttcggccacatggtcagaagctttcaaacgccctcactgaccagcttcatgattcattttaccgagttgggaaattatcagtcactattgggtttcacaatcggtgccggattgattttatttttggttcgcaaaatcaaatccgccttattcttgttgattaacggcgtcgtcttggcagccccgattgataccctggtcaaacacatggttaaccggccgcgaccatctctgacccatctggtggctgttcacagcagtagtttccccagtggtcactcaatgagtatcatggtggttgccggcagcctgattttgctggccaaccgcatgcttaaaggaagtagccaacggctgatcgttgatctgattttgatcatcatgattgtcggtatcggcatcagccggatatatgttggcgttcattatgccagtgacgttctgggcggctggagtcttggcctagtgaccttaatggtgtcacaatgggtatttaatcgattcgcgggaggtatctcatgaaaatcaaatcagcattggaatatagccatgaactgttatcagaaactgtcgattccggagataccgtcgttgactgtaccatgggtaacggccacgacaccctgtttttagccaatttagttggcaaacaaggcaccgtgtatggatttgatattcaagcccaggcagttgaaaataccaaagcacttctaaaaaccaatcacgttcgcaccaaaaacgtctacctgtacaatatcagccatgccaaagttgatgaaattttaccatacgagaccatgatttccggcgccatcttcaatctcggctatctgccgggcggcgataagacgattgtcacctaccctgaaacgacgattgcggcgattaaaggctgcctcaaccacttatgccataatggcgtgatcgtcgtggttgcctactatggtcatccaggcggcgaacgcgaaaaaaacaccgtcctcgaatttggcagtcaactcgaccaaaaacgatacagtgttttgaaatacagcttcttaaatcagcagcattttccaccaatattgatggcgattcagcggatcgattaattgattcgctgttttttatttttgcggtcaaacaaattgcagatataggcaatgataatcagaatcaagccgaccacaaagacattatgcagggaattgtacaaaatatttcgcaactgcggcaaaattttgtcacttaactgattggcagtcaatgggttaatcagtttgtccatcattttcaaggatgtatgttccgtttgccggaccccacgcagcatggtggtgttcatgacgataccaaagattgaaatcatcagtgtctgacccagcgttcggcacaaagtattaaaggaagttgccacaccaatctgagttggtttaacctcattttgaacgctaataatcgacgttgtcaccgttaagccaaagccggtcccacagatcattgaaatccccaagaaggccacaaacggcgtatatgccggaatcagcaccataataatggccccaaccaagataaagaagagactgaggttaataatgcggtaaggtgacgtcctggccagcaatttaccggccaaaaatgagccgacaatccacatcagggaactcggcgtcaccgcaaacccggccatcgatgcccgcaggcccaaaattccctgggtccagtccggcagataaacttcgtagccgatcagaaagccactgaccaaaaaaaccacgatattttgaacgacgaaggtccgattatcaaacagttccatcggaattaacggatcggccgccagtctttctgtccgaataaacatgaccgtggcgatcactgtaaccaagaagcagaccgcaacgatctgccagttgatcggatcctggccgaccaactggaacgcatacatcactgccaacagcatcatcgtcagccaagtggtcccggcaatgtccattttagtggtactgtggtgtttgtcttcatgcaggaaaatctggaccatgaccatgacaatcaacccaatgggtaaattgataaagaaaatccagtgccagctcaagtgatcaacaatgaaaccacccaatagtggcgcgatcacagaagcaattccccaagcagacgagttcaggcccaacacctgagcgcgcttttccaggggataaatatcggcgataatcgtattggaaatcggcatgatggagccggctccaaccccttgcacggcccgccaaaagatcaaaaccaccattgagtgcgataacccggacatcaccgacccaaagacaaagatcaaaattccaccaataaacattggctttcggccaatactgtcggccaatttaccatagattggcgtcgcaattgcattggttaacagaaaaatggaaaagacccaattcattagggaaactccccgcaggtcaccgacaatcgtcggcatggcagtcgaaacaattgtcccttcaattgcggccataaaggtggccacaaagagggcaatcgttactaaggttacattacttttggttgctgttttcgtcatgaaatgacctcttttctttaaaattaaacaaaaaaatgcccttgaattttcaagggcgttttgcttgtcagctgtttataacttgaaatagtcttttaacgcatcaaccttatcggtatgctcccatggaagatcaatatcggttcttccaaagtgaccatacgctgcggtctgttcataaattggtcgttttaagtccagcattttgataattcctgccgggcgaagatcaaataatgctcgtgtggcatcaatcaattgatcttcaggcactttaccggtaccaaatgtattaatgtcgattgaaacgggcttggcaaccccgatggcatatgccaactggatttcagcttcgcttgccaaaccggcggcaacaatgttcttagcaatgtatcgcgccgcataacttgccgaacggtcaactttggtagcatcctttcctgaaaaggcaccgccaccatggtgggcgtaaccaccataggtatcaacgataatcttacgtccggttaacccggcatccccttgaggaccaccaatgacaaaccggccggttggattaaccagataacgggtcttgtcgtcaagatacttggcaggaatcacctgtttgatgatttggttgatcacatcggtccgaacttgatccaatcggacaccatcgtcatgctgagtgcttaagacgaccgtgtcaactcggaccggcttggcgttgtcatcatactcaacagtgacttcagccttggcatccgggcccagataaccaatctcgccactcttacgcaagtctgcctgctttctcatcagcttgtgggctaatgaaatcggcaacggcattaactcgggtgtctcatcaatggcatagccaaacatgagtccttggtcaccggcaccgatttgatccaacgggtcggtattgccttcacgttgctccaaagcgtcatcaacacctaaggcaatatcaggtgactgaccatcaagggcaacgataacaccacatgaatcaccatcaaagccgtaacggccatcggcatagccgattcgcttaatcgtgttgcgaacaactttttgaatatccacgtaggcagtcgtggaaatttcaccgaaaacaaacaccagtccggtggtaactgaggtttcgcatgctacccgagcatccgggtcttttgctaacaaggcatccagaattgcatcactaatctgatccgcaattttatccggatggccttctgaaactgattccgaagtaaataaatgtttttcgcgcattctattttccccctattattttttaaggttacaaggcttcttcacgcatcacgtgaatcctatcgggaactcataactctacaatcttatcatatttgatttgcttttcaagccttattttcagctgtccattgaccatctgacagaaaaccagtaggattatttttataattagctattaaaaatgtgaggaagttgaggatttgttaaaatttgaccgctccattttaattcaatcaggactgcgcgccgtcagcatggtctttatctggatgctatttgccaatatctcgttaaagggatttttcgtcaatccgcgccttctgcatctcctggtgatcgggttcgtgtttgccgttttattgaccgccgtcagccgaccgcacaaaaatgccgtcatggtcgtcttaaccgatattttactgggtatcttattggcatcgctgtacctcgatacgccgagcattaacgtctggctgattctgatcggctttttgctcgccaacctgctgttagtctctaatttaatcgatgaacctcactgtcgttggattatttatgggttcatttccggaaccggaattgtcttgttgttcacaacgacctaccatcactatttttccctggtctcactgatgtatatcaccctgatgatttttgcaaatattttcttttcctactacgcctttatgaaacaaaacaatcagctgtccatgatgatcgtgtcggtgctgattttaatgttgtgtctcacgctcaacatctcattttttaaaatcattcttatcgccggcattctggcattctacgcttattttgaatcccgggttaatttccgtaattttgaaaaacgggccaatgtttcgacggtttccttcctgttgttttcaatgctggtctgtttttaaggttcatttattataattttgttaatatggttaattttaagaaaagaatcaccaactttgtcacccaccgtcattcaatcgtgtagtatggcgttgattgataaattcgacaaggacggtgacaagcgtgaacattaaagtagttggtgatatccgagtaggcaaaatacaaccttcattaactgggaatcccattgttgacgatgtcctcattcaacatttttgtgatcgactcaaagaaaaattaaattcactgcaaccatccgttgatattattcccgaccatttcttcgatgctaccaagccatgtgccgacatcattttgatggacaggcgcatcatcgatgatctccccgacgaactgctgatgaactttaaaataatcgacattgaccataatgatattttacgaggtaacattactgaggctgtgaacgcactcaaacgatatgattccggcaagcacgtttttgcgatgtagtcgtgaaacttacccgtcggtatttgcaaattgccccatacaaaaagcccgtcatcttgaatgacgagctttttgtataccgaaaaatccacgaagcggctttcagttatgttctatttcttgaagcggcgatccttcttaatatacacaatcatcaataagaccattaccatcgttaaaacgactgtatagaaccaagcttccccacgacctgcaaatggtagtttaacgttcatcccataaaacccggaaacaatcggcggaatggctagaatcagtgaccaaatcgtcagaaactgcatcgtttggttcaatttattattcaaaatattcccaaatgccgactcggtttcccgaaccacgtcgccgaccacatcaaacatggtttgacactgtttgtattcaattaacaggtcaccaatggattcattggttttgctggcaagttccggagacatcttcaagttatccttgatggtggcttgtaactcctgcagggcgatcaagttgcctgccgtggccgagcgcagatagaccagactggtctttagtgctgccaattcatccaaactgtggttgctgattgcccggttgtgcatcccttccaacttctcggctttctgactgatctcgtctaatttatcgaagaacggcgaaatcaatgcaaacaggattgccaaaatgtgctcggcaacactgtcatatgccaacttggaatggtctgaaaccagcttagcctgctcttgggcgtgacacaccgtaatcagcagggaattactgaatcccagaaaaatcggcgatgtgagcattcggctttgcttaggatccgcaattgccctgaccaccagtgcactaaaccctgacagatcatcaaaagtggcccgtggctgctcatgacgatccagcatatagcctttgaacttggctggtgcccgatagtcaatcgtaatgtcgtttaattcgtcttcagttggtgaaattgcctcgacccaggtgtaagtgtcaaacttatgaattttaatcatggtattgcctcttcaatcgtcattttatgaataactaaagtctaattttttccgaaagcaatttcaatccccaactacctgccgccatgacgccgttggatcacctggtaaatcaccagcatcgagccaattgaaatcaatgaaatgaccatcgccacccgtgttgagctgttcaccaataggaatccaagaatgaagacaaagaatgccagtgtcaaataatcactcaacggatacccaggcattctaaagacctcactgcccttcggatgagctcggcggtatttaatgtggacgatgattaaaaccacccacaccacgacaaagttaatggttgaaacacttgaaaccaggttgaagacacccgctggaataaagtagttcaaaacaacgatgattaacagaaaggcggttgaaaagttcagggcaatgtttggaaccccgttacgccccaatttggttaaaaatgatgaagcattcccacccatactcaacgcgtacattgtccggctggtactgaataaacaactgttagtggcggagaccgcggcagtcaaaacaacaaaattcaaaatcccggcagcacccacaattcccactcccgagaacacctgaacaaatgggctggcggtcgtggtgattttattccaaggataaacactcatgactgcaatcatcgaaccaatgtaaaataaaccaattcggatcggtaaactgttaatcgcctttggcagattggctttgggatcgtcagtttcgccggccgtcaacccaaccatttcaatgccgacaaaggcaaacaccaccatttgaaatgacatcaagaacccgtgggcgccagttgggaaaaagccgccatggctgaccagctggctgaacgaagccgtcgagccgtcaacattcacgtggaacacggcgagtcccactccgacaacgactaggagaataattgccacgactttaatcatcgaaaaccaggattccatctcaccaaacaatccgacattgaccagattggcggcgaacagacataagagaataatcagcggtggaatccattggggaactccgggaaaccaatacttgatataaattccggtggcagtcaaatcggccattgccaaactaatccagcagaaccagtaagtccagccggtcacaaactcccagcggtcacccaaatacatttttacaaaatcaagaaatgaatgtttgctggtatctgacagcagcaattcaccaatcccccgcatcagcaggaaacaaaagatcccaacaatcaagtaggataaaataattgatggccctgaagtgtgaatggccgatccggaccccaagaacagcccggttccaattgccccgccaatcgcaatcatctgaatgtgtcggctttttagtgaacgcgatagtgaatttgtttgatccttcgtttccatagtgtcctccttaaaaatgtccattaaaaacgcccccagtacctattacagtaccaggggcgttcttcaacgcggttccacccaagttccacaatacaatatgtattgcctctaattgcagataaggctgccgccattaagtattgccattttagttgccggctttcagcaaatgccagctctctgtgaatatttaccagtatacggttcatatttgaaatgtcaaccccaaatcgtcaacacatgttcacggatgaagaacaaagacgaaatttaatcagcaaattagttgatttttcggccaatatcgagtatctttgagccaataaaagttaattggacttttaatcgagtcattatggagggatacatttatggaatctcatacagctttactgattattgattataccaacgattttgtggccgataaaggggcactgagctgtggcggccctggacaggtactggaaccgcatattttaaaattagctgacgaatttgtggccaatggcgactgggtgattttaccgaccgatgtgcatacaccaaatgacccataccatcctgaaaccaagttattcccacctcacaacgtccgaggtacttggggccgtgaattttatggtggcttatcaccttggtttaaagagcatcaagcagatgataaggtgtatatgtatgacaaaacccgctacagtgcctttgccggcaccgacctggatatccggctgcgtgaacgccacgttgacaccgttcatctagtcggtgtctgcagcgatatctgcgttttacacactgccgtcgacgcttataatctctgctacaacattgttgttcacaagagcggcgttgccggattgacccaagccggcaatgactgggcattggatcacttcgaacatgttctgggagccactgtagaagattaatggcgagttgctttgcaaaatttcccgatttagtgtttaatgttcttcagtagacaaaatatattttcgatcgaagatgggatgaaacgattgttttgtgaccatcttcttagtgtttgtgaatttattttggactagggaggaacgacaatggctaataaagtgtccagatacaataatgaccagtgggaaaccgctaaagaatctgttttgcaagagtatgaagattataaacaaaccctgcgggatcaaggggtcgactatacaatcaagaatgcccggaaattattgatctaccaggacctagttgccgagtggcagcacaaattgggaaccgttatcaccgaccttgaagataacctgtttgcattaacgatttttgatgaccttaaaaaacgaaagcaaagctcgcttttggcgcgcggatatgaacatatttccagttggccggacttcaacccgacggcgctggccctttggttggagcttgaggaagacgaggccatggcttagtaagtgaggtggcaaaatgtctcattttgatatttccatgttgatcacaatcgcgattggttttattttgatgaccgtaaccaacaaccgtccgttcgcaatcactttggcggtgttagcaattggcttaaccatcatgctgacaatcaaaaagatcctgaatcgaaaacaatcgcatagttaagacgacaaccacaaggggctgcgacaaatctgtcgcagcccctttgctgtctggttgatcaaaatggtctttaattattttttcttctcacccttatctttcttctggttcttttttagaaattcatcccgtgtctgtaaatccttcacgtgaattttaatttcggttggcttcaaatcggtcatttcggtgattgtctgagttaatttagtggtaattttgttaaagaccgttgggatgcatttgccatattccaagactgcatccattgccaatttaacttctttatcatcgttgtctaaatctactttcaccccagttgagggatccgtctcgtcactgaaacgatcagtgaccgaatcaatcaggttcccctctaaagacagcaccccatccacatcacgaacggtattaccggcaatcttggttaacacactgtcatcataagttaatacggttgctacactgctgttttcttgtgtcatggtttttccctccattggctattccaccctgtcatcattgacagtgtttgcgatatcgtctttctttcgggtactttgctgttcccattcttttttggtcagaacatcgttaatatttaaattaatttcaacaacgtccaaaccggtataattcttgatggctttttgggtccggctgcaaatttcatcaaagatctgccgggcgtcggcgccatattcaatcgttgcttccatgtccaaggcaacctgtttttcaccaacctcggcgtcaatcccctttgtcggatcagtggtttttgagaaccgatccgctaattcactcatcatcccgccatcaagcgacaggacgccgtccacatttctggaaaccagtccggcaattttttcaattaccgagttttcaaaggttaacttcttgtttaaatctgatttttgaatcgttgcatccatcacagtcatctcactttccttctgttatttaatcatcactcactaattggctgattaagcgcttgagcccgccaaacttccagataacggtcccgatcaaggcaccaatcaaggtcagtgccaacaccgtcagcatgccgctgaggccgccaaagacccacacgacgcctgcgaccattccgaagacggctccgtacataattgcattcatcgacatcctcctcctaaactactcgtgggcgactggctttttcgcgtctgcttgaagcttcaaacggggtcactttgacccgcactttcttgacttcaacatccatcaactgctggatctcatccacgacattgttctgaattgcctcacccagtttgaccagatcttggttgagtttatcaacggcgttgacgctaacgcgaaccacccgattccgagtcctcaatcgcaatttgacagtcacatgattgacgttgttttgcgtcataattcgattctgcaaaattttttcaaccgctgacttggaaatactcagcctgccgtgtggagactcaaaccgcaactggtcagccttcctcggcgcaaagattgccgttatcaacatcatcagactgactagggcgacgaccgcggatacaatcgcagcaccaatcatcatccaaggagtatccgtttgaattgtctgagtcacgactggtgacaaatagtcgattggaatgactaacccaaccagccaaaccgattgggcaatcccaatcaggctgacaatccagatcattaatcttgaaaacttattcaatttgcaacctcctttcttaaaagaggtaaccttaacgtgccattccccgagtcaccattgaaacgaccaggactaaaatgacagctccgacaatggccggtaaaattgccatcccagctaattgaggcccccaggaaccaaaaattgcttctccgagccaggcgccaatcaggccaccaacaatgttgccgatccagcccatgggcatgtcacgactggcaatcgctcctgcaagtgcgccaatgatgccaccaatgataagtgtccagagtaaactaaacatgataatcatcctttctacaaatagtattgtggaaattatagctcccttgctatagttatattttataataattaatatcttattgtgtgaataaggtgtgaagaaaagatgaaaagagtgtgaggcaagctgattagcttttgagcattagggtgataacagtagttaacgctagttttgcgttgactgctgttatcggactaagcggagaaagctggcttgtcgaacacatttagagtgtgaggaccaacgggtggcgcgacttctaagggagctttgactgaaaccccgggtttgggtttgggtttgagttaaagatcccttagaaacaagcgtcagttgcggcggaacacgtttagagtgtgagtccgagcggttagcaaccggagcataagctgacttgcggggaaatcgagtttgatttcgccggaagttggcttatgtgcaggttgctgcttgggggaacacatttacatcggagtgtgaggcaagccggtttgggggaacacgtttgccttaaccaaaaaaaaggcgtcaaccaaacggtcaactcctcaatccaaacattaagcaattccaagccctgccagcacccccacaatcactgaggcgaccaacatcaagccgagcatcaccaaatgaaatttcttatgcatgacaaccagggccaggtattcacgaatgactgcgttcggcaggtaataaaatggcgttttcgacccaatcccaaaagcatgcataccaacttcccgagaaaggataccggctctcaaagtatgataattgctggtaacgaaaacaattctatgattagtcgaaccggcgtccttatcaatcaaggctttggaaaacttcatattttgaaaagtattcactgactggtcttcaatcaaagtgtctgcccctctggcaccatgttccaaggcgtagtcacgcatggcgatactttcagggagtaactcgtcaccaccctggccgcccgaaaagaccaatttggcgcgcttgttggttcgatggatttgatgattataaaatgcgattcctttattaatgcgaccgccaagcaggcgaccgactttgtgtccatcaaccaatccagctcccaaaacgatgatgtaatctttattgctccggggaaaatataattgatacaacagcatcgaagacaacgtattccacacagtcagcaaaatataagcaatcagcatcgtcaaaaaagtcatgacaaacgcttgaatcggtgttggcaggtcaattgggttaaagaaaatcaaaacatcaatgaggacaacgccgatcccgacgattaacgtcaacgacccgctgagactataaccttcttttcgccaaacgacgattgcgttgataaaccagaaaataaaactcaaaattaatcccaaaataacggccagaccaacgattgcgacggccacggcaatcaccaacgcattatatttttcgccaaacacctcaaataattgaaccaggagggccaataatgccagtaaatccaaattggccagccaaccaagaaccgacgtgtttcggttcttgatcaaatatgtacctaaagccaccgtcaaaacggcaaaaacgacgcctgtcaaagccaccatccacatactcgttcccccttttgaattcaacagattcgacaaataaaaggccggcagcaaagcctcagttttgccccggtccagatggatcccagaatgctatttgttggtgtaatctttgctattcatttcttctgcagcgaattccttaataaatttcaaaatggctctgaccttgtcgtccccataacggctgatccagctgtcaaaacgtttggtgatcagatcgttgacgtgcttttcagtttgctcaccggttggagttaaatgtaaataaagtcgacgacgatcactttcagctggtttttgaaaaatataatcatgctgtaatagaactttgatttggcgtgaaattgcgcttcgggttactcgccgttcactggcaatatccatcaatgagacgttttgtttttcagcgattgtatgcaaaattaagtattgttcaaacgacaatccgtacttagttgcgggttcagaaacaaagttatctaagtatttaagtgacgacaaataaacgtcgattgcttcttttaatagatcctgatttgttttactcatatctgtcaccattcccctttaattattaaaccttatatcaccttaattatatattttagtaaccagtgtcgcaactaaatggattaactttatcgttttatggcattatgctttataattatgacataacaaaaaaggattgatatttatggctgatgatgcaatttcactaattcaccaagtagaactggatcttttcaaacaatttgccaaaatcacccaccaacaccacatccattacattgctttgggtgggacaatgctgggggctgttcgccatcaggggttcattccctgggacgatgatatggacgtcggaatgctgcgggtggattacgagcaatttttgaaagtggctgagcaagaccttaaagggactcactattttcttcaaaccccatggacggacgagaattacgctctgagctattccaaactattggataggaataccttcattgaggagaagaacaacgttaacaacgcccggaaaggcgttttcctggatatcttccccttggatcgaattccagactctcctgcccgtcaacggcggcaaattttggacatgcgaagactcgacagccgaatttatttgaaactgcgttataacgtgatcgataatccaattcgcaagtttcatgcctccctttctgccgagcaggcagagacggcagaagatttcaaaaaacaacgcgaaagcgtcatgaccatgtataacgacaaagcggcgttaatgaacgtcaagaatctcgcctcacaatatgcctatgaaaaagaaattctgagcctggaccaactaaatgatacgattgtgttgccatttgaggacacttatattcgggtccccgctgattacgatggcatcttgaccaaaatctatggcgattatatgacgctgccgccggaaaatgcccgaactgaaaagcacattgtccgtttaatcactgataatcaagagtttgaactctaactaattacttgcgttggcctgattaatttggtaggttacatatgacaagcaatgcagaaatgaaggtgttatgaatgtttaatcccaatgaatccagattcgccagctacacgatcgtttcatcattacccgatgaggcaattgataacgtttggtacatcatcgataacgacctgcaaggcgttttccaattatcaaatctgatcacatttaatttagttaataacgatggcaatttgtcctatgatttcattcaaggaaatgaattggtggcaacttttgattcaccatatccttacgacaatggttatccaaaatccctggtcgtctatgacagtggtgaccggcaaatcattgcgaccccatctgaaatcaatttataaagttactttgcatgttgtaagacctgaccggaagttttttcggttaggtctttttgaatgccctgagagaatcattccacttaagggccatcggttagattgaagattaaataaccagacttctaaatgaaaaaatgataaaaagaaaagagcaggcaaattgcctactctttgtgtaactgctccggctgggttcgaaccagcgacctcttgattaacagtcaattattctaccactgaactacggagcaaaaatatttacttaacgaccacttagataatatatcatatctaagagtgactgacaactacaaaattgcataaaaaaagattttgggggatcaaccgcccccggaagatctttactgctccggctgggttcgaaccagcgacctcttgattaacagtcaattattctaccactgaactacggagcaaaaatattttctttaaaaacgacatatatatttatatcatatccagcgaaaatatgcaaactattttatcatctaaatttcatcaacccactaactaatgtgattttctttaagaatgatgtcgacttctttctgcatttccggggttttgtgccattcttcaaagtggtccatatcttcagtcggcatcgtataattttcgttaatatattgctcatatttggccacatgaggagaatgtgggatattaagctgtaagatcctgacctgcttaataaaacctcgctcagctgccaattctgcccgaccattctgcaccatattgctgatctcaatatacttgctgccatcgtttctggtaatttcttcaattaatgtcaatacttcatgactcttcaacgtgtgacctccccttatttactcacgaagaacattatacataaaaaactgacgttataaagacgtcagttttttaagagagaaagagaattgattagaaggtatttatttagtacccgaacataatatactcaatattgaaagcgctgtcaactaaatttcgaaaaaaggttgccaaacaatcatctggcaacctgaaagtcattctttacccggcagatgaagcgtgtgcgatggatgaacaatcgcagaaggattattaatcacgtgctcgactgaatggccggaaacgttaaccaagcagaagaagaccaccacaatcaacacagcccaggtcaataattgattccaaactgacattttttcgctaatgaccgagccgtaaaaacgtttatggatcttagcgggaacatccttctcatccgggtgagcattttgttcctgttcagtgatttgcttttgataatttttaatactgaaatttttctgaacactcttgcgttcagtttcaaacttatgtttttcttttttgcttaacttcttaaaccactgcgtgaactcgcgatacttctgggtcacttctttagtgtcaccaaccattttgagttcaccatagttgatccaagcaaccttgtcacacaacatttcaatctgtttgagagaatggctgacaaaaataatcgtcttaccttcctgcttaaattcggtaattttgtcgacacacttttggtagaatgtatcatcaccaacggataaggcttcatcaatgatcaaaatgtccgggttgatgtggacggcaatcgcaaacccaagccgggagcgcataccacttgaataactcttaactggttggtcaacaaaatcgccgatatcggcaaacgcaatgatatcaggcattaattcgtcaatttcttcattggttaacccttgcatcaaggatttcagacggatattttcacggcctgtcaaactgctcctcaagccggcatgaattgccacaatcgaagtttccccgcgaacgtcaacataaccggtggtttgggggataattccggaaatgatattggaaatcgtcgattttccggacccgttaactccgatgaggccaagggtttcccctggtttaaccgtcagagaaacccccattaatgaccaaaaatgaggaacctgttttttggtaatcgaaaagaatgagcgtaatttttcagactgggtcttgaataattcatactctttggtaacattttcaacttttactttataatcgttttccattgctccgctcctaatttaagagagactaaattcacgagtaacattataacaaactttgcaactgaaaaaaggattcccaaataaactttgcgaacccttaaacatctatcggcgaacaacgcgctgcaaaggcaaactattaaattggatcacggcgtcgccttgattgatggcgacggctcccttgtcgttaaaaacaaagttgggaataatccgctttggaatactgttaattttggaacgtgaattttctgctcgaattaaagctgattttttggagtcaccagctaattgcttattgagagaggcatcaattttagaaccaatgtccccggtgctgacagacccatcaagtttgtttaaatcatacttggtaataattgcatttaatttattaccataattcatatcagtggcataagttagtgacagtgccatggcggcatcactggaagaaatggcgttcgtcgtccaggttccctcataataattcggatcggacaatgtcccgtggcgtaacagataagcattatctttgattgaggcttcaacgcttggatattttttaaaagcggccgcagtcatataatgcttccccttggaggtatattccccggtactcatagtcacagattggccattataagcgcctttaaccccgaagtaattgttggcgtccaatgatagctcggaacggccaaagtcgctctcaacgattgcctgggccatcatcacggatggatagagatggttagccttactaatcttcaccaccggcgttttcagctgattaatgaaatcggtttccacgctggcatgcgagtggtttgcttggacaaaacaaaagccggtaaccgcaaccgtggcgattagggctttcatcatgacatgtttgaattgcttaatgatgctaaaaacctcccaataccgatgttacgacgaatggtcaacaacatcggctgtttccatattcaattatgataaaaaggcactggaaacccaatacttggttgaagaattaggcgttgagattcgataccaaagtgaatggtcgctgaccttatagccaattttatcgactgtcaccttagtgccaacttgtaaatcaacctgattgagcttgtaatgcttctgcaaattccccgtcgagtttgcatgatcgtacaaataagtcgaattggcattcttagaaatcgacttggtctccttgtggttcacaaccgcaaccgatccaggatatgatactacatctgaagctttaatccaaccctttgtcttgccgtccgcaatccgataccagagaataagccccttggtggtcttttgaagggcggttttattaacattgtaacctttgttggcggccgcaatcgtctttacctttttaaccggttttgacagatagctggaacccacaatgtggttatagatgtaccccgaagaagttttacttggcgttaacgcaccagtcgccgttccagaataggtcgtggcaaatgacaatgccggagcactaacccagaactttttggctttggcattgctatagaagcgtagacggtaccagttagttgagctgttagtcttgactccgcgcatatccaggtagacttgaacccgactgttaacacccagctgtgaccaagtataacgtttctcagaggtggttgaccccttcacatgattatatacgtaatatttcttgtatttactggaaagtggtaccaaatctttgcctgaagctttgtagtatttaactttggcaagttttggtgctgtaggcatcgaagtctcggtagacgaagcagttgctgagctggcacttgagctgcttgctgttgaactcgatgctgcagatgatgatgaagcagaggtcgacgatgatgctgacgacccatccccggtctcgccaaacagctgatccaaattataggtttggataactgtaatcaacgactgaccatatccaggtgctgtcgcatatttaccagtcaaagcatttgcagcgtcttgatacgttgccgcgttctctttccaagaaccggaataatacttggggttccagctggtgccgtttcttaaagtggacccattgtcggcaaaagaagcgtacgcggttggatactttttaaaattggcagtggtattaatcatctgaccattgctattatattcggtcgtcggcatcgaaaccgaggcaccattataggcccctttaattccaaagaaattattggcttcgatcgtcagctgactttgcccccagccgctttccaatccggcctgagccatcatgaccgacccgtataagttgtacttcgatgaagctttggtaacgtcatttttatattttgagataaaactgcttgctgtggaagcataagcttgttggtatgtactttgggcagaaaatgctgtgaataaaacccccatccccgtaacaagtaaggcagttagtccatgcttaattattttattcaatgatccacacctccgtttaggccacatccctatcatattagataacagagaaaaaatgaagccctaaatagaattaattagccaaagaagctttagactttcttaataactttaacaactcttataatatatcattttctgtttgaaaacaaaaaaagaaactaccattttgagatatcaagaaaatttttggacaatatctcaatttatccagtgtgtctgttttatggcatgcctcatcaaaaaatgattgataaacaaaaaggacaagcattctctgcctgtcctctatagaaacgctattcaaatttactcaacagtgacactcttagccaagttacgtggacgatcaacatccagtcccttgttcaaacttgtgtaataagcaatcagttgtgcaggaaccacgctgagcagcggtgtgatcaactcattgacgtctggaatgatcaaagtatcatcttcctcagccaatcccttacgaacgatggtaaaggttgcagcaccacgtgattcagtttcctgcaaattgctgcgggttaagttagccgtccgcttttgtgtgataatcccgacgaccggtgtcccttcttcaatcaaggcaatcgtgccgtgcttcaattcaccggatgcaaagccttctgcttgaacatatgaaatttctttcagcttcaaggcagactccaatgaaacggtttggtcaattccccgcccaatatagaaggcccggttggctggaacaaaatactttttagcgagatcatcaatgacatctttctcatcaataatcgcctgcatcccggttgcgaccaatcctaattgctggcgaatatcaaactcttcggcgatcgtttgctctttagcttcacccaacgccttggcaagaatcgcttcaaccccaatttgggcggtgtaagccttcgttgaggccacagagatctcagggccggcgtgcaatagcatcgtgtaagttgcttcgcggaatagcgttgaattttcaacgttggtaatcgtcaagctctcatagttattggcattgacgttcactaaaacttcacgactgtcggcagtttcaccactttgcgacaggaagatgaagaacggcttcttggacaacagcggattgtcataggcaaattcagaagcaatatgaacttcagttgggacgtgagccaatttttcgaataatttcttaccgactaacccggcatggtaactggttccggcacccacaatgtacaaacgatcggcttccttcattgcattgatcaattgtgaatcaacgtttggcttgccggattcttcagtgtaaagggaggccaatttccgcatcacgtttggctgctcgtcgatttcttttaacatatagtatggataaggacccttatcggtctcttgggcatccatatcaacatggaaagtgtcccgctgaactttgtggccgtcacggtcttcaatgtcaactgaatcaggcttaattgtcaccacttcaccgtcatgtaattcaaggaagtcatgggtcacattcagcatggccaaagcgtccgagcagaccacgttgcagccgtcaccaaccccgatcaaaagtgggctcttgttcttggcaacgtacaaagtctcaggatctgtgctgtcaatcaataagaaggcatatgaagatccctcaagtaaactcaaagtcttcaagaaggcttccttagtcgtcatcccctctgtttgaacaaatcgatcaaccaattgaacaaccacttcagtatcggtttgactggtaaaggtggtgttgctcaagtacttggcttttaattccttgtagttttcgatgaccccattgtgaaccaagtaaaaacggtggtcttcagaatattgtggatgggcattgtcaacgctcacaaccccatgggtagcccagcgggtgtggccgattccgacagaaccgtgaacttccggtccaacggcagcttcgagttcggagatgcggcccttacgcttcaccagatagtcgttgccattcaaatcgttgacataaataccagcggaatcataaccacgatattcaagtttttcaagcccttccaataaaattgaaacagcattatcatttccagttactccaactattccacacattttagtattctcctcaaatttcataaattggtatatacagaatatgaactctatatatttatataacacgtataatctacctaacttcgagataaaagtcaacaaaagatgtcaaatggtataccaaatcttaaaaattgatatatcaactttggcagttgcgcggagaccaaaataaaaagatgttgcagtaaactttcgttttacttacaacatctgctcaaaatcatatttaaataaatgattctctgaaaaatgtctaaactattcaattcccatttcgtcacgaacaacatccgcaatccgtttggtgtaatcatcaaccaaatcttgcgttggtgcttcggtcatgactcgaagtaggggttcggttccactgggacgaaccaagacgcggccatcaccatgcatttcttcttcaacttgggcgatcacgtctttaaccttgtcattgtccaaagcgtgtttcttatcagctactttaacgttaatcaagcgttgcggatattttttgatctcgccagccaactctgatagtttcttaccggtggctttcatgactgataatagttgcaaactggtcagcatgccgtctccggtggtgttgaaatccaagaagatgatgtgaccggactgctcgccacccaaattgtagccgtcctgattcattttttcgacgacgtaacggtccccaacctgggtcttcacgctggtcatcccttcacgttccgttgccttatacattcccatattactcatgacagtcgtcacaatggtattcttcttcaagcggccacgttcagccatgtatttaccgcaaatgtacatgatggcatcaccatcaaccaacttaccgttctcatcaactgcgatacaacggtcaccgtcgccatcaaaggcaattccagcggaaacccctttatccaagacaaacttctgcagttgctccggatgagttgagccaacatgatcgttgatattaaggccatctggattagtggctaacgtttcaaattcaatgcccaaatccgcgtacaacgtggtaaccagcttgctggtggaaccattggcagcgtccactgcaaccttcatgccggaaaggtcctcagaaattgtctgctcaaggaaatgaatgtacttttgactaccttcaagataatccccaacgactcccaagccatcggcggctgggcggggtagaatgtcttccggcctttccaggatgccttcaatctcttcttccagttcgtcggacaatttgtaaccatcggcaccgaagaacttgataccgttatattcaaccgggttatgtgaagccgtaatcatgacaccggcatcagcttcctgatttctaaccaggtaagcaactccgggtgtcgtgacgattcccaggttcaacacttcaattcctaccgaaagcaggccggcaaccaaggcttcttcaagcatctgcccggaaattcgggtgtctcgtgcaaccagaacctgaggctgtttacgttctgaatggtgggtcagcacataaccgccggctcggccgcacttaaaggccaactcaggggttaattctttgttcgcgataccgcgaacgccgtcagtaccaaaatacttcatgttaaaaattcctcatttcagtttaaatattttaaatatttgttagttatttctggtgattttgaccgaaatccgctctggatcaaatcctttaacgccgtttaatttaggatccaacgtcacctgcttggtcttagtcttggtgacatcgctggtgtcgacttcgactttgacagaggccagcttggccaattccgccttggttccaaatacccgaacccgcttggttgccgaagtgagcgtgaagctctcgttgtcatcagtgacaccctttggttccagtttgatcggcagttctttactattgcccggcgtgattggtaaggtgacgtccgcggtagccggggtaatcaccacgttaaccgtgttttgtttggcgtcgagggcttcaataattgcctgactggaaattgatgacttggcattttgcggaacgttaagctgggcgacaaccgacttaatccggttaatctgatcggacgcaccggtaatcttgacgttcttgacgtcagcgttggcctcgcctgcctgatatcccgaagcaatatttctttgagagtatttaacggtcaatggatacgaaacggtttcccgcggctgaatatcaaccttaattgtagctggttcgaagcgatatctcaaatcattatttaaaccgtcctgctgaatcctgacggtatgtgtccccactcccaatttggagagatccgcgtaggctttgaaattttgcgtattcgcagtggtggtcaccaacgcggatgggccggtgagatgaactttgaccttctgtggataaccggtcacaaaatatttgttactatttacggttaaagaaagtggaactgaaaatgtctgggtccggtttgaagttagtgaggttgaattggtgttgccggactgattgctggttgtgctggattgggtactgccaacatacatgaataacaggatggcaaagaacagcgacagcaaacgatatgcccagttttttaagagccattgtcgcatattaccgtccccctttgaaatgcttgtcaataaagccggataccgtactaagaaatgtccggtgggtctgatcatcttcatcggtaaacaattgatctttgaagtatttcaggtagtcatcccgggtcatcccacggagtaattcgttattttgagtaattgacacttcaccggtctcttctgaaataaccactgtcatcgcatcggtcaactccgagatcccaacggccgcccggtgacgagtccctaattccttgggaatcaggttactttgagaaagcggtaagtaggctgcggcagccgcaacccggttattcttaatgatgacagctccatcgtggagtggtgtgttcgggatgaaaatgttgattaacaattcaccgctcacatcagcgtccagcgcaattccagtctcaatatattcttccagacccgtattcatctgtaaggtaatcaaggcaccgattcgccgtttggacatatattgaattgcccgatccaaagcggtgatcatcttttgcgcagcttcgttttccttgcgccctttgacaaaaatggatccacggccaaggtgttccaagccccgacgaatttccggttggaaaatgacgatcagcccaataacaccccaattaatcacctgatccatgatccaagataaagtggagagcccggtataggcactaataattttaaccaccaagatcaggacaatcccgcgcaaaagctggactgccttggtatctctgacaatcaaaagtaaattataaattagaaaccaaacggccaaaatatcaatcaggctcgtcaagttatgtatcgtaaaaatatctgaccagttcattacgctctcccctaattagttttcagaaatattatatcattgtcgcctgtcaaactgataatcgattaaaatttgtgacgatgtttaaataaaacattaaaaatgaccggatcgatcaagtattgatggtatttctccgcgaaaaatagtttaattatatattgatagggggttttaacgtgaacacaaaaacaaaatggctggtccggggactttttctggtctggatcgccttactatattcatatttaaaacaacccccgtttaattttttagtgttaaatacgtttctggcatttatcccaattgaactcagcttccacattgacgttggcaaaccccaaaacggcctgctgttttgggtgctgatcatcgtctggctgttgttttatccaaataccccttacctgctgacggatttattccacttgtcactactgaatccttatggtgtcaacggattgctaagactggacgatctgatgtggttcaagtttgcgctgctattgatttcaaccattttctcaactttggtcgggctttggggcttggataaggttggcgatgcgattacagccaggttccatgcccacaatctgttggtcaaacacgccgtcattgtggcgctcaccattctggcatcaatcgggatcttcattggccgtttcttgcggattcacacgatttacttgttcttaaccccggaattatttatcagaccgttattgaacatgtggagccggccgacaattgtgtttattgttttattaacggcagttcaactggtattctactacacactcaaactcattcaaaaaccacaatcaaaataaatgggatgctaccgtaattcgacggttcatccctttttatttgcttcaatatcaatccgtcacgaacttttctctaaaccgcgcaatgtaatcgctgggcagatccaacccatttttcaaatacccatcaaatgagccaaagtgttccagcaaaacatcgttggcgtggcgtaaataatcggcatcaaccagcaaggctgtgtgcaggttgtccaattgctgctgattcatttcatttttgaatcggttgagcaaatcttcattggccttgacccgaagttgattggtcagcagataatcatccataatttgttgatcgtcagcgccagccacctttaaaatcacggccgctgcaaagccggttcggtcttttccagcgaagcaatgaaataggatcggtgcatcatctgccagcaaatccgtcatgaaatcatgatacccctgttgggcagactgacttaaaacaattgattcataagttttaagcatattctcatgaaccttgttgccgtcggtaatcatagcccccagactagccccattagacgttttatcagacaaaatatcaatatggtaatatttggcaccagaaatcgcactatccggtgcctgtttgacttcatccgtactcctaaagtcgtaaacatcccggatccggcactggtcttgcaggaaggccgtttgttcctggctgatcccggcaatttgaccgcttctaaaaaagtatcctgactgcaattttccggaaggaactctgattccgccgatgtctctaaagttcactaaccctttgtcattcatttgaagtccccctactcgttttgataatccataatcaaaactgtttcagaatagttaatatattgtcttaagtgggcagccatcgaccagtcaatattgccttgttcgaggagcacctgcacgccttcacgttcggcagccaaggccttaattctcaggctctggtagttcatcgcctgatcattgatctgctttttggaatgatccttggccagctcaatctgatttcgataatgcacaattaaatgataaaccgactgactgtcaaaccgttgattgtcaatatcgtcacgggcaaagtagtcggataatgccgagatagccgccttcgcctgttctcgctgaatcagggccagctcatcagaaatatcttcattcgttttgcgccgaatcaaccacaaagagacgcgattccgcagtttaatgaaattccgcgcggttccatgcccaagtttgactttccgaccaaccgagcggatcatccgattttctaaacgctgcagcttggcattggcaatcaagaaagcctgtttggaaattttttggtcgtcaaataatttctgaacggcagcccgttcaccacgaagagcaacccttcgaagtgccaattcatcagcaatgatggagtccatttcttttttatcttggagttttaattccagccttcgaatcagaaactgataatcgagaattaagtcaaaagcctctttttgattattgggccgccgttcttcttcaattcgttgaactgccaatttcataatatagacgcgggcctcatcttcagaaatgtattccgcatcgctgtcggctgaaccggtatcaatttcatccggatcatccgttgagttggctcgagtcaacagtggtgccttatcctcagaaatcaacggcaaggtgacggtggccacgaccagtgaaatgatgatcacaccggcagcaacgaataacgccagtgatctggacggaaacggactgccattatcaatcgtcatgggaatcgataaaactccggccatggtaacggccccccgaacgccagacaatcctgccaacagcgccgccttaaaggtgggcatttgcttggtttgaattgatttgatttttcgggagcgaatactgctgaccgcttggtaggcgtagatccagacaactcgaatggccaacaaaatcagccaggctagaaaagaaattcccagtgcagcaaaggtattaatcttgttattttgaatcacattggtggttgctaacggcagttcgattcccagaattaagaagacaatcccgtttaaggtatagataataatgtcccaggttttttcactgaccaatttgagctcgggttgactgcgatccggtgccgttccgtaaaagtggaagatgatccctgcggcaaccaccgcaatcacaccggaggcatgcaaaaattcttcagtcaccaggtacaccacgaaaggcgttgtgacctgcaggaccgtgctaaaaatgacatcgttgattccctgtcgatacagccagttttcaatcatcaaaatcagccccataatgaccagaccgctgacgaagcccataatactgatataaacaaagtcaatggcggccgttttaatggagaaaacgccggtgaccgtggctgcaattgcatatttaaaggcaatcaggccgctggcatcgttgatcaggctttcgccactgacaatgtgtaaaattccttccggaagctttgcccgtttggaaatcgactgcacggcaaccgggtcggtcggcgacaggatcgctgccagcgcaaaactgaccgaaaacggcatagttggaataattaagtgaaacagcaagccgcctaaaattgtcgtcaaaaaaaccaatacaattgcattggccaatatgggtccccgcaacttccacaactcctgcttggggaacctgcgcccgtcgttaaacagcaacggcgcgataaataatagcaggaaccaatcagtttcaagcggaatggtcacccgcataatcaaagcggctcccagtcccaaaacaacttgaattaaactaaccggaaccgctggaacaaaatggtcaacaacgttggaaaaaacaaccaacgtcattaacagaatgaccgcttcaagaatgtgcacgcattaccaactcctagtttgacttggggtcttctccaataattctgacttccgtctccagatgcacgccgaatttgtcgtaaacggtcttttgaacatgggcgatgacgtttaaataatcagtggcagtggcaccatcgacattaacgataaaaccggcatgtttcattgaaacctgggcgccgccgatctggaagccttgaagtccggcatcatgaatcagtttaccggcaaaatagccggttggccgtttgaagacacttccacaggacggcagttccaacggctgtttagaggcccgcagagcattgagatgatccatccgcttttgaattttgtcagcaatgccgacttctaaagagaaggtcgccgaaatgacgatttgatggttttcttgaacgctgcaatgccgataaccgaaatccagctcttgatgattcaagtgaataatgtggttgtcgggtgtcaagacttccgccccactgacaacattggcgatctcaccgccataagcaccggcgttcatgaacaccgctccaccaacgctcccggggatccccgctgcgaactccaagtgagttaacgaatgggcttgggcagccttggtcacgtcaatcaaagccgctccggcatccgcgacgacctcattatcatgtgacgaaatccggttcattttggttagaatcattgtcaggccacgaatgccgccgtccttgacgattaagttgctggcattgccaaccacagtgaccgggagcgattgctcgttggcataatccaacatttcttgacattctttaatcgatttaggaaaggcaagaatatctgccggaccgccagtcaacgtgtgggtgtatttggataaaggttcatttaacagaatctcaatttttggatataaatctacaacagtttttgattgcatcatttttcaattcctcggtttcaaaacatatacattaattttaccacgaaacaagttatctatggggcggaatagccgggaagcactccggttgcgttttcacgaggttctttgtacaatgtgattaacttgaggtgaaaaatatgaattttgttgcgatggatttcgaaaccgcaaacgcaaaaagagccagcgcatgttcaattgcactggccatcgttcgagataatcaaatcactaacgaattttattcattaatcaatccggaaatggactttagttggcgaaatatcaacgtccatggcattcatgaacgtgatgttgtcgatgccccgacctttccggaagtttggcgccacattcaaccgctgttttcagccaataaattggtgattgcccacaacgcatcatttgataacagcgtcttgaaacgaacactggaacgttatgaagttcaaccgccgcactatctgacactggacacgttaaggacctccaagcaattctacccgacgttggaaaatcacaaacttaacaccctttgcgataagctcaacatcgttttggaacatcaccataacgcgctggacgatagtgttgcctgtgccaatattctattaaccgaacaggcccaatttggcagcgatatgctccggccatttgtcaaagcaatctaaagagattggaacgaacttagtttcatcccagcattcaacaaaataacgcaaccattccaagattagggatggttgcgttatttcattaagtgcctgagatcaaccagtcatcacgtccgtttaataaaaaagtggcggtcttagttgcaataagcaaccacgtcactcaaggcttcaatccttttttgggacatcaaaggccattctcacaacttcacgaccgtcttgaaagtacacgtcggtatcgtgaaacccaactttgtaataaacatgaatggccggctcattcttcgagaaaacagtcagcaccagttgatcaagcgagctaaaatctgttgcccagtcaatggccagttccatcaagttggtgccaatcgagtatccttggtaacccgcaagaacggccacgccgacttccccgactccattatcaacactgtcaacggtcacaatcccaatcaattcggagccataggtggcaaccgccatcaaattggtccgggaatgattgatcaaattaatttgttgggcttcgtcggctgcggtaatgtcatccaaatcagaatcgaccaaaaacgtatcggactcgccttgaagaaccttcaacaaatccaaaattgcctgaccgtcactcggttctgctaaccgaaagtctacttcttctgccacatcattgctcgctttccattgttattctgaaaatatatcatcaattagttgttcaaaacggtgcccggtggcctcaaaagtcaatgttctcacgttgtcgccctcagaatcatcccgccgaaaaataatccggagatagtcatccggtagttcgtcggcaacaaactttgaccattcgaccacgttgaccccgtcgccattaaaatattcttccaagcccagatcatcgccaccgccttcttcaagtcggtacacatccatgtgatacagcggaattcggccgtcttgatattcgcgaataatggtaaatgtgggactcttgattggtcgcgtaatccccaatcctttggcaagtcctttggtaaaggtggtcttcccagctcccaaatcaccatcgagcaaaatcaaatcttgtggcgccaagtatgcggctaatttctcaccgatcgtcatggtttgatccgcggaatggactgttatcgttttagtcaattaatcacctcattcaaaaaggaaggattgcgacgcaataaccaccgcaatcctaccctgtttaattatttctattataaggcctgagctgctgtgatgatagcaactttataaacgtcttcttcattgctgcctcgtgacaggtcagaaacgggtttgttcaatccttgaagaattggaccaatcgcttcaaaaccaccgaatcgttgagcaatcttgtagccaatgttgcctgattgtaattcagggaaaacaaagacagtggctttaccggcaacatttgaacctggtgccttcttctcggcaaccgttgggacaaatgcggcatcaaactgcatttcaccatcgattgccatatcaggtgcctgttcttgagctaatttggttgcctcttgaactttggtgaccatatcacccttggcagagcctttggtcgagaagctcaacagcgccactttagggtcaatatcgaaggtcttggcaaccttgccgctttcaaccgcaatttctgccagggcattggcatctgggtccaagttgatagcacaatcggcaaataagtatcgttcgtcacccttttgcataatgaaagcaccactgattaatttaacgccgggcttggtcttaatgatttgtagagctggacgaaccgtgtcgcccgttggatgattggcacctgaaaccatcccgttgattttgttcatgtagaccaatgtggttccaaagtaatttggatccttcagccaatcgcgcgccttagcctcatcggtcttgcccttacgacgttccacgatagctgcaaccatttcatcgatttgatccgctggttggttcaggtagtcgataatttcaacgttccccaaatcaatgtcagcgtctttagcaactttttcaacggtgtctttagcccccagaatcactggattaaccagtccgtcctttgccagacggctggcggcaccaaggattcggacatcgtcaccctctgggaaaacgatactaatgtttttgcccttgatcttttgcttaagactttcaaataattccatgataaatcctccaattctacaaaatcagtctaagatgtttgcgataccttttccggcagctgccagttaatcggctcctcgcccattgcttccagtgcttcattggtctttgaaaatggtttcgaaccaaagaatcctcgatgagcagacaatggactgggatgggccgattgaatcaccacgttggtcttcgtatcaatcaacgcaatcttatctcgggcagctctcccccacagaataaagacaacgggcttctcacgagcggacagtttttggatggccgcatcagtcagttgctcccaacccttccctttgtgggaaaaggcctggccattgcgaacggtcaaaactgaattcagcagtaatacgccctgtttggcccagctttccaaatcaccgtgttcaaccggtttgattccgaggtcagactgaagctccttataaatattctgaagtgacggtggaattttaacgcccggcatgacagaaaaactcaatccctgggcttgatgaggctcatgatagggatcctgtcccaaaatcacgacctttaccttgctgaaaggggtcagctgaaacgcctcaaaaatgtgattcatatcaggatgaatatattgcgtcttgtattctgatatcaaaaattggcgtaactgctgataataagttttctcaaattcgggctttaaaacatcccaccagtcattttttataaacggtttcattcccaacacctcacgttttattctaccataccatttttaaaataacaccagcgtaaataatttcagaacgtgttaaaatgaaaataatacaagtaaaggaaatgcgtctatgagtcgaaaattacagttgaatttaaccgaactggatcacacccgttcgactaaggtcaccgatcaatatcgagacacaaaatatttaattgtcggcaagtggggcttgattgacgacactttttcaatttactcaatttcaggtgaagtcgtggcaaccgtccgtcaacaatctctgggcatgacgcctaaatttgatttgtattacctggaccaatttgtgggcggttccgtgatccattttacgatgcactacacaacgatttttatcaacggaattaattggttggttgccggtaatcaggacaaacaaacttaccgaatcatgcacggacgccagcggattgcgacaatcaagtcatacagtcagtccgatcaagtcattcggatcatggatgtagacaataccaatcatgagccactggtgcttgccattgccgccattctcaatcatccctcgttggcacatgcttcccgattgaagttgggtgttttgaataaagcacccgtcaaaccaaatcttgaaagtgaaaatatttcgaccctgcacaatgaaaataagcgatgaatcagtcggcagcttgccaattgatttcatcgctttttgtttgagcttgattaataatgtttcataactcgttcaatttgacgcttttgatcacgtcgcttgatggtttcacgcttatcgtactcatgcttaccagttgctaccccaattaaaactttggcaaaaccatttttgaggtagacctttaaaggaacgattgtaacccctttgtcttgagtaatttgagccaatttgcgaatttgctttttgtgcagcaacaactttcgattgcgcagcgggtcatgattaaattggttcccctcagcgtactcactgatgtggacgttcatcatgtaggcctcatcgtttcgaatttgaacgaagccgtcctttaggttaatccgccgagcacgaatcgatttaatttcggtacctgtcagcacaattccagcttcgtaggtttctgaaatcgaataatcatgacgggcttttttattttgcgccatcaaattatcgttattatgctgctttttgcctttggccatcaaatcacctcgcttacagcttaatgtttattatggttccgatgtccgttgttgccatggttgttgtttctcccacggttgttgttggcgtgattggaacgggaattgttattcgaattgccgtggcgctcgttattgccatgatagttattattatgataagtccgctttggcagcatgttactttgtggcgtcttttcaggatcaacaatatcaaagtcaacggcactctgcttgacgtcaacattgaccactttaactctgattgcctgacccatcttgtaggttcgacgagtgtttcgaccgaccaaggccataaattgttccacgtattggtagtagtcgtcgttcattcgactgatgtgaaccaagccttcaaccgtatttggcagttcaatgaacagaccaaatttcataactgaactgacaaccccatcgaattcttcgccgatgtgatcgttcatatattcagctttcttcattgaatcggtatcacgttcggcatcaacggcccgacgttcgtattgagaagtcgtcgtcgcaatttcatccaacacgttggcataacgtttcttggtctcatcgttaatcccgttatcttgataataatgaatcaatcgatgaaccattgtatctggataacgccgaattggcgatgtgaaatgggtatagaacggtgctgccaacccaaagtgtcccaaagactgatcggcgtaacgagcctgcttcaaactccgcagcagcatcactgaaaccatcatttcttcaggcttgccggcaacttttttcaagacattttgtaaagtctttggggtaacgtgctctggatcacccttcacattaatcccgaatgcggtcaacgtctcaaagaaggttctgattcgatcggcatccggcgtttcatggacccggtaaataaagggaacgtgtttttcatagtagtgcttggcaaccgtttcgttggcggccagcatgaatgattcaatcatccgctcggcagtaccacgaacccgcagcttaatatcgattgggtggcctttgtcatccacgataatttctgcttcgttatcgtcgaagtcaattgccccacgcgcttttcgatgcttgtataaaattttgtgcagctcacccatggtttcaaacatgggaaccaatttatcgtaacggtccatggttttttgatcgtgagattccaaaatgttgttaaccgctgtgtaggtcattcgggcggttgaacgcattaaactggggtgaatccgatgcttgatgatattgccggatggatcaatctccatctcacaactcatacataatcgtaattcgccttcgttgagggaacagatcccgttggataaacgtcttggcagcattggaatcacacggtcagtcagataaacggaagtcccacgacggaatgcttccttgtcaatggcgctgccgggttgaacataatggctcacgtcagcgatatgaacccctaaatgataattgccattggggagtttccaagcggtaaccgcatcgtccaaatctttagaagattccccgtcaatggtcaccaagtcctgatcagtaatatcttctcggccaatcttctcggcttcagtcacgtgatctgggatggcatccgctgcctgaatgacatcttcagggaactcagcgggaatatcatgggcataaacaatctgtaaaatgtcaattccagggtcatcaactgatccgatgacttcatcggcaatccccaccatgtaatcagggtgcttggtagatggatattcggtaatttgagcagtgatcacttcaccaggtgttggtttcaggccaacgtcgttgatataaaatttgtacttggcaattttcttatcgttgagggttaattgaccaatgtatcctttgtcatcatcagtcttttcaaacggtccaaccacgcgggtatatttgtgttcggcaattttagtgactttaccttccgggccccgatcagatcccggttgcgccggccggacaatttccatttccacagtatcaccattcagtgcattcatggtgttatcgggcgcaatgtaagcatctggagcattttcatcataagcgacgaaaccaaaccctttgtcattagcgtggaaaataccacttaattgttgtttatcaggattcaattgaaacttgccgtcttcagtcacaacggcgactttatcgcgttccaaagaagccaattcttgaacaatcagcttaaaggctgctgaaccatgcgatctcaggacgtcagcaattttctcgacagtaaacacgttatccggataggttcggagaacgttttctatttgatttttcaaatcattatcttgcaatctatattcctcttattattcataaagttgtgttaaaaattcggttaaatcagcctcaagctgcttgtgagcaggattaacggtaatcatgtgactggcgttggggtattcgtggtaactgacccgactgttcaccaatccatccctcaaagacttggcactttcaggattcacgatctcatcgcttaacccctgaccgatgaagtatggttgggtgattttaggtagatcctgcgccacaccaactgtgaaatcagcaatcttacctaatagtatatcaatattttcgtcaagccacttgagttttgaattcataatcgcttcattggtatcatactgaacaaaattggctttggccatttgcataaaggtattatgaacactaaactgacgctttcgaacaattggtgatccaaacgaaccgccgccgagtaaagtcggatcattctccagcgttttagcggcaaaaataccgcccagcgagatgccaaagatactgatttggtcatagcccttgtcctttagaaactggacggcccgtttggcatcattccaccaacgctcgggcgttccctgaatcaggatatcggtaaaatcagccgtcccatggcccgtaaacattggcgcatacacggtataattctgacgctccaaatacctcgcgagcattcgaacgtcaaccgggccactggcaaaagcatgcaacagaataattgctctcggtccgtgttcaaaataaaaagatttgactggtgtttgcatagcacccatcctttcatgtccacccattcaattataataaaaatcctcctgcatttaaacaggaggattgaatactaatgagatgatatccaaactaatgcaagtgctaagagaaagaaaataatccctaaaacaagtgtagttttttgcatgaatgcttcaaagccacgtggcttctgctttgcaaacaagtcgtcggccccaccagttaaggcggacatggcgtcattagtctttgatggttgcattaacactgcgattgtaattaaaacacagtcgatcagcaataatgttaacaaaaagttgtacacgttgatagcctcctaccgttaaatcggcttaatactactcttactaaactaacacattatagcagaattcgctaccttttgggattaagtttctgttgttaaggcaataatttgttgagtgatcgcgtgctgatttttagtcgagacgttaatgaacaatgtatcgccccatcgaatcaaggtgccgccagcaggcacaatttcgacaccatttcgttgaatcttggtcagcagtgaccccattggccatttgatctgacgcaccattttgccatccatctgtgaaccggcatacacagtttccataatttcagcagttcgacccaaattcatcttggtctgaactttcagcagctgctgaagcatcgagtaatagactggtttgccgtttaacaggtctaagacgccgtatgcgattaaagacacgaccgccaggccaaggagatgggtcagagtcccaaccatctctgtaatcaaaagaattgccgtgaaaggggccttactgattgccgcaaagtatccggccatccccataataatgaaactcgagaaatacagtggattcatcaacccaagattgacagcgatactgccgacaatcgcgccgattaaaccaccaaggcaaagaattggcaggaaaatgccgccgggaaggccactcccgtatgaaagcattgagaaaacaaaccgaattatgaaataaagacataaaatcagagttggataatttgccgaactcaacctcagaataatgtcactcccgccacccaacaagtgcgggaaaaacgctcccattgggatcaccaacaacagcggaataattccgttgaagtaccagggaatatgagtatgccgataccactttcccatccgaagaataaccatctgatataaccggcccaacacgccaaggacaattcctaaaatgacaacccacaaaaaatatttgagtggcagtggcgtacttcgcatgtataaaaccggcttgagtccaaaaacatacgtcgcaaccatgtcagaagtgaccgcagatgtgagcgaaacaatccaaatattggtggaaaagttatgataaatctcttccaaaacaaacagcgtactggcaattggggcgttaaaagccgcacttaagccagcagcggcaccactggaaatgagcacttggcgatcaaacccaacttgtttggtgaaatgggcaactccctgccccaaagttgaccccaactgaattgagggaccttcgcgaccaaggtataaaccacttccaatcgccaaaatgccaccaacaaatttccgccacagaatcgcccaccagccgtaatcaacctcacctaacaattgaccttcaacttgtggaatgccggatcctttaatatccggctgctgctttagaaaccagccaaccagtaagccaatggcaatattaatgacaattgtcgtcagtagaaacgacagatgatggatcgaattgatataaagatagcgcatcaaatccgtcatatggccaattgaccaccgaaacattgagactgccgaaccggcaagtacaccaatgacgatcccgttaacgattgtttttacttgagacagcttgtaacttcctcttacctgcaattttgctcatcctttaatgatttctgatatccattatatcataatcaaatgagtcgtttgaaaagttttttgccgattaacgcgccaagaagtgccacccccgataaaacaccgacaacggactgcgattcaccggtttggggaagcttttctgaaacttccgaagtgtctttggtttcgctgtgtcgctttgatttggtttcagacggattccggccactgatagctgattgacgcccttttttgtggccagtctttgagctgagtgcagtcggttcagctaatggcttgtttgatttgtcagctaatttgatgtaagtgaagtgcacatcttcaggcatcagattgtcagccttcagttcctgagttggttgctgaacccgataacctgaaataaacttggccgtgtaagtcttggtttggccatattcaagttccactgagtctttagagatggttttgccatcctgatccacgttgataatattaaaggtgacttttttagcagtataatgcaatgtcagggttttcgaacttgcatccaggtcggtggactgtaattcatagccataaaattcgacgttctttgaccggaatgcccgagcctcttctgaagtgagatgcagggctttattgaagagtaagtggccgtgagtgtcgatcccatggagttgataggttgtggtcattggttgcatttcctgatgatcggttgatttttcgggtacctttgtctggttgattttcggaattttgggttttgtttgaacgaccggtttttctgagtcttttgaatcagattcggaagtcttaactgtgttctttgtggagccggattgatctgtggttttaccaggaaggtcggctggcttttcagacggcttcgcagacgtttttgaaattccctgcactttttcatcgggtttgagtgattcggctgtggtttctaccggcttggatgatggggattttttgccggtttcggactgaacggatgatgtcgactttgcattagtcgacgaatctgcaactgcgccttcctttttgctttcaggtttagtaacacgagtctctttatcggaccgtgatgacgccccattggttttagtggtgggctggatttttggttcaggatccggcaatttggttcccggcgccgccactggtggggttacttggctgttttcagtccctgtggcacccactaccttcacctttttatcatcatgtttggggccggacttggaagcggtagtgtccttgacttctttatcgggcgtttcgactggtttgacagccggttggtgcgttggttcagtttgggtaaccgatggaacgacatgattgccagcctcgctcggtgtacttggtgatggttgcatgtcagttgtcgcagtcgttgaaaccaccggcgttgaagcagactcgctcatgggcttttcactaacgagctgaattggttcgcttgtctgcccagtttcaccagacttggaattaccaggttctggctggtctggtacaaccacattagccaaccaatccgcagcaatcaatggattaaggctcttatatttgagggtcacatcccagttggtctctttgatttttccattgatatcctttgaattgagcagttcataacctgaaacgtcaaattcgtttttattaaggcggtaggtcccaaagatagttgcttgattgaaaaccttgttgtcctgaattggttggttgttttcatcaaggtacttgatggtcaccacagcatcttctgccatatagttaaccaccattccgggagaataatgcacttcggaaacgaccggatggtaatgtggaacgttgtccggggcactaaaggttgacgacttactcttatcaatgtacatcttgactgtggcttgtttgtcaagcaccgacttgtcaccacggatgtttctaacttgaaactgttggtggatggtaattttgtcaggaaactcctgggtagctgtttgactgatttcagcaccaacaatctgctcatgcaccagtggactggcgaatcccagcacgcctaacgaaactgataataaaagtgtttttttcaaaataatacctccattatttatgatctaagagttagatacgcaaaaatggaggcgttttatgtacaaaaaaagtcgctttcacgacttttttcaaattacttgtttaagatgtcttggcgtgcttgttctgacaagttgtagaatgagtgaattcctttgtaatcggcaacgtcaccgagttggtcttcaattctcatcaattggttgtacttggcaattcgttcgccacggctcattgaaccagtcttgatttgaccggcattgaggccaacaaccaagtcagcaatcgtggtatcttcagtttcaccagaacggtgtgaaatgattgcagtgtagcctgcttctttggccatttcaacagcttcgacagtttcagtcaaagtaccaatttggttaagcttgattaagatcgcattggcaacgcccatgttgatacctttcttgaggtaatcagtgttggtaacaaacaaatcatcaccaacgatttgaactttcttaccaaggcgtttagtagccatttgccaatcagcccattcgttttcatcaagaggatcctcgattgaaataactgggtatttgtcaacgatgctttcaagcaaagtaacaaattcatcagcagtgtatgacttaccgtcaccctttaaatcatatttcttagtatcggtgttgtagaattctgatgctgcacagtcaaaggcaatggcaatgtctttacctggcttgtagcctgcacgttgaatagcttcaacaaggatttcaaatggttcctcgttgttcttcaagtcaggcgcaaatccaccttcatcaccaacggcagttgagtatccgcgttcgttcaacaagttcttcaagttgtggaatgtttcagaactccaacgaatagcttctttgatggttggagcaccaacaggcatgatcatgaattcttggaaatcaaccttgttgttggcatgcttaccaccattgataacgttcaacattggtgttgggagcaagtgaccattgaaaccaccaaggtagttgtacaatggaacttccaattcatcagcagcagcacgagcagcagctaatgaaacacccaagatcgcattggcacctaacttacccttgttgggggtaccgtccaattcgatcatagccttatcaatagccaattggtcagtaacatcgtagccaacaatttctttagcgatgatgttattaacgttgtcaacggctttggtaacgcccttgcccatgtaacgatccttgtcaccatcacggagttcaacagcttcgtgttcaccagttgaagcacctgaaggaacgattccacggcccattgcacctgcttcagtatacaattcaacttcaacagttgggttaccacgagagtctagaacctcacgagcataaatatcagaaataattgacatgtttttttctctccttagcgaaagttgtgaccttttgtacaaggttcaacttcaattctattagtttctcgccgaagtttcaacataaatcagcgaatttaactatttttgtaaaaagtttgcaagctttaagaatgaatccggttttaagctggcaccaccggccaaaacaccgtcgatatcagtctgtgacagaatgtcatcggcgttttcgtcgtttacactgccgccatacaagactcggacttgatcggcaatatcatcgccatacaaatcagcaatggtttgacgaattaaataacaaccctcttcggcttcatcgctgctggcggttttgccgctgccgattgcccaactgggttcgtaagcaacaatgatcttctcagcttgttgcggggtaatcgatttaagggcgttggtcacttgactgaccacccaggaaattcgatcagcggattcacgccggctcatcgtttcatcacagcagatgattggtgttaattggttgcgaaaagcagcgtgaacctttttattaataatgtcgtcggtttcgttaaagtacttacgacgctctgaatgaccaataataacgtgggtcacgcccatttcggcaagcgctttggggctagtctccccggtgtatgcgccctcgtcttcataaaaacaattttcagcggagataatcagtggtgaatcaccattttcttcgaccatgctctccaaaaagagtggtgaagccgcaatacaggtctcggttatcttaggatcgggtaattcaccctcgatggcttgaagaaatttgactgcttcagcgactgataaattcattttccagttacccgcaacgaacggaattctcataagaatcatcctttacattttttagcttaatgccattgtaaccaaaagagaatttaaaagccacatttttctcctataccaatttttagtaaaagaaaaagagctcgctaaatagcaagctcttcgtcaattatttgttgtcaattgctgcaataccagggagtgttttaccttcaagatattgaagtgaagcaccaccaccagttgaaatgtgggtcaatttgtcagcaacgcctaattgtttgacagcggcagttgaatcaccaccaccaacaattgtagtcgcatcgtttaacgttccaaggaacttaccaatgcgaagggttccttgggcatagttaggcatttcaaagacacccattggtccgttccaaacaacggtcttagcatctttaagaacattttcaaagtcttcaattgacttaggaccaatgtccaaagccatccagccgtcatcaatgtcaccggcaacaactttgtgttctgcgtcgttcttaaattctttagcaaccacgttgtcagttgggagaacgatcttgtcgccacccttttcaaggatcttcttggcaacatcaatcttgtctttttcgatcaatgagtcaccaatcttgattcctttggctgcatagaatgtgtaagtcattccaccaccgatgatgatcttgtctgccttgtcaagcagattatcaatcacaccgatcttatcagaaactttggcaccaccgagaatagcaacaaatgggcgctttggattgttaacagcttcgcctaagaactgaatttctttttccatcaagaaaccagcagcaactggcttgccgtctttgtgcattgcttcggcgattccagcgtttgaggcgtgggatctgtgagcagtaccaaaagcatcgttaatgaattcgtcggcaagtgaagcccagtattcacctaatttaggatcattaccggattcacgcttgacgtattcaccattaacgacatcttcataacgagtgttttcaaataagagaacactgccgtcttccattttgttgatggcgtcttcaagctgtttaccttcagtaacgggaacgaaaataaccggcttgttcaataagttggaaagacgttctgcaactgggcgtaatgaaaggcccttcttgtcgtcttcttttttgattcggccaagatgtgagcaaagaattgctttgcctttgtggtccaaaacgtacttaatggttggtaaagcagcttggatacggttatcgtcaccaataacgccgtctttgatcggaacgttaaagtcgacacgcatcaaaactttctttccttcgagatttaaatcagaaactgttaattttgccaatttggaaacctcccaaaatcgatttgatttgtgatctagagaacatagcgagatagtaaaagacggagaaggccaccctcctccgccaattacaattaattattaaagtgaagcgaacttcaacaaggtacgaaccatgttgcaagtgaagccccattcgttatcgtaccaagcaacagtcttaacaagttggctgtcaccggcagtagtaacttcagtttgagttgggtcaaatactgaaccatgtgaatcatcaatgatatctgatgaaacaatttcgtcagcgttgtaaccaaatgcagggttgtcagcggtgtgcttcttcatagcatcgttaacttcgtcagcagtaaccttcttgtcaaggactgcaactaattcagttaatgaaccatcaacgacagcaacacgttgtgcgtgtccttggagtttgccggcaagatctgggataaccaaaccaatagccttggcagcaccagttgaatgaggaatcgtgttagcactggcagtacggttgttacgcttcttcttagtcttaggaccatcaagaatttgttgtgaagcagtgaatgcgtgaacagtcgtcatagtaccaactttgataccaaagtctttgttcatgaagtaagccattggtgccaagcaattagtggtacatgaaccagctgaaacgatgacatcgtttgagttcaattcatccaagttaacaccaggaacaacagtcttaatttgaccagcaggtgctgaaatcaaaacacgctttgcaccagccttgatatgagcttgtgatttttcttctgaagtgtagaaaccagtacattcaagtacgtagtcaacaccgtcatttttaacccaaggaaggttagaagcatctttttctgcgtaaacaggaatttctttaccgtcaacgacgatacccttgtcagttgctgaaacatcaccagggaaacgtccatgggttgaatcatacttcaataaataagccaacattgatggagtggtcaaatcgttaattgcagccacttcaatctcgtcggagtgtaattcgtggatccgcttgaaagccaaacgaccaattcggccaaaaccgttaataccaatctttacagtcatactaagttttcctcctttaggaaataagaaaatattaagacacagtacacgttaatcgtaccatgaaatgaaaacaaagtcagcacccttgtgaacgaaagttcaaagtatgcatcgagtaaccataaaatattacccaaattcgagtatagcagaccgcgggagaattgcaatgcaaatggatttagtaagcgttttcacaatcaatttttctttgttcttgaaaaagttctcactttctagtatattggtataggaagttgcgcccgtagtgtaatggatcgcacgtaagattccggttcttgaaatgagggttcgattccccccgggcgcatcagatttcactgacccatcgcaagcaaggattcatgtttcattaggtcatttttgacacataggtaattgtgttagtggtgaaactaggttcagtggacacaaaacaattttaatcaacgaaacagcgaggcagatgccccgctgttttttgtaagcaatcagcttgatcgtcattccgcttttttcatatacagaattggaaagtgattgccctgttcatcaaattccgtgcgcttgtaaacttcaaatcccatgtgctcataaaatccgcgcgcaagtgggttttgttcgttcacaccaagctggtcgatcgaatactgctgcatcccataatccaatagtcgtttgcccaaacccttaccacggtattgatttgagataaacaacatttcaagcattcggtcattaattcccatgaagccaaccggatccccattgtcgttttcaatcacgattaaatgctggacgccgccaatagcttccggaatgaccttcttaatcttttgaatctcgttatctgtcaaaaataaatgggtcgccttgacggaactctcccaaaccgtcaacaagtccttcaccaatttgggactgaccttggtttcttcgacaattttcattctctttctcactttcatgcaaactgactagcgtgtgtctgttcctatgccaaacaattcaatttatcgcttctggagtgccaaatcaagtcccaaaatatcttaggtaagtcatgggatgtttctgaagtttggtcctctcaatggtcggcttgatttcacaaacaacaaagaggtccaagcttaatccttgaacctctttttttgatggttaatcttttcttcgcaattcaacaacccctggttaatccgggacggacgttggctctcgaacaccttcggtaaaatcaacgccttctttagcatagaagtccatgatctcttgacgttgggactcaaatttcggtggcaatgacagtccctgccccatcgtcaaaatgggttcttcgagactaaaccccggagtcgtcgtggcaatttcaacccggttatcaccaggatctcggacgtacaaactcttgaaccagccacgatcggcatactcttcaatgtttaagtgctgttctttggcaatatcccagaatttgaacaaggccgccttagttggggcttgaatcgcaaaatgatcaatactgccccggccaaaccgagtccggacatcttgctggtcactttcaaataattcaatggactggccgtcctccaattggacaacattattttctaccggaatgcccaaccaattatggaaaaaggcactggtagcttcaggatccggcacgtggagttctgttcccattaaatgcgtaatttgtttttcagcggggatcccattatcaggaaccacccgcatatcggttaaaacttccgaagtctccaataatttaacttcgacatcatcagggtcagcgaacaccaggccatggtcaatatcttgaacagccactgaatggtcggttaaccgtttcttccaaaaatcagtgctcccggttggaatcgaaagtttgatattattgaagaaatgcttaccgtcagtccgatggcctaataatggcaccacaaaaaatgtcaccactgatcctggtgttcccagatagtcaccgtagaataagtgacgaatgcggatattttcctgattgacggtgttttttaccaggcgcatccccaaaacccgggtataaaaatcaatgttttgttgagcatctctggttaacagtgaaatatgatgagttctcatagtatatcctcccgactcggtatttgctgattaccgttattgtatcacgaatgaatccgctttcttattataagcatttctttatcgaagcacagtgaagattgaccggaaaaattaatgatttgatgtgagcaaaacatttgaccttttttgaccaataaactatcatattaacatgaacttggcgtaagccatctttcataaaacctataaggaggcatcttgaatgaatttagtgccaaccgtcattgaacaatccgcaggcggtgaacgtgcgtatgatatttattcacgtttgctaaaagaccgaattatcatgttatcaggccctatcgaagacgacatggctaatgcgattatcgcccaattacttttcttggatgctcaagactcagaaaaagatatttacctctacatcaactcacctggtggtgtgatcacctcaggcatggccatttacgataccatgaactttgttaagtcagacgttcaaacgatcgtaatgggaatggccgcatcaatggcttctgtccttgcttcttctggagcaaagggtaagcgatttgctttgccacatgcccaagtcttgattcaccaaccttctggtggtgctcaaggtcaacaaactgaaattgaaattgctgctgaagaaattctcaaagctcgtaagatgatcaacaatctcttagctgagaattccggtcaaccaattgagaagatcaacaaagacaccgagcgtgataattatctcactgctcaagaagctgttgattatggccttttggatggcattatgaccagcagttccgaaaagcagtaattcaattcgttaattgaattgtatgatgcctttcaaagcagtcctcattttgtgagggctgctttttttacataatccacctgattgataattggttgatgaccgactagaatataggtgaagttagttaaaaaattaacatgatgaatgatgaatcgaggccattaatatggatgtcaatcaaacaaaagaacaagttaaacaaactgctgatgaatcaatccctactgagatgaaggcctgggaaattgttaagcccggttcaattaacggtgcggtttctcctttacgttacaccaccaagccggtgccaaaaccaaaacgaggcgaagttttggtcaaggtcatcgcttgcggggtctgccacacggatctccatgtaactgaaggcgatctgccggttcataaggaacatttgacgcccggtcatgaaatcgttggtcgggtcgttcagatgggtgctgaaacccgtcgatttaaattaggcgatcggattgggattccttggttacgttggacttgcggggtttgtgaatattgccggtccgggagagaaaatctctgccccaactcactttataccggctgggatcatgatggcggctatgcagaatacgtcactgttccggaaggtttcgcataccggattccggcccggtttgattcactgacggctgccccactgctttgcgccggaatcatcggctatcgggcatatgaacgggctaacgtccctgcaggcggcaccttgggcctgtatggcttcggcggctcggctcatttgaccgcccaaattgcaatgaagcaaggcatcgaggttcacgttttaacccgtggtgaagatgccaggaaatttgccctgcaactgggagctgcctcagccagaggaacctatgatatgccacccgttaagctggattcggcaatcaactacacaccggttggtgacgtagttccaaaagccatggaagcgctgaaaccaggtggcacgttggcaatggccggtatccactcaacagatattccgcaaatgagttatccaagtcacattttccatgaaaaaaatctcaccagtgtcgaaagcaacacccgtcgggatggtgaagagttcctgaccttagctgatcgactcaatatccatccggaggtcactgaatatccgttggccaaagctgacgaggcgctgaaatatattgccaaaggtgatattcgtggtgcctgtgttttaagagttagtgagggctaacctctgtcattaacagttaaatgattggattcaaaaaggattctaactatttcacagcgaaataattagaatccttttttaggtttaaaaatgtgttgaaactttactagcttggtcaaaactaaacttcaggggtcagtccctgagccagcttgccggcatattcgttaatctttcgcaatcggtgattaactccggatttggaaattggtccaccctccaccaagtcgcccaactctttcaaactgacttcgggatgtttcaagcgcgcccgggcaacttgggccagcttagggttcagtttatttaatccgaccatctcgtcaatcagtttgatattttcaatctgcttactggcagcgttggcaaccttgttgagattggcattttcacaattaaccagtcgattcacggagttgcgcatgtcgcgaacaatccgaatatcttcaaatttcagcatcgagctggtcgcaccgatcaattgcaaaaagtcggcaattttttcagcctctttcaggtaagtgatgtagccgcttcgccgttgcgtagtgcgggctttgaggtgatacttgttcatcatttctgcaatcatttcgttatgattttcatacagggaatagatttccaaatgatacctggaagtttccgggttattaacagagccgctggctaaaaaggctccccgcagatatgagcggatctgcgaatcttctgtcaacatatgactgggaacccgttcaacgattgaagcaccatcaaaaatacccagatcatccaacagttgggttgccttattttcaactcgtaaaatatataaattattctttttcagcttcattttacgacgaacactgagctcgccagtgatcccgtagaactttgaaagcaacttgtacatccgcctggcaattgccgggttttcggatgaaacgtttaacacaaagtggtgattggatattgaaagggagccattaattcgaatcaaggccattaattcagccttggcattatcccggtgaacggtcaaagaggttaattcctttttgacctcacttgcgtatgacatttaatcccctccatttcttgagtgactggcctacttatggtcgtccaatgatcgacccagtaaattgatcaattcgtcagcgacctcttgcccattgtgaaaggcaccgcgatcctttaattccagaaaatcggctgagataacccgacagcccatggcccgcaatccggcaaaatcatgtttaaccggttgtgagacttcattccatttttggtaatcaatgtattcagccggcacttctttgatgttcaccaagacggtattaataaagttcatccctaaatgacgattcaggacgcgaacatggtcagcttcagtgaagttctcggtttcacccttttgagtcatgatattacaaatatagacgatgtcggcgctggtttgtcgtaaggcttcacccacgttttcaatcattaagttgggcaaaatactggtgaacagacttccgggacccaagacaatctgatcagcgttcataatcgcatcaatcacttgatgaaccgcctctggtttatgagaatcatcggtggtctcgacccaaacgcgcttaatcaatttgccggcagcggttatttcagattcaccgctcattgtcgtgccgtcactaaattcagcgtttaattccaggggctcgttggcagccggataaatatggccatccaccttgagcatgtcactcaatatctggacggaatcaaaaataccgcctttcatctctgaaagtgccgcaataatcaaattgcccaaagcgtgaccggcaaagaattggtctgaacttcgaaatcggtattgaaacaaatccaaatacaactcaggcatctccgatagtgccaccataacgttccggatatcgccaggcggaacgacgttaatgtagtttctcaagataccagaagaaccaccatcatcggcgacggtgacgattgcagtaatgtcgacgtgtcgatttcgtaagtttttgaggataactggcagcccagttcccccaccaatcacgacaattcgcggttggtgcgtatgaagtgcgtcaagcatcagttaccctcctttgttttatggcggtcaatatcccgatgggtgatgttcaccggatactgatctttcaagtcatttgccagctgttgggcaattgccacagaacgatgttgcccgccggtacagccgatcgcaatagttaagctggccttgccttccttttggtaaccgggcagtgtgaagaccatcatatccaatagtttttgataaaattctttggccccttgggagttcatgacataatcacgaactggtttatcaaggccggttttgtaacgcattttggcatcataatatgggttgggtagaaatcggacgtccatgacaatgtcagcgtccaacgggagcccatatttgaaaccaaacgacatcacttccacgtggaaagtatgtgtttcatcagttgattcaaaattgtgaaagacttcttcacgtaaccgccggggcgccatattagtggtatcgacaaccaggtcagcagcctgtttgacgttggccaacaattcacgctcttttttaataccgtcaatgacgcgtccattgcgagcaagcggatgggcccgacgcgtttctttgtatcgggaaacgagtttttggtcagatgaatcaagaaaaatgatgtcaacattattgtcatcatttttctttaaatcgttaaacatatcgatgatttcatcgtaaaagacctgtgaccgcaaatccattactaaagcaattttattaatatcccgctccatgcggattaattctttaaactttggcagcaaggttggcggcatattatcgacgcaaaaataccccaaatcttcaaaactttgcatggcaacagtcttaccagcaccactcattccggtgatgatgacgaattggttgttaacagccataatgatttcctttcgtataacgaacttcaaccagtataacataccgggtgtgtcatgtgaatgaaagaaacacccggaggtacttgtccccgaccgaatgagcattctagcagtaatggggcaacttcagacagcaaaaaagagccacttccaatcagttcattgaaatggctcaaccaaattatttacttgctttgactgcctgcttttcagcctgcttggtcaatttcttatccctttcaaggacgggcttaaggtactgaccagtgtaactctcagggactttggccaactgttcgggagtcccggtcgcaacgaccgttcccccaccatcgccgccttccggtcccaaatcaatcagataatcggcactcttaacgacatccaagttgtgctcaatgatcaaaacggtattgccttgatcaaccagcttttgaaggacacctaataatcgccggatatcctcactatgaaggccagtggttggttcatcgagaatgtagaagttttggccattggccttcttatgcagctcagaagccaacttcattcgttgagcttccccaccagacaaagttgtggccggctggcccaaatgaacatatcccagaccaacgtctttaattgtttgcagcttgcgagaaatttttgggatggcactgaaaaaatccacggcttcgtcaacggtcatgtctaatacatcggcaatattcttgcctttgtattcaacctcgagggtctcagcattgtaccgcttgccatgacatacttcacaaggaacgtaaacgtctggcagaaagttcatttcaatcttcaagatgccgtcaccatgacaggtttcacagcgaccgcccttaacgttaaaactaaagcggccctttttgaagccccgaagtttggcatcgttggtattggcaaacaagccgcgaatgtcgtcaaacacaccggtataggtggctgggttggatcgtggtgttcgaccgattggcgtttggtcaatatcgataattttttcaatatttttgtaaccggaaatggacttgtatttacccggcttctcggaattatgattgagtttctgggcaagggcctttttcaagatatcattgaccagagtcgacttaccggagccggagacacccgtcaccacaaccatcttgccgagcggaaaatcaaccgtcaaatccttgagattgttctcagcagcaccagtaacacgaattttcttaccatttcccttgcgccgcttatctggaaccggaataaaccgcttgcccgagaggtattggccagtgatcgattccggtactttttcaatgtcggcgggtgttccgacggccattacccgaccgccttgctgaccggcacccgggccgatgtcgacgatataatcggcagcccgcatggtatcctcatcatgctcgaccacgatcagggtattgcccaaatcgcgcattttcttgagggaggcaatcagtcggtcattatcccgttgatgcagcccaattgagggctcgtcaagaatataaagaacgccagtcaaatttgaaccaatctgagttgccaagcgaattcgctgagcttctccacctgataaagtccgtgcggaacgggagagggtcaggtaatccaacccaacatttcttagaaaagtcagtcgatcagtaatttctttgataattggtttggcaatcattgtatcctgttcaccaaatgtcagcgactgaaagaagttcaactctgcagtgacatcaagagctgaaatttgggccacgttatgcttgccaaccttaacagccagtgcctggcggtttaatcgatagccgtggcaggtctgacaggttaattcggtcatatactgacttaaattgtccctggtaaagtcgctgctggtgttgtgatagcgtcggtcgacgttgttgacaaccccttcaaacgggccgtccacatcacggatgccgccaaagtcactttggaggacaaagtggaatgatttggtctttgaaccgtataacacaaagttttgctgtttcttcggcagtttgttaaatggcacgtccatgtcgatgccttgagcatcacaaacctgcttgagcatattcggataccatttggaactggcggaattccaaggtgccagagcgccctcggccagagtcttggttcgatcaggaaccaccaaatcttcatcgacttccagcttcatccccaaaccatcacagtcaggacaagcgcccagcggtgagttaaaggaaaacagccgtggttcgagttcaccgactgtgaagccgcaaattgggcaggcgtagtgttctgaaaacatcagtggatcgcgctcgcccaaaaagtcagcgacggcataaccgccactaaggcgcaaagcagcttccaatgaatctgacaatcggttattaatgccatctttgacaataattcggtcaataataatattaatgtcatggctcttatttttatcgagttccggtgcttcatcaatatcataggtttcgccatcaacctgtacccgaacaaaaccttcacgcttgatcttttcaaaaatctttttgtgttgaccttttttcccacgtacgattggtgacagaatctgcaattttgttctctcaggcagtttcatgatctggtcgatcatctggtcaactgattgactggaaatcaccgagccgtcgttgggacagattggtacccccactcgggcccacaacagtcgaaaataatcattgatttcagtgaccgttccaaccgttgatctggggttcttggaagtggttttttgatcaatcgaaattgctggactcaagccatcaattgaatcgacatccggcttatccatttgccccagaaattgacgcgcatatgatgacaaactttcaacgtatcggcgctgaccttccgcataaagtgtatcgaaggccagcgagcttttccccgagcccgataagccagtcatgacaaccagtttattttttggaattgtcacattcacattttttaagttgtgggcacgtgccccacgaatgacgattttatccattgccaatatgcataatctcctttagattacttactcgtttgaccctttaattcaataattgtatcacgcaaagtagcagcctgctcaaaatcgagctttttggcagcgtcacgcatttcttccgtcaaacgagccagcatatccttttgatccttcttactcatttgttcaaaatcactttcgacaaagtcgtccttttcgccggcatcatccgagcctttggtaatcgaaattaagttacgaattggtttgacgatggtggttggcgtaataccatgtttcttgttataagcaatttgaatggcccgtcggtgagcggtttcgtcaatggccgccttcattgaatcggtcacggtgtccgcgtacataatcacagcgccatgttcattccgggatgcacggccgatagtttggatcaacgaacgctcattacggaggaagccttccttatcagcatccaaaattgcaaccaaggaaacttcgggaacatcaattccttcccgcagcaggttaataccgaccaagacgtcaaacttacccagccgcaagtcacgaatgatttgagttcgttcaagggtcttaatatcagaatgcagatacttcactttgatccccaaatctttgagataatcagttaaatcttcagccattttcttggtcaaagtggtcacaaacacccgctcgtgcttgtcaacccgcttattgatttcaccaaccaaatcatccatttgccccataatcggtcggacgtcaattgttggatccagtaaaccggttggtcgaatgacctggttaaccacatctttggtctgatccagttcataaggccccggagtggcagacatgtagacgacctggtggacgtgctgctcaaattcgctcaatgtcagtggccggttgtccagtgcacttggcagccggaatccgtagttgaccaactgttgttttcgcgcttggtcaccattatacatcccccgaatctgcggcatcgtctggtgagattcgtcgacgactaacaagaaatcgtcagggaagaagtcaagcagcgtaaacggcggctgccccggctttctgcggtccataaaccgtgaataattctcaatgccgctcgtgtagcccatttcacgcatcatttcgatatcgtaagtagtccgttgcttcaaccgttgtgcttccagtaatttgccctctttttcaaatttggcaacctgcttgtccatctcgtctttaatctctggcagtgcaacgttcatcacgtcatcactggttaaaaagtgagtcgccgggaaaatcgcaatatgatcccgatcgccgatgacttcaccagttaaagtatccacttcgcgaatccggtcaatttcatcgccaaaaaactcaattcgaaaggcatgttcatcccaggatgccgggaaaacttcaacaacatccccatgaactcgaaaacgaccacgctgaaaatcaatgtcgttgcggtcatattgaatatcaactaattggcggagaaaatgatcccgttcaattgtctggccaacccgcaatgaaaccacgtgatttcgatattcggatggatcacccaacccaaagatcgatgaaactgaggcaaccacgatgacatcgttacgctccagtagggaactggttgccgagtggcgtaactggtcaatctcatcattaatcgacgaatccttttcaatgtaagtgtcactggatgggacataggcctccggttgataataatcataataacttacaaaatattcaacggcattgtgggggaagaactctttaaattcgccatacagctggccagctaaggttttattatgcgataagaccaaagttggcttgttgacctgggcaatcacattggaaatggtaaaagtcttcccagttccagtagccccttttaaaatttgggcttttttgccttcgttaatacctgccaccaacttcttgattgcatcaggctgatcaccagttggtttatatttggatactagatcaaattttcgatctgcttcacgttcaatcaatttgaatccccctaacctctataccaaaatgacacaacataaaagggctgcaagcaaaatcatattttgtttcagcccactattcaacgctattttaccatacgaacatactttcgccaatcattattccttggaattgtcttccttttttaaaactttgcgggtgagtcgtcttaatttatcctgagtcgtaaagttttcggccagcatatccggaatgactttcgtcaaaacatactgaacacaatgcatatcacggtactccagcatcgttgagagactctctttatacatctcagggtagacttcctcgggattacctttttgaatttcgccaaaggattcatacaacaggtcaactttatcggccaccgctaaaatacggccttccaaactatcatccttgccttccgacagacgtcttcggtaggcatcttgaaattcatccggaatttcattttggacaaagttttccgtcaatttgtcatccacatcagccagcattgaacgcagcttgggtgttgcatacttgaccggcgtcttgatgtcaccaataaaccgctcggtataatcatgattgagggctttttcatacaacccgcgccagtcgactttttcgccggcattttcctcgacgtcacctaaaaattgggcaatttcagttaccttgaatgaatgggcagcaaccgaatgctgttcgaatttaaagtagccaggtgctcgattgatcaattccaactcgtctaaactttccaaatactgatgcattcccattgataattccccgtccttttcctcgcaaaaagagccgtgaacaaaacaactgtttgtacgcggcctccctttgattaatcattaaattagtgttccgaaacactggcctttgatgtgtcagccaatgattcaacatacttgaatgcttgttgaccggcaatcccaccttcgccaacagctgttgcaatctgacgaagatccttttggcgaacgtcaccaatggcataaataccaggaattgacgtttccatctgatcgttggtttgaatccaaccatcctcatcagtaatgttcaaatctttaaaagcatcggtcattggcagcagaccaacgtaaataaagaccccagacgtctcaagaactgattcttcatttgtctggttattcactactttaacgccggtaactttgttatcatcacccaaaacttccgtgacgttggaattccaaacaaaatcaatcttgtcgttggcgaatgcccggtcttggataaccttttgggcacgcagttggtcacggcgatgaataactgtcacatgatcaacgattccagcgaggtaagaggcttcttcaatcgcagaatctccaccgccgacaacgacgacttctttgttcttgaagaaggccccatcgcagacagcgcagtacgaaacccctttgccaccgtattcgtgttctccggggatccctaatttcttatattcggaaccggttgcgatgatgaccactttggcttggatttcgtcttcgtcagtcttgacgagcttatagtcaccgtgatcttccacagcactgacggttccataaacgtattcagcaccaaagttaattgaactgtcatacatattctgagcgagatctggacccatgattgatttaaaaccaggatagttctcaatggcagctgtgttgttcatctggccgccataaattccccgatcgatcattgcaactgacaggttggctcgtgaagcatatagagccgctgtcatgccgccggggccggcaccaataatcacgacatcatattgtttagccatatggatcctccctttaattaccaaattttacttacacgttaatttactatgaaaaagtaagtctgtccagtagatacacttacttctttttgtcttcttcagttaattgggcgcccaaatctttgagataagttcgcaagccatcagaaatttctggatggcgcagaccaaagatgatgttggttttgagccagcttaatttgttcccagtatcgaatcgttcacccttaaattcatgagcaaagacccgctgtgtctggttcaaggtgtcaattgcagatgtcagttgaatttcaccagttttatccggtttggcgttttccaaaatgccgaagatttcgggcgtcaacaagtagcggccaataatcgctaaatcgctgggggccttctctggcgttggcttttcaacgaactttttaacgttgaacaagcctgggcggacctcttcagagggatcaatgaccccatatttggagatatctttgtgggcaactttcttcactgctaatgtggaagctccagtctgctgatagctttccattaattgtttggtcagtggcactttgtcctgcatcacgtcatcaccaagcatgaccacaaacggttcattgctaatgaaactgcgggcggtgtaaattgcatcacccaacccacggggatgagactgacgaatgaagtaaatattcatgtcgttggtcttgcgaatggtttcaagaatatcgttcttgtggcgctcttccaaattcatttccaactcgggattcgagtcaaagtgatcttcgattgagcgcttgcctttaccgatgacaattacaatgtctttgatgcccgcctgtttggcttcttcaacaataaattgaattgtcggtgtatcaacaatcggtagcatttcctttgggagtgccttggtttccggtaaaaatctggttcctaagccggcagccggaatgactgctttggttacttttctggtcatagtgagcttcaccttctctgagttattcaatttctgaacggccttcacgggtcatcagttggttaatcgtttctttaatatcagcatgatcatataaaacgtggtaaattgccgaagtaattggcatttcaacaccgcgcttcttggaaagttcataggcagcgcgagtcgtcgcaataccctcaatgaccattcccatattattaatgacttcatccagggaatgacccttgcctaattcgttaccagcccgccagttacgggagttggtactggtggcggttacaataatatcgccgacgcccgacaaaccgataaaggtcaatggattagccccaaacgacgttccaaggcgggaaatctcggctaacccacgggtcatcaaggcggccttggcgttgtctttataccccaatccatacaaggcgccggcgcccaaagcaataatattcttcaaagcagcgccaatttcgacgccaatgacatcgtcactggtataaacacggaaatagttgttcatgaacaaaccttgaatttcagtagcagcttggtcactatcactggcaacggtgaccaaagtaatgtcatgggtcacgacatcttcagcctggctggggccggatagaactgaaattgatttgcggttctgaggatcaatttcttgagccagaacttgagataatcttaagtaagttttttcttcaattccctttgaagcatggatgatattcactttttgattccggtcggccaaaatttctgcaacttgtttggcaactgaacgggttacctgggtgggaaccacgaataagatgtaatcaacaccatcgatggcgtccttcaaatcattggtagccaccagtgaatctgaaaacgtgaaattcttgatgtattttgtgttggtatgctgttcgttaagttccttaacttgtgtcgggttatacgaccataatttgacgtctgacccattctcgtccaataaactggcaagaacactcccccaagaacctgcaccaagcactgcaacttttttagccatgataaatctcctttattagtaaatgatcaattaactgttaatttggaaccctctaaataccaaggattatgtggctggcgtaatcgacgataaatgatgattccaattgcaccaacaaataaaatgattgaaagaatctgcgatacccgaaggccgccaagcatcaaactgtcagtccgcatgccttcgacaaagaatctgccaaaagaataccacatgacataggttaaaaagacttcgccacgtttaaacagatgggaattgtgccgcaaggttatcagcaccaaaaaacctaagaaactccacagcgactcgtagagaaaggtcggctgccgatacgcgccgctaatgtacatctgggtaatgatgaaatgtggcagacgaagcccagtcagaaagctcaaagatgttacctgaccgaaggcctcctgattcataaaattgccccaacggccgattgattgtgccaaaataactgttggtgcggcaacatccaacatcagccaaactggaatgaagcggtggcggcaaaataggatcaccacaatcatcgcaccaattaaagaaccataaatggcaataccaccgtcccagattttgatgatttcaccagggttatctttgtaataagaccactggaagatgacgtaatacaatcgcgcacaaattagcgcagcgggcaaggcccacaaaatcatatcgtaaatatcgtcggctttaatcccacgtttatcgccttcgcggaccgccaaccaaaccgccagaatcacgccactggcaatgataataccataccagtggacttcaattggacccaggttaaaggcgatcgggttgagggctaagctcaataaatttgtcaaaataacgatctcctattttttatctgaatctttgtcacgaccatcgatgagatctttatttttctcctcaagatgttcctgttcttctttatgcttttcgtcgtttttgctgttgaccttgattaaattattcaagttacggtcaaaggtttcagtcgcgtcatagcccatgctttgggcacggaagttcatggcagcggcttcaatgatgatcgccaaattccggccggttcgaacgggaatcgtgattttcggcacatcgacatcaaaaatatggacattctgagtcccgttgcccagacgatcaaacttggcttccttggtgtagttggccagatgaataattaaggcgactttcgtctgactgcggacagcaccggcgccaaataaagtcatcacatcgataatcccaattccccgaatttccagtaagtgacggagaatcgcaggggcagtccccatcaaggtttgttcatcttgttggtaaacctctacccgatcgtcggcaatcagccggtggccacgtttaaccagttccaacgccgtttcactcttgccgattccactgtcaccggtaatcaggattcccaatccataaacatcgaccaaaactccgtgaagcgacttgcgttctgctaatttatcgtcgaggtaattagtcatgttactgagaactcgagacgtcgtcaatttggaaccgaggacgggaaggtgctgttcttttgcggcctccagcaattcttccggcggatccagttgggtggacaccacgaacgccggggtctgtggttgacacatctgctgcatcacatcgaggagctcttcatgagacatccccttggaatatgaaatttcagtaatgcccaacagctgaattcgtttgacagggtaataattaaagaacccggttagctctaggcccggtctggaaatatcagcagtggaaatggtcctttcttcaaggtattccttcccataatagacatccagcctggcgtttttaaccaaatcagcaaccgttacactttcagtcaagaacatccctcctcaattaatcaatataattttatcactttgagcctgacaagtccttatggcttgcggaaatattcagcaatgatccagctaaccgcagacatcagaatggccacgccaattgcgacccaaaatgatgagaatctgaaattagccccaacaatcgtcgccgtcagttcaagcatcaacccattaatgacaaacgtgaataatcccagtgttaaaaggttaatcggcaaagacaagatcgtaatgatcggtcggaccaaccagttcaaaacggctaaaaccaccgccgctacaaaagcaattcccacgctggcaacgtagaagttggcagggaaaaagccactgatcgcaacaaacaggatcgtatcgaccaatacattggttaaaaatctcaattattgaccccttttcttgtcatcatgaacgtctttttcttcgacgttatgaatgacttttctggatttgtcgttagaagttccgccggataaagtggttttgaattggtcaaaggccgatccactaccaggtgtatcactgggaattgcgaacatcataatgatatacccaataattgcgaccacgttgatcccgggcgtaaacgccaagaccacatacaagattcgaaccaagacagcgttccagtccagatactcggaaattccgccaagcacgccggaaatcacccgattggtactggaacgccgtaattttttatgactattcatcctcatgcctccacaataaaacttctagcttaagattatctaaaaaaggcactgcaatcaagtatgcagtgcaaaatatcaaccattcttaatttaattcaataatttttccggttgccagataaaccgtccactcacaaatattcgtgctgtaatcactcacccggcctaaatctttggcaacgtttagataaataatcgctgaactgacaatctctggatccttggccatcgcttggtaactgggagaagcaatgtcgttatagagctggtcaatttttttatcgtactgttgcgcggtccgcttggctttgtcctgatcggcatcaccatatgactcaattgaatcagcatactgctcgctgacttcttgagacattgtagcaataatttcttccactgaagcgatccgctgcttgcctttaatatcaatcaccgatcgagcaacgtttcgggcatggtcaccggcgcgttccaaatcagtgacggcttttaaaattccgaccacttcccggaggtcccccgtgaccggctgatacagcgcaatcatttcaaatgaccgcttttcaatatgaatctggaggtgattaatctcgtggtcgttggtgatcaccgtttccgccttttgaatatcatggtcgacaaacgactgcccggcgttggtcacggcttcaccaaccagtgcccccaatttcataaaatccgcctttaacgtaataatctcttcatcaaaaactttccccataagcttctctcctatccgaatcgtccgctaacgtaatcctccgtttgtttttcctcaggattcacgaacatcttagttgtgtcatcatattcaaccactctgccttccataaagaacgctgtcttatcagaaattcgggaagcctgctgcaggttgtgagtaacgattattattgtataatcttttttcaactcaagcaaagtattttcaatcttggcactggaaatcgggtccaatgcactggtcggctcatccatcaaaataaccgatggcgaagtggcaagcacccgggcgatacaaattcgctgttgctgcccgccggaaaacgacagggcgttatcgtacagattgtctttgacttcatcccaaacagccgcctgcttcaaacttttttcaacaatttcatctaatttttgtttgtcacgaagtcccgcgatccgcaaaccataggtgatattatcatagactgaaaatggaaacgggttgggctgttgaaagaccatcccaatcgactttctcaattctaccagatttgtttgcggagaataaatattttctccgtgaaattgaaccgctccggtaattgtcacgccatcgatcatatcattcatgcgatttaagcagcgcagaaatgttgacttcccgcagcctgatgggccgatcagcgcagaaatttggttaggcaggaaatctaaatggattccgtaaagtgcctgaaaatcatcatagaataaatccaaattgtctgctgaaataattggtgttgccatgattgttcctcctaaccaaagtttcctgatacatagtcgtctgtcatctgtactttcggccgggtgaagacctttctggttttgttgtactcaatggcctcacccatgttgaagaagaccgtgtagtcactcagacgggctgcctgctgcatgttgtgggtcacaatgataattgtataatcctttttaagttcacgtaaagtcgcttccagttgttgggttgaaaccgggtccaaggcactggccggttcgtccaacagtaacacatccggttgaactgccaaggctctggcaatacaaacccgttgtgcctgcccaccggataaggaaagggcacttttattcaaactgtctttgacctgatcccagacagcggcttgttttaaagtggtttccaccacttgatccaaggttttcttatcatgaattccccgtcgctggagcgcgaaagtcacgttgtcatagattgatttggcgaatggattcggtcgttgaaaaaccatcccgattcggcgccggacctcataaacatcgatcttgggctgattaatgttgacgccttgataaagaatctcacctttcacagtagcgacgccatcattcatccgattaagggcccgtaaaaaggttgatttacccgatccggaaggtccaatcaaggccgtaatggtattttttttaaacttcaaatccgcgttgtgcattgctaaagttttgccgtaataaatttccaaatctttggtctgcatcgtaatgtcattttcttcgggattaaaatcataaataaaccgcttgggtttgttgtttaattcagttgtgttttgcattttcagccacctactttactgaagtcattcgttcaaataccttccggccaatccatctggccgacaaattaaagattaaaatcgccaggaccaggacagccgctgaaccggaggaaacctgtgtcaaatcaggcatgattccttctgagttgattttccaaatgtgaacggccaatgtttcagccggccgcagcggcgacaatgggctatcaatgttgaaggggttccaatcggcaaaattcaacgctggggcgctttgaccggcggtatagatcaaggcagccgcctcaccaaaaacccgtcccgaacaaagaatgatcccactgatgattccaggcagtgaagcgggaacgacaatgtgaataatcgtctcatatttggaaagtcccaagcccaaaccgccttggcgctggtcatcggaaacgttggaaagtgaatcttcaatatttctggttaacagtggtaagttaaaaatcgttaaagtcaacgcacctgaaatgattgagaaaccatagttgaactgaacgacaaacaataagaaaccaaacagtccaaccaccacagaaggcaaggaactcaaaatttcaattgaagtcttgatcgtagcggtaaaccagttatctttggcgtattcgttgaggtaaatcgccgccccaagtgcaattggcagagaaatcaacattgctaacaccaagaggtaaaatgagttaaatagctgaatgccaattccgccgccggcattaaacgctttggccggggacgttaagaaatgccaactgatattgggcagtccggtgataaaaatatagccaatcagaaaggctaagatgaccaccacaaagccagcaacggcttttaaacaggcaatggcaaatcggctttgcttttgtgttcgattcatttcttaaacgcccctttccgaccgatcatgtgaactaataaattaaagaagagcgacatgactaacagaaccagtgctagtgaccagagggcgtcattttgaagcgatcccatgacggtgttccccatgccggcggttagaacagaggttaaagtggaagccggtgacgttaaattttgcggcatcaaagctgcatttccaatcaccatttgaacggctaaggcttcaccaaaggctctggccattccaaaaaccacggcagtcaaaatccctggtgtggcggctctcaagacgactttccaaatggtctgccacttggtagcacccaaagccagtgaggcttgacgataaaacttgggaacgcccctgagggaatcgacagtcattgatacaatggttggtaaaatcatcacgaacaggacaaaggtcccggataggataccaaacccactgccgccaaacgtatttcgaacgaaaggaacgactactgagagcccaataaagccatagacaaccgagggaattccgaccagtaattcggttaccggctgaagaattttagctccccgtttaggagaaatctcggtcatatacaccgcagtcccgatggcgaacggcgtcgacagtaaagcagccagaatcgtcacaagaaaagagccgacaatcatgggcaacgcgccgacggcttggtgcccgttgggagtcttggtaccaggattccacaacgtgccggtaaagaagtctttgacagaaatgccgtctttgaagaaggtcgccaatcccttgctggcaacgaagacaataatgccaagcacgatcgccataatcagcagcagcgccgaaagactgagcaggtgcccaaatcgttcgtaacgggccgttttggattttttcatcagttgtttggctaatttttcattttgcacgattattcccccgatccttttgtaattttgccctgccaggttctctggtaatgcatatctttcacagagatgtaacctagtttgttaaagagggtcgtttgaatatgatcgtttttcaagtaagttaagaattttttagtcaatccggtgggtttcccacgggtgtaaatgtgttcataggaccagattttccacttattgtccatcacgttttgttccgtgggcttaataccatcaacgcttaatggatgaatgctcttattgaagtagccaaatgagacgtagctgatagcccccggcgttgatgagacaatctggcggacagttcctgaagaatcctgctcctgggcggtggcactttcatggcctttaagaccatattgttcaaaggttacccgggttccgctcccctgagaccggttgatcaaagtaatcggcaggtcgggtccgccaagctgtttccaattggtgtatttcccagtaaaaattgcaatcaactgggcggtgctcaagttgtcaatcccaacgcggtcattggtaatcggagcgactcccacaacagcaattttgtgatcgaccaagccggcgggattaatgcccgccttttcctcagcaaacaaatccgaatttcccatctgaacggcaccggactcgatttgactcagcccggttccagatccaccaccctgcacattaatgaaaatgccagcatgatcagcagaatattgttcgctggccgcctcaaccagtggctggagcgcagttgaaccaacagcggtgattgattgctgattggttgaagtcttgctgcgggcattgtaagcaccaattccggcaacaattaccaccacacacagtaacagtttaacgatcgtccgttttcgcatctcaattcctccttgaatcttcaattaccattgtattaaaccaatgtaaatatttgaccggacaaatgtaaatgttttgtaaatagataaccgggtgttggtaattaatggctgaagaaacgcaaaaaagccggagatgctcccggcttgattgatttgaaaatgtaaatatttggttgaaattcagcaaacatcagtctgtttgtgtgttgggctggttacgatctttgacaatcggaaagtttacagtaaaagtggagccaacgccccgctgacttttaacatcaatcgtgccgccaaccgcatcgaccatttccttgacgattgaaagacctaagccggtcccactgaccttctgcttggttcgggaatcgtctgcgcgatagaagcgttcaaataatctggaaatgtctttttgggcaatcccaattccggtatcggaaacgtggagctgccaataactgtcgttgtcactataggtaatgttaacctcaccatttgggcgattatatttaaccgcgttgctgaccagattgcgtaaaatccgcgtgagcgtggtggtgtcggcaatgacttcaacgtgttccgggacttgattatgaattgaaacgtggttaccttggatcattgattgatatgaagcaagctccgcatcaatgaaatcatgtaaagctaatggtttgtaatgataattagtaccgttttgaatatgggaaatcgtcagtatgtcttgaaccagcgaggccagctgatcactttgttgatcaataattttcagaaactctaccaaactcttcttatcgtccatcgccccacccaacagagttttggtaaatccggagatggcagtaatcggcgtcttgagttcgtgactggcatttcgcaaaaagtcaatctgcatctgtttgacgttaataatatctgaaatgtcatacataatcaccaggatgtgaaaatcgttttcgagttgattgaacaccacgctggtgtcccaggtaacagatgtcgccccgacgctttgaatctcttcttgctgagacttgtgactgtcataaacattttcaattaaagacagcaattgataattgcggatgtcttgggtatagggatgaacctgagtcaaaatatctcgtcccagcatgacggacattttatggttggcgaaaatcacatcgtgagttgaatcaattaccatcaccccgactggaaggctggaaagaatcgtaattagttcggcgttactgtttcgaatactctttccttcgtcctgctgcctgctttgaagttcgttgagctggtcggcaacgcctttgagtgggttgtcgggttcaacaaaaagcggcaccgccggctgatgatgaacaatattttcggtcattatttggagttgtttgagcagcttatcatgctggcggtattgaatgatgagaataatcccggcaattgcatcgaccaaggccaataaaagggccaggtcagcccagcccaaattgccgctcgtaaaaccataaaaaagcacggccagtgtggcaatgcttaagattacaacggttaaaatttgtttataaattttactcagcgtcatcatcccccgtggagaactcataaccaaatccacgaactgttcgcagatatttcggccgttttggatccggttcaatcttttcacgaagatgggcaatttgaatatcgaccatccggctttgacctgagtagtcaaacccccaaacaccctggagtaattggtcacgactaagcacttgattttcgtgactgaccaagtactgcatcaattcaaattcttttggtgttaactttaagtttttcgaatcggcactcacgcggtattttttgtggtcaatggtaaacggcccagtggtttcgacattttcggctgatttggcagctggcgtttcggatgccgcagcactcttttcataccgacgaagcaccgcgttaatccgcgcaatcacctctcgcggactaaatggcttgggaatatagtcgtcagcacccatctcgaggccaaagaccttatcaaattcggtatctttggcagttaataaaatcaccggtgtgtcgtttcggtccatccgcagctgcttgaggacttgttccccactcatctgcggcaacatcaaatccaaaagtacgatgtcaaattggccattttcagccattgaaagcgcatcgactccgttagtagcactctgaacttcaaaattggcttgcttcaagttatattccaataaagtaacaattgctggttcgtcgtcaactacaagcacttttttcacgatagccctcctaatgactaagctgtgtatatgttttgaccccaatttcatgaggtgaattcttgaagatcgccgattcggtcatcttcaactgatcgtttcgatcgcgaactttaaaccgacaataagttgagttggtgctgagcgcgcgataaaaagaatcttcatcagtcaccgaaatgccattgacctcaaggatcacatcgccaactttgagatccatcttggcggctggggtttccggttgaatgccaattacccggacaccatccatcacttcactatattcaaacgactgctgattgtcacggtgtttggcaagcccaagaatcaaatagtagcccaacaacaggataaccacggcgggtaaaatgaggtgcggtacgaagtagccggcaatcgccaggcaaacaccaatccccgccaataagtaaataccgtgactcattattttaaataaggccctgggaacacttcttttgacggtaaatttaagtccaatcaggattggcaccaataacaacgcatagaaatgattgtgtacttgaaatagcggcatcattggtaagctggtatggatccaatctccgggaacaaacagcaggaacggaaaaatcgtcaattcgttaaatttataaacggccgttttattgtttcgttggttgcgcaccaaggtcggtgaatcaaatcgaccaccgttaacgttcaagaaaacggcgtttgccaagataatgaccacaaataaaatcaacaaattgagcggggccacagttgttgagttgattcccagtccttcaaaccaatgaagcagtggtcgcaattccgatatatttggcaatcccagcgccaacaaactggcgataccggcaacagtcaccgacagcagccaccaatgaatcagcgtgagtgaaatcagcagtaagccttcataaatgatcaaccattccagtgaaatgcttaaaaagccacctaaaacgacggaggccagtatcccaaagatcagccccattctgacaaaatgtcgaccttcataaaaatcctcataaatcgcggagttaaaaatcccccgctctttcttcagccgcctcgtatgaattaaataactgcggataaccccgatccacaaggcgggttgcaatccataaaaaccacaagcaatcaaaaatttcattatgtcttcctcaccaataattataaggctagtatatcatttattgacagctgatttaagctgatttgaaatccgaaagactaatcaagatggtggcttaaccggcagttgctgcctttgggtgcttggtagggttctccaatcatcctgtcgttgataaaaaaaggcccttaacgcaatgtggcgtcaagaaccttatcgtatgattcgcaccgggctaaagcaaacgcggctttaataaccgattagtctggattcttttgacttaattgccattgtagataggcgttgatgaacggatccaaatcaccatccatcacgccgttgacattggcagtttcgtaattggttcggtgatctttgaccatcgaatatgggtgaaagacgtaggaacgaatttgagatccccagccgatgtctttttgttcaccctcaattttggccttttcttcggcctttttctcttcttcaagttcatacaattttgacttcaacatgttcattgccgtttgccggttttgaagttgtgatcgttgcgcctgactggcagccacgattccagtgggtaaatgggtgattcgaacagcggaggaagtcttgttaatgtgttgcccaccagcaccgctggatcgataaacatcaatccgtaaatcatccgggttaatatcgattgagacgtcatcatttaattcaggcatcacatcaacggatgcaaatgacgtgtgtcgacgaccagctgaatcaaatggcgacagcctgaccaatcgatgaatccccttttcggaccgtaaataaccatagacattttcaccgctgattaatagtgaaacactgttcagaccggcaacgtcaccgacctgataatccaaggtctgcacggtgaacccatgggcttctgcccaacgggtatacattcgcagcagcatcgaaccccagtcctgggcttcggttccgccggctccaggatggatttccaaaatggcattattatgatcatatttgccgttaagcaacagattcaaccggtagcggtccagtttagttttaagctgcttttcatcagtctcaaattctccctccatcccggaatgagcatcctcttcgatcaattccaaagtaacttttagatcatcgagtttatttttgaggccgacgaaattgtcgcgcttggtttttaactgattggtttgatcaatcaatttctgagcggcttcttggtcatcccaaaagcctggctcggccatcttcgactcattaatcgcgatgctttcacttaaggcatcaaggtcaaagtgacctcccaaaaccatcgatggctttttgcatttcagcgatttgtttttttgcttcactcaattcaaatgacatattactctcctctaattttgttccaattcaaagaaagaatccaaacaatcgtcattgccggattctttccaatacatattaacgttgcatgttttgacgaatttcagccttcatgaacagacgggttgcgtcatattcgatatcggcaatcatttcttcaaacatcttgtaaccttctcgctgatattcaaccagtggattttgttgaccataaccacgaagaccaattgattgacgtaattgatccatgatgtcaatgtgatcagtccaatgggaatcgacaactcgcaagataacaaccttttcgaattcaagcatttgcgattcatcgtagagttgttcttgcttttctttgtattctttgtttgccagacccatgagcatactcttaatttcgtcagctgatttgccttggaaatcttctagagaaatttggtctgggctgaccatcgcactgatggcgaagtccaagatggtttgcagatcccaatcttctttttccccttgagtatgcaaatcaacaattcgattgatggtccgttcgatcatcggcatgatgacccacttcaaatctttttgctcatcaatgacttcacgacgctcaccgtaaatcacttcacgctgttgtctcataacatcatcgtattgcaaaacgttcttccgtgaatcgtagttgttaccttcaacccgcttttgagctgattcaacttgcttggtgatcattcttgaacgaataaccgcgtcttcaccttcaacattcaaatgctccaggaagtttttgatcttttcagaaccgaaacgacgcatcaagtcatcttcaagtgacaaatagaactgtgacaaaccaggatcaccctgacgtcctgaacggccacgcagctgattatcaatccgtcgtgactcatggcgttcagtcccgataacagctaagccgccaagttcaacaactccgggtcctaatttgatatcggttccacgaccagccatgttggtggcaattgtaacggcgccccgttggccggcattggcaacgatttcagcttccttggcgtggtttttggcattcaataccacgtggggaatcttttcttcatcaagtcgttgtgacaagtattcagaagtttcaacagcaacagtaccaaccaacattggctgaccctttttgtgaagctccttgatcttgttgacaacggcctcaaatttggcttccaaagttggatacaaaacatctggatgatcaacccggacaaccggtttgttggttggaaccgaaataacttccatgttatagatctcacggaattcttcagcttcagtcttggcagtaccagtcattccggcgagcttcttatacatccggaagaggttttggtaagtaatggtagccattgtcttactttcctcgttgatcgtgacgccttcttttgcttcaagggcttggtgaagaccatctgagaatcgacggccttccatgatccgtccggtaaaggaatcaacaatcttgacctcatcatcttgaaccacgtaatccttatcacgaagcatgataaagttggcccgtaaagcctggtccaaatggtgggtcaaggcagtattgtcggtgtcataaagattctttaagttgaagtacttctcagccttttcgattccctgatcggtcaatgaaacagtcttggtttccagatcaagcttgaaatcatcgccttcgtgcaacgtcttggcaaatctgtcagtccgttggtaaaggtcggaagtgccgcttgattgaccagaaataatcaatggtgttcgggcttcatcaattaaaattgaatcaacctcatcgacaatcgcgaagttcaaaggacgttgaaccatttgttccttataagcaaccatgttatcacgcagataatcgaaaccgatttccccgttggttgagtaggtgatatcggcagcgtaggcttcccgcttctcatcggcatccttttcagtggtattaacaccaactgtcaggccgagccaattatataactcgcccatttcagtggcatcacgctgggaaaggtattcgttaacagtaaccacgtgaaccccttcgcctgcaagtgcatttaaataaaccggcatggtggcagttaaagtcttaccttcaccagttttcatttctgcaatatttccttcatgaagaacaattccacccataatttggacgtggaatgggtacaaacctaagacacgctttgcgccttcacgggcaacggcaaatgcttccggaagcaaatcatcgagtgtttcgccattttgatagcgtttcttaaatgccggtgtcttggcttgtaattcttcatcactgagttgacgatactcttcagcatacgaaccaactttatcggcaattttactgagccgcttttgttcgcgtgtatcactttcaacccatgttcttaaaatattagccattagtaaattcccttctaaaataaaatactgatcaaattgttcttagtatttgtggactacatacttatttagtgtaacattttaggccgcccatgaaaacacaaaaaacaatgcatcagcggcatttaaccatgataatacattttgaatagatatgaaaggttaaacgatcagattggttcacaaatgtttccggaaacgaaaaagaatggggataaattaagctgcaatttatccccattcttttgacggtgcataatacgcatgcccgttaattgattaacttaattattcttcgccggtctcaatcaagccataacggccatcattacgacggtagacgatgttgatgcctgaagtttctgcatcttcatagatgaagaaatcatgccccagcatgtccatttgaagaatggcttcctcgttatccatcggctttaaagccagttgcttggtacgaacaacctggaatttggattcgtcatcagaatctgactcgctggcagaagtatctgcagcgggtgcaaattcaagattcttaaatcctttttcacgagacttgcggttaaccttggtcttgtacttacgaatttgacgttcgagtttgtctgtcaccagatcaacacttgcgtacaaatcgttggacatttcttcggctctcaaagttaagtatggcaaaggaatggttacctcaacttttgcttgcttatctggataaacctttaaattgacatgagcagtatttttcatgtccttttcaaagtatttctccagtttactgatccgtttttcaacataatcccggatcgcctgggttacctcaatgttttcaccacgaatgttaaaaattagcatagcgttctctcccttcaccattaaaggcttaatggtccactaatgaaatcactttcattactggctacaactttagtataattgaaagttcgaattttaacaatcattgggtctggatttctttatcgagcaagggtaaatcctttcacggaagctgccccggcttgttggatcaaagcggccgcatgcctaatggttgtcccggttgtatacacatcgtcaaccaataaaacggcctgatttttaacttgatttttttgtgattcaatcatttcaaacggttgatcaagcaataaacggccctgacggtttttcgccgactggcggacggccttcttgtcgaatctgacgcttaataggttcaaatagcggtcattttccaacagcccggtgacctgattaaagccccgagtggccatggtgtccttccccaccgggattggcacaatgatcgcagattgcttcttcaactgctcgtgaatttgatcggaaaaaaccttccgtaatcggtaatccccggcaaacttgtatcgtttcatgtaatctttcattgccggattatattcgtacatcgccgagttaataaatttgaattggccgtccttctcccagcgcagacaatcgtagcagggatcgctcatatcagttgttcgccgtcgaccgcagctggaacaagttggtagcaggttaagcgctgaaaatgtgggggaacacgcctcacagatcgcccgtttctgcagtggggttaaccgaatcaagtctgcaagtgggatttcctgtcttagtctggagccacacaataaacaggctttcataattgagccgcctttcgattcatcagcttaatctggcggtcacaggatttgatgttggccgttttaaattcacaataaaagaggacttgtcctgtcggccgatcactatttcgacccacccgaccagcgatttggacgagtgcagccgccgaaaaaatttcactgtcagcctttaataccaagacgtcaatgcctgggaaggtcacgccccgctccaaaatcgtcgttgtgatcaggaaatccagttgttgactgcgcattaacgctactttctcaattcgctcgggatcagcagaatacaccgttttgaatttcgctgctatcccggcagccttgatggcagctgccgcttgactcaagtctttaatgtggggaacgaacagtaagaatcgctgcttttctgttaccaggtcagccaccatccgcaagattttttgaggcagtttgccagcttgaagctgctcgttaagacttttgacccgaatcgccgagatttctggtaaataatgtccatgatatctgattggtaaataactgaccgacaactgttttctagaaattgctttaaaaagtgcctgatcgggggtcgccgttaaatacagcgttgccccagcgggtttaatcgcattttgaacaccaaaatgaagcattgggttaccagaatatgggaagacatccacctcgtcaataatcaggacgtcaaatgcatggtaaaatcgtaacagttggtgggtcgtacaaacggtaatctgactgtactggtaccgctgctcactcttgccatggagtaacacgattgaaacttgattgaacgcggcttgaattcgtgggaacagttcgatgcatacgtccacccgcggcgaagcaatcccgactcgcaatccatttgaaattgcccagctaatccctttaaacagcatttccgtcttgccagcccccgttactgcccacaacaagtgacgctggcgttgttgaaacacttcaatcactttgtcggcacactcattttgtaattgggtcagctgcccggaccaggataatggatccggattctcagtaaaatgatttggctcttccaaataagccagtggcgacaaggtatccacccgccccatttgaatacaaatgtagcaataaaagtggtgattaggtaaactggcaagggaacggcgcaattttgacccgcagcgaccacatttcaatccatggtcgtcactgatggccggacgtaagcgaatgtccggtgaattttgcagtgtcgcggccagatcacgctgtggcatttggcggccatacaactctgatagatcattaatcatagatcatcacctcaatcactaattacgtaaataatggaggaatcctttttgaaaaatgaatcactgacaattaaatcaaacggtacccatgaaatcgaaattaaaaaatcccgttttctctgcacgatggcacgaattgataacgagaaccaggcaaaaaaaatcattgatcaagtgactaaagacaatccaaaagccaaccacaattgctacgcctacatgttgggtgacgatgaccatattcaacgcgaaagcgacaatggcgagccatccggaaccgccggggtccccatcttggaagtcctcaaaatgaatgagttacataacgttttagcagtggtgacccgatatttcggcggcattaagcttggcgccggcggtttaattcgggcttatagcaacgcgacatcgacaacgattgattcgcttgggatcgtcaaattggtcagcaaacaagaattaaatttgttaattgattacaatcaatttgatcgattaaaatacttcttggaaaacgccgctataccagttgaagaaaccaattataccgacaaaattgaactagtgattgcagttagcgatagtgaatttaaccctctcatcacacaaatcaccaacttattgagtgatcaatttacctacaagaaagggcaatacaaaattttcgaggtaccctattctcgtgaagaccgtcaaaaagatgaacgaaaataacatctggttaattttatcaccttcaaatttgtcaaacatacctcatgaaacgtggtcacttcgctgatcatgtttttttatttacagcaataggataacggtgttatcttgggttaagcaggggatgatacagatcgcaggaaaaacaaaccacacgaaagaaacgattatctcacaaacaattcgaatgattaatgaacatgggtatcaaaacatttctcttcgaaagcttcttgggactctcgacttaaccacaggagccttttacaagcatttctccagtaaggaagacctgtttaagcatgtcactgtcacaatttccaaaaaattctttgtacaggcatccaatcaccttgccaaaggaaacaaggaggatgcattacaaacgttgattgatttaggtgaattcgttattcatcaaatcgagacagttccaaatttaatggattttttattgtttaatcctggaattgtcaagatatattcacaaaattttgatgataactcatttagctttttggttttaacacatgaaatcattcataatcttgccacacagcattccttaagagaaccggaaaatgacatttttatcaaagtctgggcgtttatacaaggttatggttcattgattgcgaacggtgccattacttaccgtcgagagttcctcgctttagcagcaactcaactgattggagaagactaacatgaatacaactttaattatttactgtcatccctataaaagaagctttaatcacgcagttctagaagctgtcatttcaacacttgcttcaaaaggaagaagttggaaactaattgatcttcatcaagcacaattcaatcctacctatgacgtggaagaattgcgtctattccatcaagggaagtctcatgatcaacagacaattgagtatctcgatgaccttcgaagagctaatacagtgatcttcatcacgccggtttggtggaacagcattcccggaatgttgaagggattcgttgataaagtcatgaaagaaggggcaggattgtcccacaccgttactaaattcggtgttcatggtgagctcgggaatatcaaacatggctacgttttaacaacttccacatccccaacgttttatttaagatttttttcgggcaatggtattcaaaaaatttttatccaccaaacactccggcaacttggcattagtcattgtaagtggattaattttggaaatatttccaattcaaccctctcaagtcgaaaaaaatacttacaacaactccgctcatacaacttttcatgattatatcaaaaaccgcctgacaaacgtcagacggctttttaatgcgctaatgattatttttactggtcgtatctttaaccaatttcttaattccgttcaacagcggctgtcgatcttctccaaccaggccaatcgtttccacaaacaactcaagaccaatcaaaacggcaatcgtcagcagaatcgatccccacaaggttgaaatcggataaagcagtgagataaacgaaaaaatcagggcaattccatagatcaccaacaccgtttgccgatgggtcaaaccaatttgcatcaaacggtgatgtaaatgtcgcttatcggcatgcgtaatcggttccttatttaacaaccggcggaaaatggcaaatacggtatcggtaatcggcacacccaggatcatcactgggattagcagcgtgatgaaagtggcgttctttaatccaaacaacgaaaagaccgacatcataaacccaataaacaacgcaccggtatcgcccaaataaattctggccgggaaaaagttataaggcaaaaagccaatgcaagcggccaccagggtaaaaatcatgatggcgacgaaaatattaccgacgttcaagaagaacatggcggtaattcccatggtggttagggcaataattgcaaccccagtggccaagccgtccaatccatcaatcaagttaaccgcgttggtaattgccaaaatccaaatccaagtcactggcaagctcagccaaccaaggtggattgtgataaacggtaaggtaatggtggtcattttaacaccggctgtaaagtaaacccacagcgcggcaattgaaatccccaaaactttttgccggggctttaagacgaaaatatcatctattatcccagtgagaataatgatgacttccccgccatacaccccccacaaaattttggttgggaactgatcccgcaataaaatcatggtcgtaaaggtgtaggcaataaaaattgccaacccaccaatcgttggcattggaattttattaacccgccgtttgtttggccggtcctctgccccaacagcaaaagcaagtttccgaataaatggggttaagactgcagaaataatcatggtagcaaataaagacacaatgatctcgaatttcaaaattgtaacctcacttatttccttccaaatcaatattaattcaattatacaaatgacaattcataaaaacaaggtatgtctgactcacaaagtaaaggagcttactcaaataattaatacggaccaattgtgtgaattttcacatttttaaattttgctaacgttttcaattgtcatatttcacaaaaacatttatactagagattgtaagacaacaggttcaattattttatatttcacaaacggaaggagtttttatcatggctgacaaaacaaatactacacaagccgagacgaaagatgcgcccattcttattcaaatgggtatcttcgccggggtattgtttgtttccagtttaatttcagcatggttggtagcagtcgcaccaaagttccctgttccaaccccagttcttggtttaattattctttatctcctattaactttccacatcgtcaaagttgaatgggttgataaatttgctacatttatgatcggaatgatcgcatttctatttgtaccttcaggaattcaattgaccgcatctcttgatatcatgaaggctcaaggtgtacaacttattgttgctattattatttcaacggttgtcttacttgttgttgttgcttacaccacatcattctttatctggatcagaaagaccgttttccatggcgatattacagttagtgaagacgtcgagaaaaagtaattaaaggggtgaatataaatgtctgctacacaaacaactattattgcgtatttagggacaccaatttttggtatctgcttgtcactgttggttttcttgtttggtcaatggctattcaagattggtaaaggattcttcttattccaacctctgtttgttggaatggtacttggaatcttcatcctctggttgatggctaagatgttcggtgttgacgttacttggttctacaccaacgcttacaaaccaggtggagatatcatcttctggttcttgaacccagcaaccatcgcgtttgccgttcctctgtacaaacgtaacgatattgttaaacgattctggttagagattctgctatcattaattattggtttgttcatctcactgttcatcatctactatgtatcaaagctcatcggcttgaacaacaacggaatcgcttcaatgcttccacaagctgctactaccgctattgcaatgcctatttctggtgctatcggaggtactcctgccgttactgctatggcatgtatcttgaacgccgtcttgatttacgctttggcaacatggctcatcaagatattccacttgactgaaccgattggtcaaggtcttggattaggtactgccggacatactgttggttcagcaaaggccattcagttaagttctgtatctggtgcgatggctgccatcgcggttgttatcatttcaatcgttgttgacatcgttgttccaacatttgccaacttcatgggaatcgctcactaattccttgcgagatcaaaagatcgtccatttgggcggtctttttgtttacatatttttcccaaagctaagcgactactcaaaccaaattatcccttccctacgcacccttcgtctcttccaagataattgcccacaatcctggtaaaaccggtacgaggcggttaaaaacacgctaaaacaggccatccgctattgcttaacggatggcctgtatcgtttcatttaactactcacgcagatggtagttataagtggaaataataatattttgtcgtgaatttaaaattgctcttaatctcaaactagtctggttatgcaggacattttcccaacgatgtcttggtacaaattgcggtaccaggactgtggtcgaatagtttcgatcagctgcccgcttggcaatgacatcacagaaacgtaaggttggttgggcaattgaccgataggatgaatgaatatcaacgaatcggacatccgggaaatcttttttaaactgctcagacgtcttgtgttccttctcagggttggagtcaaaagaaacgtgcattgcgatgacataatcaccaatcgattgggcataactgatagcattggcagtcacccgagtgaccccgcttaccaggacaatgacagtcgagccgtcaaagtgatgagttgtcgcaatttcagtattctcttcaaccacccgcagctgttcggcaacccgcttgtaatgatgattgatcttgtagaaaatcctcaaaagaatcggcataacaatcaaataaggccaaacatttggaaatcttagtaagaacaggcaggtaaccaacgtcagtgaaataaaggcgccgacgaagttgataactgacttcagctgccaattcttaccccgatttctccgccaatggataatcattccggactgtgacagcgtaaatggaatgaacacacctacggcatacaatggaatcagtgaattggtccggccaccaaaaatttgaattaagacaattgcaccaacggctaaggaaataatgccgttagagtaccccaaccgatcccctttgtcgagataggcatgaggtaagaacttgtctttagccaagttataagccaaaattggaaatgctgagaatccagtgttggcagcaaccgccaaaatcatggcggttgataattggaggatatagtagacaatgccatggccgaaaacagtttcaccaatttgtgaaaggaccgtttcgtggctgtttggcataatgcccatgtagtaactcaggaaggtaatcccgccaaagaagcaggccaagatggtcgccatgatggctaaggtcgccgcagcatttttactcttgggtttgttaaaattgggaacggcattactgatcgcttcaacaccggtcaatgaagatgatccagatgagaaggcccggaagaacaggaccaaagtcatgccttcgacaggtgccccgatatgagcagccgcatgatattcgatgttgccggtcacaatattataaccgccataaatgatcatcgcgataatcatgatgatgaacaaatacactggcaacgtcaaaaacgaagcagattcgcggattcctcgaaggttgaggagcataatgcccacaacgatcaaacaggaaatcagcaccccgtgtgaatataatgacggaatagctgatgtaatggcttcagtcgctgaagttgttgatacggccacggtcagcatataatcgaccagcaacgagccgccggcaatcaggccagcctgctcaccccagttggtgctggcaaccacgtaggcaccgcccccagagggataagcatggataatttgctggtatgacaaagtaatggcagccaacagaaccaaaacgagggctgcaacccaaatttgatacatcaacgcagctgcagacagcgtaattaaaatggtcgtaatctgctcagtaccatatgcaactgacgagagcgcatcggatgatagtaaagccagtgctttaaatttggttaaagattgaccaccctcatcagtggtctttaatggctttccaataaggagccgtttgagatagcgccacataaatagttactcctttatttaataatctaccattcttgtgaaccataaaatgatagtccttctgacaattaaaaacaagtcttgatatgtacgtctgaatgggctcacagcaaatcaccatccagacaagctaaaatatccgtcagctgtgcactcagagtcaaaatatgatctaagccacatgctaactactttaatattgaattgattaattcgcaagcacaaaataagcaccaatcccgatttggaatcgatgcttattgtacaatactttcattcaaatcaacgatttaacgcttcattacatgcccataccaggttgtggcattggagcagctggtgcgtctttcttaggctcatcagcaacaacagcttcggtggtcaacaacaaggctgaaacagaagcagcattttgaagtgctgaacgggtaactttggtaggatcaacgattccatcactgatcatatcttcaaatttaccattggcagcattgtagccaattccaggcttttcgtccttgagcttttcaacaatcactgagccttcaacaccggcattttcagcgatttgacgaacaggttcttcaagggcacgaagaacaatgcgaataccagtctcttcatcaccgccagcttcggcatccaacttggcgatttctgggatgacgttaatcaaggcagttccaccaccaggaacgaatccttcttcaacggcagcacgggtcgcattcaaggcatcttcaatgcgatacttcttttctttcaattcagtttcggtagcggcaccgacacgaacaacggcaaccccacctgataacttggcaagacgttcctttaacttgtcacggtcaaagtctgaagtcgtcttttcgatttgggtcttaatttcagcaactcggttggcaatttcatcgtttgaaccggaaccgtcgacaatcgtggttgaatccttggtaacgttaactttgttagcttgaccaagttgttcaagggttgcatccttcaagttcaaaccaaggtcatcggtaatcaaggttgcaccggtcaaaatggcgatatcttggagttgatccttacgacgatcaccaaatccaggtgccttaacagcaacgacgttgaatgttcctctcatcttgttcaatacaagagttggcagagcttcaccgccaatgtcatcagcaatgatcaagagtgaacgaccttgttcaacaatcttttgcagtaatggcaaaatgtcttgaatgttggtgatcttcttatcagttaccaagatgtaaggattgtccaagttggcttccatcttgtcattgtcggtaaccatgtattgtgacatgtagccgcgatcaaattgcattccttcaacaacgtccaagctggtatcaacaccacgtgactcttcaatggtaataacaccatcatggccaactttttccattgcatcggcaatcaatttgccaacttcggtgttagcagatgaaattgaagcaatttgtgcaatatcgtctttggtcttaacatcatgcgacattttgtgaagggcatcaacagcggctttagtagccttttcaataccacgacgaattccaactgggttggcaccggcagtgacgttcttcataccttcattgacaattgcttgagttaaaactgtggcagtggttgttccgtcaccagcaacatcattggtctttgaagcaacttcagaaaccaatttggcgcccatgttttcaaaatgatccggtaattcaattgatttggcgatggtaacaccatcattggtaattgtcggtgtcccggcactttgttccaaaacaacgttgcggcctttaggtccaatcgttgccttaaccgtatctgctaatttatcaacacccttgagcattgcgctacgggcatcttcagaaaactttacttgtttagccatttcaaatttcacctcaaaaaaatatttttgattattgattcattgaatgattcaaatgattcacttattagcaattatctcgttaaaatataattattcgacaattgcgacgatgtctttttcatgaagaacgagataagtttgatcgttatcctcaatctcggttccggcgtacttatcaaacataaccttgtcgcccttttttacaacaggtgcaaccttggtaccattatcaagtacacggccatcacccacggcaacaactgtaccggcttgcggcttcttttttgcattgtcagcaagaacgataccgccaaccgacttttcttcttctttttcagtttcgataattacgcgatctcctaatggttttaacacgttagtccctccgtttgcaacaatttttagcaacattagcactcacatgataaaagtgctaatcactgtgtataatatattattttttcagaccaattgcaaggatttctgcacatttcttggtgaatttatctgcagattgccttgctgacggtaaatgaacgcataagaaaagaccggcgttttcaagatcaccggtcttttcttcattaatttgttcgatattttacttgccaaagttttcgatgaaataaatcaaagtttgcaattcattagttaagtcaacgttctgaaccaggacatcttcaggaacctgaagccgaattggcgtaaagttcaagacaccctttaccccgccggcgacagcatcgtccgcaatggactgagcgacttttgagggcacggtcaaaatgatgactttgatctgttgatcatgcagttgatgtgaaagttcctcaatcgggtagacaggaacaccgtcttcaattgtattcacaatcttgtcgtcagtatcaaaagcagcggagattcgaacgttgccgtctttgtgaaaattaaagttcaagagcgcatggcccaaattgccgactccgatcaaagccacgttggtcagatgctcttgattcaagatcgttttgaagaacgaaagcaggttgtccacatcgtatccatacccccgcttgcccaacgcaccaaaataggaaaagtcacgacgaatggttgctgaatctacctgcaccgcctcggccaattccgttgatgaaattcgttgctttcctgtatcatgtaaaatatttaagtatcggtaatatatcggcaatcgtttagcggttgcgcgtggaatattttcagctgtcaagaaaatttcctcctatttgtcattttagttaagagaactttgtgaattcctatttacatctcattctaccataagatgacatcttgtgaaatatatttcaaatattacttacaaataattcctgaaatcgtgtaaattatgataaaattgattgttggtagttacaaaatgaaaggtggccaaacacttgataatcttacaagcacaagatctaaccaaacgattcaatggcgaaactattttctcaaaagttaatttggccattcaagaaaaaagccgtgtcgcactggttggccgtaacggtgccggcaagtcgacactggttaaaatgatcatcggcgaacaatctgtcgacggcggccaaatcagcactaaaaagaatctgtcgattggctatttggcccaggataccggactcaattcagataaaagcatttatgctgaaatggcatcagtctttgccagtctaaaagagcaggaagcaaaacttcacgctctggaaaaacaaatgggttctttgggcgttgacgccaataccgaagaatatgaaacgatttcctcacaatatgacaatatccgtgccgactttgaacagcacaatggttatgggtacgacgctgaaattcgtggtgttctccacggatttggattcggggaagctgactacgatcggccaattaatgaattgtcaggcggccagaagactcaacttgccttagccaaactgttactggaaaagcccgaattattaattttagatgaaccaaccaaccatttggatgtggaaacgatcacttggctggaaggttatattcaaaactatagtggtgcccttctgatcatttcacatgaccgttacttcctggacagaattgtcactgaggtttacgagatgtcacaaggtaccctccaccacttcactggtaattacacggactacaccaagaaaaaagaccagttgattgaccaagaatggaaagaatatgacaagcagcaagctaagattcaaaaactgcagaccttcgttgaaaaaaatatcgttcgagcatcgaccaccaaacaggcacaggcccgccgaaagcaactcgaaaaaatggataagctgcaaaaaccgacggctgattcaaaaactgcccgcttctcattttcaccaaaatccaaaagcggcaataacgtcctgaacgttaccaacgcagcggttggctacagtacggtcctttgtgagccggttaatctggacgttaaacgtcaccaagcgatcgcaattgttggtccaaacggtgtcggcaaatcaacgctcttaaaaagcatcttgggcatcattccgtttttaaagggcaaggcgcagtttggtactggcgtcgataccggttactacgaccaggaacaagcctcactacacgcctctaaaaccgttcttgaggaactatgggatgatcacccaacgaccccggaaggcgatattagaagcattctggggagcttccttttctccggtgacgacgtgagcaagatggtccatgatctgtccggcggtgaaaaggcacgattgctcctaaccaagttggcgatgcagcacaacaactttttaatgttggatgagcccaccaatcacttggatatcgacagccgcgaagtgttggaaaaagcgctcaatcaattcgacggcacgattctctttgtttcccatgaccgttattttatcaacaaaattgccacagcggtcgttgaattgtcccgacatggcaccaccctttaccttgggaattatgattattatgtcgataaaaaagatgagcaagaagccatcaaggctcatgaggctgaaaagaaggcggcgggccaaccgaccccagttgccgtgccgaccaccgataaaaagaactacgagattaataagcaaaaccaaaaagaacatcgcaaacttgaaagagaagtcaaggctctggaaaccaaacttgatgaattgacacaatcaaaggatcaaattgaagcagaaatgacgaagccggacgtctttaacgacctgggaaagttgcaagatcttcaacagcagctcgatcaggtgactgcccaaatcacagaaactgagtccagttgggaaacggccagtttgaagctcgaagatagtgagtagcataatccacaagaggcaaaagatatccgattcacatcgtctactttaccaattggcgacaacccactaaattaaaaagcagcctgaggaaaaggattttatccttctgctcaggctgcttttgatctaattattgaattatccttcatcacaggatcgctgacgatttcataatcacctcaaaaaattggtcaattatttagcctcatctgccagccaatcaaactccaaacccggatctgcatttaaagtggcatcaccacgaacaccatgccgatacagcatctcaccggcagcaccaatcatagcagcattgtcgccacacaaagacagtggcactaattcaagtttggtatcggcaaacgcggcaacctctttggttaaccgctcccgaagaccttgattggcagcaaccccaccggcaagaattaattgtttgaccggaaattctttgagcgcgcgattggttttgtcagccaagacgtcaacaacggcttgctgaaaactagcggccaagtcttcacgactcaatttctcgttaatttgatcagcatggtgcaccgtattgataaaggcactcttcaacccactgaaactaaagtcaaaattatcgtcagcgtccattgcccgtggaaaatgaaaagtatcctgacctttgtgagctaattcatcaactggcttgccagccggatagttaatccccaaaacccggccaattttatcataagcctcaccggctgcgtcatcacgagtttcgccgataatttgaaattggttttcctcaggcatgtaaaccaattctgtgtgcccaccagaaacaaccaaggccattgctggaaactcaatgggttcgaccagccgggcagcgtaaatgtgcccagctaaatgattcactggaacaagcggcaaattgtgcgcccaggcaaccgccttagcggccgtaacaccaattaaaagcgcaccgactaagccaggaccgtatgtaacagccactgaagtcagttcatcataagaaacgtccgcctcacgtaatgcatccccaatacagccggttatctgctcgatatggtgtctgctggcaacttcaggaacaactccgccaaagcgttgatgactcttgatttgcgttgcaacaatatttgaaagtattcgattgccattctcaatcactgcgaccgacgtttcatcacagctggtttcaaaagcaagtactaaatctctagccacttaattcatcccatcccttttaaccgattttggtgatgtccaaaaccatatttaaagcgtcttcacgatcgttaaagtaataatcttttttaatcccgttatcaacaaatccaatatcccgatataatttttgtgcacgggtgttactgacgcgcacttcaagcgtcaccttggcatattccaattgacgggcctttttgataattgttgtcaccaaaaaataccccaagccatgattctggaaatttggggcaaccgcaacgttggtaatatgacagtccttagtatgatcgtttagcgagcagccaataaacgctaccagccagtcgtttcgacgcaacactaaatagaggcgatccgttttgcgcatcagttcggttcgaaaggcccgatcatcccacggagtctgaccaccgtaaaccgcccgctcaatccctagaatctcaggaatatccggaatcatcgccttggccaaaaagtactcagttccattaatttcaacatcgtggtttttgatgtcgagatatctctcgcgaagctgaacctctttgttataaaattgttggttaaaccactctttaaactttttcaacatagtcatgcgtatcctcattaggatgtaattttttccaatcagcctcagccttggttaaccgcaaatatcgtgggacaaccgcatcaacgaccggtactggtgactgactcaatccatacaagcccagtaaggtcgcactgggaattcccaaataaggattggcaaccaccagacggttatgcagaacgtcgcgcatcgatctttcaaatggatcggtatcccctaaaatgataatccgttgatcataacgactaacggtttccaaccattttgttagattggtgtgctgatcctcaatcacggtttgaatccgacgacttcggtagcggtataatccagtaaacatgttttgattccggccatcaaaaatcgggttgatcagcacatcttcttcttgaacattcaaggcaagatttaacaagctggaaactggtaccagttcgattcccaaggtgcttgcaatcgttttggctgcagtgacagccatccgaatgccggtgtaagatccagggccggcagcgacaaccacccgatccaaatcagttggcttcaaatcggccttttgcaccaagtcttcaatgaccggcatcaagaattcggcatgtttgcgatgagtggtgatggttgtttgcgccaaaagttggtcattatccaaaacagcaactgaaagcggttgatttgaggtgttaattgctaagattttcattattaatcgttaccctttgctttgatatctttccaaacaattgtggcacttgcggaaagaacatcatttgatttaatttcgtgaactgttttaattttagcattatctgaagaatcaacaagcactgagctggtgacccgattgccatacttaacctcgttctcaaagcggatgtcaatgttagtgggttcgtgttggttcaaaaagtccattggcaatgaatccaacatccactccggatacctggaattattgacgtggccattaaaatcgatatcgctccaacgaacttggtattcctttgcgctaacatcatcagtcgcttcaattcgttcaggacgtgccaatctgggaacccgtttgaccttctccgactgatatggcgcaataatcgtttcgtcaatcggtgtaattttgcgggtctgttcgttcattaacacccagatactctccaccttgaccagctcgttgccagcttgatcgtgcagccagaattcccgaaaggcaaaataacgattatatgacgtgcctcgggttgtcattttgacgactgaatctttgcgtggcaagtgagtgatatgaattgagtaagaagtaaccacccagccaactccataatgatcaattaaataagtttgatcaagtcccaaattttcgttctggtgttcggacgccaaaatcaaaatattgatcaacattggaattgaaatccggttgttgacgttacactcgtaaaacggaatcgtatgcaattcgctaaaactgtgagcaggcatggacattacttctttctatttgatgtcatggtactggttatagatgacctgtttttttaaatgatgatctttggcaacctttttgattgcttcattaacgctcaaaccattttcgatgtaaaagtcaacttgttgatcaacgctcatcccggcaagcggatcatctccctgcgtttgtggatgggcatttcctgacactataataacaaattctccgcgaatttcagttgaattggcccattcattgacctgatcaagggttccgcgaataaattcttcgtgctttttggtcaactcacggcagagagctgcctgacgatcccctccgagctgagtcaataaattcttcaaagtttttttcaatcggtgcggggcctcgtaaaaaatcattgtttcttctcggttacggagctcatcaatttctgctcgctgttccttcggctttcttgataagaagccatagaaataaaatggctgcggcaaaagcccggaagcaattaaagcagtgatcccggcgttggcgccaggcagcggcacaacgttaatatgctcacgaatacaggcaaccaccaattcatggcccgggtcgctaatcgacggcatcccggcatcgcttacctgggcaatcgtgattccctgcttgagtttgctaatcaactcgggaatccgctcggcagtattgtgctcatgaaaactgatctgcttggtttggacatcgaaatggttcaacagtttctgtgtgttgcgggtatcttcagccgcaatcaaatctgcagactggagaattttaaccgcccgaaaagtcatatcatccagattgccaattggcgttggaaccaagtacagcgtgccatattcacttaatgtgtcaaaactcttttgtgtgtccactgtttacctcttaatcgcgtttgccatagataatgtccgtacagaaaatacaatcttcaccgttctcccgtcgcttaccgtaataagaactgcagacatgaaatccttcattgtacagtttttcgagattcttgcgagactttgacaaacgtggcgaattattgtccattttttcggttatttcgttaatccgatcgcgcaaatgctgattttcaatctccagctcagcgtttttttccatcaacccaataagtgattcatgcaggtgagaaaaattttcagcactcgcactgagctgtgtatccatttcttttaattcatcatataagttttgactgtccacgattttatcaccctttagtaaactatgattgcccaattgcgagtatctttagtgtcaaagcttcaattatgttttgaaaattgacgttaactgccatccggctattcatatcaagcagctcgtcaagcatggttaacagttgatcgttattccactgattggccgccaatttggtctgtgcaagaatcgccgggtacttcacccgatcatccgccaaagtcccgtatttcatttccaaaacatcgtcaaacaaactcagcatcatggaaataacaatccgctgacggtccttgttggtaattagaggcatcaaagacatttggatgaaaggcattgccatgttgttttctttgaccaaataggtaaaccatttctccaaaagccgctgcatcgaggcaaaccaatcatctttggacagctctttaatctgatccaaactattggtaatggaaatcatcaagttgacttcactcggcttgacgccactattctgtaattcttggaccatctgctttttactgaggctgggaaattccacaacctgagttctggaaataattgtcggcagaaccagattgcgattctgactgatcagaaagctaaccacgttgccggtaggctcttcgataaactttaagagactgttagctgccccggtagtcatcttttcggcttctgaaataatgaaaacctttttggatccctccatggcacttttggtaaattcacttttaacgtggcgaatctggtcaaccttaatactttgaccatcaggttcggtgatgacaacatccggatgatcatgattcatgattcgcacacattcggcacattttccacagggcatgccattttgaacattcgtacaaaaaagccgcatggcaactcccattgcgactgaaaattggccggcaccatcttcgccggtaaacaagtatgcgtgtgacaattcattgtttttgattaaattcatgaattgggtaaagatggtcggctgtttagtttgagcaacgttaacaatatcgtgttccataacgttcccttctagaactgtttaaaatcttcgattggcaaaatcataaccgtagcaccaccaacttgaacttcaattggaaaggtatgttctgccgtatcaccgttcaagctgaccggcggtgtcataaattgttgtctagccgaacaggtttctttgattagtttcaaagttaaatcaacttttgaatcatcaacagcgaccaaataagtggtatttcctgctcgcagaaagctaccggtggtcgagaatcgggttgcgatgatatcgtgagcaacgaaaactgatcgcaacttgttggcatctttgtcttgaacgatcgcaatgactaatttcataatcaactctccttaaaatactcactggcaatttggtggataatcttaattgtatcattaacgacgcgattaatcggttgagttgcatcaatactgataaatcggtcggcattttcgtcacggaccttcatataaccctcatgaacccgtttatgaaattcattggtttcaacatccaaccggtcaattttactgcggtcgcggtgttcggcgatccgatccaggccaacgtcaaccgggatatcaaagtagatcgttttgaacggtaacaacttttccgttgcaaactcattcatcttggcaacttgtgccataccgatctgacggccggccccctgataagctactgaactgtcaacataacgatcacacagaaccaatttgttctgcttgagtgcgggtaaaatggtttcaaccagatgctggcgacgagcggccgcataaagcaaggcttccgttcgataatccatctcagtattctcacggtcgagaatgactttgcggatttcttccgagattttattgccaccgggttctcgggtgaccaagagttgatcgccgatttcctggttaaaaacttcaatcacgcgattcatcacggaagttttgcctgcgccgtccggcccttcaaaggttataaacttaccattcaaaacaattccctcacttttaatttaaattaattgtacttgctgttcgtttgcctgtcgattcagccaacgcttaggtggtccggattattcaaaattgtcatgatcataactgataaccgagggctgaatttggtaattcttaatttttcgaattcgtgcctctttatatatgaagaaatatttttgacgggccaacgcagtttcctgctccatctccatatcactgtcagcaaccgcttcttgggtttgagcagcatgatcccactcttctttcaaattgttgattaactccaacaagcgatcgtcgtattcacgtttaacattttgccgtcttaatcgattaaaaaacattcgaaaaccccaccttgtcaaattaaatttcagtccgtccttggactgccttaaacaacgtgacttcatcagcatattcgatatctgatccaactgataatccgtgagccaaacgagtcactttgatcccagcgggtttaatcaacttgctcaagtacattgcagttgcttcgccttctggggtggcattggtggccacaatcacttctttaacggctttattttgctggagtcgtttgatcagtgagctgatattaagatcttcaggtcctttgccttcaattggtgacagtaccccatgcaaaacatgataaaggccgtggtactcctggaccttttccattaccatcacgtctttgggttcttccaccactaggatggttgattgatcacgggttttatcacgacaaatttcacagggatcttcatcggttagattaccacaaatcgaacagtaatgaaggtcgttcttggtggcaaccagcgcctttgaaaacgctttgacatcatcttcattcatatcgacggtgtaaaaagcaagtctggtagctgtcttactcccgattcccggtaacttcatataactatcaattaactttgcaattgcttcaggatattgcatactttccccttttttcgtgcagactacattcccggaatccctttggtgtatttacccatggtgctttcagtcgctttatcaaccttggaaaggccatcattaacagcggctaataccaaatcacccaacatttcggggtcatcgggatcaatggcttccggcttaatctggatatccttcatctttttgtcaccgccaaaagtcacttcaaccatgttatccggtgcaacgcccttaaattcctgctgtttaagattctcctgctcttcacccagttgcttttgcatctttttcatttgcttcatcatcttgttcatgttcataccgttcatcattttcttttcctccaattaatcatctttgatatctaaaatgtcggtgccgaaaagttcggcagccttcttgacgactggttgactgtccggctcttcttttgacggttccggatcgtcatcagccggttcagcttttgggtcgtttgcttctttggactgggagccagtcttttttatcttgtctttgtgactggccaaatactcacggcgaatatcgggccactgattttccggaacaaacacaatttgaggggcttttcccacaatgcgatccaaattgttttcaagagcatccttcaaatcagtgtcaccttgagccttctgatacaaaaatgggtattcgaaggcaacgattactccgccggcactggcagccaccggcgatgacacgtgcatgacagcccgttgagtcaccgacagggcatccatcaagtccggccaaaccgatttaaattgatttaattgtttccgggtggctttacccaaaattggatagattttagccagctcaatgtgattgtccattgagtgagcctcactgactttggcaggctccggtgtgctgactgttggtgactgaggtgtcgactcccgtttgagatcggcaacttcagccttgagttcggcaacttgctgcgtcaattgttgaatttccgcattaacttccgggggcacggccgttttagccgactgctgtgattgtggggctgaaacagccttgggctgatttgtggcatccaaatgggtaattttgaccgtcaagacctccagataaacatctggatgagcggtaaaccgcaatgaattagaaatcgcattcaattcattaatcatctgataaatcgcttgatcgctgatctggccgcttaaggccttgaactggtcatcaatgatccctagttccatttcttcaacgattccgggatcctgttgatataacagaatatcctgacagtaactggtcaaatcttcaatgaatcggctagcgtctttaccctcatccaatattttttgaatggtaatcagcgcgcttttggtgtccttcttgaccacctgctgcatataggtggttaataattcattggtcacgctgccggtcacaagtaaggcgttctcataagtaattttattatcgccataagacatcgcctgatcgaggatactcaaggcatcccgcatcccgccctcagcagctttggcaattaatttcagggctttgtcgtcgtactcaacctttttttgatcaaggatatattccattctttccaaaatatcctgaggtttaatccgcttaaagtcaaatttttgtgtccgggagatgatcgtcgccggaatcttgtgcggttcagtggttgctaaaataaaaattacgttagccggcggctcctccagcgtttttagcagggcattgaaagccccagttgaaagcatgtgaacttcatcgatgatgtaaactttgtaatcagcctgagtgggggcgtatttcgccttgtcccggatatcccggatttcttcaacaccgttgttggaagcggcatcaatctcaatgacatcatttaaactgccctcattaattgctttacaagtctcgcactggttgcagggctcaccatcttttaagtagtgacagttcactgccttggcaaaaattttggctgccgaagttttacctgttccccgaggaccggtaaacaaataggcatgactcgtttgtttagtaattagcgcattttttaatgttctggtgataatcgactggccgacgatttcatcaaatctttgtggtcgccaaacccgatataatgcttgatagctcattaccaaatcctccaaaatagaatgccgaattcttaaaatcgttcaatgaaacgtctaaataattatatgatgaatctaaccagagtgcaatcaacgaccgtctgactttcaagaaatttctccaaaaaaatgccctcagcaaagttgctgagagcaaaagttctatgtacaagaggcacaaggttgatgatacttagtgctgcttccttccggacctgacacagttcgtaacccgacccttgcctcagggccttgcggcaatatctatcataacttaaatgattcagaattgccagccttattctttcttttcttgcgcgcagccttgaagaaatctttcatgatccgcgatgccgcatcggcataaagcccttcaacaacgttgacttgatgattcaatcgggaatcttccaacactgcgtacaaacttctggttgcgccggctttgggatcacgagagccaaaacaaacattttcaatccgcgaattaataatcgctccggcacacatcaagcacggttcaatcgtcacataaagatcgcaatcaatcagccgccaactccgcagtgttcgacaagcctcttggattgctaaaatttcagcatgcgccgtaccgtcatttaaatgttctcttagattgtgaccacgcccgacaattgtcccgtcatggacgaccacggcgccaatcggcacttcaccaattaggtaggccttggttgcttcgaccagtgcagctttcataaaacgactatcagcttgaaacatttcgaaccctcacgatttcttgatgctttgaagaatgtagtaacctttgtcccgttttaaaatctgacagtcaccaaatagtttggtcattaattttttggcagatggtgcgccctgctttttttgaagaaccaccgtcaaggtgccgccatcaactaagtgatcgactgccccggagatcatggcatcgacaactttcttgccagctctcaccggcggattggtcacgatggcagcatactgatcagtaatcgcttcatatatgttactttcaaaaatatgaacgttatcaacccgattggcgtcggcattctttttggcaagcgccaaggccacctcattgacgtcaaccatatcaatctgccgatccggaaatgctttggcaattgaaatgccaatcggaccgtacccggttcccatatctaacagtttgccgtcaggaatgagatcataattaatatgattaaccagcacccgactgccgtagtcgaccgtatgtttagagaacacaccgttatctgaagtgaacactaagttgtttccaagcaacgcaaagttccatgtaatcggatcggatttcacgttgggattctttgaataataaaatgattgttctgacataaaattctcctaaaatgatcttttataatcgttatctatatttggtgcttacaattagttttgtcacaatatattgtgttttaatcgttgcatttcacactatttagtgtaaacttgaatcataaattaaattttaacgaaacaggggaagtgttaacaatggctaaaatcacactatattcaaagaacaactgtatgcaatgcaaaatgacaaaacgttacctttcagaacataacgttcaatttgaggaacacaacatcaacgagcaaccacaatatattgattacctgaaacaacgagggttcatggctgtccccgttgtcgatgttgatggtaagcaagcattcagcggctttcgacctgatcagctccaatcgattgccggctaattgccttcatccattctaacatattgatttcagattagcgggcgaaaccacaaacggtctcgccccttttattcgcaattataagaaagcgtggtactaaatatgtcacttcacaaccttaaggatgttacctactttgatttgaacaacgaaattaacatccccgtcaacgggcagattccactgcaaaaggacaaggaagccctcgaagcctttttaaaagaaaacgttcagccaaacttaatgaagtttgacagtctcagcgatcggtttgattacctgatcaaaaacaactattacgaagccgattttattcataaatatcaactatcctttatcgaaaaattgtaccagtacttaaacgatcaggatttccacttcaaatcatttatggcagcctacaaattctacgcccaatatgctttgaaaaccaacgacaatgatttatatctggaaagcttcctggatcgggtcgccgctaacgccctcttcttcgctgacggtgatgaacagttggcaatggatttggccgacgaaattgtccaccagcgttaccaaccggccacaccaagcttcttgaacgccggccgggaaaatcgcggcgaatttgtatcttgttttctgattcaaaccaccgatgatatgaatacgattggccggacgattaattcggccctgcagctgtcaagaattggcggtggcgttggaattaacctttccaatcttcgtgaagccggtgccccaatcaaacatatcgaaggtgccgcttccggtgtggttccggtgatgaaattgcttgaggacagcttttcatactctaaccagttgggtcagcgtcaaggtgccggagtcgtttacctctcagtctttcatccagacatcatcgaatttttgggtgccaaaaaggaaaacgccgacgaaaaaatccgcctcaagactttatcattgggagtgaccgttcccgataagttctaccaattgattaaagccgatgctgacatgtacttattcagcccctatgatgtggaacgcgaatacggcgtgccattctcttacgtcgacattaccaaggaatatgataatttggttgccaatgacaagatctccaaaaagaagatcaaggctcgtgatttggaaactgaaatcagtaagctgcaacaagaatcaggttacccatacatcattaatattgacactgccaaccgctccaatccgattgccggtcgaattgtgatgagtaacttatgttcagaaatcctccaggttcaaaccccatccactgttgataaccagcagcattacatcaaaatgggcaaggatatttcctgcaatctgggatcaaccaacattaacaatatgatggctggcgatgactttggccattcagttgaaagcatggtccgggcattaacatttgtcaccgaccactccaacattgacgtggtcccttcaattcaaaaaggcaataaagaatcacattcaattggccttggcggcatgggactacacagtttcttagccaagcaccatatgtactacggctcgcctgaatccattgaatttaccagtgtctacttcatgctgttaaactactggagcttagttgcatctaacaagatcgccaaggaacgcaaagaaactttcgttaacttcgaaaacagcaagtacgctgacggcagctattttgacaaatatctggacggatcatttgcaccaaaatctgccgaagtaaaagctttgttcaaagacgattggattccaactaaggaagattgggaaaacctcaaggaatcagtcatgaaagacggcctataccaccaaaatcggttagcagttgcgccaaacggttctatttcttacattaacgatacgactgccagccttcacccgattatcaaccgaattgaagagcgtcaggaatccaagattggtaagatttattatccagccccatacctttcaaatgacacaatgccttactatacttcagcctatgacatggatatgcgtaaggtgattgacatctatgctgccgcacagcagcatattgaccagggaatggcattaaccctctttatgcgttcaaccatcccagaaggtctgtatgaatggaaaaacggccggacagacaagatgacgacccgggatctcaatatcttgagaaactacgcatacaaaaagggcgtcaagtcaatttactatattcgaactttcacggacgatcaacaagaagttggttccaacgaatgtgaaagctgcgttatttaaaggagaaattcatgactgagaattataaagcaattaattggaacgccatcgatgaccaaatcgacaaggccacttgggaaaaattgaccgagcaattctggctggatacccgaattcccctgtcaaacgacctatcggactggcggacgctggatcaagatcatcagtgggttgtcggtcacgtcttcgggggcttaactttactggatacactgcagtcccaagaaggaatggcatcgttgcggaaagatgttcagactcaacacgaaaccgccgttttgaacaatattcaatttatggaatcggttcatgccaagagttattcctcgatcttttcaaccctcaacacccctgatcaaatcgatgagatttttgactggagtgacagtgaggaattcttacagaacaaagcactcaaaattcgcgacatttatgccaatgaaccagacccactcaagaaaaaggttgccagtgtcttcttagagactttcctgttctactctggcttctataccccactttggtaccttggccacaacaagattccaaatgtggcggaaatcattaaattgattctccgtgacgaatcagtccacggcacctacatcggatacaaattccaaattggctacaatcaattgccaaaggaaaaacaagaagacatgaagaactggatctatgacttcctgtacaaactgtatggtaacgaagaaaagtacacccatattctgtacgaccaaaccggctggacagaagatgtcctcaccttcattcgttataatgccaataaagcgttgatgaatttgggtcagaatccgctcttcccagacacagcagaagatgtcaatccagtggtcatgaacggaatctcaacatcgactgccaaccacgatttcttctcacaagttggtaatggctacctcttggggaacgtggagtcgatgaaagactcagattacgatatttaaataaatacctcacagtaactcaataaggctgatgcatcccagcggggatgcatcagccttatttgtctttaacaattactaatcaaccaaatcctttggtgtcttaccattaaccatcgtctcaagattccccagtgagatatcaatcatatttttcacagcttcactggtatggaatgcggaatgtggcgtaatcaagacgtttggcatcaacgccatcttcaatacatccggatcattgacttttttggtggacctggagtcttggagatcagcagattcattttcaattgtatcaatcccggcaccagcgatttcaccgctctggagggcaaaaatcaaatcatcggtatcgacaattgaaccgcgagcagtattgatgagaattgccgtatctttcatttgctcaaacacctcatggttaaattgatgataattatcatcagttgccggcatatgaattgagataatatcgctttcttgataaatttgttccaagcttttggcatatacaaacgaattgtcggtatttttcagcggatacttgtcataggcaattacctttgcccccaggcctttgaacagcttgatagctgcctggccaatccgtccggtcccaatcaccccgacggtctgttcactgatcagacggcccatgaagttgggtgaaaaatgaaattcatgcttttgatccaactgctgacgcatatagcccacttttctagagaggtacagtgacatcatcactgcaaattcagcaatactttctggactgtacgccggcacattggtaattttaacgccattggctttagcggctggtaaatcaatgttatcaaccccgacatttctgagcgataagtatttgattcctaagcgtttaaatgactcaaataattcagctgaatattgaatcgtttgaaggcaggaaataccgtcaaagccggctgcttcttcaaccgtctcctgattcaaagttgtggtggtgtatttcacttcaattccgtgatccttaccccacttctcaataaacggtatttcatcatctcggacattgtatacaataaatttcatagttgcctcctagtgatttcagcttaaatttggttccgcttccattttaccaaaaataattgttgaaacaaaatccaagcccacctgcagaggccaaagttgagtgaatcccttttgacaataaaaatagagctggaaatcaaggacgcttatttccaaccctattccaaattatttaagttgctcaatgaaacgatcaaaggccgcttgacctttgtcgtcccatttgtaaacgccggcatcttccagaaccctgccaaagactttgccaacttcttggtcgactacctcttcaacattgtccttggtaaagtggtcacgtttcatcaattcatctgcccaaggcttatgataatcagcaatctgattatcttcacccaagacatacttttcgacttctttcatttcggtcttcagacgagcaggcaaaattgcccggcccatgacttcaatcaagccaatattttccttcttgatgtgttgaacatcttgatggggatggaaaataccatcaggatacttgtcagaagtttgattgtcccgcaagacaatatccatctcaaactggtcatcattcattcgggcaatcggggttaccgtatgatgtctcgttccgtccgtgtaggcccgaatgtcaactgactcatctgagtagttcttccaagtttctgcaatccgattggcagcattcaccactttattggcatctttgctgaccaggcgaatggttgccattggccatttgacaattcctgccgacaagccgtcaatccccaaatcaactggtcgatcaatcttggccttcatcatcgggaacgtgtggcgaccaccttgatagtgatcttgggccaataaggaaccaccaacgattggtaaatcggcgttgctgccgacaaagtaatgtggaaactgcttgataatgtcaaccaaattgacaaatgtccgttgatcgattgacattggcacgtgcttttggttaagaaaaatcgcatgctcaccaaagtatgcataaggtgagtattggaatccccacggttcgccgttgatcatcatccgaataacccggtgattgcttcgggctggatagcctaggcggccgagatagccttcattttcaatggctaacgggccgaccggataactggttgactttgcccggccagcggcagcaatcgccttaggatccttctcaggctttgacaggttaatggtaatttccagattgccataatcagttttagtttcatatgaaatatttttggcaatcgcccgagtcttaatataatcattgtcttggctcatatgatagaagtagtcggtggccgcatcaggagattgttgatacttgttccaaaagatctgattcaaagttgatggaattggtgttaacaggtccatcagttgatcttcaagaatctccctgttggtaatcgaatcttcgaccttaccatgttcaatggcgagatccaccagatcgttggctaagtcgacagccgatgaatcctcggttggctctccaaaaccatcaccgatcagtctaaaaatcaggttggtgacataaatccggtcaacatctgaatatggtgaatcagatttgataattaaatcgacaaacttttcaactgctgattggctcatgattactgatttcctttccgatcgtcatagccctttgggtgggtttctttccaattccaggcggtcttaataatttcgtgaacgtcgtcaaattgaggcttccagccaagaatcttgcgggctttgtcactcgctgcgatcagcgtgcttggatctcctgcacgacggggacccattttggctggaatcggcttgccagtcacatcacgggcagcatccaacatttgtttgttggagaagccggttgatgagcccaagttaaaggcatcgctatcatgaccagcttggagatacttcagtgccaagatatgcgcgtcggccaaatcaagcacgtggacgtagtctctgacgttcgtgccatcaggcgtatcataatcgtcaccaaaaatcgtcaactcatcacgttcgccggcagcaacttgtaaaatgatggggaccaaatgggtttcagggtggtggtcttcaccaattgagccatcaggcttggcacctgcaacgttaaagtagcgaagggcgacaaacttaatgccgtaagccacatcactccagtgcatgatcttttccattgccaacttgctttcaccgtatgggttggttggaacttgcggatcagtttccttaattggaatctgcttgggttcaccataggtagccgccgttgacgagaagacgatcttcttaacgttatgggcgttcatcacttcaagtaaactaatcatgccaccagtattattgtcaaagtacttcaatggcttttccatggattcaggaacaactgagaatgctgcgaagtgaatgaccccttcaatctcttctttatcaaagacttgattcataaagtctttgtcacggacatcaccttcatagaaacgggccttgggattgatggctgctttatggccggtaaccaaattatcaaccaccgcaacgtcatagccattttcaattaatcgatcaaccgtgtgcgaaccgatatatcctgctccacctagtactaaaattgccatttaaatatcctccttctaatcaattcgttacttaatctctttaggaccatctgaaatttctgcaatgtagaattctgccggatggccaatctctttctcatagacttcgccaacattcttggtaaaggcatcgacttgatcacggtcaacaatcgcaattgcacaaccaccaaatccggcaccggtcattcgcgcaccgacaacgcctggttgtttccaagcagtttcagctaatgtatccagttccttaccggttacttcgtaatcataatgcagtgaaacgtgagatgcattaactaatttaccaaaggtttccaagtcattattgaccagcgcatcctttgcctgaagggttcgttgattttcgaataccgcgtgacgggcacgacgaatcaaaacatcatcattgatcaggtaactattttcatcgaattcgctttcactcaaatcaccaagagatttaattggcaatcccacttggagacgcttcaaagcctcttcacattcagcacggcgttcattatatttggaatcttgaagctcacggtgtttcttggtattcatgatcacaatgacccgatctcccaatttagcgggaacgtaatcatatttgagggtattcgtgtccagaagaattgcttgatccttcttccccatcccaatggcaaattggtccatgataccggaattaacaccgatatatttattttcaaccagttgaccatatttaaccaggtcaagttcgtcgatccccagtgaaaagacatcattaacaatctctgcagtcaacagctcaatagatgctgatgaggatagtccggcaccatctggaaggttaccataaacagcgagatcaaaaccatggccaatcttatagccgtgttcgagaatctgaacaagcatgccctttggatagtttgtccagccatcttctttgttatatgccaaattgtccaacgatacttcaacaattccagcatcagaaacgtttccggagaacatgcggatcttgttatcctggcgttctccataagctgcgtagatgcccatgctgattgcacaaggaaatacgtggcccccgttataatcagtgtgttcaccgatgaggttaattcgacctggtgagaaaaatactttgcttgagtcataaccaaacttgtcattaaatagcttttgtacgtcatcagaaatcataaatttcatccctctacatatattttagtaaactttactaaccaaaatttaactcattttggcagcgttgtcaaccttaacttcacaattccctcacttgtaaaatacaattgagaatccttgatatgattgaaccacttggatgttggggaagacttcgtgaatgtggattattttttatgaaaacgcttcatcggtttccaaacaaagcctcttatatcaaggtaaatttcagtaaacattattttgatgaaaaattgttggtatttttacatttaaccgcacaaaaaagccggcagatatctgttaaataccttccggctgctgtttaatgcgattgcctgccaggttacttaaccgacaatcaattaattttcgactcagtccgccttatttgggctgattggcgtccataatgtaccagagagccttggagaggcctgccggctttttattgcgcggttgattaacaaccaggataatctgcagaaccgcgtaaaccagcccgcttcgacgataatacgcaatatattttgactcccacttatcaacgtacttgtccttataagaccggagtccctcaaaactataaagcttataaccgtattgatagatgagatgaacaatccgctcctgagtgaagctgaagcgggaagtgcccacattcgagaacggtgacatccccaagtcaaagtacttgtatcctttatcgtgggatatttcataaagattaatcaaaatgccatccatgatgcctgatggggcatcggcggaggaacgcatcagatcaatcgaggtgaccactttattaccatccggcatcagattggcaaacgcaacaattttgccggcatggtctttcatcacagcaatcggcgcctgttgaaggtagtattcgtcaaaaaagccgagtgagaaacccttttctgctttattatccaaccactcgtcagaaatcttccgcagagtggccagtaactcatctgaaaacggtggctgcagaatctcaaactggtagccttcgcgatcgaatttgtgcatcaatgcccgttcgccgcgatgccgtttaccactgagggtgaactgatccaagtcgactaatccatcctcaccggtcttgataaagtcaaaaccggtttcgtgaaggctcatggttaattcttcatcaatttcgtagaataccagcttcagatcggatttgtcagcttccttgacaaaatcatcaatcgcgtcggcaaattgggcacgattgccaaccggctcgcccataattaacagtttgtcagcaattttcttgaacatgaagaaaacctgatcttcgccgtctttgctgtaaaagtaaatctgcttatcgcgcaagaatgccagatgactatcctcattgccaccaaatttatcaatcacagccttcacccgatcggcatcaaatcgctgtgtcagccattctggatgaccggcagtcaagtaggcattcatgccaaccagaaccgccagggcgatcaataagccaacaaaaccgaccagccaggcacccgcagatggaaaaagataggctttatcaaaatggagatgaagatttcgattggcagcaatcccgatgagggtataaattgcaaatgtgatgataaaaattgacccattaaacaggaacacaccccaggaattagccatccggtcccggtataacaccgccttggagagccgcagagtgattaggatgatcacgaacagcaagaccatccgccaggtaaacgcctcgttaaaccatgtgttaaatatcgaaataatcagtacaaataccgtaggggcatatgccttcttggttcgagtccagataccactggccaaaccgattaagaggaatgcaacgataatattcatcatatgactgacgaaaaaaatcgaatatggcaatagtttgacatacagtttattaacaaccactacattgggaaccgtggcaaacaacaacatcataattccggaaaaatacataaagccagttaagaagacttgggcaatccgttgaaacagaagccgtggtagatcatcaagaaaggtgttgagtttggacccagtatcgtgaatgaacagaccggtgcccacaatgaacggtaacaagtaataaaacagacggtaaagcagaatccagaccagcgcatcacttcgggcaacaccaatgaatcccagtccaatgatgacaaagatatcaaaggatcctaatccacctgggatcatcgagacgactccggcaacgttggcaaccacaaaaatgggcacaaccaatcggaggtcaacaggtagattcatgagataaccgatcaaaataaagaaccccagtgcactcccccattcaaggaacgagccggcggtcatgaccagttcctgcttggttgacaggtcactgaaaaactgtgaattagtcacttgggtaaaaatcatcacaccgggaaaatacacggcaccgcctaatagccaaatccaatagtgggcaaattcagtcccgatcccaaagccaaagatcatgatcagtgaaaccaagcagagtaaagaaagccctgatatcagaaacaaggcaactttggaaatcgcatagaggatctgtttgcgagtggcccctttgccatagaaatgcgcgcgtaaactggcgcccaacaatccgccaaaccccagtaaattcgtaaaggtattcaccacccagccacttttaacgatgtagccgggggaaaatttagtgggtaagaactgaacaattgaatagtcgtacaccagcatcggcagaattgaaataaagcccgccaccagcattatcaaaagagcgccgcgactttgactggccagaacggttttgaactgttcaccgttgacttcacggataatcttagccaactgtcgaataacaaaaatcaaaacggagaagacaaaaatcagcttgatcatggtcatccgtttgtcgatgaattctttgacacgtgtcattattgttccaccatcatttcattttgaatatgtactcttcgtctattatgccaattaattgaatttcacacaacaaaggtgcacaaaaaaactgtgcatcgacaatgtcgatacacagttctgagaacaattatgattagataatgaattacttaagggtaacagttccaccaacggcttcaagttgttccttgatcttgttggcttcgtcttctgaagcgccttccttgatgattgatggaaccttatcaacaagtcctttagcgtctttcaaaccaagaccggtgatgtcacggatagccttgatagctttaaccttttggtcacctgattcagttaattcaacatcgtatgaatctttggtagcactgtcaccaccagcagcacctgcagcagcaactggtgcagcagcagaaacgccgaattcgtcttcaattgacttaaccaagtcgttaaggtcagagattgaagcatcttttaattggtcaataatattatctttatcaaaagccattttattttcctccattaattggaatttatttagttctgattaggcagcgtcgccatcgtcagattgtttcttgtcagcaattgctttaaccccatatgcaaagttacgtacaggtgcttgaagaatgttagcaagagtagataacaattcttcacggctaggcaatgcagcataagcagtaatttcttcaagactggcaacttcaccatcgataacgccacccttaagcttaagtttgtcgttagtctttgcaaagttgtggacaatcttaggtcctgcaacaggatcttctgacgagaagacaacagcagttgggccgttgaaagttggtttcaaatcatcaaaaccggcttcagcagcagcacggtccattaccttgttcttgataacttccatcttaacgccttcatcacgtaattgctgacgtaaatcagttacctcggcaacagttaaaccacggtagttaatgataacgatagatgaagcattcttcaattcttcagtaacagatgcaaccttttttgctttaatcgcaacagtttgttcactcacgaatttcacctcccaaaaatttgttgggacttaataaaaaatccctatgcccacccagacataggaaaaaagtaaacttactttcctcggcaggatattaaggcgtagaagccacctgagtcttaggcgaatatatcagcaactaacagtctatcacacaaagtaataaaccgtcaattagggattttttatttaaatcgaaactaattaagcttcaacacttgagaatgagtcaaggtcaactttgacgccagggccaaatgttgttgagattgaaacgttgttaacgtaaacaccacgtacagaagctggacgtgccttcacaataacatcctcaattgtcttcaagttaccaacaagcttgtcggtatcaaatgaagctttaccaactggaacagcaacgttaccgtcacggtcagtccggtaagtaaccttaccagcttttgattctttaaccgctttggcaacatccatggtaacagttccagtcttagggtttggcatcaaacctttaggtccaagaactcgacctaaacgaccaacttgagccatcatatcaggtgttgcaatggcaacatcgaagtcaagccaaccatcttggatcttttgaactaagtcagcgtcaccgacaaaatctgcaccggcatcttgagctgccttggcattgtcacccttggcaaatacaacaacggtctgttccttaccagttccattaggtaagacaacggcaccacgtaattgttgatcggcctgcttagtgtcaacgtttaatttgaacacaatttcgacagttgagtcgaatttagcaaaatcaatatctttaatcaattcaacagcatctttgattgggtatgctttttcagcatcaaccttttcaagggctgccttgtagtttttacctcttttacgagccatgtgtgttttcctccttgcttgtggttataacggattaacctcccacgcgatgtgaaacagtgtgtcatcgttaaagtaacgacgtaaccgggttgactatccttcgacagtaaagcccatgctgcgtgcagtaccttcaaccatgcgcattgctgcttcaacatcagctgcgtttaggtctttcattttagtttcggcaatttctttaacttggtctttggtaacagttgcaaccttgttagtatttggttcgccggaacccttttgaacaccagcagctttcttgagtaacacagcagcaggtggagtcttggtgatgaagtcgaatgaacgatcttcatacacagtgataactacaggaataatcatccctgcctgatcggcagtacgtgcgttaaattccttagtgaatcccatgatgttgatacctgcttgacctaatgcaggaccaactggaggggcaggtgttgctttgcccgctggaatttgcaacttaacaatattcgctacttttttagccacgagacataacctccttaagtccgtgtgtggtaaatggagatcaaaatttctcctcccacgttggtatgcataaacataccatactaatataacataaacattttcattcaacaacctaaattattggttccaaagaaacttggcaatttcttggtcgacaatggcattttcatgaagcagccgatgggttgcccgtttgcctcgaatcaccaattcatggtattgcgcggccggatcctgcagtaaatagcgcaatgaaaaagcactgttcaccgagacttctccgtcattttgctgggtgttgctgatccggccggcaatattgagaaccttaatgtcccttggaattgcaaaaacgcgttgtgacagcgcccgataaatcggcattcgtttggttggccccttggcgttcaaaggataagcgtcaactttatcagtacttctggcaatctctgaatcattgaatggtccggcaatcgccacaacatgctccacgctgacaggcgtcattttgctctgatgggtcagaaaccaaaaaatggtaatacagcccatggaatggccaaccaggttgatctcttcaacaccatagcgggtattgagcacctccaaaacttcagagagccacactgcctgctgccttgggcgggaagacttgtcggcaaaaagaacttggatcaggacctttgactttgccagatggcctgaaacatggattttaccgtggcggtcaactttgatgaccatcgatttgttagctccatactgtcgagttaatcgattgatgagtctgccaaatgacaatcgattaccaaagtagcccggaataaaaagtgtgggaatcgcctcaatcccatttgccggatcggagtcattaccaacctggttgggcgttccaagccgaatcagccggccgacaaccaccatcgcaatcagcaaaacaattatcaaaccagccatccataccatcgtgaccacctactttaagttaaagggttgtatcaatttgattgaagtcaagatcggtactggtctcacggccaaacatttcgatattaaccttaagtcgttgcttttcgttatcaacttcggttaccttgccatcaaggccggtgaaggcaccatcgacaattttaaccgtatcgccaatgttgacatccaaatcttcatggcgagaactcatgccaatccgtttgagtaccaagtcaacttcatccggcagcaatggcgttggcttactcccctgtccgtgagagccgacgaatccggtcactccgggagtatttctgacaatgtaccaagcttggtcggtcatgatcatttccaccagcacgtagccggggaaagtcttgtccatcttaactttgtccttaccgttctttacttcatgttcttcttgttcagggacaaccgttctgaagatgtaatcctgcatccccatagattcttttcgactgtccaaattcatcttaactttgttttcgtatccagaataagtatgcaaaacataccattgcttttctgctgactcgaccatgtttttctgctccttcgtaattccattaaatgagttcaaataaaaaaacctgacacttttcgcaggtttcaacaacttaactatatcaaagattgactcaaaaggctatgccagaaattggagtgcccattgaacgatccaatcaaccaagcctaaaaagatggccatgatgattgaagtcccgataacggtactggtatcagtccgcgtctgagatgcgttgggccaagtgaccactttcatttcctgagcaacttttttgaaaaaattaattaatcgcaaaattttatccccttatatcatgattaacgagtttctttatgcaaagtatacttaccgcaatacttgcaaaacttattgagctccaagcgtttggttcgattggggttggcgggaatcgtataattccgtgaaccgcaaactgaacaagccagagcaacttttctttgtgccatagcggcacctccttacaagcatagtaataatagcattcaaaaacaattccgtcaatttatctcgccgtcaaatttgcgccggcagcgttcaaaagcgttgataattcctctttgggctttgggatccaaatccgcataaccattttcactgagcatcaggttaaacgcccgcttttccaatggtgaacagctgctgtatagtttgcggagtgcatcatcgacgatcaccgcatcaattggactactagctgagttatcggcgattttggcagcgtaaaaatactcgttggcttcaaatgatgtcaatggttctaccggcacccgtttttgggcattgttggtgcgaatcaggtcaaacaagcggtttcgcagattgtgactgaaaaaggttccaaaactgacttttctcgcagcttcaaaccggcacgccgagcgaaacagaaccattcgggcttcctggtccaggtcgtctttatcgtagccgttgatataatactggcgtttgtacttgcggacgattggataatattggtgaaatagctgcgcaaaggcctcttcatttcgtttagctgtttgacgaatcagttcaagtcgattgttaggtaacatattgttatccccctcagatgtttttattaatcagattcgattacgaaaaacattaacggaggattcaacttccggcaagacgaaccagcgttcattcagtgaatatcccacctataccaattttaaaatatcagcatcctaatatttttattgaccatcatgtatcattttgtcccgcagcttctctaattcaaggagctgtttggcgtcaaatggcgtgtggcgaaacacttggccttgatcagtcatcttgcgcgcttcagtatcaacttcctgtttggcacgctgaacgtctctgagcaattctctagcggggatccgcaatgcgccggcagcaaaaatcgtccattgctcggcttgatcgctggtagcaacgatcacctgggtaaatcgattttgcttacgatgggccaaggcctcaatgtaactatcggcagtctgatccttactggtccagacaatctccatatcaaacttacggaagctttttgaattaccgggaacatacatcgcgtcaaaaacgacgatcatattgatgtcccggtactttttatattccgacaattcagccagcagttgatcgcgggcatcttctaaacggttggcctgcttgagcttgttgaggtgcggccaattaccgatcatattataggcatcaacaattaacaggtcttctttcattatttctcaccgactttattttgataatgggtggcgggaattaaagccctgataaatcaaaatgctggctgcaacgctcgcattcaggctttgaatatctcccaccattggaatggtcaacatttcgtcgacctgtttcttcaacagcggggaaattcccttaccctcgttgccgataataacggcgattgagcctttggcatcccaacgacggtaatcagttccggaaacatcagtcccaaaaacccacattccgcgttgttttaattctttaatggttgccgacaaattggtcacgcgggcaaccggaacccgttcaatggctccggctgaagttttggaaaccgtggccgttaatcccacggctcggtgcttgggaatgataatgccagacaccccggcagcatcggcagtccgaataattgaccctaaattatgaggatcttcgatattgtccagaatcacaaagaacggttcaaccgcttgcttcttggcattggcaaatagatcgtcaatcgttgcatacttaaaggctgcaattgataataccaccccttgatgattttggttattggaaagcttgtccagcttttgctttggaacctttgaaatcaccagccgctttttatgcgccaatttcatgatttcagagataatattgtcgtcatctttgattcctgactggataaacagtttgttaaccgggttttcactctttaacgccgcaaccacggggtgtctgccaatcacaaactcttcgggctgatcctgactgtcatcgctgcgatgatcttgactacgattatcattcttcatgtttgaggttcccactttctacttgttcaatgcaccaatttgcgatttctttcattcgatccgtctggtcacttaatgataggtagccaaagaccgcttcaaacccggttgaaatgcggtaggtaatcacgtcggtattcttggcgtgggtgtgactgttggcatttcggccgcgtttgaaatagtcccactcggtttcattaagcagaccatctgttttcattaaatcaattaaagctgcctgcgcctttgcggatacatagttggtagcaacatgctgcaggcgcttaggcttggtcaacccctgggcaatcaaatgccggcgaatgaaaacttcgtacgcggcatcccccatgtacgccaaggcaatcccgtttaactgggaaaaattatcaatcattaaagttgttattcctttctaaaccgggttccctgtggcgtatcttccagcacaattccccgggctttaagttcttctctgatttcatcactgcgaataaagtctttgtcatggcgagcctgttcccgttcgtggatcagtgaccaaatctcatcatcttttagttcactttgctcaagcttaatgccaaagacaccggacaattgacgcagggtattgataataaactgcaggctcaatttgaagacagtctcgcgttcactataagtgttggcaaattttgccagttcataaacggcggcaatcccgttttggacgttaaaatcatcgtccatcgcgtcagtaaagtcagcgacaatctggcggacttcctggtcggttttgggatcatcaccctcgtcagcattatgaagccgatattcaaggttattgaaagccgtctgcagctttttcaagttgctgctggcttctttaacactggcatcactgtactggattggacggcgataatgggtggtcgacatcaatagccgaatcacttggccgtccaaattcttaagcaaatcatgaaccgtgatgaagtttcccagtgacttactcattttttcgttatcgtcaccaattgtcacgaacccgttgtgcatccagtatttaacaaacgtctggccggtgttggcttcgctttgagcacgttcattctcgtgatgcgggaaaattaaatcttctccaccaccgtgaatatcaatcgtttttcccaagtacttggtggacatgactgagcattcaatatgccatcccggccttccctttccccaaggagaatcccacgaaatttcatcgcctttggactttttccacaaggcaaaatcaatcgggtcttcctttttagccatttcttcaggattaacgtgctggctggcaccgatttccaattgatcaacgttgatgtgtggcaaggcaccataacttttgaactttcgagcccggaaataaacgtcaccgtcaacatcgtaggcatagcctttatcgaccaaggttttaacgaagtcgataatttcaggaatgttcttagtggcccgggggtgaatcacgttgcttgaaatgttcagcgcagccgtgtcctgcataaatgcgttgatatacttgtcggcaatcgcgccaactgtcgtatggttctgtcgagcagcattaatcatcttgtcgtcgacatcagtaaaattcgaaacgtacttgacttgatacccccgatactccaagtatctgcgaacagtatcaaaggcaatcgcgcttctggcatttccaatatgaatgtagttgtacacggttgggccacagacatacattttaacaacacctggggtgatgggttcaaatttttctttttttcgcgtgagggtattaaatatctgcaacatttcgaattcctctctttatcttttatattcaaataatatcataattcacattgttttattactttaactataacccataataaaaggtctcgctgtaaatgcaacgagaccaatcgaatcaataatattttttataaattacgctttatcgatttgagccagtgtttctttgatatgcgcgatggctttttgctttccgaccagttcaacggactctggtagttccggaccgtgcatttcgtgggtcacggcaattcggattggcatccataattgacgtcccttgatcttagtgtccttctggatggctttgatgactttaaagatttcaacggagtcaaaaatgtcgagtttttgaattcgctcaagaaattcttttaagaccaccggagccgtttcattggaaatctctgccaatgcatcaccgtcaatttgttccggctcttgaaagaagaccgaggccatgtcgttaatctgagccatataactcatttcacgcttatagagcataatcaactgacgagcccactcgattgttttgctgtcgggattttcaggaatattcccaccggcaatcaactggcgcagcgccaaatccatgatcgtactgttatcagcttccttaacgtactggttgttaatccattccaacttcttggaatcaaatttggcaggtgacttactcaaacgagtctcgtcatacatcttgatgaattctttcttggtaaagatttcatcttcacctaccggagaccagcccaagagcagaatgaagttaaacattgcatcaggcagataacccaatttgcgatattgctcaataaattggaggactgattcgtcacgtttacttaatttcttaccggtatcagcgctgatgatcaagctcatatgcccaaatcttggtgcctgccagccaaaagcttcgtaaatcatcaactgctttggcgtattggcaacatgatcatctccacgaaaaacgtggctaatcttcattaaatgatcatcgcagacaacggcaaagttgtacgtcggcatgccatcacgtttccggatgacaaaatcaccgccaatggtatccgaattaaaggaaactttgccctttacgatatcatcccaagcatattcatggttcttgggaactcggaatcgaataaccggctttaaacccttggccttggcgtcagcaattgcttgggccttctggtcttcggtcattccttcgtattcatattcataatgaggcatttcgccgcgtgctttttgggcatcacggtcggcagtgagctgctcctcagtccggtaggattcataagctttaccctcatcgatcaactgttgaatcaatggtgtgtaaatatcttttcgttctgattgacgataaggaccataatcgccaccaacatcgggaccttcatcccagtcaagaccgagccactttagattatccagttgactcttctcgccgtcggcaacatttcgtttggtatcagtatcctcgatccgaatgatgaatttacccttgttgtgacgggcaaataaatagttaaaaatggctgtacgtgcattgccgatatgcaagtggccggttggacttggagcataacgaactcgaattgcattgtttgccaatgtataacgcctctttcttaaaaataatcaaaattttgtcagtgtttaaagtgtacaatgaacttcgccaaaaataaagggaaggcggctacttcttgttatttgacccattcttgccattccctttattctgatcaggcttatcggtaatgttcttggtcgaatgttccggacgggcgaagaccattttacctgcatctgtttgaatagcactggttacgacaacatcaatgtgatcattcaagaagtatcgaccgtcttcgacaacgaccatcgtcccgtcatccaaataagcgaccccctgttggcgttcggttccgtttttaacaaccatcacgttcaacttctggccgggcagaatcttctgccgcagcgagttggcaagcgcattaatgttaaatacctggacgttttggaattgaatcactttgttcaagttgaaatcattggtgataattacaccatcaacgtctttggcaagctggatcaacttactgtcaacttctggaatgtcctcgtaatccttctcgtaaatttcgatcggaatcagatcttcgttctgcagcttgtttaaaatatccaggccgcggcgaccgcgaacgcgtttgacactgtcactggagtcggcaatgtactgcaattcatacaacacaaacttgggaactaacaaggtgccttcaataaacccggttttgacaacgtcataaattcgaccatcaatcaaaatgttggtatccagaattttgtagtgatgatagttcttatcgactggtttatcgataatcttttcgtcgccggccttggcagtttctgacttccgccgggattgaaacatttttcgccagcgatcactctgcgtattgccaattcggaaaccaaaatagcccagtaccaacattaagatcgttggaatcatggtattcaagaagaacgtgcgggttctgaagaatacaatcgaaatcaggatggcaaccaccagcccgataatcaggcccaaggtcccaaaaaataacgacaacggactttgctttgtcaatctgacttccacccgatcgaccgctttgagaatataattgccggttaacaacgaaataaaataaaaaataattgcacccacaactgcgtttgtcgcagtgttgttaaacagcgtcccatagcggacttggaatatcagccagatcatcggaaaataactggctccaattgcggcgccggctaatgtaaatacaattctaacaattctctttcttttcaaaaatatcgccttctctcaattttcctttaaccaagtgcaagctttaaagcttgagcaagggttgaaaccccaactaccgaaatgccagttggtggattccagccctgaagattgttggctggaaccaagacccgtttgaaaccgagtttttgggcctcggcaacccgctgctcaattcgggtaacgcggcgaacttcaccggttagcccaagttcgccgacataacactccgtcgggctggtgccgcggtttttgtaggatgaagcgatgctgaccgcaattgccaaatcaatggccggctcatccagtttaacgcccccggccgcctttaagtaggcatcctgattctgcagcatcaatcccgcccgcttttccaaaacagccataatcaacgacacccgattgcggtccagcccagtggcagttcgttgcgcattaccgaaaaccgaggccgttaccagagcctgaatttcaaccaggattggtctggttccctccatggaaacaacaatggccgacccggtagcgtctttcagccgttcttccaagaagatttctgaaggattcttaacctccctcaggccgtcagtccgcatttcaaaaacgcccagttcattggtcgagccaaaacggtttttgacagtccgcaaaatccggtaggaatggtgcaggtcaccttcaaaatacagcacggtgtcgaccatatgctccaaaatcttcggcccggcaatcgcaccacctttcgtcacgtggccaacgacgaatacggtgattccctgacccttggcaatgttcattaaatcggcggtcacttctcgaatctgtgccaccgatccagtcgctgactgcagctctggaatctgcatggtttgaaccgagtcgatgacgacagcatctggtttcatctcgttaatggtatctttgatgacatccatatcggtttcggggtagacataaagattttccccattgacaccaagccgatcagcccgcattttgatttgggaagcactctcttcacctgaaacatacagaatcttaccggatttactgagctgaccggaaacctgcagcatcaaagttgatttaccaatgccggggtctccgccaattaagatcagcgatcctggaaccacgcctccgccgaggacccggttaagttcttccatgtcggttttgaaacgaatgtccttatggaactcaactttattaattgattcgggcttattgtcatggataccgtttctgcgaaggctttgggttgccattgtgctattttttggggtgatggtttcttcaaccaaggtgttccattcattacagttcgggcaacgtcccaaatatcttggggaaatgtagccgcagttctgacatacaaattgggttttaacttttgccaactaaattctcctcttatacttacactatcaatattttagcactttatgaatcaaggttgacgaaatgccggcggactttacatcatcttataaattattgacctgatgaaccaaaaccaccgcttcgggtctgttttttgcgttggtcgtcctggtccgccaacagatacggcaggaaaatgccttgagcaatccgttcgcctttcttgatcttaatgtcagtgatcccaaagttgaggatctgaacaaagatttcgccctcattactgcgattattataataatcagaatcgatcacgccgataccgtttggaatcaccaatccacgttttaatgggttgctggatcgattggcaatcacgagcacttcatcaggctgcatataggacttaatccccgttggaattaagaatggcttaagcacttttttggcctcggcaatgctgtcttcccgaaccgttttctcatgtttaagtgcccaaaggactttcaaaaaattcaatttccagatagatggaatcaccatatcggcagcactttcaaagtcatatcctgctgcgttctccgtcgttcggtaaggcaggcttaagttttcgtctgcatattttgagacaatttcaaatccacgtttcatatgtctggctccttctgtcaatatattctattattgtagtataaactatgtgaagctgtttgcacagattgacaaagatggtaaagtatcgcagtataatggtgtagtaaaacctttaaacaactttgaaatgagggaacaaatatgaaacatcaagacgagttgaagcagtctgtggggaaggccgctgttaagttcatcgaagacggcatgaccgttggtttgggcactggatctaccgtcaaattcatggtcgatgctttgggcgaacgagtgaagtccgaacacctctcaattgtcggtgtcccaacctcagaacggacccgtgaacaggccaacagtctcggtattaaaaccaagggattagacgagattgaccatattgatctaaccatcgatggcgctgacgaaattaaccggaccttccagggaatcaagggtggcggtgccgctcatctttgggaaaagatcgtggcaattaattccgataaaaacatgtggattgtcgacagcagcaaaatggttgatgagttgggttcattcccactccctctagaagtcatcccttacggcagccatcaactgcttaaacgccttgatgccaaaggttatcacccaaagtttaggatgaatggcgatcagtacgtcaaaaccgactccaacaattacgtgattgatttgcacttaggccaaattgaacggccccaccatttggcgcttgaattagaccaaatgaccggaatcgtcgaacatggactgttcctcgacctggttaacacagtcattgttggccgtgaagatggaccgcagaccattcaagcccgctaattgaataaaaactgacaacagccggaaatgcgatcaaaacgattcgcagccggctgtttgccgtttaaaagcaccctgctcactagccctttttaataaatgagcgtaaaataagattctattaaggagagtgatcatttttgacagcagaaattaatttagatcaaatcagcaagtaccagaagaatcttgataatcgaaaagattcgaaagtgattgaacgggcagttacccatcagggcattttggaaagcagcgaggactttaccgctgaaggcaaaatgagcccggtattttcaatcgatctttcaactggaaaagttgctgatcaaaagcaaagtggtcgatgctggatgtttgccgccctcaatacgatgcgcattcacctcatgaacacttataaagttccggatgatttcgaactatcccaaaactacaccaacttctgggataaatttgaaaaggccaattatttcttggaaaacgtcttaaaaactgccgaccagccgctagattcacgcaaagttgcctggttgatggcaacgccacaacaagatggcggtcaatgggatatgctttgtgccctaattgaaaaatatgggatcgttcccaagtcggcaatgccggaaaccttcaacagtaatcgctcatctcagctcaacaagttcttgaacctgaagcttcgtcatgacgccgttgccttacgtgaattggttgctgacaaggcatccgaagctaagattgccgaaaccaaggacaatatgatgagtgaagtataccgcatgttgacctacgcactcggtgaaccagccaccaaatttgacttcgaataccgcgacaaggataagaattatcactttgacgctggcatcaccccacaagaattcttcaaaaaatacgttaacttaaacttggaagactacgtttccctgatcaactcacccactgatgacaagccattcaataagacctacacaattgaaatgttgggcaacgttgtcaatggccggccggtcaaacatttgaacctggaaatgtctgaactcaaaaagttggcaattaaacagctgcaaaatggcgaatccgtttggttcggaagtgacgttggccaaagttccaacaccaaaaaaggaatcatggacaccagcctctacgcacccgacgaattattcgattcagatttgtcgatgtcaaaagctgaacgtttggattacggcgaaagcttgatgacccacgccatggtgattaccggagtcgatctggtcgacggccaaccaaccaagtggaaggttgaaaacagctggggcgaaaaagtcggcaccaaaggctacttcgtgatgagtgacgactggatgaacgaattcgtgtaccagttcgtgatcaacaaaaagtacctcaccgacgaacagcttgaagcccaaaaacaagaaccaactgttttgaagccttgggatccaatgggtgccttagcctaagaatttgttcttaaatgataaatacgacaagtcaggttatctgatttgtcgtattttttatggtctattaaattgcaacgaactactccatgaacgatttactgataatgtttaattgctcatcaaaatcgtatcgaatcggcttgccgttaggaacctccacgttggggatttcttcatctgaaatattttccagaaatttgatcaaagcgcgtaaggtacttccgtgagcaacaatcaattggttcttgttgtctaacaagttcggcgcaatctgatcaacccagtatggaatcaatcgctgttgtgccatttccagactttctcccaatggaatttggacaccgtaacgctcataacggggatcctcgtcccgcttggtcaaaagcggcggcacaacggtaaaacttcgccgccaaattttgagctgctttgcgcccactcgttctttgactttaagtttatttttcccacgaaggccaccgtagtgacgttcgttaaggcgccaggatttatgctcaggaataaagttttgaccaatttcatccaagacaatgttggtggtaataatcgcccgtttcagaaacgacgtatgaacgtcatcgaactgaatctgagatttggcgatcactttcccagcactgtgagcctgtcgaacccctttatcggtcaaaggtacatcgctccagccggtaaaaatgttgtcccggttggcttggctttctccgtggcgcatgatgactagtgtcggcacgtttacatcctctttgctcaaattaatttgttcacaaataaatccataaaaaagatgaccgaagccaccttctaatcttctcaacctctcaagtcgttgtgtgaacagactcagtgtagcatttctcctaaagcttctcaaccaaaaccattagaaccggaatcatgatcagactcaacaacgtggtttcagccaccatgattgaagcatattcagaatcagcatgatacaacctggaaacaaccggcgcattggtcataatcggcattgcagactgcatgatgaaaacttgtttcatcatcaccggcattggcgttggaatgaccaatagcgacataatgattggggccagcataaaccgcccaaacaaaatcaagaagttgctgcggtcaaaatgaacgttagttaagtcaacactattgatggaaattccaataaaaatcatggacagtggaatcgttaaattccctatgtaattaaaatcctgcatcaaaaaatcaggcagggtgacgtgcatcaataccaatacgacaccgaccatgaaaccaagcaaaggcggtgaaaaaaccttcttgagggtttgcttccaattaaatgaagcctcacctttgccatctttttggatcaaataaacccccagtgtccaaaagaatgtcgtgttggccatatagtagaccaacacaaacggcaaactggattttccaaacagcgccatgttaaccggcagtccaacaaaaacggtgttcgagttggaaaacatggacatgaacaacccagaatgcattttggggatcttggcaaatttgaccacaaagattgaaacaatgtagagtgacagcatcgaaacgattgggaaaaataagtcaggaagtgtggtcagcagcttcttggcagtaaatttttccataatggttgaaatcatgtaggccggtagggcaacctgggttaccaggcgcgcaatcatgctggtcatcttaccgtcaaaccaatcgtttctggctaacacaaaccccaaggcaatcataatcaggataattaaaaccccagaaacagcattataaaaaacttccataaacattcctcaattctaaaaatcaataacaatgaattattataacacaattagaatccacagccggttataatttttggtataattgaacaagttggtcacaacagatgttacaattattaaataatgtttaaataaccgaagatttctgcaatcaagtccaaatctgccatatacttttgggagaattttttgtaaatgaggagtcaatatgccatcagataaagataacaataatgattttgaaccagtgtattctcgtcgatcggacaagaaaccccactataagaaaaagaaccaccgtcgaagaagaattatcggctggagtatctttttcgtcctgctgatcgccttgggcggtggcctggtctggggatacggcgcatacaagagtgccaagtcgaccttcaagaagacctacgattcaaccaatgttaccaaagctcgaaacgtttcgtcagtgatccagcaaggaaagccactgtcaatcctgctattgggaactgatacaggtgccttgggtcgtcacgacactggtcggacggatacgatgattgtcgcatctgtcaacgcaaagaaaaagaccattcatttgaccagtattgcccgggacaccaaggtggtcgtccccggcgacacccagccatatgaaaagattaacgccgcttatacaattggtggcgccggaacagccgttaagaccgttcaaaatctgctcgatattccggtcgacttctacgcgatcatcaacatgggcggtttggaaaaaatggtcaatgcggttggtggcgtggacgtgaccccaccactgacgttccagtatggggctgcaaatgtcgtcaaaggcaagaaaatccatctaaatggtcgccaagctctggactactccagaatgcgtgatgacgatccacgtggtgattatggtcgccaggcgcgtcaacgacagattatcaagaagttagtcatgaaggggcttaacattacctcccttccccgttacaaatcaatcctctcgtcactgtccggcaacatgaagacggatatgactttcgacgatatgatcgccatccgggcaaaatatggcgacgccactcatcacattaagtcacaaacccttcagggagaaaacgcaatgatcgatggtctttcctaccaagtggttcctcaaaacgaactgctgcgggtttccaacgacattcgaacatcccttggcttggcgaagtcaaccaagcttcaaaccagtcaaacagataccgatgacggtcaaggggcaacccaatcatcatcgacatataatggctattaaataatcatgaaccataaaatagcggctcagataaaagcaaaccaacttttatctgagccgctattttttcacaatcaattttatgtaacttttgctttttaaaccaataccccggcatagtagccaagaactccgataacgaatagccccagaataatccagattggcgaaattcgcctacggatcagccagacacaaaccagggtcaaggcaaccggagcaatcacgttaaggccgccattaatcatcgtgtccacgaactgggaaatcgttgaactgccaaagagtccccgaactgatgcaaaatcaacggtgacccaccgagcaacaatcacgcccatcataaagacgccaaacattgaagtggcgctcccaacgtacttaataatcccggtattaaacaggttaataatatcggctccccgacgataaccggccatttgagtcatataacgaaagaccagccgtaaaacgttccacgcaataaagaatagaattggtcccatcatgccatagccactcaaaaccagactggcagcaaatgccgatagaaccggacggatcgtgcctaaccaaaccggatcaccaaaaccacccattggccccatcatagcagtcttaacggcattaatcgtgtcatcactaatatcggcaccatttgcccgctgttcttccattgacaaaaccactccagtaatcagggactgcataattggtgcggtgttaaaaaagcccaaatggcgcttcaacgcagctttacgttggttcatatccggatacaatcgtttaatcgcaggcgccattatataagcaaatccgaggttttgcatccgttcaaagttccacgatccctgctcagtgccagagcgccaaaaggtccggaaaaaatcgatctgacgaagatgaatcggttgatgggaatcgtgaatcatattttgattatttgccatttatacccaccaactcctataaatcatcaagttctttgtcaaagtcatctaaatcgtctttaccttccccatcgccgccggttgagccatgtcgtctactcttaagccaaacaaagctgatggccgcaaccaagcctaatcctgctaaaataaaaagattaatcttcgtaaaaatggcaattaaaaaaccaacgataaaccaaatccataaagagcggctgaccatcatgttaatcaggttggcgaatccaactgccgacaccatcccaattgagatggcaatgccatttgtgatccccgctggaatttgctgcattaactgatgaatcaattgaggagatatcagcatcacgagtcccgtcggaatcaggactctcagcccttgaattcccaagctcagcagatgaatgcgatcaatctgctggatttgaccattttcggcagcttggtcggccgtatggataaatttgacaattgatttacggatggtgacgttcaaaagttggccaacaaccgcaaagggaacggctaaggcaatcccgtgtttaatacttaaggcggccggaccgcacactaaaagagccgagacgactgccggcagcgcgatatccggtgcaacagaagcaccaatattgatccagccaatcgtgatcatttgtaaaattgcgcccagcataatgccaacaccgacgttgccaattgccaaaccgatcagcgtacaagcaatcattggctggtacacctgccattcgtcaagaatgccatccattccgaccacaaatgcgaccaacaaaaccaggctggttgaaactaagctcattgaattcccctcggttccttaaaagccctttttatccaacagggtcaacaaattttcctttttttcagcaggaattttttgagcatagacatctagatgaaagtcatttgccaatgttcgaatttgtttggcgatatctccattcatcgaaatggcgtcggtaagcatcgtcattccgtcgttataggcaatgctgccgatattgatgccaatcttggaaaaatcgatgccgccttctgctaatttcaacatgtcagccaccgtttcggtcaacaacaacgtgttgaaggaatcaaacctggagtcgaaataggctcggatcatcttgttaacggtgacgacattggctttgacaccaggcggtgccacttgggtaatcaatgttttccgcaaaggatctttggcaacagaatcagagaccaccataatccggttcggcgtcaccgcccgtgtccaaaaagttgccacttggccgtgcagcaagcggctgtcgactctcgcaaggcgaatatccattgtcattataaatcatctcccaaatcgtcatcattatcagtagaaacttcaaactgacggatcgaatcgtcagcaatctcattgatcttattaactaattcactcagggttgaatttcgggccatgtaggcctccaatagaatcggcaggttgactccggcaactaatgcaatcgattgcggattcttggctgcaaattgggcggcggcattaaacggcgacccaccccacaagtctgccaaaatcaacgttggcgtgtcctcaggaaagtcagccaatgcagaagcgaccttatcactaagcgaatccaccccgtcatttgcggccagacttacccaaccaacctgttcctgtttgccggcaatcatttctgcggtcgtcactaagcttttggcaaaattgccgtggctcacaaccagaattgaaatcatctactcacccatttcttaaatttgacaaagtctgttcacaccaaatatatcacaaaataacaatttcgtttgccggaattactgaatagttagtaagtctgcgggcgtctttaaatcgtaatccgtgtccgcaaagtccgcggttttcttggtccgccaaccggccagggcaaactgcacgttggcagcgtgagcagcttggagatcaaatttggtatcgccgatataaatggtggctgccggatcagcgtctaatttctcaatgccctttaaaatcatgtcaggagcaggcttgccttttttaatttcgttggaaaaaacaaaggcatcaaagtattgatccagtccaaattttgtgacatcccggtgaaattcagcttcaaccttggaagtggcaatcgcggttttgatagtcggatcagcatgcagtttcttaaccacatcctcaatcccatcataaacgtgggcatattgggtgtaatctttaattttggcaaaccattggtcccgaatgtcaaccgggttcttgacaccaagaattcgaaccgtgtccatggaggtaatcccaaagagcttaacgacatcttcataagagaagtcatagccgttttctagcagtgtcttatgtagtggtaacatatacatcttttcggtatcaatcaaggttccgtctacatcaaaaataaaatatttcattcctgtactccaatcgcttattatttgagcaaaatatcacatgctacacaataaaaaagtccgaatcactattgagatgatagtgattcgaactttaaccatgcggccaagaagattcgaacttccaccgggataattcccgacaagatccttaatcttgcgcgtctgccaattccgccatggccgcatcaacaattaaaaattatagcagaaattttggcaattgacaaatggtttttgaaaattattcaccgcgaacggtcgcgccttctgtatcaatttgcagcagccgcaaactaccatttagattttgttgtgccaaatcaattcttaactgggttaaagcagctttcttacccagtgtggcaaccgtaggaccggcaccactcaagtaagtaccaaagatgtctaacttgtgggcagttgaacggatttgatcaatttctgggaccagctcttttctgtagggctcgtggagatgatcattctcaatcagcttaaccgcctgctcccatttgccctgggcaaccaaggcgatgaaaacattctcctggctgctggcatggacggccacgtcataatcgatttgtttcggcagcttcttgcgactttctacctcgctgacaccatccggtcgaatatacattaaggccgagacgtctgggacaggaagagtcgcagcagtgacggtttcaccgtcatatgtcgaaacaaccaagttgccaagcatcgcagcagcaacgctttccgggtggccttcaatcttagttcccaaattaatttgatcttcaattgaaagccccagatcccctaacttgttggcaattttaatcccggcaaccactgcggttgtgctggagcccaaaccgtgcgcaatcggaacatccgagataacggtcagttgatgcggatgaatatcagaatcgacctttaagattgtctgaacaatgaggttgtgctcatcagttggaatgtcgtgtcccaaagcatggttgaccttccattcatctgtcttttcctcaacaatcaccgtgtaatacagctgcagtgccaacccaaccgaatcaacacccgacccgaggttagtggtcgttgcaggtactctgataataatttttgccatgtgatggctcctttctacgctccgatttgccgcgtttggctgattaaatgaagcttaccgcgacatctgccgcagacatacttcaccagattgattcttcgtcttctatgatactccaaaccgcagtcttcacagcgataaatataacgcgtttggaccctggtactctggactctgggagcgtatctggagccgccgaccgcttttaacagctgtttaaactgcttggtattgtgtttggcgctgtatcctgccaaatggagatgataatggcaaagctcgtgtttgataatcccaattaataccgcatgatcagccccgtcgtccatttttggattaatgtcgatgttgtgatcattgaggtggtaacggccgccagtcgtctttaaacgggcattaaaataggcccggtgggtaaacggtttggcaaagtattgcagcgaaatatgttcaacgagttgctgtagttcttgatcagtcatgagttctttgttcacctaaccttcaggatccaccatggttaattgaatccggtgacgatccagatccactgagtcaatccaaacggtcacgatgtcgccgaccgaagccaccttgctgggatctttgacgaatgtccgactcattttggaaatgtggaccaaaccgtcctgcttaacgccaatatcaacaaagacaccaaagtcaaccacgtttctgacagttccctgcagtttcatccccggcttcaaatcttccatcgtcaaaacatcttttcgaagcaacggcgcaggcatttcgtcacgcaggtcacggccaggcgtttcgaggcccttgataatatctttcaaggtggcaaccccaactccaatgctttcaacttcctgagccaaattaagctggctcaaagcacttgaaacggccggctcgccgagttgattaatggtcaatccgtgctttttcaggaggcttttggcggcagaataactttccggatgaatatcggtgttatccagtggatttttgccgccgatgattctcaagaaccccaccgattgctcaaaagctttcgggccgagccggggaacttgtttgagatcagagcgggcactaaattcgccattttcatttctgaatttgacgatattgccactggtcgttttggtcaacccggaaatgtggaccaacagatcgggactggcagtattcaaattgacgccaacccggttaacggcagtttcaaccaccgtgtccaactgttcacccagttgtttctgcggaacatcgtgttgatattgaccgacaccaattgcctggggatcaattttaacgagttcagcaaggggatcttggattctgcgggcaatactgacagccgaacgctgttcaacactaaagtccgggaattcgtctctggcgacttgacttgcagaatagaccgacgcccctgcctcattaacaattacgtaataaatgggcgttttgatttctttaattgcatcggcaacaaattgttcagactcccgactagcggttccgttaccgatggcgatcatttcaacgtgattttggttgatgaaatcaatgaacagccctttggcagccttacgtttggcttcactggcgggcttatggggatagatcaccgttttgtccaaatacttgccattttgatcgaccaccgctaatttacagccggttcgataagccgggtcaaatcccatgacaattttgcctttgaggggcgcctgcatcagcaagttgtacaaattcttgccgaagatatcgatggcgtgatcagcagcgacttcggtcaactgcttgcggatttcacgctcgattgccggtccgatgaagcggtgataggcatcttcgattgcatcggtaaccacatcggcagcaaatccttgatgactgccgacggtgttggcctttaaatgccacatgattggtgcctcattgacttcaattttgaccgaaagcactttctctttttcaccccggttaatggccaaggttctaaacgaaggaattgatttgatgggttgattgaaatcgtaatactgctggtaggtgccttcttcgtccaactctttaccaccgcgtttaactttgacgaccaactgaccgtattgttgggtgttttggcggacccattcgcgaaaatcggcccggtcgccagcgtcttcagcgataatttcgtggactccggcgaagactgcgtcaacatcaggcagttctttgtccgggtcaacatactgggcagcctgttgcttcaaatcgggggcaaacgacatggcggatttggctaagggctccaaaccatgttctttggcaattgtcgctttcgtccgccgtttttgtttgtagggcaaataaagatcttcaacttgctgaagaaccgaagccgcctcaatctgctttttcagttcaggggttaaggcattttgttcatcaataattttgatgacttcctgcttgcgcttgtccaaagtttggatgcgatgagcagcgtcttgaatgtctcgaatttgaacttcatccagattggaagtccgttcttttcgataccgggcaataaaaggaacggtgtcgccttcatccaacatcttgagggtttcgacgatttgtttctcccggattttgggtaagtcttgctgaatcttatgtgctaatgtgttgtccatgtatttccacctcatcaatagtgtcacgtttaattatagcagaatgaagcaaatgccggggactccaaccaggttttctcaggaacataaaagcccaaactgctggcaggaacacttgtctgcagtttgggcggaatgttgaatgttaattttttaattttgggagctcctgttgtggagtgggtttctggttggttggtttgaggaaacgtgcttcgatgcaactgacactgcgatctaagcctctttgatttaaacccaaacccgggattttaatcaaagcgaccttagctctccgtgtcaaagcattgcttgtcgcactctggttgaaacgtgcttcgcgggcctgacgctaacctctaagccaactttgatttaaacccaaacccggggttcaaaccaaagttggcttagaaaccgcgtcacccagcccgcttcgcactctttaaatttctcccataatccgcgtagtcgtactggaaaccttagcgatactattttcctgatccttctcagcttggttgaacttatcaacgtccaccgttgaagcctgcgggtcaatactgtccgtcattgcctggcaggcgttggcatagtcctcataatgacgaaccagcaacttgtgcttgcctaacaatttaaccggcacagccacctgctcaagcttgttcacgttatcttggtacttatcggttccggattgaaaatgggcttgaatgcccgccagctgatcactggtcaaatcagcaaccgtttggttatcaattgcctttctgagtgtttcataatcggcgtttaaatcctcaccgttttttgacgtctcatcaatcacgtccgagacggtttttgcatatcgctgcatatcttgtggtttcaaaatatcagcctccattcaattttatttatgggaaatgtgtctctgaatgtattttactacttctgaaacaacaacgatcataaagccaccgaagacgacgaccagccactgtgaagcggtcaactcagtcacgtggaacatctcgttgaatcctgggatgacaatcgtcatgatcaacagcacggccgatcccaaaagtgcccagttaaagaatttattcttaaacatgccaattctaaagattgactcatggatggtcttcgagttaaaggcatggaacaattgaatgagtcccagagttgcataggccatcgtcaaagcatccgcatgggccaacgcatctgaagcatgaaccgggttggtgatggcaaatgcataaacacaaagggtaataaagccctcaaaaaatccctgatacaagatgttgctcatgatcccaccggacaagaagttggacgttcgtcccctgggtttgcgtttcataataccgggttctgccggctcaacgcctaaggcaattgccgggaatgtatcggttaccaggttgatccacaaaatctgaaccggcgccaagatctgccaacccatcatcgtcatcacaaacaaggtcaagacttcccccaagttggcggaaagcagatactggagtgacttttgaatgttggcaaacaccttgcggccggctttaaccgcagttacgatcgtggcaaagttatcatcggccaacaccatgtcagaggcttctttggaaacctcggttccggtaattcccatgccaacaccgatatccgcggtctttaacgctggtgcgtcattgacaccgtcgccggtcatggcaaccaccttgccctgtttctgccaggctttgacgattcgaaccttatgctccggtgcaacccgggcgtaaacggaaatgtcagcgacttcccggttaaattggtcgtcggacatctcatcaagctgagccccattgatgacctttccgccaggattgtcaccccgacccaagattcccaaccgtttcgcgatcgcttgggcagtatcttgatgatcgccggtaatcataatcgatttgattcctgcagatttggcttccgcaactgcttgagcaacttcgggccgttcaggatcgatcattccgatgagaccaacaaagatcatatcgtgctcctgggcggctgatgtgagctcagttggtaccgtgtctacaagacggtaggcaaacgccaacacccgcagcgcctgagtcgccaaatcatggttggtgacactaattaaccgtttgtcatcgtcagtgatgtctcgaacattgtccccatcttgaatcttggtgacccgttccaacagctgatctggtgcccctttcatggtcattaggatttggccatcgtccatttggttgtaggtagacatcaatttccgctcagagtcaaacggaatttcggccagtcgccgatgggaattgacaaacttttggactggctggtcttgatgtaagtaaaacgacaccagagcggtttcggttgggtcaccagccaactcattttcttgatatttggtgtcattgttcaaaaccatgatttgcgctaatcgatcgtttaaagttaaatgggtgtcagcggaatcttgcagtttttcattcaagaagactttttccactgtcattttgttttgggttaaagttccagtcttatctgaggcaatgacatcggtgcttcccaacgtttcaacagccggcagctttcgaatcaaggcgcggtggcgggccatttgctgggttcctaatgccaacgtgacggtcacaatggccggcaggccttccggaatggctgcgactgccagggaaatcgccgtcagcagcatgttaatcaagctctcttgtccccgccacatcccgacagcaaacacgatgacggcaatcaccagaatcaaaacggttaacatcttacctaatgatttcaggttctcctgcagcggcgtggtggtttcttcagtggtgtttaacatatgggcaattttgccgacttcagtattcatccctgtgccaatcacgacgccggttgcccgaccagacgttacgttgctgttcatgaagcccaaatcctttcgatctcccaatggcaggtcgtcttccacgattgggtccacctgtttgttaaccggcacagattcgcctgtgagggccgcttcttcgatcttaagggaattagcctcaatcagtcgaacatcggctggaacgacatctcctgcctctaagaggacaatgtctcctgggacaatgtcctcactcttaattgacatcggttgattatttcgcagaacggtcgccatgggtgccgacatttcttttaatgaatcaatcgcattttcggccttggattcctggaaaaccccaaacaccgcgtttaggataaccacggccaaaataatcgcagcatccaccgtttcaccggcaaacccggcaataatcgcggcaataatcaagatgatgatcatcaagtctttaaattgggaaatgaacttctcgattaacgtggtccgccgctttgacgttaatctgttggcaccaaattgttcccgacggtctttgacctcctgatcagacagaccagtgggatgggccttcatttgactcatcacatcatcgactgttcgttggtagaacatcttcttctcctgtgtcataaacttcctcctctaaaagaaaagagacccacaaattcctcgctaaaagaattcataagtctcaccatttaagatttatcccggaaatacgagtatttcacgttgacgagataatcgcaatcgaaattgctggttactccctttatttatggtaattatacctaaccactaatgaaaagtcactaaatatctatttccaaaatgtgtcataaacattaatcggggtgtgacgtttgtgttgcgtcttatcataccagctctcaatggtctcggcagccttctcagaaacttcgcgaccttcaagataagcgtcgatatcctgatacgtcacacccagggcaacttcgtcgggcaatgctggtcgattatcttccaaatcggcagttggcgttttttggtaaagatgttcgggggcaccgagtaattttaagagctgcttgccctgctctttgtccaaacgccaaagcggcgtaatgtctgctgctccgtcaccaaatttggtataaaatccggtaactgcttcggcagcgtgatcggttccaaccacggcaccggatttggcaccggcaattgcgtattgggcgatcatgcgttgacgggctttgatattacccttgttaaaatcggcgacttcgatatcgtttgcctcaactgaagccactgcggcgtcaacagccggcttgatgtcaactctggcaaccacatcggcgtccatccacttgatggcttccaaggcatcagactcatcggcttgaacaccatatggcagacggaccgcaatgaactggtagtcaggatcgccggtttcatcccggagctcggaaatggttaattgagccaatttgccggccagcgttgagtcttggccgccagagatgcctaagaccaatgtttttaggaaagaaaattttttgagatagtctttcaaaaagtcaacggaacgacgaatctcggctttgggatcaatcgttggtttcacttttaacgcgtcaataatttcttgttgtttagctcgcatatgcatccctcgattacaaatttagtagttgatatcttgaatataattgcgaatcttttcaatgatgtcacgcttgttatcccaacacttttgtgacagatcgactggatacttttggggatttaactcccgtttgtattcaggccacaatgatgccaattccttttcggcgtagtggacaatctgctttaagtttggctggtcatatactaatttgccgtcttgaaaaattggtttgagtagtggcattgcatcaaaattatcgacagtcttattgatgtaagtatagttgggatggaacatgaagatcgacttttcttttctgggatcttcatcggccagtgtgacgtaatcgccttccgacttgccgtctttactgtcagtaatgcgccaaacctgttttttgccgggtgtcgaaaccttctcagcgttaccggaaatcttaattgtatccgtcattttgccgtcagcgtcttcaacggaaaccatcttgtaaacagcgcccaaggctggttgatcaaaggcagtgatgactttggtgccgacaccccaaacgtcaatcttggcatgctgcatctttaagctggcaattgtcgtttcgtccaagtcattggaagcatagattttggtattcggataaccggcattgtcgagaacttcacgtactcgtttggaaaggtaggccatgtcgcctgaatccagtctgacgccggcaaaattgatcttgtcacccatttcattggcaacccgaatagcactgggcaccccactttttaaggtgtcgtaggtatctaccaggaacacgcagtcgtgatgggtctgagcgtaggcattaaaagcgtcataatcattaccaaacgactccaccaatgaatgagcatgagtcccgctgattgggataccaaacttcttaccagccaagacgttggaagtcgcgttaaaaccgccaatgatggttgcccgggttccccaaagggctgctgaaacttcctgggctcggcgggtgccaaattccatcaacggatcgtcaccgaccaccgtccgaattctggaagccttggtcgcaatcagcgtttgataattgaccatattcaaaatggccgtctcaaccagctgacattcacacaagctcccctcaacttggagaattggttcattggcaaaaacaatatcgccttcataggctgatttgatggtgcctttaaattcaaagtttcttaagtattctaaaaaactgtccggataatctgtcacttcgcgcaaataatcgatatcatcatcagtgaattgtaaattttcgatgtatgaaataatgtgttccaagcctgcaaataccgcgtagccgttgccaaacggcagcttgcggaaaaacacttcaaaaaccgccttacgattttccatatgcttttcaaagtaggtggccatcatgttgatctcataaaaatcggtatggagcgttaaattatcgtcttctgacatattgtgtcaatatcctccccggagatttgttatataattagtttatattctatcatttttccgattattaacaaaaaataatcttgcaattcgcatgaaacaaagtctaaaggagctgctatgaataaccaaagtcccacccaaccagttgatatcttgggcatcccttttgaaaataccaccgaaaaggatttccaagcaattttacataacgtcatcaatcaacaccaaaatacgtttgtcgtcaccgccaatccggagatcgtcatgtatgccaaggcgaatcccgattacgaaaaactcattacgaccgctgactacatcgttcctgacggtattggcattatcatgggtgccaagatgctcaaaacgccgctcaaagaacgggtgaccggatatgatctctttgtccatctactggaatggggaaacgccaaccaaaaatcggcgtactttgtcggcgctcagccagcagtgattcgcaagctcaaaaaagtcgtccaggaaaattatccgtttctaacgattgccggcacccacgacggctattttggcgatgatcgcaacattgtccacgatatcaaacggacccagccggatatggtctttgttgcaaccggttatcccaagcaagaagcctttatcaataaaaatcgacgggctgccgacgccctttggattggaattggcggttcatttgacgtcttagccggaactgtcaaacgagcacccaaagcttggcagaaaatgcatttggagtggttgtaccgggtcgtcaaggaacccagtcgctttggcaggttgatggtgctgccaaaatatttgtggcagatcgttaaacaaaaatattcaagaaaatccaggagggctcaatgaagaaagtttcaccgaagttttggacctattttctaattatttatgtcggcgttggcatcattgttaatttgctccatcatcaggcggccattcaagacacccagtacggtatgctgggaatctttgcgctggcttatgtcaccagttatctgcggatgcccagattaaacttctatgtgatttactttgtgctgtggatggtgattcttcgtcaaattggcggttatcgtgattggacgtcttggattatcttcgcgtttatgtctgctgtgatggcctgggtcaccgattggattcggtccggctatgctcagcggtacgatcggccaaagaagaaaaatcagaaaaaacaatcataggacgataaaaccaggccaacaaatgtgatggcctggtttttgtgtgaaaagtttttgtgttgctggatttgtccgcttgggggacggctccgacgacccagatgctcacttctaaggggcacttggtatatggcggccgcctatctcgttactcggagatattatgtcaccttgtggtttagtcacttctgaggacggctccgacgacccagatgctcacttctaagggtactgggattcaaatccctcaaaaccggtatttaaatcccagtacccttagaaaacgcatctcccgggtctcgtcgcccactactctttttccaaataaaattcaaaccgatcgcccacatattgggtgcggacatactcgaacgggcgaccgtcttgaagtgaagtaatctgtctgagtctcaaaatggcatcgcctcgtttgatgttcagatattcagcaatccgctccgatgccagcatcgccgacaccgtctgctgggccttgccgatttgcaggttcttcttttgctccagggttcgataaagcgaactggttacttcggatttttccaagccctcgacaatattttcaggcaccgtggcgacttcaaagcaaatcggaatgtcgtcgccataacggattcgttccatccgtaaaaccgcttgttcctgactgatgtgtaatttttccatctcgctcaaagacggttccatcgtgtgatacgaaattgttttgctggaaggctttttcccctgagccagcatcagatcggtgaagccggtaaccccagacattttctcctgcactttctgattggccacaaacgttcccgaaccgactcgacgctctaaaataccttcgtccaccaaggtttgaatggcttgacgcaacgtcatccgactcacaccaaagtcggtcgataactcacgctcagagggaatgcgatcaccaattttccacctatttgcttcaatgtttcgtttaatctcattatgaatttgaatataaattggtaaacccactgataccaactcccttagtttttattcactaatttgccataactatacgttgccataaggtctaggtgattgtcaaacaaatttagatcggcatcatacccattctcaatgaatcctttgcctttcaggtgaaattcctccgcctgattggtcgaggtcattttgacggctgaagcaattgaacaatcggtaaattgaatcatatttttaaaagcgtccgcaaacttgagaaccgatcctgctaaatggccattagccaaggttgcccttccccgaaaaacattgaccggttggccgccaagctgatacatgccatctggctgccctttggcttccatggaatcagtaatcagttccagccgatcggggccaatggtttgataagcaatttgtaccgcttcaggcaccacatggaacccatcacaaatcaactccactttggcttgagaaagcatcgcataccccaccacaccaatttctcgctgatggagacctcgctgggcgttaaataaatgggtaacgtgcgggggcagagcttgattaagcaactgataggttgcatcagagtggccaactgccatttgaatcccgtgttctcgacaataactgacggctgttgggtcaacgcgcatttccggagcgtaggtcaaaattttgaccagcccacccgagagagtattccacctggtaattttatcaacgtcaagcttttgaatcttttccgttggctgggcgccgtggtacttgggtgaaataaacggtccttcaagatgaatacctaaaattcgcgggttggtttcagccgccattttaatcgtctgcatgctcttagcaatggcatcggcactttgagtcatggtagtcagaaaaacgccggtaaccccctcgtgggccatcaggttgacgatccggctaataacttgaggatccaaattcatggaatctgcaccataaccaccatgggtatgcacatcaatgaagccagggacaattgtgcgttgagaagcatcgatgatccgatcacttggctgctgttcaaaattagttattgggccaacgttgagaattgtttgaccaaatctgatgtagccgtcttgaataattcgtttacctgtatagatctttgcatgaattaatactgttgacatatctgctccacaagtcgactaatggttaccggttgacttggcaatcgtcgcgtcaattcccttgatgacagaaggtaggaatccagcctcttccatcgccagaatgccggcgatagtatcaccacctggcgaactgactttatcaatcatttcagctggcgacttcttggatgccatcaatgagtgcgcagagccgagagttgtttgggcagcaatttgggtggccatttctttggtgaagccatacttgaccccggcccggctgagactatcgataaagaagtcaacgtacgctaccgcactaccggaaatggcgctgaataccgaaaattggctttctttaagctccaacacacttccagttgcttgatatagcgagatggcttgggcttttcgatccccggttaagttctcgttagccgcaacagcggtcatcccctgaccgaattcagagttgatatttggcagactgcgaagaattggcaggttgtaatcggtcaactcttctaatcgatccagcgaaacccctgaaacaattgagatcaacgtcttcttggctgacagtgcaccacggatttccgccaccacatcggtgacaacggctggtaccactgccaaaaccaccagatcactgccgtcaacaaccgccgtgttcgattctttcggggtcaggccatattgagccgcatatttttcgtaatgatcttggtgagcactgtgtaccaaaatgtcttgagcaggaacaaattctgctttcagcagtccttgaatgatcgcttgagccattgccccaacgccaataaaaccaattttcataagctacctcctgaatttacaatcggactattccaattcttctaacactgacaatagcggaaaatgcaaaattttgcaatatcaaaatggtcgatcgttgaaaatacaaaaaaacgcccgcgacgagttcctttcgtcacagacgtttagtaattgggctagctgggttcgaaccagcgcatcacgggatcaaaacccgttgccttaccacttggctatagcccaaaaataaaatggaggggagtggattcgaaccaccgaacccgaaggagcggatttacagtccgccgcgtttagccagacttcgctacccctccaaaagagtgttgctatcaaaccaacgaatataataatacaaaattttagtgattccgtcaagcgcaatcatcaaaaaatttggaacattttcaactgctttgcccattcagatatgaaatcattcgtctgccactcattgtgacgatggttgtggtatcccaccgctgcattatagtatgtcgtcgccttaagcctaataggcaccagtcgttgatgaatatgcccgaaaacgacccgttcaacctgatagttctcaatcaatttttgaaaatgcagactgcccatcatggcattggccatattccagaagcgaaaatcattcgtataatgaatgaagtgttggttgggaacaaagtgagtcatcaaaatcactttcttgcccgctgattgcgcgttctggagctgttgggtcaattccgaaaggactatctgctcccgttcaggatcgctcataggctgcgaaatcagcccgtctatccagtaagccattttccaacgatgaaattcatcttcagttttatcttcattcactgcaaaagtgtagtcataccagccgttcatgccaataattcggtagtcggtttgagggacgtcaaagaattgattgttcagataccccggccactggccattttccaattcatcataactgacacctttgatcatgtcgtgattgccggcgatgaaaaaaactcggattggatcaacggctgctgacagctgctgaacgtaatccaccgacttctgaaaatcattgaatagatcgccggcaatcaggtaatcgtctaccccttggtcttgcaaaaaagttgcctgctgtttaattgtatcggccagtgtcaccttattcaaatctaagtgattatcactggttacggcaatctttaccatcacgttttctccccaaaataaaaatgtgctatccaaattaggataacacattcggtcgttcttgaatctaattgacaccttccattaaccgcttaattggtttaaccaggaatgccaacaaaactccggcgacaattgcaaccagaccaacgatcaagaagtaattaatttcattgtccggtgtatagtatttaacaatttgtgagttgaccgcttgaccagctgaatcggctaagaaccacatactcatcatctgagattcaaaggcttttggtgccagtttggtcgtaacagagagtccaattggtgaaattaacagttcagcaatttccacaatggcccagcttccgagcagccatagtggactcacttttgcttgtgcgccaaataaggcaactggaatcaccataaacagataggataatccggcaatacctaatcccagtgaaaatttggatggtgagctcggctgctttttgccaagtttaatccacatccaagcaaagaatggcgtgtacagcataatgaacagtgggttcaacgattgaaaccaacctggcgaaatattgaaaataccgccaacattattattcgtttgggttccggcaaatagtgccaaaacaacggatccctgctcttcaattgcccagaagatcgcagctgcgataaacagtggaatataggcaacaactcttgagcgttcggtggaagagatttttttgcttgaaataatgacaacaaagtaaataattggcgtggccacggcaatgatactcagcaaggtaataaatgagctgagtgataatgcccccatgacctgcatgagcaacaggatcaagccgaagacaaccactcccaaaccaacccggatagtcaatttcttggcatcgttgggttctaatggatcgcttggatacaggctggcactaggcaaatgttttttgccaccgcgaatatattgcagtaatccaaagaacatcccaatagcagccagtgagaagccaaggtggaagttgacgttgaatccgagccaactaaccagcagcggcgcaatgaatgatcccaaattaattccgaatacgaaaattgtgaatccggaatcgcgccgtgtatcatactcggtatataacccaccgaccatttcagaaatgtttggcttcaataatccagtcccaatcgtgatcaggacaattgaggtgaataatgccggcgcacccattggcaacgacagcgcgatgtgcccaaacataatcagaacaccgccatagaacacggtccggcgactacccaggattcggtcactcacaaagccaccgataaccgaggttaagtagactaacgagccataaatcgacataacagacgcagctaatggcttatcaaaccccaggccgcctttagttacactataatacatgtagtaaagaagaatggcacgcattccgtagtaactgaaccgttcccacatttccgtgaagaacagggttgagagtccccgaggctggccaaagaaagaggcatctgcgcgacgttcctggtctgtttgatcttgttgttgcatgtgataccctccaaaaaataaatctaatcttattaacaaaacaagttaatcagattagatttttgattttaaattactcctgaagttcattacaagaataaatcatacagaccattataggccagattgaattttaattcaacagaatcggaggtcacgacaagttatatacacagcaaaattaggcaagacctatttcgtaagtagtatcaaattaataaccggatgccggattgaacttatgaatgatttgtaaatgcagcgatagactttctaatcacaaattcaattgtttctgtattcataagggtatcttgcgcatgtgtgaagagcaatgagtatccaactgtctcagcttcggcaatcaccaaattttgttgctgatgtgcctggaccaaccactgatgagcttcgtttaattgggcatcaatatcactatcatgacttgatgagttgagatgatccatcaagtccgataagatgctctttgctttgccagaataagtcagcattttcatggcgatcccgtttaactgctcatcagtcatcttaagcggccccaatcggagataattgggccatgatgaacttaacgagtttctcaccgtttgcccaaccataaatctcgtcaggaattgttttaatttgcgttgcgcggtcaaacaattcaagttcttttttgtgataactggcttgaggagcaacgagcactaagtcaattggatcacccaaatatgtgtccgcattgtcaatgttagttggaatcagttcaatctttgcatcatacagttcaataaagggcctagccgatttagcgagaaagttgctggaaattccactctcgcaaattaataatacttttttcattttgttcactcccaaacaatttgtatttaccagtacagcataacgcaaaacaacgtataccacaagcccaatttttcctgattatccaatcgggtaccgttacgtcgggctatttcaaaatattattatcatataccaatctatgatatttcttgtataccaattctcgtctgacatcgtccgcgaactttatgatggtgtttcatggagatattacaagcaggaatacaaaaatagggaacccaacaaattgtcattcgttggtttccctatttttacgaaatgttatgccgactgcaggcacaagtgccccttacaaacgttgatataaaggaatttataattttaattgaccgttatttgaccgttatttgtcaattcaccggtaaaagtgatatttctataagaaattattatggtatgcataatattatcaaaagcacaaaataatattaattaatatataccaatatatgtattcccccccccaaaaaaataattatccaagggggattcatctcacataaatttctcaattaaataaataatcaacggtacaataattcccgttgccactaaagaaattaatgcatagttaatatgtgtaagattatcaattcgatgttcattttcaatagacttagccaaagctttatcagctttttcatttaagtctgcttggtcacttagctgctgtttaatggaagaaatatcttctttaatgccaatgagcattttagtcatattgatttcatcaggaacttccaccattatttatcaccagcctttaccgcaaagataaacttaactttgtctttattagctgtatagtaccctgttggtgtagagagccgataaattttaccatatttaattggtgtagcgtaaaatcgacttcctttaattaaccgtgtatgacgtttagatttgaattgaacgtcgttaaattggtgaagtacgctttgcgttgcttcgtataggcctggagtttgataatattccggtttagcaggtttaataactaccccacttccggacagtgaaccatcaaaatctaaactggcgtcaacctttaatccatcatagttatcggtatattgccacgcattcgcattatcaattcccggttgactaacaccatacgccgctacccaaatatgcttatcaataagtttcgctcgatcaattcgcttttcagcaaaccatgaaccggatccataagtaataacgttggtaaatccgttggcttttaactcctttaaaaaggcatttacttcagctgtggtcttccaaggaaggtcttgcgcttccacatctagggccaagactgtggatttatccaacccaaagctttttacccaagctaagaaatacttagcttctgatgaaccatgaccatgaaagaaatgataaacactcacagtaccaaatactttgaatccgttagccacttgttctctagctttagggttaatgtatccagtgccttccgtcaatttaaccaccgtggtatcaattccgtgacttttcagtgacttcatataagactcggagcttccttgaaatactgataaatcagcaaccttttttgtcattttcgtcacttcctacttttgttcagatgattggggttcgttaaatacttccggatcgtcatcgactggaacgtcgggtgtaacgtcattggtaggcgccggagtaacaggtgctttgtgattatctccctttagagtgtgtttataatactggtaagcttgttctgctaatccttcaattgtttctgctttaaaattaaagccggaattttttaaattggaatcaataaattggttaaccgcctttttgcgatctgagttacttaaagcaggcatacttgccaccacaggaacgaaagcattcgctaatttcaagcctaattccatcccttgcttgatatgagtattcttttcagttttaattttagcttcaatcaacggtttaaccaatttgtaagttgctggaattacagcaattaaaaaagcaaccagtccggttgctttaagagaattaaaaatatcgacaatttgtgtgtacataaaattacctccataaaatttgtgtaaaagaaaacgccccgctttaaagggcgtcctcaattcttatcatattgaagaacatgaaattccttcttggaggaatggaattccacgaacacattgtatcacgattatatagtcgtaacaactaattattaaaaacaaacacgcccatcttatgacgggcgtgtatacatcacatacattgaggggaatgtatgagcatggggcattcataaatgctcagatgaatattcgaatgcgtaggcaccaaaggggttaacgcctacgaaaatgattataccactgttccaaaaaagtgacggactttaatttaattaaacttgcattccgccaagagatcacatgtgggtttactaaactgagtaatcgttatgatgagcttgttacttgggcaacgctaccagtgtcataattcttaccagtaatatcagtaaactgatcttttgttaattcattccaaccaacgaacagtttcaatttatcataagataaccaaccgttatcatattcaattttaagcattccgtgccaatcaatattaaacattgtattacctccttttattaagctggtgaattagttgtatttgctgctggtacagtagttgctttttcagaagcatttaattgagtttgaatattttgtagttctccgagaatttgtccttgaaccactgaaatgttacttaccaaagctcccaattgtgaatcagtttgcgtacctgttgattgcaaagattgtaactgagtttgtaaggttgttacatctgtacttacttgattcaatgaaacgcttggtaagtttcccggattgagtaatttctgattcgttgcatcataccgaaatttatctgggtattgagcgaactgattaatccacgagtctaaaacaaatacttttgtgtaaccatctgtttcgacttttttataatcagtgacaaaaccatttgaatcaaacgtaatataaataaacactatttattatctcctttttaaatttaatcataaacaaaaggtctacctgaatagataaaattaatatatcaagaattatattagtaatgtatcataatagactctagcaaatccatcaattttataggaatttatactagccctaccagcacctacacccttagtagttaaaaatgcccccgtagaatttactccaccaacggagtaattccctacaaaggcgttataccctgacagtatttccatgtctatgctaacaatttcattgataattgatgaaagatcaaaaagagttccaccgttattatttgttgtaccagaggcacaaatttcaagatatttttcatcagaattaattttatatattccttcataattgtcaaaaacaccactgggaacatttaattgacgccaagcactgtcttcaacgctttttaagtcagccgccgtggcgacatcgatacctcctgactgcaaacctgccgtaaagttggctaatttattggttgtaaccacattacttgtagcggtattaacagcatttttaacatccgttgtggttgccacgtcaattccagacttttgaagttttcctgtaaaattggcatccttagtcgtatctgcaagtgttgatggaactgctggaacgccgtctttagtgatgtacggattaccacttgccttgtcaattggcgcagtatcaaaagtgttcttacctgtaaactcttgatctgaacccgttcgtgctaggtcagatggtaaactgcttgctagtaataacggattattattaacagttggaacggtatcaaaattgttagcaccagataggtgggctactttggaatcgtcagcaggtgtgtaaccaattttatcttgcttaacgttaacttcttcaatcccagctacgtcactagctggtttacgcatgtcagtaacattaactttagtgtttaaagcattgttcatatcagccacttttacatagtcagctaaatcaggcgtaatactccccatattttgccatgaaccatctatccaaatatataagtccgttccgactaagtaaccatcaccctggttgttacccgttgtgggtaaattttcctctttatcagctttccccctaacaaccaaaccatttccttgttttccttgtggtcccactggtcccattggcccctgactaccggtatcacctcggctggaaacaaaattagtttctttagttgttccgtcatcgtagataaaaataattttagtccacagataaggaagttgatcagttgttgccaaaatagtatctgaccagccccctgtgggaactgtaactggtgaatcacttaactgatactgattgttggcagacttaataccattaccaggattaccttggtcacccttatgcacattttggactgcattctccatttggctacttagatcatcaaattgttgcttaaaatcatttaaagtgattgtcggaattacttcaccagtatcactcattaggttctcttcaattgaaaatcccaacgttccatcgcttgggaaaatagcctgtgtaccatcattcatagtaacccaaacttcaatatcataatcgtctggaaccaatgtgttcatgatatcctgattaattggaaagcttagtgttccaccaagcggactagttacagtggttagatcaatagtttgttgcatgatgtagccatcgtcattagctattttaaccagaattgacttagcattagttaaatcaaaggctaccccatcggccgtaagtgccagattaaaagcagtggttgtatctaaatatttaaccacatcattatcatccgtgaatgcgagttccttactcattagttttcaccttctttctaagctgattattttcaatttttaataacgcaatttgttgattttttgctgccatatcttgactgtactcattaactaattggtttattaaatcttgcgcgttaatatcattcatcagatcaccttacatcttcaatttatttttaatcttattaatttcactaagtaaattggttccatgtgaaatgacgtctccggcatgaagatcaatcgtcgtaccagcttcattgtggaaataaatatcagttcctgaaactgatgaaatgtaacctccaggaccacatttaattccttctgccaaataagtccatgcattttcactaccaatatgagtattgttgccgccatatgcttgaaaagtttgtccttcaatgattgaggacccaacgttaattgaatcaacatccaagccaccgcgaatttgagtatatccattactatttccagatacaaattgaagatatttaccattactaatggcacaaaaaccgtttgtgtctaatgtgatccttccattattaccatcttcctcgattgatgcccctgtaattgttgaagttgcatcaattttggcagctttaatgattgacgaatcaatttctaccgagttcaaatatccggcttcaatggttcctaaatcagcagataacgctgaaagttggccaactgacaaggctgtttgggacatcttagtcttaacccaatcagatccatcataggtgtacatttcactagttatatggttactgtcttgaacataccaaatatcaccttcatcatgggttttcccatcatcaaatggttcttgagatgaaacagtgattttcccatccaaagaagttttaattttacccgcttcattagctgcagagttagcagcatttttggcgtcatcagaggcttgttgagcaagcttagcattttcatcaatattcaatgttcccgttgcaataatcaattgctatcaccatcctcaattttggttccttcaccaattgactcatcaccatcttcatcactatctgagcttgcatctgaatcatcagcattatcatttccggtaattactggttgttcagcttcatcattttcaccctcgtcttgttcaggatatttaacaactaagtctctagaatcatcacggattccaagtggaactgtatataaggcactatgagcaatagaaatagtatgtgcatcatccctatattcagaaacgttgaagccaacaattaacctggaattagtaatatcttcataaacaccttcgggttccaaatgcccgccattttccaatggcactgctaacttaatgtcctgcattggctccactacatagtcaaataccattgactgcgtaattaaattaatacacataacatgcttgtcatcagcgttgttcatatcaccagccgtaaaaaaagcaaatggataactaatcccattcgcttgaagagtattataagtgccagtattaatggttctagctggtaatggtttccacttaaaatcttgcaatttaaattcaatgattggtttgaagtttcctgcctgcaaatcgcttatctgacaaacatacactttcccactcgtcgtacttcccagccacagattgttcttcaaatcaacgttaactcgaaaatattgttttacttggcaccacttggttatattactagcacttgtattggcttggtatgtcattgttaccaaataatatttcccatcaatcggatcttttatttctgtataaatcgtattggaactttcatcatagccaaacgatccgcaatgaccacctccagttacaaacatcatgctttgtaatgttccatcggcattccatttaataaattcacaatctgaatggcttttgtctttagtgtagtgataactagacaacactgaaccatcgctcaataaatatgaaaattgtaaggccccaatatgttgatcgccattaaaatctttgttggcggcatctttagtttcccaaagcttattccaggaaccatcagctgaattgctggtatcaatccacatctctgcctcatctttcacataagtatcatcaatggtgactaatagtgtcccgacaaatggtggttcgatagtaacctgataaccatcttttgcatggtcagcttcccagccaatatcacgggtgccatccatattaattttttgccaattaaaagcttgcggtgacaaataagaagttacattctcgccttcaataaatagtctcgcaatcacccgtttggaagtatccgtgttataccaagttgaacctaatggtgtaatcaaactgactgtggctgcattggcattctctcgggcttcttcaaacagtttcttaacatggtcattccaacgctgttccatattacggataaacgccggcgtaattactttaactgtgctaaactctcccaagacgactttattttgacttggatcactctccgaagtggtttgctgaatgactcgcgcttccgttgtcaaaattgggttcatagataaatcaatcaccttaatagtatcgcccaagttagcttgaaaatcttgagtaacctccacagcatagttaattcgtggatgattgtataatcttaattcgcgtaatccccaatcaagtaatgctttaggttcagtaatagtgtcactagtaatcgttccttccagccaggtgttctgatcagtgttataaagagaatttgctgaaacgtcagtaatataattcttgccgttattaaccgaggcaattgaagcattatttgcgcccacaatgtaaagcttggttactaaattagtatcaactgtttctcgttggacagatagcatgttttgcccataggtaattgacttaccttcgtcttcacccaattgatcagccaattctaaaataagatcagtcacaataccgtttgcatcaatatggcaataagcatcagcttccgcatcgtaagttgatagaaccgtctgtaaggcagcttgactagaagacgttccatcaaaattaatatcggcaaataatcccgaagaacaattattttgtaaatcccaaccggtatctgccatgatccattgcatagcttgatctaatttacaatctttaatttctttttggggtggaatggtcttatttaatttatagattgctaggttaatagcatcaaccgttaccagatgagctccactagttgcatcaatgttttcgtcaacctgatagattcgataaatacgccaatgattatgcacatcatcatacactgcgacactattaccaaccgttaagtattgagccgcaggggcactttgcaacatggttagtcctgttaatgtatcattccaacttttggagttagcattcggatccgtactattaaaagtgctaacgccagtaatgccatcatccgagttactgttatcatcggcaatttggcgttcaactacttcgccccaaaacgggttggcgtctgaattagtcgataacgtagcaactcgctttaaatttttatccaggataatatacaaatctctagcctccttaatgtatgtatgaaaaaagtagtcgctttcgtgactacttaattgctggtcgatattcgattgttacatcagcatttttgggatccgggaaaaagtgtagagtttgtggaaccccaccggttaatttagggaaggtcgataaccatgaaacgtatttatcggccggctttccatcaatagtaactttattgttggccgtatcaataataatttcttgaccagccttggcaataatatgtggcgtatcatctggatcagtagagccatcactgcaccattcctcataattggttaaagcctcataatctgatttatatgccaccactggattaactaagtcctctttaatatcatgcttaccaaagaaaacacctaagttggctaaagcaaagccaaacttaccggacttatccaacttttccttatgcatatgagttttatgggtattattaacactatatggttcaccagttttaggatcccactggttaatttctgctacccaattgtcgtaaactttaccagacttatccgattttttctgtcgttcaagaataaattcaccataaaaattcgagtaagcatccttattcatgtacgaagtttcagttacatattccttttcctttttcttctttgtcgtagctttgggggctgatgtctttttgcctcctttgctactacttttcttgccaccctttttggcttttacaactcgtttctttttagtcttagccttcttacgagtttttcgtttctttcgcgcaaagaattgtagattcatttatatcacttcttctttttggctgtcttcttcttaacgatgaccgtttttgtgtaggcaactttaacatgcttggtagcctcattttgtttctcctgaccattaccttcatcaaaaagcaacgttaagtagctatcagagttactactatcaaaattattacctaattgaataaacgcccgtggataccgtcccattgagtaatcttcaattcccatccgaccacaaacattaccattgttgtccaacaaataggcttcaattttccccattgcccgctcatttttcattcgtttaacatgatgcaaacgcaccgaaactttccaataaggagttatcttaggtaagccattatgcataactgctgggccgtaaaagttcttgtgtttaccacgagtgccccattcataatggtcatctttatctttagccaccataattgaagtaccggtggccgctgagcttccatctatctcgcccttataaattggaaaggcttgcgtattttcgctacattgaatccacgtggctaatgagttgcacgggtcgtctacctgttgagtttgggattgtcccatgactgtgacgttgccatcactatccgtagtcgtatcaccgtcatcaacattatatccaaccgctacatagtcatcatttgtttcataacccacataataaagatcagttttcggaataatatgaataattggatcaacttccgtatttccttcaggaataatttgctgatcattgtccgtaatttttatttctttttgcggcaggaaaccacgaggatccgccagcatgaagactaacgtggtttgaaaatcctgaacaccttcattaataaatgtcggtgttggaatactcgtaaagtgtccataataagttacatctggatcgtcattaaacctcaacggatattcagtatcagcatcactgctggtattaactaaaacgttagttaatgttttaattcgttcgttatattcatcgcgggtggtacagaaacaggtaattggaatgtcaaattctttttcaccgtaatctgttcccaagtacacaccaccataacgtttagggacgtcttgaaatgactcagtaatattgggggctaacggtttcgatacatgatttagaaatatgcctaaatcgtcttccgaattaaaaccaccatttccatcttcatcaaacgcaaaatcaaatgtgtttacatcataattatcgttattagccaaaggttacacctcttccccaattattcttagccgttgttcgtttgttatgcttattgactgcctgaacaatttgcttgtcagtcactactgccggaatcggattgttttggccatcgaccaattgactcataagtttaatcattgtatcaaacttagcttcaagtcttttgacagcctgaccatccgaattgcttgattggttggtgtgctgatctgtttgcttaaaatgagccatagtatcagctagcaattcataggctcgtcctcgtttattaatatcccacggaatgatggtttccggtttgttacgttcggctactttaattaactgttcttgatcaactaagccaccattcgcatatcctaaataattagcaactttcttcgcaccgttaacgtgttgccccgtatagccaccacgttcccaatcttcagaaaattgactggctaacgaagcaatcgaaccatgaccctcaaggattcgtttaaatacagaagaatcagaactgtcatcgcttaacgcaaactttaattgggtagctgcattgcgccagttttcaccatgacgttgagcatatgatttcaaatgattcagtctaccacctaaccactgcccaagcccagaagctccaccagatgaatttcttgcgttaggatttaatcctgactcaaattcccaattaccaagaattgcagcaattcctgccttagttgcgcgtggatccagctttttcaatgctttagctaaagttttggctctagctgccacatcaccacttaatccaaagctgcttaaactaccgaacaatttttgccataatggttttaagttttttgatacccaactccaaaccccggaatgctttaattgcgactttactagtgcttgtaatccggaactttgtttatgagatttagttgactttttaactttgtcaatcaacccaggcactcttcgaatcccaacaaaatcaccgaatcccttgatggtagaatatttaatcccgtcctttggattttcagcactgaacatatgtccagaaccactattatcgaccacaataccaacgtgttggcttcctccagcaccgaagaaagccaaatcaccagtcttagcattcttccacgatacgggttttgagtatttatactccgggactgtggtagatccacctggaaccgtaatccccatgtgcttcaaagtctcgtaaaccaagccagaacaatcataataatttggacctaaacggagattagaaccttcagaatatcggtgatgagcacgagttgccaatttcttggcctcatttaaaaacgctgaatcagtctgaccgccaccttcggaaaccatgccatgtagcatattccaggcagtatcccaccaaactgatccctgctgcttgtcccgtttgccaaacatattggcaaagttcttcccaactgttccctttatatcgccaaaattaggttgaaaaacttgtttgaaagttgcatcagaatgattagcaatgtgtgatagtgccgacaacttctgttttaaagaaccccaaatgcctttaaagagtttcccgataccaccaaataaaccagtgcctgacgcaaagtgctgcatgccatttaaagccattaacatcttagactctgtagcatttaaaacgccggaaccagcttctaggaaccggtgagtatctttaccttcaactggttctaattgcccatctgcgtggacaatgatttctttattatgtgtttctggtgaatcgtgaccatcattaagcttagccaaaactggtttggttaataagccatttttcaacaatccggtacctgttgcccaagctaccgctgggatctgatccaaagtttgtgaaccaccgtattgtttaaagactttgttctgggctgaaatggcattcttattcatcccatttaccagtttgccaatccaattaccaactgacttccaaattccatgccaggaaagactgtaattatctttagttttggaattgtttttcttgatgttctcatattgagaaacagcttgatccgttactttatgattttgattatgtgcgtaatcgtacactttgtcagactgctgtttggctttagtgattgaatcgtttttttgtttatcggcatgattaatcacaccaattctttgtttacgagcctcctcaataattttttggcgttgtgccttggcagccgaactatttcccttgtactcttcatctgctgctttaactgtatttttatatttcttccaagctgaattatagacactatgatattcatcgttagcttttttgctgacagacttttgttcttcatcagcgtttgccaccaatttaatcattttttctttggaatattttttactcttttcagtgagcgttttataatctttagcaatcttattagtagacagtttaatctgaccagctaaggttgtatgcagtttggcttctttagcagtcacttgagtagcaaacttaagatgttgtttctcaagtgcttctttcttttccttctgcattttttcaacttgaacggaccctttaccgtatttattctcagcttttagaatctttttattccacgattcggttaatcgttgccgtgattgcgcataatatttggcaattgcctgctgatccttttgactcatcagagttaatcggttggctttagatccttcacctttaataatttgcaggcgtttttcgtactcttttttagtaatgtccccgtttttataaagtaattgtaagttcttcttgtcctgagcttcacggtttttataatagcttgtcgcttcatcagaaagtttcttgaaagaagacttagtagataatttaggtgtatggattttttgtgctgaaagtcctttttgaatagctttaccaaacttacgaccaacaccttcaccaaccaagccacccaaaccagcgccaacagctgtgccaattccaggaagaatagctgtcccgattgctgcacctactgcagtaccacctaatgaaccggtagcagcaccaatgtgggaaccggcagtcttctttttcataccaattaaatcagttgcagaatttaagacgtctaagacacctacggaacctgcagcaacctttccgaatttactaacacccttaaacttttcagctaatttagcaaatcggcctaccctcccggtatcttcggcaactttacttgtatcatctatatcgtggatggccgttttaccatctttttcggcaccttcggcaaccttaccttcgccaccagagttatcagcaatatcatcaattgcactggtaccatttccggcatccacattagcttctttagccttagtgttacgttcaatagctaaagtttgatcatcatatgctgatgtcaatcggttcacctttagcttttgaccgccaaagacagaggtaatatcactaaatattttaaaatatttataaactttaccaactgcccaaattgcagctaatgcttcaccaaaatgtttgacgccttcataatgcttaacagcaaaaataccaatattggcaattccttctgccacatgtgcagttaaagtagccgttttaccaatatctttctgaaatcctttttcaccaaaaagcttggtcatttgattagctgcttttgtcatatacggcaataacttagacccaaacataattgataattgatcccaggcttgcttaaatcgtttctgagacatttgggcagtttgagcatttttgttagctaatctttgaacgtacgtcccagctttgcttgctttagaaacattgttggttaaatcagccaattggccattatatttagctaagatttgagctgcttgcatgccggttggaccaaaaatatttttaaagatgcgtgctgtatcagctccaccaagttttttagtatgttcctcaataattttaaaaattgcaggcaacgttttgaaattaccattggcactttggaatattttagttgatttaattccaatttcatttaaagcgcccatagctgaatttgttggagctgctaaactagtaataatttttcgcagacctgtcccagctttatcagcttccagaccgtggttacttaattcgcctaaagcagcagaagtttgctcgatactaaagcccgcattattagctgaatcacctacatactccatacctttgcctaaactttggaagtcagtagcagtcatgtcagcagaataagctaatgcattaactacacgtttagtgttgtgcatcatttttgccgtattattggttttcatgccaaatgcttcaatcgcctggcttgatactttaaccacatctttaaagtcgtcacctgaagccacactggcctgtagctcagttttcataaccgctaacgactcagctcctgtatgaccacgcttgattaaatcctggtattgatcagcaatttctttttgactaaccccatatttgagagcgtacttagccccatctttttgcatttctgtcacggttttaatagcagttttagccttgtcgccacccgtaaccagtaagttttggtttactttataaacattttgaagttcagttgcttttttagcgccagaaaaagctgctgctcccaatgtccccatcgctacgctggcacctagtaaactacctttaattgatccaaatgaatttttaaatttattcttagcaatgttagctttatcgcccaatcgcaccattgcatcactcatgtgaccgacttgtaaatcgtacttgaccacatcagaacgcacattggccagtgaagtggctgttttgttgactcgtacttgttgggtgttaaaagcttcgttagcaatgtccaagctaccttttaattgattaagtttttccttttcttgaacatattcatccgcattcttgtgggtatcattggcgaggcggttaacaacattttgttgtttttcataggccaactgggcttgtttataagcctgtgagtttttactgagttcactattttgtaatctgtactgatcagataagctattcaatccttccttaaggcctttaagctttacttgaccagcctggttaatctttccttgagcctttagcgcatccacataagaattagttacctgattaaggttatgatagttacgctgcaatccagatagtcctgaattaaggtattcaaattgcttttccgccttagactgttgatcatttaatccagcaatcttctcttgtgctttagcaatctgattagcatatttagcatatttttctgatccttggttggttgtttgatcaaggcctgactgtcgacgtttcagctcatcaatttttaagttataacctttaatttcttctgatattccttgatacctagtttttaaagcatctagtttatctccagaagactttaaagccacctcctgagaacgccatgcattggtattagctttaatgtaattggttaaagtctttaatgaccgtgcgggttgtactgcatccaagcgaattgaagtactcattacatcattaatagtagccatcagtcagtcccctttcgtttatttaataattcgacaaccggatctgttacttgtttcttcttatctttagcatttaagactgccataaattcaaagtaatcttgtcgatttaattcatctggtaagattccctgcttcatcatttgttgtttaaaaaaaagcatatcttgttgggatatgcttaggtcattaattaatttggctaatcttaattgctttcttttgggtctgctgattcctcagtttgttgtttagtaacagtttcccaatcttcatcgctcattccttgaaatctaaatagtacataggccatgaaattttgaaaatccgtaaaatccaaagttgatttaatcttttcaacttctttgtcggatagcttaaaaatatcaatcataaattgcaataatccttgaaccattttcttttgcgtttccaaaactgctagtgggtcatcattagtaaaatcaactgcatctgatttcaacaattgaatttgtaaattttgggctttctcaacaacacccacagtggttttaacttcagctgactttttacgtaaacctaattttgtaatattaattttcatgatcaaagctcctttattttatttgattatgtatgcggggaatatcccccgccttgatctattttcctggtgttgtaccgccagtcgttgagccagttgtgctacccgtagtcgatccagtggttgaaccagtcgtgctaccaccggtagtagctgaataaccaccaaagacttcagccagcattttggctttatcaaagccagcatcttgagacatccaaatcttgtacggttctccgttgaagattgtattgtcagctggtgttaatgcttggtaagttaacgccgtattggcatcagtttcagcattattatccgttgcatgagaactaccagtttcaattagttgaccattagcaaagccttcgtacatatcaatgttcgtgtatgaacgaaaatgtaacaacattgctacatggggctttggcaattgacgtgtccaaccaccattagccgcatcctgaatatatcctttgagtttttgcaactcgtcaaaatcaatatccaagaattccaatgcgacctgtggttgtgcctgaccatttgaaactcgttttgcttcatcattagcataggcgacagtaccctcggcttccaagccagaaactgtggccgtcgtagcaccttcttcgtcaccatcgactaaatagataccattagttcctactcctgcatcgctagtcagtaatttaccattagcatcaactaaaccaaaggtgacatctttaataccatgtgttgacatttaaaatccttctttcttcattgtaattgtcttagaaactgaaaaagttgccgtaatttgatcggtatctggatccacagtgttaggctcatgtgagctaaccagccaatcctgattttccaaattattcattaaagtaacttcttcattaaaaatattttcttgtatttcttttttccaaaatatttgaatttgaatattagcttgcatattgctaaatcgatcgttccgatatccacccaacggttcagtaactgaagtaactaatacaatggtctgctttccagaagtatcagctccgggaggaatgttcatggaataaagctggtcaatccaaccatagtgcaaagattgaattaactgataaacagtcataactggtaattccattagtgacccagctccttccacttaatatattcagattttaatatatcagaacgagtttcctcacgggtcttttccacaaagtggtcaccgacaatgtaaacagtgccatcatttagccagcgagcaatcactgcttttttcttgacccagccaactgtcgctgtcccatccacatcaccatcaacatttttcgaactaactaatacactatcagccaagtgaggatcatttccggtagcaattcgattactataatgtagccgtttagtttcatcagctaatttcttttgcaaaacatcggcaccggctttagtgattatagttctttccgcccggttgggtaccaatcgttttattttcgctaaataatcgtctaattgttcggccatactaaccatgttttttaccaaccctctcattaatctgtagagtcaaaatgtcataagtcacaattttattgctatcatctaaactcaaattaacgatttgatatagttggtcctgatattgaactagcagacctttgtcaattaacggattgtgtcgaataacaatttgaatagtatcttcaaaatctgttcccaaaagcgaaacgttctgtgtgttagttcgcgtataaggcatgcaccataacacgaactgtggtttaaattgcgttcctgatgcaccagtattaggattaattgttggtaaagccgttccaaactgggcttgccgattaaactgctccggactaaatttattaagtgccatccggatcacttcctgaaaccattccttggagttgatctagcatcatcaacaaaccagctgacatccctttagataattcccgatcataatataattgagttgccagtgtttttattgctaggtcgtaaattgatgaggcttgatattgggtttcagttgaactgactgaatgattgacaatctcagttgcctcattaatcaaattggtaacagtcgttaattcagtcggactttggtcaatatgcaactcatccattaattctgtcggattaaccgtcacatgacacccctcctaacagccgcccatcactgtattgtttatttcattggcgacttatttaaattacttgccagttgaactagtagtcccactagtctttgcagcaggagttaaatctgctaatccagtaaatggcgcataaatgaccgattcagtatcccacaactcaacatcaaagcgatcaatggcacgaatcttagtcaagtcactttcaaaagaaccagcaccaatattagtagccaacaaagacatctgttggagatcgaaaagtctaactgcttctttcaaagcaccgatgtacagtgggaaactgttaccatcgtttggcaaaaaggcatcagcaataactgtaattgtcttaccagccagcatcttttgtgatgggttaagcgggttaggctgaatgacgtattgtccgttattatccttgaccttgtccaagacagcaaagcctgattggttagtaataaaagcagattcattccaaattaatgggtccagttccttgttgtaaatatccttaatggcgtcaaaactatcaactgtggttttttgtgtggttggcaatttagccaatgcttttaaaatttcactgttccgggtaataacatccttcttagcaatccaattttccaaatatgccaagaggtttgcatcactgtcattcatcaaagtgttggtaatactggaaattcctgcatatcgatggattttgtaagttaaaggcttaaaggctgccggctcatcgttattcccaatttgagctgtttcatcgtccaaattagcaaatggagttaccgactgacgtggttcaataactcgtgaaccagatggtgcgctaactccttccacagttactaatggctccagcgacgtaaaggtttgcttcaaagtattgatggccgtttggacatcttctggaattgtcaagccaacaccgtttccattggcatcaagtccactagacatcaaattcaaaaactttggatcaccctttaaggctcctttaacaatattaataaatttaggtttgtcttttggtgtaacatttttctggccaccagtagctggtttacctggcttagccagtttagccgttgctaaagcatcatcatatgcacctttagcaaaatctcgggtcttctttgctttatcaattgaatcagcaattttagttagatcctcatctgaatatttttcaggagaatcgttcagttcaactgccatttgattgcgcttttcttgaaggtccgttactttttgaccagcttcaagccaagcatcgtgcagcttatttaaatccataatttaatttccttctttcttaaataaaatagccaacttatgtgatcgtaattggtcactagtttggctattagtttctttaggcttttcttttactttggttaacaatgatttaattttactaattgcctgattactcaacatcaagggcgacatcatgttagtaactttggctggttgatctgcaaacatcatttcgtctgcaaatccttgttcaacggcatcttttgcattgatataagtttccttggccatcatttgcatgactgtttgcggatccaaacccgttcgttgcacataaacatttgcaattgattgatcagtcgagttcaacccctgcaaatcgctggataaatcatctgcattcccttgagatacagtggaagcccgatgaatcattaattgagccgttggcgaaattttaatcgtatcaccagccattgcaatgacactggccgcactcgctgctaatccaacaatgtcaacttccacattaccggtataattcttaagtgcggtatatatttcagaacccgcaaacacatcgccaccaggtgaattaatttcggcaacaatattttgaccatttgcagtgcttaacgcatctttaactgcggaaggagtaactgttgaatagccaaagaattcatatacttcagcatcatcatcactagatacaacacctttaattggtactgttgtcattatcatcacctccttccactgctgaaactttcaaatcaggaaaaactcccgcttgtttcagaattgtttgcgcttgttgcgacgttaatgctggtgactgaccagtacttaatttagtaatattactaattaattgctgatgatcaacatcaatagccgaattaatatccattttaatgtcgattcccaactttaaagacaattctgattcaattggccgaatatataggctcaaactattttgatacaaagaacgaatcatctcaattgatgattgttcgtcaccttgaccatttaaataactatctggaacacaaaaagccttggcaatctgggtctgactaaacgtggcattatttaataatttagctatatccggattaatctgtaaggaatcaagctgagcagattgatccaaaacaattggtcgaccagcattcgaaccagaattctgattctcaaacgattttctaatattttctttagcttccggttccaatttggccgccggaaccgtaatcgtataactaggcgcaattgcattctttaaactgctcagtgacaattgattactatagttctggatgttaatttctttagctaaactgtttagcggactgctacccactagttcagtggcaacttgcccagaaacaaacaagcgaaaatgtaaaatatcggcagctaaatatgtcacctgccctcggtcatcaccgtaattaactgtgtaataaagaacattttgttgattatctaaagtaatgctgacctggtaaaacgggattaaggtcaaccctgctggacttccattgccatttcgctgaattagaacaaaggcgttgccagttaacatcatttgagcactaactgcttgccaaaaattataagcactcaataatgtgctgggctgatttagcatgttgctatattggtctgttttaaattcacagctggccacatcacctgcaattcgattaatcaccgcataaatatcactgttttgcagtgctccgtctgcatccacagtgttagtggataacaatgtaccatttaacataaatggtgaatacccggtggtactaattgtttgtgtttgttttgacataaaatttttaaaggggttcagcattcaacgcctcctttcacgaaatgacataggctaaaacgattaaagcaatcccggccactacccaacctacaataaaattaataaggcttgcggcaaccacaaatgcaattaacccaaataaaaataatataaaagacaggttagtgattaaacctgtccatagttgtttcagattcaactaatctgcctccctaataatttattcactacatatatcacccaacaagtgttgaaaatattaaaaactaaaatgatcactggtaaagaattcgttgacctcctcattactcattccattaaatggattctttttatcttctttaagtccatgattaggattttcaaaataaaaaagggcttgagacatggcatcgatagtggcatcggcacaatcaattttcgaagtcaacgccgttcgatcaattttaataccatatggattagccactgttacagcgttagccaagcaggtctgcaaaatcggatcagccagcatctcaatatttcccgcaataaactgatttctcaaaaatactgtgggcgagctcaaactaaccgtcccttgctttaaagtaataaaaggcacttctggcatattattatccaaccaatcagtaattgcgctagcttgataaggatcataaataaacgctttgactctcaaatgatgatcgttaacaaaatccaggaaccagcgcccaacaaaatcttcatcaattaagccataagaattttgcgaaatatcacaaaagcctaacttttctgcgtttgagtaattaattccatcttgtttttctttcacaataatggaattatctgctcgggctaacggaacaaatgaatgctgcaagatgaaatatttcttttgttcgccattcaaatgtgggaaaacaaaactataagccgtatcatctgaagcatgtgataaatcaaaacccacatagcaatcttgattatcaatttcgaaatcagaaacaactgacttttgtatatcctctaatttcaaatatttatctttagcagtctgcaaccacatattgaggttacggttaatgaaatcatttagcgtaccgtcttccagcttagaatcacgttcactaattaaccctttcagtagggtatcatgcttagccggtaaatctagtaatggattgcttttcacccatgtttctggattctcaacttcatcttgatcatcctgctgccaaattaatgccaacgttgaatcttccgttcggttagaatctttttccatcaccttagtaagtcgtctaacatcactatacatcgggactttagggttactgtatgccgtactgataaaaaatgtttgccggttactagtttgaacttgtccagacgtgactttagaaatcacatccgaattaaaattttcatccccgtattcatccacagtggcaaagagaaaatgaaaggcatctaattgtgcactaccagctgtcattcttaatatctggttttgagtcttcgtggactttaaaacatcatcattaatagcaatattttgatccttgatcaatttacgaaagccaggcattgactgtaaactattaaaagtctgtttaatgtaacgccaagacttcttagactgcttatcaaccggcgccaagtaacacaaatcagcgttaaactggtcactagcctcgaccaagtaagcgtaaagtatcaagatattcaataaatatgacttgccattagtccgagccactgaaaccatacatcgctcaaatcgcttttgcttgtcttcctttgttcgccatccctgagaaaggcacaagattgcttgttgccaaatcatcaatggtatcggcttgttttgagaaacatcagggcacatgcgtgcgaagttacagatatttcggcatttatccaaatcatagtaatacggaaaattaccttccgtggatcgctttaaatcatttaaatgtctaaacgctgctagtttaattgttttgcaggctaactgttgaccagttaatacccggtaacaataaacagtggccggatcacggtatttccttttaatttcatcaaaataaccttcaccatcaagtcgctgaaagattttatccaagtcaatatttctttgagtaaaatcaaattcctgtaccactaaaactcacttcccccatttaacatctctttaatattgggttcctcatcgttgtcatctgagagttgcagtaatgaggctcgtgcagatggtgttaagcctaattcgtgtgctaagctgtttaattttgccgtagcagaatcaataatttgtgatgccggattacgtttccagcctgcgttgtcttcatatgtttctccagttcgttgattgaccacagttttagaaactttggtgacaacaccatctgttttaattgagtcatagcctttccgcaataattgatagttaatacaaaacgcttcaattgttcccttgtcggcctgtttaacatatcctgatgcttgcaaaattggtacaagtttcgtccacattgctcgcgcataacttgacagatattttggacaactcttttgaatcaaatccattccagaagtttccgttattagtttttgagttctaactcgctgatccttgcgagcatgcttgtctgtagttagtttcatttgttttggcattttttagttcacctccaagcaataaaaaagagcccccaatagggactctttcaatctgattcatttagactaatgaatcacaaaaaaatcattaaacacactgttcgaacgtatacaccctacaatcgtgaaaaaacgtctaattatattaacttttaggaggtaaatatacatagtcattatagtagggttattcatataagcaatttgtgaaattgcgtccacccagttatagtaagcccataaaaaagttttgaatttacaacttttaacgtgcgctactgctgggcgtgcgctcccctaggctttcaccacccggggggggtgtttaaacattcacctaaattgtatatttttttgtaagattcaaacagtaagctttaaacaattttttctttatatctatatcacccagaggaggttgaaaaaattgtttttaataaataaatctcatcagaaatatttattccgattacctacatgataccacctgaaaaacactttgtcgtttcacaaagacatctttttttaattttgttgatgaagatccccaccatccaagctggcaggagttttctacatcagggatgtttatttcgtgcgttcagataacactttaatccaccagcgtttgttgcagtgtttgagttggttttggttaagtgattgttcaatcttggttttggtattatgcgtagtcggtgacaagcaccataagttatccatgtctaaccatttatcaacagatagtacacgtctaggcacaatgtggtcaacaataatcttatcgtttgagactggcaagccagtgactgcatctaaataataatctcgtgcagcaacaaattgccgaatctttttccattcctttgagtgataaaactgattcgctgtttgatcacgatagtacatattgtactctcggtttcgtgcagaactgactgcatggttgggcttctggtgctgtgtaacgtgctcactgcaatacctttgccccattggtatcaatgcttgacagccaacctcatgacagatatgtagcttcatataagctcacctgtccttctttcggtacgaactgtttacttaattcctgctgtaaatcaatgattgaatcaattaatttgtattcatccagtttcaattgatgatcattaattaaaccaaacgatttccaaacaatgccttggtatttcattccatatactttagttgcgtaatcgaatatatcattgaacaagtcgctattgctgataaataaggtgtgaacttcgctgtttaatgtcattggatcagcgtatttattaaggcaatattcaaaatcacctaatacctttagcttatctaacgtatcctgatgatcgaagacacttaactgttcagtaaacatttgtgcatttgatttaacgtaagctatacgatcatacaatgcatgttcaaactttttatcagtcattgaaaaaatatccattgtagctatttttccatatttaagcaggctttttacaaacagtttggttttatccgtcgggaataatgaaataactttattcactaatgaattctcaaccgacactgaacttttacaatttataggcgccaattgtccaagttcatcagatttatcaaaattctctaccaataacgtcttgtgaccataataatcttcaaccacatctttagcagcataggtaattgcccattgcttattcttaaaatctggattgctatgatcgctgaatgccttaatcaaggtattagcattgttataattccaaaaatgaattcgtcttaatacttgctcaattaatagactaaaagcatcgtcttttgaacaatgaattgaataatgaatccggttaatgccgttttcaaaattccggctctcagtaattgcttttactaagttttcatttcccattttttcaccgcctttaaacttggtttacttacagctagacattgacgataaggagaaactaattattaacggattactttgcgtttatttcagaaattgtccatccacagatggtttgatgatgctgaacagatttttcaaccatccaggttttgattggcaaaccagtttctgctttcaaaactgcttgaatgctgcgaaactctttcagtttatgaactttccctcgctttgttatcacatacgtcatataaaattcctctaatcacataattttacatatacttattgtgcacatttaacagctaattggcaagctttcataagtcttgtggttctaatttcatccctccacactttgaatgcttgaattatttaacaaatccttcagaaattcagcttcatcacgtgtaaattgctgcgtaatttcccctcgacaaacgcgcgggttacgtactccacagatgaaatacccaccacgatcatctactcgtcgagatacatattgttgcccattgctaccaatcatgccattcattttcaagcgatacattggtgcagacaatttcactgtttcatgatttaaaattgcatctataacactggctaaatcatcacggttagaaatagtttcatcattggcatatttatcaatgaatttggcgaatttagctattcgtttccaatcagaaatgttttccgccattgcgcattggtacattttgaacaattccttatcaacaatctttactgtcattttatttacctccaataattttcaacgcgtcatctacagaacggcaaacaccatataacactggatattgcttaataaattttgcaaaccgcttctgatcgtcacgtaacttgcctcgttcgtttttaacttcaatcaaaatcatttttccactatgatgttcaaaaccggtaatgtccggccaacctctcggaaataacataattcgtctgccatcatcagttttaatctttccagcattactacgacaaacagtacaatcatgtcgagataatgctaaaagaatttctgtttgaatttcatgttccgacttaatctttacacgcctccaaataattatgacggatgggaggataaatgggaggatgattcagtcgctgtatccattgcggctgtaagaacaaagcctgtttttgggtgtatgggaggatcttttcaccaaacctttatatatatctttttttactcttttatcttatatacttttattaatttatcctcccatagtataaaaagagtatataaatgtagttgtatcaagggttttagcttgaaaatgatcctcccattatcctcccaaaaggggttttatcctcccatttttatttaatccagcccagtcttggatcgcctttaattttcaatccaatataaaatatggatccacttttcttggtttcaaatttctgcttcatctcacggctaaacttctgtttactcatagaatattcggaattatcttttgcccaggattgatatttcttaaaaagttcacctgcaggtgctcgataactatcacttacctcacagcaatcatctacaaataaactaataacatccatttcatcacgatattgccggctagcacgagtaacacttattggtggattcaagccttctcgttgccataataagcaaccctcaacgatccaattaaggattcccacggattcgcgttttaatttatcctttaagttcttgtccacttgaccatcgggtatttttaccttaaaaggaattaacatcagccgtcgccaaattccgtcatcagtaccacgaataattggtttatggttagtagctaaccacagcttaaactgtggtttaaactcaaattccttaccatataaataccgtgcggttactttatcaccaccggttaattgtttaaccaatccctcgtccaatctcacaccctcattaggctcgcttgaggtaactaatcgggcgctttccaaccgagcaatatccgagttggctcccgatttgttttgtcgtaccataattgaatcggcctgcatcgacttggcataagttcccagaatatcagaaattgtatcgatgaaaattgatttaccatttcggccatttccatacaatatgaacatcacttgttccttaatacttcccgtggccgagtacccaaccgctttttgaatataatggattaattcctgatcaccagcaaaaatttgatttaaaaattcatcccattctggacaatcaattttgtcggtatattctacgcttgtctgatgactgaacattttcttaatatcgtggtcttttaagatacctgaagttaaatcaatatagccattaaccgtattcaataaagttttgtcttgatcaaactgcccatgtaataccggaacccgatgttgcacttcgcttatcatggcttgtttggcagcatgactacgcgacttcttcaaaaacttttcccaagctactttagccttttcaggatctacgccggcagcaacatgcaacttctcattcttcatattatccacggtcatatcaacgaattgagctgcttttccctgatcgtccatttcccaataactgccattatagaaataccaggacttatcaatataggaatatttgactagatttccaaaaacatcaataaatcgatcagcattcccagtatcatcccaacttctaggtggtaatttctttttaggcttagattgtaggaatttaagattatatttatgcaagggatgctgctgtggattaaaggtttcccgtgtttcgttgatagatttgttaagaagtgaaactccataagtggttttcccatgtttttcatcatatttcggtcgcataaggctagactttcgaaatatttcatccattttattaaaatcacggcccgtccaaaaggccaaatcattggaaaaggctagatcagcttctgaatgggaagtatagaagccctcccaaccaccgtgcataaacatcttgaaacgtttaccagtccgcgaaagttccgcgcgtttaacaatctcatcaacacttaaatcattaggcctgattggtgcctgattgggaagttttaccacattactttcaccaaaatagtgtttataaataagtttcattacttgcggttgtggtgtgtttattcgatcactatatggaccaatggtttttccagttaacgcgaagaatcgtccggactcatacatttcaacgttgcctttgcgacgtcgatcaccaggaatcttgcccttaaaaatggcatgaattcctttaccggataaactaatttccacataggatttagtcatcgttaacacatcttgaacttcattttgttgataatcctgtgcagcgtatctttccagctcatccccaatgtgatcaatatccaacccaatataaccattagcaaagtaaaacgcgagaccatccatttgatacgttttaagtgcttctaatgctgtttgataatcagtccaggtacttgggtcattcgtgcgtccagctccaccatcgagcgcattgtggggtattttggtgtacttatttcgctcaggttgccagattttttgaaacaggccccattgttttaaggaccgtaattcatttggaattttttcatatgccactgtttaccctcctagaacggtaaatcatcgtctgaaatatcaattgaatctccagaattatcaaatggattatctgccggtgctgatgctggttgattaccagtaaatgggtttttaccgtccttttggtctttccatacatgctgcacttgtggataatcgctcttgctaaaattccaaggggcaatctgattgatgtctttcttttcaccgccataatcatcaaccgtttttttgacatacactttggctggcttgttagcaactgctttagtaaaatcattaattgtattcaatggtgttccttctggaatttgaacagcttcaagaatgtattggaaactatccaaatcgtactgattagtagttttgcgtttccaattgtccataaagacatgacggttatggtacttggcattggtattttttaatccagtaaccccatctaagtcatttcgaaccactaaatctaattgcagtgattctgccccgttcttagttgccttctcctgagctgacttaataatcatctcgtagtttccacttggtaaagctgaaaaatctttgtgttcgttgttcttgtaatttgcttgcataaatgccatttttaaaattcctccattagttaaccatttttagtcgtttagcttgtacataggcccaaccagctttatacccacgggctttagcgatttctagtaactctttgtaactttgtgcatcttccggcttttttcttgccgtctggatttctgaataatcagtagtcagtttaaattccccaactttttcaatactggccgtttcatcaatttccattccgtcagcgtcatatttaatctcattaccacactgtgggcaaacacggcattgtgtcggtaccacggcaaaacaatttggacaagttttgaccggaattgattttgtgttattctgccgttttttcttaggccgtccttcaaggctccattgtcgtagagtatcaggcagaccaaaacgggtatagttagccacatgatcaataatcgttgccactttattgggcttatatcgcatacaacgcatggattgctgaatgtccaatactaatgattcggttggccgtaacataatgactacagagcaatctggaacatcaaagccctccgagatcaaatccacgttacatagaaccttaatgttgccatttttaaaatcatgcataatttgatcacgtttggctttgggcgttttggcatctgcatgaactgctttaattccagcggcacaaaatgccgatgcagttgctttactatgttcaatgtcatgggcgtatacaattgcctgttgaccaggaaccttttcacgatatgttttgaccacatccccaaaaattgttttcccaatggcatcatcgatcgagttattggtgtaatcaccagtgcttgatttctttagtttactgtcatccactaacttaatagaatagtacttgtatggggcaaggtgatgatgttgtattagccaagtaacattttgtccttcaaccatggccgaataaatatcatcaaaccccttaccattcattcgccaaggactcccagtgaatcccaatcttggcacgtctctataaaaatcaaatatttttaaataggactttgcccgactatgctgtgattcatcacaaatgattaagttaggccttggcaatttccccagtcggttaacgatcttgcccacagtcataattgtgcagtgcattaaatcaacgtcttgtttctgaaaagattgggttatttgattcacgagttcctgtctgtggacgaaaaacattacttgtccacccttagcaaccgttaatctggcaatttctgcaataataactgacttaccacttcctggtggtgaaacgatcaaaacaccttgattgccttcagcaagcttttgacgggtttcgtctactaatcgttgttgataatcaaataatttaaatggcaatactattcaccgccaaacctaaataagtccttagcagcacacatggttcgattgtccaaacgatttttggcataaatcgagtcatttccttgcagcataacgccacgaccgttagtcttcggattaataatcaaccgaccaaccacatcacataatcccagcattccatccatcacgctttgacgaatttcgggtgcatattgattaaattgctgaccattttcagtagtaatttggcgttgtgtctcccaagctgtggttagcacattaactggcaacgcatagatagcagtcatcactctagaaaaataattagtccactgtgaataatcctgcaattcatttgagatgccattatggctacccttccccttttccacaaaccaatctttttcaaaacttgatacattatcaataactaaattgtcgtaaccaacaatcaattctgatgcctgttcaagatactgcttcatgtcttcttcggggtgagttcgatccatttcatcgactgtaacgttgctaatgccagctaatactttagaggagttatccaaatcaaaaattctagttttaccaggtaaatatttaacacaagttgttttcccagttccgggtttagcatatagaatgactcgccagttccgggttcgctgtaaatctttagcctcaatcgtcttcatgattaagcacccactctttgataacgaatttggttactatccatgaaagccctcaacagtttcatttgtggaattgttgccgttatttttaaagacactgaatgggaaacaacttcgccagtattggtatcaatcgttttacctttctgctgaatttgatgtgtttgtgcttccgctgcttgtgcttccagagtctgctgtttttgtttatttagtttgacctgattatcaattgcttgaagcaaataattaacatcttggccttgcttcaactggtcgatccaaccagctggatcaatgtgataagcttgagcatatttggtaatagttttaatgcctgcttccaagtcatcgtgttgctttttaatgtaacccatcacatcagcaattccttcggttactttcttcttggtggtggttttatttaaccaagtaggatcaatttcaacctcgcctggttccacatggtaattaggtgccatttcagcaatcaaagcattaacatgctttaagcgaagctggcgttgctgatcttccaattcttttagcccagcgtcaattgggttaatcgaactatccagggtcatttccaaatctttaatttgagctgcaaaccgttgatatggttcagcatatttttttctaatttccttacgtttatcatcaagagcttgcttcaatttccgaagctctgcccggctagactttgattctttttctgtggaagctgttactgccattccttgatatttattggcatatgcttctacagctgtttttaattgatcaaaattattaattgtaatcacaggtagctgatagtcaatcgtgtattctggtagggataattcatttgccatttatatttacctccatcttttaatgtaaatagtgtcgttgatcaatggaatccttcattgacgctatttcttttcttttagattttgtgattctaccgcagatcaatctaattggttcgggataaattgggactcgttctttccgcttcttcataaaatccttgtcggtcccagttacgacgtaagtcggatactttatgctgagctttcgcataacgtcggcacgagagacaccagtttctaatatttgggaatccattacaccaactgctttccaaaatttagtcattattccacctcgtgatgtaaaatatattcagatagtcgttgcttttctttatctaggacaaagaaatatgccaacaagctatgatcgttttccacgggtgtgcgtccaataatcatattcaaacgtttgatacggttctgtattgttaatgttttcattctgatgaccctccaggtgttataatattagtagttatagttgttagctggtccacctatttgcggtagtgggctatttagtgcatataattaaggtggtgaatttttatggatttttacaattggttaatgcgctttaaagacgttagcttaccagttggtgatgtagcaagagaaataagatctgatagatcgtttcctaaggggaatttagattggaaacatttaaaagaatatcttaagtcaattggtttttcagattccaaattagaaattgttaaaaaacgtcttcaactattatctagcggagaaaagtcgctaattaataaaatccagtaatcatttggaagcttcatattttcttggccatatttgcctcgtatttcagtattggcataaaggccaccatgaaacagtcgggcttcctttctttttcttaattcacctattaattcagatgtcgaatacttttgcaatttattcatcgatatgattcctttctattttttagtgacgcccagttggtataaagtattcaatgaccagggctgctaagaacaataaaactagtacttccaatgattccattaatcaaatcactcctttttaatatttgtagaattttgaattcaacccattaaggaggctaagtcgtatgattcatcaaattgttgctattcgattacgaacttattccaagggaaagcaagcatcaccagaaaatattgatttaataaaacaggccagtgggaaaattgaacttattcaagccacagcagccaatattattcgtggtgatcactacttttacattctcggtaatggtacctatgaaatcacttatgattacgatcatgacaatgctttatatattaaaactaagaattccttaagccgtcacgatcgattattagatttgccaagaatttaatttttttaccaattgaattcactccaatgatcctccaggaactgctgcattttggtagctttaaacaaccagggactacctttactgccacgatggactaaatatctatcatccattaaggcttgcatttcccgtgaatattttggattttccaagaaattttcttttaaccattgtggtgatttgttcccacaccatttacgaagatcgtttaaattccaagttcgtccgaaggttgattcccgttttaacttttggtaatcttccttatttatcaattcaaaattatcaggaatttgaattgatactttagcactaatgacttgagacattttgtcacttcctttagttgtataatttatttattccaattaatcgagatgataaatatgaatttaaaacaagcagccctatttgaatatagctttgaatatttcttgagtaagattcacaatgcagaagccaaaaaatgtatatgggaatttaatgggcagttattgaccgctacttttcacgacagtactctatttagtggagatgaatttagcaagcaacttttcaacgaccgattgaaagaagatgctctaaagctcaatacttctcatggggattcacttggtaaatttcaacgaaattttccgttattaattaacacgttatcaacgttcgttgtcgatcttgataattctcaatatactttgactgatttttttctggctaaaaacgtttcatttcttgggaaaaacatagataacttagatttttatcttttccctaaagatgcagattttaagattgtatcaatcacttcatccgaaactcgggattaaagtgcttgatatgattcagcacatctcctagctcagcacttagctgctgagctttttttatttctgaaagaagaatacttccattctccaagatgagagaaatatttgtgctttttgcctgatctaataaatcaatttgttttaattcaaaactggtgttcttatcgatcatctttctcacttccttttgataagatctgacgtggattaattaatcgtcgtttttgttgtcttcaatttccacattcttcactccataagcgataaacttattaactaccgctgtgacagttaatccagtttcgtgcttaatatccattaactggttatacaaatcagtgttaatgctaatcaatcgtgatactcgtggttctggtgtaaaaggcacccgtaaaatgtaggaaaacggcaggttagaactgttggttttcctacattttttgtatcatgaatcacatcagagtgtaggaggaatttgatgtgagacgtgatttaagagaaggagtgacgatttacgtgactgaaaatattaagcctaacttcgccgagattgcccggcaatataatgttgattatcgaaccgttaagaaagcctatgaggaagtcaaagctggacttaagggccgaccaagtggtcgaccgaaacggccaagtttactggatccattcaagcaaaccatcgattcaaagcttgaactaaattgttcggctgcttcaatttttaaatttatccagaagaagggctttaccggcagctataccctcgtgaaagattattgtcgccaaacccgccgagaacgagttaagaaagctaccattcggattgaacattcccctggtctctctgctcaagttgactggaaagaagaaatggccctagtgagcagcgagggtgagctgtttaaattcaatattttcttgtatgtattgccttattcaaaactcaaatatatgacactaacctttgatcggagccaagataccctcttttcttgcttacacgacgctttccttcataccggaggtattccgacggaaatctggtttgataatatgaaaaccgttgtggatcatacaaaatcccagtttggccacgctgtctttaacgaacggttccacgaattctgtaaagatgccggtttcacaccaattgcttgtcgaccattcagaccacaaactaaaggtgcagttgaagcccttgctcgcacggttgaacgtttacggccatacaatactgaatttgctgatggaactgagctaatcgaactagttcatatgctccgagatgatctaaatcatgaaacttcgcaggccacggacgaagtcccgtacctgaaatggttagacgaagaaaaagagtaccttcatcgcgttccagttaatctccttgaaccatacttcgaagaaaacattacccgtgtcgtttcgaaggaggccatgatcaatttccgcaaatgtaagtactcagtagatccgcgatacattggttgtacggttgctgttgaaatctccaatgatgagcagcgcatccacatttattataacggagaagaaattcgtacgcactccataactaccaattcgctgaattatgacccccaagatcagttcaatatcctcaaatctgatttgcttaaagggcggacagatgaagacatttcagcttacattcgtgaacatatgactgattacgacaacttataggaggctaccatgaccactaataatcaaattcttttaaataatcttgagcgcttagggttaaacaaaatccgtgaatacttgccgaattaccttgatcaaattcacactgataatctgtcattaactgaggcgctaattgatttaactaattcggaactccagaatcgacacgaaggtcagattgcacgggccattggccgtgctcggttccccaatacaaaatccctagatacatttgattttagctttcaacccagtattaatcgccaagaggttctggaattccagaatctggcttttatggaaaagtctgaaaacttaatctttattggcaatccgggagtcggtaaaacccacttggcaattagtattgggattgaggcctgtaaacagggctgtcgggttctctttattaattgtcatgagctgttgattagattgagagcagcttacgaaaaaggactgcttgatcgatctctaagccgctattcgcgctatgacctattaattattgatgaaattgggtatttgccaattggtcaccaagaagctaacctcttatttcagctagtcaatgcccgctatgaaaagcattcaacgatcattaccagcaatagtgatctatccgcttgggttgatattttccagaacccaactgtgacagcagccattctcgatcgcttggttcatcatgttcacgtagtgaagatcactggtaaatcttaccgattacgtggcctcaagtaactgccgaaaacctacatttctttctgccgaaaacctacatttttaaactgcccttgacattctggtgctttcttttctaaaactaaacgtggttttgccattttttattacttctttctattatttactgacgtataatttaattaattcaagtaatcgaggtgaaaattgtgacttataaacgtgctgaaaaagttttgaagaaactactatcattctcaaaagaaccgaatttagcgtttgaattcaatcaaataattaaagactctttaaaacgtatttctggcgataaattggagatcgacttagattttttaaccaaagaaggtttaattggatccattagtattaactcctatcaggcaatttatgttacaagccacggttacacttactttgatgaaaagcacagtctggataaaggagttcacctgacagaattaagagttcatgtgctttatccatctatagttgcgttcataacattttggcttggcttctttctaggacatatgaccaagtaagtaaccaattgtcataaatagaactcctatcgccacatttaaaataggctgaatattactatcaaagtactgatgcagtttgcctttttccatttaactcacctcctttctatgctggctgtgtggacgtatccggactaaataaaaacttgattgtcactctgaaaagctaattcaagatcagtcacgttcggtgtcttttaggacactagttcagcaaaaaaaatatccattacgtcttcggaatttaaatctaatactttagaaagagccattatctcatctgctttaaatgggcgaatatctcttaagcctttatagaaagtggaattagacattgaaactcccatattgtttacagatttaataacatctgaaactctctttcctttgagcttaatggcagccaatagtttatctttattcatgtaatcatctcctttgtttcctttaggacacttttaattaaaacacctgtcattttctttgtcaatagaaaaatgtctttatttgcatttaatatgcgtaaaaaaatattatgtgtattttaagacacttttgtgatactattattgtataggagtgatgaactttgtctattaatttaagaaatagaagaaaagaattaaatttaacattggaagaagttggaaaaatggttggtgttggtaaatcaactattagaaaatgggaaactggatatatcgagaacatgaaaagagataaaattattgcactctcaaaagcacttaaagtaagtccaatggatataattgatcccaataaagaaatttcgaatcccatgattgataaaattgaagaaatatcaattcagctccacccttctcgtcaagaaaaagtttacaattacgctagtgatcaattaaacgaacagaataacgaaaaaataacttcaatgtttgaccacaagccgatgattgaaattcctgctgggcgttcaactgctgccgggtctcctattaacggtgaggatcaagatacccaattaattcataaaatgattgccggcgaaaaagttcctgccggtgcagatgaattaattactgtggatggtgattcaatggaaccgctcttaaaaaagggtagtcaagtttttatccactaccagccagaagttgagaatggtgaaattgcgatcgtccacattcgtgatgttggtgttacttgtaaaaagttttatgtaaatgaggataataccgttaccttaaaatcaattaacaaggcatacgatgacatggtgtttgattgtgatgaagttaatgtaatcggtaaagtgatcttatgagctcccaaatgtgggggcttcatttaaagttttaaaagaacatatgtttcgactaaccaggtggtttacttaggttcgagtcctaaatagtcaatatttaaccgaaaaaaataaccaacgtcctctggataaacgttggccacaggaaagaatcgatcgtgaagcagctaatatgtattacaaatttttggtaaatatccacgataagatcagcagtaattttaaaggacttgccaaacatgatccgaataaatggcgacactttatttcaattaatgaaatgcttgaacagttggaagaatccgtcgttgagatagaattcgaataaaaaattccacccatcggagcaattagcggtatcattttaattagagttgtccaaatactgaagacagtaaaagctgaactataagggagaatgtttaaatatgaaaaaaacatttttgtacgttggattatcacttccatttttatttatttctatagctggtgctaagggacttcaccatggatttgttgacacccattcgcaagtattatccacagctcataaaattagtggccgcactgaaaagggagcaactattcacgtactacaagataaacatataattgccactggaaaagcagatcatacgggtaagtttaatatccatatcaaaaaagctttgcctcttgaccataaatattttgtagtctcttcaaaacacggctataaggttgctaagaagggatttttagtttatcggacgaatgttccttccacaacaactacgccggcttcaggtagcagcaatacacaagctcctgtggcaagcagtagttcatcctcatcttcggcatcgtcatcaagtagttctgtacaaccaactaaggaatcttcacttgatggaaaaattacaatttcatccattgcaccagacaacactactgatatttccggacatcaaaacggcgatctgtggtatgtccaagatggaagccataatacaacagcaatgtacgagtttaataatggtaactggcaattaaaactttcatcaaactagtagatacgatatattgatataatgattaggaaaccaaaaatggtgcattcccaactaatcaaaactagatatatacgtttaaggttggtactgtaaggtatcaatctttttgaatacaaatgctcctatgattatctgaattttgaccattatcgaactagtgttcaaatggaattatttgcttaatttaatcaatgcaaaagaaaaagcaaatcctttcggatttgctatatgagctgatatcaacctcagttgacaaagagcccgaaaacattgacacttctttattttacacaagcttatattgattatctaaagcaaaaattaattaaacggtgtaacagtaacagttgaagtggaatcagatggtttagtaacagatgatgcatcaggataagtatatactaccttaacactaccatttgtattaaatgaaccattgtcagcactattagcagtataagtaaactgcttatatcctgtaataactaattgcttagatgtgttacggccaaatacagggaaaacagggctcttaagggtatccaaactctttgtcttcaaataacttaaaacatcactcgaagtgaacgtttgacctgaagcaccattaaacaaagcagaaggatttaaattggatggtgcaatatactgagcagaagctgctgacgatacagctttattcaacttaaccaaagttggagaatcaatttgagttgtatttacttgaagttgacttgcaacacctgtaactgtaaattgcttaccattccatgcattagtgatatcatcatttccaactttagcaattttatttgaagttactggtactaaatgactggctggagtaggattaacagtagaatcacttgctgaacgactatatggtgttacttgaacaaatacttggttcccctttgaaagcaccaaagtaaccgaagaaccagtggttgcttgagctaattgagcaacttgactagcagttaattgaccattagtcaatgaataggaagtgccactaagagcactatttatatcacttgtaattgtcttttgtaactgagaatccaatgaccaagtataagttccagttttattgatctcactcaatgtacctaaagtatcaccctttttagcattaggcttagttacatcaagagatttaatagcagtaccatcagttccaactaaattgatccgtacagcattgtcagcaactgtaggagcagctggtgtagcaaccttcaaagcactgaacttgatccaaccattagccttagcattggctgagtcagtagctgcaaccttaacccaaaggtcaccttcacgagtacgagtagtttggtctgtaatcttgaaagtagcatccttatatggagttgagtcggtaattacgcgaccttttttatattcagtccatgcagggtaagtgtaagttacttgagtaccatcattggcagtaccagtggtagcaatcttgtaagtagcagctttttgtgcatcagttaaagcagtagtttgttctgctgaagatgcagagcttgcagaacttgctgatgctgattttgcagctgcaggtgctgtagtagtgttgaatgaagcaataccaccagcaaatgcagtaactgacttgccgccgtagatccagccacggtaagtcttatcaaatgaaacaaccttgtagtaaactgagccacggttagtagtagctacacgataagcacggaagttcttttgaccttgcttagagttcttaagagcagctaatgtagtcttagttgcaacggtcttagcacccttcaaagtaccagcctttgtataaagagcgttagtaccgttaacagcaacgttacgagtagtagcatcagttgtcaaagctttgtttgatgtaactttggcatatgattttgcactagcatttgtgctagatacaccggcaacagctacaaatgataatgcagctacaccagcaaaaagagtctttttcaatgactttttcatgtataatttcctcccaaaaaaattgttttttcaagctacctaggcatgcaaaaacatgcctcaactaacttgctgtaaatagtataacataatcaaggttgaatgcaaaagaaaacaggagttgtaaaggctttaacatttttttgtaatctatatgccatgataattaataaatgatcgctctattaaggagtttccccccactatgtgttagtatattatccaaaggagggtaataatgccatcaatacgtaaacatggtcatggataccaagtaagatactactattatgatgccaatggccaggaacacgagaaaacaaagagcggctttagaactaaatcagctgcaaaactatttgcgagtcaattagaaatcgatatccacaatggtttggatctcgttcctaaagatcctaagtttgctgactattttgactatttttatcacacgtacaaagagcctaagattgaaaatcagactaagaatcgctataaaataactagtcgcgtattacataattatttcggtgatgttactttaaaaagtattgaccgcccacaatatcaagcatttattaacttctatggtcattctcatgcaaaagatactgtttataaagttaattcactgattagagcaaccgttcaaaatgccattcttgacgatctgattcataaagatttcacccagcgagtcagtcttatttatgataagtcacgtgataagcatgtggaatacctcaacgtggctgagattaagcgtctcatcgcttatttggagaatcacttaaactatcactttacctccacttttatgatcctgacggccgttttaactggtgctcgcttgggggaaattcaagcattaacttggaatgacgttaattttaattttaaaacgattagcattactaaatcttggaattcatccgaaggcggtggattcaaagataccaagacggctggttcaaatcgaatcattgcagttaatgacgaattgctgaaatcattaaagatcttgaaggatcacaataatggagaactaatttttgttaatcaatataaatccattccatcatcctctgccgttaataaaaagttgcgttctatactaaaagacttaggaattaaaaagcaaggctttcactttcattctttacgacactcacatgtagcttacctactatctcgaggaattgacatttacatcatttctaagcgtttaggccatgctgacgtatccacaacaacaaagatttattcctatttaatggatgaatataaagcaaaaaacgatcaacagattcgtgaagagttagataacctttcctctcatgatgaaactataccaattaagcggaacctttaataaggttccgtttttattttgttattttactctgtatcaggttaaacttcttctgcccgtttggccgttatttgcccgttattatttatattttaatactttctagtacgtttttataaattaaaaaaatcaagaatgccgttaaataggcattcctgattttaatatttcttctaatttgcataattatgccgactgcaggagtcgaacctgtgaccctcggtttacgataccgatgctctaccaactgagctaagtcggcaaatccattgtacaaaaaatgctaacaattaagttagcatttcgacaaagctccggcaggcgggctcgaaccgtcgacaacctgattaacagtcaggtgctctaccaactgagctatgccggaataatcgcgtggcaacgtcctaccctcgcagggggcgatcccccaactactcttggcgtgcagaagcttaacttctgtgttcggcatgggaacaggtgtatccttctggctatcgccaccacactatttttccttgaaagaacttcgttctctcaaaactagctaatattaattttctgcccttgaacaccatttctacttggttaagtcctcgaccgattagtattggtccgctccgtacatcactgcacttccacttccaacctatctacctgatcatctctcaggggtcttacttccatataggaatgggaaatctcatcttgaggtgagtttcacacttagatgctttcagcgtttatctcatccatacgtagctacccagcggtgcgcctggcggcgcaactggtacaccagcggtatgtccatcccggtcctctcgtactaaggacagctcctctcaaatttcctacgcccgcgacggatagggaccgaactgtctcacgacgttctgaacccagctcgcgtaccgctttaatgggcgaacagcccaacccttgggaccgactacagccccaggatgcgatgagccgacatcgaggtgccaaacctccccgtcgatgtggactcttgggggagataagcctgttatccccagggtagcttttatccgttgagcgatggcccttccatacggtaccaccggatcactaagcccgactttcgtccctgctcgacctgtctgtctcgcagtcaagctcccttctgcctttacactcgttgaatgatttccaaccattctgagggaacctttgggcgcctccgttactgtttgggaggcgaccgccccagtcaaactgcctacctgacactgtctcccgccacgctgagtggcgcgggttagagtgttcacacagcgagggtagtatcccaccaacgcctctgccgaaactagcgttccggcttcaatggctcctacctatcctgtacaagctgtgtcaacacccaatatcaagctacagtaaagctccatggggtctttccgtcctgtcgcgggtaacctgcttcttcacaggtatcttaatttcaccgagtctctcgttgagacagtgcccagatcgttacgcctttcgtgcgggtcggaacttacccgacaaggaatttcgctaccttaggaccgttatagttacggccgccgtttactggggcttcatttctgggcttcgccgaagctaactcatccacttaaccttccagcaccgggcaggcgtcagcccctatacgtcatcttacgattttgcagaaacctgtgtttttgataaacagtcgcctgggccttttcactgcggctgtgcttgcgcacagcaccccttctcccgaagttacggggtcattttgccgagttccttaacgagagttcactcgctcacctgaggattctctcctcgactacctgtgtcggtttgcggtacgggtagttgatgactcactagaagcttttctcggcagtgtgacgtcggttgcttccctacttaaatttcggtcctcatcaccacttgtcaacccgccaaaaagcatttaactctttgactgactcgtggcttgaacatccctttccaactggatgcacaacttagcctcctgcgtccctccatcgctcaaacatcatcaactagtacaggaatctcaacctgttatccatcgcctacgccttgcggcctcggcttaggtcccgactaaccctgggaggacgagccttccccaggaaaccttagtcattcggtggatcagattctcactgatctttcgctactcataccggcattctcacttctaagcgctccaccagtccttacggtctggcttcattgcccttagaacgctctcctatcacttgaccgaaggtcaagtccacagtctcggtaatatgcttagccccggtaaattttcggcgcggaatcactcgactagtgagctattacgcactctttaaatgatggctgcttctgagccaacatcctagttgtctatgcaactccacatccttttccacttagcatatatttagggaccttaactggtggtctgggctgttccccttttgacgatggatcttatcactcaccgtctgactcccggataaaaatcaatggtattcggagtttatctgaacttagtaacccatgacgggcccctcatccaaacagtggctctacctccatgattctacgtccgaggctagccctaaagctatttcggagagaaccagctatctccaagttcgtttggaatttcaccgctacccacacctcatcccagcacttttcaacgtacacgggttcgggcctccagtgcgttttaccgcaccttcaccctggacatgggtagatcacctggtttcgggtctacagcaacatactaaaacgcccatttcagactcgctttcgctgcggctccggcttttaaaccttaacctggcatgttaccgtaactcgccggttcattctacaagaggcacgctatcacccattaacgggctctaactgcttgtaggcacatggtttcaggaactatttcactccccttccggggtgcttttcacctttccctcacggtactggttcactatcggtcactagagagtatttagccttgggagatggtcctcccggattccgacgacgtttcacgtgtgtcgccgtactcaggatcctgaactgagggtcattgatttcacctacggggctatcaccctgtttcgccaaccttcccagattgttcgattatcaacaactttggtaactcaaatgttcagtcctacaaccccaatgagcaagctcattggtttgggctgttccccgttcgctcgccgctactgagggaatcgaaaatttctttctgctcctgtgggtactgagatgtttcagttccccacgtctatctctatacagctatgaattcactatatagtaacagtcgattaaaactgatgggtttccccattcggaaatctccggatcaaagcttacgtacagctccccgaagcatatcggtgttagtcccgtccttcatcggcttctagtgccaaggcatccaccatgcgccctttttaacttaacctgtacatcacgacgtgatgcaaagttaattgagtatttgcgatttttttctagttaacaaactcaaaataacgcggtgttctcagttgaaattatataaatacaatttcaaaaaaattattacagaaaattaatattatctagttttcaaagaacgaattgagagtagacctctcaaaactaaacaaaactttcgacaatgtgcaggattccgtttttccttagaaaggaggtgatccagccgcaggttctcctacggctaccttgttacgacttcaccctaatcatctgccccaccttagacggctggtccccgaaggttacctcaccggctttgggtgttacaaactctcatggtgtgacgggcggtgtgtacaaggcccgggaacgtattcaccgtggcatgctgatccacgattactagcgattccaacttcatgtaggcgagttgcagcctacaatccgaactgagaacggctttaagagattagcttgacctcgcggtttcgcgactcgttgtaccgtccattgtagcacgtgtgtagcccaggtcataaggggcatgatgatttgacgtcatccccaccttcctccggtttgtcaccggcagtcttgctagagtgcccaactgaatgctggcaactaacaataagggttgcgctcgttgcgggacttaacccaacatctcacgacacgagctgacgacaaccatgcaccacctgtcattctgtccccgaagggaacgcctaatctcttaagttggcagaagatgtcaagacctggtaaggttcttcgcgtagcatcgaattaaaccacatgctccaccgcttgtgcgggcccccgtcaattcctttgagtttcaaccttgcggtcgtactccccaggcggagtgcttaatgcgttagctgcagcactgaagggcggaaaccctccaacacttagcactcatcgtttacggcatggactaccagggtatctaatcctgttcgctacccatgctttcgagcctcagcgtcagttacagaccagacagccgccttcgccactggtgttcttccatatatctacgcatttcaccgctacacatggagttccactgtcctcttctgcactcaagtctcccggtttccgatgcacttctccggttaagccgaaggctttcacatcagacctaaaaaaccgcctgcgctcgctttacgcccaataaatccggacaacgcttgccacctacgtattaccgcggctgctggcacgtagttagccgtggctttctggttggataccgtcaagatgtcaacagttactctgacacctgttcttctccaacaacagagttttacgagccgaaacccttcatcactcacgcggcgttgctccatcagactttcgtccattgtggaagattccctactgctgcctcccgtaggagtttgggccgtgtctcagtcccaatgtggccgattaccctctcaggtcggctacgtatcatcgccttggtaggccgttaccttaccaacaagctaatacgccgcgggtccatcctaaagtgacagccgaagccgtcttttaaaccaaaaccaggtggttttggttgttatacggtattagcacctgtttccaagtgttatcccctacttcaagggcaggttacccacgtgttactcaccagttcgccactcgtctcaatgttaaatctttcaagtgcaagcacctaaaatcattaacggagacgcgttcgacttgcatgtattaggcacgccgccagcgttcgtcctgagccaggatcaaactctcatcttaaattgtttaaaatgataagcctgtgatagctcatgatttaaatttattatttgtttttacgaattgacttcgcaaatgtttggttccaattccgaagaattgaaacgccctgcacatttgtttgtcgaaaattttgttcagttttcaaaggtctacttggttgtggaagagatgaatcatctctcgcgacaactatttaaatataccacgctgattgctcagagtcaacaaaaacttttttgattaacacgctttgttgtgtgttccgttcaaatcagcatatataaatatatctgattctcaccgattcgtcaagtaaaaatcgaaagttaatttgcaatcacaattcaaagtggtctacgtgaaggtgacagctaaaaagtttgaagcttcttcgaaaaaatcgccaaaacaaaaagcaatccaggttggattgctttaaaaaattaatcgttattcgtattatcctcggggcgcatcgttgggaacagaatcacgtcacgaatggatggtgcatcggtcaataacataaccagtcgatcaatgccgattccaagtccacccgttggcggcataccatactcaagggcttcaatgtagtcttcatcaattccttcagcctcttcgttaccagctttacgttcagcaacttgagcctcaaatcgttgacgctgatcaattgggtcattcagttcggaaaatgcattggcgaattcgttagttaaaatatataactcaaaacgatcggtaaatcttggatcatcatggttcttcttggccagtggtgaaatctcaaccggatgcccataaataaatgttggctgctccagcttaggttgaacgagctcctcaaaaaatgcattaataatatggccggtcttccaccatggttcgtaatgaatatggtgttcatcagccaattttttagcgtcatcatcagacattggttgccagaaatcaattccggtatattccttaattgcatcaaccatatgctgtcgtttaaacggtttgttcaagtcaacggtgtggccttgataagtcacaacattatcatccgtaacagcagctgctgctgccttaaagatgccctctgtttcatccatcacatcatggaagtcataataggcaacataggattcaagcattgtgaactccggattatgacgggtatccattccttcatttctgaagacccggccaatttcgtaaactcgttccagtccacccacaatcaatcgcttcaaatgcagttcaagcgcaattcttaaatacaagtcgatattcaaagcattgtgatgggtaataaagggacgggcattcgcaccacccgcagaattatgcagaactggggtttctacttcttgataatcgtttgaatccagatacttgcggacagcagaaacaatcttcgtgcgcttaacaaaacgatcgaagctgtcctggttggaaatgagatcaaggtagcgctgacgataacgctgttccttgtcctttaagccatgaaatttatctggtagcggccgcagcgcctttgacaggaaagtaactgactctgcacgaacagtcagttcacccatgtctgttttgataatttggccggaaattccgaggtgatcaccaatgtcggatcgtttaaaaatatggtaaatgtcatcgccgacaatatccttacgaacatatatctggatttttccagttcgatcctttaaatcggcaaaaccgaccttacctttaccccgcttagcaatcattctgccggcaatggtaactttcttgtccttttccattaattcatctttatcttcatcatcaaaatcatgatgcagttgttcagcaagatatgtacgcacgaatcgatgtccaaatggatcgattccttccttgcgtaattcgtccatcttctggcgacggacgatcatttggtcattcatttctttgtctttggccactgtgaaacctcctaaatgaaaatttactattaataatcataacacaaaaagcgccgaatttattgtgctatccggtgctgacgtgcttttcgctgttcgtttttctccaaaaattcatcaaaaatatcatccatcgctgattcgccggatgcgttagtcaaggcaaccttggttcgagctgaatgaggaattccctttaagtaatagccggcttggccgcgaaattcgtgggaaccgatataatcacctttcaattctaccaaacgatgcaaatgttccttggcagtaaccaccttttcctcaggtgtcggctcagctaacagctcgccggtttccaaataatgctgcgtctgctttaagatccacggattaccttcgaccgcgcggcccatcataacagcatcagtgccaacttcagttaacatctttttggcatcttgcggtgttctgacatcgccatttcccataaatgggatgtgaatctcctgcgcaacctgcttcaaaatgccccagtccgcatgcccctcgtacatttgtttccgggttcgcccatgcatcgccaaagctgaagcaccggctctttcagccgctaaagcgttctcaaccgcataaatgtgatcttcatcccaaccggttctcatcttaacggtcaccggctttttaacggcatcagttacataagaaaccatctcatagactttctttgggtccagcagccaacgagcaccggcatcagttttaacaaccttattcacagggcatcccatgttgatgtcaatgatgtcagcagcagtattttgatcgacaaatttagcggcctgaaccaacgtttccttggttccgccaaaaatttggatactcatcgggtgttcgcggggatcaacaaacatcatatccaacgtttttttgtttttgtacataatcccacggtcagaaatcatttcacaaacaactaggcctgccccatattctttacagataattctaaaggcagaatttgtaacccctgccattggtgcaacaaccacctgattagggattgtgacattaccaatattccatttcatactttcacctcaaaattcgtttgcaattgtgaaattccgcttgctatattatcacatatttgtgaaaaacgacagccaactttagtggtggccctcagctttggcgactttaatgatttttcccagctcttcttcattaaaatggtacttgctttcgcagaagttgcaagtcacgtcaattcctttatcctctttgagcatcgtttccaattgggggacggggaggccctcaagatctcggccaaaccgattcttcgagcagttgcagaagaattccaccggaacagtttccaaaaaatgcaactgacctttgccaaaaatgagttccaaaatatcttcaggactttgattgtccaataaaagctcagaaatcatcggcatctgtttaattcgctcgatgacttgattaatggcgtcatcagttgcatccggcaatacctgcacgaggtagccgccggctgcgccgattgtattatcatcgttgacaaacacagagacccccaccgctgagggaatctgttcagattgggcgaggtagtacgtgaaatcgtcgccaatctcacctgaagccagcggcacgcttccagtatagggatcctcaccttcggcagcgcgactcacctcaattaagccgttgacaccaaccgccttgccaacatcaattttatgatgggcattaagtggtaggtgcacatgagggttttgaatataacctttgacatggccgttcgaatcactatcagcgacgatttggccaactggtccttgaccattaattttaaccgtcacagcttcaccatttttttcaaccgattcagcaagcataactgtgccgactaatgtccgtcccaaagccgcggatgatgcactccaagtatcgtggtcttgctgggcagtcgttacaagttgcttggcattcacagcgtatgcccgaaacatgccatcggtcgttgttgctttaactaaataatcatccatatcttgcacctcttctaaaaaataaaaacgagtttagagataattctaccctaaactcatttttgaaatattcaactaattgttatcgtcattgtcatgattgttatcttttggttgatcattgttagagacgtcatctggtttttcagagccatccgtgctttgatcatccgaattgttttggtcagtgtcttgagtttgatccccagttgtatgacccttttccaattcagcttgacgttcagcttccttacgttccaattcacgcttggcttcttcaaaggttgccgcacgctcacttggaaattcacttgtatcggaactttcaggcattttacctgtgtgccaaagtgaaaggatctgcttctcatcaagggtttcatacttcaacaaggcttccgcaatcagcttgtgcttatcacgatgctcctcgataatcttcttagcagtgtcgtgagcttcgttggttaaacgacgaacctcttcatcaacagcagcaccggtttcttgagaatatcttggaccataagtgtcttgggcaggattttcaagctgtaccggaccaagtcgtttgctcattccatactgagtaaccatggctcgagcgatgttggttgcctgttcaaagtcattggaagcaccagaggattgtgagtcaaagacaatttcttcggcagcacgaccacccatcaaaccggcaatctgttccatcgcgtccttcttagacatcaactgctggtcttcacgcggcagcataatcgcataaccaccggcacggccacgaggtacgatggtaaccttgtggaccactcgggcatcattcaagaccaacccaaccacagtatggccggcttcgtgataagcaacggtttcccgttcctcttttgaaataacccgattccgtttggcaggaccggcgatcacacgatcttcggcctcgtccaagtcactcgcatcgatttgcgtcttgttgcgacgagcagccagcaaggccgcttcattcagcaggttggccaaatcggcaccaacgaatcctggcgtttgcttggcaatctcgtgcagatcaacgtcgtttgccaatggcttgttcttagaatggactttcagaattgcttcacgaccgttaatatctggacgtccaaccaagatcttccggtcaaaacgacctggacgagtcaaggcgggatccaaaacatcggcacggttggttgcggcaatgacaatcacgccttcattgccactgaatccatccatttcaaccagtaattggttaagggtctgctcacgttcatcatggcccccacccatgccggcgccacgacgacgaccgacggcatcaatttcatcgatgaagatgatggcgggagcagccttcttggcttgatcaaacaagtcacgaacacggctggcaccaacacctacgaacatttcaacgaaatcagaaccggaaattgagtagaatggcactccggcttcaccggccaccgctttggcaagcaaagttttaccagtaccaggaggtccctcaagtaacaccccatgtgggatggtagcccccaaagttgtaaatttccttggatctttcaggaattcaacaacttcgaccagctcttgtttttcttcctcttcaccagcaacatctgagaaacgaaccttattttgcttactgtcggctggtttggccttggatttgccaaagctcatcactttgccgtttccgccgccttgaccgccagcacggcccatcatcatgtagaagaaccaaacaaacaataacagcggcaagacgtaaaccaatagatttacccaaaaaccgcttgactcttcaggcttggcattcatcttaacattgttagattgagctgccttggtgatttcagcaattgaggagttattctcgaggacagttgtggtaaatttggtaacattcttagactgagtctggtttccaccaatgagtccagattgcacctgtaccttctgaccctgtctataagttccagttaccttatagacaccgccacttggctgtactgaaaagctttttactttgtcatccttcaagttcttaacaaactggcttgattggatttcctgcgatgtggtctggttggtatttccgttaaagaaatagataacccccattatcagcagaaatatgacaatgtaaaacagactatttttaaaaagcccatttctattcgagttcatcaacgtcctcctcaaaactaaatattttcatgttgatagtcaaaatactaacacacttgaccttttttgactattaattgtttgtataaatttcaggcttcaagacaccaatgtacggcaggttacgatacttttcgtcgtaatccaaaccgtagccgacgacaaattcgttgggaaccttaaaaccaatgaaatccgactcggcatcaacggctcttccagcgggtttgtccaacagggtacaaaccttaattgaactggcaccacgatcggcgaacgtgtccagcaggaacttcaacgtccggccagtatcgacgatgtcttcaacaattaagacatcacgcccatcaatgtcggtgttgatatcctgcagcaattccaccgtcccggaagattcagtcgcaccatgataactggaaacgtcgataaagtcgatttgcatgtatgaatcaactgctcgggcaatgtcggtcatgaagaaaatagcgccctttaagacacccactaccaccggcgtcttgcctgcataagtctgagctatttcttttcccagcctttcaacggctgcttgaatttcttccttgctgtaaagtacctttaagatgtcgttattcattacaaattccttttctttccaatcattatttttgtcggacttcaattaaaaaataaggcctcgtgtcctcggaatcccgagaaacaacggcatttttcagacccaacactgataatacggtacctctggcatcgaccagcaacaaggtccgctcacgttggtcgttgggaactttggcattgatcagcacccggctgaccttttggtgttgtccgtgaccgattgataatcgatcccctgcttttggagagcgaacctgcaacggtaaatctgtatcctgcaggtaaaaagttgtcagtttattgttagcaaccgttttgtgtgcagtgaacacaccaaatttggtggacggactcagagaataccatctgtctaatattaccataaaagttcgatctttttcaggtttaccaacgattttttgtggttccttacaaattattagtgattgatacacccgcctgacctgccatccagcctctaaatccattttggcttgcggtctggcggtctgctggatcagccccaaaacttcgtcaagttgatcgactgaaatgttggggattcgaagataatgttcgaacacttcttcaagcaaacacttgacgacactgtcgggaaaatctttgagggaatcgagatcaatttctgcccggtgcttttcggaaaaaccaactgcggaatgaatcagcggctgaatcaagaatttaatggcggccaagttgtcggccaactggttggtataactgagcacatgaggcaacagctgcggattctctgctttgagtaatggcatcacgccatggcgaattcgattacgttcaacagccggttgctgattggtttcgtcttcaaaccacctgagtccagttgtttgagcaaatgattccaactgctgcttgctaaacgacaaaagtggtctaatcatcttggcatctgcaaacgatcgggtttcgcgaatgccggtcagagaagctaattgaccgccgcggaccagcttcataatgacggtttcaaccagatcatcgccatgatgagccgtcaacaggcaggtactaccggtttccttcaaaacacgcttaaaaaagcgataccgaaaggtccgggctgccgcctcaatccccgtcgttgggtggtcatctttcgaccagacggcttgtttgagtaaaagcccgtattcactgcaataattcgatatatagcgggtctcttcaacactttgttcgcggagctgatgatccacataggcgacaataatcttgggccgaacagctcgcggcaggtgctgcagcaaatatagtaacgtcatcgaatccactccggtggaaacggcaaccaccactgcatctccagcctgccaccacgctttttgcttaacaatgaaattaaattgtttctgtaaatccactgtggcctccgcttatgacttgcaggtataaaacaaatatggccggtggcaaatgattgccccagccacaaacttattaattgtcaaattctaatcgattaactacgccggccgccgcgaccaccacgtttgccttcggtgttcttacgcagtgtggacaaacggtcttcactttctttcaaaaagccggacatcatgtcatcaaagctctcttcatgattattcgaatgattgttgtgagcagaactgccgccacgggaatgataaccgtgactttgatgattcccgtggttctcatgactttcgtggttattctcgtggaaatttctgtgagaatgattttcattcttagaatcttcatgttcatgattgtcagaagctttgcggatcgaaagactaatcttgttgttgccctcaattttgaggacctttaccgtgacatcatcgccgaccttcaaaacatcatgaatatccttaacaaatccgtcagaaacttcgctgatatgaaccaaaccggttcgatgatcacctaaatcaataaatgcaccaaaattcgtaattccggaaactttaccgttaactttttctccaacttcaattgccatctaaaaaaatgttcctcccatgtaatagtgttaccagtatatcatattttattttatctcgactagcgattgtcaaaataaaaggcgaagacaaaagtacaaatacttttggcctcggcctgcttgactcatcttatttgacatcataatcattaacatcttttggtgccttattcgggaaactataaactgtttcaccaggttttgtatagtaataacgatcacgaataatttgttccacgtaattcttgtcattcaactgggcgacttgcgttttgagttgtttctggtctgccttttgttgttttaaggtcttttgctcacgggcaattcgaacatgcacgtcagcgtaattcactttggcacgaacaatttggataagaaaaattgacgcaaagaacaggaaaatggcactaataactaaggcccgcttttttcgtcgattagacaaaacagcagtcacccttgagttattcaattcaatctctcggcgacgagtaaaatcgttgtcgagcttccgtactttcccactttgctgcgtcatgctaaatcccccgatcattcgcacgttctagataaattataccaatctatgggcatttgtctaggtgattccacatgttttcgggatttttatgaatatttatttattcgttgcgaaagtcgcgttcatagtcctcggaggtaatctcgtacatccgttctgcatcatcctttttagttgtatccaacagttccttgaccaagatcgtcagagtcttgttaccaaatttgatgacaacctcatcgttaggtttaacttcggttgaagacttggcggcccgcccgttgataaagatccggcccttgtcggcaatttctttggcaacagaacggcgcttaataattctggaaacttttaaaaacttatcgattctcatgagttgtgactcctttaatttttaagaacttaccaacaaacggaatggccaaccattcacggacagtaaatacgtccaacagtcgacaccccgcaaaaaatatgatcacgccaatcggaatggcagcgcagacaaccaacaaagcagcgattcttggattatcagccaagtcagccaggttaatcccaaataccgttgtccgaaccgcaatgaacatggtcaccagcacaaccgcaagcttgccaagctgcttaaaagaaatcaatttggccaactcttttcgactgagcaggttcatcaataacaccattaccattaagcttaacagggttgcaagactagcgccaatgattccaaagtgtgccacgaacaattgattaaccaacaccttgatcaaaaagccagcaagaatggcgatcattgtcctcaaataattatccttgctctgtaaaatcacgttataggtcatcaacacgctggttaaaacgatgctgatgcagtacaggctaatcgtcaaatttaactcagacgaagcaaataacaaccggttaatttggggcattagagcagccaacccgacactcatggcaagtgaaacagccaaattagttctcagattggtggccgcaacgtgttgaaacgtgacatcttgacgatgtttgtttgccaacaccaaaccaggcaaaacggcggttgcagacgcaatgctcaaaacttgtcccagttgaacaagggtctgagaacggtcgtaaattcccttgatattctgggcagcaaccagcgaatagccaaacgatcgcaatccagacacaacggaaaatgaatcagccaactgaagcaagagcatcactgccgataccaagcacagtgtgccgccctccagcaaaatgcgcttaattaacagccgcgtttcgatagtcggacgtcgatttcgccagtttgttggcaatgatctcgatttcatccaaatcaggatgaacaacagggcaatcaggccggcaattggtgctgacagcatggccaactgacccattcgatacgggctaaccgtcgatttgaaggcccagtagccaaccaatagaatactcgatactcgaacaacctgttcaatcacttgcgaatacgccgtcggccgcatttccattttgccttgaaagtatccccgccaggttgacagaaatgggacaaacaggaacatccagctgactgattgaaccaccggtgccaatcggggatcatccattttcccggcaatgaatccggcagcaaattgcaatatacaaaaagccaccaggcaaaccacgattaggatgttttgaattcgaatggccaacccgacctgatctcttggatctttggtgtcgaccactaatttggaaataaaaaccggtagccccgtcaaagcaaaggtcatcccaataccataaattggataaatctgttgataaacataaaagccgatgttaccaaccatgttttggaagggaattcgatacacagcacttaacaatttggcaacaaatgacgcgaccgtcagcagtaaggttcctttaagaacgagttgtcttcttgacctatttttcatcagactttaccttaccggcagtaccatgatgatgccgggtttttgatagttgtttgactaatgcaatcagcccgtccaaccactttgtcatgttgggctgaacagttaattgaatttgatacctgtcattttcggtgttaatggttgcccggaacttggtttgggcaatcgcttccaacaattccttgctggagaattctgtccctgcccgaggtgaaaatgtgatggtaattttgggctgattttggtgaatcttatcaaccaacgcgtaatcggagaacatcttcagctgagagatctttaacaggttggcgacgggttcaccatagtccccaaatcgatcgattagatcatcttcaacttcgtggagctgatcttcattttcaatttggcggatccgtttatacaattcaatcttttgttgattgtcctgaatataatcactcggcagataggcttccaggtcaagctcaatagttgcatcagttcgatactcaaagttcttgccgcgttttttggcaacagcatccgacagcatctgggtatacaggtcgtacccaaccgaatcaacaaacccgtgctgctgcttaccaagcaggttacctgctccacggattgataggtcccgcatcgcaatcttgaatccggatcccaattcggtaaagtcacgaattgcctccaaccgtttctcaccaatttctgtgaggaccttatttggtttgtacataaaataagcataggccactcgactgctgcggccaatccgcccccgcagttgataaagctgagagagacccattcgatcagcattctcaacaaatagcgtattaacgtttggaatatccaccccggtttcaataatcgtggtagttaccaaaacatcatattcaccatttatgaaatcatacaaaatgtcttccatctggttttcggacatttgtccgtgaatgtaaccgactctggcggaaggaaccaaggcactgatttgttcaactgtcttttcaatatcagaaacccgattgtgaaggtaaaagacctggccgccacgcgacatttcccgttcaatcgcctcccgaattgtgccggcgttttgctcgatgacataagtctgaatgggataacggttggatggcggcgtctcgattacagacaaatcacgaacccccatcatcgacatgttcagcgtccgtggaattggtgttgccgtcagtgtcaagacatcaacgtcagaacgcatttccttgatacgttccttgtgtttaacgccaaaccgctgctcttcatcaatgattaacaggcccaaatcattaaacttaacgtcttttgaaagcagtcgatgagtaccgacaaccacatcgaccttaccgtcttttaagccttggagggtctccttgacttgtttggcggtctgaaatctggaaagcactctgactgtaatcgggtactctcgaaaacggtccagcatggtttcataatgctgctgggctaaaattgtggttggcaccaaaaaagcgacctgtttaccaacttcaattgctttgaaagcagctctcaaagcaacctcggtcttaccgtaaccaacatccccaaccagtaaacgatccattggatgctgggtttccatatcccgcttaatttccgtcgcactccgcagttgatcgggcgtttcactgtaaggaaaggcagcttcgaattctgcctgcaacgaatcgtcttgcggataggcgtaacccttttctgcgcttcttttggcgtataaatcgattagttcatcagcgatgtcttcaatcttggaagcaactttggccttggtctttgcccactcactgccgcccagtttgttgatccgcgggtgcttatcttctgaggaaacatatttttgaattaaatttaactgggtgactggaatgaacaacttggcgttatctttataggaaatcgtcaaataatcctggtgcttaccgtcgacttccatggtcttcatgccttcataacggccaattccatggttgacgtggacgacataatcgccaggcttcaaatcggtataactcttaattctttcagcgttgttaaaggtggtctggcgggggcgttttttagtcaccgtgccaaacatttctttttcagtgatcaccacacaactggccaacggcagctcaaagccattatccaggttgctggagatgagctggacttcttgttttaaaagatgatccttatcagtctgtgtcgccgtaatttcaaaatcgttcagcgttgaagcgacctttgccagtcgtttctcatcttgaaccataatgatgaccgtctgcttcattttctgccagcgcaaaatctcggttcgaagcatcggaatttgggagaagaactgctgcatcggccgtacagtaatgtcttcaatggcatccagtcgcatccggcccatccccttttggaacagtgacagaattaaggtggcgtgatgattcgcgctaaaggctttcttgaaatcgttggtgtatgtggtagacttcaaaacctcatagtgcttaatcttgtcgttcaaccactcatcgtcatcgctctcaagctgtctggcagtttcagtaattctggcataatcgtcgaaaataacaacgccatcggcagccaggtaatccaacagggaggactgttttttataaatcatatccgcaaataacaaccagcgtggatcactcaacccattttgcagatccatgatttgtggttccaagttgccctgaagttttttggccgccttatcatccagtttactttgttcagcaattaaccgtttggacagctgcttgctgacggcttttcgctggtcatcggtcattaataagtccgtggctggcagtaccgtgattgacttgatgtttttgatgcttcgctgattggaaacatcgaatgtccgcattgagtcgacatccgtgtcaaaaaagtcaattcgaaccgggtcttgatggtttaatgggaaaatatcgagaatcgacccccgaattgaaaagtctcccggagccgcaaccattttttgaaaaacgtaccccatttgatgaagttgaagctttaattgctccaggtcataggtgccgtccatttcaagcgttaacttagcggcttgaaactgctttttctccggcaccagtcttctgataccggaaacagaggtcacaatgactgcgggatcgccgctggcaagcttgtccaacgctaatacccgttgggctttgtattccggtgaactggtcgccagctcagctgctcccatttcttccaccgggaactcaaacaactgatcgtcatcaatcaagttagataagtcattcaccaactggtcagcatgaaataacgagtcaactaccacaacagttggtttgtcagtcgaatgaattaaattatcgattaaaagtgtccgggccgaaccgccgactccggtcaccaattgacgcgtgcccggtttcaaggttgcgaccaactcctgatactgaggaattgttgttagtaattgatctaacttcaaaataatgtcctttcgttaattatactgattttccaaatccggaatcgacatcccatcaatccaatcatccaaggcattcacggcgtgatcagcagcctgcttaaagattggggcttgatctttgctgaatcggcccagcacgtaattaaccaccgtattgccatgatccgggtgatcaattccaacccgaatccgatcgaaattttgggtgccgacactggcaataatgcttttaatcccattatgaccgccagccgaacctttatccttaatgcgaatcttgccaaccggcagatccatgtcatcatgcacaatgatgagatcttcgattgaaacgtcaaagtagtccattaaggggcggacagccaagccggagtcattcatgaatgttgtcggctcgaccaccatcactttggtgttgttgacaaacccagagccatacttggcgttcattttacgcgtcttaattgaaatgtcatggcttttggcaaattgttccactaccataaagccggtattatgtctggtcccatcatattggggaccaatatttcctagtccaacgatcattttcattgtttaaattcttcctcacgtttcttccaacacaaaatgctgaacaaagactgttcagctgtcgaaaaattaattaacataaagattatatcatatcagacaagcttttaagtcctggaaaaaccggaaaattaaaagatgtttatcagtgaagacgccttcaaaatcatgctataattggcgtgttctaggaattatatattaatgatttggagatgatttttttgactttacaacgccaaaaagtagctttaatcggtgacggtgccgtaggttcctcatatgcgtatgcaatgatgcaacaaggcctcgctgaagagtttgtgatcgtagatgtgattaaggaacgcactgagggagacgcactcgaccttgaagatgcacaagccttcacctccccaaaacacgtttactcaggtgattatgcagattgtaaggatgccgacttggcagtcatcactgccggcgctccgcaaaagcctggcgaaactcgcttggatctggttaataagaacctcaagatcatgaaatctatcattgatccacttgttggctctggattcaacggcgtcattgttgttgctgccaacccggttgacattttaacttatgcagctcaaaaattctccggcttcccaaagaaccgtgtctttggaagcggaacttctctggatacttccagattgcaggtcgctttgggcaagaagttgcaagttagcccacaatcaatcagtgcttacattttaggtgaacacggtgattccgaatttgctgcctattctgcagctcaaatcggtggccgtccattcttggacgttgccaaagaagccggtttatcaatggataacttaaaagaaattgaagaccaggttcgtcataaggcatacgagatcatcaaccgaaaaggtgccacattctatggagttgccacctgtttgatgagaatttcacgagctattttgcgtgatgaaaatgcagttctgcccgttggtgcgccaatggatggcgaatacggacttcatgatgtctacatcggttcacctgccgtggtcaatgcatccggtattcaaaaggttgttgaagttccacttaacgccgatgaagctgccgcaatgaaggcctctgctgagacccttcaaaagacgactgctgatggcatggcagaactttaattccactgtttgtaatgacaacaaagggatgatgaatcagcatccccagcctcaataattaatcaaaacggacaattatttctatcacataggaatgattgcccgtttttttaggaagtcctagcaagtcaacagatggaacatttccttgtgaccagcttgtcaccttattcaagtcagattttcaatcggcattctaatttatttagagattaatgagaataattcaagtttaaatgttcttttctaaatttctctatgttatcatggttgtatacaggttaagttggaggaattaaacatgctattaaaaacattagtaaagcctaaggaacgactggtgaccgtcaaagaagacgccaccttggaagaggctttacagactctcgaagattccggttatcgttgtgtgccaatcttagatgaaaccggcaagattttccgtggcaatatctacaaaatgcacatttatcgtcataaatcacggggtggtgacatgtcacttcccgttaccacacttttaaagaatgcaaccaagttcatcaacgtgaattctgcgttcttccaagtattcttttcaattaaggatctcccctacatcgcggttttggacgaacggaataacttttatgggatcttaacccatacccgtctcttggacatgctgtcacagtcttggaacgtgaatattggcagttacgtgttaaccgtcgttgcaagcggcgagcgtggtgatcttgaagaaattgccaaaattatcaccaagtacaccaacattgccagtgttatttccttggacgctcaagaaggtgaattggttcatcgcattatgttcaccctgcctgccgaagtggatcaggatcgtttaaacagaattattgctgctttggaacgcaaggaattcagagtgcctgaagttgaaaatctgcaagaagaaaaaaattaggcacgttgtacgtgcatatcaaaagaagaggccaagacacaactaattggaggttgtgtcttggcctctcctgcgttccaacgttacctagttcaagcgtggaactatcggctgatcccagccatttaagcaaagaaacgagtcattccaagacaggaataactcgtttctttgcttaaattccgggatcaaaacgcctcgcgtcccactccctcttgattataattgtattcaattgatctaagcgttgtgtgatgttttatgtattgcggtccgtcactagcctttagctaatcccaagcttatctttatcgctttatcgaccttactcataataggcggatcgagatgggttactttatccttcaatcgctgcttatcaatggttctgatctgctcgagtaaaataactgaatctctttctatcccatttccagctaagatccccacatgcgttggcatcttcggcttggaaattctggcggtaattgcggcaacaatgacggtgggactgtaatgattgccaatatcattttggacaatcaagaccggtcgcatcccgccctgctcggaaccgataactggtgatagatcagcataaaaaatgtctccacgtttaaaaataacgtcagtcaccctcatacctcccatcatcgtaacttacattactgtaaattccgtaatctttgacgatactgagttaaatggatatcagcgtcttcttcacagcaggaaaagtccttactgatctcacggttcaaactacccatttcgcgatatcccctcattaagccatcaatgactttcgggtcatcaaaaaagtagttgattgcaatctcaaccgctgcactttcggatattccaaccgttgcgctaaactgttccaaacggtctgcaatttgatcattgatcataactgaaaaatgctttgaattagttgctttttccattggtattttcccctatatgttccagattactgtactgtctaatataccatgaaattacagaaaaatcatacatattttcgacgcaatcgcggactcaagccacaaataacctcataactgatggtatgcagataatccgcaacatcatcggcagtaatctgagcatcacccgattgaccgatgatggtgactgtcgtgccgtaaggataatcatgaggcaatcgaatcataaactgatccatgcaaactcggccaacgatcggacacttgtggccatcaaccaagaccgaaaaaccttgcattgcccgaggaattccgtcggcatagccaaccggaacggtcccaatccactggtcgctatcagtagtgtaagttgcaccatacccgattgagcggccttttttaactaattttgaaaaatcaatttcggaggtgactgataaccctggcttcaactgatatggaagctgggtaatatctcttccggacgggttcaagccataagccgcaatcccaaagcgaatcatgttgccgccgcatactttgtgccacaagctggtagcggaattggccacatgaacatacttcgggcgtttatcaagaactgccataaagtcctgaaaattctggtactggaatttgaaataggtatcgtcaggactgtcagcggtggcaaaatgggtaaagattccttcaaaacacatccgatcggaatgggcgttgagaaccccaacggcagctttaagctcatccggagtttgaaagccaattcgacccatgccggtatccagtgccaaatgaatgtttaaccggcctttaaatgcgctggtgtcgagtaacttggcagcttgattaagccagtcgatcgaaccgacagtcagggaaatgttttcggaagccgctaattgggcacattcgggatcagtaatccctaataccagcaccggcagcttaattcctgcctggcgaagttggagagcttcatctaaaatagccacacaaaagccagtggcccccgctttttcagcaatctcggccacttgaaccgccccatggccataaccgtcagctttaaccacttggaacaagtcgtctccgtcatccaaacgctgcttggcatggtgaatatttgaataaattgccgccaggtcaacagttacctgggcatctcgtaaatttccaactgtcattacctaaccccgattctctaaaataacttgggtaacgacaatgtcatcggtgtgagaaatcgacacaaaagcgttcccatcaaacggttgtttcgaaaagaagggtttgccctcctcgttattaacaatacaaagatcctgaaatctcactttcgatccaaggccggaaccaaaggccttcgaataggcttctttggccgaaaaacgaccagagatatattcataacggcgcttatcagacaattcagccaattgtttcatttcatctgctgttaaaatacgctctgtgaaatgctgattccgttccacggctgcgacaattcttctaatatcggtaacatcaattccaattcctgcaatcattttctagatccctcgcaaaccaaaaagataggataagtttaacataaaaacggcctcctcggggcagatttgaagacttgtcacaaagtcaatgacgattaaccacatgcttgcattacaagttggtgcatacaaggaccttcatcaacgcaatcaaaaaaagtgaccattcatcatcgaatgatcacttcgttaaaaatcttaattaactatttttaatggtaaaacggcgtttcttattgcttgatgaccgtctgtcagaatgcttacggtcgttactgccttcataatggccccgatttcggctgccattattccggtcgccattacgatgactctttgagcccttgtaatgaccaccatgaccgccaccacgacgatcgttacgatgaccaccgtgtccatgaccatgatgtggcaatgggcgttcaggggtaatcttaaccttaacgttgtcgcgggtaacatcgttgagcagagcagcaaccaaatcagttgcttcatactcatcgagcagcttgtcagccatcttttcatacttgtcagtattagtcttcttaattaagtcggcaatatctgattcggcagaattcaattgaccaacgaaggcttcttgaattgttggtggcttcaaaggcagcatgcgcaccttggtcaacttttcaatttctcgaagataatccatttcgtttggcgttgcaaaggtaattgaaaccccatgcttaccggcacggccggtacgaccaacacgatggacgtagccatcaggatcttgaggaatatcgtagttataaacgtgggtcacacctgaaatatcaattccacgggcagcaacatcagtggcaactaagatatcaatcttggcagctttgaattcctgcatgatctgagtccgacgagcctgagtcagatctccgtgaagaccggcagccttgtagccacgggcctggagtcctttggatacttcatcaacccgacgcttagtccgacagaagacgatagttacttctgggtcctgaacgtcaaagaaacgggtcatggtgtcaaatttttcgtattcttttacccgaacatagtactgatcaattaaatcagtggttaattctttagccttaatcgttacttgatgagggtcacgcataaactgaaccccaacccgtttgatttgggcaggcatcgttgctgagaaaagcaaagtttgacgttcctttggggtttgcttgatgatatcttcaatatcgtctaaaaatcccatgttcaacatctcatccgcttcatccaacactaatgtcttaacgtgctctaactttaaagtatggcgtctaatatgatcaagaattcgacccggagttccaaccacaatctgtggatgaccctttaaggcgttgatttgacggcgaatatctgcaccaccgtaaacaacttgaaccttggctttttcatcttttcctaatcgatagatttcttcttgtgtctggattgccagctcccgagttggtgaaatgatcagagcttggacatttggattgtcaaaatcaatcttctgcaagattggtaaaccaaatgcggcagtttttccagttccagtttgagcttgaccgataacatcctcacctttaagaaccattgggatggtttcggcctggattggcgtagcttcttcaaacccactgttattaatcgcagttaataagtggtctgataatcctaattcactaaacttcaaatatgtttcctcctaatattgaaacaatcaaggttccgcggccgactggggaaaaatccgtttcccggaatgcgttggccacttgacctacaatcatttattacaaaataacctttttagtttacaccgtcacataacattaagcaagcaaaacaggccaactcatctgttgaccgtgcttatttaaccagtttggcaacaacattttccaaatgcagaccgtggctggccttcaacaagacctcatcgtcagctctcaattcggcttgaagatcagaggtcaattcatcaagctgatcagcttggtaatagtggagattctccggggcatagaccggcttgagtttctcatatagggcgtccatatcggcgccaatcaggtacaccacgcgaatggaggccggatccagggcatccgctagcgaagcgtgcatcgcttttgattgagtcccaagctccaacatgtcgcctaaaacagcaatccgtcgccccttggttgtcgtgttcttaaaagcggtcaacacttctttagcggcggtggggttagaattatagacgtcacttaaaattcgctcgccctttgaaccactcaaccactgggtccgattcttagtcagatcaaatttagccaacttgtcagccatcatctgcggataaattcggaaaattcggccaaccgaaatggccgccagggcattgttgacattataatcaccgatcatcggaatcgtaaaatcaatttcgggccacaaattgacgtgaaattgcgtctgatactgaccatctttggagtcggtggcaaaaacatcattgctgtctttcctgccaaaagtcgatttgatcacactctcatccacttgttgggcacgctctgtgagcagcggctcgtcgccgtcatagacgaagaagccgtcagctttcaggccatgagtgatctccattttggcgtcggcaatcttatcacgggtgccaaagaactcaatatgggcttcgccaatcatcgtaataacggctacatcgggccgagccagtttggatagaaaatctagttgcccgggtcgatccatccccatttccgccactaaaaactcggtattggattccatctgcagaatcgtataaggcaggccaatctcattattaaaattgtcctgggttttggtgacattaaacgtactggataaaatcgcggcgatcatatccttggtggtcgtcttgccgttgcttccggtgacggcaatgacgcgtggattaatcttatcaagataatacttgctgagctgttgaaatgctgtcagtggatcgtcaacaaccagtgccggaattgttaggggtaagcgatccgcgtggtcactggcccaaagggtagctgatgcgccgcccgcaattgcattgtcgatgtaatcgtggccgtcatgttctgcaaccagtggaacaaacagttgacccgtttgaatcttccggctgtcaaagcacaccccggtcaaagattcgtccagcattgctttgtcaaaattttcagtgttggcattaattgcttgagcaacttcgccaatcgtcattttcattattgaacgctccaattgttaaatagttatgttcaattataacaaaaaatcaaacggctaaacacccaccgtttgatcctgccattctaaatgccattttgatgtttgtaaattataggtcaagtccccggcatagacggtattttcatcgactttaccggttcgcaaaataattgaaacctgatccgggtccttcaaaatccgtaatgggatatgataagtccgggaacgttcacgcaaagaatcaaaggaaataaacaggccgtcgttggctttggtaatcaaatccaagaggatcgagcggtcaatgtctttgatcgccaagggacgcagaaagactctcaaagtgttatgggtttctcgcaaattgcgcttaatggcaatttccaagacgtggttaaagtctgagaagcgccggtaatatgaacgaatcgttccgttgtcttgactcaaataaatgtaatgattgttcaatttggaagaaaaaggccgacccattggcgttcccatgtgggccagatacaacagttccgcaatttcgaatggtgacaagttgttaacactgtcttccacgtcaaaatcaataaacttcttcttttggtcgggattacggaggagataggtccgaatttcacctgtgccattgatcagattgaacttggaatgagagttgtacccgttagcagcctgatcatcattatttaacaaaatgatattttgaggcaattcatccagtccattaataaaatcggccgcagtgatccctgatgataaaatcatgttggagattggattcgtatttataaaaatcaaattgcccttcatcgtttcattaccccgtatttatatctaaactaattgtactaccctcacgtttagttgtcttataattaagacagaaatgtcgtaatttgcccttttcttaattcattggtaacatggtggttaacgcaatattagtgtgaggttattaatatgactaacgtattatttgtttgtctgggaaatatctgccgttcgcccatggctgaggtcatgttccgtcaaatggtgaaggatgcccatttggaaaatcaaattaccgttgcttctgcagcaattagtaccgaagagcatggcaatccgcctcatccaggtgcgattgccgaattagccaaacacggcttgtccgtcggcaataagacgtcgacgcccatcaccaaagaagactttgatcaggctgattacattattgccatggataatcaaaatatcttttatctcaatcaaatggccccaattgccgatcggaaaaagattttcctttgctacaacattattcccgacaagcagggaaaagatatcccggacccctggtttgaccacaaatttggccgaacttaccgccagttatcagaaaccctgccaaaatggttggataaaatgaaaagccaagtggcttaattattgacgggtcccaataaggctcgttttaattttggtgtcgcatgactgattcgataacttttttggagtttaccgcgaatcatcaagcgtcccgcgccggtcgcgtcacaggtgatcaacgtgacaatcggccgcttggtttggcggacaacgtcaacccgggtcgctgcgataaacttgcgctggtaaaccttgtattgatagactttggtcatattactgagatagatccgatcaccaacttgggttttgaagtacagcgggccaaataaaacgtggcggttaaccatgtggtgccctgccaacggatagttgcccttgcccatctgctggtcaggccgcatggtcccggcagcgagcgccaaggtattattagccactcccaacccaattggcaaatgaatatgtgatttgggcaggagaatttcgccgataacctcaatggcgttagtgttcatccgcgcccgcgcagcagtttgaaaatcaagggatttgacttttttaaaatcataactgacattttgtttgtgacgcttagtttgcgctttttgccgccgttcagttttggcaacggtctggcgggtgatttttggatgataagatttgatcaattcatttttgattggccgattaaaaatcatccccaaagcgacaattaccaacaacacaaaaaccacgttaatcaatattttcttgagaagtccttttctcataactacctccactcaacaacgaattataatatgtacaaataataaaggaggaaccgcattgttaacaaaacaagttggtccaaactcctggcggcgcaatttagccgttctctggtttggaaccttcatggccggaatcggcttcagcgaagtgatgccatttctgtcgctatacgttgattcgctgggacatttcacccataacgaattgagcctttacagtggattagcctttgcggccagttacctagtgaccgcaattgcttcgccactgtggggaaaattggctgatcgaaccggccgaaaattgatgttggtccgagcatccgccggaatggccattgtcttcattttgatgggattggtcaccaacgtctggcaattaattggccttcggctcctgcagggtgtcttttccggatacatcagcaatgccaacgccctgattgccacccaggtgccgaaacgcaaaagcggccaggccctcggcactttggtaaccggtaacgtgtccggtgccctgcttggcccgctgttaggcggaactttggcctcattcttcagctatcgggtcacattctttattaccggtgccctgtttgtcggtgtcttcctggtaacgacgttgatggtccacgaagatttcaaaccagtcgccaaatcgaaaatgctcaatacgcgtggcgtaattggtgaactggccaattcaaaattggtactgggaatgtttgttaccaccatgattattcaagcggctaacaactccatcgttccaattttagcattatatgtccgccaaatcatgaataatagcccggcgaccaccttctatagcggaattgtcgctgcggtccccggcattgccaccttggcagctgctccgatgctgggacggctgggtgatcggattggtgctgatcgggtcttgctggtcggctttctgctggcaatcgttgtctacgttcccatggcatttgtcactaacgtctggcaattgattggtcttcggttcctgatcggtgtcgccaacgcgtcaatgttacccgctgtccagtcgattctggctaagaacaccccacctcacgttaccggccgtgtgtttagctggaaccagtctttccaggcgatgggcaacgtggctggcccaatgattggatcagtcgtctcaacctcatttgattacgcaggtgttttcatttcaactgccgtcctagtagttattaacctcaccttagtatttaacaatacgcggggaatgcgccgagcacgcaaacaacggattgaataaacccgtttacccattagtatgagaacgaaaaataggagttggacagtcagtatcgcttgtccaacccctatttgtttgcataaaaaacggggaaccgttaagctcctcgtcttcgtcatgcttatttgttgtctgtaagaccgtatttcttgttgaaacgatctacggcaccatctacttggttgaacttttgcttaccagtgtagaatgggtgtgaatctgatgaaatttcaacacggatcaatgggtaagtcttgccatcgtccatcttgatcgtttcgtcagaggttttagttgatcctgagatgaacttgaaacctgtagatgaatcttgaaatacaacttgttgatatgctggatgaattccttttttcattatctatcgctcctttgccctgaatcaatccgatgacccagagattatcgattagtcaactttgttagtgtaccataaataaaatcgtcaatcaatcatcaattgactctttcttcaacttctaatttaacgtcggcacccacaccccgcagcttatcaacgatgtttccataaccgcggaggatgttatcggcatggcagatttccgtggtgccatccgccatcagcccggcaatcactaacgatgcgccggcacggatttcacctgcctgaactttggcacccattagcttgggggagttatcaaccacaatgatgccttcatcggtatcttctgatttgactttaccgcccaatttattcagttctgtaatgtgcttaatccgtttggggtaaatcgtgtcaatgatcacactgcgcccctttgccttaaataatagcggcgtcaatggctgctgaagatcagtggcaaaccccggataaggcatcaccttaattcgaattggtttcaggtcatgtgatggtccgacataaatgctgtcctcatagaccgttaagtcgcagcccatctcttctaatttggcaacaaaggcttccaaatgttcggggatgatgttggtaatcaaaattccatcccccacagctgcggcgagtgacaaataagtgccggcttcgattcgatcaggaataattgtatgagtattacgagcctgaagggttggcacgccttcaattcgaatgacatcggtcccggcaccacgaatattggcacccatgttgttcaagaatgtcgcaatgtcaataatttcaggttccttagccgcgttgccaataacggtggttccaggcgccttgaccgacgccagaattgtattgatagtcgcacccacagaaacgatgtctaagaaaatctgggcaccatgcaggccatccgggccggtcttaatggtcactgtcccatcgtgttcactgacttcagctcctaaagccttaaatgccttgatatgctggtcaattggccgcggcccgatattatcgccaccgggaaaactaacggtagcacgctgaaaacgacctaacagagcgcccataaagtagtaggaggcccgcaagcttttaatcgccttgcttggcagtggtgcctcgacaatattggtcggatcaattgttaggacatcgcctttgaactcagacgaaacgttcatcgattttaaaattaacattaagttgtgaacatctaaaatgtctgggaccgagtcgaacctaacgggggtatccgctaatatggcagcagggataagcgcaaccgtgctgtttttagcaccgccgatcgatatctctccggacagccgtttccctccatttatgattagtttactcatcaaaaattcctcactttttgtattcgcacatttttcatgtcaagaaatatattatccaatatccacataaaaaacaatacctatacttgaattatacaatctgtaacaattaaaacaattgttccgtacaaacgttttcatttaatgagtgctagtcgggctaatttgacgccgttttcagcgaattattacaagacaaaatgagcacctgtttgcagtaatcgataaccagcgaacccgaaagcgcttttaaaatccaacaattcagtcggtttgtttcatcacccaacaaatggccagatctacttctttaactatccctgaaagtccttagaatattcaggcatacagaaaaaaggagcggttagaaatgaaacgactatttacgacaattggcgaaaatattcatcggcaccacaaactttggatcacggtcatcttgatcatgaccatcggttttgcatttggattgccaaagattcaaatgaaaatgggcaacgacgtcttcgttagttccagttcaaaaacctatcaggattcccaaacctatcagaaaaagtttggtggtgactccctttatctgttgctcgacggtaaccagtcgacattgttatcccacaagacaatgcagcaggtggccaaatttgacagtaaagtcagccaagttgataacgtcagaaatacgaccgacatcgtcagtagtttaaatgatcagttatcccatgccgggaccggaaattccagtgctcagttcaacttcaatagcaaaaagcttcaacaagatctcatggctgaactgagttccaaacaaaaacaaagcattcagtcgaaaatgcaacactcgttaacaagtacgcaacaaaatcaggttcaaacatatttgctgaaacaactcacgcccgcccaaaagaagctgatggcagcagctggtgcccaggcgcagggttccaagcaacagcagcaagcaatgcttcaaaagcaattgaccaccaaacagcaagctgcagtccagtcctacaccatgtcgctgcttaaccatcagcagcaatcacaattggcagacacggtcatcccgatgctgccgaaagttcaagatatgtcaaccaaactgctgcgggatatttttctcagcgataacggtcatgttcccagtgcgatgaagcaattattacctaaggacggcaagcatctattaatcattatcaataccaataagaaatcgtcggatatgaacaccgcggttcagattaatcacgacgctaatcaggcaattaagcaaaccaacttttcctcaagcattaagacccgattgggcggccaacctgcagttcttggtcaggtccgcagtaaagtcattaccagtatggcaaccatgttggcattcgcagtagtcttaatggtgatcatcctcctattgatattcccggtacgaaagcgtttgttgccactcatatttgtcctggcctgcctcgtatggacatttggtttgatgggttggcttcacattccgttgaccttggcaaccatggcaacgttgccgattatcattggtttggggactgactttggtgttcaatttcaaaaccgatatgaagaagaagtcaggaaacgacaaaattcccaggaggccatttcagttgccatttcgagcatgggaccggcagttggcgtgtctttaatcgtcatggtcttcagctttttgacgatgtatctctcaaaggcgccattgatgcagcaatttggcctcacgttggccattggtgtcgcctgcagctacgtcgttgagtttggactgatgttttcaagcctctcactcttggataaacacgcttcaacagctaagttggcacccaagaagctatctcagccgtcgcgtttatcactgttcctaagtcactatgctgaatgggtaacccatcatgcaggcattctgctgacaattggcgtggtgttggctggactaggtttttcatttgaaaaatccatcaatattgaaactgacttcaccaaaatgattccccaaaatatgacggccctgaagaataccaaatatcttcagagcaaaattgggtcgacaacctaccttacctatttggtagaggggaatggtcgagatatcagggatcaggacaatttgaagacaatcgatcaagttggtcaaaaagtggaccataagtaccatgacgtcaccgatgtcaccagcttatcgaccgcctatcaacagacgaacggctcattgaacacttctcaaaagcagttaactgtgggtgttgacaatttgccaacgtctttaaaacaaactttgattagcagcaaccatcacgatgcaacaatccaattcaaaattaaaaacggtctgtcctcaaaagaacaacttaagttgatgaatcggattaatcatgacattaaaggaacccatcatggcttaaaaatttctcctgcaggagcccaagtcatgatgctattggggattaataatatgtccgctaatcatgatctgattattattgccggtctttcgatcattttcattgtcctattccttatttatcgggactggcgactcgcgctgtacccagtcattccaattttactggtattaggactttctccattaaccttaaaactgttgggaatttcctataacccggtcacaattgccctcagttcgctggttcttggaattggaaccgaatttaccatcttgattctggaacgataccgcgaggaattacaacggggaattagtacccgggacgcgattgtttcagccaccgcgtctgtcggccaggcaattacagtttccggcttcacggtcatgggcggcttttcggccatcatgttctccagcttcccagttctgaagtcatttgggctgattactgtgctggacacaggttattcactcatctgtgcattgacgattttgccggcagtcatttatctgctgcgaaaaagaaagccggcagccactcaatcctcatccgaacaggcaactgaaagtaaggattaatcgacccattgaaatacccttttctaactaaaaaatggcttccataaatgaaattgattcatttgtggaagccatttttgtgtttgacgctgtttcttggcatctttgtgccatcaatcagccgccttaattactgagcgtttagtttattaatgattgaaatgagaaacgactccaactgcggccaatcaatattcgccttgagaagctgctcttctaaaaagcccattattgtattcgccaaaaaactgatcatcagcggttgtgaagacgattgcttaatcaacgttacgacaggatcattttgataggctggattgttggcccgttcattaaacaaattctccaaaatgttccgaaattcatcatagaacttgctttggctttcgggaatcagatggcgaattaaatcaatgttgtcggaaataaaatgggtaacctgggttaaaacaacggtttccctgaaatccgtccccagcaattcttcagacaggttatagataattgtatttgccagatcaaccttatcttggaaatatcggtagaacgtgctgcggtggatcatcgcttcatcacagatttctccgatcgtaatatcatcaaatttcttttttctaagaagcgtcatcattgcctgcaaaatatctcgcttggtgcgctgttgagattgggtgtcggccatagtcaaagtcctttcaaaatttagattataaaattaagtatacatcataaccaactattcttaaagaaaccaatgacaactttcacaaatttgctgccaacaaaaaagccccgacccgccacgggatcagagcttcatttgatttgttaaccgtcaatcagattcaccctaaaagtgtatcgtcagttacagacggtttatttatttttttcgagatacaggtcatttgccgcagcaacgaagtccttgaagagcccctctggacggttgggacgggaaataaactctggatggtactgtgaaccaacgaagaaccggttctttggaatttctacaacttcaaccaagtgattgtcaggtgaagtcccagaaatgaccatgccatttttctccattgcatcgcgataggcgttattaaattcgtaacggtgacggtgacgttctgagatgacatcggcattgtcataagccttggcagcaaccgttcccggctttaatttacatggataagcgcctaaacgttgagtgccgcccatatcgtgaacatcttcctggtcagccatcaggtcaatcacattgtgtttggtccgcggattcatttcagtcgagttggcatctgggtatgacaaaacgtcacgggcaaattcaacacaggccatttgcatccccaggcaaacacccagatatggaatgtcttgttcacggacatatttgatggccgtaatcatgccttcaattccgcgatcgccaaacccgccgggaacaatcaccccatcggcatctgacagcaagtcggcaacgttatccggtgtaatcttttcagaatcaagcatctccaaatcaatgtcggcgtcgacaacgtagccggcatgtttcagtgcttcggcaacagaaatgtaagcatcttggaggccaacatacttcccaaccagggtgatatgaatcgtccgtttgagatgttgaacgtgatgctcaagctgcttccattcagtcatgtcagcagctggcttatcaatgccaaagtgatcgaggatctgttgatccatcccctgcttttgcaggttcaacggaatggtgtacaaggttggcacatcaagtgattcaaccaccgcctgtggcttaacatcacagaacagtgaaatctttttgcgcattgagtcggtaattggcttttcggaacgaacaaccaacagatttggctgaatgcccaaaccacgaagttccttgacactgtgttgtgtcggcttggtcttcatttcaccagccgctctcagataaggaatcaaagttgtatgaacatagaagacgttttcgtcgcccacttcggtcttcatttggcgaattgcttccaagaatggcagtgattcaatatcaccaaccgtcccaccaatttcggtgatgacaatttcagcatccgaaaccttggcagcccgcataatcttttctttaatcatcccggtaatgtgaggaataacctgaacggttgccccaagataatcaccatgacgctcttttcttaggacttcatcataaatcttaccagtcgtcacgttggagtatttattgaggttgttgtcaataaaccgttcataatggccaagatccaggtcggtttccgtaccatcgttggttacgaaaacctctccgtgttggtagggattcatcgtgcctgggtcaacgttgatatagggatcaaacttttggatggtcacattcaacccgcgatttttcaacaatcggcctagtgatgccgcaacaattccttttcctaaggaagaaacaacgccaccagtaacaaaaatatatttggtcattatataatcctctcctcttgatagttagccggggaattcaaaaataaaaaaatccctatccaaaaaagtgaatagggaacaatttaatcatcgttcagatgtccttgaaactcaaggagcccaaaaaacataatacatactttttaaatattagtcaagaattaatggtcgtcttttgaattgaaatcatcatcgtcatcatccaatgaatcgtcatcatcattcaattcgttaagttgaccttcgatgccatctggcaagtcctcatcgtctgagtcatcgtcaatatcctgcaagtctttgttgtacttgccaagatcttctgattcatcatctgaatcgtcgtcatcatcagtatcgtcatcaaagtcatcgtcgtcctgatcttcaggatcatcgtcatcataatcgatcacgtcgtcatcatctgaagcgtcggcaagaaaggcattcaccttacggcgcttctttcgcttgggacgatcctcgtcttcttctgtatggacagttgcttcatcaattgattcataagggtaccatgttcgtaagccccaaagattgtcaccaagtgagataaagctgccatcaatgttcaaatcggtataaaattgtgataaacgatcacgaatttctttgttactatcacctaaataagcctgcaccgcattggctaaatcggcaaatggcattgtgtctccacgttgtgccaagattgcgtgtgcgacctcaatcatcgatagttcatttttgttttggcctttaaagacttctaactccaaactggtacacgtcctttcaacagtctaacaacagtctaaaaattactatactcgattaaattgtaaattgcaatcgaatattgtatttccctaataaagcatcgccggcatacagcaaataatcaattccgatgttgccccgaagcggtgcatccaaaatttccatgtccaaagcagaagtaacggtttgaacatccatcaagccatatggggttcgatagcgggcagcaattcgtttgccgtcgctaaacaataattgcaggcgattctcacctgagcgggtcagtttgacattaccgttatctgaaattttaatggtaaccggaaccccgccatcctcagtttcctcttcataccgaatatacaagctgctgcctactcgaactaattggccggtgacatcaaaaacaaagtttgatttctggccttcctgtaaaatgttagtttccaaatgaatttgaactggaacgccagttgttaaattgtccataatacaccttcttttaaatctcgttctaactaatttattatatatcccacggcaacattttgcactcatgttaccctgacgatttccggcaactttacctatttatttggtggtgtctgttataattaagaagattgtttattttatgaaacggagagttggcatatgtcttttacaaacgttccgattaccgtcatcaatcaaatttattctaaaagcaccaagctggatgcctttgcagacaccaatgccctattggaaatctgtgaccaaacgttgaagccgttcatccatttttggacgacttccgaagcaactttgatcttggggatcaatgaccgccatctgccgaaactggccgacgggctcaaaagtctgctggccaaccactatgattattttctgcgcaattctggtggtctggctgtcgtcagtgatccgggaatcctcaatatttccctgttcattccccaaccggataccgtctacacaattgatcaggcatacgaactcattaaagggttgatcagcatgtcgtttccacaactggacatcaagagttttgaagtcacaaactcctattgtcccgggaaatacgatttatcggtcaacgggcaaaaaatcgccggcatcgcacaacgacggacaaccaacgcgttggtgttgatgctttatttaagtgttaatggcgatcaagatgccagaagccaaacggttgctgaattttatgaaactgccgatgcttattcgcagtctcgttggacctttccaaaagtcgacaaggacacgatgaccacggttcaagatctcggcttcccaaatatcacgctcgaggacgtcgaacataaatttttagcgagcgttaaccagcaaaatatcgaagtggacgtaaccagcggccctgattttatgctttcaccggctttcactcaagagcgggccaaacagttacgcaaaattcagctgagaaatgaccaattaccaattgtctaaggaggcaattttttggattacgcacatcaacagttaaaaagagaaaaggtctttcgagatccggttcataattacgtttacgtcaaatatcaagtcatcttagacttgattaacaccaccgaattccagcgcttacgtcgggtacatcaattgggaaccacgtcactgattttccatggtgcggagcattcccgtttttcgcattcggtgggggtttatgaaattgctcgaagaatcattgaatcttttcaaaagaactttatgtcacaacaacctggcgatggtctctgggatgattcagaaaaattagtcgccctctgtgctgccctgttgcacgacgttggccatggtgcctattcacacacctttgagcacatctttggcaccaatcatgaacagattacccaagccatcataacatcgcccacaacggaaattaaccaggttttacgaagggtctctcctgacttccccgaaaaagtcgccagtgtgattaacaagacctatcccaacaaacaagtcgtcgaaatgatctccagccaattggatgccgatcggatggattacctgcttcgagacgcttataacaccggcgttaaatatggcacgtttgacctttccagaattctggaagtaatgcggccgtacaaagatggaatttgctttgaaatgagcgggatgcacgccgttgaagattacattgtcagtcgctttcaaatgtaccaacaggtgtatttccatccggtttcccgggcaatggaagtggttttgaaccggttgttgcaacgggcaaaagttatctttagcggggaggttcatcacgatccacagaccccctacctattactgccgtttttcaagggtgattttaacctggacgactatctccaattggatgacggggtgttaaacacctacttcatccattggaaacggtacccggatgatattttaagcaacctggccagccgttttatcgaccgaaagccactcaagtcagtcaaatttgacaagtcgaccgctgacttgttgccaagactcagagagattatcgaacaatctggatttaacccggactactacacggcgaccgacaacagttttgacttgccttatgatgcctatcaggcggacaaaaaacaaattcatttaatgcaggatgacggtaccttggtatccttgtcatccgttagcccattggttcgggcaatttctgatcgacagaccggcgataaccgcttcttcttccccagagaaattttgaagccggatgaaaacgtcgatttgttccaaccagaatacgatgaatttaatcgccacattcgaaacgataaattaattaaatagctaaaggagattctcccatggatatcaaactcattgccatcgatattgacggcacccttttgaacgaaaaaaatgaactggcgcaaccaacgattgatgcaatcactgaagcccgcaaaaacggcgttaaaatcgtcttgtgtaccggccgaccgctcagcggagtacagccctatttagataagctggccatcaagggtgccagtgaatttgcaattacctttaacggcgcaatggcacaatcgcttgacggtcaagtcatggtcaatcacacgatcagctatgataacttcttggagaccgagatgctcagccgcaaattgaacgtcaattatcaaattgagacaaccgacagtatctatacgaccaaccgtgacaccaacccctatggaatcgccgaaagcttcctggttcgcctgcccatcaaattcagatcaccagaagaaattccgcgtgacctggtgatgtcaaaggcaatgtttgtggactacccggaaaatatcactaaagccaatgacctcattcccgccaagctgcgtgatgagatgtacgtggttcaaacggaaccgttcttcattgaaatgatgaataagcaggctagcaaaggaaaaaccttaggtgaattagctgatcagctacatttaaccaaagacaacctgatggcgattggcgatcagggaaatgatttaaccatggtaaaagctgctggcttgggagttgcaatgggaaacgcaattgatgaagtcaaagatgcagcccaatttattaccaaaccaaatacagaggatggcgttgcatttgccatcaacaaatacatcaaccattaatggctgagtatacgaatagaggctatgaacaaaacgttggttttgctcatagcctctttatttgtatcaatatctgttattatccttgccaagtacaatcaacaactcagcatcaaattgttgaccgcttattggggcaaactggttaggatgacccctaacacaatcaaaaagccacccacgcccaggcaatagcgggcgtatttattaactttgattggctgatttttaattgaaccgacatcctttgccttgggatgcttgggatcattttcagcttccaagtcgcttttcttgcgaatatggaatcgccaaccggtaaataggtgccccgagccgacgataaagaccgatcccaaaacaatcaggaacaatccaaccaaaaaatcaaggttaccaagcaccatttccggcattcggaaaagaatcagcaaaaaattgatgatcacaacaacaataatcgaagaccagactggcgattttttaaccaaatcgaccattaattctcttcaccacgaaatcgattgttgaacagcggactaaccggtttgttttcattgatgcgtttaattgcatccccaattaacggtccaactgagacctgttcaattttatcgatttgtttttctttgggtaactgaatcgtatcagtcacgaccagttgtttgattgcagaatcttgaatccgctgaatggctgggcctgaaagcaccgggtgggtacagcaggcgtaaacctcgctggcaccggcatccattaatgcctgggcacctaaggtaattgtgccggcagtatcgatcatgtcatcaatcatcaaacagcgcttgcctttgacatccccgataatattcatgatttcggcaacgttggcccgcggacggcgtttgtcaataatggcaattggtgccttcaagaattccgccagagctctggctcttgatacaccaccatggtcaggcgatactacgacatcatcactgccaaagccttgcttaataaagtgatcagctagtaatggagcacccattaaatgatcaacgggaatatcgaagaaaccttgaatctgagcagcatgcaaatcaagggcaacgacccgatccacaccatcggtctgtaacatgttagccactaatttagcggtgattggttctcgtgaacgggctttgcgatcttgacgagcgtaaccatagtacggaatgacaacattaatcgtgccggcacttgctcgccgcaaggcatccaccatgatgagcaattccatcagattgtcattcaccggtgcggacgttgactggataatgaaaatattgtcgccacggatactttcgtcaatattgatgcggatttcaccatcactaaatcggtcaaccgaggtcttgcctaatggaacaccaaccgtttccgcgattttctcagccaaaggccgattggaattcaaagcaaagatctttagtttcgaatcaaaatattgctgagccatatgatcctccaatatgttttttgttaactcacatctcaataacttaattatacaatgttttaattaaaattcagagttaatctttctgataaggcaattttttgaaatagccggctttatttgtctggcgggcacgggcaatcgccatgtcgtattgattaactgtcttattaatggtggatccggcagcgataaatgaatggtcagcgacttccagcggcgcaatcaaattcgagttgctgccgatgaaggagtcgtcaccaacggttgtttcatgtttgtgagcaccatcgtagttggcgaagatgaccccgcagccgacgttgatattcttgccaagtttggcattgccaacgtaagttaagtggccgactttggttccctcgtcaatcgatgacttcttgatttcaacaaagttacccaaatgaacgtgcttgccgattttggcttctggccgtaaatgactgtttggcccgatgtctgagtgatccatcatttcagattcttcaattagtgaagatgtcaccgtaacgtgatcatgcaggactgagtcgcgaatttcggagttcgcaccaatgtagcagtcattgccaatgacggtgtggccctttaattggacgccgggttcgataattgtatccgaaccgattttgacatcggcatcaatatacgtgcgttccggatcaatcattgaaatgccgtccatcatatgttgacggttaatccgtgtccgcatgatcttggtagctctggctaaggcaatccggtcattaacgcccattgactcgtcaaaatcatccatcttgtaggcagcaatggtttcgccctcagacttcaaaatttcaatgacatcggtgaggtaatattcaccttgagcattgtcattggtgagcttatgtagtgcctcgaataatgcctgattgtcaaaaacataaacaccggtattaatctcatcaattgcttgttcttctctggtggcgtctttttgctcgacaattttttcaacaatccccaaatcattgcggacaattcgaccatacccggttggatcaggggcttgagacgtcaaaattgtcgctttggcttttttgttttggtggtaggtaaacaaatcttcaaaagtcttggttgtcaataacggggtgtcaccactgacgaccatcgtcatcccatccaagttgcctagtagtttttctgcctgcaaaacggcgtgcccggtcccgagttgtttttcctgaacgacatattgcgttcgcttaccaaggttttcccggacggcgtcggcaccaaagccaactaccgttacaacgttatccatatcagctttttcgacggcggttaaaacgtgatcaaccatcgttttgccgcagaggcggtgaaggaccttgtaaagtttggacttcatccgggtccccttaccggctgccaatatgattgtgttttttgttgccattatctatttctccccaatgcttaattaaatattttctcgatatagtttccaggttgtgaaacaaccgtgttattctcagcgtcaactcgcatcaatgacgtgtagtcgccgatcgtccggccgtttggtgccgtactttctgccacaacgccgacaccgatcagattggcgtcaaactcttcgaccatcgaaatcatgccaccgaccgttccgccgccacgcatgtaatcatcaacgattaaaacgtttgaatcgggtttcagacttcgcttggatagcgacatcttttcaattcgggtggatgatccggacacatagttgacgttgacggttgagccttcggtgatttcagtatcgtgtctgacaatgacaaacggcacgtttagaaaatccgcaacactctgggcgattggcacccctttagtggcgatggtcataacggcatcaacattttggttcaggtactgagtcgcaaaaattcgaccaatttctcttagagtcgctggacttcccagcaggtcggacatgtagacatacccacccggaagataacgggtgtcggaagacatctccgcaattaatttgttgacgacctcttgggcctcttctttaagaatatacggcaaaaacctggtcccaccagcggcaccaggaatcgtttcaagcagaccggtcccccggttctgaaatgttcgttttaaaattgttaagtcttcactaatcgaggacttggctgaatcgtaacgatccgcaaaaaaggtcaacggcacaagtgtgtgtggccgctccaataaataacgggtcatatcgatcagtcgatcacttcttcttactttcaaaaattccacctcgagtttatgtaatatctatttgattttatcataaatgttcgtctttcggggaagatatagcaaaatataatcacagtttaaacttagcggcttttgttggcaattgaattataaatcagtgccaatccatagatggccgcttcgatgctggcaataaagaacgtgaccggccaattcgtgacgtaacccagataaaggccaaaccaaacgccaaagattgcaaagccaattgccaaaagcatcatctggattacggtgtgggcaaagtactttgaactggcagccggtaatgtcaacagaacaaagatcaaaagcgaaccgacaatctgtgcggcaacactcacgctaaatgccaataagaccagaaaaataattgaaatcaaagagctgtgaatgtggttggttttggcaccaacggcatcaaaagagtcatccttaagatttctaaaaataaaaaagagcacaaccagtactaaaacagacagggccgccatttgaacaacctcttggtgactgatgccgatcacacttccaaataaaatgttggtcgcgtaactggaatttttgttggataacgataaaaacaagatccccagcccaatgaaaaggcctgaaatggcactgatcaccgactctcgacgggattccaccgcgccgctgagttcaccaaccaaaatcgaactgactgtggtaaacgccagcatgccgtttaatggtgtccaaccaatgaagattccaaatgctgccccggcaaacccaatctccgacagcgtatgggtcataaagggcatgttgcgggcaacaacgaagacacccataatcccgctgacaatcgcgattaaagtgccggcaaggtacgcgttacgcataaattcaaaactaaacatattcgccctccttagaatcattatgcagttcactgattggcccagcagtgtatccgttcttagtcagccacaggaaatgatccggatattcatgaatgacctgcatgtcatgagagacgaagatgatcgtcagtcccaaagtttgattgagccgcttaaccacatcaagtaactcccgcttagtgttgggatcaagactagctgtagattcatccaaaatcagcaggtcgggatcgttaatcagtgcctgtgcaagataagctttctgcttttctcccccagacgccaatcccaatggccgtttggaaatgtgctcaagattaacctgcttgataacggtttgaatcttttgcttctcttttcgcgatagccagggcagtttaatgccggtgaaattaagcgagataaagtcttcaatggacaatggatactcgacatcaacattacgaaattgtggcacgtagccaatttttaaaccggctttaagcttgatccggcctgctgaaggcttcaattgattcaagatgaccctgaccaaggtggtcttgcccaccccattttcaccaatcacgccaagaaactcaccccgatgaaccgcaaaggttaagtcagaaagcacttggtgattggggaaacttaatgataaatcttcaaccgaaattaatgtttcactcaaatggaaatccctccacaactttgtaaaaagtaattattactattttagtttagattaaattgaatttttgtcaatcgctgttggcaaattaaaaggactgcttgaacaaaacttaagctttgtcggcagcccgttctgatttctttaaatgaccggatgtgaatcgcattccggctgggaaatgtaggcttcattacagaagccggaaatgctattgtaaacgcggcgagcgcgggattcagttcggcagatgccaaaaactgtcggtccgctgccgctcatttgggagccgtcggcaccatattcaatcaaccgcgatttgagcgttttgatttggggatgaccagcagttgtaatctcttccaatgagttgccaatgtttgccacaatgcggtcataatcctgattttcaatgcctgctaataattcgtcaattggcggatgactgacagacgttgtcgcaagctgtttgagaattttgggtgttgacacactcacgtggggtttggccaggacaaaccacattttaggcagtttggtgagtggggtcacaatttctccccggccgctgaccaaggctgtgcgactgtagacacaataaggcacatcggaatcaacctgaacgccgatttgggctaattcttcaaatgacagcccagtctcaaacatttcgttgagtgcacgtaaaacggcggcagcatccgatgatcccccacccagtccggcagcgaccggaatattcttctcaatggaaatctccaggccaaccttaaagccaaccttgtcaaaaaataaccgggccgcctggtaggccaaatttcgccggtcattgggcagaaaactgctatccgaaaaaatccgaatcgccgagtgactgctcttggtttcaatttggatatgatcacttaacccaattgacgtcatgaccatccgccattcaattgagccatccggatggacaaagggggcatccaagcccaggttcaattttgctggtgctctgacaattcgtttcacttggatcgacccccttcatttattaataacaaaattatactaaattattaataaaatgtcagttattggctgataaaaggcagtcggagcaaaaaatggccaaaataaaaaggcctcaatggcccccacgctgactttgactccctgcagttaaactgcttgggatgcatcaaaatcgacctcaatatttttggtcaaaatatccgtatagctgtacgaaacccgttcaaaattcgcgttgcccggatccaattcgacaacaaaaacagccggaaacgtttccctcaaaattccccggcgcttggttgtctttcttcgcccaatttgagaagttactaggacgtgctggccgatatgatcgtccatcttatgcttgataacagataaagtcactggcattctactcacctcacgatatttaattataccataaaagtaatagaaatgcaattttttaccacaaatcacactatctggcaataataaaacactaagatttagattaaatttttcaaagtgtgaaaggcattcgccaaggtcacaaactgatcaacagtcaaattttcgggccgaacacccgcgtcgatattgacactggctaaaacttctttaatgttggccttcacttccggtgttttgccaaatatcccctgtaaattattccacagggtttttcgctgatgcataaaacagccacggacgaaactgataaaagccttttgatcaaagggttcaacggcccttttaacccgcggtgtcaatttaacaatggccgaatcaactttgggctgtggaataaaagcggttttgggaacaacgaatgaaatctcgacctgatttaattcctgaacaatgacagacaacgacccatagggctttgttgacggttcagcgttaagccgctcagcaacctctttttgcatcatgacaacaatcgcatcaaactgggtttcgccggtaatcaagtccatgacaattggcgtcgtgatgtaataaggcaaatttgccactactttgagcggcttttcagtgtcaaagacgtcatcaatgatttttggcaaattagctttgagaatgtcctgattaataatctcaatattatcatatggcgccaaagtttcatccaaaaccggcagtaggttggcgtcaatttcaaaggcgacgactttgttggcagccttggccaactgttccgtcaacccaccgatcccaggaccaatctcgatcacgttgtcggctttggtaatctttgcggcagcaacaatattgtccaacacaccgagatcgactaaaaaattctgccccaagcttttcttggcggataagtggtaacgattcaggattgcctgagttcgtgtgggacttgcaatctgtggatattcagtcatgagcttcctcctgattaatctgttcaacagcggctaaaaattcatcgtgtttgatgccaaacattctaaggcgatgctgcagctgtttgccgttaacatagccgattcgcaaaatttcaccgaggcgttcccgccgttttttggcactgggattacccatgaggccgtacttcattaattcagccttggaaatgagttcaccagctgattcatcctcagtataaacctgactcaaggcttcgcgaatcgattccacactggcgtgctcgacacctaacgacccatcggatcgattcggaactccctgcttcttggtgataaaggcatgcttagcgttgggaacttccgcagaaatggttttgcgaattttttcaccagaaaaatcaggatccgtgaacacaataatcccccgagtttgagccacctttttgatcaggtccaaggtctcttccgggatcgccgagccgcgggtttcaatggtgtcggcatcgactgctctttgaacgcgtttggtatcgtctttgccttcgacaacaatgacttctttaatttttttcatgattcctcgattccaaataaccgcagcgtattttcataggtatgcgccgcaatgacatccgggttgacatcacaaattcttgccagtgcctctaccgtgtaaagcgaataagccggctcgttttgcttgccccgcaatggttcgggtgataggtacggcgcatcggtttcaaccagcatgctgtcaaacggtgtttgacggacggcatcgtgaacttcatgggttttcttaaaactggcaacgccactgtatgagaccagcatccccaagtcaagaaacttcttgagccattccggatcgccattaaagctgtgcatcaccccgcggatatcggagacatccatttccttcaaaatggcataggtatcctcaaaggcatcccgattatgaaccgaaatcggtagatgcagttgtttggcaatatcaatttggcgtttaaagacccgcttttgcacgtctctgggagaagttgtttgatggtagtccaagccaatttcaccaactgcaaccaccttttggctctggagctgttcaatcaacagctgttcttgttgttcatgataatggatagaatcttccgggtgccaaccgatgattgaatacatgtcagggtattgggctgccaattccaatgatcgatcgttcagctgttgattagaaccaacgttggccagcttaacaacccccaagttctgtgcgtgcttgaaatatttagccgcttcaggataaaggtgttcgtcattcaaatgggtatgtgaatcaaaaattttcattatttgctcccaaactatttagatagaaatagggattgtgacaaaactcgcgtcttgttgccaatccctagtctttcacgatgttaactttgccacaaatcggcaatttattccagtgtgacaccattttccaagtgagatccgacggttaccaactcaacgttgccatctttatgttccacggacagtaacattccttggctgacttgaccgcgcatctttcttggtttcaagttcgacacgataatcacttttttaccaattaactgcttataatccggataccattcagcaattcccgacaaaatttgtcgatcgccgtcatcaccggcatccaagcggaattgaagcagcttgtcggcgccttcaaccttgttaacgtctttgatttcggctactttgagttcaatcttttcaaaggcttcaaaacgaacttcttttttggttaaattcaaattggtttcttcaggattaaaatcagcttcagcagcttctttcatggctgcacgacccttggccttatcggtcttggtcatttgctgcttaatgtagtccacctcatcgtcaacttcgactcttgggaagattggggtccccttggcaacggctttcacaccggcaggaacgtcttcaaacttcaaatcttcgaggtcaatgtcttctgtaatccctaattgagcaaagatttctttaggggcgtgagtcataaccggactgattaattcagcgatgacccgaagaccggctgccagatgagccatgacagcgtcaagcttatctttgtcatcaggatttttagccagattccatggttcggtctggtcgatgtacttgttggtttgggaaacgagtttccaagtttccgctaaagcatcggagaagtgcaaatcattcattaattgcttgtaatgggcaatcacggtggcagcagtctcttccaattctttgtcagcttcgttaacgccggcctggtatgcaggtaagatgccgccgtcatacttgttgatcatagaaactgttcggttcaacaagttgccgagatcattcgccaaatcaaagttcaaccggtcaatgaagtcctctggcgtaaacagaccatcattggcgtaaggcattgcgcggagcaagtaataccgcaatgcatccaaaccataacggtcaactaaagtttccgggtaaatgacatttcccttagacttggacattttaccgtccttcatcagcagccagccatgaccataaacggttttaggcagcggcagtcccaaggcgtgtaaaatgattggccaataaatcgtatggaaccgaacaatttccttaccgaccatttgcacattggctggccaatatttcttaaagttgctgtcatctttgccgtcataaccaagagcggtaatatagttggtcaaagcatcgatccaaacgtaaaccacgtgctttggatccgacttgaccgggacaccccaagtaaaggtcgtccgcgaaaccgctaagtcttccaaaccgggttcgatgaagtttttgatcatttcattcatccgggttgccggctggatgaagtcaggattgtctttgtaatattgcagcagccaatcagcatacttactcattttgaagaagtatgactgctcgtgaaccaattgaacttcgtggccgctgggtgctttaccaccggttaccttgccgtttttatcgcggtaaacctcggcgagttgactttcagtaaagtactcttcgtccgataccgaataccagccggtatattcacccaaataaatgtcgccattgtccagtagtttctggaagatatcggcgaccgctttttcatgataatcatcggttgttcgaatgaatttggtgttggaaatttccagctttttccaaagttgtttgattgatgcagccatctgatcaacataatccttaggcgacatccccaactgctctgctttttgttcaatctttaatccgtgttcatccgtccctgtcaggaagaagacgtcatagcccattgcccgcttgaaacgtgcttcggcatcacaggcaattgttgtgtaggaattgccgatatgtaacttcccggatggataataaattggtgttgtgatataaaatgttggcttactttctgccatgaaagtacctcttttcatgcttaattattctttaggatattacaatccagtatagcaaatattttttggaatggcgatgagaattggatttgggtgagatggtcgtagtcgaagttcaatatcgctttgaatcggtggtggtttgcttttacctagtggtaacagcagcaacctgcacctaagtatggtcggacaaaaatcaaaatgattttcatccaaccacactcaggctccggttgctaagcgctctggatcgcactcattcaaaacaaatccatctgtaccggcgacaggccgccaaattcaatccccaacatctttttcaactgcagggcgttgtctgctgcgtccccgccgctattattattgaagatgacacaaacttctttggcctgtttgtccagatccaggactacttttcgaaaagctgccagttcttcttccgaataccggtacaacgtccttttcccgcgccaatctgctgactgctccgtccagcctttgacgtttcgaccgtgaagccgcagcaacgccagattctccgttgtcaccagcggttcgaaaggcacgccggcattggtggtatgcggttcgtcaaccgccaccaacgtcattcccagttcgctgagatagccggcaacgtcatcggtaatctcgtcaccataccaagttgagttgcgaaactccactgcaacaggatatccggccatcaactggctaattcgacgcaggtactgaatcgtcgcaatctttctggcaaagtatggcggaaactgaaacaggatcgccttgagctgaccggtgtccattaatggggcaaccgcccgcttgtattcgttgaaagccacaaaccgctgctcattatcaaccgggtcggcgctgccctgatcgtgcatggtcatcacccggttggccttcaaaataaattgaaagttatccggtacctgtttttgccagttggtgaccacttcaattttgggaatcgcataaaacggcgtgtccagttcgacgaccggaaaatacccactgtattcagttaagcggactttacgtttagcaccgtcgatcagtgaaggatgctcggaaaacgtcgttaacccaatggtaatcaatcagcccacctcccggctgtttagacattcaccgtcaaatctttgaagaagtcaacggcattttctttgaccatcgtaaacggaaaaccaaattgaagcggctcttcattaaccgccagaactttggcattttgagaacgataatcaatcaagccggcaaacgggtaaacccgcattgatgtgccgacaatcacaatcagatcagcttgggacactgcctcaacactcttggaaatggcaactggatcaagcccttcaccgtataagacaatgtctggtcgtaaaatgccgccacagttttcgtgatacatactctttaaataatcctggtaattgactgtcttgtggcacttctgacaatacactttgtatagattgccgtgaaactcgactaaatgctgcgtgttggccttgcggtacaagctgtcaatattttgggtcaccacaacggcattgcgtttctgggtaaactcagcctggcgctcatgaatcacatttggcttggcatccgggtaatacatatttgatttttcgtattcccagaaaactttgggctcatcacgaaggcaatcggtacttaaataatactcagcgggtttatcagatttgtcattggtatacagcccgttctttgatcgatagtcaggaatccctgatgccgtggaaacaccggcaccagtcaaaaagacaattctttttgcgttatcaaattcagcttgcagcttagaatcaatcatcgtattcctccttcaaaagttcattatttgcgaacgatataaggcattttaagatcgtcgaacaactgcttggcgcttttatcatagacccctttgaaaaattccggatcgtcctggttacccttggggttggccagcacaaaggagttctgatcatctacccgattaaagccgacgtaacccttggtgttgctggtaacctcggtcaagtcggaatgataaatttcaaatagttgtttaactttcaatcccagctgccgttccgacaaaacactggtaagggtggtgaactccgtgttgtgcagggccggcagttcccagtcctttaactgttcgtcaaaggctttaaagagcttgacgacgttgcggcgcaatccaaatggtgaatccgtcggcttatcggtgatcacttgatacaacttttgggcagcctcaaaggaaaccgggaagtcttgtttgaatttgtcagccaccttgtcaattccctcgccgtaaaagaccagcgcatccaataatgtggttaaccgtaacatcatctgatcgtccagtggatccggttcaggtttgatggttgcatagacacctttgagatacatctcttcgatgtcgtcattgatcaaattgtgctttcgctgctcggatacaaccacaaaatgagagacaatgtcgtagagttccgttcccatcatttttaattgttcatccagagtatcatcgccagtggtcagtgaataaaagacctgtggaaaaccacggaggaccatcaataggtgcagcagttcatgtgaagccgtgtagtcgggagcgcttaagtctgcgatttggacgatgatatttttgccgtcctgaaccgtttgggcctgatcgtgacgtacatatcctgattgcagcttgccgataaaagtcaccgtcaccgtcccgggaaagaagttgttaacggcgtcaattaagccgtgaacgtctttgtttaactcgatatcaatattgttatccatcatgttctccatcatgttctcctatctgcgaagtatttttaaaatttctttaactgtttgtgaactgggatgatccatcccctgaagcttttgaacaacaactggcaactcctgcattgtggttccatttgaaagagctaaggaccttaattgaagattcatatggcccttttggatgccatcggtcaccaaagcttttagggcagctaagttttgagccaaccccaatgcggcgaccacctgcatttcctcgcgggaattgtcgatctgagcgatctgtttgttaatgccggccaacggcaaaaccttgctggcaccgccaacaaatccgattgggactggcagcgacatgcgtcccaccagttggtcttcgtcaatctcccatgtactcaggccttgatacgacccacttcgagccgcaaacgcatgagctgcgctttcaactgcccgccaatcattaccaaaggccatcacggcggcgtcaacaccattcataattcctttgttatgcgtcgtcgcccgccgaatatccaactgggcgatctgactggcatcggcaattttttgggccacctgagggccagataacgacttggttcctagtttggccatcgccaccttaccggaaacttcaacgatggctttatcagcaaaattcgttaagattgccatcgtggtttcgaccgtcaactgctcagaaagccaattcgacaccgcttccaacatcgtgttgatgatgttagcacccattgcctcacctgtatcaaccagcaggtcgaccgacaggaactgctttgagagaatccggacatcgaggcctttggcacctccaccatactttaaaacgcttggatgactctggtccgcaatttgaatcagctgctgctgataatcatgaacaaactttgtcacctgatgaggatctgcgtctttgacgatgacctggccgctcaccaggttatcagggacgctgcaatgaatgcctgctcctgccgataacagtttggcaccattgctggcagccgcaatcactgacggttcttcagtcaccattggtaccaaatgttcgtggccgttgacaaccaggccaactgcgattccctcggggagtggataatccgtcagattgttttcaattaattctccggaccttgggttcaaggaccgtccaagcaaatcgagttgagcctttgataaattggcagcttcagcgatcagcgaaagacgctgctcgtaagactttttatagaaatgatcccatttgttttccatgatatcaccatcatctgttagaggcacaaaaagctggtacaattgccagctttactcgatgccgtattctttttgaatgtactcggtaatgatgccttctctgacaccactttctgaaaataagacttttttggcatcaattttgtccattaaaacaatcaacggcaacaggccgccgacaataatgtcggcccggtcgtgctcaagcccctgaattttccggcgccgattgacgttgcccttcaataaattcagataggttcgattaacttgttcagcagttaaatgataaccgtgaattgcatcaattcgaaccatattttgacgacgacgattgattctcgccaaggtccgattggcaccgcccaagagaactaacggctgatgggccgcacgattcaaccaatcaattcttgaataaatcttcctgatattaaattgggcgttaaataaattcgcaccggtaatattatcatttaaatgatatctttcagtgatattcactgcaccgattggaatgctggtgagatttgagcttttgccctcattgacccgaatgagttcacaactggcgccgccaatgtctaggatcagacaattcctgattcctaatcggttaatcacgcccagataatcgtaataggcctcttgattgcccgaaaggacctgaagcgaaatgccaatacgctcagaaacggcctttaaaaacttcgcctggtttttggcttggcgaacggcggctgtggcaattccaatgacccgtttggcttcatattgagaatagatttgtttaaaatctaacagtgacttaatcgtccgttccatggctgccggctggaggatcttgcccctgcccatgccttcggaaaggcgactgtcgcttttgatgcgtttgatttcacgataactgccatcatcagaaatttgattgattgccattctgaccgaatttgagccaatatccaaaattacaaggttttccatccctgccaccctttctggacatattagtcaaaatagttaatgccaatggcatcgcgaacttctttaagggtttgattggcaacctcgttagcgtgttcactgccctttttgagaatctggtagacaccctgttcatcttcggcgtaacgctgacggcgctcacgaattggtttgagctcggcttgcaggacatcgtttaagtaacgtttaattttaacatccccaaggccaccatggctgtattgatcttttagttcctgaacttttcgtttgtcaggatcgaaaatatccaagtaggtgaagaccgtgttgccctcgacttggccgggatcttcaacgtgaatgtggtttggatcggtgtacattgacatgacctttttttggatggtgtcttcatcgtcggccaaataaatcgcgttgcccaaagatttgctcattttggcatttccgtccaagccgggaattcggcccattccctttggtgggaagtaaccctctggctcgactaaaatgtcatcattataaacggagttgaaagttctgacgatttcacgggtttgctccaacattggttcctgatcgtcaccgaccggaacagttgtggccttaaaagcggtaatatcagcggcttggctgattggatacatggcaaagccaaccggcacactttggccgaacttcttttgtttaatttcattcttaacagttgggttccgattcagacgggaaacggtcaccaaattagaataatgctgcgttaattccggtaacgccggaatctgggattgaaccagaatagttgatttttgggggtcaattccaacggccaaataatccaatgccacttgaatcaaactgtggcggatcttttccggatcacgggcattgtctgttaatgcctgcatatcggcgatcataataaatgtttcgtagtccccggagttttggagctcaactcggttctttaatgagcccacataatgaccaatatgtagtttgcctgtgggtctgtcacctgtcaaaataattttcttcgtcattgtaaccatcctttcaaaaaacgccctattgctttaacaataggacgcttatacgtggtaccacctaaattgtaacttatatcaagttaccgctcgagacgatatgggcgtcaccctttacatactccaattcgtttcgtcgtggccgttttcagcaagtcggcctctctgttgctgacgattctactcagtttttaataacaatctaattttactgataaaccgctaaaaagtaaaccccgtttgcgggtaaaatacgggaagttttggcttaatatcctgcagataaatcaaccttgttcacagcaactttgccggtttgaatgaaactggtcaggttttgatacaaaatgtcaaatgcctcatcaccatattcttgaaagccaccggaaatatgtggcgttaaaataacgttatccatcccccagagtggcgaatcactcggtaatggttctgattcaaacacgtccagcccggcaccagccagttggtgttggtccagtgctgcaatcaacgcctcggtgtccaccgatgggcccctcccgacgttaataaagattggctggttgcgcatttgatcaaagaacgcctggtcgaagaaatgatgagttgctggggttaatggcatgatattgatcacaatatctgccttggcagcttgcactactccttgatcgtctccaaccacttggtcaaaatgcgccgttggtttgccatgccggctgacgccaaccgttttggtaccgaaagcttggagtttttcagcgattgcccgaccaatatggcccgttccaaaaatcaccgccgttcgatttttgattgtgtagttctgcattcgaacctggtcaccgagccacttttgatcgcggcgggccgcttgagtggtgacgatgcccctggcaaatgccaaaacgtatgcgatcaccatttcactgatgggttcggcgtggatgccactgacgttggccaaggtaattcctttatccgcgaagtcgttcaatggcatgtagtcgaccccggcagaatttgactgcacaaatttcagcttcggcgattcactcagcacggtgcgggcttgctgattccaaccatagatggcatcgacacttttgacattgctgctattcaaatcagccggttcgatgacctgcacatcgccaagcgctgtgagtttggcctgctgttcggtcgttaaattgaataaatccagaatcttcatggtcccatccctttcattcgtcttgatctcaataaaaagtatacgcttgaaattggttcaaacaaagcaaaatccccaccccacattgaagggcaacacaattgacaacggggttaataccaactaaaattgtcgaagcattcttaattcacagtcgagtcgaatccgaatggaggaacccttttggaaaataatgaaaagcaaatcgaacagtcacgtgtggacaaagtggtgaccaaaattgaccagaaaatcatcagcacggatgacgaacttaaccgtgcccacgcagaaaccaaaaaggttcagcagacttattccgacaatacctcggttaactattttgaggtggatgatcgaattgaaaccagtgccgaactccagcagcagcggggtttggtttctcgtttaaccgaaaatgaaagcatcttaaaaaatcagctttcaactttgaaagatctcaaaaaatccccgtactttggccggatcgatatccaagacgatgacgaggatcaaaccgaaaagctgtatatcggcattgcttcatttgaaaatgaagacggtgagtttctggtgtacgactggcgggcacctatctccagtgtttactataacggcactctgggtgaagtcgcctacgatactccaatgggccgacagcaaaccaatttaaaaaagaagcgtcagttccaaattgtcgacggtcaaatccgcaacatgtttgacaccaacgaaacggttggcgatgaaatgcttcaaagtgctttgggtgagcaaaacgacgaatacatgcaaaatatcgtcgccaccattcagcacgaacaaaacgatattattagagataccaccagtaatctgctggtggttcaaggggttgccggatcggggaaaacctccgccattttacagcgaattgcctttttgctgtatcatagccgcgatacgttggaagccgatcaaattattttgttctctccaaataaattattcagccactatatttccgaagtcctccccagcttgggtgaacgcaatatgcgccaggtcacctttgatgaatttattgataaccgactaaagggcctaaacgtccaaagtttgtttgaacgatacgaaactgatggtgacttgaccgaacagcagcgactggttcgcggcttcaaagaatctgccaaatttatggacgaactccaggaatactgtgataagctccagccagcccaaatcttcttcagtgacatcatttttaacgaatcaaccttctttagcaaacaggaaattcaagacattttcgacagttttcccaaagcagccaaagtttatgatcgcttcttacacaccaagaatgaattgatcaagcgactcaaacgccggatcgacgacgaaaccaaggctgattgggtcaacgacgaaatcgatcaaatgagtaatgagaagtaccacgatctcttggccggcaaagaactgggtgagttccaaaatgaagatgccgagcgcttcttcattgcccgaaaaatcgtcagtgcccgcctgcgggtggtctacgatgcgatctttaacgacaacttcttcgatgcctacctgcagtacgccgacttcttgaaaaaagtcgacctgccgcaaaacattgaaacgccccagtggctgcagtccgttgatgagtttaatcattcaattgaatttcatgccatcaaattggacgattgtgcgccgttgctttacatgcgcgactatatgtccaacagcggacagaacaacactatgaaatacctgtttgtcgatgaaatgcaggattattcagtggctcaactcaaatacctgcgctacgcctttccaaagacaaagtggacactattgggcgacagtgagcaggcactgttcaaagacgttgaacagccaaaagaaattcttgataaattaaacgccgctttccatgtgcgccggtcccgactaatcagtttgatgcggtcgtatcgctcaacgctgccgattaccaactttgccaaatccattttgcctaacggagatgacattgaggcgttcacccgccccggcgacattccggaattggttttgacatccgacttcaatgacggcatcaaccagctgcaaaaagtgattgccgaccaacgcaagcaatacgccaccgttgctgttttaaccaaaaatatgactgaggcccagcaggtctatgaacgactgcatgctttaggagatgtcacgttattgcaagatgcggaccgaacattgccaaagggcattttagtgctgccaatctatttggcaaagggcttggaatttgattccgtgatcgcttgggatacctctgagaagaactattccgatgaaagtttgcttggaaccctctacacgattatcacccgggctatgcaccacttaaccttgatcagtctgggcgacgtaaccccgctgatttccgatgagagtttaaccgatcgcaagattaaaatcgaaaaaaagattcggaagtaattggtgtgaaaacatctgattataagcaaacccggagctgtggtcattgatcacgctccgggttttttagtttcacttagattgtctggggatagacactgttcacttttatctcgcaaaaacgtgctctttgagccagctttctcctgattacactagttctcagaagctaaacggctcaatagcactctagatcaaatactgcacatcactcgccagagttggataagcgagaatttcccggttgaagtcgccgattttcatgtgctgatcaatcatcatcgtcaaaatattgatcaaataatcagcgtgattactcaacacggtggccccaacgacagtttccgtatcgcgattgatgaccactttagccttggcgagtggctcattgagtcgatgataactgtaccacttggtcatgtcattggtaatcagcatatagcgactatcgtgcgtcgcgatactcgacggcagtcccacttgaccgagtgagggttggccaaagacaatcgtgggaatggatttgaattgaatcggatccgttgacccgttaaagtagccggccaagtagccagcttcaaaaccggcaaccggtgttagcttgggacgtttggtgctgacgacatctcccatggcaaaaatctgtggatttgacgtctgcaggtggtcgtccacgatcacaccgtgttggtcggttttgacaccaacattttggattccaatcgtatcaacgttgggaatccgccccgccgtgcagaagaccatgtcagtcggcagcttaaaattgtctccggataaaacaaactgctcgcccacttgggtaatttcttgaacatccgtatccagatgaaaatcaacgcccaacgtggtcagtctgtcaatttcttcgtggactaattgttggtcaaactgtttgagtggccgattgttatgatgaatcaggtgaaccgtcgctccggccgcgcgggcaatcccggccagttcaaagccgatatagccaccaccgacaaaagtgacgtcgtttggcagatcatcgaggttcaaaaagtcggtactggttttgaaaaattgactaccgggaatatctaaaattcttggccgctgaccagttgcaataacatattgatcaccggaaaggctttgatttccagccgtcagcagcccatctgaattgaattgggcatgctcatgatacgtgtcgaccccatctgaaatcaacccgttgttggtggcatcagaaattggattggtatactgccgcttgtggcgcatgagatccggccaattaaccgataccgagccactgatcccgttaccctgcatatcattgacaacttgagtgatctctaaaccggacaataaaattttcttcggatcgcacccgcgattggggcaggttccaccaaacaaattgtcttcgacgaccgccacggttttgtgctgtcttctgagtgagtgggccaaagacccgccggcaaccccgccgccaagaatgaccacatcatattgttttgtcatttagtattcctccataagcacctaattcatcgttgattgacgatttcacacgactaatttcataatcttaaatccattgtagaacacttcggaattatttccacgttgccttgattgacaactccccgcggaatttgtatcttagataatgtaattaaaattttattaaattgaggtatatcatggtccatgcactttggcgtcaatttccgcgcattaatttaaaactaattgctttggaaccctatttgttaaacgccgtcaatcttcccaaccagcccattcatcataagatcagccagttgctcaaatccggcggaaaattcctgcgtccgggcttcttttacatttattcagaatttggtcaagaggtggatccagctaaaattaaggctggtgccgccgcagtcgaattactgcatgtggcaactctgattcacgatgacgtgattgatgagtcgccgatccgaagaggcatcgagacaatccatactgaatatggccaaaaaaacgccatttatgcgggggattacctatttacctgttactttacgcaggtactcaaatcgactcaggatccggctaatatgaagcgacacgttgatgccatgcaaaccattttagccggcgaattggatcaaatgaaatacaacttcaatcaacaaatgactgaggcagattatttccacgaaattaccggcaaaaccgccgaattattccgcctttgtttccagcaaagtgccttggtaagccaagcttcggatcaaattttcaaacttggcggcgaaattggtctaacgatcggccaagcctaccaaattttagatgatatcttggattacagcggtgatcctcaccagaccaagaaacccgttcttgaagacctcaagtccggcgtttacaccctgccattaatttttgccctgcagacggctcagaagcaattaaagccactgctggataagcgtgaacaactgacccacgaagacattgcccaaatccaagccatcgtcgttcagtcgggtggcttacagcaagcaatcaaatctgccaaccagttaactgctaaagccgaaaagctcattgcccaattgcctgagcaaagggccaagcgcgacctccagaccctgacacagctattattaaccagaaagcaataatttattttgaaatatcaattgccacaaccagaggaccgatatctcctggctgtggcaatttttgcgtttgatgcggttgattgaaatgttgtgccgttgaccctgtcccctactgtgtaaaacaaaccgcccaacgatgaactaaacccgttcatcctttgacggttcgctttacactccggggccaacccgggtctcgttacactcttcctctgtccaagtcatacagctgcctgaatcttggttgagccttatacagttcctgcggggtgccctgcatatcgaactggccgttttccatgaaacgaacctggtcgacgtgggcgatccctgccaaatgatgagtgacccaaataatggtcttgtcatgaagtaattcaaagactttatccaacaacttcttttctgtgatcggatccaagcttaccgttggctcatccagaataataatcggtgcatcctggagtaaaatccgcgccaatgacaatcgctggcgctccccacctgagaagcgtttaccagcctcttgaacttgggtgtcgtattggtcgggcagcgactcaatcaactcttttagtccaacggctgcaatcgcatcttttacctgctggtcactggcattcacgttgcccaagcggacattgttcatgaccgtcgtgtcaaaaagatacggttgttggtcaagaatgccaaacagtgaagagcggacgtcctggaggcttaaaatattttgctggttaatcagcacttggccatcggatggtgtcaaatctccaacgaccagcttcaagaaggtactcttcccagttccgctgggtccaagcaatgcgaccttttcgcctggatgaatggtcatcgagatatgttgaaccacgtcccgatcgccatcggcatacttgaacgtcaaatcgttaatcgaaagttccttgaacggttcagccaacgccgtctgcttaacgggtttgaccgtgccggaatctaaggcgttaacccgctcaatcgaccgtttataaaccggccactcactggcaccttgactcatgttgacaaatggtgacaccgctgggaaaatggccagcgcaaaggcagccacccagttggccaaggatttggaggcggtgaactgattagccgaccagaccagcagaaccaaagtcgttagtaaaataacaaattgaaccagaaatgatcgccaccactggaagtaatggtctcgtttccgcagggctgcaatggccttaattggtttcttctgcaggttgatgaagtcgttgtaacgaccggaaatcagccagtcgcccaatcccaaaacttcatcggttaaattcgtatagaattcgtgttgaatttgatgctgtttaaattcccgaaccccgttggtggcaactgacgccaagggcatcacaatcgtgataatccctaataacagtaacatcagtaaaccgaccacccagttcagtgaaccgacaccgatcaccacgaaaatgtacaacagccaaccgattaccataggaaaaacggttcgcagatacaagttttcgatgtgatcaatatcgtcggctaaaatactcaagatatcaccggtttggtgagagcgttgaatggccgatgccttttgctcaacggtttggtacagcttttttctgaagtcggacacaattcgcagcacccaattatggctggttaaccgttcaacatatcgaaagactggccgagcaattccaaaggcccgggccaaaacaaccggtacataaatataaataatacttgacggctgtctggcagcctcactgatcagatatccggagttaaacatcaaagcgccgccagagaagaaggtcatgaatcccaggaataagaccaggatcagtaagcctttgtatttacgcaggtaaggcatgacccaggtatcgttttcgaatgtttttctaaaatttttcataggtctgccgcctccatttctgaacgaagcttgacgtaatcaccatttcgctgagcgagttggtcaggtgtcccctgttcaaccaaacgaccatgatccatgactaatacgtagtccatctcaccaatccagtgaagccgatgggttgcgaagaacaccaggtgatcattgaagaccggcagaatatcctgcttcaaaccggcttcagtttcaatatccaaatgggcagttggctcatcaaataagagcacttttcgattgggatcaagaaaagctcgggctaaagcaatccgctgtgcctgaccaccactgaccgtccgggcaccttccccaatcatggtattaagcccgtccggcaaggtattaatccagtcggtcaggcccgccttgtcagctgcatttgaaatcgcagcttcagtagcatccgcgacgtaaaacgaaatgttatcggctaacgtggcgtgaaagagatagggattttgtggaatatacagaaagtttttctgccaattagcttggttcaagtgtggcagcggctggccgttaatcgagatttgattttgaccgtccggggataagaagcccccaatgagattgatcaaagtcgatttgccggatcccgatgcaccgatgatgccgatcttctgcatccccttgatatcaatcgaaatatctttaagcgtcggttccttgcttcccgggtaggtcaaggaagcctgattcaatttcaaggttgaatcgttgttccatttcaaatcaggcaaaacttcgcgttggctcatctcaggctcatgaaggacgtccaagacggcgctcattgcgttcttaccattcaaagttgcgtgatagtcgttggcaaaattccggattggcagaaaatactccggcgccaataccaaaatggtcaacgcaggtaagagcatgactttaccatccatcaaatcaaatcctagaaagactgcgacgactgcgatcgacaaagtggtaaagaaatccagggcaaatgtcgatgttaaggcgattctcaacgtggacatcgtttctgtccgataagattcgctgacttcatagacattgtcagcatagcgcttagaaaggcccagctgctttaaagtcggcagaccccgtaaggtatccacaaagtgattagacagccgctgatagctttcatattgccgatcagccttactctgagctgcaagtccaagaataatcatgaataaaatgataattggaaaaatagcaaataagaaaatcgcttgttcccaacgcaggaacaggacgtataacaaaatcagccacggcgtaatcgacatatccaagatcttgataacaactaacatcaaataagtctgaacctggtcaattccttcaagggccatcgtgacgatgtttccagttccccgtttatcaatttcagcgggtccgagtcggaaaatcttggccatcaaatcttcccgcatatcgccacttgtcttttcaacgaacggaaataatacgtggttttcggcgacggtcaacaaatgccgccctaaaaatgcaacggtaaacacaacggtgggccaaataattgtgttgatcgactgcagattccacaggttcacgattgcaattgacagtgcgcgagcctgagcaattattgcgattgcctgaatgaagaccagtatccctaaaataacggcatactttttcatccccggcagatcaaacaatcttttatcaatcaaacttttcactcccccagaacaaaattaattacaattcctagtataaagaattattgcgcacaatgaaatatgtgagcggtttatttcttgatttatttggtttttaacacagctttggggctcacgggttaccgccaaaaattccgggcaaaacaaaaaggccagcgataagccgaaacgtttatcagtggcctttcagttgatacgcatatcattaactgaaaatcatttacccggatcgttggattcagttaaatactattcagcaacttgctttggtgacttgattcgcttgtagaatacccagtaactccaaatgaagtagatgagcacaatcggtaaaatcgtgaatgtcaaaatcgtcatcaagtgcagcgtatacggtgaacttgaagcatttttaattaagattgaatttgcgttgttcgtcgcaatcataacccgtgggaacaatccgttgaaaatcaggacaacgacactgattaaagaaagcccactggcaatgaatgatgtccaatcatggctggactgagcgccccaccatgcagccaaggtaaagatgaccaaggcgatcaagattccccaggttgacattggtttacgagtaaagaagtcagttgttaagtaaagtaagataacaaagacaacttcaccggcaagcagaaccggatagagaactttactccacttttctgctcgttctcttaattcaccgctggtcttcaaacgcaggaagtttaatccatgaatgaagcaaagcagtgaaacggcgacaccgccgacaatcgagaaccagttgacataagtggtgaagcttccaaaaatatcgccatttttatcaatcggaacaccttgaatcatactggtgaacatcatcccgaataagaatgcggcacagaaactaccaattgatgatgcccattcccagaaattacgccaagtatccgtctgcatatttgcacggaactcaaatgacacgccacggaaaatcaaggcaaccaagattaagaacaagacaaggtagtatcctgaaaatagtgaagcataccacattggaaatgatgcaaacatcgcaccaccggcagtgatcagccaaacttcatttccatcccaatgcgggccaattgtttggatgacagtatcacgttcagcccggttcttagcaaagaatcgaacggacatgccgataccaaagtcaaacccttcgaggaagaagaacccactaaacaacacaccaattaataggaaccaaataaattgataactagtcattatgagccgcccccatttcgtatggatctaccttttgatcagctgcttgtggttcgctggagtatccgtcagtctgaactgaatccggtccttgtttgagaacccggtgactcaggatgatcatgacagctccaagcgatgcaaagatcaagaagtaaacgatgttggtgaacatcaggcttgccacggtagacgttggcgataccgcatcggcaatggtcaaaagtccgtaaacaacccatggataacggccaaattcagtcacgaaccagccacaggtgttaacgataaacggcagccaaaccatcaagcccatgaggtataggaaccagcgttgcctcataatgctttgtgacttcttacggttgaaccataacccaatgatggcaactaagccgaataagccggcagaaatagccatgattcggaagctccagaataaagtccgagtcggaacataatagttcttcgtttgatcattcttattgtactttgcctttaattccttgttgaccgtttgttggcctttgaaagtaccgttcagactgtgatgaccaagaatgttcaagacataaggaatttcgattgaccaagtcttatcgtgacccttaaatcctgaagccaaagcccaatcacctttattagtagaatctttatagataccctccatagcagcaaacttcatcggttggttattaatcaggtaacgtgtttgcgtatcacctgaccatacagaacctaagcaggcacaaagcccaatgatgagtgaaaccttcattgacttgcggtagaagtgctcatgatccttcttaagtaaacgccaagcagaacagccggcaacaacaaatgcagccgttaagaatgctccgaaaataacgtgtggaaattcgttccacaactgacggttcataataacagcagagaaactggtcatttcaactttgtgttgagcaacattcattgcgtaaccaactgggttttgcataaagctgttggccgccaaaatccaaagtgcagacagcgttgaaccaaaagcagtcagccaaatgaacaaacagtgaaccactttgttgaaacggtcccacgtgaacatccaaaggccaatgaatgtcgattccaagaagaaggctgccaaggcttcaattgccagtggcgcaccaaaaatatcccccataaatcttgaataatccgaccagttcattccaaactggaactcttgaataataccagttacaacaccaacggcaaaactatacaggaaaatcttcccccagaattttgtcatgtttttgtatgtttcatccttggtcacaacgtaacacgtttccataattgcaacaataaaagctaaaccaatggaaaacggtacgaagaagaagtgaaacacagtggtcatcgcaaattgaaaccgcgacaacccaagcatcgtgacgccaatatttaacattgtcgtatccccccttactaaatattaatgagttatcctcatatacccttattgtatatagaaatggttcaacattcaatcaaaatactaattaattatcagcaattactcataatcctgcactgttgttgacacaatcccgcctgaaacatgtaaacgtcgtcaatcaatcaatgtgaaggacttagattagggaagaaatgcttgtgaaattattgcaatggctttcattagacaattgtcaaagccacatttataataagggtgataagattagtttatgctattattgtaattttctaaagcaatcttattttaattattccaaagggggaaaatttcatgacaaagaacatcgtcgtcattggtgccggtttcgcaggcgtttacgcaaccaagcaattggctaagcgattcaagagcaactctgacgtccaaattacattgatcgatcgtcactcgtacttcacttatctgacccgattacacgaagttgcgaccgagcgggttgacccaagcagcatccagtatgacctgcaacggatttttcacaagcagaaaaacgtgcagctcgttacggataatgtcacgtcagtcgataaggacaagaaaattgtcaacggtgaacatggcacgtatccatttgacagcctgctgatcagtatgggtggcgagcctaatgacttcgggacacccggcgttaaagaaaatggcttcacactctggtcaatggaagacgcactccgacttcgagcgcacattcgtgaaatcattggtcgaggagccgttgaacgtgatcccgacaaacgtcgtgcaatgctcacaattgtggtctgtggttccggatttaccggtgccgaaaccattggtgaattaattgattacaagaaagtcctggcaagagattacaagctggatcctgacgagattcacattctcttggttgaagctgccccaacaattatcaacatgcttgatcgaaccaacgctgctcacgccgagaattacatcaaggatcacgacgttgaagttcgaccatcatccatgattacctcagttaatccagacagcgtcgacattaaggatcaggattcaattccaaccaacaccttgatttggactgccggggttaaaaccaaccacgttgccgacagtttcggaattgacgccggccgtggcggtcgattgattaccaatcaatatctccaggcaaagggctttgaagataaaagtatttacgttgccggtgatgactccaacgccactgagcaaggtgctgaacgtgccgttccacaaactgctcaggaggctgaaaatgaagccgttgtttcctctgccaacattgctgctgacattgaaggcaaccacaactacaccgaattccatgacaagaacatgggcttcaccgtttcatttggtgctcgttacggaattgcccaagtattcggcggcaaacgagtccgtggctggctggcaacgattatgaagcacgggactaacctcctgtacttcatgcgaattcactccggctacttcatgatgcagtatatcttgcaagagttcttccgggttgataacaaccgaactgtgctgcctggtattactgcccgtcaggggaacgctttgtggagtgttccgctaagaatgttcttgggaatcgtcttaatggttgatgcattctcttacaacgccataattccagttggctttggcctgactgcgattgaaggcattattggctgcctgttgttcttcggtctattcacttggattgccagtttggcattaatcgtgatcttcttcatggggattgccagctggccgcatgcttggatcgtctttgcggcgattgccttaatgaatggatccggtcgttccattggtttggactactggttcgttccatggctgcaaaagacttggggccgttcacgttaaggcattccaaagtcactttacaaaaaataaataaccgttaaatgaaataagaggctggaacaaaagattttgttccagcctctatttgtgtctgaatgttatctagcacttatgattcagcttgagtttccggtatctcaacaatgtacttgccataatgagggacatcgacaatttgaatattagtctcaaaaatgttggctagtaattcacgatcgtagcattcttccggtttgccgacttttaccacttcaccccgtttgaccagccacaaaacatcactgatcttaaatgcctgattgatatcatgaatcaccatgataatcgtgatgtgcttctgctcattaagctgcttcaaaatccccatcagttcggcttggtagtgaatgtccaagtaagtcgttggttcatccagcaatagatatgtgggatcttgggccaaagctgaagctaaccagaccctttggcgttggccgccagataacgacgatagtggccgctgtgccaatgatgtcaaatgagtggcctgaatatacttggccacctcggcgtcagaaattgttgccagcaggctgtggtgtgccaacctgcctgttttaacaacatcaatcactttcatatcatcaaaaatatcgttttgctgactaacaactgcaaccttggtcgccaactgtttccgaggaatcgaactaattggctgcccgtcaagatcaacctcaccaccggacggttgaagaatgccagccatcaattttaacagggtcgacttgccggcgccatttggaccgataatcgatagaatgtgccccaccggaattgtcgcactgatctcatttaaaagggtcggttgttgtggataatgataactaacttgatttaagtccattaaaattcttcctttgcaacatcaagattaagaatgggccgccaatgacggtcataatgaccgcggcggacaattcactgggcaacacgacaattcgaccgatggtgtcaacaactaataacagccaagcgcccatgagcatcgacagcggaatgatggtttgataatctctccccactaaataacgaacaacgttgggaacaacgattcccatgaacggaaccgtgccgacaactgaagaaacgcccgaggataagtaaacgaccaccagcagtaaggccagacgcatcatagaagccgaaaccccttttgtctgtagctgttcggttgataatttgagatagttggcccacggtgaaataacgactgccgcgaacatcccactgacacccaaaaataacagcacttcggtctgcgaccaggtaatcccgttaaaagagcccgtcgtctggccgccaaatccattggcaaacagctgctcgaaaccggtaaaggtcagcatcatcgccacaccaatgataatcagccggtatgggctcttgagtgccggtccccgggttaacagtaagagtgcaaataagccgccaaggatggagaaaataaacttgctggcaggaaatgccggtagaagcattgtcccaatgagaatgaagaagtctgaagcgctggtcactcccagaatactggggtctgccaacacatttcgaaaggcagcctggctggcagctcctgctaccgcaagcatacccccacacagcatggttgaaagaatccgcggaaagcgaatgttaatcaaaatgtccagttgattgggattgccaccttgaaaggcggtcatcatttgttgtggagtgatgaagctggcccccaacatcatcgcaaacaaaatggtgatgaccagcatcaccaaaattgtcgaataccatattttttcagatttggtcaattcgtttggctcccttcttgaggatacagccaattcgaaacgatctgcaaggctttggcagcccgcatattggcagttgcatcaaagttgggttcttccagatcataaacgcgatgattcttaacggcaggcagcgtcttccacatcggatcggatttaaattccgagttaaattgtgggatcacgatattgggtaaggcgtgtgccaatcgcaaaataacctgtggctgcgcttttttgatggcttcatcgttgggagagacaaactcttgtgtctttgaagagaaaacattgtgaccaccggagattgcgaccaaatcaccaacgtaggattgattagtggcaatcatataggaagccccgggtaatcccatcaagacaagcacacgaggtttggtggcatgacgcttggcaaccagtttgacatgctgttctgcctggtcaatttgatcaactgcgtgtttggcctgggcttttcgctgatattgtttccccattgcggtcaccgtttgtttcaatttggcgacactggttaaattcagaaaatgaggcgtaatatggcgttccttaaatgcctttccaaattggtcctgcagggtcgtcacggaatagacgacggtcggttttaaactggcaattttttcaacactaggattcatcggattgccaacccgggcagcgtgcgcataacgcgccggaattttattttgagttgtcggtacaccgaccagcgggagatcaagcttatctgcaatttgaacgaccgcaaaagtcgttgccacaatccgagcttttttctgatgattggcagcaccgattcggctcataaaaataccgcccaacacgccaactaccaaaacaagtgagagcacaattaaagcgatcttacgagatcctttcattatccttattgccccctctaatgtttaaagtaaatccacaatcctgctgaaagtccggcaatcacagtcacgccgccgacaatccaaggaaccccgctcttttttgcttggggtttgtctgaagtctttttagctggtttggtcaggttactgctggccttacttggctgtgacgaggctttcttggcggaagactgttttgctttgggttgctttgtcttggttgagctagcagtcttagcagcttttttggtcttctttggtgcattggctttgggtcgactgttggtttgctttgccttcgtacttggactagtagccgccttaggctttgtcgttgacgtagccgtcttaggtgtcgccgctgcggcgtgcgtccttcccaagcttggcagaccagcagtactaaatttgaacgaaatcaagtgatgggccttataaaccttgggcacgtcaatagcgagcttggcattgatccgtttcttcaggttattagcataaaatgaatagtacagcagcgaatctccggcccggtctttcacgcgacggacatttaatggcgctttaccgttgacccaattcactttgactggaaatgatgacaaactcttggcagttttaatttccatcgtgacatagtagagatgatttttcaccaccacattggccggcttaacaaaatagccgtctgccattgacgtttgattggttccatagcgcaatgggtgataggcaatggtttgagcactagctggaataattgaaacgatgaacagtccaatggcgacaaagaggcccaatagccactttgatctatttgacaattccatgattactcccccaaacaaaagataatcctgatacgagtgctaatccaagcattgacaagctgttttggctggcatcaccagtttgtggtaatttagtctggctggaagtactcagcttagctgaagtggctgttggtacaacagcaacatgcttgctggccttggcaggtgctttttggctaaacttgaaacgaattggccaagttgtattgatttgggcttgagggacaaccacatggattgaacctttgataactttcttcaaagttttgaatgatgaaacgttaaatgaataagtcatggtgtagtaattagtcgtttgaccataactaacaactgaggatttcactttgcggccattgatggtcactgggcgaacagcttttgaccccaactttaagttcttcttgtaagcaaccttcagttggacgttgtagtgcttagcaatttttttaatcacggctgttcgagtgtaatattggttagcaattgaccttgaatttgagtcaccctttaaaaccacatactttcgagttgtggttggcacctttgctttagcggtggtcttctttttggtggtaacagttgacgtggtcgttgtcgtcggagttgtagccgaactgctggtagctgcaggcgttgtggcactactgctggtggctgcaggttcggtcgtggtacttgaatcacttgtcgtggttgttgcggcatctgatccagggaccttgacagcatctgcccagtcaaacgaaaagtcggcagattcttgcatttgtccaagaattggaatgttatgaagcgtaaagctaaccggcatagtgctgcttggattggtcaaattgaacgttaaggttccattgttcccagaggtcacaattggcaatgccgtttgatcccccatcgtcatgctggcaatatagttggcaccgtttgtcgtaatgacggtcgtataggttcctttagacactgtcacctgggcagtttggtcaaaaaaatgattggcaatcgattgagaactgctgccgctcttcaataaagtaattggtacagtgtacgaagcgtcacttaggttgacagaatcagccttagcattggatgaaaatgcaccccccacaaatgcgaaaataattgctacaaaaacaaactgaataaaatgtacaaaacgttttttcatgcgaaaatccccctttaggtataaaaataattgtacacagtaagtttaccattagtttggaggtaaataacgtcaaatttgtgaattgataggcaaaaagcattactttttctcaagcgctttcttgccacattgtttatggattttgctcttaaacaactgacgaagttaattaatcaaaatatttgtctggttaatgaacaacggctgatttgttaggaacgcactgaacaaagaaaacccagccagtacttcacatcttttgccggaacaagcggtcttggggacgtgtgggctctagtctcacctccggtatcacagcaagcgaagtccatataagagcgtcatacatcgtctgttgtttgagatacttcgataccactgagccttacaaaaaatgcctccagccctcatcataagaggctggaagcatctgtgcggttcatcaatctaaatgtatctgacagccattgccaggatttgaacctgggaccttttccttaccatggaaatgctctaccttctgagctacaacggcatggttgaatcaaagaacataaatcgatattatcaaaaaaagcaccgatagtaaatactatcagtgctttaggattgcgtggcaacgtcctaccctcgcagggggcgatcccccaactactcttggcgtgcagaagcttaacttctgtgttcggcatgggaacaggtgtatccttctggctatcgccaccacactatttttccttgaaagaacttcgttctctcaaaactagctaatattaattttctgcccttgaacaccatttctacttggttaagtcctcgaccgattagtattggtccgctccgtacatcactgcacttccacttccaacctatctacctgatcatctctcaggggtcttacttccatataggaatgggaaatctcatcttgaggtgagtttcacacttagatgctttcagcgtttatctcatccatacgtagctacccagcggtgcgcctggcggcgcaactggtacaccagcggtatgtccatcccggtcctctcgtactaaggacagctcctctcaaatttcctacgcccgcgacggatagggaccgaactgtctcacgacgttctgaacccagctcgcgtaccgctttaatgggcgaacagcccaacccttgggaccgactacagccccaggatgcgatgagccgacatcgaggtgccaaacctccccgtcgatgtggactcttgggggagataagcctgttatccccagggtagcttttatccgttgagcgatggcccttccatacggtaccaccggatcactaagcccgactttcgtccctgctcgacctgtctgtctcgcagtcaagctcccttctgcctttacactcgttgaatgatttccaaccattctgagggaacctttgggcgcctccgttactgtttgggaggcgaccgccccagtcaaactgcctacctgacactgtctcccgccacgctaagtggcgcgggttagagtgttcacacagcgagggtagtatcccaccaacgcctctgccgaaactagcgttccggcttcaatggctcctacctatcctgtacaagctgtgtcaacacccaatatcaagctacagtaaagctccatggggtctttccgtcctgtcgcgggtaacctgcttcttcacaggtatcttaatttcaccgagtctctcgttgagacagtgcccagatcgttacgcctttcgtgcgggtcggaacttacccgacaaggaatttcgctaccttaggaccgttatagttacggccgccgtttactggggcttcatttctgggcttcgccgaagctaactcatccacttaaccttccagcaccgggcaggcgtcagcccctatacgtcatcttacgattttgcagaaacctgtgtttttgataaacagtcgcctgggccttttcactgcggctgtgcttgcgcacagcaccccttctcccgaagttacggggtcattttgccgagttccttaacgagagttcactcgctcacctgaggattctctcctcgactacctgtgtcggtttgcggtacgggtagttgatgactcactagaagcttttctcggcagtgtgacgttggttgcttccctacttaaatttcggtcctcatcaccacttgtcaacccgccaaaaagcatttgactctttgactgactcgtggcttgaacatccctttccaactggatgcacaacttagcctcctgcgtccctccatcgctcaaacatcatcaactagtacaggaatctcaacctgttatccatcgcctacgccttgcggcctcggcttaggtcccgactaaccctgggaggacgagccttccccaggaaaccttagtcattcggtggatcagattctcactgatctttcgctactcataccggcattctcacttctaagcgctccaccagtccttacggtctggcttcattgcccttagaacgctctcctatcacttgaccgaaggtcaagtccacagtctcggtaatatgcttagccccggtaaattttcggcgcggaatcactcgactagtgagctattacgcactctttaaatggtggctgcttctgagccaacatcctagttgtctatgcaactccacatccttttccacttagcatatatttagggaccttaactggtggtctgggctgttccccttttgacgatggatcttatcactcaccgtctgactcccggataaaaatcaatggtattcggagtttatctgaacttagtaacccatgacgggcccctcatccaaacagtggctctacctccatgattctacgtccgaggctagccctaaagctatttcggagagaaccagctatctccaagttcgtttggaatttcaccgctacccacacctcatcccagcacttttcaacgtacacgggttcgggcctccagtgcgttttaccgcaccttcaccctggacatgggtagatcacctggtttcgggtctacagcaacatactaaaacgcccatttcagactcgctttcgctgcggctccggcttttaaaccttaacctggcatgttaccgtaactcgccggttcattctacaagaggcacgctatcacccattaacgggctctaactgcttgtaggcacatggtttcaggaactatttcactccccttccggggtgcttttcacctttccctcacggtactggttcactatcggtcactagagagtatttagccttgggagatggtcctcccggattccgacgacgtttcacgtgtgtcgccgtactcaggatcctgaactgagggtcattgatttcacctacggggctatcaccctgtttcgccaaccttcccagattgttcgattatcaacaactttggtaactcaaatgttcagtcctacaaccccaatgagcaagctcattggtttgggctgttccccgttcgctcgccgctactgagggaatcgaaaatttctttctgctcctgtgggtactgagatgtttcagttccccacgtctacctctatacagctatgaattcactatatagtaacagtcgattaaaactgctgggtttccccattcggaaatctccggatcaaagcttacgtacagctccccgaagcatatcgatggtagtcccgtccttcatcggcttctagtgccaaggcatccaccatgcgccctttttaacttaacctgtacatcacgacgtgatgcaaagttaattgagtatttgcgatttttttctagttaacaaactcaaaataacgcggtgttctcagttgaaattatataaatacaatttcaaaaaaattattacagaaaattaatattatctagttttcaaagaacgaattgagagtagacctctcaaaactaaacaaaactttcgacaatgtgcaggattccgtttttccttagaaaggaggtgatccagccgcaggttctcctacggctaccttgttacgacttcaccctaatcatctgccccaccttaggcggctggtccccgaaggttacctcaccggctttgggtgttacaaactctcatggtgtgacgggcggtgtgtacaaggcccgggaacgtattcaccgtggcatgctgatccacgattactagcgattccaacttcatgtaggcgagttgcagcctacaatccgaactgagaacggctttaagagattagcttgacctcgcggtttcgcgactcgttgtaccgtccattgtagcacgtgtgtagcccaggtcataaggggcatgatgatttgacgtcatccccaccttcctccggtttgtcaccggcagtcttgctagagtgcccaactgaatgctggcaactaacaataagggttgcgctcgttgcgggacttaacccaacatctcacgacacgagctgacgacaaccatgcaccacctgtcattctgtccccgaagggaacgcctaatctcttaagttggcagaagatgtcaagacctggtaaggttcttcgcgtagcatcgaattaaaccacatgctccaccgcttgtgcgggcccccgtcaattcctttgagtttcaaccttgcggtcgtactccccaggcggagtgcttaatgcgttagctgcagcactgaagggcggaaaccctccaacacttagcactcatcgtttacggcatggactaccagggtatctaatcctgttcgctacccatgctttcgagcctcagcgtcagttacagaccagacagccgccttcgccactggtgttcttccatatatctacgcatttcaccgctacacatggagttccactgtcctcttctgcactcaagtctcccggtttccgatgcacttctccggttaagccgaaggctttcacatcagacctaaaaaaccgcctgcgctcgctttacgcccaataaatccggacaacgcttgccacctacgtattaccgcggctgctggcacgtagttagccgtggctttctggttggataccgtcaagatgtcaacagttactctgacacctgttcttctccaacaacagagttttacgagccgaaacccttcatcactcacgcggcgttgctccatcagactttcgtccattgtggaagattccctactgctgcctcccgtaggagtttgggccgtgtctcagtcccaatgtggccgattaccctctcaggtcggctacgtatcatcgccttggtaggccgttaccttaccaacaagctaatacgccgcgggtccatcctaaagtgacagccgaagccgtcttttaaaccaaaaccaggtggttttggttgttatacggtattagcacctgtttccaagtgttatcccctacttcaagggcaggttacccacgtgttactcaccagttcgccactcgtctcaatgttaaatctttcaaatgcaagcacctaaaatcattaacggagacgcgttcgacttgcatgtattaggcacgccgccagcgttcgtcctgagccaggatcaaactctcatcttaaattgtttaaaatgataagcctgtgatagctcatgatttaaatttattatttgttttacgaattgacttcgcaaatgtttggttccaattccgaagaattgaaacgccctgcacatttgtttgtcgaaaattttgttcagttttcaaaggtctacttggttgtggaagagatgaatcatctctcgcgacaactatttaaatataccacgctgattgttttatgtcaacaactttctcaattgattgaattgatattggttggtcacgaacaaaaacagcacctataaatatatcgaagtttgatcaattcgtcaagccccaatttcaaatcaattgaactttaacgatcgggactgtttatcccaaacgatgacttgttttaatccaaattaaaagtggaacatccctgttccactttaattcgcaaacctatttcaattcaggtgcatcggtcttgtacaaattcatagttgatttaccattgttccttgcttcaatgctggttggttctttcttttgggcctgcttcaaattatcaagagcctttgtatattgataagtaaaatctttgcgattaacttttttgaatcccttaggtgtgtagaacctgagtaaatctccccagatgacccgatcggataatgataattccgttgtcacatggttttggatgctagccaactgccgtttttgagcggcatttggcgtaatcagtttgcccgtcttagtcaaataaacgtcgctgcccaccttggtatatttcggtgtaacaaagtcgccatcccggaatgcaacccgctgatcatgctgcttggataacagatcggttccaaactgaatcgtattattattcttgtcgcctaacagatgcaaaatagttggcaagacatcaatctcaccaccatatgtgtgattgaccccacccttaaggccaggtgcatgaatcatgaacggaaccttctggaactgtgccaaatcataattgttaatcgacttcttatgaagcagctgggcaatggccgggcggtgattattggaaataccgtaatgatcaccgtatacgacaatcatactgttcttcatcaaaccggttcgcttaagataattcataaattccgcgaaggcctggtccagataatgggcagtttgaacgtatgggtcaaccgttttatccccggtcttagtggcaggaaaatcagtattttgtttatccagcaaatatggataatgattggtcaaagtaatgagtttggcataaaacggctgaggcagctgctgaatataattggcagcatctctaaagaaaatcttatccttgagaccatacccgacactgtaagacggcttcgtcttgtaatattgagagctgaagaaataatcatatccccaggacttgtacgtactgtcccgattccaaaagctgggaacatccccatggaatgcagctgttgtgtagcctcgttgatccaagatagcgggcgccgcctgatacgtgttctgggcaccatatgtcaccatggcagatccttgaggtaacccgtacagagaattttccaacatcatttcggcatcagaagtcttcccttgagcaacctggtggaagaagttatcaaaaccaatggtatttttattgtggaaaaaggcattcaggtggggcgtcacttccctgccgtcgactttataatcaattaagaactgctggaaactttcaagatgaataatgaagacgttctcgcccttggccttgccaaaataagccggattggccttggcccgactatgatctaagtatttcaaaatactatccatatcgctggccttggcttttgatcgggtagcggattctttttgggtttggtatgcattaaaagcggcatactcgtttaaccctaagtatttaacaatataattattgtcgaaagttcgggtcaacaaaccagaccgatccgtgcttgccagaccgtattcgccacccattaagagaaaagaaacgatcgtaatgaaaaatgcataacgcttcttaaatggagcggcgtcaattcgaatcacgtgaaaagccaacaacgcaatcaaaataatcacatccagaaaaacaaaaaagtcactgaagtgaagaatttcaaccaggctcttccccaagttattttgaacattgccggatcctttgatgacacccaacgaaagaaagtcggaaaactcacggtagtacagaatattggcaaaaatccagatgctctccaaagtatcgatgatcatcatcaaccaataagatagccggccactaaaataaagggcaatgcccaatgtcaatagtgccgccgggatggggttgactgccagcaagaattcctgcatgccgcctttaacgcccagcgtaaatttagtttgatacgcaatatacgtcttgatacaaaataaaatgacaaccagcaaaaagaagccaattctggtgtttaaaagatttgaaaaacgatatttcttatccgttaacattcctgttcctccaaatgtttccctgcccgctatttaatgcggttatcgggatcatcaactttatctggtttgactaataaagcacaggccccagcagccattccaaagtaatacgttaaaattctccaaataatcattgccaataccaatttgctgttactcgaaataaagctatggaaaagtgattcaaaactgaattcggcaccaccagaaccaccaggaattgggaacaacgaaataatcatcacaatcatgatgtgtaaactggtaaccataatcacgttgatactagtatagccgagcgatagcataatgaaatatgggatgaggtaataaaaaagaagttgaaaaaatgtgagaacaacgatttttaataatagcttgggttgacgcccgattctgacgctttcctcaaacaaattatcaattttggaatacatcgtttcacgcattgaataaaatttctcgtccttgatgaaccatttaacaggatgaaaaagtaattttgaaagtttcttggtaaacgacggccaatacattatcaacagtaagccaacgatgacaaatagatgaattaaaaagccaaataaaacgaacagcgccaaaaagtgcaatttggttgcgacaaaatggaatccaatgaccaagctgataaaaaagttgatcacaatcattccttgatacaccacaaacttcatcaacagagcggagcttgcccgaccgccatcaatcccagtctgcagcatgacaaacaactgtccgggttggcccccagatgaaaacggggtaatcccattaaatagctgttcaaccagcggaacccgcagagcatccttaaacgtgaagtgttcaacgcgattggacaccaagacttttgtaattacgccctcaattaataaataggcacagatgcaaagaaaggcgactaaaatccaccaaggattcagggtgaacaggtcatggatcagcacactcaatttaacgtccctcaaagagtatgcaataattgcaatcccaattatcaccatcgtaaagagggtaattttattatttcgtgacattattaaccttccttagattgttgattataaaaatcataccaaactttggcgagatgatcttcagaatagcgttcactggcaatcgtcgtttcatgctgtaaagccgccaatttgtcaggattcaataacagttggtgcagctgttcgttcatctgtttttcatcagcagcaggaagataataaccgctgatgatcgacttgtataaatcaaggtcccgaagcatcaccggggtattggtcgaaaacgcttcaagaaccgacattggaaacaattcattgtaagacggaaggagaaataaatccgccatattataatattgaaccatcttggcgcggtcaataattcctggaaacgataaattacttgggggatccttgacgattttttccaaatcagcataaccctcggtaattttgccaaacgaaaaaccacccgtccaaataaattggatcgtcgggttttgcttggccagctccacgaaatccaacacccctttacgagtttgaatttggccgctgcctaaaatggtgaatcgttttggatcgtatccatgcttgactcttagggcttgtttttgttggtcatcaacatcgtagaactcggctttgctgacgaaattaggaatataagtaatccgttgcttgttaattccgtagcgttccagcttgggaataaacgatgggttaaccacgacaatgtggtccatccgcttataaaaggcaattacatacttataaaaaatcgccttaaacggctgggggattttaatgctgccttccaaggtttccggcaggaaatggacatagccgatttttcgccctcttcgcctggaaaatgtcgagaggtagaaactgggattaattgtatggtaatgagtaatatccgcaggtgcatagctattaatggtgattttaaaatcgttaggaaagtggtccttgagcattctcaccagttccacataggcactgccgacgccttgacccttgaccttatccgcggttgaaaacatattaatccttaacatacaaactcctcacaaaatatttagtcgatattagtagtggcattgtcttgtaattcttgagccaccgctactgaatgataaaagttaatcacccgtttgccaaaggtttctgcagaaattgcagtcagtttctttttcaagatttgtttggctttgggtgtctgagtattgacctcgtgctttaaataatgggtcacaatcccaacaaattcatcgtcgtgctcaaatgtctgccccaaagtttcggagctcaacaatccattggtataatcactggccgaaacgactactggaagtccggcagccatcgcttcaatgtaggttagtccttgagattctgatttagaggtggaaacaaagacgtcgcatgcccgatagaaagcattgacatgatcattagcaacttcaccggtaaagatgacatgatcatccagctgcagcgcatgcacctgactcatcaaatcatctttggcgggaccgtcacccacaatcattaagatggcgtttggaacctccgtcaaaatttttggcaggtagtcaattacctctaagatgtttttttcgtatgccaaacggctaatcgaaagcatcagcggcgtatctggagaaatatgatactctttgcgaatgtcggtcttgatttcttcagcgtacatatcaacatcgattccggttggaataatccgaatctcgcttttaacaccgtaatctgtcaacttgtccaatacgcgatcactgggggcaattacacccgacaggtggtagcaaaaagccaacgtcccttctttaacgtggacgggtttgagcaacttgccattagccacatagtgcaaataatcttcatacattgtgtgataagtatgcacacaaggaatattcaggtttttggcgacaaatttgccgatcattcccatcgaaaactcggtttgcgtatgaacaatatccaagttgagttctttggcaatttcgtaagcttgaaataatccgcggaccgcaatccgccgatccgtaaatgagataaaggggatacttgagaaacggaaaatattctgctcgtaggtgtccttatcgacatgcggatctgttgtggtgaaaatatagacctggttgccctgtctctccaattcatttttgagagtcttaatcgaggtcgcaacaccgctcacctgcggaaaatatgtatccgtaaaaatcccaatattcacggctgacacccctttctgataaaaatcgattaattatgctcgtgaaatgtgccgtcaggccgttacccggtgtgacgcatagtctcacaatcattgtaattatattggtttagttctgctattgcaaaccacccgaataaaaagaacaagccgaaaacagacggtttaacgccattaacagcttgttctttaagttatttataaatctattggacgttattagtggcctggtgaacaaaggcagtgacttcttcactggcgctggccatggtaaccgccttgttggcaagggtgaccatctctcttgaatcgagccgtttgattaacgctcgggacttgagaattgaagaagcgctcattgaaaattcgttgagccccattccaaccaaaattggaatcgcggtctgatcgccagccatctcaccgcacatataagcaggaagattattatcatgacaagcgtcgataatatgcttgatcattcgtaaaacggctggattataaggctggtaaagatatgaaaccatccggttgccacgatcggcggccatgatgtattggattaaatcattcgtcccaatactcatgaaatcaacctcattggcaaattggtcagccaaaatggcagcggccggaacttcaaccataatcccaatcttaaccggttttacccgaaccttttcccgaatcaatttgatccgttcctgattaaaaatattcttagcttttttcagttcattaatggtcgtaatcattggaaacatcactgacagattcccaaacgaagaagcccgcagcagcgcgcggacctgggtgcggaaaatatccggcttatccaggctcatccgaattgcccgatatcccaaaaatggattggcctcctttggaacatccaaatacggtaaatccttgtcaccaccgatatcagcagtccgaatgatcaccggctttttatccatcttttgaagcaccgtcttgtaaacattgaactgctcatcttcagtaggcaggtgattagagtccatatataaaaattcagttcgaaacaggccgattccctcggcaccgttttcgatagcgccgtccagatcgtccaaagtgccaatattagcagcaatgattggatgcttaccgtcagaagaactggtcatttgatgtttgaaatcagccaacttgctcttgcgttgacgatagtcagcctgcttttgagtatattcgtctgtttgggcttcagtcggattaacgatgacgttcccagttgatccgtcaacaatgaccgtatcgccattcttgatatctgccagccggcccttgaatccaacgaccgcaggaatctccaatgaacgcgacattatggccgaatgagaagtccgtccacccatatcggacacgattcccaacacataactcggcacgaattgagctgtgtcgctgggagttaagtcgtgggcaatgataatgaccttgtggtgaatcaaggccggatcaaccagcggcactcgcagcaggtgacttaaaacccgcttggtaacatcacgaatatcgcttgaacgttggcgaatatattcgttatccgtcattgaattaaagattttgatgtagccgtccgtgactttggttaaagcatattcggcattcaccttctctttttcaatcgttgatttgatccgattgagtaattcaggatcagacaaaattgcgccatgagctttaaagacctcagcttcactgctgccgaggtcttcaagtgttcgttgttgaattgttaaaagctcgtcttttgagacatcaatcgcagcataaagccgcttaatttcatcagaggcatcagtaatgctccgctttttaaagcttaaatcaggttcagttaaccgaaatgcagatgcaatggcaattccatcacttgcggcaatccccttaaactctttcatgaaattattcagtcagtccttctgctttcatcgtttcgctaattgcatcaatggcttctttttcgtcatcgccgtcagcagtaatcgtaacagctgcactttgaccaactccgagtgacatcacacccataattgacttcaagttaactgacttttcttggtattcaagggtgatatctgagttgaacttgctggcagtttgaaccaacaaagtagctggacgagcatgaattcctgtttctgcgatgatattaaattgacgtttttccattattaatcaatctcctctgataagattataaattttgaagatgatgctcaaaatttaaatttgttctttacttaattaagaatagcaatatataagggaaaatacaagtttaaacttaaccgcttacagggtttttaagaacttttttgcttgtcgtctctctcataaacataggtaatcacaccgccttcggtcgcggacccaaccacccgctttcgatggtcaaagttcatgtatgctgtctgaaaggccatgaatgattccggcttgacttcgattttttcaatctcacctgattccaacttttctaacaactgattgtagtcttgattctcttctgccacaacgtctcatctcctttcaatttaagtgaagttcaattacttgattacatataatcatgttgtataataatttcaaaggtcaaagttggtcagtgattaacagatcctccttgtccttttatttctatattaaaggaggaaagcaattaatgctatgtcaaaattgccataagaacccagcaacgattcacttgtacactaatgtgaatgggcaaaagcaaactattaacctttgccaaaattgctatcaactcctatccaatcaacaacgtaatacaggaggtgctcaaaatatggctcaagatccatttggttttggtggattagatgacattttccgtgcaatgcaaggcggaaacgttgatccaaccaatggtcaacaagtgccaccaacccaaccaatgggacccaacaatggcggccccaaccgaccaagaaccggcggagcgggcggaaattccctgcttggtcaatacggaattaatttgacccagcttgccaaagatggcaaagttgacccggttatcggtcgtgacaatgaaattcaacgggtaattgaaatcctgaaccgccggacaaagaataaccccgtccttattggggaagccggtgttggtaaaactgctgtcgttgaaggacttgctcaagaaattgtttccggcaacgttccttcaaagcttcagaataagcaaattattcgtcttgacgtggtttctttggttcaaggaaccggaatccgtggtcaatttgaacaaagaatgcagcagttaattaaagaagttcaagataatcccgacatcatcctgttcattgatgaaattcatgaaattgttggtgccggtaacgctgaaggtggtatggatgccggaaacgttttgaagccagcattggctcgaggcgagttccagttgatcggtgccactactttaaaggaataccgtgatatcgaaaaggactctgctttggctcgtcgtttgcagccggtaacggttgatgaaccaagccccgaagaatctattaagattttgaaaggtatccaaaagcgttatgaagattaccaccacgttaagtacaccgatgacgcgattgaagcggccgttaagctgtcagaccgttacattcaggatcgattcttacctgataaagccatcgacttacttgatgaagccggatcacgaaagaatttgaccatcaatgccgttgatccacacacggtcgatgaaaaaattcaaagtgccgaaaagcaaaagcaagctgcgttgaagagtgaagactacgaaaaagctgcttactaccgtgatcaagttaccaagcttgaaaatgccaagaagaacggcagtgtcgactcggcagcaacaccaaaggtcactgctcaagacatggaaaagattgtcgaagagaagactgaaattccggttggtgaacttcaaaccaaggaacaacaacaacttcgtaatttggcccctaaccttgaaaaacacgttatcggacaaaacgaagcggttgaaaaagttgctcgggcaattcgtcgtaatcgggttggcttcaacggtaccggccgaccaattggttcattcctgtttgtcggacctaccggtgttggtaaaactgaaatggctaagcagctggcctatgaactgtttggttcaaaggattcgatgatccggtttgacatgtctgagtacatggagccgcattcagtggctaagttgatcggttcacctcctggctacgttgggtacgaagaagccggtcagttgactgaacaggttcgtcgtcacccatactcattgattttactcgatgaagttgaaaaagctcacccagatgttcttcatatgttcctgcagattcttgacgatggtcgtttgactgatagtcagggacgaacagtttcatttaaggataccatcattatcatgaccagtaacgccggtcagggtaatgcggaagccaacgttggtttcggtgctgcagccagtgggaagacccattcaattattgataagttgaccgactacttcaagcccgaattgttgaaccgtttcgatgacattgttgagttccactcattatcaaaggacaacctgatgaagattgtttccttgatgattgacgatgtcaacggtatgcttaagcaacaaggattgaagatcaacgtgactgacaaggccaaggccaaattggttgacttgggctacaatccagctatgggagctcgtccacttcgaagagttatccaagagcagattgaagacaaggttgccgacttctacttggatcacgaaaatgctgctacattaacagctgacgtagattcaaagggcaacattgttatcaagagcgacagcgcggctgaagtaaaagcttcaaccaaagcaaagcctgatagcaaggattcagataaataagtattaaaacattaaggggtaacggtcagagtttgagactttgatcgttaccctttttgtattctcaccatgattccccaactatggtactaactgtcgccttttctgggttgaatcgttaaaataatccttaaattcggtggtgccaatgctgattatgctataatttttattagaagattgtagatcggagcatttatcaaatgaagttcatggattgggtcaaacaacaattaaatatctttgtgtcgccgcgatcccatcggcaatcaaatcgtcggggccgtcgccgggactatcaccaacgaaagcggtggcagtctgcacaagtggacccggataatagtgaccaaacggcagaagtagacaactcttccaatcaagacgcggttaaagaccaagcggatgggttgctcaacgacccttcccctgcaccttctcaagccgaggagacaattcaaatcaagtctcaagtgaccttcttttatctcgatgaaaatgacgatccaatcaaaaagcctgacattttaattggtaacgatggtgagcgcttttcccttcaacttcccagctttaaacaatattacctggtctcaattgataacttttcgacttattttgcagataccgatcaagaagtgacattccgatatgctctcaaacaagggttgccggtcctagcctattatttggacattgataccggtgaaacgttgcatcacgtcacaatccactcaggcaaactgggtgagtcttatgacgtttcagctgcggatatccccggctaccgcgtcatcaatgatgtcggtcccactcacggccactttgatgaccgcacccatggaatgatcttttattatcgacgaatccattggcaaactgtccaaccagttgagtattatgtccgtctgaagaagcgacacgctgtcttggaccaaccaaatggccatgcgttacaaaccggattaccggccaatgttatcaccaagatttttgcccgcatcgaaacgacggacaatcaaagctggctgaatattggcggttttgaatggattaaaaatgccgaccttgaacccagtgacccgccgaccaatcatctcgttccaccgattacgaaaacttccaggaatccggtcatgctgtttgggacagttgatttcgtagctggcaggccaattgaggtctttgataaaccgtatggcaccagtactggaacagtggcagacggacaacgggtttcaattaaagcccgaattatcgatgatcagggcctgatttggtacgagctggctgatcagtcagtcatctttagtgaatatgttagaattgattcctaatttaatcagattgggatcaaagtcgatttgatcccagaatttaagtaaaaatcgagttattcctgttttgggaatgactcgattttttgcttaaaaaactgggatcagccgtttgccaggtggcttggcaagcacgctggccggcgccgcaagttttgtcagtataaacgtggtgatcaaagctgacggctatttaaaaatgacaaatatgaaaaccgatactagcgcaatcatgcaaacgacaaccgcaaatccaccaacaatcattaatttttccaaccgattctttgccggatcccgcttttgccgttgctcctcaacatcttggccatccgtgaaggccacgatttcagcataagttctcaagtttttgcgtttctttattcgctcgacttgagatgcgctaatgaacatgaccgcaaaacagatgatcggcaccaaaataatcaacgtcgattgctcaaagtaaataactaacccgattgacattgtgcccaaaacagctgcgattagcatcacccaagtataagctgacattgccgtattgactttcttatcagataatttagctttcatcgcttccaaatcccccttgatgagttcatctacagaaacgccaaataaaacacttagtagtaaaacgttttgaatatccggatactgtttgccggtttcccaatttgaaattgtctgcctggaaacatatattttagatgctaattcttcttgagaaagaccacggacttctcgataagcccgaattttattgccaatgtccatttcctcaactcctcatccaaaagtatacctgaatgttgggacgatttctgtcacgttgccgtatattgtcaccaaaatgatcaatggaaagtcaatgcgacacctcgcaggttggcgaacgcaaaccgcaatctcaaagtttgccttttttatataaacacgttgtatctagcgcttcgctttatcaaccatgacttaacacgttggacaaaaaaagctggtgaacaaatctgttcaccagccagttcttcttcatgagaccacaagagtgaaattgttccctcgttggttgaaacatgttccgaagctaatcagcttggtcttgtctctaaagatttttatccatattaaacgtcaacttggacagtgtcagtcccttttcaatcaattggtgattgaaatgttcagtggcaattcgcatcattttgacaacttcatgattttgctcggtcaagtagctggtcaattcttcacccttcagtgcctgactttcatcaatcgcgctttggacgtggcgacgcagttgttccttcatgtcagttaagaaatcaacatcatcttgaataaattcagaataatgggattccactaacatcgacaatttgcggtacatccaataggcgctgacatcatcgcaatggaccggcgtgttggcataagtatcatcggtatccgttgcattagcaaagaatggcacatatggtgaaaatgccggtaccccaaagcacagccacataattgcattactgttatttttgagatcattacgaatctgcaaaacatgtgaattttgggtccgattcattgaaattggccgaaacagcgtcttagtgtcctcatggcctttactaaacggatcatagggcgtttcgttgtaatgagagctcaaaatgtactcaacatcttcgacactaattttatggtccgtatgacagatgaacggtaaatttgaggaagttggtgactgctcaatttccggattcaggtatttctggccgaaccaaacccgaggcgtattgtaatgacggtccttctcgttatccgttccaaagatgtggcggaagttaaatccctgcttgtcagtgttcaaatgatacttctcgacaaattcttggatgccgtctgaatacatgaagttgtctggatcatcaaatttcacctgttggatagcaacttgattggcggcaatcgcataggcgtcatcaggaattcgttgagcaacccagtgatgaccggtaacaatttccatgtaccagacttcattgttatcgctaaacaaaaccccattaccctcgggtgatccgtactgcttgattaatttaccaagatactgaacaccgtctctggcagaatcaatgtaaggcaaaaccattgactgcaaagagtcctcagctaggccgtctttgaccaatggatcaaaggccagcgcccgctcattcccgtaaacactttcagtggcactcatggcaacgttcttttcgttaaagccactttcggcgtagacaccttccttatcaacttcaacgttgggcgtcaatgagtaacgataggcctgctttggcaatggtgccttaaaaccgttttggttggaaacccactcaccggtttggtgatcattggcgggttcaacatagaaacgttggggtgttagcggcaaaaatgtatcatcatttctggcaatcatcgttgagccatcgatggaagcttttttaccgacaagaactgtggtgcatgcggacaaatgtttggaaaccatcatatctcttctttcaaagttaaattatagtttagcggtcaatgtaacatcagggtacttatccttgaaccagcgaagggcaaattcattctcaaataagaataacggattgccggcgcgatcctttaccaataagtttctggaggacgacatcttttcgtcaagttgatcagggtcaatccagcgggcaatcttatggcccattggatccatattaacctcagaattgtattcgttcttcattctgaattggaaaacttcaaactgcagctgaccgactgccccgagaatatagtcattggtggtataggattggtaaagctgtaccgccccttcttggaccagttggtcgattcctttatggaatgatttttgtttcatgacattcttagcagaaactcggacaaatagttccggagtaaattggggcagcttttcaaactcgacttttttcttaccagtataaatcgtgtcaccaatctggaaattaccggtatcgtataatccgataatatctccggcaaccgccgtctggacgttctctctggtattagccatgaattcggtcacattggataatcgcagtttcttctgtgtccgataaaggttaacgtccatccccttctcaaactcaccggagcaaacccggacaaacgcgatccggtcccgatgattcgggttcatgttcgcttgaattttgaagacaaagccagagaaagtatcgtcatccggcttgattaaatcgccctcttccgtcttgtgggcacttggcgccggtgcgtatttcaaataagcgtcaaagaacgtcttgacaccaaagttgaccaaggctgacccaaagaataccggagtcatatcaccagtcgcaattttaccctcgtcgaattgattaccagccatatccaagagttcaatcgcgtctttggcgtcttcaaactgttcgtcctgggcaagttgatcgttgttcaccggatcattattatcatccaaatcaacaatttctgaagactggttgtttttttcgtgattataaagttcaacgtgatggttatagcgatcaaaaattccagtcaaggtcttgcccatgccaattggccaattcatcgggtaggcttcaatgcctaacacattctctaattcatcaaccagatccattggttcgcgaccatcacgatcgagtttattcataaaggtgaaaattggaatgccccgcatcttacagatttgaaataacttcttagtctgcggttcaatccctttggcggaatcaatcaccatcacggcagagtccaccgccatcagtgtccgataagtatcttcggaaaaatcctcatggcccggggtatccaaaatattaattcgtttgccaccgtaatcaaactgcatgacggaactggtaaccgaaatcccccgcttctgttcaatttccatccagtcggatttagcaaaattaccggtctttcgggcttttaccgttccggctgaacgaacgacgccaccaaagagcagcagctgctccgtgatggttgtctttccggcatcggggtgggaaatgatcgcaaatgtccgccgggtactgtcttccttttctaattgttgggtattcatgtttacttcctttcaggcgagtcaataactaattaattttaacacgttttaggcgactctcctagaacccacgtcaatttcgttggtgcaatccaaaacaaagaggatggaaacaaaacatcagctttgtgccatcccctctttgatgtgaaattacatgccactttcaatttgatgcatgacgtagttcaccactttcaatgaactcagaccatcgttaatcgcacagaagcggttatagaagttcatgaacttctcgttggctgacatatcaggatgcgccaaggcatggttgatttcggctaacagctgcttggagttttcagcaattttacctggcagatccttctcatagttgagatagaacccacgcagttcctccttgtacaaatggtaatcgtaagggtagaacaaaattggccgctttaggtaggcatagtcgaagaaaactgacgagtaatcggtgatcaataggtcggataccaaatacaagtcactgatgtttggataattcgaataatcgtaaacgaagtctgaataatcggaaatatccaaggcattggaaatcaaataatgcatccgcagaattaagaccgtgtcatcgccaaacgacttccggaagtcatccaaatcaaacggcagctcgaaggtatacttacccttctcggcaaattgattgtcccgatacgtgggggcatacataaccacctttttatccaacggaattcctaactgctctttgatagcatcaatatcttccggctgggtattgattaattcatcgtttcgcggatacccaatctttaagatttggttgttgaagccaaatgcagaacggaaaatctgcgttgagtagtcatttggtgaaaccaaggcatcccaacgattggcttctctgacaaagttcttgtgatatttgacggtggtggtcccaggcattgaaacgttttcgatatccaggcccaactttttaaggggcgtcccatgccaggtttgaatataggtcacatagttgggcttcttaacccaagttgggaagcgggcattactgatccaaaattgggacttttccaagacccgaacccacttgttggttcgccgaatcacgtaggcaatttgattttccttacaaaacttcttctgagagcgatcaattgaccagatcatattaataccaggatataacgttttgaagaccttataaatggcgtacggactgtcactaacctggcggccgccaaagctttcaaaaataatcgtggtgttatcgtatggtgaatggcccgacttgaacaggaaccgcattctaaccaggttcaatttgtcttgaatcatcttaataacatcaataatggtgccggccttgccgccagctgcacccaccttctggagcagagaagcgccagcaaattccttgactaaaatgccattatcatatcgtttttccaaagtgatctcacggttaccagccagttgaatgtcggttgattggccggctagtgacttggagataattaatcgctgcttgatagatttgccgttcaactcgtattcgatgaaaagttctccgattgaattttggggaatgtcggttagcggaatggcaaccgtaaacatcccttcaaacagctttttggtgactgggtattccagtgtgccctcggtcgtgtggtttttcaggatgatgcgttgatttttgattagcgtcccgttgatcttgttataaccggtaatttccaagttttcatcggttaagttgaccgaattgatcatgaattcttcatcggattggtgagtccgaatgttaaacaacgccattccctgggcatcgctgttgaattggtaataactggttaattccagttgatgacggtcacttaaatattcactttcaacctgaatcacatttttgttggtcaagttgttgttgatgagaaaaatctgccattcaaattcagtttgatcctctgattgaaaatggaagtcctgggcatcgatgttgacccggataatattgtgggacagcactttgctgatcggcttcatgatcgaggccaagctatttttttcgacaaataaaacgtaagcagtatctaatgacaccgcaacgtctaataattcaaattcaaggacttgtttgcccttcttttgatggacacctgataatatcgctcgcaatttaatttccccttaataattaaagattcgtttgcctggcaggtacttggatgcatcgacaatgttgtcgatatcgatgtatgtccgggcgtcttcaatattcatgtttaacaagacttgatgataaaaggcattaatatcgtcgtagcgatggtaatcgctgtatgataatgctttggtgaaggtcgacttaccttggccttcgtaggctgtcagcatttcgtcctttgaattagacttgtcatcttgaatctcgcttaattcctgaggggcagcaatcgttgaactgggggtgacgttataactcaccttttggtccttcacgtagttggtaaatcggtaaaccagttcacctttggcattcagcagcaagctttcagtcagtgcatcatcaacatatttttcaatcccaaataatcggtcggcatcatcgtaactgttgatttggctgatccggctgcttttgtcaaagtaaagggtatgtatccgggtgttgtcttcggtaaataaggtttcagcgacgatgtttccgtcagcgtcaatgtatctggtcaccggcaattttccttgatgcgccttaaaggtctgtaatccagacagatccggatccatgaaatcggcggcctttagactcacaccgtcatgttctgcgtaaatatccgccagtgaaatcaagcgcacactaggagttcccttcggtaggtcaatcttggaaaattcacgctttgcctgccagatttcatcaaaatcggtcattgccaacaagacaaccacctgatactgattattaattaacgataacagctgtcgtcgaaatgtcgctttgcgaattccgtgaatcgttgttgccaaaaaaattgctcgtcccatgattctcctcctgaataaaaacgaggctggaacaaaacatgtagtcttgtcctcagcctcatttgaatcttgtgtgctacacatttgattgtgggtattggtttggaatgtccgtggcgggaaagcccgtccagattggccaagtgccgggataatcagaatctcagatgttaagctttccaatcctcggtatccgttaagcctaaatcttctttgatcttggtggttgaaataccttccgttcttggaaggtatacgacttcgcaataatcctttaagaagtcaaacttccctttccagtcatcacccatcacgaagacatcaatgtctcggtcctggacgtcgtgaattttttgatcccagttggtttctggaatcacttcatcaacgtatttgatggcttcaagaatgtatttgcgatcttcgtatgacgtgtatgctttcttgcccttctcagcgttaaactcatctgatgacaagcacactgtcaggtggtcacccaacgcctttgcccgcttgagcagacgaacgtggcctttatgcagcaaatcaaacgttccatacgtaattacttttttcatagaatctcctacttaatcattactctgaatgtgaactaaaataaacacatcttaaatagtagcataatcaccgacaacgtcaatatttattaaagattattaacgtttttgtgttattccagttgataaatattatacatgtgcacaaccactactttgaccactgcgtaaagcggaacagccagaatcatccccatcagaccggcaatgtttccagcggccagcaagatgatgatgatcgtcagtggatggatttccagggattttccaatcacgtttggatagaccaggttaccgtcgatttgttgcacaatgaggaccacgatgatgttataaaccacggaccacaagccaccgtgtgaaaacgagacgatcagtgccggggcaattccgatataagggcccaggtaaggaatgatgttgcagatcccggcaatcacacctaacaataaggcgtacggcgtgccaatgatgacatagccaatggccgtgaaagtaccgacaaacaaacattcaatcatctgaccggaaatgtatttggaaatggtgtggctcattttgcccagtaaatccatggtctgttcacggtgacgttcaggcaggaatttcttaatcgttggggctaatcgatagccgtccttaagcatgtaaaacaggaccaccggcacagttacggcgataataaccgcattggcggcagcagaaataatgccccccaagccgttggttacgccattaaaaatcgtttcagcatatttattgacatttgccgacaacttattcgtcaaggtcgtaaaatcaatcttcttgagcatctgctgagagttcatgtccttaaacagtttatcgaccaacttctgaccctggctggcagcgtcaggaatctgattggccaacgtaatcaactggtttaaaattttgggaataaagacggttgcggctaacgcaaccaatcccaacaagagtaagaacaccaacgtggttgcccaggttctggtgatttggtgcttaccgaatttgatcttggtaatcaaattgacgattggattgagcatgtaaaacaaaatccccgccaacaagatgggaataaagaccgtggaaaagaagatggcaattggcgaaaagacaaaattaatcttcgtagagatccagatgatggcgaccacaatcaatatttctagtgaccaaaacatcagtggggaattttttaatcgttcgaacatcgaatgactccttaccttgattatttgaatagtcataacggatcatgataattgcttataacggtaattgtaccatacatcgtaagcgctttggagattttcattcaccgggaaaccattcttggccagcgaaaaacggccacaataaaaggctgtcggcaaaatcctcattttgcggcagcccatccctgaagagttgattatttattttgacgagccagttccaaatagcgttcgtaccaaatggcgataaattctttggaaaagggtcccttctcattttcaatccaatcaacgagaatgcggacatttcgttttaagatatgatcaatttctggaccataattccaacgcttactgaaggccaaatattcatcggcatccagtaatttgcgccggccgtctggaaagactttgacgtccaaatcataatcaatatattttaaagcttctttatccaaaacataaggtgatgctagattgcaatagtaggcaatcccatcatctcgaatcattgccaccacgttgaaccagtaatgcttatgaaaatagaccagcgccggttctcgagtgacccaatggcgaccatcgtcctcggtcaccagggtatggttgttacatccaatcaacgaattctcactcgtctttagtaccatcgtatcccgccaaacgcgatgcaggctaccatcatgcttgtagctttgaatcgcaataaactgaccttctccaggtaatttttgaagtcgtggcatgtatggtacccactttctgactaacctaaaaacatcgattgttcccaatccatttttcattatatcagagtgggcattattttcgaaattattttattcagtcagcttcgccatggcaattgtgatgtcatccatcaaaaagcctttccggaaaagtgcctgtttcactttttgattgcgttcatagggctgaagtttgcgatactggcgccaatacttttctgcgacttgatcaatgaccgcttgatcctttgttgccatgtctgaagtatcgacttgattcataatctcctcaatatcaccataagggaacccccgacgcatcaaaagctccttggtcttgttgatggccattttggcagaatcgcggcgatagcgtttcaactgtttttcggcaacttcaccgccaatttcaatgacctcttgagccggataatattggttcagcgaattttccgcctggtcggaagcaacgtgtttgtctttcaaatgccgccgaatccaatccgggccatttttgcgttcacggaccacagtgcgaacaaagctgtctgcgtatcgttggtcgtcaattaaggtttgatcagccaggatatcaatgacctggtcgatggcgtcctcatcttcagtcagctcagcaagcttttgtctgacttcgtactcggttcgcaggttgtgagcgagataattcagcgcccggctgtgaagtttggaaatgttatcggcatttttcagggtttcgattaattgatcgtccagttccattcccttgaaaacccgatatttgatgaagacttcttcactgattggaaaggcgtattgaccgtccacatagacgttgaagcggcctttacgtttctgggcttcaattttagtaattgtttttgccataagcgtcctttcttttctgcgtgattgaaattcactttgtcattttgatttggtatactgagaacaatttaagatagaggatgaaaaatatgattactgctcatgtagtttacgcaacaattaccggcaacaatgaagatattgccgacatcgtgactgaagcattggaagatgcggatgttcaagtcgaagaaaccgaaatttctcaaactgacccgtccgtttttgaaaacgtcgatatttgtgttgtctgcccttacacctatgatgagggggctttgcccgaagaaggaatggacttttacgatgatctctccgacctcgatctaaagggtaagatttttggggtcgcaggttcaggggacgttttttatgaagaattttacaacacatcggttgataaattcgaagaggcgtttgaaaagactggggctaccaaaggcgcagagagtgtcaaaattaatttggaacccgaccaaaaagatatcgaaaagttggatcagtttaccgccgaactggttgccaaagtcaatcaataaccagtcggttgaatcatcaatgggggaggctgagacaaaagtatacgcttttgcctcggcctttttttgtgatcccatattatttatcaacaacgtgcgacgacggccagcatgcttgcctagcctacatggcaatcggctgatcccggccatttaagcgtacagatcaatcattccaaaaccaggaataatcgatctgtgcttttaaattctgggatcaaaacgcctttagtcccactctctcctctttggttgtcaagattacctgaccggcctcatttatgtttcctgatcttgcgggcccgtttccaaacattttcaatggcgtcttcctgctcctgaattttgccctggcgaatttcttgaatcgtagcattgaccaccccgccaaacagcatgatgactccggagaagtccagccagaacattaagacaatgaaagttccgattgtcttataagcatcgattctctgagagaagaatttcagataaacggtgaaggcttgggccaacagcatcaagcccaaggtggcgatcaaagcgccgacccagacatagcggaatttaaccttggcagtcgggacaaaataaaacagcagacttaatagcagccaggaaacggcaattgttcctggccatttaacggtactgatcaggttcaatatccatcccgggacgttcaaaatcggcgttaaccactggaaaaacatctggccaaacgcaaaaaccatcatcaagaccaccagtgcgagaaccaacaccagcatccaaacgaaggaaatcagccgattcgagattgctgtttggtcggcagcgacgccgtacgttttattgatactgcgctgaaaggccgcaatcgcccggctggctgaccaaatggtcacaattaaaccaactgataattggctggcacccccactttgcaaggtcgaattgatgatcggttccagcatggaataaattcgatcaggaaacagcggccgcagatagacttcaacttcagtgatatgaatatgaaacaagttcaaaatactgccgacaatgaagaaaattggaaaaatcgacagcaatgtataaaacgctaacacagcggcggaatcggaaacgtctccggatgaatagcgtttaataatgatttcgataaagtttttaacggcttcgtataatcgtttcatcaggcatcgacttcccgcaattattagttgaactggtctcggatcgcttttaggattcgttcggcggcatgaccatccccgtatgggttcttggcttcagccattttctggtattctttgggatcgtcaagcaggcgctccatctctgacttaacaactttgggatcggttccaaccaaccgcaaggtcccagcctgaataccctcgggtcgttccgtagtgtctctaaggaccaacaccggtttcttaagcgacggggcttcttcctgcaccccaccggaatcggtcataataaagtaactccgagcggacatgttatggaagtccaaaacatccagcggttcaatcaaatgaacggccttgacaccgtcaaagacttcatgagccaccttttgtaccgctggacttaggtgaaccggatagaccacttcaacgtctggatggttcgccaagacttctttaatggcttcaaacgttcggcgcatcggttcaccctggttctccctgcgatgcatggttaagagaatcatcttcgagttttccttcagctcatcaaacacagaatgttggtagttttcggtcaccgtctgcttgagggcatcgatggcagtattgccggtgacaaaaatatttttatctggatgattttctttaagtaaattatccctgcttaatgaagtgggggcaaaatataagtctgccaacacatcggtcaattgccggttcatttcttcaggatacggtgagagcttgttccaagtacgcagaccggcctccacgtggccaattttaatttggtgataaaaggcgctgatactggcagagaaggtcgtggtggtatcgccatggaccaagataatatcaggctgggccttttcaataatcgggtccagttcggtaatgacccgggtggtaatgtcgctcaatgactggccctgtttcataatgtttaaatcatagtccggcgtgatatgaaatacatccagcacctgatcgagcatctctcggtgttgcgcggacacgaccgtaatgggttggaattcgtctaaatgctgctgcatcagtaggataattggggccatcttgattgcctctggccgggtgccaaagatggtcattacttttattggtttcatcaattaattctccttttatgtggttaattatatcaaaaatggcaagaaacttaacagctacttaattttgtaaaaaatatgatatggtataatctgttagatgttcatttttacatagcgaggtgggattcccacttcagccactgatttggtctgctgctccaaacggattccagcttaccaataaaaattggcaaaagcaaagtcattaacaaacgtactggaggaaatattttgaaaacgatcagtctaattgttccttgttataatgaggagccaacggttgaacttttctacaacacgacagaaaaagtattcgataaattaaacgcgtcccatgaagaacactaccaccctgactacctgttcatcaacgatggttcggcagacaaaacactggacgtgatgcggcggcttcattcacagcatcccgacgaagtccattacatttcattttcaagaaacttcggtaaagagtcggcctttgctgccggcttagccaacgcccatggcgattatgtcgctgtgatggatgtcgacctgcaggatccaccggaactgttgctgcaaatggtcgatattttggaagatcccaaacaggattatgacgtcgtcggctgtgttcagaccagccggaaacaaaatccaattcgtgcatttctttccgccagtttctacaagatcatcaacagaatgtcaaaggtccaaatgaaacaaaacgttcgtgactaccggttaatgagccgcaagtacgttgacgccatcttaaagctgcccgaatacaatcgctttagcaaggggcttttctcttgggttggtttcaaaaccaaataccttgagtacgaaggggttcctcgcgctgccggggagacttcctggtcaattttccagttatttgaatactcgatggaagcgatcgtcgatttttcggatgtgccgttaaaattagcgacctttgtcggcatcctgaccttctttttgtccattatcggtctgttctttgtcgtcattcgggccttgttctttggcggatccgtcaatggttgggcatcaatggtctcgattatcctgtttctaagtggtgttcaactgtttagtttaggaattttgggaacttatgtcggcaagatttatctggaaaccaagcatcgccctaaatttgtgattgcggagaaacgttaatatgattgatcgattgaagaagctatatgataaatacgaagaggttatcgcctatcttttttggggtgtcttgaccaccctcgttaatgtcgccattttttcgggattacatctgtttaccaacatcaactacatggtgaataatttcattgcttgggtcatcagtgtcctgttcgcctacattaccaataaagcctatgttttccactcaccttccaagtcgtttgtgagcgatttgaaagagatgggttcgttctttggcggtcgggtcgccactttggtcattgaatggattctgttatggatcggtatttctttgatgcatcaaaaccaaattttggttaaaatattcgaaaatattgttgtgattatcttgaattatttctggtcaaaatgggccgtgttcaaaaacagcaccaacagaaaccagcccaagcaaggacggtgagttaatgccaaaaatcaacagacaaacgctcagacagcaacgccaagaatttcccgaaggctattacaccaaagctgacggcttcaagctgctggcaatcgctgcggtaatgattctaattttgatcgtggttgccaaatatcttatgtaaaaacaatctgaaaaaggtcgaaacacaattaatctgtgtttcgaccttttttgaaccaattttttgtatcacagttatcgagccaactcccgttccaactgggtttgaccaatcgtcatcagccagcagaagaaccaataaaccaccgcaatcgtgatgtaaatggtcatgtaatcctgattggcaccggcaacaatctgagcgtccataaacatttcactgaccgtaatcatcgctgccagcgaagtccctttgaacagatccagcaaaatgttgcccaacgccggaatcgcaattcgaaaagcttgtgggaaaacaatcttggaaatgactttgcggtatggtaagcccagtgagtatgcagcctcccactgtccgtgatcaaccgcactaaatgatgaacggtaaacctcggacacaaaagcgctacagttaatcgtaaaagcaattaccgcagccggcaatgcatcggctcgaaagccaaagtaaatgataaacaataaaaccagcatcggcactccacgcataaaggaaataaatgcccgtgcgggatagtgcaacaatttgtggtgacttaattgggccagcgttaagaacaatcccagtattaatgacaaaataaaactgatcgcggttaatccaatcgacatcggaaagcccgctaaaattctgggaattgaacgaaacgctaatggtgcgttaaaaaaatccggaattgataaatacttaataatatccaacagcaccgccccttacttaatcgtaaaggtctttgaaatgtggacatggggctgtttagtaacgtcagcgtgataatacttctctgacagcttcttcaaagtaccgtctttcttgagctctttgagggctttgttgacctgcttttgcagcttggtattgcccttcttcattaagataccgacacctttgccatcttcattggttctgaagtacatgtttggcatgatcttcaaagtgttgttgggaacggcagccaatgctaatttctgcagatagtaatcattcataatcagatcagtcttgccgctttcaacgtctcgcagatacacatcgtttgaaacgttgttgtagttgacggtcttggcgcctaactgcttggcaagtcgttgatatcctgtcccggcctcaccggcagcttttttacctttaatgtcggcccaggaatgaatgcctgaatcccccttctttcgaacaataatactgttaaatgagtgcttgtaaggcgtcgaaatagcaaactcttttgctcgttgtggtgatacggcaaaatcattagccgccatatcagccttacccgtcttcacagccgtttcctgaccatcaacgttcatttctttgaaatcaacttttctccccaactttttggcaactgcacgaacaacttcgacgtcaaagccggttagcttgttagtcttttgatcatgaaatgatgttggataaagcgtccccgatgtggcaactgtcaatggacccttatctgctgattttttctgaccgcagccagtaatcaccaagcccagaaccgcaaatacgcctaacaacatcaaccaacggaacttaattctgcgcataaattgtcaacctcctaaagtttttggatcattatcattataggcatgtgaaaccgatttcacaatagctgataaattaattgttaaatattataaatcccctcaatttttgataaataattgttggtcgccaaagtgatcgtcaatttagcgttggctccaaatgctttaaagtcgcatattttagccaatcagtatttagtcatattagaattgcccttgaacgacacttagattggtatataataaaaacatttgaagtgacaaacatcacttgttaataaatttgaatggcggcttttgatggacatcagaaaagaggctgttcaggcaaacgcaaaattatcaacgcttgagaaagtcagttattctttcaccgatatggctggaaacttgttgtacgtcagcatgtccagttatattctttatttttatacggatgtttttgacattccggtttcagcagcaggcatgattattttgattgcttgtattgttgatgcggtcagtgcgattttttggggatcaatcgttgaccacacacatactaaatgggggcagagcagaccatactttttgtggcttgccgtcccttttgcgttaagcacctttttggcatttaccgctcctaatatttcaggtgtccccaagctcttatatgccgggattacttatgtattggcggctggagtgatctacaccggcatccaaacgacgatttccgcaatcctgccgaatttaacccttgatcccaccgaacggattggcgccaactcttaccggatggtcggcagtctgattgggtcatttgtaaccagtacctttaccctgccgctggtagcgttctttggcaatgggaatgacaaacacggattcatgatgacgattgccatctttggcgtcgcagcaattctcttgctgatcacggcatttaagaacatgcgtgagcgggtcccggtcagccaaaaatcactgccgttcaagcaaagtttaaaggcaactgtcggcaacgttccttggtacctcttagtgatttcttttgccaccttttggatcgcccaggctgatcgcaatagtttctcgacctactatgccaaatacaacctgggtaatactgaacttgccgcggtattcaatggcctacaagttctggggatcatctcaagcattgcaattccgtttattgttaagattaccaacaaaacagcaactatgttaatcggcttgggaattggtgctgttggccagacaatgatggcactggttggcggcaacttcatcttggtgattgtttcttggttgatcggcgttttgggatcggctctggcaatgtcaatgccatttgccatgttggccgacacggtcgactttggcgagtggaagacaggcgtgcgggccccggtttcttaaccgccgtggggagcgcattctgtatccaactgggatcaggctttggcagttttattccgtccaaaatcttggatatgactggctttatcgccaacaagacccagacaccagcagcttcaggtgcgattaacttttattttatctggctgccggttatcatctacgcgattgtcgccggcattatggtctttcatctcaagtatgagaagatggagccaaaaatcaaagccgatcttgtcgcgcgtgctgaacaacgtgacgcttaatcaaattgaattgatccgataaaataagaacgtcaatgatgaacaatatccattcatcattgacgttcttatttttacttcgtatttcgtaaaagcgatcgaatacgccatgaccccacccggactcgaaccgggatcaaccgcttaggaggcgggtgccctatccagttgtgctatggggccaaaacaactgcactacaattttctcatttatctcagaggctgtaaagagaaattatccctccgtgcgcttatggtgcatgcccttgcgtttggagtgtttgtgcttctttttgccgtgcggtttggcgggcattggctttcggccagtttttttagcctcactgctccgcttgacatcttgagacgatgcagcctttgaagttttgggttcatcatccaaattaaccggctgcttaggtcgagtatcagacaactgattaccatcgaagtagatgttgctcaattcatatccgtaaggcttaaccaacttctttaaatctctcaaatcgtggtcgtcacccatattgatcaccatgccgtcttgatgcatgcggccagtccggccaacccggtgaacataagttttcggatcagacggcaaatcaaaattgaccacgacgggcagcttttcaatatccatcccccgagcagcaacatcggtggtcaataacaagcgaattttgccatcgcgaaaatcgcgaagcgccttttgtctggcagtttgccgctgttcactggtcagctgtgcagcctctttaatgtgtcgatgagacaggaaaccagcgactttttgcagggtatccaattggtcaaaaaacactaatgccttgaagtccttcatgtgaaggaaccgcaataacatctgagcctttttccgattggaaacttccagcaaggtatgtttgacttccccgcgggtatcgtcaatgtcagagacatcaaaggtctgaatatcttgaccaaaccagcgattcacatgtgccaataagtcgttttgggttgcggagaaaaagcccagcgtcactgagtcgtcagccaaatccaccaatgatcggatggaagcaagcgtatcttcacttaataagttgtcggcttcgtctatcacgatcgccttcagtgaatccaatttaagtttgcctaaatcgattaagttcacgattcgaccggtcgttccgacaatcacgtttgggtgctgttttaatttatcaacttgacgattgatattggcaccaccgataatcccttgaactgataagccgattagcttaccccattccaataaaactttttgggtctgcatagccaattcggcagatggttcaatgactaataatgacagcccgtcttcaggttgaatattttccaacaacggcagggcaaaggcaactgtcttccccgatccggttggtgccagccccaggacactttgaccgtccttgagtggttgataaaccgcttgttgaatcgcagtcggctgattgtagcctaattctttggcatgttgcttaaattcttctatcaatatggttctccattttctaatcgattactttttctcgcccacaaatgagatgtgagcatcctgtctaagattataaattaacttattaacgtacacgctgagttggcgccagtagtcataatcatgtttgttttgcgggttctttggatcgttaatcactctggcgaaatcttcaacctctggcagcatcggattctcatcaatagtgttgccaatgacctgcttgttgcgatcgtcatcaatgtaaatgacggcgttaatttctccggcatcatcgatttcgattaagtctttgaggccgtaaatctccgatgtcatatgtgagttggtgatctttgagaagtttaaagtcacattatactccggatactgcaaaattgctgttccttttccgtcaaccccggtgcgaatcagctgtgggtaataagcagcctcttccggcattccgaacaaggcaacggcatcatagacggtatagacgcccaaatcctggagagcaccgccggcatatttgagtgagaagacgttgggttcttcaccctccaacaccagatcatacctggaagagtattttgaatacgtgaattcagcgccttgaaccgttttaagttgaccgagctttttttcgatcgcatgaaaattttcggtgtgaatattgcgggcggcttcaaaatagagcacttgtggattctcgtccaacaaagcttgaatcttcgccatttgtttttgagtactaaaggccggcttttcaacaatgacatttttgccgtgttgaatggccatttgggcctgttcaaaatggaggctattgggtgaggcaatgtagaccgtctcaaactgccccttggtaaagaacgcattcagatccgtaaaggtttcttgggcgccgtttttggccgcaaaagttttggccgtttggtcgtgtcgtgaatagacactggttaagtcgaatttgcgtgatagtttaattgcgtcaataaattgctgggtaatccagttggttccaataattcctaatttaatcaatttgataaccgcccttctttaattaaattgtaacaaggttttaacccaatgaaaacgaaatcagacactctctgttatatttatcgactatactgggtttctactatgactagggggatgattttttgcgcaaaagaagtttttttatttttatggtgtcgtttttaattagtctgttccataccaaacggacaccaaaacaccgtccagatcctgcagacccaatgtttttcgttggaacctggcagtttaaggaccaccgggagcgtgtccatcgactggaaatcgacccggatttaaaattgctcattgacggaaaagatatgtcggccaaggtttcattattaaccagatatgaattgtcgtacgttgacaaatttggttataaattggaaattcgggggaatgaagcccggccaatcaaattctacgatgaatctgaaaactatacctatgatttacaatcggccaatgaaattgaacagtcaaattgagtgaggacttactgtggtaaggcctttttgttttggcctgttccatacgctttaattgatgtattcccgccactgtctgcgattaccgttaaagaccgacatcggcagaaagatcagttgcgagtcaagcttaaagccggccttatcgtctgcctgaataaatgttgcatcggcattgggccggccgatcttaccgtcagtcaaccagaattgggtcttagcattcgcctttaactgcaggctcttgatgatttgttgggtcgccgaaatgaccaccggccgtttatagtactgtcttaacaagtgcgaaagctgccggacttcttttctggccgcctgccaatgaattgttgactgatcaaacgttccgtaatactgaatttgaatacagatcggtaaactaccggtattgtacttgacttgccggacaaagtttttgaattgggcagttggtgaactggtaaaactaaaataatggtagaccccaatcggcaactgggaaccctggctgcgttcgaaattactctgaaagctgtcatcggtgaaggcagctccctgagtggcctttagatagacgaaactgatgcctttacttttcaagctttcaaagtcgatatagccattactttgatcaatggtcaccccatgaattgggtattttttcagctgctgattttcgtgccagcgcaacagcaaaaaggtcgaaaagccaatcaagattaacaaaaaaatgccgaaaactaccctgcgtgtgcgtttcctgcgctggtaagtttcagcatatattggttgaatgtctcttcgcttcatataaaggtcatctcagttacccgaaaaatccagttaaattaagtccgggtactttcaataatattttgaacgttgcgaatcgcgtcttctgtcgccggacccatccgaaccgttgccatcataaataacgtatcgacaatagccagttgggcaagcagtgaatacatcccttcagaacggtaattggattcatcactagacgaaataaatgtaatatcactatgcagtgcgagcggtgagtccggatagctggtaatcccgataaccggcacctttcgcttctttaaggtttccgcaacttttaaagtttggcgatttttgcccgagtgggaaaccacgattgcgcaatcttcttcacccaattttacagcttccatcaactgtacgtcaaagtctggataatagaagcagtcaatcgacgtccgcaagaacttatgataaccgtccagggccgcaactgacgagccgccaaggccaaataagcccagacgacgacaatgaataattcgtaggactgcccgagcaaattcatcttcatcaattcctgcccgggtatcttgaattgcccgctgactgctgttaaaaatcttgtcggcaatcgttcctaaagaatcgttggcatcgatatctttaaaaatcggcaggttctggggccgcaactgcgtgtaggccagcgccaaagtaaactcacggaaattgccatagcccagtgtcttcactaaccgggaaaccgaagcagttgaggtttcagtcacttctgccaaatcttcaatattggcttctgaggccgcttgaggattctccatcacatattttgcaatttttttattggttctgcttaattcatcaaacgattgttttaataattgaactggcgagctcataatgatcacctttcatggattgtaagtgtcttattttcatcaatgtaaatattttacaacaaaattcttgcattgtgaaattgtttttcatataattgtgtttgcgtttccattaccaggaaattcaatggtcgaaatatttgaagtctcccggtgataatgatatttttagtgagaagcggtaccgagccaattcttcagcactcgacattggtttaacgatgcagctatattttttgccattatttgaaagcgcttcggccgttgactcaactaatacagaagggaagttatttacatggattatacgctaggtgttgatattggaacaaccagtgttaaaaccgtgctctacgatgttaagggtaaggtgcatggatattccaacaatggatatcccctataccaggacacccctgatatggccgaggaagaccctgaagaaatcttttcagcgatgtctgacggcattaccgaattggttcgaaaggccaatatgaaaccaggagagctgaagggcgttgcattttcctgtgcaatgcatagtttaattcttctggatgagaatcacaaaccactcacccgggcaattacctggggtgacaaccgggcggtcaattatgctgataagttgaaggccagccctgagggaatggaaatctataagcataccggaacgcccattcacccaatgaccccactcaccaaactgatttggctgcgcaatgatcatgccgatctattcaagcaagcccgctggttcgttggcattaaggaatatattctttacaaattattcggtgtcttaaaagaagattactcaatcgccaatgccaccggaatgtttaacatctacaatatggactgggatgaacaagccctgaaacttgccggggttacacgggatcaattgcctgatttagttgacaccacttatcaattaaaagggatgcgtgaagagtacgctaaagtgctgggaattgacatcaataccccatttatcatcggtgcttcagatggtccactggccaacttgggggttaatgcgattcaacccggggttgtcgctgtcaccattggaacttccggtgccgttcgagttgtcactgataaaccgcataccgatccaaaggcccgggtattttgctactacctcgccaagaacatgtgggtcgttggcggccctgtcaataatggtggcgtcgtcttccgctgggttcgtgatcaactctgtgccccggaaaaagtcactgctgaacaaatgcacatcgatccatacgacctcttgacagaaattgctgccaaagtgccggctggatccgatggcttgctgttcttcccattcctgggcggtgaacgtgccccaatctgggacgctaatgcccgtggctcattcttcggccttaaccggacccacacgcgtgcccacatgattcgggccgttttggaaggtatcgtctacaacctttacacggttgccttggcccttgaagaagtcgttggtcaaccaaccagcatccaagccagtggtggttttgcccgctctgcgctttggcgtcaaatgctgaccgatattttcgaacaggacgttgcaattcctgaaagtttcgaaagtaccgctttgggggcagccactttgggaatgtacagtttgggcctgattgacagcctttccgacgtttccaattttgtcggcaccacggttgtccatcacccagatccaaagaacttccaggcgtaccgggaattgattccaatctatattcgcctaagtcgttcacttcaacccgaatacaagaatatcgccgagtatcagcgtcgtcacgaacacgaagatgaagacgccgagaagtctgaatagcacctgtccgtttttatttgaaaggggaaaactatgatattaaagctgctagccttgctgatcggaattattttcctgttggttctgattatcaagttcaaaattaataccttcgtttcgttggtattaaccgctgtcgttactgcgatcatgctgcagatgccactaggtacgatcgctgattccgtctcaaatggtattggaagtcaactgggcgaattgtccatggtcttcggctttggtgccatgttagggcgattggtttctgattccggtggtgcttatatgatcgccgaaacgctgatcaaacgatttggtaagaaacgcctccagatcgccgttatgttggcttcatttattttaggaattgcgttgttcttcgaagttggaatggttttactggttccaatcgtcttcgcaattgccgttgaagccggtgtgccaattctttatttaggaattccaatggccgctgccttgtcagttacccacggatttttgccaccccatccagcaccagttgccattgcgcaggtcttgggtgccaacgatggtaaggttctcctgtttggatttgtcattgcaattattgccgcttatatcgccggaccattgttctcaaagatggctcgtaaatttgcacccgctgcattcgagcgaaaaggaaacctttcttcgatcggtgaagttaaacaatttacccctgaagaatcaccatcgtttggactgtcagtattaactgccctgttcccagttctgctgttggcgattgccacaatttataaaatgaccgtcaatggtggagttgatccaaagaacccttctgtgattgattcaatcattgaattcattggatctccaagtatcgcaatgttgatttcattattcttcgcaatgtataccatgggctggggtcgtaaacgaaccactgctcaaatcatggaatcccttgaaaatgcggttaaatcaatcgccatgctgctattagttattggtggtggtggtgccttcaaacaagttctgatcgacggtggtgttggtaaagccgttgctcaactgttcattggttcaccaatttcaccattaatccttggctggttggttgccgttgttctccgaattgctttgggttctgcaaccgttgcttcattgacagctgcaggaatcgttgccccattgatggcccaagctggggttgacccagcattgatggttctggccattggtgccggctcattggccgcatcacatgttaacgatgccggcttctggatgttcagagaatatttcgatttaacaattaagcaaactcttcagacttggaccgtgttggaatcaatcatttctgtcgttggtatcatcatggttatgggactgaacttgattttccattaatgagagagtgtgaactcaggcgcttagcttttgagcattagtttaatacaggccgttaacgctggttttgcgttgacggcctgtattggactaagcggaaaaagctgcctgagagaacacattttaatcatagtgtgaaccaagacggttagcttctgagcatttatttaacaagcggtttgatgcggttttagcatcagaccgcttgttggataaagcggaggaagctgtcttggggaacacattttaatcagagtgtgagctcaggcggttagcttttgagcattagtttaatacaggccgttaacgctggttttgcgttgacggcctgtattggactaagcggaaaaagctgcctgagagaacacattttaaccagagtgtgcccccaggcgcccagcttttaagcaccacttcaatcatacaaactccaaaaagactcgagcaaaccaatcatgtttgctcgagtcttttgtatccagtcaattaaacctgcctagctgctcgactcagcactttcattcggacagccaccaagtatgcaacaactgccttcagcgtgtcgccagggataaataacaggcctgaagtcaatgcaccgatcagtgagattggcgtcacccaccacagccagagggcacccatcaggttaacgatcaaaacaccgctgatccaaatgacaattagttgaccccatgaatggctcataaacggccgcgagcggcgataacccatcatgagaggtgttatgagccaaccgaacaaatagcccgctgtggggccgataaagactgctgggccggcttgaccgccggagaggaccgggaaacctaaaaatgccagcagtaagaataccccaactgcgatcgtgccgttctttgaccccaaaaagaggcctgccaacataatccctaagttctgcatcacaatcggcacaggaatgatccctaaaggaattggtggaatcatccccaatacgataatggctgcgatcatcaaggccgtttgcgtcaattgtctaattttcatatcattttcctttcaaaaaacggttaaccgacttctatacgccgcttaaccgtcattggatattaaattagcctgaataaccatttccaggcagataaactttcgtcacttcaccgctcgaaacggtaatgggttctccggaatcctgcttgaccaccaaggcaccatcaccggtaaaacgatcggccagcccagtgatggttcgatttcccatcacaatttggactcgtttcccaagggtttctgataacttggcgtactcctggaggaaattaccactggtgtaagtttgatacatataaaaaaagttgtcgatgagactggcagcaatccgattcttgtcaattgctgtgttggtcacaattgccccggctttatgggcaatttgatcaggaaaatcagtggaatcaatattcaacccaattccgaccaccacattttcatgaagaccgtcttcgagactggaaatcgtttcggtcaaaataccaccgcattttttatcatggaccaaaatgtcattgacccatttgacccgaaagtcctcatcgggaaaaaactgttgcagggttcggactacgcaaaccgcggttccggtggttatcaacccagagtgaatggttcggcgattctgtaaaggaatcaaaatgctcaaatagattccacccttcgccggcgaatagaaatgtcgccccagtcggccatgcccctgagtttgcgtatcagccacaaacacctgtggaatggtaaagtcctgactgctgccaaactgcttggcgtaatcgttcgttgaggaaatgctggcaaacgcatggatcgccaccgggaaagtggttgtccgataatggtcgatcacagcatcatcaaaaaattgggatttttgataacaataacccagccctttgcgtgtggtaatcacatgaccgcagtgcgataatttttgaatattgttgtagacggccggccgactaatttgcagtttcttagccagttcattgccggaaacatagcggccagccgccgttagcaatgcatctaaaatttgtctttgatgattgaccattggccatcccccacttacaatcgtcgttaaattaaatggacacctttatcaacgtagaccacgtcaccggtcataccggttgaaaggtcactcatcaaaaaggcggcgacgttaccaatttcactggtggtgacgctcttttgatcaactgtccgtgactcggattccttcaacaattcaccatgatgtttaatcccagtaactgctaaggttttaaccgcgccggcagaaattgcgttgacacgaatgccattttcgccgagatcagatgccaggtaacgcacgttggcttccaaagcggccttggcaacacccatcatgttgtaatttggaattgcccgggtggagccaaagtaggtcaaagttaaaatgctggctggattattcaagaccggttgggcataacgcgccacggcaatcagtgaataagcactgatgttttgtgccaaatcataaccgtccttggtcgtgttgaccagtccggaagtcaaagtatccttgtcagcataggcaatggcgtgaatgaccccatcaattttgccatactgattgccgatagtttcaaaagcctgcttaacgtttgcgtcatcggcaacatcacactcgattaaatccaagtcgtccggcacaaagcgttccagactttttttaatgcggtcattttgataggtcaaaataaccttggcgccttgatccaaaatcgcttgggtacagccccaggcgatactgcgtttatttgcaacccccatgatgacgattgtctttccatctaaaaagccactcatatttgagcctccaaatcttatcttcaattaaaaattccggtaacgtttatttcgacggtccaccaaatcatcaattggtaacttggccaattgagaaaattcctgatccaagaagtcacgtaacgcactcaaatcttccccgggttgatactcatgaataattttatcaataatgccatctgctaataatgcttctggagttaatttgagttcttctgcggcttccttgaccttggatgaatctttccacatgatgctggcgtatccttccggtgagagcaccgaataaatgctgtcttcaaacatgaagacccgatcgccgcaggacagtgccaaagcaccaccagaaccgccttcaccaacaataatggtgatatacgggacccttaactgcatcccctgaataatattttgtgccaccgcggacccttgaccatgatactcggattcaacatctggccaagcaccgggggtattcaccagcgctaaaattggccgatgaaatttctctgcctgcttcatcaaccgcaacgccttgcgataaccttgaggcgttggactgccaaaatgtctggcaatattctgatcggtatctgatcccttttgaatcccgactactgtgattggtttatcattcaacaagccaataccgccaatgattgccgggtcatcagcttccagtcgatcgccatgctgttcaaaaaagtcactggttaaatgattgatcaactcggcagtcgtgattttatcaggacggcgagctgctttcacccgctgatatgctgttttatctgccatagacgttctcctttgtgtgcagagaaattaagcgactcaaagttgctttcatttgtttacgcggcacaatcgcatcgataaagccatgagccatcaccgtttcagcactctgaaagtctttgggaggcttttgcataattgtctgttcgatcactcgccggccggcaaatccgaccaacgcgtgaggctctgctaaaatgacatcaccatccatggcaaaactggcggtgaccccgccagtcgtgggatcgcataagacaacgacataaaacaggccggcccggctgtgttccgcaaccgcccccgatactttggccatctgcatcagcgaatgaattccctcttgcatccgggcaccgccggaagcggtaaacatgatcaccggcaattttttccgggtcgcttcttcgaacaatcgcgtaatcttctcaccggttgcacttcccagactgcccatgacaaagaatggatccatgatgcccacaccgacttgctgcttatcaagggtgccaatacccgtgaggacactttcgttgattccggtgacttttttagcctttttcactttggccaaatacttttcatcggtgtactggtccggaaccgtcattgatttgtcaatttcatcaaatgaatcaaaggtaattttggcccgtcgtttggccgtgattcgaaaaccatagccacaattgggacaggttttcgtgctgccagcccttaatgaaaaaaaggttgcgtgacaaattgggcattcccgcagcacatgatcgggaatggcatccatccgctttaccagttcttcatggcttggcatattaaaccgactgcgtagcatggaatccctccttatcgctcaacacttcattttgaatgtaactggtcgaataaatcccctgatgaaatttgtcggtgccaatcaagtaatccaaaaagctttgattggtccgaatgccgtcaatttccagttcccctaaaattcggtgcatctttgagataacggtatcgcgatcgttcaaatgaacaatcactttggcaatcattgaatcatagaacggcgaaataaagctgccattggtgacacctgaatcgattctgacgccgagtgaaccggcggggaaaaataaatgattaatctgaccgggttgcggggcaaaattgttagtcggatcttccgcattcaaccggcattccaaggcgtgccccttcacggcagcatcggcttgggtaaacggcagttcttctccggcagccaccgccaattgccctttgaccaattcaattccggtcacttcttcggtaattgtgtgctcaacttgaagtcgggtgttcatttccatgaaatagaagtgatgctcatcgtccattagaaactcaaaggttccggtattggtatatcccagcttaagcgtggcgttggcgacaatctcacccaaatgccgccgctcttcagctgaaatcaaaacacagggactttcttcaatcaccttttgatgattccgctgcagtgaacagtcacgctccggcagataaacgacgtgaccaaaattatcggcgataacttgcatttccacatgtttggcctgacgaatcaatttttcaacatagatatcttcgtcgtcgtatgaaattcgggcttcctgctgggtctgctcaaaagcacttttgagttcttcaggtcgatcaacttcacgaatccctttaccgccgccaccggctgctgacttcaacaacaccggaaagccgatttggtcagcgacttgttcggcttgggcaacggtattgactaccccgtcacttccgggaatcacagggaccccggcttttttcatcgcttctcgagcgttggccttgtcgcccatcagagcaatcaactcatggcttggaccaataaatttaatgtggcaggtttcgcataattctgcgaactcggcattttcggataagaatccgtagccagggtgaattgcttcacatccggtcaaattggcggcactaataatctgggccatgttcaaataagattcactgggctgcggcccgccgatacagatggcttcgtctgccaaatggacaaacaaggcgtctttgtcggcactggaatacacggcaacagcggtaatccccatatcgtgcaaagcgcgaataatttgaacggcgatctccccacgattagccactaatacttttttaaacatgcgctcacctctattactcaactgcaaaaattaaatctgcttcacaaatctgctgtccttctcgatgaatggtgccgtggccaaggccgatattgtgctttaacttctttaattccacggtaaaggtcaatttgtcaccagggcggaaatcatcttggaagactgcattcttgatgccgccaaaaaaggcgtttttgccttgatattccggcattgacagaattgcggctaccccggtctgggccatcgattcgatcataatcggccgtgggaccacgaggttattggcttgtttgttggcaaaaaaccattcattaattgaaattaatttaacagccgcggcactctcccctggcttgacatcaataaacttgtcaatcatttggaaggggtagcgctgtggaatcacatcttgaacatctggtttcatctcattaccccttcgttacttgaaaaattggttgatcgtattcgaccatgctgccatcttcaaccaaaatgttggagatcgtcccggtcacatcacttttgacttcgttgatcattttcatcgcttcaatgacacaaaccacatcgcctttttcaacgtggtcaccctgcttcttgaaagccggcttgtcaggacttggggcaaaatacacaacgccaaccaacggtgccttgatttcggcaacgttttgggcgaccggtgtttctggctgctctaccgtggttggttgactattttgtccatggcctaaaccatttgtgctggcagatgccgcttgcgcagaatcttccacgacggcgtggtcatcgccctcccgtttgctgaacttaagcttgaagtcatcttgagccaattcaaagttcttcagtgacgaacggtcaaatttatctaataaacgttcaatttctttctcatccattacctaatcacaccctttaaatgcaattacggcgttgtggccgccaaaaccaaacgagttgctgatggcgtagttgacttcggcatttttattgctgtcgtcaaccagctccacgtcacattcttcatcctgattaaccacaccgacgttgacaggcatttggttatgcaaaatggcaccaattgttgcaacggcttcaatggcaccggcagcccctaatgcatggccggtcattcctttagtgctgctgaccttgacatgatcattattggcaaagacttcgttaatcgccttggcctccgcgctatcattggcgtgagtactggttccatgggcattgatgtaatcaacctgggtttcatcaatcccggcttctttaacagcctgttgcatggcgcgtttggcacccttaccttctgggtccggcgcagtcatatgataagcatcgctggttgtcccatagccgacaacttcggccaagatcttggcaccacgggcttttgcatgatcgtaatcttcaagaattaaggttgctgacccctcacccatgacaaacccattacggtctttatcaaatggaattgaggcctttttcggatcggtttccttggaaagagcggtcaaagccgcaaacccggcaatcccgatttcgttgacggaagcttctgtcccgccggcaatcatgacttgggccttgccctgcttgatgtattcaaaagcgtttccaatcgcgttagtccctgaagaacaggcagttacgattgcttgactggtatttttggcattaaaggcaattgaaatgttaccagccgccatgttaatgatggagtcaggcacgaataatggtgacacccgtttgggactcttatcgtgcatcttaatgacctgttgttcaattgttgtcaagccaccgatcccggaaccataaatgacacccagttcttcggggtcaacgccaccgtcaatcaacccagcattttccatggcttcagtggcactgtacaacgcatatgtacagaagaggtcatttcgtttggcaaacttcttatcaacccgttttaaaggatcaaaatctttaacttcaccggcaaccgtaatgccagtgggctctgaatcaaatttggtaattggggcgataccaaccttggatgcaaacaggttttcaagaaagctgtcaacatcgttgccgattggcgtcacagcgcccaaacctgtaacaacgactctactcatttaattactcctttaacaatctaaattgtcaacccgccatcaaccgtgatgacttggccagtaatgtattggttacccaccaaaaaggcaaccgcatcggcaatttctgtcggttcagcgaagcgcttcagtggaatttgatcagtgaattcgctttgtctgcgttcactcattttttcagtcatgtccgtcttgaccattcctggcgcaacggcattggcacgaatatttcgcaatgcgccttcacgggcagccgtcttggttaacccaaccaagccggctttacttgcggaatagttggcctggccaaggttgccgtggaggccggaaatactggaaatgttgacaatcgagccttttctggccttttgcattaatttcatcgcaaacttggtcatgttaaaagcaccgactaaattggtctccaagaccgcctgaaaatcggctaatttcatccgactgagcaatttgtctttggtgatcccggcattattgaccaaaacatcaatttggccgtatttctcaaccaccgaattgatcatttgctcagcatctgcttcactggcaacgtcgccaactaagacatcgaatgaatacccggcagcggctaactgctgactgtcttcgtcgcttaattcatgatgggcattgataaccaccgtcatcccatcgtcagccaaccgtttggcaattgccaaaccaattcctttggcagccccggtcactaacgcaacttgttttgtttccgtcattatttcaccagctttttgtttgatcgaacttgatttaaggtttccacactatcgacatggaatttgtcagcgttacaaatgagcggcttggcaaatttcatcaaggtatcaccagggccaatttcaattaaaacattggcatccaggttcaacaattccttgaggcattcgttaaaatgcgttgggttaacgagttgattaaccagcgtttgcttgacgttcagccgcgtaaacggcttgataatcgtattgctgaacaccggaaaatcgggatcttgaaaattgaccgtctgcagtcgctttgacagctcgtcgctggcttcctgcataaatggtgtatgggaagccacggtcattttcaaaggaaccacccgcttgatgccgtgctcatggagatactcggtcgcagcgtttaaaccggctgccgatccaccgatcacaatttgggtatccgtgttgtaattggccggatagaccggtccgacttttgagccgacccggcaggcctcatccacaagattggcattagcttttaaaacagccgccattttacccggataatgctgtccagcctgatccatatagtgattgcggtcgccgaccagcggcagaccgtcttcaaagctcagactgtcagcagcgatcaggccgctgtattcgcccaaactcaatccggtggcgccgactggctgccctaaatcatgtgccagaattcgataaattcctgtactcaggatgacaattgaaacttgtgtattggcgggatcatcaaaaatctttgaatcactcatgtcttttccaagtatctgagaagcttcttcaattgtttgacggtaaatcggctcctgctggtagagatcctgtcccatcccggcaaattgtttaccctgaccgctaaataaatatcctagtttcaaattatctacctgcctactttctgactacttggtttgttgttttaaaacgtaatcaaccaactcgccaacggtttccataccttcatcggtgtcaatttcaatatcataagtatcttcaatcttgtcgacaacttcaaagatgtccaagctgtccaaatcaaggtcattcttaaagttggtatcttccttaaccttgtctgcgtcaacgtccaattggtccacgataatatcttttaccttgttaaatacttcttctttagtcattttaatttcctccaaattttatgttattccaatttttatttttagtacttgataatcattgtgccaacagttaatccgccgccaaatccggatagggcgatgacatccccccttttaatgcgttgtttggcaaccagctcagcaagtaaaatcggttcgctggccgctgatgtgttgccatattcattgatattgacgggaaattgattcattgaagcgcccaaagtatcggcaatcttttcgatgatccgttcgtttgcctgatgtaagacgaagcagtcgatgtcatcaacggtcaggtttgctttctcaagggcacggttaattgattcgggaacattcttaaccgcgaaaccataaacgcgatggccattcattttgaaaaatggcgagtagctggttttcggtgcagcaaatggtgacttaacgccaacctgcccagccgttaaatgcttacccaacttacccagcgtcttcaagtcttcagcgataaacgaaccggaatcaccagattggttggtcatcaataccccagcagcgccatcgccaaacaagacggacgtcgaacgatcatgccaatccaaaagcttacttaatgtctcggccccaattaaaatagcgtgcatcggccggtcagctttcaacatctgacgaacgaccttcaagccgtagacaaaccctgagcaggccgcgtcgatatcaaaggcaatcgcctgatcagcacccaggttgccttgaaccatggcactgactgacggcgtcaaataatccggtgacatggtagcgacgacgattagatcaatctcagtgggtttgaggccgctttttgccaacagctttgtcgcaaccgcggtcgccagtgaactggtcgtctcttcgacggcaacgtgacgccgcttgattccggttcgttgagtaatccacgcatcagaagtatccatcatcgatgaaagctcatcgttatcaaccacgcgctgtggaactgaactggcagtctcaatgattttgaaatcttcaaaggtcattttgcagatacctcatcaataaagtcttccaggttaaccatcgcctgcttgatcaaccgaatgtcgtcatcgtcaaagcccctcaagaaccgtttgaccaacaatttatgaaacgcgtcatgggcccgatacaacaatcgccccttactggtcaatcccagattgataatccggtgatcttcctggttggcgattcgcatcacataccctttacgttccaaattattcaaattggcagtcaaagttcctttgctcaatttcaaaatgtgggccacttccgaggtcgtctttcgatcatgcaggccaatggtatgaaccaagtgaacttccttcgcagtaatgtctttgaaccgactttttcgaatttcgctctcctcaatccgcatgatgctgtcgtagacgttgatgagcgactcattgataaagtcggtatctttttttatttcatcactttgcgaattcatttcttagctcccctagactgataattaaattttcttctttggatcagggacaataaaggttaattctgcagagcaggcgactttgtcgtcaaccttggcttcacacttaactttgcccatgttctcacgctgcttttccatggtaacgtgaagttttaagacatcccctgggcgaacaacttttctaaacttggcattgtcaattgcgccaagataagctgttttgcctttgtacttttcagttttcaaaatcaagattgaggccgcttgagccaatgattcaataatcaagacaccaggcatcacgggatttccggggaaatggccctggaaaaattcctcgttgatcgtgacgttcttggtaaccacaattgactcaccggggtttaattcatcaactttatccataaacaaaattgggtatcggttgggaattaaatccataatttcagatgcatctaatacactcattgatttcttcctttcacttacagggtggtcaatgccaattaaaatttagttcgactatcaaactattagctaaaactaaacgcacaaaattgacatttaccgaggttcttttcggaacacacaacataataacctaatttagtttgaatatcaaactaaatttcaataccacgtgttgcgtttctgaagtttaccacaaaaggccttctgtgactagtcgtccggaaatggcagacgtctttcttttgaacttgcgggttggcctaacaaaaaggccgagacataactcattatcggttatatctcggcttcgctggtgtgcgacttttgtgaattccactgttatctagctaaaacgtgtgaaagaggacagccatcgaaatttaagccgcttcagtcgaaaacctgactcggtttcctggtgtcttacttttatttggattaaacctgtgaaagaggacagcaatcgaaatttaagccgctccagccgaaaacctaactcggtttcctggtgtcttacttttatttggtttaaacgtgtgaaagaggacagcaactaaattttaagccgctccagccgaaaacctgactcggtttcctggtgttttacttttatttggattaaacctgtgaaagaggacagcaatcgaaatttaagccgctccagccgaaaacctaactcggtttccgtctggagcggcttaaatttcgattgctaaacgtcctctttcacactctgtttttattcaactgtttcataaaccaacgttggtttgttggctgactcagagatttcgatattgtcatacaaccgcttcttaatgtcatcgacatcgtcacgattgctatatattgtcagcagtgactccccggttttgacctggtcaccaatcttcttatgcagcataatgccaaccgcatagtccagctggtcatcggccttctgccggccaccgcctaagagcatgctggcaatcccaatttcatcggccacaatcttggaaacgacgccgctgcttggtgcgggcaggtcaatcttgaattgagcttgcggtaagacatgttccgggtcgtctatgaccgccgggtcgccgccttgatccgcgatcattgcgcggaatcgctccaacgcctgaccgttatggatcactgtggcacatttttgctggccttcttcagtcgtttccgcttggccacccataactgccatgtagccgccaatcacgacgatcaatttttccaaatctgccggcccattgccctttagcaaatcaattgattcttggatttccagcgcgttaccaactgcatcacccagcggctgattcatgtcggtaatcagcgccatacactgcatgccgacgcctttgccaatctcaaccaaggctttagccagcgctcttgaatcgtccagggtcttcatgaaagctcccgcaccggttttcacatcaatgaccagcgcatctgcccccgaagcaatcttcttactcataattgaactggcaatcaatggaatagagtcgaccgtatcggtgacatcccgcaaggcataaatctttttgtctgccggggcaatgttcccagttgcgccaataattgccaattggtcttttttaagttgggcaataaagtcatcctcgctaatttcaacctgataccccgggattgcttccagcttgtccaatgttccgccggtatgtccaagcccccggccggaaatcatcggtaccggaattccaagagcggctaccacggctgccaatggaatactggtcttgtcgccaaccccacctgtggaatgcttatcgactttcacgccgggaatttggctcaagtccaagtggtcaccggatttcatcatcgtcatggttaatttggcttgttcctcgctggtcatcccttggaaaaagatcgccatcaataacgcactaatttgataatccggaatgtcgcccgaaaccaccccgtcgacaaaaaattgaatctgctcatctgtcagctgtttgccagctcgtttggtgtgaatcacgtctaccattctcattgtcgattctcctttgatatttcgtttaaaataaagcgttctcatttgagaattgaacaaacgcccaaccctgattggttcaaatatggattgggcgttgccgttaataatctagtaagagttgtgccaaactttgatccaaaattgcgcaattggtgtagtgcgcattgattgccgcatggactgctgccgcctttcggttgccgctggcgaccaagattgcgtgtggcttatcttttaaatcatccagctgaatgccgatggtccgatcgttgatttcttttgagacaatttggccattttcatcaacaaagcgtgaaaaaatatcgccgacagccagtcgctgaatttcagctttttcctgatcattgaagtacccaagttggaaaatcaatgcctctgatcgaacagtcccgacagtgaataaggcaacgttggctcggcgcccaagatcaagaatgtgcttgatatgccggtcggtttcaaccatttccttagtgacttggttatcaaagatcaccggcagcggcagatactcgggatgggtatgataggctttcgccaattcattgactgactcataggcccaagttttttcctgggaatgactgatactacctttgagttgaaccacctgaacgccggcaacatcctgctcttcgagttgcttggtgaccgaatggatggtttccccccagccaatcccgatgatgtcaccagcttgaacgttggcagacaaaaagtcggcggtatagcggccaacaccatcttgaatactgacggtcccgccgtaattgtttggcaccacatggaattcaattccgtacttatcactcagctgtttggacaacacctgcgaatcaaccaagggattgacaatctggatcttcaccaaaccgttatccttggcatattgcagcaatcgtgacaccgtcggccgggagacccccaatcgagcggcaatttcgatttgactcaaattatcctgaaagtataattctgccacgcgcaagctttgtttgagtttggtgatgtccttaatttcatccatgtgatcgctccaatttctctttatgacatatttttaatggcggtttctagtgataatctggccatctcgtcaaatgacgtttcccgttccttggcggagagggcttcgccggtcagcaaatgatcactgaccgtcagaatggtcagtgcgcgaatgtgatgtttggcagccagcagatatagcccggaggtttccatttcagttgccaaaacgccgtaatcaattaatttgtgaatatccaactcatcgttgtagaaacgatcagcggcaaaaatgttacccaccttggtgttaatgcccatttcttgcgcggtatggtaagcagaatccagcaggccaaaatcagcaattggcgagtagtacattcctggaccaaaggtgttttgaatgatcgatgaatcggtggtcccggattggcccaaaatgacgtcacggatctttacgtccggactcatcccgccacaggacccaacccgataaatggtcttaaccccatattctttaatgagttcagtcgtataaatggccaaagacggaattcccatcccagatccctgaaccgaaatccgatgacctttataagttccagtatacccgaacatattccggacttcactgtagcggacaggattatccagataggtttcagcaatgaactttgcccgcaatggatctccaggcattaaaactgtgtcggcgatttcgccgggctttgcgccaatatgtgtactcatatgattgcctccgtttatttcaaatcagccagaaaactatcgccaaccccgttgccggcaacgttaaagttatccagcacggttgcgccaaagtcggcaaaggttttacggatgcctaagctgccagcgtgttgcattgaaggtgaataggccagcaatggcaccagttcgcgggtatgatcggtacctttaaaacctggatcgttgccgtgatcggccgtgatcagcaacaggtcatcgtccttcaaattcttcagcaccgttcccaaacgtttgtcaaaatccattaaagcttgaccaaaaccgattggattgcggcgatggccgtacattgcatcaaagtcgaccaggttggtgaagcaaaagccggtaaagtcttctgccattacgtggtcaacgtgatccatgccgtccatattactttcattatggtagccttcatcaattccgtggcctgagaaaatatcgttgattttaccgatcccgacggtgtggacccccgccttctgcaggtcgtccaaatcagtcgtgccagtcggctccaacgtgaagtcgtgccggttggcagtccgagtgaaatgatccttatcctgaccaacgtatgggcgggcaatgatccggccaaccgtgtatttgggaccgttgaccaacgttctggcatactcgcaaattttatagagttcttcaagcgggatgacgtcttcgtgggcggcaatttggagaactgagtcaccggacgtgtaaacaatcagatccccagtcttcatctgttgctccccgagttccgcaataatcttggtgccggattcaggccggttaccaataattttacggcctgaaaaatctgccaattttttgagaatctcttctgggaacccatttggaaaggtgtttaagggcttttcaaccggcaaccccatcatttcccagtggccgtccatactgtctttgccggcggaaatttcttgcatcttaccatagtagccgattggtgaagtcactttgtcgactccttcaattgccgtttggcgcaaattggaaatgccaagtttttgtaaattgggaatctgcagctttccctgataagcttcgccaacgtgtcccaaagtgtctgacccgacatcgccgaatttagcggcatccggtgcttcgcctgttccaaccgagtccattacgatgccaaaaatacgtttatattttttaactgtcatctaaattcctcccctacaaccagctgcttaagataaaatcttgacggttgcgctgacacctaaccggctggcaccagcttcgatcattgccaaagcttcttgtcgagaatgaattccaccggaagccttaacgcccaacttgttgccgacagtctttctcattaaggcaacgttatgaagggttgccccttccgtgctaaagccagtcgatgtcttcacataatcagccccggcagcttcggaagcgtggcaggcgttgacaatttgctcatcgttcaataatgacgtttcaaaaatgactttgagcattttgtgctttgcatgaaccgcttcagcaacggcttgaatatcggcagtgacgtaatcaagattgccgccgatcagttcaccgacatttaaaaccatgtcaatttcttcggcaccgtcatcaatcgccgtaatggcttcgtaaactttggtttcagtgttggttgctccgagtgggaagccgacaaccgtaattgggttaacagttgtgtcctttaaaagttcggcggcaagtggaatccagtgtgaattgatacaaacagaagccgtattatacttgattgcttcttcacaagtttggcgaatgctggcctcagttgcctctggttttaagtttgtgtggtccaaatactttgcgagttgagcggtcgtgatttcttttgtcatggtcatgtaacccctttcatttctttacaaggatagtttacaggaatttagaacatatgtaaagatgtttgttgaaattttgttctgttatgtgaacttatgagcttttagtggattgataaaagccatcgtccttgaggggcggtggcttttgggaggtgggaatattgattagttttactttctgttgttgaaaacatccatggttgcttgtgcatgttaaacgagctggttggtggagatatcgataatccgagccttggttgtccctacttacatagtgaaaatgtgctccgacgaccctgatccctactgactgcataaagcgaacccttcaataaggcacagaaccacgccttattgaagggttcactttatgctccgggatcacccgggtctcgtcgcactctgttctgaaatgtgctcctcagcccagcccctaacgtataaggccgaagcgcaaatcgataagcacacatcgcttatccattcgcccttcggccttatacaccggggctaaccgggctgactcgcactctacttcaagtctccaatcgtattcacattcttcatatacgttggaacagccaagccgaccttggcgccatgcaagttgacacccaaatcgtcaaacttgcccttgtagtccttataatacagtccctgagttgtcggcagccaggcacttaccatcccatccgctgcatttgtagcaattgatgcccacagtggttggacttccattgcttggatttccaccttgtaacctaatgaccgcaatacgttggccaccacattggttgaggcaatttcagaatcccaggcgacatacgtcagcttgatcgattgaccatgaacgtgggcaatgcccttcgtccaggtatcaacctgcttttgattggccttgatccaatcattggcagctttatgtggatcttctccattattgactttcaacatcacatctgccatttgttttggccgccaattaaagcggttcagcatttcatacgcctgtggtttgtccttcttcaatccttttcgaacgatggtgtgaatgtcttcggctttgccgtatacgttcttaggatctttcaaaaattttaaattgtatttggtaaacatccagtgcggagtccagccggttacgacaatcggctgatgatttttgatagctttacccaaggtactggtcattgccgcggtggaactggtctgcagctgccatttacctttgtccaaaccatatgccttcatggccttctgcgtactggacatgatcccggcaccggcctcaatcccggtaattgtgtagttgatctgcttgccaaggctttcgttagcatgataccgagcaggcttactaccacatgccgaaaggagaatcatcgagaagaacaaggcaatggttaatagaaatcgattgttcttttttcgcatagtaacccccttctatgacttagggacttttgttcggttaatcgcctgtgtaatccggtcaaggatgattgccagaataacgattgccaaaccggcagcaaaaccgccaccagcatcgtttcgaccaacggcaaagtagaccttgtttccaagtcccatcgccccaatcatcgaagcaatcacaaccattgacaacgacagcatcatactttgattaacgccggccattaaggttgatttcgctaacggtaattgaaccttaaacaacttttgccaaccagtagatccatacgaatctgcagcttcaatcaagtcattgggcacttgacggattcccagattggtcattcgaaccgtcggtggcattgcaaaaataacggaggcaatgacccctggaaccataccgatcccaaagaaggcaaccgctggaatcaaataaacaaaggctggcattgtttgcataaagtccaaaattggcttattgatcaccgcaaaaactttggatttagccatccagattccaagcggcaccccaatcaccaacgcaatcaaactggatgtcagaaccagtgtgagggtctgggtcatatcccgccagaaaccttgattccaaatgtaaaggagaccaatcgcttcaaaaatcagtaatgtccaatgcttggtgttgcggttcagccagtaagtagcccccagaacaatcagcatgaacagccaaattggcaggatgtcaaagacccattggaaaccgttaatgatgccgccgataaaattggtgacaccgttaaagaagccttcaaagcctgagagccagtcgacaaatttatcaatccagctggagactggtaattgtggaatgttattcatcctctgtcacctcatttcctgaaatggcgcccagaacggcacctcgaatgatgattcctagtaaatgtttttgatcgtcaagcaccgcaaatggaatcggtgtctgcgagattttttccataatctccgtaatcggtgtgtcgggatgggtcgttgggacatcggtttggacaactgacatcagatcagggtttttctgtttaattaatcccatcacgtgatcagcatccgcaacgccaacgaattcccgcttactattgacaacgtaaacagacgaaatttcattctcacgcatccgacgcattgcgatccgtggaccatccttatcgatattgacaaaagttgggcgaatcatcacattggaagcagttaagaccttggtccggtcaacatcttcgataaatttctcaacgtattcgtcagcaggctgagtcagaatctcttctggagtcccggtctggacaatcacaccgtccttcatgatcataattcggtcaccaattctcagggcttcgttcagatcatgagagataaaaacgattgtcttgtgcaggttctcctgcagatccagtaattcatcctgcatatcttttcgattcaaaggatcaagggctgaaaaggcctcgtccatcaacaggatttcagaatcagttgccaatgctctggctaagccaactcgctgctgcatcccaccagagagttgggttggatattggtcgtcgtagccgtgaagaccaactaattccaaggcatcgtgggccttttttaagcgttcatccttgtcaacgcctttaacttccaatccgtaggcagtattttcaatgattgtccgatttgggaataacgcaaaattctgaaagaccatgctcattttgttgcgacgaacatccaacagttcttttttattcagatctgtcagattctcgccatcaatcagtaccttgccggatgtcggctcaattagacggttaatcattcgaatcatggtggacttaccacttcctgatagtcccatgatcacgaagatttcaccatcattgacctcaaagttggcatcgctaacgccaaccgttgctccagcattttgtaaaatttcagcttttgacttaccttgttttaatagttcttcagctttttgaatcctgcggccaaagattttggtaagatgttgcacttgtagttttgctgtcatgtgctcctccttacatcattcatgataaataaaaatcaattaccggcctaaagcacaaacgtatgtggaagccagtaattgaacgacttataaaaccttaacaaaaatatgcattcagttcaaccaattagcaaatccgtcagattccctcattgggggaatgtaaccggttttatggttgaccttatctacataatagcaattttatacatttgcactgtatcttgttgccggggttgctacatttacttttagaataggatttcaacgggattggaaaatatttttggctttttttaaatttgctgattccctcacacattctctgttaactgcaacattgaatgacctctggcaataatgaaaatcgatggaatcatcaattcgtttttgtaaattgaacaaatatccgttggatgggctcattcaacgcttaatgaccacgttccaagacggtaattgattcaacatgcacggtctgtgggaattggtcaacgggttgaatcggttgattaacctgataaccttgctcagtaaataatttaacatctcgtgccaaagttgccggattacatgacacatagaccactcgcttgggctgcattttcaccacgctgtcaatcaaactggcatcaaggcctttacgcggcggatcaacagaaatgacatccggctttaagccgtcttcctgccatttggccatttgcgtctcggctttgccggtaacgaagtgcacattggttaaattgttaagcttggcgttcttcttggcatcttcaacagcttcagggacaatttcaaccccataaacctgcttggccacgcgggccatggaaagcgaaatcgtcccgattccacaataggcatcgatcacaacatcgtcagccgacaagtcagctttcttggtcgccaaatcatataatttttccgtctgcacagggttgacttgataaaatgagctggctgaaatatcaaacttcagtccaagcagggtatcctcaatggtactcttaccagccaaaactttatttttcttgcccatcaaggcattcgttttttcaggattgacattttggacgatactcttcacttcgggcagtgactgttcaatttcagccacaatctcgctactgcttggcaatttctctgttctggtaatcaaaacgatcatcatttcatgagagtaatggccgcggcggaccatgatgttgcggacaacgcctttgttagtttgttcatcatagggttgaactctgaacttgcgcaaaatgtcacgaacaaccaccactgcctcatcaatcttgggatcttgaatatagaagtcttcaatcggcaccaagtcatgagagtgtttccgataaaaaccggtttgaagctgcccattaattgagcggacaggaatttgagccttgttacgatagtgggtgggatcgtccatgccgatcgtgggattaacagtcacatcaagcttcattttatcgaagtcaacttgaatttgatgttgcttgaattttaattgcgcatcatattttagatgttgaagcggcgcaattccggtttgggtgtatgctttatccaccaattcaacccggtctttactcttttgattgatcttaactacccgtccgaaggcaaagttctttttaaccttaataaccttcatggtcacgttttcggttggaagagcattttcaataaaaattgggaaatcatcaatcttggcaactcccagaccttgatacgttaaatcagtaatatcaacgtcgtagttctggttcttttcaactggtaccatctttttcatttattcacctttttaattcctagaaacaaaaattgcgaaacgaaagcttcgtaacgcaattataacatcttattaaactattctttatcagggagtttgtcaacgcctgtgacgaagttcttttcaactctgcgcatctcattggtttcatcagaatacgcatcatcaggaatttcgtcggtattggcaaaaaattcaatgtgttgtttgagatcaacgaaagtcatcggtgcatctccaccatattcaccgtccagattgatctgcattcgatcatgaaccggcttggcagtgactttacgcacctttttatagataatccgtggatcatcgacatgccggccaccgttgaggacttttgatgctaaatggagaatttcaaccaagttgctggttttaacgataattaaagtgaattttccatcatctaaggaagcgtctggaacaatttgctcgaacccgccaaccgagttggttagtgccaggaaaaacatcgaggccttacctttaaactcttcatcgtcatacttcagatccatctcaatcggcttaatgcgtggcaacagttcagctccacgaaccaaataagctaagtaaccaaagaaggttttcaagtctgaaggaacatcgtaggtcagttcggttagcaatccacccgcagcaatattgataaagtaattttcacccgctttaccgatatccatccgcagggtttggtccttcaagaccaccttggcagcctcgacgggatcttctctgggaatgtgcagcgctcttgcgtaatcgttagtcgttccggcgggaataatcgccatcttgggacgcttcttcagtggcgcgatgccgttaaccacctcgttaatggtaccatccccacctgcagctaccacgagttcaaagccgtctttggcagcacggcgagcctcgtttttagcagagtccttggcgggggttgtcgcataagcgctggtttcataaccagcttgctcaaaaatattcaaaatgtcgactaacttttgcttgagaagttcccttcccgaagttggattataaataacccgggcccgttttcgcatatccatcctgactttctatttactcattgaatcctttagcattttgttgattacttgcgggttagctttcccgtgggtttgtttcataatttgaccaaccaagaaaccgatggcccgatccttaccgttatggaaatcttcaacagattgtgggttagccgctacgacttcatcaacaattggctgaagtttggctgggtctgacaactgaaccatgcccttgtcttcaacgaatttcttgggctcttcaccattggtgatggctttaaagactttcttagccatctttgatgaaatcgtgccgtcagaaataagtttgatcatagttgccaaatgctcaggggtgatcttggtatcttgtagttcaacctgattatcattcatataagcattaacgtcgccttgcaggtagttggcagccaatttggcgtcagcaccggcagcaatcatcttatcaaagaaatcagacatttccttggtctgggtaatgaccatcgcatcgtaatctgtaatcccaagttcattgacataacgctcacgacgttttgcaggcgcctcaggcagttctgactgaatctcgtcaatccagtcctgtgaaatattcaaaactgggagatcaggttctgggaagtaacggtaatcatcggagccttccttagtccgcattaagatggtttggccggttgactcgtcaaaacgacgggtttcctgggcaattttgccgcccgacatcaaaacacgttgatgacgagcttcctcaaacgccaaaccttttttaacatacgtgaaggagttcaaattcttcaattcagtcttggtcccatattcctgctggccaacggggcgaacagaaatgttaacatcgacacgcatggaaccttgttccatcttaacgtcggatacacccgtgaactggataacctgacgtaattgttccaagtaggcatatgcttcatctggagaagaaatgtcgggtttggaaacaatttcaatcagtggcgttccctgacggttcaaatcaacgtaagaatattcggaagcatgcgagttcttaccagcatcctcttcgatatgcatttcagcaattccgattttctttttcttgccgtcaacatcaatttcaacccagccatcatgggcaattggggtttctgattgagtgatctggtaagctttaggattatcgggatagaagtagttcttccggtcaaagtgtgggtggcgttcaatttgggcgtgaagtgccaaaccagccatgatgccgtcatggacaactcctttattggtggttggtaaaacaccaggatatccccagtcaatgacgttggtattggagttgggttcatcaccaaattctacaggagatggactaaaaattttggaattggtttttaattcaacgtggacttccagtccgattgtcgtttcaaaattcattagttgttacctcccatctttggtgtttgttttgcaaaattagtttcttgttcaaatgcactacctgcttggtaaacggtcaattcgtcatatgggcgaccaatcaattgcacacccactggtaagcccttggagaacccggcaggaattgacatccctggcaagccagccaagttaaccggcagggtcaacacatcgttcatatacatggtcatcggatctgagacatcctcaccgattccatatgcaggcgtcggtgcagtaggtgccaaaatcaagtcatagtctttgaagacattggtaaagtcattaatcatcaacgtccgaacttgagcggcttttttgaagtaggcgtcataaaaaccagctgaaagtgagaatgttcccagcatgattcgacgcttaacttcgtcgccaaaaccttctgaacgggatttaacgtacaagtcttccaagtctttgacgtcttttgcccggcgaccataacgaatgccgtcaaaacgctgcaggttggaagaagcttcggatgaggaaatgatgtaataagccgccacaccgtacttggtatgtggaagtgaaacttcttcaacggttgcccccagctttttgaaggtttccgcagtatctaagacggtttgcttgatatcgtcatccagtccctgggccataaattcagtcggaatcccgattttcatgcccttaacacctttgttcaatgtgctggtgaagtcaggcacttctttagtcgaagaagtcaagtcatgctcgtcgtggccggcaatggcgttcataatcgttgcattgtcgctgacgttacgagtgattggcccaatttgatccaaactggaaccaaaagcaatcagtccccatcgtgaaactcggccataagtcggcttcatgccgaccacaccattaaatgatgctggctgacgaatagaaccgccagtatctgatcccaaagcggcaatgacttcaccggcagcaacagcagcagctgaaccacctgacgaaccaccaggaactttggttgtgtcccaagggttatgagtaatcttaaatgcagagttttcagttgacccgcccatggcaaattcatccatgttggtcttaccaactgtaatggtgccaagtttgttcaacttgtcaacagcggtagcatcataaatcggcttgaagttttccaggattttcgacgctgcggttgtggtcaagcctttagtcaccatattgtccttaatggcaattggcattccagataaaaggttatcggcatcaatgcccttagcatcaacgtcggcagctttcttcaaagccccttcatcatcaacagtaataaaagcgttgatgtcattatcaacggatttaatgttatccaaagtttgctgggtcaaatccttcgcagagatttctttgttgaccagttgtttgtgaatgctggaaagtgattgatcgaaataattcattattcgttatccccgctttcatcaataatggttggcactctgatgtagccatcggccgtgtccggtgcgttatcaagcaatgcttggcgttggtgccaatcttcggcgatatcgtctcgcatcacgttaatttgatcagtcacactactggtaggttcaacgccgtcagtgtcaacttcgctcagtgtttcaaacaacccaatgatttggtctaattgagtggtgaaatatggcagttgatcgtcggcaatttttagctttgctaattcagcaacgtgttttacttgatcttcggagatcttttcagtcattgaaatccttctctcttctgaatatatccaaaatttaataacaacaataattctaccatataaagaatcgcattttttagaaattaataactattgaaaatatgggcagaaaatttcttctcattttgcttacggctcaagaaactctgaatgccttcagtcgaagataccgtaatgtcaattggtgcattggccggcaaatatcgctgagcggcattttgaatgtattgggtaaaactgatgatctcagtctgactataaaattgagtcgtaatgctgatattcatcccactgagtgagccatcggtgtattgtgcttgagcagtcaccccactcaaattcgggaagaagccttgaatttctgatttgaagttatcaaacgaatcagcatcattttggctgggacccttcttgtcagattgtaatgggaagacatagttcttttgattaattttgtcccacttggcaactttggtttcaccatcgtcattcatggaatatgcaaagaagttcccgccgaccaggctatcatctgaagcttgcttgtataaagcaatgatgattggaatgttcttcagcgatcgccgttgtcgcagccgcttaatcacttggttggcgatagctttaccctgctttttaacttgggcatcggaaatgtcggtttcataagttggcccataggccgtcttcttatagtaatcaaccgagttgattcccagtccgatggtcatccctgacaagcgaagcgatttgccgctttgggtcatgaaatcctgctcatcaatttgggaaagataaattggatttctagtgttagggttggtcgatttggacttaaccggattttaagccggttgggtttgatttcgattgacggcccaaccaattttcaactgtgctggtagaaagatattgaccttcttggaaaatgtattttttagttgaaaattcttttttggaaatatccaacaggccgttttcaaaccccttaatattgaactgatttgattcttgagaaacactcacaccacgagatttactggtctgataacggccattcttgatcacaccttgataatagtcggtgttcgtttggccggttaactgcgtcttggcttttgacccactggaattgctggtatccttcgacagattatcaacgctcccacacgctgccaacataaatcccgacagaatgattgaaatccccaggataatttttttcacgattcgttcctccattgtcacttttcatcggccatttcttggtggaaacgggcttcgtcccatgtctgaatgccgaggcttttcgccttatcatacttgctgccggggtcttcacccacaacaacgatgtctgtatttttggaaactgaactgctgactttggcaccatggtcctcaagccattgagttgcatccggccgggtgatattttgtaatttccctgtcagaacgaacttcttgccggtgaagaatgaatcactttcagcaagttgttcatcagtcacacccagataatccatgttgacgcccacttgtttgagttggtcgatcaactgcttggattcaggcattgagaagtaagtaaccacgctgtcagcaatgatcattcccattgtagcaatttcggcgatatcttgcgcgcttgcctgcataaccttatcaatatttttaaaacgttgggcaattaatcgagctgccttgatcccaacatggcggattcccaagccataaagcagtcgttcacaagaattcgatcggctgttatcaatggcagccagcagcttagtggctgatttttcaccaaatttgtccaaagttaatagttggtcaaaggacaaatcataaagtccggcaacatcggagaccatgtgtttttcaaacaactgggcgatgatttttggccccaaaccgtcgatattcatggcatccctggaagcaaagtgggttaagccttctttgagttgcgccggacactgaggattaatgcagcgaagcgcaacctcttggtccaagtgaaccagggtggaaccgcatgatggacactgggttgggatttcataggcctgactgttggcaggccgtttatctggtaagtactgcgagatttcagggatgatgtcgccagctttatgcagcttaacggtatcgccgacccgaatatctttttctgccaaataatccggattatgaagtgatgcccggctgacagtactgccggctaatatcaccggatccataaccgcagtgggtgtcaccaccccggtccgtccaacggtccattcaatgtccctaacaatcgtttgaacctcttctggtggaaacttgtatgcaatcgcccaacggggaactttaacggttgccccgagtgagcgctgcagcggtagtgaattgactttaatcacaatgccgtcaatcccatagggcaaaccatcccgtaaatctttgtatttatcaacgtaattgtcaatatcagccatattgtgggcaactttgaaatctggattgatcgtaaagcccaattctttgagttcggcaagcatcccgctttgagtgtcagattgcaaatcatcgatatcggcaacgttatacataaaagtacttaatttgcgactgcgggtcacacgtggatccagctgacgcaaacttccggccgcagcattccttggattggcgaatggttcttcaccatccaactggcgctgttcattcaatttggcaaacgattctttgggcatgtaacattcgccacgaacctcaatattgatcggtcgagtcaacttttgcggaattgacttaatcgtctttaagttacgggtaatatcttcaccaatttgaccgtttccgcgagtggatccttgaacaaagaccccgttctcatatcgaaggttgattgccaaaccatcgatttttaattcgcaattataatcaaacgcgactgaatcattttcacttagacggtcgacgaattccgccaactcttccttagagaaaacatctcccaatgaaagcatcggaatttcatggttaaccttggtaaaaccgggaagcgtgtgatccccgactttttgagtaggtgaatcaggggtcacaatctgtggaaattgattttccaatgcgaccagctgctgataagtttggtcatacacggcatcttcgacacttggtgcgtcataggtgtaatactcgtcagcccactggttcaattgtttcctcagatcgccagccttagcagcggcctgttgctcggacatattttcaaatgccacaataacaccttctgttgattaattttcctgcttcttaattggggcaaatgcagccaacagccgcttgatgccctcttgcttgaatgcaatatcgagctccatatcctcgccggttccggtaaccttgacaaccgtgccggttccccaagccttgtgtgacactttatcaccaacggcccaagcgagtttgtctgcaccggatcctttagggctttcgacgacttttccaggtcgccgataagtagttgcagttgcccgcctggttcggcgatcaaacggcgtgcttaggggggactcagtttgctgttgattatccgaatggataagctctgggctaatttcgttcacgaagcgcgactctggattgttttgacgacgcccatacaacattcgtgagtaggcattggtaatatagagtttttctttggcacgcgtaatgccaacgtacgctaatcggcgctcttcttgaagttctgattcgtctgctgcggctcgtgaaagcgggaataatccttcttccattcccatcaaaaagaccactggaaattccagtcccttggctgcatgcaaagtcatcaaagtcacttgggaattgtcttcttcgagactatcctgatcagaaaccaaggccaaatcacttaagaaattcactaagttctgttgaccggtttcgccctcgttttcttcatcatacttttgagtcacagaaataaattcttccaagttttcaagcctggtttgagcttccaaagacttcgaagctttcaaggtacttagatagccactcttatcgagaatttcttcagtaatttcagtgattgataattgtgccatcttctctgaaatcgttcgcatcgtctgttcaaattcagcaatcgaattttttgcacgggtagaaatctcattggctaagtcaacgtttttagcagcctcaaggagactccactgatgatcgttggcgaatagtcgtaatcgttcaatgctggcttggccgatcccccgtttaggttcgttgatgactcgttcaaaactcatggagtcatttggattggctaacaaagtcaggtaagacaaggcgtctcgaatttcttttcgatcatagaacttgtgtccgccaaccatggtgtagggaatatttgatttgagcaaggtttcttcaattacccgtgactgcgcattggttcggtaaaggatcgcaaaactgccgtaattgcgttttggcttggccatttcttcttggattttggcaacaacgtatcttgcctcgtcgttttcggtctgaccacgataatacgaaatctgatcgcctttggggttttcagtccacaaatttttgtcggcacgattgtcattatgggcaatcaccgaattagcggcatcaagcaccgttttagttgaacgataattttgttccaataaggtcacatgggcatccggatagtcttttttgaaatcaaggatgttctgcatgttggcaccacgccagccgtagatactttggtcggcatccccgacaacacagatattacgatttttcttggcaagggtattcaccagtcggtattgagcctcattggtatcctgatactcatcaacatggatgtattgaaatttgtcctgataggattccaaaacatctggatgttcatcaaataattggatggtgatcataatcaaatcatcaaagtccaatgattgattctgcttcagctctgcttggtagcgatcataaacgtccgccacgatttgatcgaaagcactattagcctgagctttgaatgctttgggcgtgagcagatcatttttggcgttggagatagccgataaaacggctctgggatcgaattttttgggatcaatattcaaatcccgcagtactcgtttaacaagcgtccgttgctcactggtatcggcaatcgtaaaagccttattgtagcccagcaaatcaatatggcggcgtaaaatccgcacacatagtgcatggaatgttgaaacccaaacatcgttaccaccttcacccaacaattttgaaacccgttcacgcatttcccgggcagctttattggtaaaagtgatcgctaaaatccgccacggcataatatggttatgttcaattatgtaggcaattcggtgggttaatacccgggtcttgccactgccggcaccggccataatgaggacgggtccttcagtatggataacggcgtctttttgatctttatttaatcctgctaataaactttcttctgccactaaatattccatcctctcgcatttatcttttcaattataacaaaaaagtcggcttcccgactctctacatgttgctatattttgttttgtaatctatgtcatgccaaatcccagtggcctccagtttaaccaaggtatctgaaatagatttggtcggaatcaagacatgcccaaccagctgatggtcgtcagttggctcgttgccataaaacgtgaagtgccaattatctttgatgacccattgggtttggacacgttgatattcctgttgtcgaatggcctgataaaccgttgcaattccgggaataatttgtgtcaaaggcaaaccggcaattgcccgcaaatgttgttcaaattcatcggcattagcagcgtaatcaaatacaaacccagccgcactcaatttgggagcaactctgctgacataaatcgaaccgctcttggccaagaagagtgtgacttcgaaagtaccgacatagtcaaggttgttggcaatttcattggtaattcgggtcatttccttcttcacactgggatcgagttttgccggcgtataggcggtcattaactgatcgccttcatacatcacttcgactggtggaaacatcacaattgaccctgactcggtccgggtaacgaccacggagtagtcagtattatgttccacataggattccaaaatgtaagttccggaatctaaaaaaccggatgccaggacaatatcagcctggttcttaatcagcaattccttgccgccgtttagtccccgctgaatgggctttaaaatagccgggtacccaatggaattaatggcttggtaaatgtcttccaacgtgacaatcgtcgagtaaggaaccatgttaatattcagggtttcaaaaaaagttcgttcaatcagtcgatcttggacaatatccaataatccgtcccgttgcgccacagccgtgtattgggaaatgtatcgaatgacatctgaatcgataaattgattgtcatagatcaccgcttcacagcgttcggcaaacattttcaaggtttccttgtcagtgtaggggccaatgtatttatagtctgccagttccatcgccttactgttttcgttggaactgtacatgccaacattaaagcccatttgttttgcgcgagccaataacgttggggtgctgatactatctccaagaatcccaattgtttgaccgggatagataacatttgcgtttgccaattaattcactactttcatatcgtcattttattaattgtaagtcatcactaaacttatcgtaccattattttcacagctctaatcaacaaatgtgactttttggttatccagagaggcaattcgggccaaagactccaaacggacacctgatttttcaatcatggtgtgccctttttggaagctcttttcgatcacaatcccaacaccctcaactttaacatttgccaacttggcaatttccaacagtccttgaacggcctgaccatttgccaaaaaatcatcaataatcaaaattcgatcatttggcttcaaaaatcgtttatcaatactgatatcgttgctaacttgcttggtataagaataaacactggcggtgtacaggttatcggttaaagttaaactcttatgctttctggcaaagatcaacggaacccccatatggatcgccgttgtcaatgccggggcgattccggaagattcaacggtcacaaccttggttaccccttcatctttaaataagcgggcaaattcggcaccaatttggtccatcaattttgcatcaacctggtgatttaaaaagttgtcgacctttaatacgtttcctggtaatacagtaccatcctccaaaatgcgtttcttaagtaagtccatctcaaaattcctttctagtcatcgtattgataaagtttgtattgtctgatgatggcgatcaatttcttggtgtaagcagggtcggtcgcatagccatcctgctgaaggccatcagcggcctgcaggtagttgtttgcggccaccacgtccttgtactgctgtgggttccatttcgtgccgtaagcaagcaatttggcgtgatcagccaaggattcattccaatcctgatatacttggaaccgagctttgatcgtcacataacggccattcacaaattcttgcgtattcaggtagaccgagttggtggtattatcctgagctttgacgccaaacagattataatacttgctcgcaagcttgctggtgccccagttggactccaaaatggcctgggctaaagtaatacttggtaagatattatattgtccctgcagccgctgggcttgtggcgctaatttgttgataaatttacggtgctcaatggctacttcgtcgtttgagctttgaatattgctcgaatgataaccgttttcgtacaaagcgtggaaaccaaaaatgatcaccaacccacagatcaccagaatcaacatcaaaacggcatttgctttttttgcgcggcgtttccgccccttcttatattttgccaatccaacctcaaactttctaactttaaaattaattctaacgataaatccgaataaagacaaacgaaatttgtgctttgttcaatttttataaatgcgtaaaaattgacaaatctgttaatttcggttatgttatcctctgacacttaaatctggagatgaaaaccaatggctaaaaacaccgaagtatcagaagctcaatcaaaatttcatgttggtgatgaggtttcattcaagatcgaaaaacagacgtttaccggcttcgttgataagagttacaccaactcatttttaatcacttttgaatcggatgatcctgagattatcgacaagtaccacaaaaaggttgtcatcaataatcgtcatctcaaaatgatcaaggcagctcctcaacctgaagttgaggatgatgacgaggacgataatgaaactaaatcctcgagaaccaaaaaatcgagcaagaaataatgattaaaagtagaccctgcatatatttgtgcaaggtctattttttatctgctggtccggtcaaaaatctttttaaccggcaccgcaatcaacggtgtgacaattccgctaaagattgcttccggaacaccattcgtaccaaccacccctagtaaatatgggaggagttctttgatattaatctgatacagttgaggggctttcgccttataaaacagataaatgagtcccagcaccaagaccgtgttggttaatgaacccaagacagccgatacagaaatactggctgcctggcttttcaagtgtttcttgagatacgtgtacgtcataccagcaactacgccaatcataatccgggggatgaccgaaataatcgggttaacgaagacaattgccgctaaagggctggtcggccatacaaaagctcggacaaaagtcgtcatcccccaaacaccaccaatgatcgctccgtcaacagttccaagcaaaaccgttgcaacgacgacagtcatcgggataatcgtaatttcaagtggaccaattgggatgtacccgatcaaaggaatcgaagtttgcaacagaatgatcgcaataaacattgccagcatgttcagtcgtaaagtatttttcttaacaggcatgtgttcttacccctttaaagttgttggaaccattatacaataacggattgtattctaatacaattttgctggtgaatgtcagtttaccaacaagcttaaaatattctcaacaaaaaaacactcctcaaaagagaagtgttttgaaaaagcaaagtaaattttaacgctttgaaaattgtgaagctttacgggcctttttaagacctggcttcttacgttctttcattcgtgcgtcacgagttaataaaccggcacgcttcaatggtccacggaagtcgggatcaactgcaagcaatgcacgggcaattccgtgacgagttgcgccggcttggccggagaatccaccaccgttaacgttaaccaaggtatcatagttacctaaagtctcagttacgttgaatggttgcacaacaacttcacgcaagttagcaaatggaatatagtcttcgattgctttgtcattcatgataatttttccagttccgggtaccaagcgtactcgagcaactgaatctttacgacggccagtgccgcgatattgtacttgagccaaagtgaattcctccttaaattaggttattaatgtctaatacttctggtttttgagcttgatgatcgtgttcaggacctgcatagacatgtaacttcaaaccaattttatgacctaatgttccatgaggaagcattcctttaacggaagtttcaattaacttttcgggattcttagcacgcaaatcaccggcagttcgttgcttcaagccaccaataaagcgactgtgatggtaatagatcttccgagtgtctttgtgaccagtcagaccgactttacttgcattaattacaatcacattatccccagtatccacgttgggtgtgaatgttggtttattcttacctcttaagattgatgctactgctgatgataaacgtccaagagatacgtctgttgcgtcaacaacgtaccatttacgttctacttcaccaggttttgccatataagttgtacgcactgtatattcctccattgttcctgtgtttgttcgacaccaaataagattccggggcttatcgtggggcaaacaataccaattaacataatacaaattattctggtgaaagtcaattagtttcctaaattatcgttgtcgttttggcaatttcgtggggtgcttcggatcttcaccctcataatagactttctttaagtacaaaccggatgccggcatggttcgtcgggcctggtcacgatctttcacctcgtataagcgcaatatatcgtgctcagggcgcatttgagacccaatctcaacaactaccccaaccatgattcgaaccatgttatagaggaaaccattgccatagaactcaagccgaatttcgttggctgatttgtccaaaatcgcattagcttcataaatcgttcgaacattggatcgtgcagtcgaccccgaagcgacaaaactggaaaagtcatgttcaccaacgaaatcattcattgccgtttgaacccgttcaatatcaatgggaaaacgccaattgccggtataattccgtttgaacggatccttaaattcgcctaaatccagccgataaacataccgtttaccggacacatcgtagcgggcatggaaagtattggataccttttccgcttttttaatctccatgtcaagcggcaggagactgtttagtccccgataaattgccttggttggcaaatcaaacgggaaatcaaaatggacaacttgtccgagggcatggacaccggcatctgtcctgccagatccgtagacgacaattggggggtcgggattttttgccatgatattcactttttgggtcaaaacaccctcaatcgttctgcgcttgggctggcgctcaaagccgctgaacaacgtgccatcataggctaacgtcactttgtatcgaatattgaacacctcaactctttcttatgaataaaacgagcaccccgactaacaaaaagactgcccaactaatggtatcttttcgctgccaccgataaatccggtatttgctgcggtgctcactgtcggtaaagccacgggcttccatggcagttgacaggttttctgcatgattgattgctccggtaaataatgggacgagcaggggaacggctgcttgaatccgatggcgtaagcttccggacccaaagtccacccctcttgaccgttgagcatttaaaatagtttccatttcatccattaaggtcggtacaaaacgtaaagcaattgaaagcatcaacgccaatgtgtccacaggaaagtgaacttttttgagaggccgaagaacggtctgcaccccgtctgcaatcgccaagggcgttgttgtcaaggtcaaaaccgtcgagatcatgataatcaacagaaatcggatgaaaataaaaccaccgttaattaagctggtatcactgactgaaaatggaccaaaatgccaatagacatgtcccccactgctgaatagaatctgcagtaagacagtaaaaataatcaaccaaataagtggcctaatcccttttagaaaataaccaatcgacacgcctgacatgaggaccaccatgagaatcaacacactcaatgccgcataagtccaaatgttattggcaaagaaaatcacaaccacgaaataaaagctcagcatcaatttggattggggactcatttgatgaacccaagaattaccaggaaggtaccgaccaaataggaaattactcatggccatgccccccttgaacaacttcgacgattgcatccgccaatttgtcaattgtcagtggaacactttttagcggaacccctgcagtgatcaatcgagaagcaaattcggcactactcggcaaatccagatgcatctgatagacccactggggatccgcaaaaatctcttgcggtcttccatgtttaacaatcttcccttgatccatcacaataacgtcagaagcgtaatcaacaacatcatccatttggtgcgtgacgagaataatcgtcatgccctgatgttcgtgcaggtcttcagccaagtccataatttctttgtggccgcgaggatccaagccagcagtgggttcatccagaatgagaatttccggcttcattgccaaaaccccagcaatcgcaactcttctcatttggccgccggaaagatcaaatggtgacttctcctgcaaatcttcgtcgaggccaactaatgccatcgcctgtttggcatcggctctagcttcttggtcagaagccccataatttttggggccaaacataacatccttgataaccgtttcttcaaataattgtttttccggaaattgaaataccatgccgacgtgcttacgaagttgctttaaattcttattggtggtcgcaggtgtaatcgttcgccctgacacctcaatttctcccatagtcggcttgagaagcgcattaatgtgctgtaccaaagtggacttgccgctaccggtgtgaccgataattgctgtaaatgacccgctggcaatggttaaggatacctgattcaaagcattttgggcaaatggtgtatcgggttgataagtatgagttacttctttgaaattaattgtttgatccatgtaattaacctctcatcattgagatattgactatgtgagtcgattccacgctttttgagggcagacagcaattcggacgtaaaaggtgcggataagccaattgatgtcaatttttcaatgtcaccaaaaatatgatccggctgatcagcttcaacaacttgaccttgattgacaacaatgacttggtctgcaccagcggcctcatctatgtcatgcgtaatggagatgacggtcagattattttcgcgtttaatctgattaaccagttttaaaatgtcttgtcggccacgaggatccagcatgctggtagcttcgtccaaaatgatgattttcggactaagggcaataattccggcaatcgcaacgcgctgcttttgtccgccagataaattagcaggaatccgatcacgaaagtcccacatgccaacctgtcgaaggctttgttcaacaatttgatgcatttgctcacgcggaacttggcgattctctaagccaaatgcaacgtcatcctctacggtcgctccaacaaactgatcttcaggattttgaaaaaccatgccaatcttatttcgaatctcaaagatatttgtatcgttgactgtcagtccatcaacaataatttgaccagacttcagaacaattaggccgtcaattaagcgggccagtgtactcttcccacttccattttggccaatgatagccgtccatttaccttcctgaatattcatcgaaaaattattgaaaagtttttcttgttcggggtaattgaaagaaatgtttttaatttgaataatatccttcatgatgttcctcacgctgtgcaaagtgttttatctatgtacaaaaaaatcacttacaggtaatcggtgcatgagataagtcccacattcaaactagactaggaactgggttccaccatcataacgttctataccaaaaacctgagtgattctcgtgataaatatgtgatttggtttaatactagttagtcaactaactctaaaatgaccattggagcaccgtcgccacgacgaggcatagtcttcaaaattcgtgtatatccaccattacgatcagcatactttgtagctaattcgccaaatactttttgcaaagcagtcgtaacgttaatatcgtcaccatcttctttaacatcagcaacaacatcacgaacaaatgatgcagcttgacgacgggcgtgtaaatcgccgcgcttgccaagtgaaatcatcttgtcagcagttgagcgaacttccttagcttttgcttcagtagtaatgatttgaccatgaataattaactcagtagtcaaattacgaagcaatgagcgacgatgtgcactactacgttgtaatttccgataacccataattggatgtcctccttctttatctttattagtcttctttacgaagtgaaaggcccaatgcagcaagcttttctttaacttcttcaagtgacttgcgaccaagattacgaaccttcatcatatcagcttcggtcttttccgtaagttcttgaacagtattaatgccggcacgtttaagacagttgtatgaacgaactgataggtccaattcttcaattgtcatttccaacattttttctttgtgggtttcttccttctcgaccatgatttcggtattcttagcttcatcagtcaaatcaacaaacatctctagatgttcggttaaaattttggccgccaaactaactgcttcactcggagtaattgaaccatcagtccaaatatccagtgtaagcttatcaaaatcatcgcgttgaccaacccgtgtactttcaacctgatagttgacacgttcgattggggtataaatagaatcgacgggaagcacaccaataggcatttcagaactgcgctttttgttttccacagcagaaacgtatccacgacctttgttggcagttaaccgcatatggaatgtggcaccttcagcaacggtagcgatgtgcaaatcagggttcagaacagtcacatcactgtcagcttgaatatcaccggcagtaacatcagcaggaccaattacatcgatttccaaattttcttcttcatcttctggcccatctaatttcaaagaaattttcttaacattcaatataatctgagtcacatcttcgacaacacctttgatcgtcgaaaattcgtgcagtacgtcatcaatctggatgctggtaacagcagcgccaggaagagatgacagtaatgtacgtctcaaagaatttccgagagttgtaccatatccacgttcgagcggttcaacgacaacttcaccaaaattatttgtttcttcaattttatgaatgttaggcttttcaaattcaatcattcttatcattaacccctttcaaaacgcgtgagtcttcatgcaaaatatcaatatgcttaaaccaagtaaaattcactatattgaatgtcttaattaaactcgacgacgctttggaggacgagaaccattgtgaggtaccggagtaacatcacgaatagcagtaacttccaatccagtagcttgaagtgcacgaatggcagcttcacggcctgaacctggtcctttgacagcaacttcaacggatttcataccatgttccattgatgccttagcagcagcttcggcagccatttgagcagcaaatggtgttgacttacgacttccacggaaacctaatgcaccggctgatgaccaagaaaccgcattcccagtggtgtcggtaatcataactaaagtattgttgaatgttgaatggatatgtgcaacaccagcagcaatattctttttagcacggcgtttacgacttgtctttttgtttaccataaaaactgatgacctccttctttaattattttcttctaccagcagcaactttgctacctttacgtgtgcgggcattgttcttggtatgttgaccacgaactggcagtccacgacgatgacgcattccacgatatgatccaatttcttgaagtcgtttgatgttcatacttacttcacgacgtaagtcaccttcgattttaagatcgccgacaacttcacgaatcttgtcttcttggtctggtgtcaaatcacgtacacgaacatcttcagaaactccagcttttgctaagactttttgagctgttgtgttaccaataccaaaaatgtaagttaatccgataacaattcgcttgtcacggggtaaatcaattccggcaatacgagccattgagcatacacctcctgtttatgtttatttaccttggcgttgtttgtgctttgggtttgctgagcaaataaccattactcggccttttcgtttaataatcttgcaatgttcacacatttttcgtactgatggtcgtactttcatttttaaccctcctcgaaaaaaaatgacgaaaaaggactacttaaatcgataagtaatacgtcccttggttaagtcgtaaggagacatttcaacagtaaccttatctccaggaagaatccgaatgtaatgcattcggatctttccagaaacatgagctagaatttcgtgtccattctccagttcaactctaaacattgcattcggcaatgtttctacgacttttccttcaacttcaataacattatctttagccactcaatacacctccaatgttaaattagattgaataaattaaattaatcttgacaaacctttgacagtttaacacattcattatatttcatcaatctaaccgactcaacacttaattagtgaggtttagagtgtgctcaagattttgtcaacatcttgccaaacttcatcaatgtctttgctgccatcgacattgaataaaagatttcgatccttatagtatgcgatcaatggtgtattcatcttaacgttaaccttaagacgatttttaacagcctctggtttgtcatcctcacgctgataaaattcatgcccaccacagacatcgcaggtaccgggaactttaggcatatggtacaacttatgataagtggcaccacagtttttacagatgaagcgacctgacaaacgctcagtcaacaacttaggatcaacatcaatgttgataacggctgtcaaaggtttatccaagtctttggtcatttgcgacaacgcatctgcttgttccaaagttctgggatagccatctaataagaagcctggtttagtatcatcttgggctaatctttcctttacaatcccattagtcacttcatcaggaactaaatcccctttatcagtaaaggatttcgccttaaccccaaggggtgtactatttgaaattgcatctcggaacatgtctcctgttgaaatgtgaggtacgtgatacttgtccacaataaattgggcttgagtacctttccccgcaccaggtaatcccattaatatcaagttcaatgacattttattgtcctcctaattaatagcggaattgctcaaatttagtcatcagttggtcgagtatcatgaatgaagccaacgtactctcgcttcatcattaaaccacgaatctgacgaattgtttcaatagcaacaccaacaacaattaacaggctagttccacctaacccaattgattcatctaagttccacaggttttgcgcaatcaaaggaatcaaagcaacaaccccaaggaataacgcaccgactgtacttagcttcatcaacagatcagacacataagattgggtctcatgccctggccaaacaccaggaatgtaactgccttgcttttgcaaattctccgaaagcttttccgggttaacttgaacaaaggcatagaagaaagtgaacatgataatgagaattgtatagaaagctgcaccggtcggcgtttgcatattgaatagattattcaatacctggaaccaagttgcagttgagtaattgttagtgaatgccatcaagatagtttgcggcgttgcaataaatgaacttgcaaagataactggaataacaccagcaacgttaaccttcaatggaaggtaactgctgtctggggatccagaaactcgccttgtatattgaattggtactcttcgttcagcttgttgaacccaagtaacaaaggttacgatcactaacacgattatcagcaatgcaatcgcaaaaaggattggttgccatagatcagcgccagaaacgccaacaaaatactgggtccacaatgactgaagtccgactggaattcgggcaatgataccagcaaagataatcattgaaatcccattccctaagccacgctcagtaatcatgtcccccatccaagttgttaacattgttccaccggttaaaatcaagccgatgatcacaaatgttttgatacttggattttgaacaagattcagactacttaattgattaaatcctgcggtaattccaacggattggaaaaaggctaggatgacggttaagtatctcgtatgttgatttaatttacgacgaccaacttcaccttgcttaccccattcaacatattttggaacaatgtccatctggagcaactggatgataatttgtgcagtgatataaggtgagacccccatcgcaaagatggaataattagtcaacccaccaccactaaaggtgttcaggatactaaccaaaccagaagatgcaacggatgttaatgctttggcattgatcccgggaacagttatgtatgctcccagacggaatataactagcacaaacaaagtaaaaagcattttattgcgaatatccttcactttgaatgcttttgctaaagtcgaaagcattaaaccacctcgattttaccgcccgcattttcaattacggattgtgcagcctttgaaaacttgttagccttgacggtcaactttttagtaagttcaccttcaccaagaatcttgatgcctgatttggcattcttaacgagtcctgattgttgaagtaattcaggcgtaacttccgtaccgttgtcaaagctttcaagcttaacaacatttacaacagcatattccttgcggttgatgttgttgaatccgcgtttaggaattcgacgatacaatggcatttggccaccttcgaaacctacacgagtcttgctacgagctttttgacctttttggccacgaccagcagtcttacctttaccggcagaacggccacgacctttacgagtacgtaatgaacgagaaccttcatcagccttcaattcatttaatttcatgaaattggcacctccttactaatttttagtctttaacttgttcaacttcgattaagtgagcaatttggaaaagggctccacgaatagattcgttgtctggtttaacaacggtactattaactcgacccaagccaagtgccttcacaattttacgttgctttggaaggcgatgagttacgctacgttttaaagtaatttttaattgagccatctaaaacaccctccttattcagctaaatgttgggttgaaaccccacgtaaagctgaaatttcttcagcactcttcaactcaaccaagcccttgaatgttgcccggataacgttgataggagtattggaacctagtcgtttactagtaacatcgtcaataccagctaattccatcacggaacgaacggcaccaccagctgctactccagaaccttcttcagcaggcttcaataaaattcggccgccaccaaatgttccgagaacttcatgaggaatcgttgtaccaacaatcggaacctcaattaagtttttacgagcagcttcaacggctttacggattgcttctggaacttcttgagctttaccagttccaaaaccaacatgaccgtgcttgtctccaacaacaactaaagcagcaaaacgaagacgacgtccaccttttacaactttagtgatccggttaatcgaaactacgttgtcttcaagctctaacttatctggatcaataaatttcttcatgtgcggttattcctcctttttagaattctagtccattttcacgagcagcatctgcaagagcttgaacacgaccatgatacaagtatccaccacgatcgaaaacaacatttttaatgttcttttcgctagcgcgttgagctactaatttaccaacactagctgcttgttcagtcttgttaccactactgattgcagaatcaagtgttgaggcactaacaagcgttacaccctctacgtcatcaattacttgagcgtagatgtttttattagaacgataaacattcaagcgtgggcgctcggcagtaccagaaattttattacggacacgattatgacggcgtttccgattcttattcttatctggtttagaaatcaaaatagtcacctcaaaattttattaggctggcatcttactacttaccagtcttaccttccttacgaataatatgttcattctcataacgaatacctttacccttatatggttctggtgaacgtactgaacgaactgatgcagcaaagtcaccaactgcttgtttgctgataccattgatgtgaatcgttgtgttatcaggaacttcaacagttagatcatctggaacagtcatttcaactgggtttgaataaccaacgtttaatgtcaggttcttgcccttaagttgtgcacgataaccaacaccaaccaacttcaaagtctttttgaagccagtagttacgccatcaaccatgttgctgacgttggcacgagttgtaccatgcaatgcacgtactttgtcgttgtaatcaccaatgggctcaaagttaacttcgttatctttgatagtcatcttgatttgtgatgaaatctcgcgggttaaagatcctttggcacctttgacagttacagtattcccatctgcttttacctcgacaccttttggtaattcgatggttttataaccaattcgactcattaattacacctccgatttgatgaattttaccagacgtaagctaacacttcgccgccaattttttgggcgcgtgcttgcttatctgtgatcacaccatttgatgtggaaatgatagcaattccaaggccatttaaaaccttgggaacagcatctgctttaacatacgaacgtaaacctggcttagaaattctcttaagaccagtgatgacacgttgcttatccttgccatactttaagaaaacacggataatgccttgtttgtcatcttcgatatattcaacatcgcgtacaaaaccctcacgtttaaggatttcagcgatgtcacgtttgatttttgatgcaggaacttcaactgtttcatggtaaaccatgtttgcattacgaatgcgagttaaaaagtctgcaattggatcagtcatagacatcagcgcacaacctcctttttaattattaccaactagctttcttcatgccaggaatttgacctttgtgggcaagttcacggacgcataaacggcataaatggaatttcttgtatacagaacgaggtcgtccgcaacgttcacaacgtgtgtaattctgagttgagaacttagcagggcgttcactttttacaattaatgattttttagccaatgtgaaacctcctctttatctggcaaacggcataccgaattgagctaacaattcatgtgactcttcatcggtatttgcagtagttacaatgacaatatccaaacctctaacacggttaacattatcgtaattgatttcagggaaaatcaactgttcacggacacccaaagtgtagttaccgcgaccatcaaaggcacgagtgctgacaccatggaaatcacgaacacgtggtaacgaaacgttgactaacttatctaagaagtcatacattctgtctccacggagtgtaactttagcaccgattgacattccttcacgtaatctaaatccggcaattgacttcttagcttttgtaaccaatggcttttgacctgaaatcaatgctaattcagaaacggcttcatcgaggttcttggcgttaataacagcgtctccaacacccatgttaagaacgattttatcgatcttaggagcttgcataactgatttgtagctaaatttatccatcatatgtggtgtaatttcgctattgaatttttctcgtaaacgacttgacatttaaaaggtatcctcctttcgctagtgattaatcgatcgctttttgcgatttctttgagtaacgtacttttttaccatcttcaactttaataccaatacgagttggctcgttggttgatgggtcaattagcataacatttgatacgtgaattggggcttcagcatcaacaattccaccttgtggattcgtctgagaagcttttgtatgcttcttaactttgttgattccttcaacaatcacacgatcttttgaagcgatagttttagtaactgtcccttccttacctttgtccttaccactaataacacggactttgtcaccagttttaatgaacatctacggcacctccttatatcctggttgtgattacagtacttctggggctaatgaaacaatcttcatgaagttgctgtcacgtaattcgcgagcaactgggccaaagatacgagtgccttggggactcttgtcatcacggataagaaccgcagcattttcatcaaaacgaatgtatgaaccatcattacgacgagtaacagccttagtacggactacaacagctttaacaacgtcaccctttttgacaacgccacctggtgttgcttgtttaaccgtagcaacaatagtatcgccgattccggcataccttctggttgagccacctaaaaccttaatagttaacaattctcttgcacctgagttgtcggcaacttttaaacgactttcttgttgaatcacaggtatatcctcccttcatcattggatcgaatacgataataatgataattaagtaaagttaaataataactgctttttcaacaatcttgattaaacggaaacgttttgtctttgacaatggacgtgtttccataatttgaacaagatcaccggttttagcttcgttattttcatcatgagccgtaaatttctttgagtatctaacacgcttaccatatgttgcatgtttcttgtaggttgaaacttcaacagtaattgtcttatcactcttgtcagaaacaacgcgtccttgataaaccttacgctggttacgttcttcagccattaattatacctcccttatcgtattctatttgttgagttcttgttgacgaagtgcagtcttaatgcgcgcaatgttcttacgaacctgcttcaagcgtgcagtattctccaactggccagtggctaattggaaacgaagattgaacagttcatctttgtaatctttttctttatcaatcatttgagcagtggttaacttgctgatatctttagccttcatttgattcgccacctacttcctcacgttctatgatcttagtgcgaacaggaagtttgtttgatgcaaggcgtaatgcttcatgggcagttgctttgtcaactccaccaatttcgaacaatactttgccacgcttaactggtgaaacccagccagctggtgtacctttaccattacccattcgaactccgacacctttttcagtatatgatttatgagggaaaatcttgatccaaacttttcctccacgcttcatgtgacgagtcatcgccacacggcatgcttcgatttgacggttagtgatccaatgagaatcaagtgcttgtaaaccgtattcaccgaaagtaaccgtcttgccacccttggcagtcccacggagcttgccacgatgttcacgacgatgctttacacgtttaggtactaacatgtttatttccctcctttagcagcgttgctgtcctttggcttttcagggagaacttcaccacgatagatccaagtttttacaccaattgatccataggtagtaaaagcttcaacccatgagtagtcaatatctgctcttaaagtatgcaaaggaacagttccatctgagtatgattcaacacgagccatatcagcaccgttcagacgaccagcaacctgggtcttaattcctttggcaccggaacgcattgtacgttgcattgcttgacgcatagcacgacggaaagcaacacggccttcaagttgacgtgcgatgttttcaccaaccaacttggcatccaaatcaggcttcttgatttcaatgatgttgatgtgaactctcttaccagtgaggtcgttaagttctttacgaagattttcaacctcagatccacccttaccaatgaccattcctggtttggcggtatgaattgaaacattaacgcggtttgctgcacgttcaatttcaacagtagaaacagacgcattagcaagacgcttctctatatatttacgaatttgcaaatcttcttttaagtaagctgcatagtctttacctgcataccacttagcttcccagtcgcgaatgattccaactcgtaaaccattaggatttatcttattacccacgcgttatccctcctctttttctgatacaacaattgtaatgtgacttgttcgcttgttgattggtgaagctgaaccttttgcacgaggacggaatcgcttaagcgttgggccttcgttaacaaatgcttcacttacaaacaagttttcactatctaaatcaaaattattttctgcattagcaactgcagatttaagaacttttgaaactaccggagaagcaccgcggggtgtgaaatccaagattgcggctgcttcagcaacactcttacctttgataagatcaactacaagacggaccttacgtgcggcaatgcgaacagttttggcagttgcttttgctgatgtaacttgttcagccatttgttatcctccttgttattaaacagtcttcttatcgtcagttccatgaccatggaatgtacgagtgggtacgaattctccgagcttatgaccaaccatgtcttcttgaacatatactgggacgtgtttacgaccatcataaacagcaaatgtatatccaatgaagctaggaaaaatcgttgatcggcgtgaccaagttttgataacggcctttttatcttggtctttttgggcatctaccttcttgagtaagtactcatcggcgaatggtccctttttcaaactacgactcattttgcaacctcctctgcacagatattaattgttattaataaatgcgttctattacatctttgaacctttacgacgacgaacaataaacttgtccgaacgtgctttcttagaacgagtcttcttaccaactgtcttcttaccccatggtgataatggtgatggaagaccaactggtgctttaccttcaccaccaccatgagggtgatcgttagggttcattacagatccacgaacatgaggacgttgacccttgtaacgtgtacgaccagctttaccaacattgataagttcatgttcttcattacttaccgaaccaatagttgctcggttagtgctaaggattaaacgaacttcgccagatgcaagtctaacaagtgaatacttgccatctcgaccaagcaattgagcagatgcaccagctgaacgaacaagctgaccacccttaccaggcttaagttcaatgttgtgaataattgtaccaacaggaatgttggataatggcaatgtgttaccaggcttgatatcagcatcaacgccagattcaaccttgtcgcccacctttaatcccttaggtgcaataatgtatgatttgattccgtcagtataaacaatcaaagcaatattagcagtccggttaggatcgtattcaattgctttaactgtggctgtgacatcatctttaattcgcttgaagtcaataatacgatattgattcttgttaccaccaccacggtgacgaacagtcatatgaccgtaattattacggccggctgttttactttttgattcaagtaaagacttttcaggcttacgcttagtaattgcgctgtagtccaagcttgtcatattacgtctaccattgctggttggcttatatgttttaatggccaaaacgtgttcctcctatattagagatttgtttgattattcttcgttgaataattcgatttcttttgaatcttcagtcaatgtaacgattgccttacgacgcttcttagtgtaaccagcgtaacggccttggcgcttgagcttgccacgaacgttcatgatgtttacacggacaactttaacatcgaaaatgtcttcgatggcctttttaacttgggtcttagttgctcgtaaatcaacatcgaatgtgtatgtcttgtcgtccatcttactggttgtttcctcagtaataactgggcgtaaaataatatcgcgtgattccattatgcgagcacctcctctacttgagaaagagcagctttcgtaataacaactttgtcgtgatcggcaacatccaaagtgttaatgccttgagcagaaacaactttaacgttttccaaattacgagcagatagaactgccttttcgttgtcgtcttccaaaactactaatgtcttagttgaaacgtctaatttacctaataattcagcaaattctttagtcttaggtgcatcaaattgtaaagtatcaacaacaaccaatttgttgtcggaaaccttttctgataacactgacttcaatgctaaacgtgaaaccttcttaggcaaacggtatgagtatgaacgtggagtaggtccgaaaacaattccaccgccacgccattgtggtgaacgaatagaaccttgtcgagctctaccagtacccttttgacgccaaggcttctttccaccgccgcgaactgcggaacggttcttaacggaatgagttccttgacgtaaagaagcacgttgcataacaattgcgtcaaacacaacattgttgttaggttcgatgccgaagataccatcgtttaatgcaacggtaccattcttgcttccgtcttgtttatataatgctacgtcagtcatctatggttgcctcccttctagttgtttgagccgtgaacggcacttctaattgtgatatatgatttatttgcaccaggtacattacccttaattaagagaacattgttgtcagtatcggcatttacgatctccaaattttgaatggtaacggtcttgttacccattcgtccaggcaatttcatgccaggaacaacacggttaataatgacaccgagtgaacctggacgacggtgataacgggaaccatgagtttctggtccacgtgattggccgtctttatggatgttaccttggtatccatgaccttttgtggttccagttacatcaacgatgtctcctggtttaaagatatctgctttaacttcatcagatactttatagtctcccagctcaacatctttgatttctttaatgaagcgcttaggagtcgtatttgctttctttgcatgaccttgttctggcttattagtaagcacagtacgtttgtctgcataacctaattgaactgaatcgtaaccgtcattttcaacggtcttgatttgcataatgacattaggtgtcacttcaacgacagttactggaactaactcgccgttttcggtgaagacttgcgtcattccaactttctttcctaagattccttttctggtcatgagtacacctccgatatattgtatttattatagtttgatttcaatatccacaccgctaggcaagtcgagcttcattaatgagtcaactgtctttggcgttggatttaaaatatcgattaatcgcttgtgagtcaaaatttcgaattgctcacgagaatccttaaacttatgtggtgaagctaaaacagtgtagattgtacgatcagtaggcaatggaattggacctgagatagtagctccagttctttgcgcagttgcaacaatcttgtctgcggattgatcaaggatacgatgctcgtatgccttcaatcgaatacgaattttttgttttgccattgtgttccctccttcgtctattttgaaaataggactaactccgtgaaaattaccgccaaacccatggcaaagcatccgggtgtgtcgcaacctttcacatcaaagctaatacatattgctttagggcaaacttatccctaaaaacaagtactcaaacagtgtactaaaaaaagccgcataaaacaagtgttaacagcaattaattcgttttgtaacattactgttacttgaaaaatgattttaacttcttttgatattcaaatgaacgtaaataacttcaaccaatttattatacattgccgtgggatgatttgacagacctttagtcaaaaaaagagaccgggattaaattccgatctctacgtttgaaattaatcttcagcaggttggttcccaccgtttttcttaataatttcagcttggatgctctttggaactggctcgtaatgatcaaatgtcatggtgaaagtaccacggccttgtgatgcagaacgaagtgtcgttgcataaccgaacatttcagcaagtggaacgaatgaatgaataacttcggcaccgcttcggctttccattccatcaacccgtccacgacgtgcagtaacttggcccataacatcacccatgtactcttcagggacgttgatatcaaccttcatgattggttccaagattactggagcagcggtcttggcagcattacgaagagcgattgaagcagctaccttaaatgcagcttcactagaatcgacttcatgataactaccatcatataacttggctttcaaatcaattaatgggtaaccggcaagaacaccgttagccaatgattctttcaaaccttgttctacggctgggatgtattcacgaggaacaacaccaccaacgatggcatcttcgaattcgaagccttttccttcttcgtttggtgtaaattcgatccaaacatcaccatattgacctttaccaccagactgacggataaacttaccttgagccttggttggcttggtaaatgcttcacggtatgaaacttgtggggcaccaacagtggcttccacatggaactcacgtttcatacgatcaatgatgatatccaaatgcaactcacccattccggcaattaaagtttcaccggtttcagggttggttgttgctttgaatgttggatcttcttcagaaagcttttgaagagcaacgttcatcttatcttggtcagccttagtcttaggttcaacggcaacctgaataactgggtcagggaattccattgattccaaatgaagtggatggtcaacatcagtcagtgaatcaccagtagtggtgttcttcaaaccaatggcggcagcaatatcacctgagaatacttctggaatttcttgacggtgatttgaatgcatttggagcaaacgaccaacacgctcacgtttgtctttagttgcattcaaaatatatgaacctgactcaagggtacctgagtaaacacggatataagtcaaacgaccaacgaatgggtcagtagcaactttgaaggccaaagcagcaaaactggcgtcatcattagctttcaattcaatcttgtcaccggttgcaggatcagttgcattgtatggcttaacatcaagtggtgatggtaagtagtcaataacagcatccatcaacatttgaacacccttgttcttgaaggcagatccagctaatactgggaacagttccaggttcaaggtagctttacgaatagcagccttgatttcaggaattggaatttcttcaccctcaaggtacttgttcataatgtcgtcatcaacatcggccaaagtttcaactaattggtcacgacgctttttagcttcatccttatattcatcaggaacatcaactgtatcccaatttgaaccaagcttatcttcatcgtagatgtcggccttcatttcgattaggtcaataaccccttcgaaatcatcttcagcaccgattggcatctggattggaagtggcttagcgttcaaacggtcttcaattgagccaactgagaaatcaaagttggcaccaactttatccatcttgttaacaaagacgatccggggaacgtcataatcagatgcttgacgccaaacagtttcagtttgaggctcaacacccgcttgggcatccaaaacagcgatagcaccatctaagacacgcaatgaacgctcaacttcaacagtaaagtccacgtgtcctggggtatcaataatgttgatacggtggtctttccattgagcagttgtggcagctgacgtgatggtaatcccacgttcctgttcctgtggcatccagtccatttgtgaagcaccatcatgggtttcaccaattttatgaatcttaccagtatagtacaggatccgttcggtcgtggtcgttttaccagcatcgatatgggccataattccgatattacgagttttttcgagcggaaactctcgtttgttagccattgtgtaactccttccgattcgtacaaaaagtggctaaatcagccacttattagtttgagctgtttagaaaaatcctgagattaccaacgataatgtgcaaaggcacggttggcttcagccattctatgtgtatcttcacgcttcttaactgatgcaccggtgttattagcggcatccatgatctcacgcgcaaggcgttcagtcatcgtatgctcaccacgtgaacgggcatagttaacgatccaacgcaatcccaaagttgttcgacgatctggtcgaacttcgattggaacttggtagttagaaccaccaacacgacgagccttaacttcaaggaccggcataacgttcttcatagcttcttcaaagacgtcaactggttcgttgttagtttctttcttaattaaatcaaatgcaccatataaaatttgtgatgcagttccacgtttaccgtctaacatcaaacggttaattaaacgggttaccaattttgagttataaattgggtcaggaagtacttcccgcttttgaacatttccttttctaggcatttcgttatcctcctcatgattctataaactaaatatttagattgcattagtaagattattctttaggcttctttgtaccgtattttgaacgaccttgacgacggtcttgaacaccagcggtatcaagtgcaccacgaataacgtgataacgaacaccaggtaaatccttaacacggccaccacggatcaaaacaacactatgctcttgtaagttatgaccaatacctggaatgtaagccgtaacttcaattaagttagacaaacgaacacgggcatatttacgtaaagctgagttaggcttctttggtgtcatagtaccaacacgagttgcaacacctcgtttttgaggggctggaacagtaacttgcttcttcttgaaactattgtaagcatagtttaaagctggtgactttgattttgaagttctagaatgacgtcctttacggaccaattggttaattgtaggcatctaaaaagttctcctttcaaattttcaatgtaagtccacacatccaggcggttcttttttatgtaaaaagaaatgtgtaccgcccaacactttttgtcatatacagtcagcatgtctgaatattcaggaatctgtcacaaaaagcaccttgtctaatttatcatgactggccgtttgtgtcaatgaatcatgttgaataatttaaatcgtaacaacgtacataaagtacagaggtaaaaattatgatgatcattattcaatttttgctgggtgcaagcctggcgtcgttttttaatttggttgctgttagacgacaacgcggggaatcgattgtcgctccccgctcccattgtgatcgttgtggtggtcagctgaagaattttgatttaattcctgtcttcagttacatcattttaatgggaaaatgtcgttactgcaaacaaaagttttcagcaaatttgttcactgttgagttggcggccggatctgttgctgcgagtttgaatctttttgagataaattgtctgtacgttggcatgttgattattttaatcgcactcagttcctttgacattgtcgaccaaacaattccaacagacggaattatcatgctgttgcttgtctgcggattatcaaacacccatccagtccaagaaattttgattgccattctgatctatctgctcatccaatttttaaaccaccacttttcctggatgggcagtggcgacatcgacatttatttttgcctgtggctggcactggatattccaagcttactttggcaaacgtttattgcttgcgtcgctgcgctgctttatttaattgttgcgccgtggccaaaagattccaaaattccatttgtgccattcatcaccatcggattttatttaacccaccaattccaatcaatcttattaccgttaatttcatagcaaataaaaaaaggattccaacccattgcaggttgaaatcctttttcaaattgattcattcaatttaatgattatttggtcgtcttgctcttgttagcatcttcagctttcattttttcttcaagctggctaattgagtaaacaccatcagttgatgaactaccaatttcttcaggcttaattccccggtaatctggcattccagtacctgcagggattaatttaccaatgataacattttccttcaaaccaaccagtggatcattcttaccacgaattgcggcatcagtaagaacacgcgtggtttcctggaatgatgcggctgacaagaaactatttgtttcaagagcagccttggtaataccaagtaagacaggacgggcagttgccggaattccaccattaacaaccgtgtcaccgttacttatcttgaagtcattgatatccatcaaagtaccaggcaatacatcagtgtcaccaggatccatgatacgaaccttacgaagcatctgacgaatcatgatttccacatgcttatcagccacttccacaccttgcatccggtaaactttttgaacttcatgaagcaggtagttttcagttgagagaacatctctaaccttcaacaattccttaggatcaacagaaccttcattgagagctgaaccacggtgaatgtagtcaccttcagcgactctcattcgagctgtgatcggaacggtgtaagttcgagtatcagattcacctttaatggtaatttcttttgttctttcagcaggattttcttcaattgactcaactgtaccagtaacttcactgatctcagctttaccttttggattacgtgcttcaaagatttcttgaacacgaggaagtccttgggtaatatcggcgttaccagcaacaccaccagtatggaagttacgcattgtcaactgggtaccaggttcaccgattgattgagcagcaacagtaccaactgcttcaccaacttcaacctcatcaccagtagccatgttacgaccataacatttctcacaaacaccatgaatggtgttgcaagtgaatgctgaacgaatcgttacttctttgattccaaggtcatcaatcttagtagcctgatcctcagtgatcatggtgtttgcaggaacaatcacatcgccagtcttagggttcttaacggttttgtgagcataacggccaacaattcgatcatacaatggttcgatcatttcgttaccttcagtaattgcactgatagtcaggccacgatcggtcccacagtccttttcacgaacgatgacatcttgagcaacatcaaccaaacgacgggtcaagtaacctgagttggcagtcttaagggcagtatcggtcattcctttacgagccccatgggttgaaatgaacatttccaaaacagtcagaccctcacggaagttggaagtaattggtaattccatgatttcaccgttaggagcagccatcaagccacgcatacctgccaactgagtaaagtttgaaatgttaccacgagcaccggaatcactcatcataaagatagggttctgtggatcttggttttccaacagacgcttttgaatgtcatccttggcatcattccaaataccaataactcgttcataacgttcatggtcggtaatcaaaccacgacggaactgcttggtaaccatatctacctttttatgggcgccgtcgataatttcttgcttatcaggcaactgtgtgatgtcggtaattccaacggtcaaaccagacttggttgactcgttgtaacccagatccttcattctatccaacaagaatgaagtttcagtcactttgtagatcttgtaaacttcggcaatgatatcacttaagaagcctttcttgaatggcaggattaatttggcattcttcagatgctcatgaatgtcctcacctggttcaaggaagaatttgtcatcaacataaccgttcaaattggtttctgaaggttcgttaatgaatggaaaatcttctggcaaaatctcattgaagacaatcttaccaacggaggttaccaaaatttttccaagttgatcctttgtaaaggtcttctttggatatgcggaagccttgattccaacacgtgtgtgccagtgaacgattccattcttaaatgccaattgtgcttcatcaggtgagttaaagatcattccctcaccttcgcggccggcttcctccatggtcaggtaatagttaccgataaccatatcttgagatggggtaacaactggcttcccatccttaggtgccagaatatggccggcagctagcatcagcaaacgtgattcagcttgggcttcatcagacaacggaacatggatagccatttggtcaccatcaaaatcggcattgtaggcttcacaaaccaatggatgaagacgcatcgacttaccacttaccagtacgggttcaaaagcttgaattcccaaacggtgaagtgtaggggcccggttcaacagaactgggtgttccttgataacatcttccaagacactgaaaacatcgtcatcttggcgttcaattttgcgcttggcgttcttaatgttggatgccaaattgcgaccaaccaattccttcataataaatggcttgaataattccattgccattggaactggtaatcccatttggttcatcttcaaatgagggccaacatcgataacggaacggccagaataatcaacacgcttaccaagcaagttctgacggaatcgtccctgcttacctttaagcatgtgagaaagtgacttcaatgggcggttacctggtccggcaactggacggccacgacgaccgttatcaatcaaagcatcaacggcttcttgaagcatccgtttttcgttttgaacgataattccaggtgcgttcaggtccagcaatcgtttcaaacgattattacggttaattacccgacggtacaaatcattcaaatcagaagtggcgaaacggccaccttcaagttgaaccattggtcgtaagtcaggtgggataactgggattgcatccattaccatccatgaaagttcatttccggattggacgaaagcttccaaaatatcgagtcgacgaacggcacgggtccgcttttgaccggttgcattcttcaattcatcttttaattcggtaacttctttttcaacatccacatcttcaagcagtgtcttgatggcttcggcaccaatttgagctgagaaccgaggaccatattcctgcttcttttcgcggtattcacgttctgaaagcaactgcttcttttccattggtgtgttacctggttcggtaacaacgtatgaagcgaagtaaatgatttcttcaagtgcacgagggctcatgtccaagacaagacccattcgacttgggattcctttgaagtaccagatgtgagtaactggagctgccagttcaatatggcccatccgttcacgacgaacctttgaacgggtaacttcaactccacaacggtcacaaacgattcccttataacggatccgcttgtacttaccacaagcacattcccagtctttggtaggaccgaaaatccgttcatcaaacaaaccatctttttctggttttaaagttcggtagttaatggtttctggctttttaacttcaccatatgaccaactacgaatcttatcaggagaggctagtccaatctgcatactttcgaatttattaacatcgaccactagtttgacctcccatttctagtcattactgttgttaacgttggttgatttacttggtgtttcaacttgatcggcaggttgtttagctgcatgatcttcctgctctttcttcttgtcagccaatttgctcaatgcgtcaacgttcacaacgtcgtcatcgtcatcaagatcacgaagttcaatctctttatgactcgcatcgagaaccttcatatcaaggcctaatgactgcagttccttaacaagaacccggaatgattcaggtacaccaggctttggaattggctcacccttcacaatggcttcgtaggtcttgacacggccaacaacgtcatctgatttataagtcaaaatttcttggagagtatatgcggcaccataagcttcaagtgcccaaacttccatttcaccaaaacgctgaccaccaaattgtgctttaccaccaagtggttgttgcgtaaccaatgagtaaggtccaattgaacgtgcatggatcttatcgtcaaccatgtgggccaacttaagataatgcatgacaccaacggcaatcttcttatcgaatggctcaccagttcggccatcgtacaagatgtacttaccatctgaaggcatgccggcttctttaactgcatcccagatatctttatcacgagcaccatcaaaaacaggtgttgcaacgtgaattccgagtctgcgggcagccattcccaaatggagttccaaaacttgtccaatgttcatccgtgatggcacacccatgggactcaacatgatgtcaactggtgttccatcaggcaagaatggcatatcttcttctggaataacaacagaaacagtacccttgttaccgtgacggccggacatcttgtcaccaacttgaatcttacgtttttgagcgatgtagacacgaaccatcttattaacaccaggtgaaagttcatccccgttttcacgagtgaagatcttaacatcctggatgattccgccgccaccatgaggaactctcaatgaagtatcacgaacttctcgtgatttctcaccaaagattgcatgaagcaaacgttcctcagctgataattcagtcacacctttaggggtcactttaccaaccaagatgtcaccatcatgaacttcggcaccaatccgaactgtcccgtcctcgtcaaggttcttcaaagcatcttcaccaacgttaggaatttctcgagtcatttcctcaggtcctaatttggtgtcacgagtttctgattcgtactcttcaatatgaattgaagtgtaaacatcatctttaaccagacgttcgctgatcgcaatggcatcttcgaagttgtatccttgccaagtcataaatgcaacaacagggttttggccaagtgccaactctccgccttccattgatgggccatcagctaagatttcatcagcatcaactcggtcgccaaccttaacgattggacgttggttgtagttcttaccgccatttgaacgacggaatttcattaatttgtatttatcaagggacttgtcgtcacgacgtactcgaatttcacgagcatcaacgtattcaacagttccttcattcttacagatcagggcaacaccagaatcatgagcagccttgtattcgataccagtaccaacaagtggtgcatgaggatcgatcaaaggaacggcctgacgctgcatgttggcacccatcaaagcacggttagagtcatcgttttccaagaaaggaatacatgcagtggccacggcaactacttgcttaggcgaaacatccatgtaatcgaccttgtcgataccaatttcaatgttgtttgacttgtgacgggccataacgatgttattgacaaacgaaccatcatcattcaatggtgagttggcctgggcaataacaaagttatcttcttcgtcagcagtcaaataatcaattcgatcagtaaccttatgagtggtccaatcaacacgccggtatggtgtttcaatgaaaccatacttgttaacccgggcgtaactggacaaactgttaatcaatccaatgttagggccttcaggggtttcaatcggacacatccggccatagtgggtatagtgaacatcccggacttcatatccggcacggtcacgagtcaaaccaccaggtccaagggcagacaaacgacgcttatgagttaattcaccaagcgggttggtctggtccatgaattgagaaagctgtgatgaaccaaagaattctttgattgaggcaacaactggacgaatattgatcaattgttgtggtgtcacagttgaagtatcctgaattgacattctttcacgaacaactcgttccatccgtgacaagccaattcggaactggttctgcagcaattcaccgactgagcgaattcgacggttacccaagtgatcaatatcatcaattgaaccaataccttcttgaaggttaaagaagtagttcattgctgaaatgatgtcagctggagtaatgtgcttaaagctcaatggaatgttgtcattaccaattaaaggaaccactcggtcaggatcgttaactgattgaactttaatgatttgaacagtcattggttcagtcacaacggcttcatctgaaggggtaaaggtgtaagctttaaattcatcgttatcaaggaatggtgccaagtccttcataacatctttcgtgacaacggtgcccttttgagcaatcacttcacctgtgtcaggatcagcaagggtttcagccaatgtcaaacctaacagacggttcttcaaactcagcttcttgttggtcttgtaacggccaacaggtgccatgtcataacgctttggatcaaagaaacgagcagtcagcaagcttcttgatgaatcagcagtcttaggctcacctggacgtagacgttcgtaaatatccttcagtgactcttcaacacgtgaatcgtcagtgtctttatgaacatctttttccaaggtcaaacctaaactgtcgttgtcgcccaagatgtcaatgatttctgaatcactgccaaagccgagggctctaattaattctgttaaaggaatttttcgtgttcgatcaattcgaacgtacgcgatattttttgcatcggtttcaaattcaagccaagcacctctgttaggaataacagtagtaccaaatgaatcacggccattcttatctttatcagcatggtaataaacgccgggtgaacgaaccaattgtgaaacaattactcgttcagcaccattaataataaatgttccttgatcagtcattaatggaaaatcgccaaaaaatacatcttgcgtcttaatttcgccagtctcatgattggttaattttaaggtaatgtgaagtggagcagaatagtttgcttcgtgttcacgcgcctcatcaacggtgtactttggtgttaataattgataatcgacaaactctaaagaaagcttgccctgaaagtcatcgattggcataatgccatcgaaggtttccttaagtccctcatgtaaaaaccagttgtaagaattagtctggatttcaatcaggttcggtaaatcaagcacttctttaattcgtgcataacttcgtcgggtacggtgttttccatatttaactaaatgtcctgccaagtttttcacctctccaaaaaattccggaatcgaaatgttacagtttgattacaaatgcactttttagcacatctgaccgggttttgggcaaaaaaaatccaaaaacaagactttcttgcttttggctttttatgcaggccaacccggacaatagatcgcgtcgaccatttcgattcacaacaaatacagttaaaagaataacaatttatagaagtaaagtcaaccttttagaccatggttcagtttgaatcgcaatttattttttatcattcactaaagttttgcgttccggcttcttcactgaaatggtaatctggttgtttctaccgccaacagtgactgagtcgccggggacaatttccttggcaagcaacttggcactcaaattatcctcgagttcagtttgaattgctcttctgattggacgagcaccgtactcagggtcaaaaccacgcttggaaataatcccgattgcagtcttggtaatcttaatgtcaatgccttgatcgtgaatccgcttgataaccggtttggccatcaggtaaacaatttgatcaagttcgtccttggtcaatgagtggaagacaaccacttcatcaattcggttcaggaattcaggacggaagcgttgcttgagggcagcttgaatcgtgtccttcattgctgcatagccttccttggcatcctcttgaccaaatccaacggtcttcttatcccgcaatgtggttgcacccaggttggaagtcatgatgataaccgtgtttctgaaatcaatctttcgacccttggcatccgtcaagtaaccatcatcaagaacttgaagtaagaggttgaagacatctggatgagccttttcaacttcatcaaaaagcacaactgagtatggcttttgacgaaccttttcggttaactgaccaccttcatcgtagccaacgtagccgggagcagaaccaatcagacgactggttgaatatttctccataaattcactcatgtcaactcgaatcatgtcttcttcagaaccaaagactgcctcggcaactgcctttgccaactcggttttaccaacaccggtcggccctaggaacatgaaggaaccaattggacggttcggatctttcaaaccgcttcgagcccgacgaattgaacgagaaaccgctgaaattgcctcttcctgaccaacaacccgcttgtgaagaatcttttccaagttgactaagcggtcagcttcggtactgctcaaacgagtaaccggaatcccagtccactcgcccacgatttcagcaacgtcttgtggcgtctctttgacggggtaatgtgcatcctctgagccttcctcggaatcattatcttgagcaagttcatcctgtaactgattggtttgtttgcgaatcttagcagctttttcgtaatcctgggctaccaaggcttcatttaattctgataacaaatctgagagtttcttatgatcatcaacggcatcagatttttgaaggtgatcaattcgaactttggcagctgcctcatccattaaatcgatcgccttatcaggtaagaatcggtcgctgatgtagcggttggaaaggttaactgcagtttcaatggcgtcatcagtaatttcaacgtggtgatgttgctcgtattttggccgtaagcctttgagaatttccaccgtttcatcagtcgttggctcatcaaccataactttggcaaatcgacgctccaatgcagcatcggattcaatgtacttttggtactcgtccaaagttgtggcaccaattaattggagttcaccccgggccaatgccggcttcaaaatgttggaagcgtcaatcgcaccttctgcaccaccggcaccgatcaaagtgtgtaattcatcgatgaacagaataatgttgccatcttggtaaatttcatcaatcactttcttgagtcggtcttcaaattcaccacggtatttggtaccggcaaccagtgagcccatgtcaagcatcatcagacgcttcttggacatgtcaccaggaacgtcgccgctgacaatccgttctgccaagccttcagcgatggcggtttttccaacaccgggttcgccaattaaaacagggttgttcttcgtccgacgagctaaaatttgaaccacacgtttaacttcgagatccctgccgacggttgggtcaagacggtcttgacgggccatttcagtgaggtcacgagccaatgaatcaattgttggtgtctttgagtcagctggcttttgttgacggccacgttgtttggaagccaggtttgaggccattgagccaccactgatgcccatttttcgaagggttacttttctaatttgtgatagatcgagtcccaagttaatcagaatacgggaagataaaatggtctcatcagtcagaagtgaaagcaaaatgtgctcggttccaacctttggaacaccgttcttcttggcgaattctcctgcttgagccaaaacttcctttgcctttggagagtatggtagataatcgttactgctaaggtccttaaggttgccatagccggcgaaacgctctacttcttcagtgacatcttcggcagttactgaaaactgctgaagcgccttgtaggcaattccattcgtttcgatcagtaagcctaatagaagatgttcagttccaattgcttggtgcttgaatttcttggcttgttcttgtgcaatggtcaaaacgttcttagcactcggagtaaataaattattcatagataccctctctttctatcgttcgtatcgcagccggttcaatatcgacaccatgatgttggcacgtaaaatgtcggttaaatcgctgttattcaggtcaattgcatctttgtcaatcgcagctaatatgatgctcacctcgcgacgattaattaattcattattatataacgtttgaacgatcgtttcactatcccgcttcgataatttgttaccaattgcggcaattaatgaattcaaaacgtcaatgtcatctaataaatgaactttttctattctaatgtagccgccgccaccacgtttactttccacaatataaccattctggatcgtgaaacgcgtgttgattacatagttaatctgagacggtacaacgtcaaacagcccagcaatttcagaacgacgaattttaacctgctcgttctcggcaaggatttctttgagataatgttcaattaaatcagaaatgttttcgtccgccatgtaatcacccaattctttgactaatattgactattattatacgaatgtgacggcaaagtgcaaggaaagtgtttgagagcgcgacgaaccccggttagagtccggagcataagtgaagagattcaaggatgaacggtccttgttcatctttgaatctcttcacttatgcagtaggactctggggtgtcggagcgtattttcgaagcgggataaagcagaaagaagcaaaacgaacatgccctagaggaaacatcaatggtgaacgaaccttgttcatcgttgatgtttccgctttgtgtggtaggggtcaagggcatcggagcacgtttataatccggatctcttcacttatgcagtaggactctggggtgtcgaagcgtattttcgaagtgagataaagcggaaagcagcagaacgaccgtgcacctaacactatgcccctccgatgcagagagactttcgaaataatccattcatggtggcaaaaaggattaaaacatcaacaccagcaaccgggattgccgttcgccgagatgtcaaaaaaaggccagacccaaagtacagttctgacctcaaacacgattcaattaatatgtaatttcccacaaaaaaatcgggaaaacaagatttgaacttgcgacccctacgtcccgaacgtagtgctctaccaagctgagctacttcccgatgatttaagtactattgagttaacaatataaatataccatatgatctatgttaaacaaagtcgggaagacaggattcgaacctgcgaccccctggtcccaaaccaggtgctctaccaagctgagctacttcccgaaaaggaattcattgcaataaaaaatgcacccagtaggagtcgaacctacaaccttctgattcgtagtcagacactctatccaattgcgctatgggtgcataataagtattaaattaaggaacctcaatcatagtacttgattgaagcggaagacgggattcgaacccgcgacccccaccatggcaaggtgatgttctaccactgaactacttccgcaaaatgccgactagacgattcgaacgcccgacctcttcattactagtgaagcgctctaaccaactgagctaagtcggcaaaatgtataaattgttaggtaactagcacctatgcgggcgaagggattcgaacccccacgtcataagacactagaacctaaatctagcgcgtctgccagttccgccacgcccgcattgttaaaaactggcaatgagccgtggcagtctcgaactgccgaccctctgattaaaagtcagatgctctaccaactgagctaacggctcaatggaggatacagggatcgaacctgtgacctcctgcttgtaaggcagatgctctcccagctgagctaatcctccatgaaactaaatgaatcaaatgttggtagcaacatcatcaacacaactattaaattttacaataccaatcaactcaagtcaagatgaattttaaaaaatcctgattggttagccgttagttaataacgtctttttccgacaaaaaatattatatcctatctcggaaaacattgctagtccaattttgaattaattgcatttttattcgcgacaaataaaaaggcgaaggacagtcagccgtccttcgccttgctcctggtacgatgatcacacccacattcaaaattcatcatgcagtgggaatgatttcattcaaaaactagttttgcttttcaattttagtcatgccgtgcatatatggccgtaatacttctgggatcgtgacagtgccatcttcattctggtaattttccagaatggcggccaccgttctgccgactgccagtccagaaccatttaaagtatgaacaaagtgaagtttcccttcatcatcccgatactggatgtgtgctcggcgtgcttggaagtctgtacagtttgaacagctggagatttcccggtacttatcctgggctgggaaccaaacttccaggtcgtgtgtcatagcggctgtgaaactcatatcactggtcgtcaatgtaataacgtggtaagccaacccaagtttttgcaggttaacttctgcttggtgggtaatctcttccagtgccttccacgagtcttcgggcttggtaaatttcaccatttcaaccttgttaaattggtgtaatcgaatcagccccttggtatcacggcccgcacttcctgcttccgatcggaatgctggcgacaaggccgtaaccgataccggcagcttttctgtcggaataacttcattgcgataatagttaaccaatggaacttcggcagttggaatcagggttaaatcactgtcctgaatctcatagccggatttgttctccaaaaattttggaaattgcccggtgccatacattgaatcgttattaaccatgtaaggtggaattacttcggtataaccggcagcggtattttggtcgaggtagaagttgtaaacggcccgctccaataaagccccgtcgccaatatagtaaacaaatcggctgccggacactttggcagcccgttcaaagtcaagaatgccaagattttcaccgatttcccaatggtgttttggttcaaaatcaaatgacgggatctgcccaatcttacgaagctcaacggatccttcttctgtgagtgacaccgggacatcatcatgtggaatatttggtagatgggcagccaaattgtgttcatcttcctcaacttgccgcaattgctcgtcaagttccttaatccgttggcccacctgtttcatttggttgatggcctctgttgcatcctctttattgcgcttcttttgtgaaatctggtcagaaacggcgttccgttttgctttaagtgactctgattcaacgatcagatcccgacgtttggcatcgtagcccactaattcatcaatggtttcgggcttgattccccgcgtagcgagcttttctttggtaaaatctggatcttttctgattttcttaatatctaacatttcaaatcctcccaatctgtatacaaaaaggacccctcgtctatgggacgaaggatccttttcgcggtaccacccaagttctcgacaatcttgccaagctctcaaagtatggtaacggcatacaccgtgcagcattacctgcccgttcacttgtgctggaatattcgatgacagttcacaccaaccactgtctctctgaaatctacttaataggcacaaaacgttttatctgaaatcgattataacgaatcaatccctaaaccacaagagcggtctgaaattaaattgccaacttatccactttggcgtcgattagatcgatcaccttgtgcttatcagcatcattttcaacaaaatcatacttgtcaccgtcaatttgaatcttaggtgatttgtcatattcttggtaccacgtctggtagcgggcattcaaatctttatagtattggtacaaatcgggatcattatcaatctgctcataggaacggccgcgcttttgaatccttcttaacatcgtttcaaacgagatgttaatgtggatcaataaatcggggttcttgctgtgatcggtttgtggcatctcctgcatcatgttctccagcaatgagtcgtaaatcgtcacctcagtttcggtggcccggcccaagtcggcattcaaatggaagagtagtgaatcctcaaaaattgaccgatccaacacactctcatcattttgccaagcttttttgatgtcatccattcgacgatttaaaaaatcaatctggagcaagaaggcatacttcttgggatccttataaaacaacggcagaatgcggttgtgttcaactgattcataataggcgggtgtgcccaaatgttgtgacagcatcttggtcagtgatgtctttccggcaccaatcgttccagcaagtacaagcataattattcccctaacgtttttgcgtgcaatcatcgcacaatattttatcaacgctacatattgtactagttagaagagataggtgcaacatattgtggaaatttagttaatgtttgagacgtcaaccacttggatgttgtccaaaccaccgtacgcttcaaaccacggtgtggcattctcagacaagatctgggttaattcagtgacgtttctggttcccttgcgtttgagccagtcaaccaggccgtctttaccgtcacgaatgtaaatgtcgacaccttccaaccaagttgcccgaccgcttaagacaccgttaaacttggcaccggcatctccagccagcttcaattcccgttggaaaacaggggtcggcactccggcactcaagaaaataaatggtcgggtcgcctcgtcgctcaactctttgagatagcctttggcttggtcttcggtgtaggcgtaatcgccaccatcagcccattctttgacgtaggtcgggttaaatggaatttccatcttcaaaacgtcaatgtgatatttctccttggtgaattccatcattgactgcaacaccagatcaggcttgatcttggcaaaatccaacgacttgctgtcgtaacggtcgtcgtaagtgacaatttcaaagaaggtcggcgtctgagctgccaaaccttccgtcccgtatcgttcagcgaacgcttttttgacgtcattgatttcatcagggtcgttaggattgtagtaaaccaacactttgagggcatctgctcccttctcaaccataatttgagctgattgatcaggaatcaagcttggtaatcgtcccggggtgtcggcatcgtatccggtcttttcataagacataatcagaccggtgtctttagccttggcctggatccccttgaaacccatttgctcgtccaaaagcacggcagaactcagtggactcaggatttcagagacaatctccttgaaatcatagaccatcttcatactgaaaagctttccgtatttttcggaggccgttttcatccccttaaccagcgatccacgttggtctaacgccaatgcatcgataatgttctgatcattggacaatttgttcattctttcaaatttaccttttgacataaactttttcatatatctttcacctcatatttttaatataccaattggtaaaattgtaccaaacattatgcccaaatatcaagttttaggctgataaaataataaaaattggcccatccaagacggatagaccaatttataattaatatattacttgttgttcaattttgaaagatcctcgtctttatgggccggggaaacgtcaacctgatccagcggaatgattttcgtatggtgcttgagcttataccaaaagtacaaaatcaataccagcggcacgctaatgtaagtgaccagaatctgcttccagtcaaagcttgcaaaggcctgtggattttgaccgacaatcaccagaatacacagaatcaggcacagtacaggaccgaacgggaagagcttggcatgatacttgagttcgctgaggtcatggccctggcgaatgaacgcccgtctgaatcggtaatgtgaaatggcgattccaaaccaggcaataaagccggttaacccggaagctgccaccagccacatatagatttggggcccggcaatactggaaataaaggtcaatagcgaaacaaaagtcgttgccaataatgaataatatggaatcccattggcagccgttttacccagggattttggcgcatatccgctgttagacagtgaatacagcatccgggtagaggcgtacataccggagttcgccgatgaaataacggaggtcaaaataacggcgttcatgacactggcagcagcggccaaaccagcccgctggaaaaccaatgtaaatggactgatcgcaatgtcagtggcacttgatcccagcagtgaatggctggtgtaaggaataatggcggcgatgacgaaaattgtcaaaatgtagaacaaaataatccgccagaacacttcattaattgcctttggcacactgtgttggggatcttgggactcgccggcagtgatgccaaccagctcagttccttgaaatgagaacccggcgaccacgaagacactcaggattgccggaaaaccgccgacaaatggtgcctgcttaatagaaaagttacgcatgccgacaaaatggccgcccatgattccaaagatcgtcaaggcacccactaccaggaaaataataatcgtgaccactttaatggcggacatccagaactcggtttcaccgaaggtactgactgacatggcattaatcaggaaaataatcactaaggcaattgcactccaaatccaggcaggcacatttggcagccagaatttcataaccaaagcggcggtactaatatcaacagccaccgtaatcgcccagttaaaccagtaattccagcccatggcaaatcctaaggccggatcaacgtatttggatgagtatgcggcaaacgagccggaaatcggcatattagtggccatttctcccagactggtcatcaggaaatagaccatcatccccatcaggacgtatgccgttaaagcaccaccagggccggcttggctgatagctgaaccactggccacgaacagcccggttccaatacagccgcccaaagcaatcattgacacgtgacgggcttttaggccccgcttgacttgtccgttggcttcttggctctcattatcgttcatcttttcgtctcctatatccaataatttcaaaatctcactaaatctacaaaaaaatccctttcaaaatattgaaagagacagtttgcgtttctcaacatcttgatagctctccgcgattttcgcgacagtccccagcttcttaaactgggccccaacaaccagctggaaggcagctgatcgtttcggcactcatccctttttacttcagtcataacttccttcaagttcctgaaatatactcttgatgaatgcgcctctactcgattagattgattaatttagttgttaataacttcgacaatcaaaattgtaactcacttgggttgaattgacaaaccagaacgacttttctcactgcaaagccagctgataaatggtcttttctttgcccaccagcggatcaatcaatgttgtcttcacttgaaacccgaccttctttaagacgcccttagaggcttgattatcgctgaacacctctgcattcaacgtctcaatcgttgggttaacagcgagttcctcaattaatttagtaagggcttcagacatgatcccttgatgccacaggtctgggtgaagaaaataactcagttccagattggcaggatcgggttggtgatcaaaaccaacttgttcatataagaggattgccccgatcagtcgatcgtggatccggatgccaaaggagttaggcgtcgcaatctgtcttttggccactgcccccagcatttgttgattactgaccagattaaaaccggcgccggcggcaatttctggaatgctgattaatttttcgtaagccgttaagtcggccagagttaattcagtcagttgaagtcggttggtctcaatcggtaaatccatggcgatctcctttcaaaaaaatgcccaggaaaaatcctcggcattttcaatcagattttagtgtgaaccacaaaccggtagcgggcaactcggggcgcgtaactggcataaagcatttcagctaccaacagccaggaatagccaaccaggcaggctcccaccgtatcggttgggtaatgggcgttcaagtagaccctggaaagcatcaccagcgccaagacgatgacgagcagtactttgatcaccactcgaatggatgcccgctcaatcaacggcaggacgatgatccataacaccccggcgaccaggaaaaatcccaggacgtggccgcttggaaaactgtagccgttgtcgacacccagatgcagcggcggtcgatgccgtctaaccagttgtttgacgactgcgccaatcacgtcgccgccgactatcgtccctaatgcccaaagtgcgggaactttgtacttaaatccccaaaggaaaaaggcgatgatgaacacccagaaaatgtccattttcgggctggccagaaatgtgattactgaatagaaatgttccagtcccggtgtcggcgcggatccttgaatggccgttgtaaaaattgaatctaaaaattgcaaataatcaaaattaaacgctaccgaaattgacagcaaggtcgtaaaacacaaactcacaatcagcttgaccaaccggtttggatcgcgttccatcagcatgtaatcttcgtttccgtacattagttcaacaaccctctcgtatgtattactcaaaaatgagtatatcacaaatcgaaaacccggtttctggtttctgaaaattcttagctatcttttaattatttacagaaagtgtataatcttgtgagttagagatcacattttaaaggagtgaaagacttgataaactatgctttattgatgattgccattggcgtgttcgccgggttcgccggtgccatcctcggcctgggtggtggaatcatcttaacgccgattttgacattgttgatgggtgtcgacattaaatacgcaatcggtgccagtatcattgccgtgattgccaccagttccggagcgacaattgcctatctccgtgacaaagtgctcaatttgcgggtcgcgatgtttttggaaattgccaccactttaggggcattgagcggcgccttgttgaccggtgtgattgatccgaaatatttgtacatactatttggattattgctattattctcaggctacaatatgattcgcaaattaatcagtcaccaggaagtccttcatcgggctcatcccgatcaattatcgtccaaattcaagctggacagcagctacttcgataatgttgaaggcaaaacgatcaactaccaggttgaacacattcccggcggcttggcagtcatgtacggtgccggcattgccagtgggttacttggaatcggctcgggtgctttcaaagtcatggcaatggacacggtcatgaagatgccgctcaagccatcgacttccaccagtaatttgatgatgggcgttaccgcagctgccagtgcaacggtctatttcttcaacggctcgatcaaaccaatgatcgccgttcctttggcactgggaatcttggtcggtgcccgcggtgggtcacgaatcatgcgggatatgtcagcacggacgattcggatgattttcgttccgatcctgttttatatcggcatcgaaatgtttatgaaggggatcagataagatggacaaaaataccaaagaacaaatgactgaagaaatggccgacgtccaattgattatcggcaagattcttcggctaggggtcataatttctgcaaccgtgatgatcattggtttggtgcttttgattgtcaaaggtaacggcggctatcctcacaacgcctttcccaccgactttacccaaatttgggcgggaattgctgaactcaagccatacgccatcatgatgctgggaattttcctattgattttgacaccagtattgcgagtggtcgtctcaatttattccttctatcgcgaaggtgacagcttgtacgtttggatcaccacaattgtgctggtgattttaggaattagttttgtgtttgggattttaagataatcaattaacgatcaagaggcgctggcaagggaacattccctttgccggcgcctcttttgcgttgagtaacatttttaactctggtgaatcgtgacatcgccaacgtcgctggtaaatctgtaagtcaccggatttttggcattgctgtcaatcttcttgttgtgtgagctgccaaacaatgatgcatcgccaacatcggcactcactgaaatctgcgttcgcttgttcttaaccacatgtcctgaaatatcgccaacgtcgctgtgggcggtaaaagacttgccgaccttttgggaattaaaattaatatccccggcaccggtttcaacggacattgagtcaaatttattggacgtcagatcgacatcgccggcaccaacatcaagatgggcgctgggaaaagtgctggtcgataaatttacatcaccggtattctccaagtccaagttttcagtggtcgtcacgtgattcaaattaacatcgccgaccccagacgaagtgatcgtcttgatggtcatatttttgatggtaattgagttggcaatgtcactgttgatcgtaccgaccttcatgctttttggaacggtgatgatggtcttgccaaaggcctggcgtgctcggcgaaagtcaccaaagaagatgataccatggtgcttacgtggacttttcaaattgaaatgaagggtattgcctgattgcgtgatcttggtagcacttggataagtcacctcgattttagaaacgttacccttcttaatttgcaccggactggccgttgacaaagaaaagtttttcacgccggaaaatttggcactggtttggtgtgacttaaccggcgtggattgatcagttgtgaacccgtgatcccaatagaccgtgcgggcaccaccattgcccaggccgagcaccaacagaacagttccaaccagggtcacagttaatcccacgatgacagtttttttcatttttggtcaccctttccttttcgttcagcccggttcttcgggacaatcttgttataaatccatttcgaaaataacgtgataccacgaatcaggccgttgacgacggctttgaagaccggcaccagcataatcatgaccccaatgaccatcagacccattcccaaatagaaaatgcccgtccaaaacgaactaaacagggtgcccaatccgacgacaaacccggtaataccaaccacgaccaccgcaaagaagatcgccaaaacggcaataatcagtgaaccggaaactgcgataccggcaaaaatcacccctgcaagcgcaagtgccagcggaattgtcactggagtcgaaagcaacgctaagataatcagccaaatggttttaacatcatttttcggctgctgtcgagactgctgagacatcggcgcgtccagtgtccgaatggaataatctgccaacaccttccgggccaattgatgaggcgttcccaactccctgatgcaatcgtcgtaactcgcatagccgccgtcttgaagatattcacggtagaaatcgactgcttcatcccgctcttcaggactcaattgtcccagcagtgcctgaaactcttcaatgtaatcattcattctgatcatctcctaacatgttatcaatcccttgcttaaattcctgccactcctgctgaataatgccaaactgtcgttttccttccggcgtgattttataataccgtcggttgcgaccctgatatggctcatcataagtcgtcaacagatcgttcttcttcaaccgtcttaaaaccgggtacatcgtcgactccgaaacagaaatcgactcttggaccttctgggttaacgcatagccgtaataatcctgaccattcaggattcccagcacacatccatctaataattccgaacttatttggatcgccatattgccacctccatagtattatacgcggcataatattatccaagacaaataatacgcctctaaccaggaatgtcaaacaatttatggcagaaaaaaagatgggttatttatcccatcctttagacacatatttaatcttaattcgaattttgttaatcaactcggccacgataaaccccaaggcaatcgatccggcaatccagacgacctctgaaagataattaaaggccacctgataatcacctaatgcaaagtttttaatcgtgttatacgcctgacccccaggcaccaatggcaccaagccggggacgtcaaataagatactcggcatttttttgaggtgggcaatcaccacggacaccaaaccaatcgtcaagccgccaaaaaaattagcagatcctaagccaccccaggtattcatgacgccatagtacaccagccaactcaaagtggcggtgatcccggcgacattcaaagcccggtgtggcaggttgacgattaggccaaagccaatgcctgaaaagtaaacacaaatacatttaataataaacagattcataagcatccctcaaaagaagtgcagcgcgattgctacaccaaacccaagcgcacaggcactaatcagggcttcaatcccccgtgccgggccactaattaagttgccggacaacgcatctcgaaccgcgttggtcaagggaattcccggcaccagtggcatcatcccgccaatgataatatcatcggctttgacgccgatcccatttttcacagcgatcagagctagtgcacccacgacaaccgcggccaggaactcacttaagaaccgtatttgaatataaatattcaaaaaatagtaaactgcccagccgaacatgccgacaataaacgtgatccaaaaatccggcagattgttttgaaacaccacgaccaaagtgccgctcactagcccggcgcccaaggtctgtaaccaaagcgggaaagttgctaccaagtcatcaatgtggactaaatcgtcacgaaactcatagatatcaatctttttggcagcgtaggccctggacaattcattgaccttggctactttttccatgtcaaaagcccgtttatcaatcgaaccgacttcagcgccaacttccttgacgccgcctgacatgataatgccggtcaaagtcgcgtagacttgggcatcctttaacccggcattcttggcgattcgcataattgtgtcgttgacccgggacatttctgagccggattcaatcatgatccgtccagccagcacacaggtgttcaaaactaaatgatcataattctcctgccgagttgcagtatcggccatttcaatcacctcacgaaaacataatgagccgttttaaagccaatcaccaatttcttcttatccgtcacattcttgacagttaccgacccttcgaagggatcgtgggaaataatttttaacttatccccaatatcgagtttaatatcgcccaacaacgttaataagtcatgattgtcaataaatcggttaacgatgacttcttcaccgtcttttgcatcagtgagcagtttatcatgatcggggtgataattaccattccgatctggaatgacgccgccatggggacaacgcttcggattgcccaaaaagtcatccaggtggtcgatcatcttgtcagaggtaacatgctccaaaagttcagcttcgtcatgaacatcggaaatgtcatagtgcagcgtgttcaccaggaaagtttcccaaatgcgatgcttgcgcacgagttcttcggcataacgcttacccttttgagtcaattgaacaccggaatacggttggtgagtgaccaatttttcagccatcatcttattcaccatttcggtgactgacccggcagcgatgtttaaactgagagcgatctgcttgttgctgaccaaatcatcagttccgccaagttcaaatattatttttaaatagtcctctttcattggggtcatttaactcaaaatctcctatactttatggaatatcattaccacggtcataaatgatgtcctcgtgctcaccacgggtcgtttctgcttgaatcgtcacgtgacacatgtggtacttgtccttcaataccttgctgatttcggaataaatcggctcagcctcactcaacttcatatcatgcatattgacgtgagcggaaaagataacgttgttttcatcaattgaccatgcatgaacgtgatggacactgaagacaccgtcgatttgcaacagatcttttttaatctgatcataatccaggctcggtgccccctgcatcaagattcggcaggtttggcgaataatcgggatggactcgtagaaaatatacacggcaaccaacacggtcacaattgggtcaaccaatgtccaattataaagatcgattaaaatcccaccaataataatcgccacagacgacagcgcgtcactcaagatgtgaaggtaggttgctttcatgttaagactgcttttcgaccccgaattcagcagaaaggccgacagcaagttagctgccaaaccaatgaccgcaatggtcagcattaaattaccgttgatcggttcgggtttactgatccgtttgagtgcttcaataatcagaaaaacacaaatcaaagccaaggcaattgaatttaagaatgcggcaataatctcagcccgtttatagccaaaagtattgcgcccgttttgccggcgtttactgattcgactggccacgtaactgaaaacaattgaaaccgaatccccagcattatgaaaggcgtcagaaatcagtgacagacttcctgacagcgccccgccgatgaactcggcaatggtaataacaacatttagcacggtcacccagaaaaacttggcaccggctaattcttcgtgattatgatttttttcagccatccattaatcactccaatctactatcattattgcattagtttatgaaaatttccataacgcgtgaacaatccttttagggataccagaaaatcgctccactaagtcgttgaaaatgggccagacagcaatcaaaagctaagccattcctgccgaaaacctgtctcggcttccgtccggagttttcctgttatctggattaaacctgcgaaagaggacagcaatcaaaagctaagccattcctgccgaaaacctgtctcggtttccgtccggaatggcttagctttcgattgctaaacgtcctctttcgcactctattaaaaatcatccgctatccgtctagcctttacctcagcatccgcaacaatttgattcgcttgatccggaaaatgatccatcccctcgacacttaacttggccactgactgaacgccgacaaaattcaaaattcccttaacatactgagtcccaaaatcctggttattgtacttgccgccggccgcctggatatggagggcttttttgccgctggtcaacgggactgcagttcccgtatcagtatatttaaacgtcttcccggcgacattgatcgtgtcgatccacgcttttaatttagttgggaccattaaattaatcaagggatttgcgataaccactttatcagctgccaaaaactggtcagttgaggtattaaattcagcgagcttcacttgttggatcgacgttaagtcgctaaactgtctgccagcttcaagttcatcccacgcagaaaaaatatcgccgtcaatttcttgaaaatcaactttgtacaaatccaatctttcgatgacatcatttggatggatcttcacatactcatccataaacgccctcaacacttttaatgtccgggactttgagctttcgggacgggcaatcaccactagtacttttgccattattcaagacctcttttacgattcaatcgggttgtcaactccgataatatagcatgatttcgcgggaatgacaacgctttcattttctggtaaaacatggttcgctgttttggtggggactgctttacttctctctagccaaaatgtgctccttggggcaatgatggggacccaagctaccttctggcaaagcctgactcggcttcaccctgctctttgctgctatctagctgaaacgtgctccttggggcagcaataagattataagcaccctcgggcaaagcctgactcggcttcacccgagctttttcctgctatctagctgaaacgtgctccatggggcagcaataagattataagcaccctcgggcaaagcctgactcggcttcacccgagctttttcctgctatctagctgaaacgtgctccatggggcagcaataagattataagcaccctcgggcaaagcctgactcggcttcacccgagggtgcttataatcttattgctaaacgccccttgtcgcactcttaaaaaagggcccagtgcactctgcactgggccctcctgtggggaatcggccactctaatggttttaatcaaatatcacttcgttcatattcgaatactgatccggtttataaccgaatactcaaagtgcttttattcgcacgatggaactcttttgtcacattacttgtgcaatctaacagttatacaaacgatcatctaattaatgacttaaagagtgccgataccccacgtgtttagaatatcattcaattcttggtttaacaataactttgtctagatcttacaacgtttaatcagttgtttgacgtcttctaccgacgaaccattttcaataaaacagttgaccatttccatccagtacatatcggtgtcgtcaaattctgcacctactgccacttgaggcttgcttggaaccaggccgtttttgatataatcatcaatcacgtcaggactgacgttaaatttggctgccgtttcattcaatgtcaatttcataaccgttactcccaaatttcgttaaaattcaaatcaaatgatagtctaacagcttaccggcaaaatgcaacagcgaattattcgaccatccgccaattgccctcatccgctttcgaaatttgatctaagaagtgcagaatcgacgccgccatgtccttgtcatgctgaaccagcatattgagcgcctcacctgtaataatcggattactcaacgaaaattgctcgccttttttctcaccagtagagaatgccaagacggtgttgccatcatcaatttcagtaataatgaagaacatactgaaatcatcgtcatctttcatataggcaggcatcgcccaaattccatcactaatttgaaccaattcttcattgttgaatcggtaatcccggtgattctgttcattaactggcttatccagcacaaacatcattttgtcaaacaccgggttgccaagcttaatattatcttccatcgaattcccctttgcattcatcgttattcaatcacgcaaaaatcattctactgataattaccggttcatgcaagttcaatgaaaaatccaatcgatgaattattctttataaaccttggtggtgagaatttcataaatcgccatcgtcgctccaaaaaatagcccgcttctgacgtttggccaaatcactcccatgttttcgacactattgagtggactggtgccgtcaaagtaccaatccattaaaatatctgcgatcaacataattaccataaagtatattccaaagccaattcccttcagaaccgcttttttaatgatctcttggcgactggctgcttgaatctcacgcgtcacaatgtgtgcccgggtagtcgcaattaagatataaatgttcaccacgaagccaaccatcacaatgttaatcatgaccagaccgatcagtgcttcttctgggtgcttttgacccacaaaaatggcgacaatgctggaaaccaataggtagactgccaaaatcatataagcgttggtgccaatcctgccaatttgttggtgcttgtactcgtcgaatggtcgtttgaccccaaaccaatgcatcaataatcttgatccaaaactttctttagctttcattattttctcctcttgacatcagattccaccacaacgatatggttgattgcttctcgggcctcccagacacaagcgaccaccaagaataaaaaggcaaaaatccctgggaagggccgatcagccggactgacgttcatccagacagcaaataggaccaccccgccgagaaagccaacccagacgctgcccatgaccgcatcttcaaccgcgtcatcatactgattggcaatcaccttgcggatatccaaacccaggtcagctgcccgccggcgaatataaaggccggagccgcccacgccaatcaataggcttaaatagacaaacagcatccaagattcgctattgggggtattctttacgaacagcaaaacaccgccggtgaaaaccaatatgtataaccacataaataaaaatgcttttgagatggcagcattcatttgttgacgggcggctttgtctaacaccccacgaatgtgaaaaaagtatcggaataattttgtggaaatcgtatcgtcttgtcgcattattttcctcctattcaactttgacaatgtgggcaatctctcgttgagtatcagatgtccaagaaatcaaaataatgaatatcgcaaagccaatgctaacgatcgagaaaaaaccgttaaattgagcaaacatcaaatacgtaaccaatccataactgatgccaaaccatgcgccatggatcacggctttatgaactgcctttggatactctttagttgagacttcttgataattcagttttaattctgaaactttatgcgtgacgtaaagtcctacgccaccccatacaataaacatattgaacagaataaagccattgatcattgacccggtcttaatggcctgtgggagaagcagaaaaacggcattagcaatccctgtatacatccacaaaaacataaaggcgtttgtggcgactttgccgatttctcgagcattatgctcatccaatacaccgcgaatactgaaaaagtatcgcatgattttaatcaagaaactctctttcatgaattttcatctaccttccaaaatagtgtgtttaaatccgtccccaattcttccgccaagctgatacacaattttaacgacggattatacttatcattttcgatcaaattgatggtttgcctggccaccccgactttttcagccaaggcaaattgggaaatgcctacctgctttcgatactcccggactctgttcaaattaaccggcctcccctggctactttgtcacatatatgtgtcatcaataatataatgccatcaacaaataatgtcaactatatatgacaaaaaagagtgggacgcgaggcgttttgatcccagaatttaagtaaagaaacgagttattcctgtcttggaatgactcgtttctttgcttaaatggccgggatcagccgatagttccacgtttaaactagataacagtggaaaacaagagaggccaaggcacaccctccaattagttgtgtcttgacctctccttgagtatgctcactattatttccctgaatcgtggaaaaatgagcagcttccggccgtataagggggtccatcaaatatccaagccctggatatttgatggacccccttatactctggaagctaagcgctcatttttccacactattatacatacaacaaactccgctgcttggcggtcttttgcatatgatcgtacaagtgatccccaatcatctgggtgcccactgtcttaaatccttttcgttcatataatttcttggcttcaggattttcaaaatcgacattcaagccgatcactgatttaccatcattcaacgccattcgcggaacggcagccaataacttactaccaataccatggccctgccaattaggatcaacggcgatggaatccaagtaccattcgtcagaattggtctcggaatcagggatatacggctctttaaaatcagcactctttttcgataaattgatcagaaccttattaatagcgtcctcattttcgctggggtagccaaagacgaccccaacaacttggccattggcctcggccaccacggtggatgccttactggacagatacgtgtctgtctggtaagccctcgtgatgaccttggctaatccaggttcgggaacgtcttctaattcatcaaggtccatctcatcaaaaataatatcaattaacggggctatctggccggcgtcatcttgctgtgcttctctaacggttatcaaaaaaatcctcctaagtaaatgaacattcagtatgtgttacgtcatatattactgaagttttcatttattgtcaaaattgaggatgaaactactgatcattttcagaatggttttcatgatcctgctggtcattttcatttagattgcttttgggattgccaaactgatttcgttgaatcatgtccaattcagtacggatttggccaagaatttcaatttctaatttctggatttccaatgaatgtggtaattgattttgtgttaaattatccaattttgcatgtaagattcgcagttcatgttcagatttctggttaacgtgataatcattttcagagctcatccgatcccggtcggcggcccggttctggctcatcatgataattggagcttgaatggcggcaatgcagcttaacgccaagtttaagagaataaatggatagggatcaaagtgcatgccaaacaactgcaagccattgatacacatccaagcaattaacacaaacgtgaaaacgccaatgaaaccccagctaccaccgaagcgggcaacggcgtcggagactttctgaccaaacgttaaactcttggccagattatcattgacatcaataatatcgtaatcatcactctgcatcgccttggtcagtcgacgattgatctttttggtctgcttgacgtcggcattcaccatcccatcgacgcgcattaattggtacttcagtaagtcatggtcacaaataaaatcggtgaccttggctttcggataatcccccttgatcaaatttctggttgccggctctaaatcctttagatatcgaccatcaatcaacatatgctcccggtggtcgataaagcaaatcgctgttttagcttctggcatgttctcaatccctccctaatgtatgtatgcaaaaaagaatgtctcaccgattattatatcagtaagccattcttttcaaatcatttaatagtcgtctaaaactagcgcctaaccaaagcgtgaaacattatgccttaattaaatctgattttgctttcaacaaagcggccttcaaagcacggatgtgctcgcgggtttgcttgtcttcctctgcggccttcatccacgataatacagacaagttagtttccatctcagcaataattttttgaaccgtctgatccgattcaccattggtagacatatctagtctcctccttaagttgatacccatactataccagaagtatgtgaaaatacaacggaaatgaacccgctttcatcgaattctaatttgaaattaacgcaagccgatcaaccattggtcttgcaatgttcatttgtgcacaatatgagtagacctctaatgaagaagtgctgaaatgtcttgtgggagttgagatttaaagcttaacgccctgttggaaaatggatcttcaaacctgagctgggtggcatggagtgcttgtcgaccaatccccaagtccatcgggccgtgatacagggcatccccaagtaacggatggtcaatcgaagcaaagtggactcgaatttggtgggtccggccggtatgcaggaccacatcaaccaatgtccgatcctcgtacgcctggtcaacccagtattccgtttgtgccggcttgccatcatcagaaatccgttgaccgtatccggtggggtctttagtaatcggccggtcgatgaagccgtgtttctccagcccaacccctgcgaccacagcttgatactgcttgtggagcgttttggccgccaacatttcattagccaaactgttggccagtcgatgcttggcaattagcaccagaccactggtaaatcgatccagccgcgtaataatatgggggaccaagtcttcagcgccattctcaaccaggtggcccttcacccgattcaccagggtatcatcgcggttcgccggtcccggcaccaccgttaggccagccggtttatcgacaatcagccagttgtcgtcttcatagataactgaaattggttgcctactgacggcaacgtttggatcgcttgcctcagcaggaaaatcaaccgttacctgatcaccggctcgcagaacaactgttgcatcaacttttcgcccacctactcgaaattgaccaccatcagttttagcgctcttgtacattcggtggctgatgcccttggtattcaaaaattttttcaacgattgtgggtcattgtctgtcactgtccaagaaaatttcaaaatggcctccaaaaaaatatttttatattgtgtacaactattttgcttacgttataaatcccgccctaacagcaatcccagcatgtgaaccacattgcataacagaaaaaggcttttgtcaaggccttgacatcgcttgcacaacttgtaatatgtaagtacaagcaaacgcttgtgaatcttttataaaacgaaggagaagttaatatgaaagttgcagttattggttgtactcacgcaggaacctttgccatcaaaacaattttagcagaacacccagacgcagaggtcaccgtttacgaaaagaatgataacatttcgtttctttcatgcggaatcgctttatatctcgggggacatgtaaaggatccgcaaggcttgttctattctagcccagacgaacttaaaaaactaggcgccagcgttaagatgaatcatgaagttaccaacgttgaccccgcctccaaaaccattgaagtaaccgaccttaaaaatgatcaatcatttgaagacacttacgacaaattagttgtcactaccggttcatggccagttattccaccaatcaaaggcgttgacaacaaaaatgtttacctttgcaagaactggaatcacgccaaagaactctttgaaaccgcacccgaaaagaaacgcatcaccatcgttggtgccggctacatcggtgccgaattagccgaagcttacaacaccaaaggacatgaagtaaccttactagatggtgccgaccgcatcatgagcaagtatttcgacaaagaattcaccgacgttgttgaaaaagacttcactgatcacggcgttacccttggcctagatcaacaggtcacagaaatttccggtgacgataccgttaccattaaaaccaccaaaggaacttacgaaaccgatttagttgttctctgtgtcggcttccgtcccaacactggtctattcaaaggcaagttggcaatgaccgacaacggtgcgttgattaccaacgaatacatgcagacctcagatcccgacatttacggtgccggcgatagtgttgctgttcactacaacccaactcacggcttggcctatattccactggcaaccaatgccgttcgtcaaggaatcttggtcggcaagaacattgaaaagccaacggttaagtacatgggaacccaatcttcatcaggtctcaagttatacgacaagaccatcgtttccaccggcttgaccatggctgccgcaaaggcacaaaatatcaacgccagcgaggtgatcatcaccgataactaccggccagagttcatgccaaccactgaacctgttttgatgtcattggtttacgatccagaaacccgtcgaattcttggtggttcattactaagtacctacgatgtttcccaatcagcaaataccctgtcggtatgtatccaaaatgaaaacacaatcgatgatttggcaatggttgatatgctgttccaaccacaatttgaccgcccattcaattacttgaacattttggcacaagccgctcaagagcaagctgccaagcttgctgggaccacttcaaaataacggttacattttagctttgtaaataagtctgaaccacgttataatatttactgcatggtgatgacgatctttctaaaccacatttagcgtctcacaaatgcatcccgtctgacttcggtcgggcgggttttcttatatcacgcttgtgctattgatcatttaggctatacttatggcagattcagacaggaaattggaggtatgaataatggcagaagaccattttatcatttcaacaactgaacacatccccggaaaagaatacgaagtgatcggtgaagtctttggcttaaccacccaatccaaaaacgtcgttcgaaacatcggcgccggattgaaaaacattgtcggcggcgaaatcaaagattacaccaagatgttggatgaagcccggaacatttccgttgaccgtctaaagcaaaacgccattaaaatgggtgccgacgcggtcgtgatgatgcgctttgattccggatcgattggtgcggatatgcagtcagtagccgcttatgggactgcggttaagtataagtaatccaccggttttatttgaaggcctgaaggtaatgatacctttgggccttttttctgtggactttttgatggtcaaaggcagaaccttttgccctccctcctccagccaaaagcctgactcggttttccgcttttctgctattttgctgaaacgtgcttcgggggacagcagggagaaaataagccccaccagacgaaagcctgactcggctttccgtgcttttctgttacttagctgaaacgtgcttcgggggacagcgattggattctaagcccctccagccaaaagcctgactcggctttcgtcgcttttctgttacttagctgaaacgtgcttcgggggacagcagggagaaaataagccccaccacccgaaagcctgactcggctttcgtcgctttcctgctacttagccgaaacgtcccccttcgcactctctttgtaaaattaaagtaaccaacacgtaaaagtttaaccaacttcaattcaaatcccctctttcacgatactatgaaattgcagaaacaaaatcttaagaattcatggagatgaaattgatgattgttaagttgaaaagttcgatctttatctcagccgttgcgctggggattctcggcgtcagttgcgttgcttccaccgcccacgccagcgccccaaaaacacttacggctgaacatccgttaactggaagccctgccagccataacgtaacctttaccgggacgtctgcgctttactctaaaccacccgttagcaaaggtgcccacgttgttgccggcaaagcgactttaaagcaattagcctcggctaaatcttctgctgacaattttgtggctgatcgtcaggccactgccaaaaatggtgccgtctactacaaagtgacttcctttgacggccaataccatggctggatttacggtggcaaaaaagctggtcagtttagtggcggtctggaacctttccggacgttcaaccaaacgaccccaccggccagtctgagtaaatacaccttcaaaattgccgctcccgggttccaaaacgacggcaaaaccgttacatacaaagcacccatcaacacgacctaccaagctggcaaacagattggcgactccgttagatatgccaataccacgtttaagattgacggcatgggcacccgggctcgcgaaggcgatgtttgggttcacatcagtgcgctgaattctgccgacgccaaagcaaatggctggattctttacaaaggcctgcgtcaagcagaatcccccattccaaataatgccttgcgaatcgacctggttgacagcaatggtaatttgatccgctacatcaattacaccagcgccaacgcccaatacgaccaaccactgggtaccccatacgaaacttcctggacgctcggcaacgacgatctcgccaacattcaagtggccgttcgtcaagcactccaagggaccggctacaacctggacacgatttctgccaaccaggccggctttcttgcccaggctaaatttggtcaccgagcctcactgaccgttaagagtgccgatcccattcccggaaacgccatccgcatcaatctggtgaacgatgccaacgcagtgatcgatactgtcgactacaccccaacaggcgcccaacctggccaattactggggaccagttcaaacgggacggcctcattaaatgatgctgatcaaaaggcaattcagtccgccatttccacggccttaaaggattctgggtaccaattgaccgacttgtcaacagatcaaatctcagacttggccaaaaccaagtttggcggggacgtttacctgaaagccaacagctccgatacatcaatcgccgataacgcagttcgtatcaattttgttgacccaagtaacgggaaagtcatcaaatcaattgactatgtcaacaccgatgcggatgatccggccaagaaaggcaccactttaggcacccaaaaatccggcaagtggctgcttggtgacagtgacgtcgttgaaatcaacgccctggctgcctcgtcattatccggaaccggttatctgttgaaccaggaacacctttccgatgaccagcagagcactttggcccaggccaagtttggcagttccgtttcgatcaatgtcggcaaggccaacaactcaactcactttaacttatacgctgccagttcttcaggagacagcgccaacgctcaacagttgaccccaaccgggctgacgtacgtgaacaacagctgggaatttccagacgtcggcggcagcagccagccaacctacagccagttaagtgcggcagacattgccggtttgtcagccaccaatctggctaacttcaaacaggcactggcaaaatacagttctgattcgctggcagcgatcaataacagttttaaatcagctgccgagatgcagtacgtcgataatggccaaactgccagtttgaaccgggcagacctggattctgccaaaagcaatttgaagaacagcagttggtcaacgcttcaatcgccaaaatatccggtctttggaaaagacgccaacgggtcgattaacattgcttggcaaaccattacctaccacgccaaatcggtcaaacaaaatgcggatgaccaatccctcagcctgacctacacattcgacgcgcaataatcatttatttagaaaaggacgagataagatgaataaacctttaagaacgatcttcacgtttgccttggcatttaccgccgcgggtgttctcgcagcctcgaccaacgcccaagccgacatcatcgacgttcccggtgcggtcaaatcaattccccaagtcaacgccggcaatgtcctcaccaactatgattcaagtgatctcaaaaatattgataatacttcgccgatcgggaacatggatcgcaaatataaccagggaaccatcgatccaactcaggacaacgccggcgacacctttgcgaccactgatgcaacgacaacaaccgccaattcgtttaaaacccagtggttcctccctgacggtttcaacgtgaccgactaccaacacggtaacttccaaagcgtcgccttagatgattccggaaatgtctactttgtcgaatcaaacggtagtgataccaacttaggcgtgatcatcaaatttgataccaataagctcaaacagctggggcttgaaaatgacccaatggccctatggaacgcctttaactacttcaatccgtatactgaagacggtgtcacccacaacaaccagtacgatgatctgtatgagtcgatgaaagatacctttaaaactgtcaagtcacttaccagcaaggaagccaccgttaaggcagcaatgaatgacctggcaaacgccaagcggacgacccaggcgaaatatcgaaagaccagcagcacgactaagaaacatttagccgcgagtctaaaagcaaatgccaaaaagatggccgctgacaggaccaaattaaccgcgttgcaaaaacaaattgcgcacggccagtcacagatcgccaaaatcaaggcgaaaaatcctgaattattcaagaacattgaaattgccgaaaccgctcagctcagtccacaagtcgatattggccacggccaaacattgaccttcaacccacaaaacaagcatttgtacctggttgaagataatacgctgaccgatctgcgcaaccgggatgaaaacaacaccgtcctggaaatggatcccaataccatggagccgatcagacaatacaatttcaaaatgttccaaggaaccaaaggcaacctccagctgcatacgttagtctttgataagaacggtaacgcttattggggtcgaaagaacggcatgggctacatgttcttctacggtcgactcgacgaaaacagtgtcaaattcgccgctgcccctgaaaagttaaagactcgcgggggctcgcctaatcaaggagttgccttcaataatgtcaacaatcgcatttacgtcgtttcagacgatgtcttgacctccattccggttgacaaactgactgccggcaccgcaaccccggatgacgtcaactactcggttttccaatccaaacgtgaatgggaatgcttggcatttgactcccaaggctacggccaccttctcgctctgtggccggcggaactgatgaagagtaccgcaccactaaactaaatttgaagggcaactaaaaagcctgcaactcagcatgatgctgaagttacaggcttttcctgtgccttgaacgtttaatgagggcataaatcaaccacaaaggtccgaaaagcacaatgagaagattcaaacacaaatttttaaagatgttaaaaccaaaatccgccgctcccttgtatgattgggtctgagtgtagcgaaactcccaagggttgacggtgacgccattagctgaccaagcacggttcttatgattagcttgaacgtcagcatgatgcaggcggagagctttgtctttataggtttcaaattcaaccgactcttgactgaatgcctgccgcatcaggattcgaaccaccggtagaatcaggagcatatctaacaaaaagtaccaatcccaagcagacaggttaaataccaaccgcagactgccttttgtggaccagtcagggaactgcagggcaccatcataaaaataaatcagtaacagcgccaccaagccacccaacagagaccacccataattcaagaaatgtctcacgatttgcaagttgatccacctctcaacggcaacagaatatcttaaagataaccgttgcgacttgggatgtaaaggtattattaaaattattcacatttatttcacattttagacggattgtgattcactgaccgcagccacctttgccaaaacggcggcaatttgatcaatcccggctaacagatcagcctcgctcattaccaatggtggcagtaaccgtaacgtattgtgcttagccgacaacgtcagcaggccgttttcttgaagttggccaataacatcctcgactttaacggcagcactcaaatgaatcccgatcatcagacctaatccactcacgctgtccacaacggttaatggcgaaatctgtttgtgaatggccgcaaagaccgcttgagatttttcttgaacctcagccaaaaatttcggggttaactgttctaagactgcttttgcggaagccaaagcaatcttgttgccgccaaaagtcgtgccgtgagaacccggaccaaacgccttcgccagttcctttttacccagcatcgcaccaattggcagtccattgcccaaggctttggcacacgtaataatgtcaggatcaagatcgtagtgttggaaggcaaacttcattccggttcgaccaatgcctgtctgcacctcgtcgataattaacagaacgccctggtcgtggcatttagcggcaactttttgcagccactcgccattgccgttaacgacgccgccttccccttgaatcacttccaaaatgacagcggccaaaccctcattaattgcgtcaagtgcctggggatcgttgtaatcagcgaaactgacctctggaaccagtggcttaaatcccgtctggatgtcgggatttccggtcaaggacatcgaaccataagtccggccgtgaaagccattgttaaacgccaagactttacctttaccagttgccttgcgggccaatttgaatgcggcctcattggcttcagtacccgagttgcagaaaaaggccagcatgccggccggacacagcgaagcagctacttcatcctgcagactgctggggtacagattggacgtatgccacacttttccaagctgattaatcacgctctgctcaatccaatcattgctgtaaccgaagctgcagaccccgattccgctggtaaaatccaaatacgatttgtgatgactatccactaaatgccaatcatgccccgaaacaatttccatcgggtattgggcatacgttggaaaaacatgttccatattctacactccttaaattgccagctgcttaaccgataaactggtccctgaatgctgcagctgattagtaattttaacttctttcacaccatgctttagtgcgtcaaatgccgctttgatttttggctgcatccctgatttaatgatctcagcctcaaacagctgattggccttctgcaggctcaattgatcaatgacgtggctgttcaccatgaccccaggcacatcggttaccagatacagcttttctgcccccagcagtctggcaactgctgcagcagccacgtcaccattgacatttaaattcttacccgacttggtcatcgccaacggggcgcacacgccaatcccatcagccaaggcgtggttgatgtattcccgattgatgccgataacctggccgacctcaccataaactgcctgatccaggtagtcaccaaccagtacaggctgaccgccggcatttaatccgacgaccggaagtccatgagcagacaactggcgacagagtgtcggctgaaccagtcccaataatacagcttgggtgactttgagggtttgcgggctggtaacccggacgccgttaattttggcgaccggcaaattgagttgggcgctccactcagagatttgtggcccaccgccatggacaatcagaatctgtttgcccatttggcgccagctccgtagctgttcaaaaaattcttctgtcagctgatcagtggcgtgaccgccaactttgacaacaattatctgactcatttccttcacctcctagcttcgatatgatgcgttgatttgaacatattgataagtgagatcacagccccaagcagttccggtagcttttccggcatgtaggtcgacgtcaatcacgactttgttctgtttaagggttgctgcgactttatcatcatcgatcccggtgcccaagctgttgtaaaccagctccaggtcattaatggcaacgctgacgccgtttaaatcaacgtgggcggttgtctggccgattgcctgcatgattctgccccaattgccgtcttcgccaaagatcatcgctttgaccaggttggagccgacaattgccttggcaacctgttggccctccaaatggttataagcgccagagacattgacttcgactaacttggaagccccctcaccgtcaccggcaatctcctgtgccaaatgggtgagtacctgcttaaaggctgccgcaaaggtcgggtaatccggatcggctttggttaagggttgatttccagcagcgccgttggccatcacgaccaccatgtcgttagtggacgtgtcgccgtcgacagtaatctgattgaaggtttcatcgaccgttgtgctgagcagctgctggagatcttctccggtaattgctgcgtcagttgtcacaaaacccagcatcgtggccatgttgggatgaatcatcccagaccctttacaaaatccggtggtggtcacctcctggccgtcaatcaaacatttgacggtcatcgttttgggatgggtgtcggtggtcaagatcgctttagtgacgccaacgttttgggtcagcttcagttgggaaatcccagccttaatcttgtccattggcagcggttcgccaatcacgccagtggaggcaattcccaccagttgcggatcgatttgaagtcgatcggcggtcattttctgcatcatcaaggcatcggtttctccttgcgccccgttgcatgaattggcattaccactattcatgaccaccgcttgtaattgatgtgccaagttgatcgtctgtttggtcagcttggttggtgcggcctgaaactggttcgtggtataaaccccggctgcgtttgcgggggtactggaataaagccatcccatatcgtcctggtcgggcttgaacccggcgtgcgtcgaatcggcggaaaagcctttcggccaagtgaactgactcacttcaatgagtgtcttacttgtcatctgcattcaaatctctcctcggtttacggcaaaaacgtttgtaggttcaagccgctggtttcttcataatcaaacatctggttaaaattttgaacggcttggccggccgctcctttcagtaaattatcaatcacgctgtcaacgaccatcatctgagtgaccggattgtagacaaccccaatatcgcagttgttagtcccgacgacctgtttgatatcgggtaaatgctcacctatataatgaacaaatggcttattgccgtaagtggtggcataggcctgatcaatttgggcaccgccaacgccgggcttaaccttggcataaatcgtactcatgatgccgcgggtgattggcaggagcgtcgtcataaattggatagcggccacatcatcgttccagcgctgcaattccaacatgatttccggaatgtgctggtgttggttgggcttatatatctgcaggttgtcattagcctgtgtgaaatgagtggcctgggcgggatttttgccagccccggaggttcccgatttggcatcaacgataatcgaccccgggtcaatcaagtcattttgaaccaatggtgccaaacctaatagcgttgccgtggcataacagcctggattggcaacgtaggtctgatgaacggctgattcgaaatctgccaggccataatgagcttgccgcattgccagttgcggcgccgctggcttgtgataccagcgttgatactcgctggcatcctccagccttaagtctccagataggtcgatcactggaaagcctgcctgaatgtacggttggctgagctgggcggtcaccccagccgacgtcgcgaaaaagaccatttgattgtccaccataattgttttaggatcgtatggctgaacttgggtgtcgtccgtgtaaaaagccgaaaccatttgcgacaatttctcattttcagttaatttatgatcatacaggttaatcccggctacttctggatgccgacgaaggagttgatacaataccattcctgcatatcctgtaatcccgactaaagccacttgcaaaccaatcgcctctcatttttctaaatattcctctaattgaatattaatgaattgaaaacatcttacaacaacatgcaggttaatgcaatgttttttgggtattattcatatttttatttgtagattgatatttattcatattcttgagtataaagatgtatatttggcttgtgaaggaaatttattcacatcagtattcatgaataatattgtcgttttattcatatcgaggttctttttgcttagactgccgtggtgctcagttcgtcggctctgcctgccatagtggcctggatttcgagcctgtagtctcgaaatgccagggtgttgtaatcgccgctttcagcgactcaacaacacctttcactatggtagtcaatgccaacgaactgagcgccacttctttggaacgctgatggaacccccgttacgagttaacatccacatggtttgaaatatccctcacctggcagcttgtaaccctcatttggcagatggtagaaaaattagattcgaatagtcgaaacccttggaaggtcttggagacttgcaaaccaatatagcttgagaactgcatgaaccaaacatcagtcattttgccttctcggttgcctgattttgccagctgggcattgccagccatagtgaaagtgctgttgagtcgctgaaagcggcgattacagcacctttgtatttcaagacgataggcttgaaatcaaagccactatggcaggcggagcccagccggcaaaatcacaaacgttaagttaaattcccccacagtttgaccaactgagtcgacaatcatccacaaaacaaaaggactaaccacatagtgcagttaatccttcgtcaaactaattcaattcaaggtttcggtgccccaactgtttcctgaacgtcttccggaattttatccaaagcctgactgaggtcggcaatcaggtcatcagcattttcgacacccaccgacactctgatcaggtcgggcgtaatcccagcctctcgcagctcttcctcattcagctgggcatgcgtcgtcgaagctggatggataattaatgatttggcatcggcgacattggccagtaatgagaataacttgaggttttgaataagctgcttgccagctttttcaccgcccttcaaaccaagggtgaagattgagccgaccccctttggaaaatacttttcagccaaatcatggtacttgctgtcttcaagtcccggataattgatccaggccaccttgggatggcgatccaagaagttgacaattttcttggtgttttcaacgtgacgttcaactcgtaatgaaagtgactccagcccctgaagtaataggaacgaattgaacggactaatcgtggcccccaaatcccgcaaagattctgctctgactttggttgtgaacgcactaccaccgagatcggcaaataccaggccattatattgagtattcggttcggtgaagccgggataacggccgctttctttccagtcaaatttgccaccttccacaatcacgccacccattgtggtcccgtggccgccaatgaatttggtggccgaatggacaaccacatcagcaccgtgatccaatggtcgaaccaggtatggggtgccaaacgtgttatcgacaatcaagataatgccatgtttgtgagcaatcttggcaacggcttcgaaatcaatcaaattaattcccggattaccaatactttcgatatagagtgcttttgtgtgctcattaatcggtgcttcaaaattggccggatcgtccgggtccacgaaatgggtcttaatgcctaatttcggtaaggtgacattgaagaggttaaaggttccgccatacaacgtgctggcggaaacaatttcatcccccttgccggcaacattcaaaatagcggcggtgatggctgccgaaccggttgccagtgtgacgccgccggtacagttttctaaagcggcaacccgcttgtcgacaacatcggtggttgggttggtcagacgcgtatagatgttgccggggtccgtcaagccaaatcggccggcggcctgctctggattgtcgaatacgtacgaggtggtttgataaattgggactgcccgagaaccggtttcatcaaccgtttgacccgcatgtacctgaagtgtttcaaagtgtaagtgactgttttcttctgtcatattgataaacccactttcttatttgcgatgattttcatccagttatcataaatctgaatactgctgtttttccaagaatagtccaccgttccggaatcctgatcaatgaagtagttttgcggcaatctgatcggcatctgctcatataaatcgcggtaatattccaatgccagcgtcccttcggaatactcgggatgaccggtgatgtaagtgctgtgaagactgtcggctgacaagatgatcgggccggtaacagcggctgaaacatccaccgtcaagccttccggaagatggtcctcgtccaaaacaatgccggtatgtctggattggggcatcttcagcaatcccccagcgccaaatccacgggcaatcggtgattccgcgttgatggtttctgccggataaacaccaaacaatttactcagcagtaagtgtttccgaacaccaaagtcgtggaacaaacaggcttgagcagcccaacattcatacaaacattcggtggcatgatcctttgaccagtcaatgatttcctcaagttcatcccaataatcaacttggttgaacgggagcgtttcgattggcgctccagtgacaattaagccatcataatgggcatccctaatttgatccaaacagacataatcccgttggatcaggtctgttgacgtccctcgaaaatgatgggatgacggatacataaacgtcaattccgcgtcggaaccaatttcactgaaccgcgttaaaaactgacgctcagtatttacccgcgtcggcatcaggttcaacaccaagattgatagcggattagtaacttcgtggttaacccacttttgtgctgccaataagaacccattaattgcatttgccgtcatccaaatcatctccttaaatcataaaaaagcttccgtccacatagttatttcaactacgggacgaaagcttcgcgatgccaccctgatttactgtcacctcacaatgacagccttaataagtactccttggaatacccggtccaatatcgcggactcgcggatatcctagccttttgaccggatatctgactcagagctcatcttcacgtcgctgcaaaccacttctctcaccaaacgaagctctctttaggaatgcgttaacgttactcttctcttcaatgtctaatgtatttttaataattgctagtaactttatcatcacaacatgcccttgtcaacaccaatttgaaaaatctttttgtcatgattaaaaacatatgagtttataatggaatgcaaagagatttttcaaggggtgaaagtatggatcaatcaatatctgaagatgagctgatcgccgtctgcggcaaggtcggtaaaattctgctcaccagcggcgcggaaacatcacgcgtcgaaggcaccgttgaatatatcggccgcgctgcccattatgatatcagctgccacgcaacgattaccgccctgtttgttggggtcaaaaatcagaccaaaacccacttggttaaagtccgcctgggggatttcaacttggaaaaggttgacgaaatcaacaccatgtcacggaaatttgtgaccggacagattgattttgccgagctcaaacgaaccatcgaccaaatcgacaagaaagtgattgactttacttggccggaaaaagtgtttggtgccgccatggtgtctgtcgcaccaatgctgctgttcaaggcaacttgggcggatctttccctagcgtttttcgtcggcatctttggctacttggccgcagccctttccagcccccggatcaagaccccctatgtggcagctggattaggcggttttacggtcggctttttggcagccgtcctgcagtcactgggaatcgccactaacgccggcaacatcattgtcagtgctttaatgccactggttccaggagtggccattaccaactcgtttcgagaaatcatcgatcggaatactatttccggggttgtccgggcggttgacgcattgattatcgctggatccatcggtgccggagttgtcttgggcgttgggctgtccgggatcattttccatctgattggaggcggcctatgaaagtcctgattgaactcatcgtcagtttcgcctcaacggtcggcttcggattggttaccaacgtcccccggagatcactgttacccgccggcatcaccggatcactggcctgggtggcctattatttagtcttgcaagtcgataacgggttaattctccccaatttcaccgcggcaattgttatcggcattctgggtaatatttctgcggtgatgtttagagtcccggtcaatattatttatgtccccagcttggtttcattagttccgggcggcattttgtacctggggatgcgcagcttcactttgggaaatgaaattcgcaccgggcaatacatgttcaatgcgctgacaattgccattgccttggcagttgggttcgtcgtggcagaagttattttttatcgaattaaaccgtttttgctgcgactcttggcaaagcagcgtgaacgataaggtgaccgccctcattaatcataaggaatccaaatcaagcagacgtccagttgaatcttgggcgtctttttgactgtcgttttttcgaaaatcagttcaaaatgatagcgtttccgtcataatggttctaaataaaatgttatcatgataaattttgaatgatggtcggtggtgggcattatctacctgtgtattcaccttttaaacaataatccgcattttatggccaaaagaatcaatatgtagtttataattattctaatttattcgataaatcacctcataaatatgttacgctgtatttagcaagtcaaatacttgtaaatatcgaatctagaaaggcggaatcgttgatgaaagttattgttgttggttcatctcacggtgggtttgaaactgtcagggggattttggcagaaaagccggataccgaaattcaatggtatgaaaaaggtgacttcatttcatttctctcctgtggaatgcagctttatcttgaaggggtcgtcaaggatgtcaacgctgttcgttacgcaacgccggaacaaatgcgtgcccaaggtgtcaatgtgtttgtccaccaagaagttacctcaattaatccagacgagcatacggtagttgtccataatttggacgatgattcaactcgtgaagaaaaatatgacaagttggtactatctgccggtgccgtaccggcaaaaattcctgttcctggcggcgatctcaaaaacgtctatgcaatgcgtggacgtgactgggccatcaaattaaaggagaagacggttgaccccgatgttcaaaatgtcaccgttgtcggtgccggctatatcggtattgaagccgctgaagtcttctccaaagccggcaagcatgttacgttgattgatattctccctcgtccattggccctgtacctggatcaggagtttaccgatgtcctttccaagacgctaaaggatcacaacatttacttggcaaccggccaaacggtcaagtcattcaatggagaggacggccaggtgacggcagttaagactgatcaagctgaatatccaagtgacctggtcatcgagactgccggcatcaagccaaataccgactggttaaagggcacccttgatttaaccgataagggtctggtcaaagtcaatgatcatcaagaaaccagccagcctgatatttacgccgtcggtgacagcaccaaagttccatttgccccaactggtaaggaactccagattgctttggctaccaatgctcgacgccaaggcaggattgctgcgaaaaacgtccttggagacgacatgaagatgccggctgtttccggttcatctgccctgtctgtctttgattaccattttgcttcaacgggaatcaaggaagggacttccgcagccaacggcgtgttgagtcaatccgtcttcgtaactgataccacccagccaccattcgtaccaaatgaggccggcaatcaaaaggtctacttcaagttgacctttgatcccggaaatcaccgcattttgggtgctcagattatgtcgaagcgtgacgtcaccgccaacatgaatgccattagtttggccgtccaagcaaagatgacgttggatgatttagcctatgccgacttcttcttccaaccaggatttgaccggccatggaatatcatgaacgtggctgctcaaaaagcactccaaactttagccaaataatcagttaaacaaaattcctccctaaaacgattgctcaccgttacgcaaacgcaaatctgcgttatagtaaaggcgtagccaaatcaatttagggaggaatttttttgaaaactgtcttaattcttggtgctgccggacaaattcccagtttcttaatcccccagctcttaaaacaaactgattttaatttgaaactttacgctcggaatgccaccagtcggcttcacgtaacggatcccaagcgcgaaacagtcattgatggtgactttaacgatcacgatactttgaaccaggccatggatggtgtcgacgctgtctatcttaatgagatgcgggacatcacatccgttaagaacatcattcaagcgatggatgccaaccacgttcgccaatttatcggtgcgaccgttctcgggatcgaagacgaagttaagggtgcctttggccagtggaataccagcatgattgaaagctcgatcaccaagcgcaagaccactgccaaagcgatcgaagattctgatctgacatataccctcttgcgattggcatggctgtacaacaaggatggcaataccaattacgaattgactgaaagcggtgaaccgtttggcggcacagaagtcactcgccaggcggtggcccagttaatcatcgacatcttaaacgacaactcacggaaatttgctcgcaagagtatcggtgtcaatgaaccgaacaccaagttcgataagccgtcattttattgattcaatttcgatggctttgattaccactgttatgttgataaaacgtgcagagtttaagcaaaggagcgagtcattccaagacaggaatgactcgctcctttgcttaaatgatgggtcaaaacgcattgcgttccacactcataaatttccatcatcaattaatcaaaaattttcttcgcaatgtcaaacgcagaccaagcctttggccagccggcataaaatgctaaatgggtgatgatttcgaccatttcgtcttttgtaaccccatttgccttcgccattttcatgtgggcttccagttgtgggaacagcccctgtgacatcaagctggcacaggtgatcatgctgcggtctctggccgacagcttcgattctcttgaccagacttcgccaaataaaacgtcgtcatttaattcggcaaatttgggtgcaaaatcacccagtgcatctcttccagcagtttgttttttagccatgattattgaacctccaattgatcgtattcttcatctgagaccggttcgagccattctggtgtcccagcggtaatcgcaatgtgtgagaaccagctgtcttttgtggccccatgccagtgcttgacgccatcgtgagtcacgaccacatctcccggcactaagtgttgagcaggcttgccggcctcttgataccagccttcgccaccggtgaccaacaaaatttgatagccatcgtggtgaatatgccaattattgcgacagccgggttcaaaagtgacgttgccaacccccacattaaccgctggatcattgactaatccctgaagataactctgacccacaaaatacttggcataagcatcgtttttcgggccagctgggaaaatcacaccatttttaacattttcattttttaccattgaaattcctcctcatcaaaaacatttactttacaaataggagcatacaacttaaagttaactttaagtcaaacattcatttaaaaataatggaggaaatatcatgccagctattcaatcagaaaccagttatgaaatcggcgaatttgccgaaattgtcggcctctccgctccaaccatccgctactatgaaaatcaggggctactcaaagcccgtcggacagacaacggccgccgatattttaccgaacaggacatcaagtgggtcaaattcctcttgcatcttaaaggcaccggaatgagcatcaacgacctgaaaaaatacgtcacttggcgggctgagggcgaccagaccatccctgaccgcctggatttactcaagaaaaccaaggccgatttcatggaagaataccgccaagtccagcatcatctgcagattctaaatgataaaattgactggtatgaagccaaagaatccggaaaagataccggtaaggaaccctttgccacctacttgcagcgactggggcaccatgaataagtttctgagaatttcacagaaacttgtcagggactaccactttcaaatgagctgccagtcactctacaatgttcatgattattcaattgaaccagaattgaggggaaattatgacgaatactatcctgctggttgaagacgaggaagcactcagctcgtatttaatcccggaattaaaatttgaagattatcaggtattgttggcaaaagacggtcaagaagccctccaagtctatgacaataaccggggcaacttagatctgatcatcctggattggatgctgccaaagcttgacggactggaagttctacggcgaatccgcaaaaatgatgacatcccagttatcatgatgaccgccagagattacgtcggcgataaagtcgccggactcgacagcggtgccgatgattacattaccaaaccatttgaaattgaagaactgctggcccgaattcgagtcgttctccgccacgagagccatcaccaccagcaaagcgaactttataccgtagaggacctgaccttaaacaccaagtcccgccaggtttcgcggggaaatcaactgattcaactcacccaacgggagtacgaattgttattaaccctcattcgccacggtggcgaaaccctcacccgtgatgagctgcttgacgcagtttggggggtcgatttcgaaggccagccaaatgtcgttgacgtttatatccgctacttgcgcaataaagttgatcggggatattccaaacagctgatccacaccgtccgtggagtcggctatgtgatgtccggaaattatcaggaataaggagtcttagtttggcaaacaaacagcatcgcaccacctatcaagcaatccgccaccactttattatcctgctaaccttttttgccctatttaccggtatcgccgttgtcttggtggtgggcgtgaatttggtccgccaaagcgaaagccaatcggtggaattactcagaagccttaatcgctcattcattgacgacaaaccggattggaaacagtggcggaaaaacagcagtatcaatactgaaaatacttatgtcagggtaacggatcaggttcatacggctaagcagccggaactattttattcccagggggcgcctcaatttttggcggcagcaccaaccccgatttcaaaaatgatccacataccggttttcccggctctcatttatgccaagggctatggcctcttctattatcgcagtggcgttcggcacggtagtcaaaagaatatccgctcagaaatttggctgagcctcaatccaatcgttcaactgttaacatcggtcattttaatcgttctgttggtttcacttgccagtctgtcactgggctggttcgtcatttccctgattgcccgccagttaacggagccgctgcaaaccctccaggaagctgccaaggctcatagccaatcaattaatcgggttgaaaccctcctaccggttccggagtccccagtcgaggcccaacagcttgcgattagctttaacgatttgttatcagccatcatcaaaaataaccaaaaagaaaaagcatttatttccaatgcatctcatgaattgcgaacaccgattgcggctatccggggtcatattgcccttgttaaacgccgcggcaaagcgcatcctgaaattatcgacagctcacttcattttattgacgacgagtcagcaaaaatgcaggcgctggtgaacagtctgctggccctgtcgcgagccgacaaggaagtcgtcaccaaaagtcattttgatttagcggtaatcgtcaacgaaaccgtcgaagaacagcgggtgcttttaaagcagccaatccaagttgtgggcgagcaatcagcaatcgttcatgccaaccagaccaatattacccagattttatctgcccttttagataatgccggcaaatattccccgccggatgcccaaatcacggtcaaaatcagcaagcatgatcatcaaacagttctggctgtcgaaaacaatggcccaagcatccccaaggctgatcaggcccacatctttgatcgcttttaccgtggggatcctgcccacaacagtcacattaccggcaacggattaggcttagcgattgccagtcagcttgcccagctaaatgatgtcggcttacgagtcaagagcatcttgccccatggcgtctcgtttgaagtcagcttttccgaccccgatttaacaaaatagcaccatcaattgcgatgcgttcttcttaactgacacctgcatccccactttgagaccttctgagaatttatcagaaggctctttttttagccctgtattttctcaccaaaaatcacagtattcttggcttgtaagttcgataaccaagtgattggaggaatattcatgcagacatcaacaatcaaaaatcatccgctgctgttcttcggctggctgatctttattggcatcacaggattggtcctcctgcaaaatgttcagttgtatttttgggaccgcgattttcttaactatctccagcgatttattaccccagacagaacaagttttttcaaaggagttgccctgttcggcagcccaatgataacagttgggttggcaattatcgccagtgtgtttctttggcagcgaaaaatgctggaggaggctctgacaaccctggtggtagtcgttaccggcaatgcgggtggattaatcattaagcagctaactgaacgcccacgaccaaccaccatgctaacccatgactcaggctacagcttcccaagcggccatgttgtcagtgccgttattctgctgttaattgtttttcaattcatcctcccgctcatctcatcggtgagattaagaatgtttttcagcatgatgttagtcttctgggtagccctgatttgcctctcgcgactctacctacaggtccactatccaactgatgtgattggtgcggtgctgtatggactgctgtggtgggaatcagcaatggcagtccttcaccaccagcaatttaatactcaaaaagtcatccaacacaatcgggggcagtcatcatgaacctaaaatacacaaccagaaatatcctgttaatggtcgctttatcggcagccctgaccggcgtggtgttggcgatgatcttcaccgttaaccaaatcaccccatttgggactcacaatctattagttggtgatatgagtgctcaatacgtcccatttctgaccggctttcgaaacgccctcttaatcgggcacttctcattattttctttttcgcttggcgtcggcgaaaacatctttccgctcatcacgtactatctgttgagtccatttaacttactggttctcctatttccagcgagccagctgccggtggccatttcctggattttcatcctcaaagacatgacgattgccgcgacgacctgctggtttctctctcggcatttcaatcgaattcatcttttactgccatttttcactctagctttcagcctttgcggttttgcttcggccaacttcgtcaatatcatgtggctggacggcctcatttatttgccgttaatctgtgacggaatcgatcagatcaaagcgggaaaccaatcgatcagtttatttgtctggctgacggcagcgatcgtgtccaactactatatcggctatatgctcggactgtttaccctcatctacgcggtcgaaacgattatccgaaccaacgatcttcacttctcttggatcaccgccatcagccacaatcgacagtttattaccagattcattttcaccgaagcggccagtgtcatgtccagcatggtagtgctgttgccgaccatgttgggcatgcttcagaccgccaaaaccagcccgtcgaccgccaatagcctggccgcggctgccaagccacaatttggtttggagatcttttcacaattgggcttgggcgggcaaacgtacgataatcggctgctacatgctccggcgattttttcgtccttagcgatcgcccttttagtgatcggctactttttccatccccaaattcctcgaaaccacaaactagcggtctcggtaacggctggaattctctcactcagcatgctgattggaccgatcaatctggtttggcacatgctcaatgaaccgtccggctctccatttcgctattcattcttgctgagttttgtcttgatctccgcggcttacgaaatggtgctggccaacccccaaggcttgtcattcaaggctaaattgagcactccaacaattctagcgggattgttaattgtcggttatctcgacatccgcctgggacgccatgtgctcacaaacgactatttggccgttcagcccaactcactcaacgtcctcatagtcaatctccttttaacggtcatcttctcatatctcctatttacagccgttcatccgatgcagcaattattaattggaacaattgtctgcctggaaatgggtgccaacttcggctacaccctcaagagtgaaccgctgcctttgcaaacaggctacgagactgcctatcctcgagttgataccatcgtttcaaagactaaaaccaccgacaatcagctataccgcattgaccagtctcacagtcagttggctcccatattcaaagaaacttacttaggctataacgatcccgttttgttcaattacaatggcattcaagaatacagctcgacgttaaccgaatcgacccgtcaatcattgaaaatgatcggtctgttcagtaagaatcagcgccgaatcagcactgccggttcgactgccatttccgacatgctgttgggggttaaatatcagctgaacccagctggaaaaattgagaaaaacgcatcctttgcgggaatcggcttcccggttaccaaccaattcgctcatctacaactcaccgccggcacactatttaccaatctggaaaggattctccaacgactggcaccttccaaccaaccgtatttagtaagcgaatctggaaccaacccacaacggcaaacaatcggggctcgagaaaaatacaccctgacgatcattcccaagctcagcggtccgctgtacttcgatacttcggataaactgctggattacagcgccatttatgtcaatcacacccgattaaaaaccatccccaatcaacttgataaacagtacctggttaaattgggaactgccaaacgtggcgtcccggttaccctacagctcacatccaaaagtcaaaacacccttcatgagagtcatttcaacagcctaaatgactcgcaattcagcaaagttgatcaacacctgaaacaaagcgcttttacccccacctataccaacgatcgtttagtggggacggcagttcggcccaattcacaatcagaatggctatataccgcaattccatatgatcccggatggacggcgactgtcaatggccaacccgttgagccaattaaggtgttgggtaactttaccgcattaccactcactgatcagtcaaaccacatcgtgatgtcttatcacgtccccgggttattgcttgggatcattctttctcttttaggcttattggcgtttagttggcgccaatttcgcaatcttgcccttcgaaaagacgtgagtcaacaggcgccaggagatggaacaccctcaaacggggaaacttactagtaatactgacaagaaacgttcgatcaacgtaactgctgcgatcctgcctacctttgaatttcaaatcatgtagaggtatactcatttcacaacataaaaatcaaaggaggcaactacatgatctattcaccattaaatgaatgtgatgttccaactatccgttaatagcgggttattccgctaatcatttcatacgaaatctaaaaagcggaggaacatcatattgaattcaaaaaaaatgctcggtgcattgctgctaagtttagctgccagtatctggggcggtatgtttgtcgttgttaaagtggtggttgagactatcccgccaattgaactggtctggttgcgatacctgattgcgttagtttgtttaatgttatttgcagtcatttttcacattaaatggcgtttcaatcaacgtgacttgggaatcatcattttaatcggtattattggcaatgccatttccatcgtgacccaagaaaccggaacttggctgtcaaacgctcagactggggcggtgattacttcagctacgccgaccttcatgatcatatttgcctggtggttgcttggtgagaaattggatgctgttaagatcatttctgttaccatggccactttaggcgttatctggattgttggggttcacttctcaggaacccatgtgttactcgggattttttcgttaatcattgccgcattgacttgggcgttgatgtcggtcctggtcaaaaaagtttcaggcacctataactcacttcaaatcacgattatgtcgacttttgtcgcattcgtttgcctcacgccatttgtcttgagccacatggatgtgattacccgagctcattatctggatcccaaaattggtctcagtctcctttatctgggaatcgtctcgacagccttgggctttgtcatgtggaataaaggccttcagttaatgaacgctgccagttctggacttttctttctgtttcagccggttgtaggaacgttacttggatggttagttttaggtgaaaccatttcgtggggatttgtctttggcaccatgatgattatcggcagtgtttgggtatcaattcgatttgctaaataatggcacttaaaaagggaaacgcaaaattgcgtttccctttaatcgtttctaaaaattttattcgcccttagcctggtaaacgtactgacgcgtcattggcagaccggttccacttggggaattggtcaacaagtactgcataacatcaatattaccggcttcaaatgaagcggcactggcttgtaagtacatgccccacattctggagaacggcacaccgtacttttctttgaccttatcgatgaccttcatgtagttggcgtaccagatttccaaggtcttttgatagtgacggcgcaacggctccaaatcactcatctgcattccggcatccatgatgtgagtcatgttttcagcgacgtttggaatgtagccgccatggaaaatatacttgttcaagaacggatcaacgccggctccctggtgctgaccagtaatcccgtggattaaggctcgtccttcaggtttcaagaaatcatgaactttctggaagtataagccaaggttttccttgccaacgtgttcaaacattccgactgaagtgacgtagttaaattggcctttgacttcccgatagtcttcaagcaaaacgtcaactttaccttcaaggtggcgttctttgatttgctgcttggtgtagtcatattgttcctggctcaacgtaattccggtggcctttaaatcaaagtcttcagcggccatgaacaacaaagtgccccaaccactgccgatgtccaataacgtattgccggcaaccggattgagtttgtgtaaaatatgcctgtctttgttcaactgagcttcttccaaagtatcgtcatcgtgttcaaaataggcacatgaataagtcatgctcttatcaagccacattctataaaaatcattaccaatatcataatgcttttgaatgtctgactcactggctttctccgagtgggaaacctttggtaagtgcttcaagaatgggttgttggttaagaagctatggtctgcacgaaaggctgaggcaaccagctcttgaatgctgccgtcaatctcaatgtcgccgttcatataggcttctgccaataccaatgttggctgtgaagtcattttctttaatggaatttctttcttaatcgtaatcttaacttgcggctcaccatctccgtagttatcggtcttaccatcccagtaagttacagatactggaatatcaaacgcatggctaagcagctctttataagtgatcttctctaacatgaaatttcctccattgtttttctatcagtaacagtgtaacgcttttaggggtataaaaagcaagcataaattcttttgaatttacttttctgttggaacgactttaaatttggtgccgtcttttttaaccactgcatagaggatcgaatcttgattatcgtccagatagcccaggtcaactgcaggatggccgtcgatttcggtcatcccttcaaatcggtcgaataggacctgtctcgctaatttgagttcgtggctcttggattcggccttttgggcagcgactgccaaagtgtagccctgatccaataaaactttcatctgatagaccttgatcagcatactataggaaaatttgcgattctggccctttccttgggtgctttcgatatagccctttcgttcccagtaccgcaatttggtctgggaaacgccggttgcgttggcgacgtcaccgatgcccaagtgccagtcgttctctttcatgatttgagccagcttctgctggaactctttatccaaaatgatccctcgtttctcattttcaaaagttgtaattgcttccattgccttaaaaccggcattccaattattaaatcgtctgataccagtgagacattaattaacattaagtatatatttttaaatatgtttgtcaacttgcttgacaattatgttgaaacattttatattagtccatgttcgattttgagagaaatcaaaattttaaataaagaaggtcctaaatcgtgggtaacgcagtagataaaaacgggaagtcatacaaccgtggtttgatgattatcgttattctggtcggaacattttgtaccgttctgaatcagacgattctttcaaccgcctttccgaccattatgaaagcattcgacgtcaacacatcgactgttcagtggttgaccactgggttcatgatggttaacggaattatgattcctgttagtgcttggttaagcacaagattcaattctaagtggctttatattagtgccatgaccactttctttgccggaacgatcgtttgttacatcgctcccaactttgcgaccttattaatcggtcgtttgattcaagccctcggtgttggggttaccatgccattacttcagacaattatgctttccatcttcccacctgccaaacgtgggactgccatgggacttgccggaatcgttattggcctggcacccgcaattgggccaacgctttccggatgggtcattgataactggacttggcgtgatctgttcggaatgatcattccattgatgttcttagttattcttgccagcttctggcttgtcagaagtgtattggataccaagaagacgggcatcgacctgctttcaatcgtgatgtctaccatcggatttggaagtttgctttacggcttctcatcagttggtgaagatggttggggcagcacaatcgtgatttcaacgttgattgtcggcgttgtcttcatcgccttgttcatctggcgtcaattaaccatgaagaccccattcctggaatttcgggtctaccgttcagtaccatttaccgtctcagcgattttgagttccgttaccatgatggccatggtcggagtcgaaatggtcattccactttacctgcagattgttaaaggaatgtccgcctttcattccggattaacgttgctggccggcgctttgatgatgggaattatgagcccaattaccggccgggccgttgaccgttttggtgctaaacgtctgtcaatcttaggaatgagcttgttaacgttaggttcaattccgtttatcttcattaccaagagcacgtcaaccttatacattgttgtcttctacgccattcggatgtttggaatttcaatgacaatgatgcctgccacgactgttggaatgaactcactgccaattaatttgttaagtcacggaactgccgtcaacaacactcagcgacaggttgccgcttcagttggaacggctgtgttgatcagtatcttgaccaacgtgacgaagagcaacaaaccggctcactcaatgctgacaagtaacccgcttggctaccgtgatcacatgatcaacgccacgttaaccggttatcacgccgcatttgccatttcactgctcttctgtatcttagctttgatcactgccttcttcttgaagaaccgtggtcactcaactgattacactaaaaatggaggtgaagactaatgatcgttatcacacttgcaattggggttgttctggcgtttgtcttcttcatctacatttcaagtaaaccggtcagttatacccttaccgctctctcactattgttggcagtcgtatcaatggtcttcatcattaagaacgaccacgatcattacggcatgaaacaagtgacgacagaaacatcacagcaaatttacccaatcggcagcaagcaaatgcagatgattctctatcagccgattggaacagctaataagcatcaagtttatatttatcaaaaatcagccaatgctaaaaagaagtcccatacgcaaacgactgataccactaacaaagtggtcatgaccagcggtacgactcacatggtcactcaaaccacgcgttgggagtacaagagtgatgccgccaaattgtggttcggcatttctggtgaaggccacaaattcgtcaaacgtcacaacatcttgtacgtcaacaaatcagttcaggttctctccgctcaacaagccaaagcccttaagaaaatgatggcaagcaaatcttaccaagctaaattaaaggcccaaggtaaagcgtttgtcaccaagcaggtgatggccgcaatgaagaagaacccaaccatgtcagctgctgaccgggccaaattggtcaagcaggccaccgctgaattccaagcacaagccatcaagactgtgctggcacagattaaaaaataggttccatttctcttccaatattaaagcgcaccaattcaacaataaccgttgagttggtgcgcttttttggattgtcatttaatttgataagacttcggtcaacttcgacaagaagaattccaattccgcatgcgtccccacggtgactctaatgtgatgcggatacccccagggcgtgcagtcacggacgatcaccccatttttcatgagggcgttgacaacagttgtcgcgtcaggggcgccatcgggaagttgggcaaacacaaaattagcttgggacggggcaactcggaagcccagaagtcccaacgactcaaccagtccttcacgatcaccgagaatttttttgcgcgccttattagattcgatttgatcaaattgaagcgcagcacttgcgccggcaatcgccgttcggttggtgttgaacggttccgtcacagtgtcataggcctgaattgcctcaggatcacccagcacataacctagtcgggcacctgccagaccatagaatttggaaaaagtccggatgaccatgacccgtttatggccgatatagcgaagaaagttcgccaagctcaagtgatcggcaaattgggcataagcttcatcaacaatcacccagacattgtcaggtaggtgatccataaaagcctcaagtttggctgcatcagtcaacgtcccggttggattgttgggattacagatccaaatcagcttggttttgtcggtgattttttgctgaaagtcgtccagatcgaactggtaatcatcggtcaatgggatttcaatgaccttggcgcccattaatcgagacacttcccggtacaaccggtacgactgtttggcaatcagcacctcgtcaccggcattaataaacatcttggcaaccgtttcgataatgttgccggcaccactacccaaagccacattctctggttttaagccgttttcatccgccaatagctgaatcaaattgacaaagtcatcttccggataccgattcagtgtgctgatacttctaatcattgcattcttggagtggtagtacggcgcataaggattctcattagagcccaacttgaccactttatccaaatgatactttcgagcgacctcatcctctgtttcaccttgaatgtatggttgagtcacattgacttcatttcgaaatgttgcatcaaattttgccatcatttcaccgccttaatcacaaattaaatatctttataagtccatcctaccgcgaattggcttggaattgtgaatgattgttctggactaaaaaagcccacctccaaaaagtgggatggaaaattattgatcaattgtgactgattccatcacaacgtcttcattaggcttatcctgagcatttttctcaacttggctaatctccttaaccacgtccatgccagagataacctgaccaaaaacagtgtgtctgaagtccagccaaggcgttccgccattcttgtaggcttcaataatttcttcaggataaccggccgtcttcatttgagaaatcatcccgtcatcaacatgttcgttggaaacaatgaagaactggctgccattggtatcagggccggcgtttgccatcgacaatgcgccattgatgttaaataactcaggtgaaaattcgtcggcaaaattaccgccaaagctgctctcgccacccatgccggttccggttgggtcgccgccttggatcatgaaatcaggaatgacccggtggaaaataacgccgttgtaataacctttttctgccaaggcaacgaagttttcaacagtctttggggcttgttcagggaacaattgaaccacaatatcaccgtgattggttttaatggtggctttgggtcccttggcattctttaaatctaattgaggtaacgtcatgatatatctcctttagttaacaaaatctatcttaaatgagcttatcacacccagttcataaagtcaggaacttcgacggtatttcccccgttttaaccccaattacggtaaaatatggataaagtttactttataaaataacggggtatttgtgatgagggttaatcaagcgcactggcggcgaaatatttatttgttcttgacgagtcaatttttgactgggattaccagcatgatcgttcagtatgccatcatttggtatctaaccaaagaaaccggctcggccaccatcctcagcatcgcgacaattttgggcatgctgccaatggcactgctcagtccatttgtcggaccgctggtcgatcgctggaacaagaaggccttactcatcgttccagacgtggtggcggcaatctttgcaattatcctgtcggtttccggcggggtgtttcacgtttttccaatctggctgatttttgtgtcgttattaatgcggtccattgctcaaacctttcaaatgccgacgattcaatcggtgatgccaacgatggttcccgataaggaattgacaaagctcaacggtcaactcggcatggtccaatcagccaatatgattattgcaccggctctcggcgccttcctgtttgcgattatccccctgcaatatctgattttgctggatgtacttggcgccatcctgggtatcagtatcttgatctgggtccagattcccaacaacgaaaagatcgacgctgctctgcatatgctgcacaacaccaagcttggcgttcaacaactcatgcacaataaggggctctggtacattaccatcaccggagcagtcttcaccctgctgtacatgccggcggccagcatgtatccgctaatgacaatgaaatatttccagggaaccgttggccaagctggctttatcgaagctttgtactccggtgggatgctggtgggcggggccatcatcggtatctggggcaaatggtccgacagaatgaaaccagtgatcattgcattcttccttgtcggcatccctaccggtttaagtggcctgcttcccggtaaccagaccgggtttatgtggtttgccattttaaatgtcgtcgaaggaattgccacaccgtttttcaacacgctcttgatggcaatgattcagcagagttatccccctcagcaactgggacgagtcctgggggtactaaattccctgatgagtttaaccgggccaatcggactaattttcgccggtccacttgcggatgcattgggagttgagatgctctttgtcatcgccggaattggcacagtcgtttgtggtatttttgccttgatgatcccaatcatgcgagaatatgatttgaaacttcaagcccgactcgccaaagaagattaattttaaattggtagttgccttaaagtggacttcaaggtctacaatgactttgtaaataaatgtaaggggagattatttgatgaaatcaacattatttgtaaaaccaggaaaagttgaaattgaagagattgacaagccaaccatccaagctgatgacgacgttattttacacattgtccgtgcctgcgtctgtggatctgatttgtgggcttaccgtggcttggaagataaggaacccaattccgaaaacagcggccacgaagcgattgcgatcgttgaccaagtcggcaaagacattaccaccgttcagcccggcgactttgtgattgccccatttacccatggatgtggacactgtgctgcctgccgtgccggttatgaaggcagctgccaaactcatagcgataacttcagttccggctaccaagccgaatatgtccgttaccagcacgctgaatggtcactggtcaagatccctgggaaaccagccgattacagcgatggcatgttgaactcgctgttgtcgttggctgacgttatggcaaccggctatcatgctgcccgggttgccaacgtcaaagctggtgacacagttgtcgttgtcggtgacggtgccgttggtctgtgtggcgtgattgcttctcaaatgcgtggtgccagccggatcatcgcaatgagccgccatgaagatcgtcaaaaattggctactgaatttggtgcaactgatattgtccctgaacgaggcgacgaagcagttgccaaagtcatggcattaaccaacggtgccggcgcggatgccgtactggaatgtgttggctctgagctttcaacggaaactgccatgaaggttgcccgtccaggtgcaatcgttggccgagttggtctgccgcataccaagaagactgacctcagcagctcgttctatggcaaccttggcattgccggaggtccagcttcagtaaccacctacgataaatcagtcctgttgaaggctgtcttagacggtgacattcacccaggcaaagtcttcaccaagcgcttcaatctggatgaaattgacgatgcttatcaagcaatggctaaacgtgaggctattaagtcgttggttgttgttcaagattaataagagtgtgaaagaggacgtttagcaactaaattttaagcccctccagacggaaaccgagtcaggttttcgggtggaggggcttaaaatttggttgctgtcctctttcacacgtttaatcaaaataacagtgaaacgcacggaaaccgagtcaggttttcggctggtggcgcttaaatttcaattgctgtcctctttcacacatttcaactagatatcaatagaacccaagagaggccgggacacaactaacaatcagttgtgtcccggcctctagtcttttggctgattattctctttcccgtttcttaccaaatccaagccaaccaaacattgccaataagatcatgccaatgattgaaaccgcttggccagtttcggtatcaccagtttgtggtaagactgcttgtcggccttcgttagttcctttctctgtagctgcttggccaacagcttgggttgttgcttgcttagcttggccggcttgagcatcgttagcaaccactttgccaggatcattgaccttcaattgttctttgctattttgagggtcttttgcggtttgcttcttcgatgcttcaggtgccttttcgccagtcttgatcattcctggttcctgagactcggtcgggtcttcatgaacgacattctcctgcggtgtcggatttgtctcattcggcgtaccaggtgtattcggtgttggcgtcggagttcccggagttggagtgcttggtgtcggtgtgactggcttattaggatccacgttgccaccaggcgttaccggatcctcagcctttttcggtgccactggggcaaccggttcttgtggctggtcaaggtttggctggtagtcggccacgactgtcgttccagcttccggtgtcgttggaccggtcacatcgaccactttggttccgttattttcgactggtgccaccggtgcaactggctgttccgcattattggttgggcgggtttcatccaaaattggttgggctggttccttggccttttcatcaacgttgacgactttaattgcggccaacaatggttccgtatagcccatttgattaaccccgacaacatatgagttgtaagccacttcatctttgagtttgtcgtttaactcgccaaccccaacctgtttgccggcttcagcatatttggagataaaggttgatttgtctggaactgccaagttaaaggtaatcccttctgccggacggccattgatggtttgccctgaagtgccgggaagcatgattctaaaggcggtgatcttcgaccagtcagtcactgaattttccagctgccaagtcactgcgctcagatccttcaacacgtttgcctggtcctcagtggtgtagtaaacgttgactttccctgtccaatcggccggcagaacaaccggaccagtcaaaccagccgtataggttgaagttctcacatcagatgttgagacaccttcaattgaaccggcttgcggtaagaaatcaagtaagtcaagctgtgacagactctcatccgtattgtcggtaaaggtaatcttgacggtcgcctgcttaccggtttcaactgcaacggcgtggtgataatcatctttgtcgctttggctgaccaattgattgctctgcagtttggaatctttctccaaaatgtagtagttacctgatgtaatcaaaggtgtcttggtatcaatcaaaccggtggttgagccatccgcaatcttctggctagttgctaaagtggcgttactaatcgctgggactgagacaatataattctcagtatcgggaccaacattaatgaagttctggaaaaccatatcttttggcgcactcttatcaatgttgacaatcacccgagtcgcgccgttctttcccggtgttaagttggaaatgtccgtccagacaatcttaagcacctgttgaccagagcctttaaagttatcaataactgagtattggttcccatacggaatgacgccggattgttttgaggcagccgcgtcgaacgtgacaccctttggcagaaccgtgtaagtttcaaatggtgtgtctctggcaaccaggttaccgagtgaactcttgtccagcacaaacccaagggtcaattgatgagcaccagtctcaagaactgagcccgtggccttgccgtcaaggaaaattgcagaagtgacgtaacgactggcatttttatttggcgccgcaatttcgattgtcgacggtttgaggaattgccagacaactcctggccaacctgatccttcatcgatggaggcttgctgttcggcctcgtcctttgccagccaacgccataagccttcaggggcattggcatccgacacccaatcctgcaaactcacataggttctggcattcgaccaactgaccttaggggtcatctgatgcacgatcgttccaggcgttgcgcctgatttgacagtggttttgaagtagacgccgccataagtgccatgcggtgcccaggatccagcaggtaacccaccatcttcgggagatttcaacagatcccgtttcaaaatcgttctttgagcaccgttcttatcggtaatggtgattgtatcattcttataagccttgtacgggtaatccggatattggtagatactttcccgactaatggtatccggattctttggaatgtcacccatgcccttcttatgcatatagagatacaattcgaccacattctttgtcggatcaagtccggctgccaataattgttggcgattgatatagatgtacccgacagagccatcgttgccgccagtcgcaaagattgggttaccatctttatccttttcgacatctgaggtgatggttggcagattatcaaataaagtgtggtactggttctgtccctcaccctcatatttcacagccagtgacaagtatggattttccttgaagtacgtccattcgccgaccgccccagatggtgtcttggaatccttgatactatttgaaggcaggtagacaaagttgtggatgataaccgtctctaaatcctcacgcggatcgatcgactggtggagtgcataatagttaaagtcacgcagccgttcgttttggggaacttccggatctacatcattaaatagaaatagcggcagcaaagcatcatagaattccaagacagcgttcgcgtcggaataaacttgtgggtccggattgagcaaatccttatccgccaatgcgccaaaaccgtcttttgagccgtagtgaaccatcggtttccaactcccaccagtcacgttccaagtggttggatcatgcggcagtaccatggtagccgcgatcttgttcattaactgattgattggctgggcaccttggaaagtgaagccgactccgacatcagtcttaagccactggaagttggcggcgtctttgttgaccttggcgatcacttggaatttcagcgtttggtccttagcaatttgatccgccacgtcaccggccttaattgtccatttaagaacggttgccggagacccatctttcagttcgccggtggaaatttcgggagctgtgtcaatcaagccgttttcagcggttccttttgtcatgccaacataggtctgctcgccagccagataataataaacgttcacatcactacctggttccagtagtgcattcttcggttgggcagttgggatcgtcacactgaagtcccaaatggcctgatcttcttgagccggattcttgtattcattaccataggaatctgtgtagacgttagccggggtgttggtcaccattgccgaatacgccatggccatcgtctgtgaggcactcagggtgacaggcgttgagatttcgtcggccttaaatgagatgcccatcgtgaccgtttggccattgatcacggtgtccttttcggtgccatagacatagtgaaggtcttgggcgacgccactttccaatgtatcccagtggtaggtcagcgttttagtggcggcgtcataagtgggtgtcacacccgcaattgcgtattgactgagatcagtggcgtcaaatgagagccctttgtcggctggcaggttaaccaccatttcagcattggtataaatggtccgaatcccattggcatcaaaatgcagatcaaatacgccgttatcgccgacatcaactattttagcagtcggtgtaacctggaggccgggtaggatcggattagcagtcttttccggcgcactttccgctaccgctttctcgaatgccattgccttggcgtaagcctcatcccagactttcatttcttcttggtaactcttcaattcaatcagatactggtcatttaactcagccaaacgggtggttaaggtatcataagccccctgggcaacactatacctctcggccagtttgtcgtgaacgcctttaacggcatcgaaatcagctttcaattgattgtaagcatcggtcttggcgataaaatcaatcccggcatcggtaaattgtttttccaggtttgcaaaggtggtgtgagcttgttgatactgctgattgattttttgatattcagcgtcgattgctttgaattgatcggcagttgccttttgtttttgatcagcatccttgaattgcggctgcaggtcgtcgatttgcttttgagcggcgtcatattgggtcttaactgtctggtattcagcttcggtcttttcataatctgctttggtttgcagataatggtcctggatcgccttaaactgagcatcggtcgaagtcccctgccctttctcatactgagctcgggcagcttcatacgcacttctggctgtttcatatttggcgagggcactgtcgtacgtcgtcttttgagccgtatgggtggtgaccgcagcttccaccttatccttggcagcttggtagtcagcggctgctttgtcattcaatgccttggtctgatcgtagtcctgtttcttttgatcgtaagctgttttggcagcttcatattcggccttcgccttctcataggccgccttttcgctggaatactgggtttgattatcctgatatttttcaagcgcctggttatattcggccagtttgtccttatacacggttaattgttgatcataagcattcttggcctgatccagctggttggtaatgatttcgtaaagctttttactggcgttatacacgttgaccgcttgatcatatgacaaatcttcggcaatggttggctccgtagttgcctgagctggcgccggtgtggcttcggttgccttagattccggtgcctgagtttctcctgccttggtgtcagctgccttggtttctgtttccttggttccggtttccttagtttctgctgctttatcaacggtggtattgttggatgttgatggcttggcagctggctggttagtgtcagtctcagctgcttttgccggctgggctgcttgaggtgtcgctgttgcctgagcaggctgttgggctgcctgtgatgtacctgggttggcagcttccgtctgaccggaattgaccggttgtgactgtggctcagttgttgactcggattgggacttgggagtctgcgcagtcgttgactgttgggtctcagctgctggcgccggttgagcagtttgtgatgctggcgtcgctgtttggtctgcagtcgctgtttggtctgcagtctccgtagttgccgtagccggttgggctgctggtttctgtgcggtagctggtgcagttgttgctgtcggtgcactctcactcgcagttgccgtagccggttcgggagctgcatttgcactaccagccgaatttccttgggtggtcggcgttgtgtctgcagatgcgtcggtgaccgtacttaactgactgccaacgccaaaggcagcaactgttaagccggcaatcatccatcgcttgccagctttatacatcttataatgtttagcagtaacatcctcctgattaataattcccctgtttgatgatttcattgttttttcctccaaaaatgacagtaaagttgtctgcttccccttagcaatattgacatcatttcttttacaatgtaattatatcaggcgtataaagataagtcataagtaatgacctaatcccgatatgacaagttttcatcatatttttccattactagtccattatcgtaatacgtaaaaaaagaacggttatgataatcataaccgttctgatattaaagtacgttaattaattcctaattttttcagcagtcaatcccattgcattcaaggccacgataatggttgacattgccattacagcagccccaacggctgggtccaaaatgatgccggcaaacgctaagataccagctgccagtgggatggcaataatgttgtagccggctccccaccagaggttctgaaccatttttcggttggtaatctttgctaaatcaaggaagtgaagaatgtcactgggttctgatttaaccaggataacgtcggccgaatcaatcgcaacatcggtcccggcaccaattgccacgccaatattggcttccgccagacttggcgcatcgttaacaccatcaccgaccataatgacgtggttgccctttgcctggtactcagagacaatcttttgcttgtcattgggcagcaatccagcatgaaattcgtccaaaccaagcagtccggcaacgtgttcggctgctttttgattatcaccggttaacatcactggcgtaatgccacgttgtttcaatccggcaatcagctctttggccccgctcttaatcgtatctccttcggcaaccatccccaaaacttgttggccttgaagcaggaaactaaccgagttgcctttggctgcccattgatcggcagtcgcgttatcaaatgaaatcccgttttttgtcagatagttaccgttgacgatcgtataattctggccgtcaatctcgcctgaaatgccgacaccagggatgttttgcgaattgttagcagcctgaaccttgatgcccttttcttcggcagcagcaataatagcctgtgccagcggatgggtagagttgctttcaagggctgccaatttacttaacagtgattgttcatcagtatccgcagctggtaccagggcgttgacagtaaatttaccttccgtcagcgttcccgtcttatccaacagcacatgactgacgtgttgactggcttcaatggcttgacgattccgtaccagcaaaccattttgcgcaccaatcgacgttgaacgggcgacaaccaatggaatcgccactcccaaggcatgtggacaagcgatcacaaagactgtgaccattcgggtcaagccggtcgatagtccttggggtaaccaggcaaagaatgcgatgattcccactgataaggcggcatagaagagatacttggcaaccaaatcagcccgatcctcagcctttgatttcgactgttgggcctcctgaaccattttcatcacttgtgacaaatagccggattcaccggtcccggtgatttcaactgtcaacgttccgttattgttggtggcaccaccaatgactttatcgccaacattcttgttaacagcggcagattcaccagtcaccaaggcttcattaacggttgattgaccattggtaatggtgccgtcagcaggaatactttcacctgagcgaacttgaaatgattggccgacttgcagatctgatacttgaacatctttggtttccccattttcagttaccaaatgagcggtcttcggcaatagagccgccattttctcaacggcatcgccagcacccatgaccgcgttcatttccaaccaatgacccaacagcataattagaatcaaggttgccagctcaaacgagaagtccatcacatgagtggcagtgtgcatcaagttattggcaatgaatgcataaatactgtaaaaatatgaaactgaaatacctaacgtaatcaaagtcatcattgccggtgccttactcttaacttcagcccaggcgcccttcagaaatggtgagccgccgtaaaaatatagtgccgtatcaaataaaagaatcgcaattccttcaatgagtggggcgtggaagttcaacacagcgacgtccaaccccatgatgggtgctaatagcaatacggggatcgccaagaccactgagacccaaaacttttgtttcaggttacccatgtgcatcatttgaccgccatgcatcatcatgtcgccgcccatatccatgccggacatgtccatatcgccatgatccatctgcatttttgaatgatccatgctggtcatatcatggtccatattcatcttagaatgatccatgtttcccatatcatggtccatattcatcttagaatgatccatgtttcccatatcatggtccatattcatcttagaatgatccatgttgtccatatcatggtccatattcatatcatctttattatttgccattttaacgatcctccccacatgtcattttccccggcagacagttgcattgaaccatttccggagcatccttggctttctcagccaatatctgctgcaattctgcaatgtcactttttgacaattcgcgtgtcttgatcacttgggcaattgtagagccggctcgcatcgcgcacatatgatcaaataaatcgtccgccgcagcggacattgattccttttcgccgacgaccggtttaaaggtaaatggtcgactatcgccgatttgttcaacagcgccctttttaatcaatcggtgcaagagtgtcttagttgttgagtcagaccagccctgtagttcattcatcgcgtcgatcagctcgcgactggttgtcgaccccattgtccaaattgcccgcataacttcccattcagaatcggtgatggtaacatttttagcatctatcattttgataacctcattttatttttcttttaaagtttacatttgtagctctcaacaactacagtttacatctgtagcctataagatgcaaccatttctgttcgaaaattccgtttcatccacaaaaaaggcgactgggacgtgtcccaatcaccgttaactcacattaaaaatgttttcccaaaatatccagactgcgccgttgcccatccatttcggcaacatccggtagatgtccccaaaccgtaaatccattgtggataaagagcttttggctcggcaggttgtggctgaaaatgaaggcaaccagggcatccagtccgaggcgttccaattctccactgacaaagtcgattgcctgctgtcccaagccttggtgacgataatttgcgtcaatgtaaatactaatctcagcagtcttctggtatgctggtcggccataaaatgattccaagccaacccacccggctatttgatcgtcaaccttcatgacccacaacggtcgggtttcatgattgaactcagcaaaccagttctcacgagaggcaaccgaaaccggctctaaatcggcggtagcaaggcgactgggaataatctcattatagatttcaacaattcgtggcaattcatcgtgcgttgcatattcaaatctgactgacattccatgacctcattttttgtattatccatctattttacgtcaggcaatcccgaggcgcaatatcacgccaacgtgtcataaatgaccaaaaagaggtggggatattactcgttattgaagctttcattgcagatacgattaccactttgatattgatcaaacttgcgtcggccattcaacaaagaaacgcagtcattccaaagtccggaataactgcgtttcttcgttaaatgctgggatcaaatcgcgttagtcccaatctctttttgacttatttcatactggcagccatccgaattgcgacggcgggatcggttgcctgcagtcgatagactacactaccagcctgccaagtaatcacttgagctgaaccgccaacgttgaatttgacgactccttgagtatccggtgccggtaatgagtagctctcaaacatattgacacttgaaagcgctaatttcttcggcgtcgtgttattcacgggactgccatgaacactaatcgaccagttgccctcgttccaagaaatgtactgctgaccggctcctgattgagtatgaccaacaatcccgtggccaaggtcaactttcgggagccctttaatttccgaagcagccgtataatcgacatggctttgagcttccgaagctgaagagtagctgcgtttggctaagaccgcatacggcttctcagctttcaaactactgtcattgagtgcaagtgcatcattaccaatgctgtagtatatggtactgttactagaattcccattatatctgatatgaacgttcttggatgaatcgctcagtcccgaattttgtggcaataacgtatctgacaacttacttgacagatccttagttagcgatgagaaatcgtacgattgaccgtccgattgagcgttgctgtcagaagaagctgttgaggcactttgtccgctggtggtatcagagctggtggtcgaactgcttgagttctgcatatcggtctttgattcattattagaactttgtttaccggaattgccattactgcagcccacaagaaccagactcagtaataacactccacctaatttatagagcttcatcgtttccctccaaattgtttgcgtgaattattgtacgtaattcttattggcagttaagtagcggccgtcggcggtttcaaaatagtatgaaccactgtctcgtttgtgaattgccgtcacgttaactttggttcccggctgaactttaacaacccggttggctttcttaaagctggttgaatcatacaggtacagtttttgagtggtcgtgacgctgctgacaacgtcggtgaaataagttggttgcgcagtatcagctgattgagctccgccgatccaccaagtaattggcttgctggaattcaggattgtgctggcgtcaactgattctttcaatgcgggaacgtacttcttattagtgtactgccacaaatcggtttgaatggttggccgtgaagaataattggcaatccattgggcatcaaaattctttctggcagtattggcatgagccgtcgcaaaggactggtaggaataaaagattaatttcttaccggttaatgaacgcatttgatcgtaccaggccttaacagcagcattgcttgaacctgaagtcacgtcattttcttcgtagtccaaaacgtagaatttagcgttcttgttggaattttggtagaagacgttggcctcattacgggcactggccgcactggtgaaggtagcgtaatcatattcaccaaatggaatgccatattggacgtataaattggtgttattggttgcgtacttgtcttgatagttagcgccatattgccggcggttaataatgaaggaaacctgactcttcaagtttgaaactttcgaagccgttaatttcccctgccactctgaaatatctggaatgacagttgtggcagccgatgccttaactgccccaaaaatcgaaaccgataagataacggtcaaaatcgataggatgatcgcccgtccctttttcctcaatgaactcatttaaaaccactccgcatttatttatttgcttacgctaaattcaattagctaaacagttgtcgtcaatttctctaccaacatatgacagaatgggtttgagcacaagaaggccagcagtaagcaaaaagaatattacagagctgagtcgcgccatgaagcctcagcgattacttcttttcaagaatgttataaatgtgtaacataactgaaaaaatatcactccgacaaccgtcaatgaataaatcggaatgcgtagccgaatcggcatcagccgataacaaaagggttccatcagctcgatggaaccctcaagataattgaaaacttatttaacagctcgtgaaactgccgcattaacgtcagctttttcggcttgaaccagttgaacccgactatcgatgacactaatatccatcttgatttcgcgagtcaaaccaggtgttgggatctttggttcaaagaattctttgaattcagccaaccgttgcggtgtgtggaagatacctgaaataacggtaatgtaggtggcaaattccatatccccaccaaccgtatcttcgagccactgccagtcttttcgaatccagtcccatgcggcttgttgaccgtcatcattggcgaggaccccgcggaaccaagcccgcaagtcttgcggtttgatggtgtcggcattctcaaattgaccaaccaacttggcaatcaaatccgggtcagtggtactcgtcaaagcagcgcaaatgtcttgcttgtaactggcatcggcagtttgccggtaagcagccaataatttgtcaaataaggcttgactgccaaagttcttaacctcatttcgaaggacaaacacccggatatcagcagataagcctgccagattgccctcgttttgtttaaacaatgtatgagcagcagccatggcatcagcgttttcagcatacaatgaagcacttaaaatataaggtcgcgtcagttgatcatcatttgactcatcagccttgggggcaaagcccaatcggtcaagttgggcagcactcagtcgatcgaagaattgcttgagtgctttttcttcattagatttaggagtcacaaatttcttcaaattgttggcaacccgatacattgccgcattgacaatgttggaatggctgtccgcaaattttggcagcaacggcacaatattagcataggaattttgacgaccatcagctaacaaacggaggtcttggagaatctggagctgagaaattgcgtccagatcacccacatgatcaagaatatctgccattaaggtttcatcatattgaataatgaaatgtgaattgttcccaacgttcaagaagaatggtttgccgttttcttgacgcaactgctgataatcaccgactgtgaatgttttatcagccatgatttcaggcacggcgtcgtaattgctgttaagcggaatctgccacttgcggtcgacatccttgccggcaccgataaagaattgttgttgtgacaagatcaactggccgttttggactttggccgtcacaactggatatccaggctgctccagccacgagttcatgatggcaccaacgttcatgccggacgcgtcgcccaaagccgaccataaatcggcaccggtagcgttatggaacttgtgggcggcaaaataattcttcaagccttcccgcaaggccttgtcgccaaccaaagctcgggccattactaacattctggcacccttggcatacacgattgccgagtcaaaaattgaatcgatctcggccgggttttcaacttggacgtgaaccgactgaacaccatcggtagcgtctcgttggagggcagccggggcctcagaagtttggaagacctcccaaatatgccaatcaggctcgatcgcatcgattgcaacatattccatcatgttggcaaaactttcgttcaaccacagatcatcccaccacttcatcgtcaccagatcaccaaaccactgatgggccaattcgtgggcaattacggtggcaaccagctgtttcatttcaaatgaggtgttcttgggatccaagagcaggtaggcttcacgatacgttaccaagccccagttctccatggcaccggcagagaagtctggaagagccagctgccatgagtgtggcaatgggtacggtgtctggtaaaagtcttcataaaactcaattgaccgtttggcgatatccaaggcaaaatcaagctcatcggccttgtgcgccttggtagcaaacacaccaactttaacaccgctcttggtggtcgtttcctttttctgcatctcaccaaatccaaaggcgatcagataagtcgacatcctcatggtcgtatcaaaatagtgaacaccattttctgtgcggacttccggcatattgctgatgatcgtctcgccggcatgctcgtcaaacttaatggctaaatcaaaggtggctttggcttcgggttcatcgacacatggaaaggcctgccgggcagcggtggtctcaaactgggttccgatcagctgcttcttaacgccgtcaacttcataataagatggataaatgcccatcatcgtgtcagtcaatttggcactaaattgaatcgctaaggtcaccacaccggttgtcggcaaatcaatattgattgcttcctgatcgtcgtccttgctaaatgaaacggccttgccgtcagcttggaccgattcaatattgagaaacttttggtgaatcgaaattgctgtcgtcttcgcatcacctgtaatcgtggaagtccccgagaactgcttcgtgtcccgattgatgtccagatagatattgtaatgacttggttgaaatttttcgtagaaatgggttaattgttctgccatgagttgcctccttgaaaatttgttaattatattatacgactctggcaacgcttatgcggctcgaatggcaaaacattgatttttagctgaacatccgcgtgaccagtcgatcttgaatccgatcgggaatcaatttcaacaatttggccgtcacttgttcttgaaatcttatctgatagcgtaacttcggtttgcgcgtcatggccgctttgacaatcactgctgccacatcgttggtagttgcccgactgtcctttaatgtcttcgctaaacgctcggccacccgtcggtatggagaatggattggagtagccgccaacagtttaccaacggcaattttttgccagccggttgctgtattgcctggttcaaccacaaccacatccactccaaaaggtttaacttccaaccgcaaaatatccgacatggtttccaatgcgtgtttggaaatatgataccagccgcccagttgggtatacatcaaacccgccagagaagaaatattaataattcgaccagacttttgggttctcatcgtcggtaagaccaattgaattagtcgaaccaacccgaataaattgacgtccatttggtgtttggcttcctcgattgtcacttcttccagcgcgccaaatgaaccgtagcctgcagaattaaccaacagatcaactctgccatatgaatccaagacaaaggccacaaaggcttttaagcttgactctttggtgacatccaattcatgaacctttccgccgagttcagtcagcaccttcatttgttcaacgtgtcgcgcaccgccaaccacgtaataaccctgcttcaaaagcagtttggcagcagccaggccaatcccggacgacgcgcccgtcacaatcgcaacttttttcatcaaaaagacctccgtttcataaacgatagttctatcgttaatacttactgtgtataatagcgatagtcttatcgtttgtcaaggttgcaatgccagcactttccaatataatgaagatatgaaaattaaaacgacagaacaatataatcggattattcagggtgcgactgccattttactgacagaggggttggccgccttttcgaccaccaaagtcgccaaacacattcaaatggcacagtcgaatatctatgtgtactttaaaaataaagatgatttgctggtgtcggtctttcggtaccaccagaaaaagtacattcaatttttagtcgatcgcattgatctctccctgccacccacggatgcgcttaggaatttggtttcaacactcgatgaattccataggaccaacaaggaatcactcgacgttatttggtcgattcggcagagcaccactttacggcaactgattccaaaagtcagcgatgatcaaatttttattgccatttttcagtggctgaaggattggcagcatcaaggaactgtccgccaactaccactcatgtatctcaccaatttggtcttttccgccattatcgattactttcagttaattgatagtaaggaaatgtcaccaaacgagctggctatcgaggaaattgttccacccttatcagcattactctttgtctgagggaggcttgtcggatggcttgattactcgtatacttgaattctgacgtgctggtgattgaacaatcagcaccaattgatgcgaaattcattattctagggggaatcgtcatccaaaacacaaaatctcagcgttgggtcggcctgatctcgggactgattttaaacgcctttggcaatgcgctgaccatttcagccaacatgggaagtgccgtttggactgcttctgctgttaactacagtcactggttcaatttgaatgttggcattatcctgttttttatcggttttttgaacacggtcaccaaccaagtcctgctgcgacatccggattggccacggttcgtcggggaaatcctctatgtctgcttttttagttatttcgtgaatatctttgcccaactttttgaccaaattgggatcggccagttaccaattgtgattcggggcatcctatcatgtttggggattatcttcttctgtacggccatctcactgtatcagcgggcaaatattctcatgcatccaaatgatgataccaccaatattttgcggtttatgtatttgaaaaaaagtgccgtggctgcccagctggtcgattttgttccaccaattatcgcgatggtgatttcctttgcggtgacccacaatttgtatgccgtcaacgtcggaacgatcttttcgattcttttcaatggcttgattattcaaaccgccgatcactgggtttggccgactttgaagcataattttaaaactttggggaatgattagtaccgtcaccaatgttctaccccttcaattgaatggtcgatacagacaaatgaaatcataaattgtcggtaaatccagttgcatcttcccttcaatatggtaaattaaacgtaaataagtcagacttaatcgctatgcagaaaggagtttggacaatgatctttatgttactcatgctttttttagtggggtatttggttctaaatgtcagttggctgttcattaaggcctcggcttggctgataatactggcaattgggtttctgatcttgtccaaactgctggtagttggcctgatagtcgctgccgtttatggcgtttatctgctttatcagcactcacaagttcagccatacaagaatcgccactaatccaattatcttgaaaatgttttacataaagagaaataaaatcattcaattgatcttatttctctttatttttagataattttacgattttctaaactttgtaaccgttttgatagaaaatttctttcataaggtatagtattacattattacttaaaattgaggagagttttgattatgaatttacttattgcgttacttcccgcccttggttgggggttaatgccactgataaccggaaaagtcggcggatcccccgccaaccaaatctttggaattggtgccgggacgaccatcatcggattaattgtcttcttggtgacccgaccggccgtcaacatgactgcgtttctttttgcaatcgtttgcggtgctttgtggacgattggtcaaatcggccaatttatatccttcaaacgaatcggcgtgtctaacacctacccattatccacggtgtttcaattagttggtaactcgattcttggcgtattgatctttggtgactggcagggaactcaatccaaaatcattggttttatcgccttgattattgtgattgccggagcgttgttaacgtctgtcagtgacgaaaaaggcggcaaaatcacctttaaggacgccacgttcttactttgcaccaccgttggttactggatctattcgtcattccctaacattccaatcattaaggcacaaagcggcacttccgttttcctgccagaaatgatgggcattttaattggtgccgttattttcggtttgttcaccgaccgtcaatcatttaaacaaaaagaacaatacctcaacatcatcgccggattactttggggagtcgctgcgctttcctacatttactctgctcaggcaaacggaaacacctccgcattcatctggacgcaattaagtgtcatcattgccacttttggcggaattacaattcttcacgaacacaagagtcgccgggaaatgatctttaccattgcgggtatcctgttgattgttgttggtagtgttgccacctcatttgcataattaatagatcagttgaaaaggatggccaccaggcattgtgcttggtggccatccttttcaatttggatttaaggttgtccaatcccactcttcgtaaaatcattgagcagacgggcggtgacccgtttaaagaagtctttcatgaacaggccgacgatcaagcccgcaatcagcatacagatgagcacgaagaagtcgagaaccacggtaccaacattgggtcctccaacggcctcccgaaagccactgacactgtacgaaaatggcaaaatcggctgaatgattctcatgaacaacggattcaattgaatcggataaattgccccacttccggccaactgaaaggcgaccatcatcactgccaacgcctttcctaagttaccaaacaccgacgccatcgtataaacgattaccgagaacgtcagtgatgacaccacgccgatcatcaccattaggaacaaactttccacgtgaaccctgagaataaagacggtcgaaaggacaatcaccatcgtttgaatcatcgacaaggtgttaaacagcagcatcttgccaatatattcttcacgcggccgcaaatttttgaaacgatgatatttgggcgccgaggtgtgcagaactgcgaccagcatcgcacaccctacccaaatcgatagggccatgtaagttggtgcaaacgcctcaccaaatgaactgacccgataaatgttctcatttttgacgttaaatggttgggccagtgcgttgcccatcaacttgggattgttctggaggatgctgataatgttggcaatattatcgtctgaagtcaatttcaactgattacttgcctgcaaaatcacgcccttatactgaagcagctggttctccaagtcgccggtggagtcactgaccagttgattgcctgaaataatcgtatccaacgacttttcgttcaagctgcgaatgtcattaacattgttcaagacacccgaagcgtgattgctggctgacagcaggttgcgttgaatcccgttcaattctgatttaacgttgcgattataactcgccagtgaatgattcaggccgctggcaactgaataggaatgactggcaattcgctgctgcaggccggtattggccgtactgcctgaactaagcgcccgctgtagttgggtgacttgctgagactgggcatccagcagattcttgacgtcattgagttggctgattaaccgactcaccccactcaaccgctgcgattgattaatcgtctgcagataagcaattaatggcgtgatctgccctcttagtaacttaatctgcgacaaaatttgactagccaaaccagtggcctgattacggccggccgcagaagtctgcttgttcaactgattggtgagggaccgcagtcgtgcggcgtcagtttgaatcccattcaagctggtttgaacgttgccaaacgattggttaacggcctgattcacactccgaatcaactgctggttcgacgagccaatcgcttggttaatactgatatcctgagatgctgaaatcaccggcttcagttcagaaaagaccatggccagcccactggaggcttcactgatatctcctaaggtattggttgccagttccatactgtctccaagattgataatcaggtcctttaaattgagaatctcggattcattgtcaccagcctttttaccagccacattcaaataggtaaaaatggtgctgttaacttggtatacgaattgttttttgatcgtgttcaacagcgtctttgaggcggcttcggtaattttgtaactcattggactggccttggtgtcagcgatatagtcgatgtgggccttcttcggattggcagtcacaatactgcccaaatcagccgaaaaggtcttgggaattttgatttcggcgtaatactttccagcgcgaactttcttttgggcagtctttgaatcaacaaaccgccagccgatctgattattgtgttttaactgggcaatgatctgcttgcccaaattcatctgtttaccttgaaccgttgtgccttgatcgttattgacgacggcaaccggaattttttggacctcgtgggaagtatacgggttccaaatggctttgacgttgaccaacgtatagagacagggcaaaatacaaagcgcactaatcgtcaataacgctgctttgtacttaaaaattgccttgaggtcccgttggtaaatcagtttgatatttttaaacattgttccatccctcaaatttccttgctacttgtttctgtcgaaaaatgcattatactgataataacgcgtatgcgaatgattaacaatggtaactatagttaacaacattaacctacttttatgagggagctataatattatgaaacattcagttattaaatggatactatcactgaccatcttaggggcgctatttgctattcaaccaaccaccgcgtcagcgaaaaccacagcggccaaggtcaccagcacccagactttaaccacggcaccctaccgtgcagtcagtggttatctgtacagttcggccaaattaaccaagaaggtccataacgccgacaattatcctttaaccactttttacgcttctaaatcggcaaatatccaacgggctaacggcaacaaggcagtctattactatgtccaaaatggtaacggtaaggtcgccggctggatctggcgtggtcatctggtaagaatgatcaatgtgactcgtcagcgacaacaactaaatcagattatcggcttgattgacacattgtccaccaataataaggaccagctgatttcaattctcaacctgatgaatcatcaaagcaccctgcccgacttgctaacccagttaaatagctggatcgaatcaattcaaaatgatccagacattgccaaactcaatcaaatctttgaaatgatcaaatccgatggtcaaacactcaattacttgtttagtgaggggatcaacaaactgtatcccaagatcgtggtcattcataacctgaacaaccgcgtatttgcgctcgcccaaggactgcttgatcgaatcaattaaaaggacccatttatgcgaacaatattaaccttactcaaacgtgacttacacaatatatttcatagccggccggtgtggataaccctgctggctttttgtctgattccggccatttatgcggtccccaacatcatggtctcttgggacccgtattccaaggccaataccagtcgactgccgatcgccgtggtgaatgacgatgagggcagcacggtcaatggcaagcagctgaatgtcggcaaacaaatcgtcggcgaactcaaacaaaaccacgccatcaactggatcatgaccaatgactggcagggaaacaatggtttggatgaaggaaagtattactcgctcattgaaattcccaatgacttttccagcaagttggccacactggtttccaccaatcctgagaagcccaatattatttataagtccaacgaaaaattaaacccggccgcaaccaaaattaccggccaggctgtcgacacgttaaccgagcaggtgcgggacagtttcatcaaaatcagtaccaaagccgccttaaaagaaatgaatgccgccggagccaagattaacacccacaaaccggagattctccaaattcgttcttctttgttggacgccatcaacacggtgaagaaaaccaatggttacctggataaggcaaataaggactcagacaatgtgcagcaatatctcaaaacggtccagggagacatcccgaaaatttcccgtcagataaccgatctgcaaaatgttgtcaatcatggtcgcaacttaaccaaggccaccaaacaatctctcagttcagcgcaaaatgatttatcaaacggattaaatgaccttcagtcagataataaccgcatcaactcattggtcgatgacctgcagactggcggacacgcttcaagtaagtcgctgttaaacagtgaaattaatcaactgaaaacactgaatgactcgacgcttaccggcatcaataatgccctgcgaatcgccgacgtgttgaataacctactgccaaacaatcagacgacttcactgatcagaagcctcagcaatgccaaacagcgcatccatgatcagcagcgtaatttgaccagcctgaaaaacgctaaccaagccaatcgatcgcaaaaatcaattaatcaactgattaagcagcttgcaaaaacgaccgacgctttgggtaatagtctgactaacgcgggatccacgttcaccaacacggtcagtcaggcgatcgacgacctcaacgataccttggacacccagttgaatggcaatgatgaagtgctgtcatccttaagaaccctgttaccacaactaaatgcgttaacttcgtctggaaaagcaatcagtaaaatttcagtttcccaggtcaaccgaattaaacatcgcttaaacggcattgaagataaactgaacgacttaaatgaccaaaccaaattcatcaacgaaaagaatttgaataaaatcattaacttattgggtgaaaatcccaagatttcaaatttgctggcatccccaattaccttgaaacaaaagcagctgtataacatgggcctcttcggctacggcatggcacccttttacacagtcttatcaatgtgggtgggcgtcttactcctcaccacgattgtctcgtggaaatacctgattccagaagacaaacggttcccaaaagccaaccggattcagcaatacgttggtaaaggccttctgtatctaattctgtcatttacccaaaccaccttcatcatgctcggtgaactggtcatcattggactgcggccacggagcttgttggcaatgttggcaaccgcctatctggcaacgaccgttttcaccatcatcatgttcacgttggtctatatgtttggcaatattggcaaagtctttagtgtcttgatgatgattgctcaactatttggaaccggtggtgtgtatccacttgaactgattccttcccatttggcaagcttggcaccgttcctgccatttacctacgtcatccaagccttcagagaggccattgccggaccgattccaagcgtctattggcacgcaatgctgatcctggcagcgtttggcggattctttctcctaatggcgccattgcggcgggtgttcgtcaaaccactttcgaagatggaaaatgggtttcataagtctcagttgtaaaattggatcattggttcagaaaaggcccacaaaatcatttgctgattttgtgggccttatttcgcgaagactgctaaaggatccgacgcatatccaacccccgggcactgcggatgttttcaatcacaattaacgcattcttatcttcactttcgatgatcggtaccaatttggtgacccgccggggaccagcaatcatgtacaacatgtgctgatcggcatcactataatagccggtgccattaaaaatcgtcatttcctgatttaattctttggaaatggtcaccgcaatttgccggtactttggtgaaaccaccagaacggcctttttagcaccaatattcgccaaaaactgattagtgaacacggagtaaacgtagaggtagatcaccgttaaaacggtattggtgaacccaataatcatgataaacggaaccacaatgaacaggtcgaatatcaaactcccggtacccagtgagatgccaaaaaagtagttgagaatcttaccaataatcgtatccccggcaattgtgccgttgaagcggaaaattaaaccaattgagatgccggttaaggcgccggctaacagcgtcggcacaattaactcatgggtgtgatatgtataaaacaccggaatcttgagaaagaccgtcatccatgcaatcgcccaaattgtcagataagtggttttcttttcaaacaacttgtagccaatcacaattaacacggcattgatgaggaggtttgacaagtacgacggcaccccaaaggcatagtataacagtgctgtgattcccatcgctccaccttcaccaaggtgagaaggcaacagcagataattataggtcatcgaatagatgaacgccccgactgctaccccaattaattcggtcgatttaatatttagttttcgccaataattccaaattgaattcatttcgcacctcaatcttgatatgtgattttcattctaccattaatggggtgcggttggcagtcccacttttcattgtttaggctgaaatcatgaaaatcacagaaaatataaaaagtccaaaatcaagatctgattttggactttcataatatcaattaatttgttattcccattcaatcgttgccggtggcttgctcgtaatgtcatacactacgcggttaatgccatcaacttcgtttacgatccgagtggagacattttgcagaacatcccatgggatccgtgcaaagtcagcggtcattccgtcaacagagttcactgctcggatggcaacggtgtaatcgtaagttcgaccatcacccatgacaccaacactcttaaagcctggtaaaacggtgaagtattgccaaatatcgcggtctaaaccagctttagcaatctcatcccgcaggacccaatcactatcgcgaacaatcttcagcttctcaggagtcacttcaccaagcacacgaatgccgagacctggtcctgggaacggctggcgccaaacaagcgtttctggcattcccagcttttcaccaattgcccgggcttcatccttgaacaacgtgttcaaaggttcgatcagcttaaacttcatgtcttctggcaggccaccaacgttatggtgagacttgattgtctgagcagtatcagttccactctcaaccacgtcagtgtacaacgtgccttgagccaagaaatcaatgccatgaagcttgctggcctcatcgttaaacacttggatgaactcgttaccaataatcttgcgtttcttttcaggatctgtgacacccttcaacttggaaaggaagcggtcctgagcgtccactttgataatgttcaagccgaatttaccgaccaaactatccatgacctggtcagcttcgttcttgcgtaacaagccgtggtcaacaaaaatactggtcagttgcttaccaattgctttgtgcaagagaacaccaacaacacttgaatcaactccaccagagagacccagcagtactttcttgtcgccaacttcttctctgatatgttgaatctggagatcaatgaaatcatccattgaccagttagcctctgcatggcagacgttgaaagcaaagttcttcaagatgtcgttaccatacttggtatttctaacttcagcatggaactgaatcccatacaaattacgctcaacatcctgcatagcagaaattgggcagtcacgactggtggcaactgtctcaaagccttcaggaacttcgttaaccaagtccccatgactcatccagactggttgctcacgtggggttcccttgaagagaactgcatcatcagaagtaatctgaatatcagcatgaccgtactcggaattggaagccttctcgacttcaccattaagggtatatgccataatctgcatgccataacaaattcccaagattggaattcccagcttgaagatgtctgggtcaaccttcaaagcgccatcttcgtacacactatttggacccccggagaaaacaattcccttggggttcatgtctttgatctgttttgcggacaatgcgtgggacttaagctcagaatatacgcctaagtcacggatccgtcttgtaatcagttggttatactgactaccgaaatccagcactaaaatcttatcgaagcttgataagtcaacgtttgccaaatcatacaccctttcaaagttcttacataaataataaacgattcacctaggtttggtcaacattattctgaaaatccaaacattaatattttctcaggtacaatcgatcgatcaaatgattgtccgtcttgtgcattatcatatcagctcgcgagcgagttggcaggatatttgctcgcaggttgggcaggtcgatggtgtcccacactctgcgggccatatcaaaggcctcctcacgatccccttgcgcgtaatcatagtaatagttgtcgggatcttggaaggccgtgtccatcaagcggccgaatcgttccaagtaccacttctcaatcaaatggacgtcagcatccatataaatcgaaaagtcagtgaagtcgctgacataaatctgctcgttgctgggtaactgcaacgtattgattccttcaatgatgagcacgtccgggcgatcgaccaactcaaagcggttgggaatgatgtcataactttgatgcgaatacaccggtgatttagtgaccggcactcccgacttgacctcgttcaaaaatgcgattaacttgcgcatgtcgtaactctcagggaaccccttcttgtcataaatgccgcgctgcttcagctcagcattcgaatagagaaacccatcggtcgtaatcaacttaatcgtctcgccggtaaaatagttggaaagcagttcctcaagcacccgggccgtggttgatttgccaaccgcgacacttccggagattccaataataaacggcacggttcgcacctttttgcgcaggaaccgagccttggtggtctgccattgatcaaagttgtttttctgcaggcgaatcatgtgcaccaacggtttgtagatgtcagcgacatcctgcagcgagatttgatcattgaaggccttaatgtgccgcagttcgttggacgtcaacggcaaatcgacttcattgtcattattaaaatgtttccactcatctttggtgaatgaataatagtttattaaatcatccatgcattttctccgcttattctttactcaaccaaataagtataacattttcagactgccccgagaaccagagatatgttttcacttgaagtctgccagccgacataaattaggtaataaaaaatcggaccatttcgatccgactcatgcttaattcaattcatattcatcttgaggcaccgtctcaaaaattggtgacaacgatttgactgccacaaccgtcaatcgatgcattgcccgggtacaaatcgtgtagaccagttggcgatcactctcgtccgggtagcaggccgtcgaagcatcccacataatcacactgtcgaattccaaccctttggcaaggtatgaaggcacgacaatgatgcccttcaccaaacgctgattttcagttcgaatcaatgttgacttgacacccagttcagcgagtttgccgcttagctcttgacattctttcagtgtcttgccaatgatggccgttgtttcatggtcggccaagttcaactcggactgctgtttaacctgctcaactgcagcatcgaccccgtccttgacgtaaatgtgcggcaggtcgccttgacggttgaatggaatgatattctcaccattggtcaacaggtgcttggtaaagttggtaatctgttctgttgatcggtacgacttggtcaattgaaccacgcgggtcttatcctcggggaacatgctgccaagttcgcccaacaatttacggctgttttcatgggtgaaaatcgcctggttcaaatcacccagcagcgtgaatcgtgcccttgggaaactgaatttcaagaatgccaattgaaaggctgaataatcctgcacctcatcaataaagagataacgaatatctttatcgccgcgtttaccagtcatcaagtcatacaagtaaatgtacgatgacgcatcagctaacgacaatctgcccttcttcaaacggccgacggtggctttgatctcttcggcccacaactcgttagaaatgccaaaatcagccagattgaggatctttggcatctctttaagcatatgaacaaactggttattgatactcaaccagtggttgcgagaaatttgccgctggacttttcgaaatgacttgataacaatccgtcgggccaggaacttgaattccttatcggcattgagaatttcttcttcaccttcggcatggaactgttgaatttcttctttagataggttttgaaccgcatcttcaacccactttttccgcatttcgacgtgaatcttgcggttaagaatcttcatcaattcttccttggttgactccagtcggttgcggaggttgtagttctcattgaaaccataatagatttcggcgattttttcttttggaatcaggatttcgccgttaaacatcaggtttctaaagcgcatgtcttccttgttcaaatggttggcgtaagcactgactgctcggaaataatccaagctgcctttgacgtcagtcagcttctgggcagtcttgtccagttgctcagtgaagcgctcagacagggtctcaacttgaacactcggcaaacggtgtgagctgtactgatagaacgtcatctgaaccatgttctgctcgcccagttcagggagcacctggttaatatagtcattaaacagttggtttggtgaaaataaaataatttggccggaatggagattcccgcggtattggtacaggagaaaggccacccgctgcagaacggcggccgtctttccggaaccagctgagccttggacaaacagtaaatcagaatcggtatcccgaataatctggttctgttctttttgaatggtggtcacgatactcttcatcttggtgtctgaacgattgctcaaggcatccagaagcatctggtcacccacgacttcttcggtatcaaacaccgtcttgatcttcgaattttcaatttggaattggcgctttaatttgacatcaacggtctgttcaccgtcgggcgtcatgtaactgacattgccgattccaccgttatagtaaatgctagaaatcggtgcccgccagtcatagatcaggtagtggtcaggccggtcggtaaacgatgccatgccaatatagatggtctcgtctcgtttttcgtccccttcacgaaagtcaatccgtgcgaaataggggttctgctcaagcttgttgagcgtcccaagttctcgggcggcatgttcctggcgattttcacgttcagaaagcatttgctgttgctgccgaatggacatggcagtttccatcatcccgctgtacgtctcagttttgagccgaacgtcattgttgaaattgcggttgatatctttaacatcccgcttggttgccttaatcttttgctcaaggtccttttgggaaatatggatttcatcaatgacgtggtccaaatggtgttgttcttgtgttttgatattatctgccattatttaccccctataacttgacttaatagtttagcataaaaacggtaccaattcaaaagacattatcgtttctggcttaacggtaacttaaatggcctgacattgttaattggtatacttgccattcgaccgatacactatggtataattgagatgttttaaataattgtatacttaggaggacacacatgacgatctcactatattttgttagacatggtcaaacatacttaaacaaatatcaccgtatccaaggagtgatcgactcacccttaaccgacaagggaattgccgacgcagtggcagccggcaagcggctttcacaaatcaaatttgatgcggcgtacagcagtgatacttccagggcaatcaagaccggccaattgatcttgaaagaaaacccggcagcaatcaaagatccagtaccaaccggtgcctttcgtgaactgaactttggctactacgagggcgaagatgacgtcaaaacctggcacaccattggcggccccatcggaatcaactcgtttcatggcttaattgccgaatttggtattgaaaaggccgaggacatgattgcagcggctgatccgtacaaagatgccgaaagcggtgaaacgttctggaaacggcttaaaccagccattgatcaggtagtggccgatgccgatgatggtgacaagattttgttggccacccatgggacactgatccggaatgtggttgccaaatttagtgacattccagtcgatgtgtcaactaagaacgggagtgtcaccaaggtcaactgggacggcaagagttattcggttgagtactttaataatgtgagtgaagatttatagaagaagcccaaacagccgcgagcaacattctgctcacggctgttttatattattagactggattgaatcagtctcctcagctgtcaaaccagcccctattgttcgttgaaccgcttcttcaacttagcctcactaaacgccatcaaactatccggatcaacctgatatttgtcacaaagaatcaggacctggtccatcacatcagctaattcttcatgcagattataattgcgttcatccctggtatcatgttcacctggatgatcgcggccgatttcaattgcccggattgcccgggacaattcaccgacttcttcagttaaaaaattcagtcgaatgaacggcgagtatttgtaccaatctcgtcgcttgtaaaaatcgaccagccaatcttgatgctgctttaacgtcattaatcaccactccattgtcttatgtctacttaaaatcatacacctcaatgcttcgttttccaggtcaacaaactaatggccgtacaagcaacacttggaatcacgaagttcggtaccattaagtcggcaatcgttgctgagctggcccacgtccagccaaaaagtgacaggacaaaaatcagttcaagtaccaaccaggctgctatgtacgggtgttcagtaaataatttatcaatcatctcctaatcctagtaaaccacataaatttgaagaaaatatgaccattccccccactcgtggtctgttataataagggcgacagggggttcacatcatgaaaaaattttgccagccgcaatcatcggactcaccggtattttgcttctcaccggctgtgggaacaaaaaagccgacatgcaggataaaacgacggccaatcccaacgcaaccaaattaaatcacttgttgtcaccggcaaccgccaaggtcccggaagattcgcaggcaacgaccaatgaccagctttattcccaattttataagagtaagggccagtggtactggaaactatcttccaaacaagacgggaccattgataacagtaaaatcaaatcacttagcgccactgatcaaaaagatgtttataatttttccatggtcagcaaccagcgcaagtcttacacccttaaattcaattggcttaacggcggccaccaggcttataccgtcaatgccagctaccatcatgtcaacagcaatttcatcttggcagacgccaatactgacactgattggcagacaggtgccccacaggccgtccagggaacttgggcaaccgacttcgctaacaattcaggcagcgatgcgcaaaagctgccttataccaaacaatttttgaacatcaccagctccgctatcagtagcttcaccaatgaatatgacaccaaccaccggctttataattcagacacgattgctaaagccagcaacgtttcctacaagcaaaccggcgatgacacttacgtcttaaaagcctacggcaatgaccaaacgccaatcgtttataacatcagtgtccaaagtaacaatcaaattgaagtgaatgggctgacctcgggcagtttgaccatgagcaaatcagccactactgaaccaaccactggttcacagacggccagttcgcagtccccatcaacgaccagcggctcgactgccaatcaagcagcgccgtccaccaaccacctcactgatcaacaggtggtcaattggatttggccctacgtgaaagccaaatatccaaatatggccgtcgattcaaccgactttacctacatgccgcagatgagaaacggtcaactgtacgtcaacgttttggagaatcacaactctcaggcatttaagaagagtggcgttgataccggcactaatccacaagtcgccagctttagggtcaccgccagcggtgctttggaacagatggacgcaacaaccggtgactgggcagttgtttccaatagctatggcggatagcaatgaccatctaatttagttttaaaaattcaaaaagtacccactccttaattgggaatgggtacttttttgtcggaccagacgcactgttaatgcgtgctggccattttaccttggtaatctttatcaatatgttcataatgatcaactttgtatttcaatttatcataggacgcctgcattttagccaggcgttcactgacggatgccagctgttcgttcaaaagatctttgcgtgcctgaacagtctgcttgccctgcttaaacagagaaatatagtcaatcaaatattcaacactgacaccggcgtctctcatacacatggcaaaagagacccagttcagatcttcttgatcatagtttcgataaccggcttgatctctggaaacagcaggaatcgcaccaacccgttcccagtatcggagcgtgtcggcggcaacgctaaactttttagaaacttcgttaattttcatcagctcacctcattactaactgatgataaaccttgaagtgcactttaaggcaagcgcctttcacattttgataaccaatgagtcgtaaaataattaatctttgttaattggcggcagctttttaatcaattttgccggaacgccgccaaccattgcgttatccggaacatcattggtgaccacagcgccaccggcaatcacaacgttactgccaatcgtgacgccgggcataatcgatgccttgccaccaatccaaacatcgttgccaatcttgaccgggaacccctgagccatatactttcgccgctgaagggcatcaaccgggtgattgaccgtatagatatcgacgttggggccgatcatgacattatgccccattgtgactggtgcgatatccaagatggtgagattatagttactcaaaaaatcttctccgaccgagatatttttgccgttatcacaattaaaggttgcctgaacggacacccgctcaccagtcttcccaaaaatctgcttaattttagctgtctgcttatcgggttcagttgccggaattgaattaaattcctggcatagcttggcggccctggcctttctggcagcaacctcatcatctaagaaatagtaaggttcacccgcatctagtttttctaattcagtcacttcaaatccactccttatagcctaactgatcagtatgtctggcagttgcgacgagattaacattttcttgttgtgccaagtaagcagccaatgagtgaccaaatccggttgaagtgccggttacaaaccatgttttatttgtcattaaattcctctccttgtttgattagattacacattcatgctacaactttaaccaaggtttaagtcaagtcaaaatattggaaagaggtatccatatgtattctattggagatgtggcaaaaatcatgggaatcagcacgtcggcaattcgcttttacgaccgcaaggggctgttgcccttcgtagagagggatgacgccggcagacgaaaattcaaaccaaatgatttgaatttcctggaagtcatcgactgtttaaaacaaagtggcgttccgatcaaagatatcggccatttcatcagtctgtgcatgcagggggacggcaccttgaagcaacgctatgactatttggatcaagaagaagctgccctgcagtcaagcatcgatcggatgaagtcgcagctcgctttcctgcgctataaaaaatggtactacaaaacatccgtggaggctggtaccgaatcaattcacttcgccccgggttccaacgttgttgatccaaagaccaaaagtcaatatcaagaagcattgcagcactgtaccgacttacgcgacttgattgatcttaagcaatctaaagctgataactgaagcaatcaaaaacggtttctcagatgatttgaagacacgtcatctgagaaaccgttatttgttatcggtaaattactgttttaacctggaatcttcctgagcacgcttttgatacattggaatttcatcctcactggcacgaacccagtgatgcggcacaatttcaactaatgaacgttccttgccgtcaaattcctggctggcatcgtaaggaatttgaactcgggcccgttcatactctggatcgggtaccggcacagcggacaagaggctggctgtatagtcatgtagtggatgcgcataaatctcatcagaactggcaatttccagcattctgccatagtgcataacgccgattcgatcggaaatgtacttaaccattgaaaggtcatgggcgataaacaggtaagtcaggttccgttcacgctgcaatttcttcagcaaattaaccacttgagcctgaatggaaacatccaaagcagaaatcggttcgtcggcaatgatgaattgcggttgaacggcgagcgctctggcaatcccgattcgttgtcgctggccaccggaaaattcatgaggataacggctggagtggtctttgttcaaaccaacggtctccagcaaatcttcaacctgcttggaacggtccgcatcatctttggctaaatgattaatatcaattccttcagccacaatatccttaactttcatccggggattaagtgaggcatagggatcttgaaagatcatctgcatgtcccgacggaatgtttgcttttgcttcttggaattgagcttggaaacgtcctggccgtcaaagacaatcttcccggatgtcggttcatataaatggatgattgcccgacccgtggtggttttaccagaaccggactcaccaaccagaccaaaggtttcaccgcgatagacatcaaaagtaatgtcatcaacggcacgaacttcatttggcttaccaatgttgaagtattgttttaggtgttcaacctgtaatattttgttttcttctgaataatcaatcacagttgctcctcctgttcttcaacatgatttcccttgctcttgttaatttcttgatgaacaagttcggcgtagtgcttctgacgttcgatgattggttcaggtggcgtcactttaggtgcccgtttatcgagtaaccaagttgccgcataatgggtatcagataccttgaaaaatggtggctgcttttcggtgtcgattttgagggcgtatttattccgggcagcaaacgcatccccaactggtggatccaataaatcgggtggcgttcctggaattgatggtaactcagtcccactggtatccatggtcggcatcgagttcagcaagccccaagtgtagggatgctttggattatagaagatctcgtcaaccgttccgtattcgacaattttgccggcatacataacggcaactcgatcggccatcccggcaaccacgcccaaatcatgggtaatgaaaataattgacgtgttggtcttggcctgtaactctttcatcaaatccaagatctgagcttgaatggttacatccaaggcagtcgttggctcatcagcaatcagaatctcagggtagttcaccaaggcaatggcaatgacgattcgttgtctcatcccaccagaaaattggtgaggataattattaatccgctgttcggcattttcaattccaaccagcttcatcatttccaaagcttgggcataagctttttcacgtttcatgcccttatgaataatcaaaggttcggcaatctgcttaccgattttcattgttgggtccaatgatgtcattggatcctggaaaatttcggcaatgtctcgaccacgaatctggtccatttgtttgcgggacttctttaacaaatcttggcccttaaacataattgttccgctgtcaatcacagcattgggcgagttcaatcccataatacttcttgtggtaaccgttttgcctgagccggattccccaacaatcgccagggtttcaccctttctcaaatcaaaactcacatctcgaatcgcttgaacagtaccggcataagtattgaagttgattttgagatttcttacctcaagaacatctttttcgttttccatctcaaaacacctactctctactctttggatcaagggcatcacgaagcccatcacccaagatattaaatgcaatcattaagactgaaagaacgatcgctggataccacatctgataaggcaggaactggaagttcttctgaccatcgttaatcaaagtaccaagtgatgcctgaggggcactgataccaattccgatgtatgacaggaaggcttcgaagaagattgcggttggaatggtaaacatcaagttaatgatgatcacactactcaagttgggcaataaatgcttaaaggcaatcttccaagaactttcacccaacgttcgggccgccaggatgaattcctggttcttcagttccagcgtctgcgcccggaccagccgggccatgttaatccaactggtaatcgcaatggacaggataattgcggtcattcctggcttcaagaccaggattaacagaaccatcacaaccaggttaggaattgacagcatgatttcgatgattcgttgcatcaaggtatcaactcggccgccgatccaacctgaagtaatgccgtaaaccaccccaaatgccaagtcgaagaaactggcaatcaaagcaatttcaagggaaattcgagttccatataagattcttgagaacaggtcacgaccaaggtaatccgttcctaaaatatagaaatggttgccggcatgagcctgcgcataagcgttaacccgttggccggattgatcaatggttccgttaaacccgttaatatcaatgccgggaatcttcggcggcaagttcgcgaagttcgggttggtcgcatttggattatgtgtttcaaataaaaatgagaagaaagctaaaataaagagaatgattaaaatcaccaaagcaatcattgctgctttattcttccgcaatcgacgccacgagtcttgtaagaaagttaaagatggcgttgcgattttttcgtcgtccagcttggcacgatcggcaccggcaatcggtgtaaaatcgtcagctgaagtttgttttgcattgtctgccattattattctccctcctacttattaattctgattcgtggatcaattaatccataaacaatatcagtaatcaacagcacaacacaaagcatcgcactatacacaattgtcagtcccatgatggttggataatcgttggtcaaaatcgacttaacgaattgttcaccgattccgggaatcgagaagatattttcaacaaccattgaaccggtcataatgttaacggccaacggtccaataatcgtgacaactggaattaaactgtttcgcagtgcgtggtggtaaataatgccaactttgttgagtcccttggcctttgccagttcaatataatctgaactcaacacgtccaccatttccgtccgcatgaatcgggcggtttcggctaatggcgacgcggccagcgccaaggtcggcaggacggtatacataaacccaccccagtcggcgattgggaataatctcaatttcaagcccaggtagtactgcaatagtacggccaaaacgaatgaaggaattgagatgaacaggattgagatgatggtagctgaagtatcaacccaagtattggctttgatggcaccaacggcaccaacaaccaatcctgcaagaacccccagtaccattccttggccaccaatgatcagagatggtccaagtcgactggaaattaagtatgaaaccggttggttactgaattggaaggaagtcccgaagttaccgtggatgatgccacccaggtagaccaggtattgctgccagacaggtttgtccaacccatactgtttataaatttgatgaatctgtgtcggtgtcaatttggcttggttagtcaatggagtaccaggcattaatttcatcaagaaaaaggtaatcgtactgacgataaacaaggtcagaataatgtagaatattcgttttcccaagtattttgccataagtgttcctctcatttctaattatgttgtaactattttttcataaaccccataataatgtaaaagaggccggatttcaataaccagcctcaaatacatcgaactgttcatttaataattacttaacgtaagccttggaccagtcgtattgtggtgaggtggtgaaggcttgaacacccttaacagatcccttaagcaaagcggcttgaccttgttgataaagtggaactaatccttgttggttcatcaagatcttttcagcttgaaccatgtcgttccaacgagcggtttcgttgttggcatcggttgattctgacttcttgatcaaagcatcgtattgcttgttagaccacttaccatcgttgtatgagttgttagatgtcatcaagtccaagaagttgcttggatctgggtaatcggcaatccatgcagaaagaccaatatcaaattgttgattttccatcttggttaattttgacttaaatggaatgtttgagttggtaatcttcaaaccaggtaatttggttaattgactttgaacaaattcagttgctcgtttggtatcatcatcatctgcacccattaaggtcaggctcaatgacttcttaccaacttgtttgagaccttttgcgaataaggctttggcttctttcaagttgtaatcagtaccggctttgacatatgcctgatcggcaaagtccttgccgttgtgtttagccatacttgctggaacaaagcccttaggggtaatgtcgccaccttgcataactttgttaaccatttgcttcttgtcaattgctaatcccatcgctttacggatattgacgtttcgaagggctgggatcttcttagtgttgaattccatgtaagtagttgaagcttgtgggaagacaacgtaatctttgttgttcttgttgttggctgccaaagttccactcaaagtggtgaagtcaagcttgccgctgttgaaactgttcaatgaagttgaaggtgtcttaacagcttggaagttaacttggtcaagtttgaccttcttagcatcccagtacttagagttcttaacgagcttccaagtatcgttggttcctgaccagcccttcaagataaatggaccgttgtagctgttcttggttgagttggtaccataatcgctaccatatttggcaaccgtctttgaattctgtgggaagaattctggttgggtaaccatgaacttgaagtagctttgtggttgatcaagggtaacgacgaatttgtagtcaccgtcagccttaacacccaacttggaaggtgacatttttcctgcgttaatcttagcagcgttcttgatgttggcaaatatgtaagcatattgtgaagccgtctttggcttaacggttctttgccaagcatagacgaaatcctttgcagtaaccggagtgccatcgttccacttggagtgacgcagattgaatgtccaagtttttccatctttagaaacgttgtaactcttggcaacccctgggtctactttattgtctttggccatgcgaagaagtccttcgttggtaccattggcaacttgtgctgaatacaggtcaatcatctttgaagtatccatggttgaaatggcagatggtgtcatccaactaacttcttgcttcttggttccttgtgaagatttacttccacacccagcaaggatcaggccagtaaccagcgctaccccaccgagtttcgctaatgaattaattttcatgttgcgatacttcccttctcatatatgaaatacttaatttgtaatgaccttattttaaattaaaatttgattaaaagcaaacactatctggtcattcaatcgatttgtccggtgccgaattggtatgggtggttaattgtgaatgtttaattgcttaaccaccagtgtttgaagattctctttcactttcaaaatttttataaatttattggtaaaaatgattctgtgctagagatacgcaccaattaagtcagatatgcgctccaggcgtaaaccgattcacagcaggaatcaatcgcttactcactatattaagagaagtgcaaggtatcgatatacatgtttatatgcataaaaagctcaccgcgaattcggtgagcttttctatgatattaaagattatttaacagtaatcttggaccaatcccactgtggagcagttgggaagaattgaaccccgtgaatctttggcttcatcaaagttgaaattgcgggttgataaagtggtacaatcccttgatcgttcatcaagactttttcagcttgaaccatgtcattccaacgagcactttcgttagcggcgtcagtgctttcggatttcttaacgagagcatcatacttggcgttgctccatttaccattgttgtaactgttcttggaagtcaagatatccaagaagttgcttgggtcaggataatcagcgttccaggcggtaatgaccagatcaaattggccactggcagaacgtgacagacgcgtcttataaggaacgttttggttggtgatcttaacacctggcaatttggtcaactgactttgaacaaattcggttgatcgtttggcaacgtcggtatcgtctgaaagtaacgtcaggttaaccgacttcttgccagtttccttcaaacctttagcccagtatttcttggcttcgttcaagttgtaggccaccgcactcttcacgtatgactgatcagcaaagtccttaccgttacgctgtgacatatcgtcggcaacaaatccctttggtgcctgtgaaccatcggcgagcactttgttggccaattgtttcttgtcgatggcaagtgagaaggctttacggatatttctattcttaaacatcgggaacttcttctcgttcatttccaagtagtagattgaggcttgcttgtacacatgatagttcttatcgttcttgtattgtttaacttgagttccgctcaaagtggtgaaatcaagcttgccgctttggtaaccattcaaggcggtgttaggatctttgatcgcctgcatgtttaaggtatcaagcttaattgccttggcattccagtactttggattcttaacgagtttccaagtatcgttggttccgttccagcccttcaaaacgaaaggtccattgtagccgttcttttgagcatcagttccatatgaagacccatattttttaaccttcgaaatttcttcagggaaatagtaactctgagaaaccatgaatttgaagtaactttgtggcttgatcaaatgaaccaccagtttgtaatcaccctcggctttagcccccagcttggatggtgataatttaccggcgttaattttgtcggcattttcgatgttggtaaagatataagcatactgtgaagccgtcttgggattaacggtccgctgccatgagtacacgaagtccttggcagttaccggtgttccatcattccatttcgagtgacggaggttaaaagtccaggtcttgccatccttggatacggtataattcttggcaactccgggcacaactgcattgcccgttgtcatcttcaacaacccctcattagtcgcattaacattttgactggaaatcaaatcagtcatcttagagacatccatggtgttaatgttggcggctaccatccaattggcagattgtttcttggccccggaatcggaggatttgctgccacacccagctaacacaaccgcggtgagcagagaaacaccggcgatctttaaaagtgatttagtcctcataaatatgaaacttcccttctgtcttatgtattatctgtgaacccattcattttaaattaaaatttaattaaaatcaatatcatttgaatattattataagactgatttgccggtattcttacgaaagtcaatgagatcaatgttatcagagatgaatttcaaataataaaagttgcatatatttttaatcttcgacaccggtcaatgatcagatccgaaaacgaagtgcactttgtccactatgtatttacatttgtgtgttatacttgaacacataatttattaggaggcaccacatggatttacaagttactttaactcctgttgtcacgattggattgaaccgcaacaccagcagcttcgagtattcaatgactgaattgaataacctggcagaagctaacaatatgaaggttgttgaaaccttggttcaaaaattagaccggccggatcctgccacctacttcggtaaaggcaagattgaagagttgacccaagtcgtcatcgatgatggtgttgataccattgtggtcaacgatgaactgtcgcccagccaaatccggaatattgagaaaaatacgcattcccggatcattgaccgaaccggtttgatcctcgaaatctttgctaaccgggctcagtcccgcgaagccaaacttcaagtcgaattagccaaattaaaatatcaactgccgcggctgcataccagtgccagccaacggttggatcaacagaccggtaccagtagtggtgctggtggcgcaaccaaccgtggtgccggtgaatcacaatacgaattgaaccggcggacactggaaaagcggattacccacgtcaatcaagaactcaaagaaaccgccaaggctgatcagaccaagcgcaagcagcgtgaccgcagtgaaatgccaaccgttgccctggtcggttacaccaacgctggtaaatcaacggtcatgaatggcatgatcaacttgtatggcgagaacgaagacaaacaggtcatggttaagaacatgctgtttgccaccttggacacttcagttcgaaaattaaccttaccagaccagaaacgtttcctattaagtgacaccgttgggttcgttagtcaactgccccaccaattagttcaagcattcaagtcaaccttgtcggaagctgccaatgcggacctgctgattcaagttgtcgactactctgatccccatcgtgaactgatgatgaagaccaccgaagataccctgagtgaaattggtgttaacggcgtgccgatgatcgttgccctcaataaagccgacaagatggaggttgccttcccatcccgcgaaggcgacaacctgatcatgtccgccatggatgaaaagtcactgcaagaattaacgacgatgatcaaagaaaagattttcaagaactatcatcgattaacgttattaattccatttagtgacggtgacgttgtttcgtatttgaatgagaacacgaatattgaaaccaccgattaccgcgatgacggaactgttatcacagcagaattaaatgacgtggatgccaagcgatttgaaaaatacctattaactacggaataagttggttgttaacaacagcagattctgatactatttgttgcatatttttttgaggagaagagaggaaaaaccatgaaagaacagaaagaagtaacgctggaccgtgaccttggcctctggtcagcgttagcccttgtgattggaacgattattggtgccggtgtctttgttcgtcagtctgccgtcctagacgatgccggctcaacgtcaatggccctatttgcctggctggcaggggggattttaaccatcaccgccggattgacaattgctgaaattgcatctcaaatgcctgaaaccggtggtctctacgtttatatggaacggatctatggcaagttatggggctttctctccggctggatgcagattattatctacggcccggcaatgatcgcctcgcttggtgcatatctggccattttattatcagatttctttggcttcccaagcaagtacaatgccattctggcaattggcaccatcgtcttagttggtattttaaatttattctcgaaccgttacggtgcgacgtttgctattattacgacgatttgtaaattggttcctgttgccgcattaatcatctttggccttttctttggtaatgaaagtgcctttggtcaaagtttggttcacgtacatcaatctgccggcaactttggtgttgcgatcttggcaactctattcgcgttcgatggctggattttggttgccaacctgggtggtgaaattaagaacccgcgtaagcttttgccacaggcgattacctttggtattttggctgtcttagcgatttacctgctggtctcttacggtgtttatcgttctgttcctgctgaacagattcatcgtttgggcaccagtgccattccatacatcgccaaccaggcctttggtgaagttggcggcaagatcttaagtattgggattatcatctcaattgtcggctgtatgaacggtaagatcatgactttcccacggattatgtatgcgatggctaaacgtggtcaactgccattctcaaagacgctgtcatacttacatccaaagtcacacaccccgattttctcaacggttgccgagttattgatcgtcacagtgatgatcatcttctccaacgctgaccgcttgtcagaattatgtatcttcacggtatactgcttctatgtgatggcctttgtcggcgtcttcctcttgagaaaacgcaatccagaccagcatcgggtattctcaacaccattgttcccaatcaccccaatcctagcaatcggcggctccttgttcgtcatcgtcagtgaaatcatgtctgacttaccaggtgtcttaacttcatttatctttatcgccgttggtattccggtattttattatgaaactaagaaataccgtgagagccaagcagctgcagcaaaagaagagtcattagataacgaaaactaatcacgcatcaaaaaaaagagctggaaatcaatttcgatttccagctctttttttatagttgagataattttatggtaagacaacgaccttgccgaaactatcatgactatccaggtaggcttgagcgtcggcggtatgtttcagatcaaacaccttggttggtgctacgtccacgtgattgttgttaatgatatcaaacaaatcatcaaacacccgttggtttagggcaccggattcaaaactggttaaataacctccattgagttgggaaatgggctcgaagtgagttaagtcccaaataccgccaagttcaccggtaacacaggtaatcccattctcctgaatgaattgcattgagttgggcagcgtcaatgccccaaccaattccaaaattcggtcaaattgtctcccggttgcctgcaattggttatcttgatccaagacaacttcatcaaagccgaccgatttcaattcatcggtcttttccagatgccgggtggagccgaccagcttgatcgatggcaccattgcccgcgctaatttaccggcagcaacccctacaccactggttgcaccacgaatgagcagtgaatctgcttcgtcgaggtgcagtttgagcagtgatccgtaggctgtcccataagtctctggaacggctgccaaatcttgaatcgcaaggtgagtgttaaccgcataaatatggtcatttggcagcaacgtatattccgcatagctgccgtcaaaagcacgacccatgccacccattacagaaaccacaatttgccccttcttcaagcgctttggatcggtggtttcaaccacttcgccgacacactcaatgcccaagattcttggtaacttgacggatggcgaccaaccatttctggtaaaaatttctgaacggttgatcccaaaacctttaactttcaacaacgtccagccgtctttgactttgggcattggcacatcttcataggataaggcggaaggtccacccgggtgacgtaatacaattgctttcattctaattgccccctaaacactctgtcgttcgacaattctaattggcgtatacattgaataaaattctttaaatgagtcactcaccagcatatccattccgttagcccccatctcaaagaaggattgggtaacactggataatttaggccgaacgatgtcacacaattgggtgccgtcaatcgtcaagattgccagccggtctggcaccttcatcccatagttggtggcttgattcaaaatcccaatgcctgccagatcacttgaagcaatcacggcagtcaactcggtttgcggaccataatgttccatggcgttcacaccatcttcataggtaaaatgccccccgcaaatccaatcctcatcaaatgacaaatggttgtcacgcatggcatcccggtagccttcatagcgcaaatggccgacaaatgaatccaagtcggtagcggcaagcccgattttttgatggcctttgccaatgagatacttggttgcctgataaccaatatcaaagtcattcgaagaaataaacggaaaggcactattcttcaacgtcatcgaaataaaaataaatgggatattcgcattttccagcaactcatcgtttgaagggtccaaatcaatcgccactagtaaaatgcccatcaccgatcgttcaatgacggttcggatcgcttttgcctggacctccgcatcgccttcaccggcgaaaataatcatcacgctcaggttgtgaacccgcgcctgttcctggatcccctttaagatctgatcagagaaattggtttgagtagaactgaccagaaccgcaatcaccttgctgcgttgcgtgaccagctcaactgcactggtgttgcgccgataacccagttgtttaactgctgcccgtactttttgggctgttttttctgaatagaaggctttttgattggacaaaactcgggagaccgtcgccggagaaaccccggcagcccgggcaacatctttaattgtcgcagccatgtgttcacctcttcatcagtatggtcggataaatcttcgaaactaattataccacaaggccgattggccatttctgcctcaaacgtttgtgttaggataggtttacgtatttgaataagcacctaggctcaaaggcaaccatttccggttgtctttttttgtttccaataagcttggcgttataattaagaaaattgttctgtaaaggagggctgcccatgaccgcttatgttttgtaccaactagaatggattttaaggttatttgtggccgcaatttgtggtggcctcgtcggttatgagcggaaggtccggttaaagaccgctgggattcgaacccatatgttagtggcggtcggatctgcgctgttcatgatcatttcgaaatatggtttctttgatgtcatcaaccacgctgatgtcagtttggacccttctcggatcgcctcacaggttgttactggaattggttttattggcgccggggcaatcattacccggaatcacaagattgacggtttaactaccgcggctggtctatgggccaccgctgcaattgggctggcaatcggggccgacatgtacgtcatcggcattgctggaacgttgtgcattttggtcacccagacaatcgtccggcagatccgggcatttaaacgctatcccaatcgctctctacttcgcctgcaagtcacatttaacggcgaactggcatcgatggatgagctgccggaccgcctgcgagcgattggcagtgccgatattcgaatgagaatcgttgcctacaaaccggattcgttctcactggaagtccgggtaaaattgcagcacaaaatggatccggacgagtttatccgccaaatgagtgatttggtcgatgtacggaagattgaagtgctggattgaaagttgcttatggatacgaaaagagtcatcaacgattttggttgatgactcttctttgtttgcatttataatcccagggaaaatcccaccaggaatgccaagattagaagcaatatgatctgtcccatgaagcgggcaaatttgattagttccattggatgaccttcttttggtggggttctttgagtattttttctattatttggatgaaacgtgctccgacgggcctgaagctaacttctaagccagccctcgtcgcactctggttaaaatgtgttccttggagcagcaacctgcgtgtaagccaactctggttgctaagcgctccaatccacactctaccgttctgctccctgcacaacttcctccacttcacccgacttcttggctgttcccagtctgtggtcgaggtactgtgacagaagtgacagtgagtaacatacgatgaagtacatgacggctaacgccaagaacattggaatcgtataattggtgttttgaccgtaaatgatttgcgcatggttcatcaaatccggcagcacaatgatagttgccaatgacgtatcctttaccaaggaaatgaattgactcacaatcgccggaatcatgttcttgatggcttgcggcagaataatatatctcagtgcctgccaataagacattccagtcgatctggccccttccatttgtccgactggaattgagacaattccggcacggacaatttcagcaaccatcgccgattcaaagaccgccatggcgatcaccgacgcccaaattggatccggcttgaagccgatgtttggtaagccaaaataggtaaagaagataatcaggattagcggtaagttacggataatatcaatcacgaaaccgacaatcgctgataaatatttaatttcaacatatctgataattcccaaaattaccccaaatatgtaactcaggataatcgaacaaactgaaaccaggatcgtgacccaagccccttcaagaaggaacctgatgttaatccatgaataagcacctaagactgttaacatatctcgattcctcctttatgccaatttcttttcaaggtaacgcatatagtaactcaaaggcaaagtcaaaatcagatacagaacaccaacacacagatatgtgctcatactttgcagtgagtcagacgcaatgacgttgccttgatacatcaaatcaaatccggcaacaaaggctaggaccgaagagttcttaaccaagttgatgaattggttgcccagtggtggaatgacatatcgaaaggcttgcggcaaaacgatataacgcattgcctgccagaatgacaatccattggcacgagcgccttccatttgaccaggatcaacagactggattcctgatcgaaccgtttcagcaataaacgctgacgagtaaaggatcaggccaatcgtaccagatgcgaatccactaatttcaacaatgtacattggaataaccacgtagaagaacatcgtgataaccagtaatggaatgttccggaaaacttcgatataaactctggcaatcactctaaagaatttgttgggtacaacttccaggatggcaaaacctgagccgatgattaatgcaaagaccaacgcaataatcgagcacaaaagggtttgtcccagtccataaaggagctcaccaccataattttgaaaaatacttatcatcgttctgcccccttaaagtcaaatccgtgaactttgtggaaccacttgtaaaggagcttgttgtattgaccggaattttcaaccttggtcagggcgttgttcatcgcgtctctcatctggccttggcctttgtcaacggcaattccataaggttccttggtgaaggtgccaccaacaaccgaataacctgggttttcgatggacatcccataaagaatcccgttatcagtggttaatgcatccccctgaccggatttcaaggctgtcaatgcctgagaataatcagacagttgaagcactctggctttcggcgcaaacttcttaatattttgaacggagttggaaccaaccaccccaaggacaatggcgcccttatgattcagatctttcacattcttgatcggactaccattcttaacgaggatggcttgcccggcatcaaagtatgagcgtgaaaagtcaacttgcttagctcgctccggggtaatggtcatggttgccataatggcatcaatgttgccgtttctcagtaatggcatccgggtttgactggttacttgaatgaatcgtgccttgccgtctttgccaagaatctgcttggtcatcgctttggccaaatcaatttcaaatcctttaatctgattgtcccgaacatccattaaaccaaacagcttggtgtcggctttaacgccccatgtgatcgtctttgtctgcttgtcatccttcagcacatttttctgtgatgctgcgctcgaacaggcactcaaagaaacgaccattaagagcagggttaacaataacccaattcttgatatgatcttcttcatgatgcgacctcccaataatgaaatttttaatgcgtaataattttcccaagaaattgtcgtgcacgttcattggagggttcaccatcaaagaatttgtcgcttgtgtcatcttccaaaatctgaccgtcatccataaagataacccggttggcaacttcacgggcaaatcccatttcgtgagtcacaaccaacatggtcatatctgaatcttgcgcaatatctttcataacgttcaaaacatcatcaatcatttctggatccaacgcactggttggttcatcaaacaacagacactttggcctcattgccagggaacgggcgattgcgatacgttgctgttgaccacctgataattgggctggcaatttgttggcttggctttgaagaccaacttggtcgagcaactgcattgccaactctttgttttctttttcaggacgcttcaacacaattcgtggtgctaacatgatattttcaagaaccgtcttgttggcatacaaattaaaatgctggaacaccatcccaacgttctttcggatccggttaacatcggtcttcttgttggccaagtcctgcccattgacgatcaacttaccttcttgaatcggttcaaggccattaaccgttcggatcagtgtcgacttaccagaacctgaaggaccaattaaaacaacggtttcgcctgcttcaattttcaaattgatgtcctttaaagcatggaaatcgccgtaatacttttgtacgtcttgaaattcgatcattgccatgtcattttcctccaatgctttcaggctatttattaaaattgcctaagaatgatactacatccataatatgttaaaaattttgataggtcaaaaaaatgttacaaaaattttattttcatgtcacattttctatcaacggggttaatccgatgataaagccattcaaactcgaccattattttggatgtataaatttgggtaattatctaattataattcaccatcagcgaaaatggaaaccccatttgaataaaatttaattggaagctcattttgtggctaaaaaatgagagcttaaaaataacgtgcaatccaaacccgggctgggttgaattgcacgttattaagatgagaaaatattaattttcagaaatgtaatcgagaatttgaaacatgacgtttttattttctgctggaacctgacgagccaaaatttcatcagctgactgattcaacaccgagccttgaatgtatgcagcgtcattgacgaccatctcgcgaacattatcttctttgggctcaaagtgaaactgcaacccgacaacctggtgattcaacacaaatccctggttagccaagtggtcgcttgagaacaataaatctgcatcatcgggaagctcaaacatatcctcgtgccaatgcagcgccgtcaattgctcaggtagtccaggaatcacgtcggactttcgatacaccggggcccaaccaacttcttttgccgggcctttggaaacggcgtagcccaagactttggcaatctgctgagccccaaaacaggcaccaaagattggtgtttgagcatccaacagttgttgaatcaattcccgttcttgttgaatccacggcaaatcgtcattaggactcattggtccaccgaggatgatcaacatatcagtctgagctgcagttggcagtaaaccaaattggtccgggtggtaaatgtacatctgatgccccttggcatgcgcccagtcctgaatggatccgggtccctcatcggcgacgtgttgtaaaacgttaattctcataatgaagccctttcgtttataacttcttgtaagcaaccattgcccgcagcttatagtcctgtggcgcttcaatcaccccagcccggccgatctgcttgtacggtccaccaactaaggtcactgatgccaagtataacttgacctgactcaaatcaagcgatcgaatcgactgcaggccaattcgcttaatttcaccgaccggatagatctctgcttggttcaaaccgcaatagaccatcaatgacgaaccttgtttttgcatttcaaaataaggaagcaatacgcctttgccaatggcataaatcggcttactattaaccttcagcagttcatagatcttccggtcactcatgccgttatagtcggccctaaacagctgttggcgttccatttgagcaactagtcgatcaatattagcctgctgcattgggctgacctcaattttagccggtaacaggtgctggtcgtcgaacaagccgttggccggcacgtttctttcatcagcgatgacggtggtgcccattttggattgcacctgagtttctcgtgggtgctcttgaatgtgcagcagcttggcaattttcggtgaaatatcgaaccacggctgcttcttagtaaagtaataaaagaagttgcaaattgtaaagtacagcaaaatgattgcgactaataaaatcgggacacccttgctaaacatctgattctgcaagaaacgaaaactgatgtaaaacaggtagacgtcaccaaagaagcctaacactgtgtaaatccggctcttaagggtcacattaatattgaagtaccccaggtagtggttaaccatgtccaaaaagctaaacattagttagttccctcccctgtattgccagtcgtcacatcagcgttggcattcgtattattgttattttgagtgttggttccgcccgttgttccagtcgtctgattactgctgtcactactggtctgggtattttgatccgagttattgttgttagtcgtattcccaccggtcgtcgtccctttattagtggttgtacccttattggtggtcgttcctttattggtcgtcgtcccggttgtcgtattcttgttgttattggttgtatcatcgttggtttggtcatctgaagagctggcgtttttttcgctctcggctttttcagacgaagccttggccgcagacgattcttccgcggccttcttcttttcggaggcttccttagccttctcagctttttctttcgcatccgaatcgttggtctttttcttattcccatagatggaatccgaaatctttttttgattggtcgtttgagtggtcctaggggttccttcattggtggacgtcacattattgaccacaacgttagtggcgccgagtgccaaagaaattgagagaatggcaaatggcgtaattaatggtggaattctattatccattcaaaaaacttccttactaaatttttgtaacctccattatcgcataagaatatgaacgaaacctaaacaattcgttaattattcattaagttgacgcactgagggcacaagccataaatctgaaacaaatgaccagtcacttcacagccagtcagctgggaggtgatttcaggactcaatgggcaatccttgagttcgatcactttaccgcagttactacagataaagtggtggtgatgctcatgttgaaaatcacattggaatttaaccgatgcccgatccccctgcacctgccgctcaacaatcccgagattggcaaactcggaaatgttgcggtaaatcgtgttatgactcatgttgggaaaagttttgcgcatgaaatcatcaatgctggtgacttcaacaaacttatgcgtcgccgtgccgactaaaaattcaatcatcgcccggcgttgcttggttatcttgaaattattctcttttaaaactttggtcgcttgttcaattgctgcaggcatactgttcacctctaataagtaattattactgtttattgcatcctaccataatctactttcagcaacaactatcccgctgtttcttaacgataattctcaacgattttgtcaatttgttgacgcgtctgctgccaatcctggttaaccacttgataagccttgccctgcagttcatgaggcatttcgagatcccggtggtattccttactgctgacccgtttagcaaccatctcagcattgtcaccacgtccctgcattcggcgtttgagttcttcggtatcgccgacctgcagaaaaatgatgatcgctttttcgcccagtttctgcttatatgtaatggctccggcagtatccaggacaatcgtcgcaaacggtgatttctcccaggcattctctaagccttcgtaagatgaaccataatagtggccggcatagtggacggactccaaaaagtgattgtcaaagaacgattggtcgtcctcaaaataatagtccaccccgtcacgttcattctcccgcggcggccgggtggtgtgggtgatcacccgggccatttgatattggtcatgtaaataatcacgaacggttgtcttgccactgccagcggctccggtgatcacaaatactcgattcttcatcaggcttcctcgatgttttctttattgcggatataggtgtcggcgtgcttaagcagctgtcggagattatcataggttaatttttcgtaggcatcttcatagtcaaaccagccaaatgagttgatctcttcatcctgctttcgaaccttgacttcaggagcgacccggctgacaaagaaagtcacgtccttgtggtggccgttgttcatatcgtactcaaccttttctttaaagttggcgtcgatctgcgtctttaagctggtttcctcgcggatttcacggattgctgtttggatgagattttcattcttctcgacgtgtcctttgggtaatccccaaaaatcagaggtggcactctgcaataacaggtaccagatcttgccgtctctaatttcataaaccactgcaccactcgcatattcagtaaccatcattaatctccttttaaactttcatcgttttcttcaataacattggtgccacaatcgtcgacaatacaatgacaataataatttcagagtacaggttcttggccatcaaattggcggacaacccgatttgggcgataatcagcgccatttcaccccgtgataccatcccggaaccaacaataaacgcgctgctccaattcattttggtgatccaagcacccagggcaccgccaaacagcttggtagcgatcgctaaaatcgtcatgatgacaatgaagcccaggttcttgatgacattgttgaactccatgtccaggccaatgctgacaaagaagatcggaatgaaaaaggtgtatccgaccgagctgacactgctggagatttcatcttgaaacttcgtctgtgaaacggccactccagcgaagaaggcgccaaccaccgaactcaagcccaaagcgtcggcggaccaggccattgtcaaacagatcaccagcgaggtaatcgctaccgagccgtggaccggcaatcgttctgccactcgcagtaccaccgggaccacccatttaaccaggacgatcacacctaaaaagtacatcaattgatacagtgtggcaaccagtaaattcgacgatccactgccgctaactccaaaggagctgacgaagatactcagcaaaatcacggcaatgatgtcatcaaccactgctgctcccagaattgtcgcgccttccttggtgttcagtttcttgaactctcggagaacttcaacactaattgagaccgaagttgccgcgaagataacgccccaaaaaattgaacgctcaaagccctgccccatgatttggccgtagccgtaaaagacaatcatgggaaacagtacgccgattgcagcaacactaattgccggtttgaaatacttcttgagcaaatccagatcgctttcgatcccggcaatgaacatcaaaataatcacgccgatttctgccccggcgtgcatcagttccgtattgtgcaggacacctaaaatacccgggcctaaaataactccggcaatcaactggccgatcacggccggcatccctaatcgttgactaatcgctgccgccaataatgttgcaattaaaatgagtgcaatttgacccacaaacgccatctaataaccctttcttttcttaaccattagttacgtactattgatattagtttaccataccaactgcccgcgttcatgggctgagaccggtaattttaagaacttaatttcacaatcaagatactttcaatttctggtaatattccgacataatgaaatcgattacaaggaaggaatatttacacttgggggtgaataatcatggagcgttccaagagactactcaactttttgttaatgatcacgacgaccgccatcctgatgtttgtggggatggtcttaaataaccaaacgccgatggtcacggccgccaatgcagccactactcaagacgaacagaccatcgacaaaataatgccgaatgagaaactgcgggaattggttttaatcaatatgaaagatcaaaagatcattcaagatcccaactttaccttgaatgacttcacgccgaccacatttaaggaagatttggcaaaactaactcagctgggctgggaaattgggaccaacgaacaagtggaccgccaagaaccggtcaatggcggcaacggttcggtcggcccagcaaataagggtaattattcactggaaggcttggaatattgtacgaacctcaccaagcttgaattgaacgcagacttaaatagaggaagtaaatttcatcatgatgacattattgatgtctcaccacttgaaggtctggaaaaactcgaatatatcaacttgtcaggtaatcgaattcaagacatttcaccaattgcgggtctgaagaatgtcaagactttatatctcaataacaactgcatcaataatctaaacacattggacgctgaacaatataccgagggatttaactacctggagcaaatcgtcattaaaccactacaagtgctccactccaacacctacacttggaaagcaccgtttgtggacgccttaccaaaaaacgttaaaaccgaggataacaaaccattccagccttaccagcaaaaatttctccgtccgggaacccttgcttatggcaacccaaccgataccaagtactctcaaattgacgtcttccgcaacggcacccgtgggactggtgtggcccagggaaccacaaccattaatggtgatgatttcacctacacaaatttggcaccgcaaatcatcccaacagatcccactaacccatgggccagctactatccaaacgcaaccgtcgttaacaatacctacacttactacatgattgcgcaatataacgtctacccaggagaaccgctctacgcagcactgagctactttatgccatacgtcattcaaccagaagaagcccagccggtcacagttgagtacgtcgacactaacggcaactcaattcatgcctcagccacgatcaaaggggaaatcgatcaagccttcgatctttcgacagccgattacaaattaaatatcccaggttacaccttctccaaatacgacccggcacaaaccggtaaaattactggagaaaagcaaacctttaagctcatttacactaagaattcaacaccggtcaacccgacgccaccgaccaccccaacaccaaatccaccaaccaatccggaaaccccaactttcccagtccacccaaccccaccaagcggcacgcagttacccaactatgccaaaaccactggtgaagtcgtctactcactgaagaagatttacctatacaagaatccaaccttcaaaaaagctgagcgactggttggttatactcaaaagccacgggtcttccgaccaatgtttgtggtcaccggctacagctattccaacgcaggccgcttacgtttcaaagtcgtcgatgtcaaccatgatagtccaactgcgggaatgaccggctacatcaccaccaagtccagcttcgtttctccggtttactaccaggcagtcccaaagttcatcaccgtcatcagcccaaatggagtcatcgaatacaacgaaaaggacctcaccaagccagtccagacgttcaagcagggaagaatcctaaaggtcgagtcaatcaccacccacaacttgaccacccgttacatgctgggcaatggtaatttcatcactgccaaccgtaagctggttatgaacggtaaacaaaagcagccaaccagagtggtcgccaaaaaaacaatcaaccgctataccactgccaatttcaccaagaaaaacggtcactacaagaaaggcgccaagattaaagtcaacttctacacctatagccatgatgcgtcgaacaccaagtccggtgccaagcgattcgctgtcaagggtggctatattaccgccaattcgaagtttgtgaaagtctattataaataatcacccaaaagaggcgagacatcattctttgtcagttatgtcatcgtctcttttgagttccactgtcatatagattaaacgtgggacaatcggctgatcccggccatttaagcaaataatccagttattccaaaaccaggaataactggattatttacttaaattctgggatcaaagcgcctcgcgccccactcttcatttaatctaaataccccttggtagctgcaataatctcctgcagccctttcttggcatccgagaacatcatactagtttgatcttcactaaacagtgggttttggacacccgcataaccggtactcatggaacgcttaatgacaacgacggactttgatttatcaacatccaaaattggcatccccgaaatggcgttacccttttcacgggccaatggattggtaacatcgttagcgccaataaccagcgaaacgtcagtattttcaaacatcgagttggcttcatccaactgtttcatttgatcgtaaggaacgttgacatcggcgagcaaaacgttcatatggccaggcatccggccggcaactgggtgaatcgcatagttgacgttaattccggcgtccgtcagcaatttcgccaattcagcgacttcatgctgagcctgagcggcagccaaaccataaccgggaacgatcatgacattgtgcgcataggccagctgcatgccgacatcatcgggtgtggtcttcttaatgttggttggcacttcggcacccgcaccggtactgccgttggaatcaccactaccgaagccgccagcaataatgttggcaactgatcggttcattgcttcggccatttgcagggtcaaaattgttccggcagcaccaaccagcgcaccggcgataatcaagacctgattgtcaatgacaaatccggcaaaggcaaccgccaaaccggtaaaggcgttcaaaagtgaaacgaccaccggcatgtcagccccaccaattggcaaggtcatcaataggccaaaaatcaaactggctaacaatgccagtaccataggccagtaagcggaaggaaaaccaatcatccaaacaccggcaacgataatcgctaacactgccaagccgttaatcaatttatcgccgggaaacgaaatcggtttgccggggacgtgtccggacaatttaccagtcgcaatcagcgagcctgagaaggtaatcccaccaataataatgtcaagcagcactggaatggaaaaggccaggctcaaagaggtaccgacagcttcgtgggtataatcgaaaatcccaattgtggcagcggcaccgccaccaacggcgttaaacagtgaaactaattgagggacatcggtcattggcactttgcgtgcgcggataaccccatacaaaattccgattaacagaccggcaaacaataccgtccagccgatcaacgtaatctgacccttggcgataatttcaactaaaatcatgacaactgccatggccatcccaagtccggaaagtaaattaccattccgggctgtctttggggagcgcatcatgtgaacaccaattacgtagcagaccgctgacagcaagtaaattagggaagcaatcgttttaaggagtgacattatttgtcgcctcccttgtcagctgaattcggctgttttttcggccggttaaacattcccagcatccggtcagtcacggtgtaaccaccggcgacgttgacagctgcaaagaatgcggccagaaatgccaacaggtagaaataccagctgctggcttctgcagcaatcacaaaggcaccgacaacgacgacgccatgaatcgcattggccccagacatcattggcgtctgcagggtcgagggaattttactcataacttcaaacccaacgagcaggctcaaaacaaaaatggctaaattcgtatataattcttgactcataatggctaatcccccttctcagctgacttgtcgtcagaatcggcaggggcagcatcgtcttcagccggttttgaaattggcaggttcagcgcttttctgactcgttcagaaataatttcgccatgatcggtcgcaaccaactggctcattacatcatcttttaaatcgatggtaatttgagcatccttatcagcaacatcattaatcactgcctgaacgttcttggagaacatttcagaagccgacgttgccatttcactggctaaattcccggccccaatcagttgaacaccggaatcggtgatcactgtttgatcgggctttgatccagcgacattaccacccaaatcactggcagccaaatcaacgaagacgctacctggtttagcattatcaacggcggcttgaggaaccagcagcggcggttttcttccaggaacttgcgcggtggtgatgacaatatcattttgtttgataaacccaattaattcgtcttgctgctgcttttgctcatcagcagacaattgacgggcataaccgccttcaccgacggcactgactgaactggtgagaaattcggcaccgagtgattcaacttcgcctcgagacgctggacgaacatcataaccggaaacaattgctcccagccgtttggcagttccaatggcttgcaggccggcaactccggtccctaagaccaacaccttggcaggcttggcagtccccgcagcagtgatcatcattgggaaataacgggcgaatttgtcagcagccaccaaagcagctttgtaaccggcaattgaggcttgtgaacttaagacatccatgctttgggcacgggaaatggtccgcggcagcagttcaaacgacagcgccgtgaccttctgtttagcaagtttttgcaccgagtccaaatcggtcaaggccttcaacaagccaattaaaatctgtccctcatgcaacttgcccaaagtctctgaatcaggtaaatcaaccgtcgcgatcacattggcctgactaactgcatcatctcggctaacgacttttgcgccggcatcttgataggcttggtcggaaaaataagcattctgaccagcgccctgttcgatcataacttcaaacttgctgtgaactaatttcgcagccacatccggtgtgattgccacacggttttcatcgccagattcctttaaagcagcaataatcgtagacattaaagcgacccccttcacaatcattttgcaaacgctttatacggttcaaggctagtcctcttcatcgagaattgcaatggtttgtgattaactttacaagcatagaaaaacgaaccaaaaagttattttcggttcgtccttgtttcaaagtatcacttgtgaccgttagttagtgattaaccatgccggtattaggaacttcagaattcaaagaatcgacaaccgaattgtcatcaatgacatccagatgttcattctgcttgcgattagtttcacgtcgttccaactctttgacaatttcggcatgtttctcgtcagtcaagtcgtagccaaagtaaaagacaatgcaggaaatcgcactggcaatcgctggcactaagaaatatacggcactaatgccggagattgtgctggcagattgaggttgattggcaacatatccggtcattgtcaaagcaagaccaggaataaagccggcgaccccttgggcaattttccgcacaaaactgtagccggaataaataattccttctgagcgaatcccggtttgcaactgaccgtattcaatcacgtcattcacaaacgcaaaggcgacggtcccactaaagcccaggaacatgtatgaaatcgtgttgacgatcagataaggaacaacgtgtgagccggtgataaaaaagttcaccagttcggctgcaatgaatcccagtgttgcgtatattgcaacgttcttcttaccaattttcttaaccaacggcgtggcaaagatcaccgctggaataatcgataaagcactcaatagactcacaatactaacgattccgacctgtcccaaaacgtactggaagtagtatagctgaatacccattttaaggaacatcgagccaacactaagaatcgtgaaaatggatagaataatgaacggacggttggttaacagtcccttgattgacttgagaccatcccccttttggcggggcttatggtcaatgatgcgttctttggttccggagtaacagagaatctgtgaaacaacgccggcggcagcaaaaatcgcgaccgtggcaatgtaaccaattttaggcgtcgcaaagatcgctaccagtggaattaccactgctccggtaagcaaggcggccatttgcccagttaagttgcgcgcggcagccaaagaagtccgatcaccggaatccatagtcatagctgctgccagcgaaccataaggaatatttacaacggagtaacaaaatcccatgatgttatatgaaacgaaggcatagatgatccgcccggtctcaccaaaattaggcgtgacaaaacaggcaactgttgcaattcccaggaataatgagccatagagaatgtatgggcgaaactttccgcgtttggaaatatgctgacgagaatccacgaaggcaccaacactggtatctacaaaggcatcgaagaatttggcgatcaggaaaatcaaccctccccaataggctgggatctgtaaaacatcggtatagaattttagtaagaacagctgagcaaattgaaacatcaagccgttgcccaaatcccccaatccataggctactttttcacgcattttgagtttttctgttttcaaggtaaacccctccttaatcatgtgctggttcttagtttgttaagcgctttcatttgaagcaataaaaaaccggcgcacgcggaatcacgtgttccggttcgaaaattaacgatattattttttataaccaaagttaggaatcttagtccaacgggctttcaagtaacggacaaccatcttcggttcccgtgatctggtgaaaattcctttcttattaccctgaacccgttgaatgccaaatttggtctggaagtcagcgaagttccacaattgttcaccgacaaagtgtggaaactcatcgaagaccttgctggccattcgatagtagtcttcctggaattcttcggagaatggctcgtcataattgctgtgcagccccggaatggtgtcagcaccgtattcagtatacataatgggtttatccgggaatttgtcagaatattcctgcagctcatcgcgggttgcttgttcagccatcttcaaatcaccattaccaacataccagccataatagcgattcaaggcaatcacatcaaccaatccgatacagttatccgtcttcggggtggccatcatgatgctggtgtaggtgcagggccgcttttgggggtccagttgacgggcttcatcaaatagcggcttgaagtattcatatgacccttttgaaaaggttgccgcttcgttagcaatcgaccacattgcgacacaggcatggttcttgtcacgatcgatgatttctttgattacctgcttgtgggcgtcggcggtctttaatttggtccaagtatcgtcttggtagtcgtcgctctcaagcattgacacatcaaacccaaaggttaccatcaatccgacagccggcgtttcatcgatcaccacaattccttcgcgatcacataaccgcatcatttcctcggagtatggatagtgggaagttctaaacgaattagcgcccatatccttcatcaaattaatatccaagacattgaccggttggttgattccccgaccatgaacgtatgaatcttcatgcttgccaaagcctttaaaataaaatggttcgccgttaattaagaactgggcgtttttaacttcaatcttgcgaacaccaaagtcttctgaataggtatcgatcacttcaccatttcggctgaccgtcacttttgcggtatagagataggcgttcaacggctgccagagatgaacgtggtcaatatgcaacgtggtatcggcagaagtgccgctgactaccggctggccgtcttggtccaaaatggtcactttaactccatcaatctccccatgggtagcaactttgacctgaacatcagcactggattcagccaaatggacgtctggaacgactgtgatatcgctgatatagtcagctggcgtcgagtagattttaactggtcgttgaagaccggcatagttaaagaaatcaaagttttcgtcaacgtggcggagcttgtggccatcttggtcagtgctttccgaatagttgccaaccggcagagtcgtgtaatcaagaatattgctgagtttaacggttaagcggttgtcgctgtcttttagataatcgttaatttctacttcaaatggtgtaaagccacccttatgatgggcaatttcctggccgttgaggtaaacccaagcttcatgagtggcggagccaaatcgcaaaactaaccgctggctgcgcaatggtttggcaatatcaaaattagtttcgtaccacacaaagccgttgtgctcacgaatcttctttgacgcggtttgatcattgaaggaagccggaaccgaaatgacatcttcagttggcaacggccgtttgggatcgattggcgtgatctcctcatcgatcataaatttccagagtcctgataagtccagaaccgttctgctgggtgttgtgagtgggtataacatagttaaaatcctccgttcgttagtcagtatttggatcactgcttttcaatgtctttaatataggctaaactgggatcgaatacttatccaatttttacttaaatcgcattttattgacttttatgtaaccgctaccagaaaggagcttgacgatgaccgtgtatgacaaccaatcaactgctgaactgattcattccctgacccaaattgatattgccatcattcaaaaagacggcacccccgtggtgcaaattcaagagaacgtgttacccgccttccaccggctcaacgagtttgatccgatctttcaacaaattgagcaattccacgctaatgagtacctgacttacacggattccgcccagctgagctacgtggcggcccgccttgaccaacctgacgaccaagttgtcgtcttaggaccgttcctgaccaccactctgaccattgacggaatcaatgacatcgtagcgatgaattcctataccatcagcgaacatcggcaactcacccagttgtaccaaagtttgccggtgctggcagaagataaaatcaacgacttggccactttgatgaccaacttattttcccgacagctagccaccgcccacgaaaaagccaaagtaacccatggccctcagccaattgaaagatcgttgatgacggttaacagcgatcatcgggcgcaaatcgaagccaactacgcaaacgaagccaaaatcaccaatgcgattgcttcaggcgatcaagttgccgtccaccgtctcaatacaaccatgaccaagatatttgattccttctcgaatcgaattccaggcaagccattacgctcctcaaaaaatatctgctttgttttcaatactatttgtcgaattgccgcgcacaaaggcggcgtccacccagtttatctcaacgacatttctgaaaagtacgccttgttaatcgagcgccaaaacacgcttcaaggtttacacatcttagtccactcaatgacgcgggaatattgccaactggttcttaccctctcaacttccggctattccccaatgattcaacgagcggctgactatatcctgctgaacttggggcacccgatcacgctcaatcaaattgcccaatctatcggcaccaatccgtcctacctttcaagaaaattcaagcaggaggtcggcatgaccatcaccgattacgtcaaccaccgccggatcgttttggcaaaacaatatttgagcagaccaacgccctcgattaccgacatcgccttgatgaccggattcaacgatttaaattatttcatcagagtttttaagaagctgacaggccagacaccactgcaatttcggcaaaagccgaccggttcagggattcaaaagtaaggtataatggcgttaacaatcatttccaggaggtatttcatgaaaattaatcagtttgcatatgttcccactgatcatcacactattgtcaaagagttggcggatgtccatttcttaaccgcccaaaccaaaaagatggcagatccggtcatgctttatcgccaattcctgctgaaattcttcattgaaaagcagagcttggccactcggattcaaaaggttgctaatttgatggcaacccccactctaaatgcctatgagttcacgacaactcaagctgccgtcagcaagttagccttttataacgttggcttgcagctgttgggatttgaagttggtctggacttcgagttgaacgacccgttttccgccatgaaaaaatatcgactgccaatggcggttgtcgacgatacgctcgaccgcaatcaggtcattgacgcctggtacaaactgcttaatacgcgaaccaaatttggccagaccttgattgattatttggcgggtcaaggctactatcaccaattcttcggaaccgatgaactgaaacagccgctcatctttaacggtaaatcccaggccgtctttgataccactaagctcatccgcgacgtggtttacgttgaagcgcccttggacaatgaccatgatggaaaacgagacctcttgaaaactgaaatcattcgtccgggagaaactgaaaacggcttgaaggtaccggttattttcactgccagcccttacgaccaagggactaacgaccaccaagccgatcaaatgacccacgacgttaatcaggaaaaattaacccgcaagcaacccaaccatctgagttatgaggacgttaagttcgattacgacaatcatgatttgccggagccacgaaccatcaaggataccaacaaagtcgctgaagaatcatttgttaaaacctggacttattcactgaatgattacttcctggcgcgcggctttgcggtggtctattcatccggtgtcggcactaaagattctgacggcgtccgaacaaccggaacgcctgacgaaaccatcagtgccacttcggtcatcgagtggctgcatggcgatcggaccgcatttaccaatcggtccgatcaaattgccattccggcttggtggtccaatggtaacgtcgggatgaccgggcgctcgtatcttggcaccctctcaacggcggccgcaatgactggcgttgacggactcaagaccgctgtggttgaagccggcatctctaactattacgattattatcgagagaacggcttggtcgtcgctcccggcggcttccaaggtgaagatactgacgtcttgggtgaactcacctttagtcgtgagcagtcggctgccgattacctcaaaataaaggacacttggttggcccagttgaaaaaactgactgctggccaagaccgggtaactggcagttacaacagtttttgggataaccgaaatcttctgaagaatgtcaatatcaaggctgacatgctgctagtgcacggtttgaacgattggaatgttaaattgtctcacgtttacaacctcagaaaaacgttaaagaatgaaaagattacccaaaaattagtccttcatcaaggacaacatgaatacctcaacaacttccgctcagtcgatttcacggatatcgtcaatctctggctaactaacaaattgttggcggtcgataatcaagctaaccagattgtgccggatgttttggtacaggataacgctgaaccggaaacgtggaacacctacaaagactggggcggcaacgttaaagaaattccccttgacgataagcgctggacagatctgaacgagaaccattcatttagcgatcaattgccagacgatttatttaaggactacatcgaaaacaccaagaagtggcagaaggccctatttaccaagaatcattccaagcttgataaacacagtattaaactcgtgtccgagccactggaccaagatatcaccgtggatggaagagcgacgattaccttgcgggctgccagcagtgcggatttaggtttattgagtgcggcgctggttgattatggggtcgaaaaacggttgaccgctgtcccccaaattttgtctgcccagcagattattaccggttaccaatggcggaaagacgatttgaaagaatttttgcctgagaaaaaagcatcggcttacaagaagttcaccgatgcccatatgaatatgcaaaatcgcaccaacaattatcaatcggacgacctgaagcccggccaatactacaacttcaccatggcatttcagccaacattttggcgcttgttgaaagggcatcaacttggattgatcatttacgccactgatatggactacaccatccgcagtaatcaggatatttcctacacagttgatctgagcgcttcaaagattgaattaccattgttgactgccgatgataaccagggataaatgtgatatgatttttataaataacaataaggataggtgattttatgaagacaggaacaaaaatcattactttggataacggctatcacttatggaccaatacccaaggcacaggcaacattcatttgttagcattgcatggcggccccggcggcgaacatgaatattgggaggacgcagccaaacaactcaagaagcaaggcttggacgtgcaagtcaccatgtacgaccaattgggttcatggtattctgacagtcctgatttcagcgatcccaagaaccgcaaagatattttaaactacgattatttcttaaacgaagttgacgaagttcgtgaaaagctcgggttggacaacttttatctcatcggccaatcatggggcggcctgttagttcaagagtacgctgccaagtttggtcaacatttaaagggtgccattatttcttccatggttgatcgaattgacgattacaccaagcatctcgaagaagtccgcgagaaggcattaactccggaacaagtggcttacatgaaggattgtgaagccaagggtgactacgacaacgacaaatatcaatcatacgttgatattttgaataagggatacattgaccggaagcagccttccaagctgtcgcatctgatcgatgttactaacaccgatatctatggcgctttccaaggcgataacgaattcgttgtcactggtaaattggctgagtggaacttcaccgatcaattaaagaacatcaaggtgccaacactggtcacatttggtgaacatgaaaccatgccaatcgaaactggtaagcgcatggcacaaatgattccaaacgccaaattcgtctcaacaccagaaggcggccaccatcacatgatcgataatccggatgtctactatgatcatctggcaacctttatccgcgaggtggagagtgatacgtttaacaagtagagtgtgacgagcaacgggtgatgcggtgtgtaaggccggaaagattgaaatcccgggcttggatttaaagctttttggacttacacgttagacaaactatattacgtcaaggaaaaataatgactttattgaagtttattaccccatttttgagcgtataagaaataagcttcaaaaatagttattttttgaatttgataattacatggtttttaggcttggttaatctctaatcaccgtctcagaccatgggtcattgtattttagaatgtggtaaataattcgaactagcttcttgactacatggcttaatgccaccaaatatggtttgccctcagacctctttttctgataatacgctcgcatggttggcgaatacattgcgcacagtctggctgcttgaaagagcgcccagcgtagctgcgttgaaccgtgcttaaccatgtgaccgtagttaccttgcatttcaccagagcgaatgattgagggctcagcaccggcaaatgccagaatctggtttggtgattgaaagtagttcacatttctaatttcggctaaaataatggcggctagtgtttctccaactcctggaatcgataggagcggcgtcttaatccgattcataattttgtggatcttttgatcagcttccttgatctgctgggtctcaaattgtagcgcatcgatcaactgcaggagttgaaatgaaagactatcagatgcttgaccaatcgtttctctggccagttcacgaactttaattgccatttcctcgccatgctgcttcatggagtatttggtaatgatgtttgtcatcgtgttgattcgtccatgagccaacttatctgttgacgggtatctcttcaaaagtgccaacaaccactgactgtactttgcggatactggcccctagatttggcgcccactcaagaaattcttggtcgaggacatttgtaaatgcgagcttggtttttctcgtttacgctaaattcctcccgataccgggtatcactcttcaattaaatgatatcggtttatgcttcaaagctaacatgagtggtatctgaccttcctttttggcaatctccaatgcatcgttgtggatttgttcttgtgagatacaaggtatcactctgcaaatcattatgattagtattgggtcgtaagctaacactagtaatatgtgacgtcgcaaatagccgatctagttatacatcataatggtcggtattctttaatcccaatttaacgtgaccatcatccgtccggacatgttcaagtgtgtgaagcagccatcaaaaaaccctcactattatttagaatttccagatcagctaatagtaccgttccttggtcatcactaattgatagatgatgttcatattttgcaacatcaattccagcataaatcatcattaccgctcctcacgtatgtaattaacgctgtgctccacaaatctcttgccctgtattcttgcattaaatgaaacatcatatcttgggatatgtgttatcaaaactaatcaacagtacaacaaaagactgtggttagagtctaacgtaaccagtatccgttaggatccgtacctcagatggactaatccacagcgcttaatatcagtttagtacaaattaatgttaccttgctgacatctttaatatacaagcatcagttgcgtcggaacacattttaatcagagtgtgacgagggctgggtgaggcggtttctaaggtagctttggttgaaaccctgggcttgggttttgaccgaagctggcttagagttagcctcaggccctcggaacacatttcaatcagagtgtgacgagacccggttagagcccggaacaatctcaaaaaccaaacaagcgccgggagaattgcatgtaaattgcaactctcccggcgcttgtattattttctcaacgaatctctctgaagtaatttaattggcaaaacatacttatccagcagttgatcgtcatttttctgaaggcggctgaacaacaaccgaaccaacaaatccgcgatgtcttctaccggctggacgattgtacttaattctggatgatactcctggacgtaatccgagccatcgtagccgatcacttgaacgtcttcggggactcgcatccccgcccggcgcgcttcttgaatacatagcaatgcggtttgatcatccgtacagaaaatgccgtccggctgatcagccagcagtttttcacgtaacgtagcccgacgaatggtgggcgtcgaattaaacggaaaggccaccatttgaacaggacagccatgttccttggcaatttgttcaaagccggttaatcggcggttattgggagcccgcttctctaaactaccggacacgaccatgaacttcttggagcccttttcgatcatcgtccgagccgccaattcaccccctgcctgattatcactgctgacagtcggaattttcgtttggaaataacgatcataggaaacaatcggcagccccgacattttatattccttaatcccctcgttatgcgaaccagtgataatgccatcaacctggttagccatcagcatttttaaatactgctgctccttttcgggattgtccatactgttacagataatcgctttatagccacgggcaaacagccgattttcaatttcctcgaccacttgggcaatcaatggattctccaggctggcaaagatcaagccaactaatttaaattgttttccttgaaggacccgggcggccaaactaggttggtaattcagctgctgcatggcagaaaagaccttttcttttgtggcagctgacaaatagccccgctcattgatcacccgagaaactgtggtcacggaaacaccggccaactttgccacatctgctaattttggttgcatgaaatcaccttctcagcgcgttttgatagtaccagtatagcatattggaaaatctttttatgttaatttatgtcaaacgattgacacatcgttatgtaagcgtgtatcatgtgttttgtgaaaggggtttcaaaatcatgagaggtgagcacattgattaataatcaacaaaatccgacttggtggcggaatgcagttggctaccaaatctatcccaaaagcttttatgacagcaacaacgatggtatcggtgacctaccgggaatcattgaaaagatcccctacatcaaatctttgggagtgaacttcgtctggctgtcgccattcttcgcatcaccaaacgtcgataatggctatgacgtgtcagattatgaagatattgacccgcaatatggcacattggatgacacatttaatatgatccaacagttccatcaaaatgacattcgggtcgtcttcgacctggtcatcaatcatacgtccgatcaacaccactggttccaagaagcgaaaaaatcggttgataacccctaccatgatttttacatttggcgaaaaccggttgccgaaaaggaacccaataactgggtctccttgtttgggggttcggcctggacttataacccggcgacagacgaatattattatcatctgtttgccaagcaacaacccgaccttaactgggaaaatcccaaggttcacgaagcggtcaaacaaattattgactggtgggccaaacatggtgttgacggcttccgattggacgccatttctcacttaaagaaaaatcaatcgtttgcagacgtccaggatcaagaagcagccatgaataacgttccaggaatcgacaagtttctcagtgagcttagtgctgatttcaaacatgatcacctcatgaccgtgggtgaagctggtggcgttccagtcacccgcgcccaggaatgggtaaacagcaaaaccggctacttcgacatgatcttccagtttgaccacgtcagtttctgggaaaagttcaccgtcggccaaatcgacgtggcgatgctgcgaaaggcgttaaccaactggcagaatggcctcgagggaatcggctggaacgcccttttcctggagaatcacgatttacccagagcagtttcttattttggcaatgatggcaatctgcgtcagcaaagtgccatggccttggcaatgatgtacttcttgatgaaaggcaccccgttcatctatcaaggccaagaacttggaatgagcaacgtggactttgacaacatcgatcaataccgcgatctggattccaaacgcttttatcaagaggaactggccaagggcgcaaccaaagatgaaacgttgtttaaactccaaaaaaagagtcgcgataacgcccgtacgccaatgcagtggacgtcaaccggcggcttcagtaatcatcaaccttggatcgaaatgaaccccaaccatcgaaccgtcaatgttgccaacgaacaagccgatccacaatcagtcctcagtttttacaagcggttgattgctcttagactaagcgatccaattttactgactggtaagtatcacttaatcgacacgcacgatcatcaactttatgtttacgtccgcgaatctggtcatcaaggctacctgattatcaccaatttgagtgatacgccggcaagttaccagatcacctcggattatcggaacctcgagttaattctcacgaacagttcggctgaacaaaatcccgctaccatgaagctccagccctggtcagcctacctttacaaatacgaaaggaaataaccaatgaaattaaacaatcaagcaatgctcattacctatcccgatagtttgggaaataatatcaaagatttgcaaaaagtcttgtcaacatacctggacggtgtcgttggtggtgttcacctgctgccattcttcccgtcatctggtgatcgcggtttcgcaccgatggattataccaaagtggacgaaaagtttggcaattgggacgacgtgaaaaagctgtccgagtcatactatttaatgtttgacttcatggtcaaccatatttcaaaacaatccaaatactttaaagatttccaagctaaccacaatcagtctgcttatcgggatctgttcatccactggaatgaattttggcccaagggtcgtccaactcaagaagatattgatttaatttataagcgcaagccaaaggcccctgttcaaacggttaaatttgccgacggtcagaccgaagatgtctggaacacctttggtgaagatcagatcgatctgaatgtgaattccaaggtaaccaaacagttcatcaaagataccttgaacttcttgatggaccatggtgcttctatcattcgcctggacgccttcgcttacgctatcaagaaactcggcaccaacgatttcttcgtagaaccggaaatttgggatctactgaaagaaatcagtgacatcactaatccacgtgagaccactttattgcccgagatccatgaaaactaccatattgtccgaaagattaccgaccatgattacttcagttatgactttgccttaccaattgtaactttgtacagtttgtactcaggtaaggctgatcgcttggccggctggcttaagaacagtccgatgaaacagttcacgactttggatacccacgatggcattggggttgtggatgccaaagatattctatcggacgacgaactggattacaccaaagctgaaatgtataaagtcggcgccaacgtcaaaaaagtgtattccagtactgcttaccataaccttgacgtttaccagatcaataccacttactactcggctctgggggataacgatcacgcttatctgcttgcccgtgccattcaagtctttgcaccagggattcctcaggtttactatgtcggcctgcttgccggtaagaacgatctgggcttgctggaaaagaccaaggaaggccgcaatatcaaccgtcactattactcattggatgaagtagctgaagaaactaaacggccagtcgtcaaagcattgtttgatctcctccgcttccgtaatcagagctcggcgtttgatttggaaggtggaattgatgtccaacagaatggtgacaatgaaatcgtggttacccgccgatccgaagatggtcagacttccgcaactttgtccgctaacttgcagacccaagcctttaccattaccgaaaccaattccgatggtgagactaaggaaatattaaccagtaatttgtcagccgttaaataagcacacacactgaaaagaggattaaaaatgaaaatgacacaaacattgcctgcgggttcccaatcactcacaaatgatgaacacattaccaacaaagaacgtttaagctatggggcatccgactttgcctgcaatatcgccaacggtatggtcggtacctacttgatgtactactacacggatgttttcggcttagctgccggggcaatcggaaccctgttttttatcgctagaatcgtcgatgcaatttccggtccaacctggggcattatgattgatcgcacccatacacgttggggtaaaagtcgccccttcttcttatggttctccattccatacgccatcttcttcattctggcattctcgtccgtcccactaggaccactgggcaagttggtttgggcatacgtcacctatattgcaattgatattttatatttgggaatcaacattccaattacttcaatgctgcccagcctgaccgccaatccacaggaacgggttcgattcagtactgttcggcaagtgttagctaccaccggggccacgttaatctcaatcatggtcctgccggcagtttcactgcttggtcaaggtaatgacaaaaagggtttcttgattaccgcaattttggtcgcaattctgactgcgttcttactgttgttaacgttcaaaaacactcgtgagcgtgtccatccccgtcaccaagaaaagctctccctcaaggagtccgctcgggcgcttaagggcaactggccttggatgattatttccttaatgtatttcttcttctggatcgggatgcaaaccaagcttcaagtaacggtttatttctttaaatacaatatgcacaatgcagacttggcttcgttcatgcttggcctgcaggcactttcgctggttgtgattgtctttacgccatttttaactcgccactttggcaagaaaggcacgatggtaattggtcttggcctttgtgtcatcagtcaattagttcttggcgtcggtgctaagatgatgaacgtccccattctggcgggcgcgacgattctcgggtactttggtaacggcttcttcgctggactgctgccagttatgcttgccgataccgttgattacggcgaatggaaaaacggtgttcgagctgagggtctggttacgtcattctccggaattgcctccaaccttggcatgggaatgggtggtgtcgtcactgggttcttgctcagcatgaacggctacgttgccaaccacgcccagactgcacaagccttaaatgccattgagatgaacttcgtttgggtgccgttcattggatttggtattggattaatcttgatgtacttctacaaattcgataaaatgcaaccgcaaattgaagcagacctcaaggcacgacatgaagctgcttaaaccacaacttaccatttgaattaataaaggacccctgaagttagtgtacagatgctagctttgggggttctttgactgttacaaatatgcttgataacccaagataattgccaagacgaccgcaaatattcccactgcggttttgataactttggatggaatataccgcacgatgatcggtccaatgtagccaccggtaaataaccccagcaacaaggggataatcactgcccagtcgattggaatcgtgaagataaacatggttgctgccacgatattattcataaacgaagcaaaattgcgcattgaattataaatggcatagttttcatgaacaatctttgaaagcaccgcaatcattaacaatccggatgccgcaccaaaataaccggtatagattcctaccaggaaagtacttacccagcttacagcggtaataattcggctatcaaatgccgatttgccatggcgtttaggcgtcaagattaaaattccggccaacatgatgaaaactggaactaatttcttgaaaccgctattggtgctatgaattaaaatgagagcacctaatacgccgcctaaagtatttagaatcgcaatttgaaacgcctgtttccagtgaccatgcagctcccttaacgaggaggttacggttcccagcccgccaccgacttgagcaacggtaatcgttgcgttggcagtaatcggtgccacgccaaccgacagtaaaaccggatacaaggtcaacgatgccatccccacaattccagttaagactcccgctaagagactcatgagcaccaaataaataattgaaagcatacttttcctttcgcatcacaggcaccgtggtttttggctacgcctgcacataccaatatttgacttaagaataacattctggggttggaattcaaacgttaacgcggcttctggctgtcgatacttatgtaccagggaagcagctcgccggctacttctctgacaattcattaataactcacatgaacatactttggactagccgtcacgtagccaccctttacttggaaacgttgacttccagtgaccctcagagaataaggatgggcataaacaactttgttgactttgagaatggtgcccattttgagctgtttaacatgtttatcgaagttggtgttgctataaagataagtggctttaacaatcttcactttctttggttgctgatatttttcagccgtgaccaatttacgattaccggtgacatagtggccatttgaaagcaggtatcgggttgttagatggtatttgataaatcccttaactttcaatttagtcccttgcttcaaatttttaaccttcccggtcaagctcttgtgcgtgtattcgttgactccagttgggttaatgaccgtcagctgttggtgattgctttggtaataaactggacggacgaatgcccaatcgctagtaatgtagccagtcttgccagctgttttgctgtgatggttgacgtctcggacagcgtacacaatctggccgttacttgccttcacctgtttggttaccacaaacatcggccgattaattcgtggcttcttggtataggtggcgattcggtcacgtgactgcatgtctttgtccttgtacaagctgatcgttttcactgcgtatacagcttgattcttttgtgctaggggatgatctggggttggaattgcaccgggttgcgaaactgcggtggttggactctctgcggcccctatcgattcacttgagcgatttggtgttggggtagtttggggatttgttggccgtggttgactgggtttcaccggtggaacgactggaatctcaggctgtttaacaactttgacaaacgcacctaagtcgtacccacccagtcgatgaattggctctggattggtggcgttctctcccaagccatcattctgctgagcttcatagtgcataatgaccgtaaattgatttggggtgtcggcaggctttggcaaatctgtcatctgtcgtttgttctgatcgttcttaaccttggcaacagtgacatccgtgtcgtttgccaacacatccacatcaacatggtcggggttaatttgttcaactccggcaatcttgaatgaggcattaattgtctttgttaaagctgcccatgtcagtggatccttggtcaccacatctaccgggagcaaatctttagaaacaagaactaaatggttctcgtcaggaccggttggaatctggaattgatcaccaaaggctcttgcactcatttcaatgtccgcctggccaagtgagatgctcgtcaatcggttttccgaaaatgccccagtcgcaagttgggttgccttgggcaaatcaactcgtgtcagtttattgttggtaaatgcccacttgccaacagtttgaacattaggcagtgacacgctggtcagttcgttacccgtaaatgattcgtcgccaattgtggtcactccaggcaagtcaatgctggtcaactgattgccatagaaggcattataatcaattgtcttaatctggttgggcgcttcaaatgtgaccgctttgatcccgcggtattctggaatcccaactcctgcttcgtcgatatttccaactgtcgataaattgtcggtagagaatgcatccggaccaatgccagttactgtttcaccttgcagtgttgctgggactaccaaatgaccaccttgaagcaattgacgggccaaatcttcattttcgacatctgtaatgatcccgtcctctatggaaacatcatcgtcagttaaagtaattgtctgattttgttgcatcgttaccttttcaatcttagatcctgcagagtcaatcgtatctgctttgaccgcaataccgccgattccaaataggagtgttgttaaaaagctgatataaataagtctgctcgtcttcatattggggacctcctcatcaatcctgtcatctctttacacctgtattttaacacgtatggttataattactataaatattgtcttatagttaatgccattataatcattaaatcagctaaattcattcattttttggcaataaaaatggaccattcgtctagtcccggcaaatggtcccagtatgctaactattgaattgtttctgtgattgcttccttcatggcttgtgtactcaactcctggccaattcctggtcgatcagggattgtgaaccagccattctcaggcatgtcatgatatttaccggaatcgatattgggctgcttcaaggaaatctcatggtactcatgaatcagagcattgggcgatactgcctccagctgtaatgcggcagccgttgcaatcggactaccacacacgtgaagttgaacactgacatcgtcaattgccgccatatcgctaatctttttagcttcagtaatccctccacaaatgccaacgtcgggctgaatcacactcagtgatcgttcatcaagaaatggcttgaacccgtatcgagttaccaatcgctcaccgcttgctaagggaatggacaccttgttccggatttctttggttagctggggattcctcggtgagttgggctcttccatatagtaaatgctcaggggctcaaccttagcggcaaacttaatcgccgaatcgacgttcaatcgagcgtggcattccaaaattatatcaacattctcccccacggcttggcgaacagccgcaatccggtcataatacatttgaatttgtgcctgggttagcagctgctggtcatgcacaccaaatgttccatctgcctgcatcataaatggatcaaccttgagggccgtataaccttcttgaacagctttttctgctgcttgagcataatcctttggtgtcgccagaaattcaacatgcttgccccagccgaactggatttgactggcgtaagctcgaattcggtttcgggtctggccacccagcagctgatacaccggggtatgaaagtatttgcctttaatatcccaaagcgcggtatcaatggcactcacagctgaataaaagacaaccccgccgccttttccccaaaacgtatcttgatagagttcattccagatggcttcattccgcaatgggtcttggccaatcactcgatggaccaagtctttcagactgccaacagctcccaaactgccactgccatatgccagtccagcttcaccaaagcctgagataccggcatcggtattaattcgaatcacaactggatgccaagctggcatgagtccaaaccactgcaattgaaagatatcaacactgataattttcataaagcgccccttttcagcctttaaaactgctcatcatgtaagcgatccaacatgatctcggccaatcgtttcgatggaatcggcccgatactagtcgtcaaatcagcccttgcaaaggcttccgtgagggctgataaattaaattcagtcccatctaaccgctcggtaatggcgtgaagattggaattcggttgcaagaaatctccataaatttttgaatcgaccacgtggttgtcttgaatcgagaacccgattccgaccgttccaataccgttaaaataaccatctctgtaatattgatgttgattgccagcgccaaaaatccaggtcttgctgccatatttagtatgagccaacgaaacaattgcctgccaatctttctcggttaatcgataggttggaacttgcgccagatcagttgtttgaaacacttgggttaaaattgtttgttgaacttgatcgattgaaactgttcgatgggcatcatcaaagtgctcgcggagatttgtcacccgactgtgaaccgattgaacgcctttagccctcaactttgcccgtgatggtttcaacactgagctggcagcctcgatatcgacatcaatcatcagcgtgccgccataggacacccgatgaccaattttggaagctgacatcccggaaaacttgcggccatcaactgttaaatcatttcgactgtcactctcagcattgacgccaagggactgcaacgctttaacgactggttgggcgtattttctgaaatggggatgttggacagttggctcagtatcaataaaaacgtacgtcagatttccgggatcaacgtagacggctccaccaccagaacctcggcgaaccaaatcaatcccgtgggcctggagataagccatattcacctcggcaaaaacgttctgatgaacgccacaaatgacaattggcgtttgcgggtggtagaaatacaccagtgcatctgaaaacttcgccgttgtctgcagatattccggaaaggcctgttcaactgttgggtccttcaaatatttcattccattggatgtatctagataatgaataatgatcccttctttgagactacttcttaatatacatatacttataattccattgtgaccccgttgtattgtgggtaatgccgtgcaaataaggccgtttcagatataagttgtaattctggaataaaggtgtggctccttgatcctgcataataatcttctcagctgccaacatcttgttccaacgaatcgatgggttggcgttgttggtataaattgactgactgatcaactggtcaaattttgcattatgccatgagccatagttcattgaattcttgctcatcatcggctgtagaaaggcggttggatcagcaatgtcagctccacgaccggtaatgtatgcttcaaaatcgccggaaactccgcgcgcatactgaacttcttgagggaccgtctgaagattaatcgtcaatccaggaagttgtttctcagcggatgatttgataaattcactcactttcttcacgttatctgaattggcaaccatgaggttaaaggccagcttcttttgaccaatttgttttaatcctttgttccaataatccttggccaacttaggattataggcaaccccttcaccgccatattgttgagaagcaaagtccttattgttggccggatcataagccaaatatttggtaacaaatccagttggcttcagtgattcacctttcaagagattgttggcaatttggctgcgatcaatcgtcaatgaaacggctttgcggatgtccacattattaaaagctttccgcaaggttggattcttgatcttttggttataaaccaaatagttcatgtatgagtatggaccgtggtataggtcggcactattcttataatgtgtgacctgatcgccaattaaaattgtaaaatcaagtttgtgtgcctgatataacgacaaactggtctgtggatcagtcacataattcatatgaattgtgttcatcttgacatgctttttgtcccagtaatttggattctttttaaatgtccaagtattggattgtggggcccattttttgatgacatatggcccggaaaaaacggccttattggcagcttggccatagctggcaccgtatttgtcaacgatctttttgtcttgtggtgaaaaggcctgataggtcatcaatttagtgaagtaggcaatcggccgatccaagtgaacaacaaacgttcgcttattcggtgccgcaacgcccagcgcgcttagcggcagtttcccaaagttgaccttttcggcattctttacgccatcaaacagataagcatgggtggacttggtcttgggattcaacgtccgttgccacgaatagacaaagctgtcagctgtaattggatccccattactaaacttggcgttctttcgaattgtgaaagtataagtcttaccgtcatttgacacgcgataccgacttgccagcgccggaaccggcttatgattcttattcatgtacaacaaactatcatagagattaccggcgttatcgaagccctgggcttttgaaatatccagggtcacgattgaatagttcgccgacaagttggccgttcgaaccaacttgctgttgtcttttgacttagtctggctcgaacaagccgctagtgtccccacactcaaaacacctgctgctaaaaggagcaaatttctcaaataatggttcatattcttaacaccattcccttcaaataatcctgttaccgcttacaagagctccccaaaataagtccaaaggacaggcgaccaaggggagaaggtcgctggctttgaacttttaacacgtgaatatcttacaacaggtttaccacataaaccaaggacaaattttggtacaaaaataccacacaaagaattatttgtgtggtatcatatttttatctcattttacgattcttctcgaatcactggtttttcctttaagctcaattgctccacgttcaagactttatcgaccaatccatcatagaagctggactcatggctgacaataatcaggttgccagggaaccggtccaatgctcgcttcaaggcctctttagtctcttcatccaaatgattggtgggctcatccataatcaggaagttggtcggggtgaactccatcatggccaatttgaccttggtttgttcacctccggaaagttccccaattggtttaatggcattggcagcatccagaccgcatttggcaagcttcgtccgaattgcccgttggtttaatttagggaatttatccgaaataatctgcatcggcgtcatccggttgttatcccattccagttcctggctgaaataactgatgtgagatgatggcgagaacttcgccgtcccccctttggcaggcagttgaccgaggattgatttgatcaaagttgacttaccaaccccgttaaatcctgcaaagccaaacttctcccccattgaaatagtgaaggtgaccggcttaagtaatggcttattgtaaccaaccgacaaatgatcaacggtcaaagcttcatgagaaccggtttcttcataaggaaaattgaagctggccttgatattagtcgaaggcgggtcaattttatccatatgggccagtttcttctcccgcgatttggccatcgtggacttggaacctgccttgttcttacggataaagcgctcggctttctcgatttcgacctgctgcttatcgtactcacgctgttggaattcttctctctcagcccgttgacgcatcgcttgtttgaaactaccacggtatttggtaatcttcccaaaagcaacgttgatgatacagttagtgattttttccaagaaatcataatcatgtgagacaaccagtgcagaaccgctaaacccattcaaatagtcaatcaaccagtcgatttgagcggtgtccagatagttggttggctcatcgagtaaaatgacgtcgggatctgccaacaacattttagcaaggatgatcttggaacgctgaccacctgacatctggccaaccaggtgatcacgtccaatgttatctaatcccaagccggtaatcgtctgttcaatcctggtgtcaatgttatagaaatcgctggaatccaagatatcctgaagtttcccagcccgctccaacaatttatcgtcggcagtcttagcataggtattataaagttcattcaattggtcactggttttgtataaatcagcaaatgctgtgcgcaaaaagtcgatcagggttaaatcttcctcgacatcggcatactggtccaaataaccaattttaatgtttttctgccactttatgtccccagaaagaggcagttcacttccggtaatgatcttgatgagcgttgatttaccaaccccattttgacccaccacgcccatgtgctcgcctttttcaagcgtaaattcagcatctttgtacagatccttctcagcaaagctcattgaaagatttgatacggatagtaatggcaaaaaagttcactccttaattaattcgaaatactacatacaatttgttacgttactcttgtttcctatagtagtcaaactaatcgtgcgaagatttcgctttggtatataatggaaacattacttttaaaggatgatcataaatgaatatcagagaaattgaatacattacaatccccgtctccaacctggaagtcagcctcagattttaccacgaggtctttgacctgcaaattgttgatttacccaacggtgataagggagcggacatgcacaaaatgttacttgatttccacgaggaagacaaggtcgacaacccaatctcatttggcttgattgctaaagacaaaatggccgatatcaaagcccatttgattaactactttgtggatattgtgagtgaaccgaccgaaaaaactaaagtaaggagaaacgttaattcgatcacgattttagatcctgacaagaatcggatcgaagttaacgagttcagataaatgaatccaaccaggtatctcatcactaaatcaacgcaaattttaaaattcgtggggtttctggcaacttatattgtagcggaatcagtttttgaaattgccggtcaatacatcaaagaccctctgagtgctcgtcaccttctgggactggcactggttttgattgccggcgccctggctttgatcggttggcgttatggtaaacagctcgctgctaacaatccacggcattttggccgacggcatccgactgccaagcggatcgcccaactgttatggatttttattttgatgacggctatccagatactttggcagtggctcattgccaaccacgtcttgacaacacccagcaatcaacaagctgtcgaagccgccgaagtcaagatgcccatgtggaacatcttttttggcgggattctcgcaccgatttttgaggagcttatttttcgtggcatcttcatgaattatttcttcaataaagataaccggctgaacaatcttttggcagtcatcgtcagcggctcgctttttgggtttgcccatgagatgagctttgacctgacttggatcatgtattccgccctcggctgctgtttatcgtttgcctacatgcacttccgggatattcgttatagtattgcacttcatatgatgaacaatttgattccataggatgagaatatgaaccgcactatttagtcataaaactaaagcacaatttaaaacggagatcggaacacagctcacaatgagctatgcctcgacctccgttgagatccactgttatctagtttaaacgtggaacgatcggccgctcccggccatttaagcaaaaaatcgagttattccaagaacaggaataactcgattttttgcttaaattctgggatcaaaacgcctcgcgtcccattctatttaattagaatgattcaacttttccttagctgctttaggcacttgtgagtaaggaatcccttcatagtcaacgacattcttcgatcttgagtaaccaatcttgatatagtgtcccttgacgaaatacttaccgtcaactgaacccacttcaagggtcttaccctgacctttgtcattgtaagccttaatcaaataataatgaacatccggattattgccgggcgaattctcagttcgttccaatttgccaacttggccatagtaaaagattctcgcataattgtgatgataccagatgccaccaattgcaccaagcacaacgagaaccgccaaaatgataattgttcttttcttcatggtcgatctccctcatattctgtctatggacaaactatatctaatcccaatcagcctgtcaatcaatttgccaggtcactatttgggcatcatttcttccaaataacgttccagacgtggatcatgggcgtgcagatacatccctttaatcccccgcctcagcaaaacgttcaacgagtttcttaacagttcaactttgctttcttcataatctttttccgacatgtcggaacgatgcttgaagatctccacgtcagtgactttactgggatcgacgcccagacgattatcagcagttaaataaaacggcggcccaatgataatcccaatgtagttcagatcaaacccctgaaccgtgtaaatgctgccgacctcgtcaatcgtttgtggctgctcagcccatggggtactggtgaaattatattgatcccaaggcagatggaagttgccttcgttgaccaaatgtttcccaccatctaaagtggatggatacccactggttgacgtcattcgcgataagccatactggttgtttttcttgatgatcgtttgaaacatcttttcagcatcggcgaaaatacgaaaatcatagtcgccaacgtcactgggaatcgcgggtataacatccccgtcaataaagtgatccagccaatccatcagcttcgggccggcctgcattctaaactgctgcttaagatgcaccaaatcgtgaggatatggggcaatcaatttttccaatctggcgttattccaaaagctcttggttcgcagcacttgatgcggatcaaaaacaacaattgtcacccggcttaaattgatgatgtcctgcagctggttgtcaccatagtagttattgtagtgatccggcttgctcagcaacaaatgggcctcatcgacaaccgtcaaattgacctgtttgccctgcttatgcatctgattgataaagctcgtcggccgctggtagtactttttcagcatgtgtggggtttgcccagccagctcgcgatacacttttaggagttcgggatgattgaccagaaaataggcatcgtcaacgacttgggccaactcggtaaacagttgattcaagatcaaacttttgccggtcccggcatcccccatcaaaacaaacaccgcgtgcccgtcttcttttaaatgttggcgagaaaaggcgtcaatttgctttaaaacagctttctggtggtcagtcagttcaatatttttcgaaaatgcatttaaggtgtgcgattccaaagattccattgagttactccttctctcaaagctcataatatcatgataacttttcgccgttttaatttccagaaagatcaagcttgcaatcgctaccaattatcatgaataatagagacaaacgaatcagcgaggagaatcagcatgccaactttcattaacggaaaaatattcactggaattgaccagacgacttttgtttcagcgatgacaattgaagatggtcacgtcacttgggttggtgaatccagtgacatcaccgatcccaacgcaattgacctacacgccaagactgtcctgccaggattgatcgacgtccacacccatcccaaatacatcgccgatgccctgcacggggttgcctgcacgccgcccaacgtcaatagcatcaaagacatgcaagctgccctgcgtcagtcaccggcatttggaaaaggcccagacacttggatcgagggctggggctttgatgaaaccaaattagccgagcaccggacgccaactgttgatgatctggatgaaatttccaccacgcagccgatttttgtttatcggtcagattgccactcatcaatcggtaattccaaagcgctggaactggcggggatcactgcaacaaccccggatccggttggcggcttcattggccattttgatgacgggcggccgaacggctacatgaaggaagtcgccgctacccaattgttaatcaaggctaaatcagcccagagttatcagggcgatgtcgataatatggcgaacagctccagacattacctccaaaatggcattgtcgccatcggtgaaatgatgggccgcattcgaccgtacgactcactcaaactttaccaagatgctgtaaaggccggtttcaaaccgaagtcatccatttactacgtctacgatgaagtagccagcaatgctaacctgaaaccgaccaatgatgatcagctacgcattgccggtatcaaggtgttcatggacggcagcatttccggtgaaaccgcctataatcaacaaccttatccgagcggccaaaatggagtctgcctgacggacgcaaccaaactcaagcaagctgtcacctatgccaaacagcagcatctccaagttgccattcacgcgatgggcgatgcagcgatccaattgattttggatgtgacagataaaatgcaaccgtggctatcggaccgtccgtcaatcagaatcgagcatgcttccattctgagcaatcaaatgctgaaacaaatcaacatggcaaccatgaactacgccctggtgacccaaccgattttcttctttgccgaggatgaatcgtaccgtcactatctttccccgcagcagttcaatgaagcctaccgtgtgaaatcaatgatgaacaccaaagccgagtttgccctgagctccgatgccccctgcacaccatgggctgaaccggatagcccatttgtgaacatttacgccgcagtcactcgaaccgcggtcaatggtgacgtcgttaatcctgaagaagccattccggttcctgatgctgtgcttgcctacaccaattggccggctaggattggcggttttagtgagaacggccagctgactcctggatatgccggggattttgttgtgcttgaccgggatattttctccgtaccgcatgaggagttgaaagatattcgtgttgctgagacttggatgggtggagaacaggtgtattaggacacaaaaaaggcactcagctgagtgtctttttttatggggttttaacagggtgctcacagatttagaaaatcttgcttattctttaggtttaccgctttcgtcacgttcaccagcttgaacaggattttctttcttcaaagcaaatgccgcaaagacagtaacaacagctacaatggcaccaagaatcaggtatgtttgatggaaaccaattgcatcatataagttaccggcaacacttgagaagatgaagactgatatttgcttggcgaagttcgacgctaaggcatacacagttgcgtatacaccaatatcgaaagcaccagcaatatacttcataattgatacaagaaccaaaggcatttcaagtccggctaagagtcgaagaacaatgacccaaatcaaacttggtgacaatgcactaccaatgatccgaatagctaagatacagccataagcgatcaaaccatttcgtgaaccaatccggttgataatccatggcattgggaacatgagcaggaattccagaccaatttgagcagtggtcatgtaactatatgcttgagttccttgagctgcagtattaaagaatgtcttgaagaagatgatgaactgttgatcaaagacatcgtaaatggctgaagcaccaatgtagaagattgataggtaccagaagttcttaattttaaagatcttaccgatttgaccccagtcaatcttgtctgaagtgttaccggctgcagatgcattttccaagtgaactttatcactgaagatcagtagtccagttaggataattgctgaaacggtacatgcccagaagattgagtatggtttccagatgaataattgtccacccaggaatgaagcacacatcccggctaaggagccacccattcgtgagtgaccatattcaaatccgttagccaaacttgcacgttgaacatactgttcaattactgaaacaccaccgttgaagatgaaactaaggaagataccagtaataacggctgcaaacatattgcttatgtgagcaaatggtataaacagccactggaagtatggtccaataaagatcgcggcgatcgcaattgtgataattaagttctttttgaataatagcttatctgaaataacaccaaatgctggttggaacagtaatgacattccggccatcattgagaatacaactccggcttctgccccatttaaatgggcaacttgttccagccaaagggttaaataaccattaataatttgccagttaaagaagtaggtaaaatgagtaaatggaaagccccaaaaatccttcttctctttcttttcaggcatttttgcactgttatccataacatgtgcctcctattaaaatttattaatcataattataaggaacaggcttgccaaagttaggcgtcccgtcttcattccaagtaaatggctgaaccttggtgtgacggtttggatcgtacagtggatcacctttaatctctgtgtaatcacggcaatggtaaaccaaaatatcggtcttgccgtcttccccaaccgtaaaggagttgtggccaggtccatattgatgggttgccatatcactttggaaaaccggcttcttggacttggtccagttgcttgcgtccaacaaatcttgatcatccgggatacttaacatccccattgcgtaatgttcatcggtggcgctggcagaatatgtcaggaaaaagcgaccattacgatgaatgacggctggtccttcattaacccaaaaaccaatcgtttcccaatcaaattcaggttttgacagcatgaccggcttcgttttgagcgtccaagggttttccatttcagcaatgtacaagttggaattacccttgatgtcaggatctttttgcgcccaaacatagtaaagcttgttattagcttcgaagcaggttgcatcaagtgagaaactatccatacctgtcttcacttgaccatgttcaaaccaatcgtcttcactgcgcattggatcagcattgtcacattcaatacagaacattctgtgttggaacatgccattcttatccaaggctgtggtttctgccgccgcgaagtaaatgaaccacttgccatcaatgtaatgaatctccggtgcccaaatcaattgactcatgggaccgctttcatgtttccgccaaattgtccgtggagctgcatgagcaagtccttccagtgttttagcacgacgaatttcaatcaggttatatgccggtacagaggcagtaaagtaatagtatccgtctgtgtgtttgtagatgtatggatcagcccgctgaacaatgagcggattcgtataaactgtcaaagtaaactcctcttttcttgattgactacgtagtattgatatcccttgtgcacatctttatgatatttcttcagtaaaacggttacaagccataacataaatgttcaattaacttttgacttaaaaccgtggttttgctaatataaagacgattagtaaccggttacaaaaataagattaacatttatattgatttaaacgtttttactgctaatcaatcaataaatgttaattggttgattcagtcagattgagagtgaggtcacaaagatggatttagatatttctcaagattcgcttgaggtatataaagccttggcaagtccagttcgaattcaaattatccaaacactttcatcaaagcggatgagtgttcaagaattgtcaaaaaaattaaaattaagcagcaccattatcctgatgcatctgagtaagctggaagatgccggaatcatcggatttgaacgtgaaggtcacagtaaaatttcctacttaaaagttgataatatcaacgtccactttccgacgaccatttatcccgcgtttgcagaatatgagacacaagtccctgtcggtcaattcactgattactcagtaaccccttcgtgcggtctggctggtaaaaatgactatattggcaaggtcgacaatcccaagtactttatgagccctgagcggattaaggctggaatgatttggtggacgaacggcttcgtggaataccagttcccgaactacttagaagaaaaggacaaactggaaatgttggatttgtccatggaactcgggtcggaattccctttctccaacaatgtctggccttctgacatcacgttttacatcaatgatgttgaaattggtacgtggaccagtccaggtgacttttccgatattcggggtaagtacacgcccgcgtgggttcccgacaacgttaaccaatatggtcagcttaaagtggttcgcatcaccgatcatggtagttatctggacggtcaaccctttaccgacgtttccattgatgacattgattggaagaagccaacgttcacggttagatttgcgattaaagatagtgcgaagcacaaaggtggctgcaccatttttggtcaaggatttggcaattatgatcaagatattcaaatgaagctatttcacagttaataatatatagaatggatggcgagatttaatggaatttgaggatcgaatgcgggaatttatcttaagctttttagacacgcagcctaaccatgttgatctaaaaacagtccagaaattgatcgattatggtaagaacaacaaatatactgcgccaatgttattaactcagctcaatcaaatggacgatgctcacgaaaaaatcctgacagtcacctttgacgttgattttattgatggtgtcaagctcttcaacaatcatgcaaccaagtggttgacggacaaaggcaaagcctatattcaggaattaaaacgggcccaaagcaaagctgaaaccattgattttccaaaggacgatacccaaactgaaagtactgaatttgatggttatttatctcaactaatgtcagtcgtaaaatcaatgaagagtcagtcggaacgcctcacactgcaggaatttgctttagagttaaggcatttattaactgacacgaaaaagctggacaaaggtgccttaaacaaattcaaacccttcgtcgatcgcaactggaacgaactttcaaccccaatgacgccgatcttggtcgaattatcaaggcgctttttgatcgaaaatagttatgatgattaaatcgcactaactaaaacgagcaccaaactcaatcaatcgctgagtttgatgctcgtttaatatccacttaaggtagaaaatctattataaagactgaagccattcaagacacaatgggaaccacttggcaaagtgttcatcggtccggtcgcgattaacgacgccgacaaattggttggctaggctgaagccatgaccgccagtggcaaattcatggacttcaaagttaacatcattcttaaacagtgcttcggtgtatggatagatgtggtcgatgtatggtgccaagccatcacttctggcaccgaagagaaatgttggtggtgtgtttttagtaacctgcttagtaacatcttcactgtgaatgccaattttttcatcaagggcctgtgttaatacagggtagcccaagatggcaaacttagctttggtatccttttgattggagtatgctgcggcaagttggccgccggcagagaagccgattacccctaatttatcggtgtcgacattcaaatctttggcatggtctgtgatataatcaaaggccatggagatgctttgcttggcatcttgataatttttcttttcgttaaccggatactccacaacgaatgcctggtaacctttggttagaaaagtcagggcaacccgggcagcatcccgttctttaaatgttttgtaactaccaccggggattaccacgattccaggcagtgcaacgtcactatcagcatcgtaaatgtctaatttaatctctttgtctttatcaaatacaacttgtttaaaattcatacaatcacctcttcttctatgataagtggtgaccggcaaaattgctattgaaaaaacaatttattattggtgatttccttgatatacgtggggttgacccacacattggaatattttatttgcttattgcaattttttataaccttcaaaagtattttgtcgtataattagaaagttaatagtaggtatattattataggtacggggagcggtatctaatcgtaattcgaatggttcctaaatatcaattttctggggagaaaattcaatgattaatttctttaatagacacatcaagctgttctttgcggccttcgttgtggcatcaatttcgtttggaatttatagccaccccaccgcagacaaagcaagtgttcaagttgaatacacaacgcagacgcatccgcatgcctttgcgctgaagaagaacgccaagctgtacacggatgttcatttggctaaatcagtcagcgccaagaagtttttgaagacggcctggtatcggagtcaagctgccaaattgatttgtggcggcaagagcaagatcgtctatcggatcagcagttctaaccaaaagtacaaattctgggtattgaattcagctgttaccgatattacgtcaaaatcatataacgtcaaattggcatccgccggcaataaatacgctggcgaaaagatcggcgtctttggtgattcaattcctgcaggttgggacggctatcacttctatttgaacagttcttaccctgactggacagccaagtatctcggcaccaacactgcggttgaaaacttcgcctgcccaagtggccgaattgttggtaatcgatatgcttatctgggaacaaccttggtcccacaagatttgtcagccgcaatcaaggctcaccgaaatgacatcaagaagatgaacgtcatcttcgttcatatcgggaccaatgattacaccaactattccggttcgggaagtttgaagaatgtcatgcgccacctgcgctataacattaagatgattcaaaagttgaatccgtccgccaagatttacggcatcctgccaatttcacggtttgacgccaatggcatgaatcgtgacaacatgagtgatatgtatggctacacctaccacgacttgcgggcagctgaagcaaggctctacaagtcaatgggcgccaaagtggtcaatttccaacagatcgcacccaacattatcactaacagcaacaaggatgtcactttgaaggatcatgagattcatccaactgcccaaacggctcagaagctggggtatgcgttggctaagtcaattgttaaataaataaacacaataagttccctgcttagcaaatactaggcggagaacttattttttagtggtggaagatgatccagaatgaatgatctgttgagaagccatctctaacctgattgatttgacatccttctaaaactcacattttccacagctagtggatcgtcgggggtttaaccttattgatttaacatccttctaaaacccattaactgaatcatcatcagaactgtcatgggtttaaccttattgatttaacatccttctaaaacccacaatctcgggatccacttatacattaagggtttaaccttattgatttaacatccttctaaaacgtctaaaatggacactatttattcatccatgggtttaaccttattgatttaacatccttctaaaacaatgatttggaagtatgtagatttgatttggggtttaaccttattgatttaacatccttctaaaacattcattgtaataccctccaattgatttccgggtttaaccttattgatttaacatccttctaaaaccataattacaccgccttttattgttcgatagggtttaaccttattgatttaacatccttctaaaaccggtgtcaatgctttgatttgtgctgccaagggtttaaccttattgatttaacatccttctaaaacaagacagatggttgaccaccatccatcaatgggtttaaccttattgatttaacatccttctaaaaccatattatatcattagcaaataatcttcaggggtttaaccttattgatttaacatccttctaaaacgggttgcggcatacaaaaagccacccccgtgggtttaaccttattgatttaacatccttctaaaacttttacagcagcgaaaaaggtgcacgggaagggtttaaccttattgatttaacatccttctaaaaccaaccgctgaactgattccttttcctgaaggggtttaaccttattgatttaacatccttctaaaacagcgatgactgaaacctgttgattcttgcagggtttaaccttattgatttaacatccttctaaaaccaattcaatattaaaccaacccaattgtttgggtttaaccttattgatttaacatccttctaaaaccggcgaatgacgaaagcgcaaaagattgggggggttaaccttattgatttaacatccttctaaaaccgattttttataaccgaattttaatgcattataaatgccaatcaacaaagtcctcgtcgatgtagtaaaagtcgcaattggtataaagctcctgtgacttcatatctgtgaattctactaataatgtcgagatccccgcggaacttgtgagcttggatagatcaattaattgctgctgattaagataatgagcgacattagttaaaccaacagccgacttcaatccacactctaaatgaattttgataattgattcaattatagcataaggattcagcatggtatcagcgttaaaatgaattttacagtatttaaacagcctctttaaatcccaatcataagtgacttccagaggtaagtcgatcataaacaaacactgctggacgaccgtatacaattgattattaatatcagttatcgatttacgctgatcatcagtcaacacagcctctaattgcttaaaaatgccagaattatacttgtcactgacaccatcgctgagtccgacatctccctgccaatcaattgcatctttaacttccactgactcaaaattgtcatcaaacactttaatcttgtcgctaaaagatcctagtccaacaaccagatcatgatagacggttgggttgttcgtggcaataaccgtgagatactttgaattcagctcaatttcttgatgaccggcatacgaaattttcatagaataatcgtcctttcagaagaatttcgaacatcttcctttggtttgccggcaataaaatgcatgtcgttgtattgcttctcggtcataattaacgattgaatcaacccttcaggagaggcaattgctgcaatccgcttctccataaaatcagcggatttcttgttgacgcagactcttacataaacagaaaactggatcatcaagaagccttcattgatcaaagccttgcgaaacttccgataattccgacgattctcacttgtttcaaccggcaaatcaaacattaccattaatcgcattattcggtacctcatttttcaattccacctcaatttgaatttcgtcagtctcaccacttaaatatttcaaacaattccggacgtgttcggaaataatatttcgaaataacatttctttgccattaaatttcatctcaagatttaacaggtccgccaagccaaatttgacatctggcgtcaattccttgaaattttgatttgccagccagtaatcgataactggtctaaaaggctccatcaggtcagagcctaagttgaattgattatcattgctgtgatgatggattcctaagtatgtgaggtaaccattggaaacgatctctcgattcacgttggatagcaaaattgaatagccataattcaaggcagcattcaccggcgaaaaatcacgccggctaaacttattatcaaacaacagcgggaaatatttccgtgcaaccaccgcctcccgattggtgatgtcatcaatttccaatttatcaagttcagcaatcaaatcactgttttcaacgccataaatcgataaaacattaacctgattgacgattttgcttgcaacaatcctcgtccaaagaaactgttggcgcttctcatcccaacaaaattgtttcttaatcaaatcaacatcccgacgattcggataatacccaacggtttcgcaaaccggctcattggcattatctgtaaaaataattttgacctgacttttcaccaactcactgatcaaagcagtggtaatgactgcctgagtagttgataccagtaataaatcaatgtcttcaattggcacttgattaatgccgtccatcgtttggacaatcatatttcgtgacgaatatgacatctttgcgtgctgtgatatgacaactgatcgccatcccataataaaatctcccttgcctcaattaatgaattggggtattattatttttgttgggtagctcccaacatgtttgaccttattgatttaacatcctgtgttaaaatcaagcaaagcgctttgcgcggagtttcaacttttgacccattatatgggcattacatatgcgaaaggaaccattcttcagttggagaatggttcctttttttgttataagtccttcagactgacggttctttcgaataagcctgttggtgactgataacgaatctttgtttcatctgacagcagaattccattaggctgttgtaattgaccaaatggcgttgtgatgccgacatccttcaaattcccgaatgttggatttgcatgtagcccattcaatatttcttgcaagatctcccgtttgccagaagacaccttagtattcccatcaaggacattatggttaggaaatgagataaatttgctgaaaccaagattcaacttgtgacgaaatttattcatatcatataaagaaaaatactgattaaccttgtctaaaatctcagtgtagacgttattgtaatccatactttcttgcagaggatctaatcttcctttgcttgcaagtgtcttgacagattgatcggagaggaccaattgcttggcgttatattgataggttgagcttccaagcatgaacttcttatcaccatcaatcatcaattgtcggtacattacttttcctaaaacaatctcaaaatcttcaatgacttgggtgatttctcccgttttccgactcttcttagtcttcgtgagctgtggtgccaatacatctttgagagcccggtcaaagtccgcatcactgacgtttttcgcggcgtctaaacgatccagtgcccgcattggaacaccgacaaccctatatttatcgcccttcttattatgaattctgacaattgccatatacgcatccgcactgccgctatatccaccatagacattgaccggtcgatcagcttttaccggaatcaattttcgtttgccggcatctgatgcaggataaacagtttgattgaacattgcgccgcgaagcgtataaacttcgtgtgaaatcagcatgaatttataatggtaaacatcctttaactgctgaattgaattttcgcggtcccatattacttcaccagtctcagcatcagcgatcttttcttgagtatcatcagttaaatcatggagaaaattaaaatttcgcatagtgactttatcttctctaaacttcttgaaatcaccatagacgaagtatggacgaagcttgatgtatcgatggtacaaatatctacctaaaaaggctgttaagtaggcgtcaaacgcatgatgatagtcattgatctcacgattcttgataaacccaaactcatctctcatctgatggttcatccgggcagtaatttcaataatcttggtatcatcattgcgatacttgtctcccaaaatgttcgcgaccagtttgataacttggctggtttcaaccaactgtcgacgaatgaatccatgcatcgcatacttactaatggtatcgggatctgtttgaaggttcttgagtttgcgcttactaatcaagcctgcttcagcaagctgtttccagaagtgccccatcttggcaccaaacattcttagaggaacgttatccgatttaccattgttaaccgccgttaaaactagtacacggttatccagtgaattatctttaataaatgcctgtggcaaaatatgatcaatgtcatatttattaagttcatcaatgttgattggctctccagtgtagatatccttcccaagttgcgtgaagtacaagtacaaccgatcagtcaggcccttcttagactttgctgcattgtccagttcagaaagtaactcgggattgattgatttagccaaagatttagcagtatcttttaaggtattttcaagttgccgttgtcgtgaaattgtccgacgtggattacggtcctctgaacgggtaaactcaatagaaatatacttaggcgcaactccgcccatggccttttggatatcatcaacgactttaaccacttggcggatggccttcttattttgtggagaagtgtacgcatctgccaacacatcttccacgtcgactgcctgcatttggtcagcattcgcttcgtgaatccgtttggcaaaatcatcatcagactgaatttgcatgaaatttttattggtattccaaagtttgtcaatgattcgttcgccttggtcattgacaattccagttaacagtttcttggaaagccggccccaaccttggtaacgactggattctaaaacatctttttgctgatcagataaccaggtaatttcgttaagcttttcccgcaggatttttttgtcctcaaatacagttgaccattcaacaatcttctcaaaatcatcttgaagatctggttcgtcaaccttactaccaaataatttcttgaaatcattgtatgttcccaaagaattgttgaaatgctcagggtctgataaacctgaaatctccggatcactgggtaatcctgttttggctttaatgtaattttgcagcttcttgaccgagacatgcttgtagttttcgaaaagatcttggaatatcgcttgtttatcagcaaccttcaataatttgccgttaacccggaccatgttcaactcattgaggactttaaacttctcatataataagctttcatctggaagaacatcctcaccaattaaataagtatctttggtggtcattcgcttgatgaatctgtttgcggatgccttccggtcaaccttttcatcaaaattccaaggggtaatctgcccagtttctgtacccttacgctccatccaagaaaaaacagtctctgctgattcagcctggtcttttggcgttatcattggcccaacataatatggaaccctaaaagcaaccaattgttcaatcttgtattttgcaaggtggagatcgtgcttattgggattgatctcgacaagccatgggtaatatttgctttgatgttcaatgatttcatcaagttctctttggtgcagttgatgaggaatcaccccattttgcgatgttcgttgctttggcataaatttttctgcatcgatcagatccataatttgctttgagagctcggaatcatccaaatttttcttcacgcttgaccagaactcggcttgttcgatgactttaccatcgtcacccacgtattgactatatgccttctttaagacggctttcttcttcggatcagcgagttgatcaattagctttttatacaacttcaagtggtcatgatgatcattgtacttttcgatcattgattctgataatgacatgccattaggaacaatttgattcaaagttacttgagaatataagttctgtaggatagcaacaattgattgttgattttcgtccatttcaggtaaaatcttttcaagtttggcatcaatgtcctcatcatcgaatttaagtgcccatggtttggaatcaactggggtgcactgtaggacaacatcaagttttgctttatagcctaaaatagcatgaataatttctgacgcgattttaccattaagtctgtccgttactttatcattcatcatgacaggaacaatctttggaatttgctttttcttgtcaaatttacgaattgatggatcgaggaactggtggccaatatcttcgctatttgcaagattaattttaaatgactcttcaggattaattgcggcatataactcgtttaactttttaaattggtcaacaaaatcaaccttcgatgccttaaaggaatctactggtgtagagtttaagaaattgccgcgatatttcacaatgtggtgaatggccaagtaaaccatccgaatatcaaattttttatcttgcgtcattaatgcatgacgtaaatgataaatggttggataatttttgtggtactgcatgtcggtcaaatccgggaaaagcatggaacccttgaattctttgcgtgaatcttttggtgacaaattggattgtttcaacctggcgaaaaacgtggaatcgacaggtgtaatatatgggtcaaatatttcctccaataacttcaatcgccacttccgtcgactcagacgccgtcgagtggttcgaaacatcctgcggtcggcagcggggttgccttcctgaaacaaccgggcgccaatcgctgtcttccctttaacacgcagcggttttccgtctttgccaattgcgacccaaccaattgatgaggtcccaatatcgagacctatatgataattattaactttcatgctcgtaaactccttggaatattgttgccctggaaatcgccttggcacatcatctattatgcattaaccggcaattatccgaaacccttttggcatagattggttgggaattttcgatccaattattcatcttgcatgcagttaaggtcttataaaaatatttaatgtagaataccgcatctttagaaccatcgatccccgccttaagcccacaaaaaactccttttgagtagacaagcgtcacctgctggtccactcaaaaggaattcattttatccatccatttcatcattacaccctcgtctaataaaatggatgtggcccttcgtttctgtgctcaaatattttgtttgcaagagcaattcggcttttttcaggcaacgttggtggagccagtaacaagactgggcacccatcatgttgggaaaatacttggtccttttcaacaccatcgattaagaattgaccatcgggcattcgataaacatcataaccaagttgagaagaattgtagccgatcgcatcactcatttcaacatttgacaggccttctgtattcgaagttagacccatcactaccccatagtcaaaatcaaagaggcgaaggcgggggtcatttgtcttgaaaattctagtttggagtttatgatgccctgactgtttatattttttcttaactcgcttaagcttatcagcgttcatttacgactgtcctcctgctattttacgtgcttttaccaagcaatttggttataggaaaataagtatctatagcatacaaccccaacggaaacgagacaatgcactttaatgaatgttaatcaatacacactttgtctgaggttgaaggagaaacgtcccaaccactggagtttagtaaccactaaagaggcattttcttctaaaattcacggcgttgtttccaccacaacaaagaatgcactcacagggatgtccctatttcacagcgaatggatccgccaaatgattctgagccttctcatcttgcacataggcgacttcccggtcaataattgcctgagaatttggatcagtatacacgtgcagcttataatcaatttctttcagattatctgccaacagccgttgctttgccaacacctcttggcgatgctttaacaacagccgtttgcggttatcaatcgaggcagctccctgcatacaataaccaatgtatttcttaatgtccttaatcttcatatcagtgttcttcaaacagcaaatggtgtgaataaaattcaagtcagaatcggtgaactcacgatatccggcctcgtttcgggaaacaaacggcagcagtccctgcttgtcgtaataccgcagcgtgtaaatggaaaggcctgtcttttcggcgacctctttaattgaataagtcatctcatcatcccttttaagtttaatgtcttgcactagagtatactctagcctttaggataaagatattaaattaatgaggagaatataaatgactaaaaaaatattggtaactggcgggaatggctttctgggcctccgaattatttcgcaattgttgactaaaggttatgacgtcagaaccacgctgcgttctctcgacaagcaatcactggtattggatacgttagccgccaacaacattgcaaatgtcaatcaactggattttgtacaagctgacctatctagagatgaaggctggcaggaagcgatgaacggcatcacagatgtcatgagcgtcgcatcccccgtattcttcggtaacaccaaagataaaaatgcggcgatgcgacctgcaatcgatggcatcacccgaatcatcggggctgcacaaaatgcaggggtagagcgacttgtcatgactgccaattttggcggcgttggtttcagcaatctggacaaaaatagtatcacggatgaaaatgactggaccaatccggatcaaaagggcctttccctatatgagaaatcaaaattactcgctgaaaaagaagcttggaagctggtgaatgagtctgacaattcaatggccctgacaaccatcaatccagtcgccattcttggaccggcaatgaacgggcatatatcagggagtttcggtattttggaaaacttgatgaatggcagcatgaaacgcattcccaatattccgctcaacattgttgacgtcagagacgttgccgatttgcacattcgcgccatggaaaatccaaatgccgccggagaacgttttatcgccaccgccgacggccagattacaatgccggaaatggcagcgattatccgacagcattacccccaactagaaaacaaagttgccgataaaattttacccaactggatggtgagggtcggttccctattcaaccaacaggcaaaagaaggccaactattactggacatgaaccggaatgtcagtaatcaaaaagctcgcaaactcttgggttggcagccaatcggcagtattgaggaaacgattctggccactcttcaaagcatggacaaatttggcctgctgaaatgagttcgtcatcaaaaaggcattaacctacgtgacaaaacgtcactgaggttaatgcctttagtcgaccatgatttaattatcaactcttccaagaataaacacatagccatatcgacttgccaaatcaccagattcaccacttggcatgacaatgttattgataatgtgaatgccgagtttgtatccggataaggaagcccgcttactgtcggtgtagccctccgcattcagcaatttcttaacaccggcaatcttggttgcattagacgcgttgtggttggtgtacagccacttttgaattgccgggaaagtcttgatgtcggtgtagccggttgtgctgatcggactcggatcaccatcaatatcgttatcaaagctgtcataattataggcagcgatctttgataaccccaaatccggctgagagttagggaataacttaataatttctctggcgagtttttgatttttcccggtttgaagatactgattaaaatctgtgttattcacgaaataacgcatattaacataattcattccggtatgatctggattcagcccaccggtgatcgcggattctgcaatgtaccccctggtactcttggtggtgccgtttaaagtcccggacaggtagacgtacttggtatcttttccattgtgccgcatgacaactgtatgggttttctggaacacagcaccaggataatccttcaggttcgcccgcttcttagtatgggtataattccatacgtaaacattttttgctttgtacgaatcctttacgtggaaataatcgtacttgttataccactttgtgctgataatttgatagccatatgggctaaatccgggtgtcaaagcatttgtccgaacatacccctgcatgtttccaagtcggttggcaacgtaataataagtcgcactcttcaatttgtgatagatgcggacctttttctcgacaaaccacgtggttgttttgtgattagcgagcttgtaaccttttttgtagaaagcattcgccttgatgttgttgtcaaattcctggttattccacactgacgccttggtcttggccttcgcgtgaaaggcaacatcttcagtatagttgctgtaattttgataagttttcagcgtcttcacccgataattatcgtgggctgcctgtgcgggctgtgggctggccaccacagcaaatacgacaaaagccagcatcacaccgacaagcttaacgatttttttcatgaatgaaaccccctctttcaataatagaatatcatgattaagttactgctgtgttaaataatgcattcattttcatgatggattcagattggtgtgttgacgaaaggtagacaatcatttaaaattataggtattctatcacgaaaggaaagattgctatgagttcacttgttaatcgcagttggcaaagccgataacaagtcacatcgacacagatgcgacttgatcttaagcatgcgatcatgaacgcatctgtgccggcaatctttcggaaaacgaacggtctggccagatgatttcggcaggccgacttatcacgagtatttcggtcagaccggaatgctcgttttttgttcgcataactaactgatggcgttacatatttattcaaattgagggagacagctattatgaagaaaaaatatttaatttcaggtgtcgtgttaatttttgtcgtaatcttgggcgtggcatttttccaagggcaacagaagcaaaagccccaggccaaaccaaccgtggggattctccagttgatgtcccatccagctttagatgccatccataaagggattatccacggtcttgaagaagagggctataaacctggtaagaacatcaaaattgactttcaaaatgcccaaaatgatcaaagtaatttgaagaccatgagcaccaagtttgccaacgaggacgccgatctttcaattgggatcgccaccccatctgctcaggcattggccaacaccattacccacaaaccggtcatcttgggggccatcactgatcctaaaggcgctggcttggttaagaacaacgaaaaacccggcggcaacatcaccggcgtttccgatcaggcacctttaaaagaacagctgaatttgatcaagcaattcatgccaaaaatgaaaaccttgggaattatctacacttccagtgatgactcggcagttgcccaatacaagatgtttgtcaaattatgcaaacaggaaaacgtccgtctcaaagcatactcaatcgccaacaccaacgatttgacccaggttgctgaacaagcggttcgttcagtggatgccatttatgtcccaactgacaacacgattgccggagccatgcagacactggttggcgctgccaataatgccaaagtcccggttttcccagctgttgatacgatggtcaagcaaggcggcgtggcaacttacggcatcgaccaatatcaattaggggttgcaaccggtaagatgagtgcccagattttgaagggtaaaaagaagccatcaaccactcccattaaattcttccgtcatggaaaactaattatcaatgaaaagcaggctaacaagttgggaatcaagattcctgccaacctcttaaaagaagcccaacaaaaaggagaattgatcaaatgagtattatcgtctcagccatcggccaaggattgacctggggaattgtcggtatcggcttattcctgacttttagaattctggatttccccgacatgaccgttgaaggaaccttcccaatgggcgcagctgcctgtgtcgccgccatttattcaggggcctcaccactagtcgcaactttgattgcctttgtggcaggcatgctggctggtttggtgactggttttctgtataccaaaggtaaaattccggtattacttgccggaattctggtgatgaccgctgcttactcagtcaacctgagaatcatgggcagagccaatttatcgctcttcgacaaacccaccatgttaaagaaccactttttggaatccttaccaccctattttgacagtgtcgttcttgggatcgtcgtggttgcgatcgtcacagcactcattgtttactttctccagaccaacctcggccaagcatttattgccaccggtgataatcccaacatggcccgctcacttggcatcagcacagatgcaatgcagattatgggcttgggtgtttctaacggtttaattggccttggtggcgccttggttgctcaaaataatggttttgccgacgtcaatatgggaatcggtgtcatcgtggttgccttggcttccatcattattggtgaagtcgtctttggcgatttgacgatgaaccaacggctgatcgcagtgaccatcgggagtatcttgtaccgatttgttattttgctggttctcaaactcggcttcaatgccaacgacttgaacctgatttcagctatcgtcttggcattattcatgatgttcccggttttggaaaaacgtttccgaatccgccatactttagcaaaggggatgaccaaacatgactgaaccaatcttcgaattaaatgacattgtggtcacggtcaaccacggcacacctgagcagattaacatcatggatcacgtgaatttatccgtcttccctggcgacttcattacgattctcggttccaacggggccggtaaatcgaccttgttcaacgtcattggcggcaatctccctgtgaccagcggccaaattctgctgaacggcaaggacatcacgagcatgtcggttgaaaagcggacccggttcttaagccgagtatttcaggatcccaaaatgggaactgcgccacggatgacggtggcagaaaatctgctgctgtctgagaaacgtggccagcgtcgcggctttgcaccgcggcatctcaagacacacatggataaattcaagcaaatcacctcagtgatgaataacggtttggaacatcggctgaacacggcaactggtaaactttccggtggccaacggcaggccttgagtttcttgatggccaccatcaagcgccccgacattctgttattggatgagcacaccgcagcccttgatccgcaaacttcgcaagaattgatgactgccacgaacgatcaaattacccgcaaccatttaacctgtttgatgatcacccaccatttggatgatgccctgaaatacggaaatcggttaattgtcttggataacggtcgaatcacttacgatatctccggtgacgagaaggataatctcaccaaggaagagttgctgagtttctttaatgatattgaagagtaacgcacgattgcttttataattaaaatgtcaacttggtcggtgcatgcgaatccgcatgtaccggccttttttcttgcttctatttttgagagaaagttcaaatcctttaaaatctgagcaaaatgagacctggcattcggtttatgagaaattttaaagcgctttctttgtatattctatatcttcctatttataatgagggcgtacaaagtgtctataatcatttgtgattgtgaattttctatataattttaacttatgtaaataattcgatttttcttcacagaatctttatagattttttgtaaactatagtcagtaaaggaaaaggaagtgaacattatgcaaaatcaacaatcaactccaaagaaacgtcgatttaagatgccttcagcctacaccatcttatttctgatcattatttttgttgctattttaacttggatcatccctgccggacagtacagcaccgacaaagccggcaatatcattgcccacacttacaaagcggtggcttctaatccgcagggaatctgggacgtcttctccgccccgatttatggaatggtcggaaatgatacgacggaaggcgcgatctccgtttcactgttcatcctggtgattgggggcttcttgggagtcgtcaatcaaactaaggcgcttgatgatggaattgcgactgttgtgtcaaaatacaaaggcaaggaaaaagttttgattcccctgctgatgattttgtttgcacttggtgggtcaacttacggcatggctgaagaaactattgccttttacccactgttaattccagtcatgattggggtcggcttcgattcactagtggccgttgcaattgtcctggttggttcgcaggtcggatgtttggcatccacggttaacccatttgcgaccggtgttgcctcacaaacgctgcacatttcacccggagatgggattatttcccgggcggtcctgtttgtcatcgtggtggcaatcagtatcctgtttgtttaccgatacgctgccaaaattgaaaaggatccttcaaggtcttacgtctttgaacagcgtgaggaagatttgaaacgatttgcgttgaaccatgaagaccaacccggcactaagatgaccggccgacaaaaagctgttctctggatgtttggtttgacattcctggttatgatcatgggcttgattccatgggaccagatcaacaagaactggaccttctttaccagtttcaccaaatgggttcaagatgtgccattcttaggtagtctggttggttccaacctggtaccatttggttcctggtacttcactgaaattacgaccctcttcttcttgatggcaatcgtggtgatgttcgtcttccatatgaaggaatccacatttatcgaatcattcttagccggaatgagtgacttcatgggtgtagcaattgttgttgctgttgcccgtggaattcaagttgtcatgaatgatggaaacatcaccgcaactgttctccactggggtgaaatgggcttgtccaacctcgggtcggttgtcttcatcatcttggcatacatcttctacatcccaatgtccttcttgattccatcaacgtcaggcctggcagccgctacgatgggtatcatcgggccaatgggtaagttcgccggtgttgacccaagcttggttgtaacagcttaccagagtgcatccggttgggttaacctgatcacaccaacgtcaggtgttgtgatgggagcattgacaattgcccacgtcaacatcaccacttggtggaaattcatgttcaaattgatggtttacttgttcttggcgactgcgattttcctgggggtaatggcactgttgtagagagcgcgacgaggcacgggagatgcggtttctaagggtactttgactgaaatccctggtcttgggattttagttaaagtgcacttagaagttagcatctgggccgtcggaacgcatttcaatcagagcgcgacgagacctgggtggccccggagtgtaagccagaaagtttgatgatggacgtttttggtccatcattaaactttttggcttacacagtaggggttagggccgtcggagcgcatttccactaggtaaaaagaaaaccacaaacacccatctacctcaaacaaaaaccactaacaacaaccaaaaaaccaaaaaattcaacttaggaggcaccaacaaaaatgtctgaaaaattagtcacagaaacagaacaaaacgaagctgttgaaggcttaaaacgcctggtcagcaaaccttcagtcaatgatccagccaccgtttccaaaacgacgccatttggtcaaggaatcgacgacgcattaaccgaagtcttaaagattgctgaagaaaatggcttcaagacgtttaaagatcctgaaggccattatggctatgctgaaattggttccggcgagaagatctttgggattattggccacatggacgtcgtcccggccggtgatccaaatgattgggattccgatccgtttaccgcaaccatcaaaggcggttacatttacggccgtggcacccaagacgacaagggcccttcgatggcagccatgttcgccgtcaaagccctagttgatcgtgggtacaagttcaactgccgcattcgatttatcttcggcaccgacgaagagaccctttggcgtgggattgctgtgtataaccaaaaggaatctccaatcgattttggaatcgcacccgatgccgaattcccactgatttacgctgaaaaggggctggagcagtcctacctggttggtcccgggatggatgatctgtcccttgatttggaaaatgcttttaacgccgttcctgccaaagccccttacaacgggccaaagctggatgaagtcaaggcatccctggacaaacacggcttcaaatacgaagaccatggcactgatggcatcaccgtcgttggtaaagcggttcatgctatgaacgcccctcaaggcaccaatgcagtcctgcggttggcaattgccttggacgacgtctttgacagccccgtactcgacttctttggcaagaaattccaagaggacgctaccggtaccaatttgcttggtgatgtcgaagatgaagcgtctggtcatttgaccatgaatatttcaagcctcaaaattgatcaaaaagaaactcgcatgcaagtcgacatgcggattcctgtaacagttgatcatgatgaattgattgaaaagctcaagaaggcggctgaaccatatgacctgcactacgaggcatttgactacgttgccccactgtatgtgccgaccgacagtgatttagtcaagacgttaatgtcaacctacaaggatttgaccggcgatgacacccaaccgcaaatttccggcggtgccacatttgcccgaactatgaacaactgcgtggcttatggtgccatgctgccaggaacccctgattttatgcatcaggtcaatgaaaattgggagcttaagagtatgtacaaggcaatggatatttacgctgaagcaattaaacgtctctgcacggattaacagtgatcttcgtgaaatataaaaagtgctcgggaaccaatcgttctcgagcatttttgtgtctctattaatctaagcgagcctatttgttttgagcagccgacttcaaagcggcatttttacgcatatccatttcaatttgttcaagcgtcttgccacgggtttctggcaccatgtagatgacgaagaagattgaaacaatggcaaagaaggtaaagacggcaaatgggccaccaacattgttgttaaacatgtgaagtaattccaagaagaattgtgaaacgatgaagtttccaatccagttggcagcggaaccgattgaagttccgacaccacggacattcaatgggaagatttcaccgatcatcaaccagcaaattgggccccatgaaaccgcgaaaccaaaaatataaattccaatcaggatcatggttggaacggcagcgtcttgaacttttaaagtgaagttcaagattgagagaattccaattgacaatgccatgacgattgaaccaaatagcagaatggttcttcggttgaatcgatccatgatattgtatgctaagatcgtgcagaggaagttgacaatcccgattccaacagaaatccaaatggcgttactttcagggaaaccaaagcctttaatgaagacttgcggcaggaaataaatcactgaattaattccaactaattgttgaagcagcatcagcaaaatcgcaacaatcacagccgggcgcgcaaaggtaaacagctctttgagaccgcccttgggttggttggcaacttcttgaatccctgccaattccttgtctggatcctcatcagtctttgcccggagttcatgaagaacgtcccgagcctcatcaatccgacccttttcaaccaaataacgaggtgattcggggagaatgattgaaccaacaaacagcatcaaagctggaatcaaagcggatccaagcatccaacgccaatcacgtaatcccagcagattgtgatgtaagaatcctaagttggaaacatatgctaacaggattcctaaagtaatcatcaactgaaacatcgtaccaagtgagccacggtgcggtgcatcagccaactctgccaaataggctggcgttaaagctgacgcagatccgacagcaaagcctaagatgattcgggcaatgaccatcgatacaaatccttgggcaaacattgacagtcctgatccaattaagaataggatcgaggctaaaaccaacaggcgctttcgaccaaaccggtccgaaagtgaaccaatcgacaacgcaccaacagatgaaccaatcaaaacagacgagacaatgaacccagtctgttcagttcctaaattaaaattgctttcaatcaatggtgaggcacctgaaataataccagtatcaaatccaaatagaaggccacctaatgcaccaaagaagaaaataaagaacgtacttaaatgacgtgctttcacgattatccctccttaggggatcatttctgaatcaatcaaatcttgtaatccctttcatttgaaacaaaaatacattaaaacagttcagtattcatactccccctttagatactcaatttgtactatcttttagtgtaaaaacgttgaggctaaaattcaagaaattacatttttgacttactaatattcagtcgataaccaatctgatttaaagccaatttgtaattcgttataatagttaggtaccgaaacactttgcttgtgttcaaaaaaattcagtgtatacttcttattgttaggtacctaagtataacaattcaaaggagaatgaatatggcagacattaataaaagagaactattaggcaagttcttcggcttccttcatggaacccaacgatttgcccgtcaccaagaacggccttaccatttgcggggccaaaacagagtcctggttatcctgtccaaggaaggcacactgattcaaagccagttggctgaaatcatggacatccgaccatcatcaatgactgaattgttgtccaagttggaagagcgcggcttgatcacccggactcctgacgagaacgacaaacgagttaccaacgtggccatcaccgacgaaggcaagaaagccatcgaagacgatgattccactgatgacatgctcgaccaaatttttgcggggctctctgatgaggaattggctcaattaaacgaactgttgagtaaattgaacacgtcactcaaagagaaactccctgaccacgacgacgaaccaggttggggacaccatttccctcaccgcggatttggcggcggccctcatggccatcacggctttggtggtccccacggcgatcctcgcggtcatggaccaatgggattcgcgccaagagattaagttgtttcatcacagaaaggctgccgatttggcagcctttttgcatacatataatactctaacttttcacacgctaactcttcacaaaattcgcaatcacatcctgtttcttactcatcttaatcttcgcctgagcggctgctaagcgagccactggtacccggtaaggtgagcaggaaacataggaaacattgatcgactcgaagaactcgattgatttgggatccccaccaacttctccgcaaacgccgattggcaggttgggtttggtaaaccggcctttctcaacagccatcttcattaattcaccgacgccgtctacatcaaccgtttggaacggatctgctttgagaagccccttctcaatgtattctggcatgaacgaacccacatcatcccgggagaagccataggtcagctgggttaaatcgttggtgccgaagctgaagaagtcggatacttcggcaactttatcggcagttaagcaggcccgcggaatttccatcatcgttccaaccgtgtatttcaacctggttccctgctcgttaaataagctttcgacctggttcacaacgatgtctcgaacccagctcatctcagccttggaaccagttagtggaatcataatgtgtggctgaatctccagtccttgggtgtgcagctccaaagcagccccgatgattgcccgtacctgcatctcatagatatctgggaaggtcacggccaatcgatcgccacgatggccgagcatcgggttgatttctttgagggcatccactcgacgaaccaggtattccgggtcaattcccaactgatcggaaacttgagcaatttctttggcgtcgtgcggtaaaaattcgtgcaaaggtgggtccaacaaacgaatcgtgaccgaacggccttccgataaacggaacaattcgtaaaagtctccctgctgcatctgcagtaactctgccaggggggcttttcgttcttcggcatcttctgcgatgatcaaccgtctcatttccagcagtcgctccggtttgaagaacatgtgctccgttcgagtcagaccaattccgtcggcaccgaatttcagggcttgggcaaaatcggcaggggtgtcggcgttggcatacacgcccaggtccccttcctgcttggaccaatccaaaattgtcgacaggtcgtcgttgacctttgaatcattggtctgaatctgcccgaaatataggttaccgttagtgccgtcaactgacagccagtctccttcgtgcagctcagttccggcaatggtggcgaccccgttttgatagtcaacctgaagatcattcaccccaaccgtcgctggggttcccatgcctcgagcgacaaccgccgcgtgggaagtcatcccaccacgggaagtgacaatcgcttcactgatgaccatcccttcaatgtcctctggtgacgtatcctgtcgaaccaggatgaccttctgttccaaatcatcgtgggcagctttggcagactcagcggtgaaatagatctggccggaagcagctcccggtgaggctggcagaccactggcagccggctggctttgctgcaaggcttcctcgtcaaattctgggtagagaatcgcgccaattgaatccggattaattctaagcaacgcttccgtccgagagatcaagccttcttcgactaaatcaaccgcaattttaactgccgcagtcggcgtacgtttgccgtttcgggcttgcagcatgtacagtgttccgtgttcaatggtaaattccaaatcctgcatgtcgcggtaatgaatttccagtttcttggcagtggccacaaactcgttgtaaagatcgggcattgtgtcggctaatgtactgatcggctggggtgttcgaatcccggcaacaacgtcttctccttgggcgtttaaaaggtactcaccgaataatttgttctccccggttgctggattacgagtaaatgcaaccccggtccccgagtcttcgccggcattgccgaaaaccatcatttgaacgttaacggcggttcccaaatcactggcaatatgattttcccagcgataaacctgagcgcgatgattgttccatgattcaaagaccgcattcactgcagcaagcaattgaactttgggatcctgcgggaactctttgccggcttcggctatgtagagttctttaaacttaccgacaattgtgtgcaaatctgccaccgtcaagtccaggtcggagtcataatgattggtgattttaatatcttcgagaatctggtcaaaaatgtcctcggggatttcgtacaccacgttgccaaacatcgctaagagacggcggtaactatcgtaggcaaatcgttcattatcggtaatcgcagctaaagttttaactgtctggtcattcaaaccaatattcaagatggtatccatcatcccaggcattgaaattgccgccccggaacgaacggaaaccagcaacggattatccgggctgttaaaacgtttccccactttagtgcttaattggtcgagtgcctgatcaatttgttcgagcgtgtcgtcattcaactgattaccattgtcatagaatgcctggcaggcttcggtactaatcgtaaatccactcggaaccgggaaccccagtgaggtcatttgtgccaaattagcccctttgcccccaagtaaacgacgcatatccttgttaccttcttcaaagcgataaatgtatttcatatcataacgtcctttctgaactaattagcatgttatattggatgcgtttatcatatatgatacgttttaataatgcaaattaaattttaaaaaacgttttattgaatgacgatgaaatgttggttttaaaagggttggcaagttgaaaaagaattttactgccaatccattttctgaaataagacgttttattggatacatatttgatcagatatgatagaattggactagtggtacggaccaacgactatcgaaagtgggagcgattaacttgaaactatccgaccggcaaaaccaaatcgtcgacattgttaaacagaaagaccccatcaccagccgccaaattgctgcagagttggggttgagtatgccgaccattcgatccgacctcagactcctgacggcattcaacattctggaagccaagcccaaagttggttacacctacaatgattctcaagccaagcctttaagctatcacaagctttatgcggaaccgatcgctaatattctgcagaaaccaactgagattcgtgaagatgccacattgaccgaggcggtcaacaccctgtttatcgaggatgtcggttccctttacgtgattggcgatcgtcaagaactggtcggcttaatttcccgcaaggatttgttacgggcaaccctgaataataccaacgcttcactgacacttgccagtacagttatgacgcgaatgcccaatattttcaccgttaccccagatatgtcggtcctccaaaccgggcagctcttattggatcgtaaagtcgattctctgccagtggtggataaggaccagccaaccaaagtcgtcggcaaaattactaaaaatcgaatctttcaacatttcattaccagtgttgactaatcatcccactcaaaagagctcaggcatttgcctttgctcttatttaattggtgcaaaatgccagaccccagttttgatttaagtctgttttaaggtcaataatgtataagtaaactagattatttttactaaggacggtgactgcaaaacagctatgttgaaaaagagaattgaatggattgatatcgccaaagcatacggtattatcgcggtggtgtttggccacgcgttagccagcggcacgaccaccaacattatttattggtggcacatgcccctgttcttcattgtcggcggattcttcttgaagccgattgacacaactaaattaactcattggaaaaagttctttaataaacgtatttaccgggatctcctgatctactttatcgcggggatcggcttgatcctgttgtatagcatcttgtatgacaaaaactgggattacttgattaaccacctctcgagactgttggtcgggggccggacattgaatctgtacacgtcaacgttctggtttgtgaacgtctacctgctgtcaattacggcggtgaccctgctgatttcgaccgttaaatccagaattggtcagctcacaattgtcgggttgggattatttgtctctacctgctatgacaaaatcgattggttgaacttgtacagttatcaaacaatgccctggaacttggatatcgtcttgattgcggcattctttacctacgtcggttatttgtttttccacacaaattggcactggattgaaaagccattgccgattggattactggttggtgcttccttggcaatcattggcttgtatcttaatcagaaattcagctttgaattttcgatgaaatctcatctgattcaatcatcagagccgaaaatcttgatgctggccaccatcccactgattttttcatttggtgtgatggggctatcggcacttaccagcaagctgtcgattggcttgttgctttcaaccattggtaagcacaccatgattattatgtatttacacggcgccctgctggacatcgcagaacaggctggtattgaaaacgtggccgtcaaagtggtgattgcgttggttatcccaatgctgctggcactgctcaagcagccggttgttcgaaggaatagtgtttatttacaaggataataaaagagagtgtgaaagaggacgtttagcaagcaaaatttaagcaccatcacccggaaaccgagtcaggttttcgggtgatggtgcttaaatcttgcttgctgtcctctttcacgcgtttaatccaaataacagtaaaacacccggaaaccgagtcaggttttcggctggtggtgcttaaatctcgcttgctgtccgctttcacacgtttaatcaaaataacagtggcactcaaaagaggctgagatgactaacaaattgttagatctcagcctcttctttatcggttctggaatcaacatcatgatcccatattcaattatttaaaatccaactctaaatactccgcgccatccaaggggttgaagcggtacgggtcgattggtttaaaaccggcggcgtgataaattttcaaagccccggtcattgatttcaaggtgtccaaacgaatcgcctgatagcccaaacgctcggcactggctaaaattctggcgaccagttcctgaccaatcccgagttttcggaagtcgtcacgaacgtaaagccgcttcatttcagcaatccccggttcaaattcatgaacagcgaccacaccagctaattggtcatttacataagctaagatgagatctcctttgggctggttataccgggtcgctaattcatttaattcatcattgaagtcttggaatcccaggtcaaacccgagtgacttggaatactcaagaaaaatctgcttagcggcgttaaagtcggccgccgtactggcatgcttatacttcagttgtgctggttgagcttgttccatgtaaccatccctcctgacaattaggagtagtgtacaaaatttgagttatttatgcaaatggcgttggtgaagcaagcgctgcttttcttcctcagcagctttatcggctaactgttgttcatgctcccgttcactggcagctttttgtggcaaaaccaaattgagaacaattccgataatcgtggcaaatgccaagccggtaaactggaacttaccgagttggagataagcattaccgacaccgataaccatgaccgtggacgcaatcatcaagttgcgcttcaggcccatatcaactttattttcaaccatcacttgaatcccggcagttgcgatcgttccaaacagcaggaagctaattcctccgatgaccggcatcggcatctgcataatcaaaacattcaatttgtttacgaaggcaaacagaatcgcaaacatggcggcacccatcagcacataaacactgtggatcttggtaatcgccataacaccaatgttttcaccataactggtcatggcaggtgcaccaactaaaccggcaaacagcgaagcagcaccatctccggctaacgtccggttcaaaccaggatccttgaagaagtcccggccggtcaattcatccaagaccataatgtggcccatatgctcggtcatcgtcacgaaggcaattggcgtgatcgctaagatggcagcccaatcaatgtgaaatttgtaatcaattccaggaatatcaaaggctggaattttgaaccatggggcactggcaatcgcatttaaatcaacgatgccacagaagactgagatgagatagccacaaacaattgctaacaaaactggaatcaggccgatgaagcctttgaataacatattaaaaataatagctaagaataaagttgccaaggcaatcataaagtacaacaggctgtacttgccatttttcatcatcgcatcttgagcggcgctaccagccaatgacagtccaataaccatcacgatcggccccaccacaatcggcggtaaaatatggtcgacccagtccgagccaaccgcccagataatggccgccacaatcatatacacaattccgacaccaatgaccccttgagcgattcccggatacccagtggtcttcataagtgccagcattggcgtgataaacgcaaaacttgatcccatgtatgcaggaattttacgttgggtaatcataatgtgtaacagtgtcccgacaccagatgcgaacaacgcgatgcttgggctcaatccaaccaatagtggaacaatgaccgttgacccaaacatggaaaacatgtgctgcaatgataatccaacccacgggaaaaatttgggcatgtcatggatgtcgagaattgcacgatcatcatgaaattcattcttgtctgccataaatatttgccaccctcaaaaagtatttgaatctttcaactccgcttcagggtggcccttttgacgaattgtggcagactctcacctggaaagccatgcagcaaaaaaggtgtccaccccgcgttaggcaaggcagacaccaagtcgagcaattgctcgttcaatatcgtcctcttaccagcctcacgggaccagagttaaagattcattcgttgtgataattataatataccgtggttgcttgtcaatctaatcttgcaactgcatttccatatcaatatggggaatgccgtcttccagatagacgtcactgacgttcttaaaaccaaacgatttgtaaaatccgttgaggtactcctgtccagctaagacaatttttccggtcttgggcatcaatgttggaattcgatcaagagcagtttgcaccaactcgcgtcccagaccaccgccgcgatgattggggtcaaccacaaccctgccaatccgggcaaccgtggcgttttcctcaggaataacccgcgcataggcggtgatgttgttttggtcgtccttaaacatcaaatgataagcggtcaaatcgtcatcatcgacttcttggtagtagcatttttgttcaaccacaaaaaccgccactcttaatttgtagatctgaaataattcttgagtggtcaattcaggaaatgttttaacttcatttctgtccatatttgccatcctttaaggtttaaaaatacaagtttttcgctatctgttataatatattcaactagatcaacatgcaataagagaatctaaatgaggtattaatttgaataggcatgacgatgaaccacaatataaaaagtatgacttcaattccgaagaaaatcgacgtcgacagcgtcgcaaacaatacagcggctggtggtttgctctgctgattttgattattgggattgtcttggcactttcaatcaattggtttgtgacatctggcaatcatcgacagggaagttcaaccaattcgatcagtaagaccatcaaaaaatccgagaaagaattgtcgggtaattccaagaagggatcgctgactacccaagttgagaagaatcgggtgaatgcattcagcagtaagctcaaggatgctcagcaaaatggactcaatccaaaagaacgtcagcaattccagcaaaccatcaacgaagagcagaaccaatccgtcaagtcccaggagcaaaacctcttgaacggcgtcaaaagtgataaaccggctaagccacagaaagctcctgaccaattctcaagcacccacacttttgcctctgttcaggatgccaagaactgggcaaatgccaccaagcagcaatggctgaaggctggttacgtcaactacacgattacctcgaacggacagggatactatgtcttacggtttatcaaatagttggattcatattattttattctacgattaaaagacatatcattgagatggaggagggatcaatatggatatacaagttcctttaacaaagggtctcttagcagataagtacagtaagtatgctgcaaaaaacgacatgcttgacggtgagccgatcgtttcatttccaattcaaatcagcaacgttccaaagggcgcgcaatcattagcactcactttattggactgggacgcggttccggttagcgggtttccatggattcactggattgctgccaatattgcccctgacgttactgaaatccctgaaaataacagtcagcaattaagggttccaatgattcaaggacgcaacagcactgccggcgggctaattggcaacaccaatcagacgactgcctggcactacaatggtcccaacccacccgacaaagttcacaactatcatttatcagtctttgcactagacacccagttgcccttgaaagacggcttctggttaaacgaattacaggacgccatgcgcggtcatatccttgaaactgccgaattcattgttccaagtaaaccgtaattttctgaaaatgattctgtatttcagtttttaagcgccattcgctggaataattagtgatataatgaacttaaattaatttgtgggaggtttcttcatggaatccaattataaaaccatcttagtgcctgtcgatggatccaatcaatcagaagatgcattggcgaaaggtgcacaatttgcaaaaaataatgatgcccatctcgatgttcttcacgttttgagcacacaacaatacggttataactatggtggaatggtcgacggggacgtcattaacaaccttgttgaagataccactgattatctgaacaaactggtcgatcggattaagaaggaatctggccttgatgatatttcaatccatattcgttttggtaatcctaagaccgttatttcaatggaattcccacgagaccacaaatctgatttaattattatcggtgctaccggtatgagtcgcctgcagcgagtccttgaaggatcagtttcttcatttgttgaccgcaacgccaagtgtgatgtcatggttattcggaccaataccgaaaacaaaccttatataccattccccaaagactaaacaaatgaaagcattcagcaatgaatgctttttttgttcttaaaaagaccctttcgttgacgttgccggtcaacacggtatgattaaattaacgaatgtaagcgctgtacttcgagaggagaatcaactatgaaagttcttgtaattggcggaattgccggcggaccctcgtttgcaacccgacttcgacgaatcaatgaggatgctgaaattatcatctttgaacgtggcgcggcaatctcggttgccagttgtgccctgccctattacctgggaggcttaattaaggaccgctcggcagtcattgaacggacgccggagatattaaagcagaagaataacattgacgtacggttatttaatgaagtcacccagattaatcccgatgacaaaacggtggcagttaataatctgcaaaccggtgacacctataccgaggattacgacaagttagtcatcgcaaccggcgccagtcccacggttccagaaatttccggaatccatgatgccaacaatgctttcgtattaagagcggtcacagatgcagataagatcaaatcatttattgatgaaaaacatcccaagacggtaactgtcctgggagccggttcaattggcattgaagtctcggaagcctttgttgacaatcaaatggacgtcacgattgttgaacaaaccggccacgttgccgcaccatttgatcctgagattaccgatatcgttgccgacgaactcaagaagcaaggggtccacgttattcttaatgaaagtgtcaaagagattcaggatcatgggcataccttaatcttagacgatggctcagtccatcaaaccgatatgttatttttaggtaccggagttaaaccgaatagtgagatcgccggtgcagcaggaatttcactttctgatgatcaccatattatcgtcgataatcatctgcaaacaaacattccagacatttatgcaattggtgacgtgattgaaacgaccagtttaatcactggcaagccaattccaagcctgctctcaagcgctgctaatcgccaaggtcacttgctggctgacatgctaaacggcagtccgttggaatataaaggattcattagcgcaggtgtttccaaattcttcgacttgacagccagtttcgtcggttttaccgagcaaacgcttcaacaaatggggattactaactatcgaaccgtgttcatcacaccatttgatcgagcttatttctacccgaatgccgatcgagtcaacttcaaattgatttatgaagataagaccggtaaaattctcggcggccaagcagttggccgaaacggaattgataaacggatcgcagaattgtcggtcgcaattaccggtaacttgaccgcgtttgaccttccatctctggaaattccctattcgccaccttattcttcaacccgtgatgtactgaatatcgcaggttatgtggccattaaccagttaaccaatcaatcagccacgatcaagattaacgatattcctgacgatgatcttaaaaacgccgtgttcctggacatcagagaagctggaaaaccagtaactggatcgatcaaaccaactttgaatattccactttcagaactccgagagcggattgacgaggttcctaaggataaaaaagtttacattaccttccgaaaaggtctcggtccatacaacgcaacccgtgtcttagctggaaaaggcattaatgcaactatgatcgaagaataatgaatcaataaaaggggattttttggacaaaatgttcatttagccccctttttctggagcatcaacgtataatatatgtagatgggagtgtgatgacatgccacgcaaactaagaccaaatgcagccgtcaaaaaagtcttgaagatttatcaacaaaactttatgaggaaccaatttacggcacctcaaaacgatgcgctgcatttaatatttaacttaggatatacagttagtccggacgtcaacgaaagttcatacggctatgtcaaagttgtcaatatggacacggggaaatcgctcgtcttgactaacctcagcggtaacaaggcgctattagatggtggaaccaccattatttctgaaccggatcttgacctggacacatttgattatgttgattatttgaattcgaaaggtgacaatccggattatctggcaccaaccgtcgcaaatctgaaaatgctgcggaatcggttgaatcaattgaatgcggattttgatcgcttgaaaaaattgcgaaatgattatcaagaacatctgaccagtattgactcagaatacaataagaaagttagttctttcattactatcgtcaatcaagttgaacgaatgtccaacaagataactgaagaagatggcaaaagtaacgattcatccaagtaaaagtgggaattttcccgctttttttattttatcacaatggttatttatttggtacatattttatttaaagagggattattatatttattttactccaagctaatcagattgttattatttttacccctaattttcatattcgctctataaacttaccctgttgcataattgtttgcaaacatattttttggagggaattatttcatgaaaatctcaagaatcgcattggcatcactcatttcatttggtgtattaggaggagccagtctcaatgcttcagcaaatcacacccattatcaacgaatcctttggaacaagaccatggcacatcaaaaagtcgctttgaagaatggtaagggtattatttggaacaaaccatacaagactgctaaaaattccaaaattacttatcgtttggcacacaagaaaggtcttgtgatgaccactcttcgccatatgaaggttaagaacgggagcatttactactttgttaaggctggtaagattagtggctggattaacaaaaagagcgtgaagttaattaaaaatagtgccggaaccaaaacgacaattgctccgaattctgcgccaattcagagcaacggcaccccagttccgaataccccctctaatacattaaatacgacaacttcaaatattcctgcaaagaattcacaaaacagttcctcaagtaatgttccaaacagctccactacgcagccaacatcgtcaaatagcaaaacatccgattcaattaacccaattactgccaccactaaagtgaactcgtttatctattcagataattgggatggggacaatcctgatagcaataaaacaaacaaatcactgggactccttccgcgtggagaaaaagtggaaattatcagaacagataagacaaaaaatggtacagccctgttagtccgatctaaggatggtgtttatggctatatgaatcaaaacgaattaaattttgattccaaagacattccatcatatgtcttgaattacaattcggcaaataatgtcacatcagttccaaatgtttctgacaaatctgtcagcaaatcagattccaaggagacgggaaatgtcgatcattctactgaagcaaccgtaaatcaaaataatttgtttctttataagaatagttgggatcacggcaaaacgcctacagataatgctacaaaaggactgatcgcaaatggcacaaaagtctatgtcctcaataacgataaatcccgtgactcagtcctcgtcataactaacgccggggaaacaggatacattaacagagaatccctgacgtttaacaaataattccacagcccattacgttaaaaaagacaaaacaaagaaattaattgctttgtctttgtttcaatggcccagtccacattactatgtcacttcctaaatccgtcaaattcccccaaccccctgttatgacaactaccactcgccactgcaagctttcattcatttgcaatcatttttatctttggtaaactagttgtcatcgttaacaggaggtatacatggattcaaaaaacacaacaaagattggactttttcaacttgtaatgctgacactgggatcactaatcggttctggctggcttttcggttcttgggaagctaccaaaatcgccggtccggccgcaatcatttcctgggttattggaggaattgtgattgctgcgatcgcatataactacgtcgaaattggcgcaatgtttcccgaagctggcggaatgagtcggtacgcccaatattctcacggcccgctgctaggattcattgcttcatgggcaaattggatttccctaatcactttgattcccattgaagcagttgctgctgttcagtacatgagttcctggccttgggcttgggcgaactggacgcattctttcttaaaggatggcacgattaccacctcaggcttgatggtcgtattcatgttcattctagtgttcacactgttaaatttctggtcagtaaaactattgaccagtttcaccagtttaatttcaattttgaaaattggggtccctgccctcacaattatcatgctgacaatctcaggattctacccacaaaattatggccattctattcacgaatttatgccatacggctcggcgccgattttcgctgccacctcagccgccggaattattttttctttcaacgcattccaaacggttatcaacatgggaagcgaaattaaaaagtcccggaaaaatattggtcgtggaattttcatttcactgctaattagtggtgtgatctatattttgctccaaagcacttacattactgccataaagccctcaaccctggccgcaaccggttggagtgggtttgacttcaactcaccatttgctgacttagcaatcatgcttggcatccgctggttatctgttctactctacatggatgctttcgtctcacccgttggcaccggcgtttcctttgccgcgtcaaccgggcgtgcgctttatgcaatggaaagcaaccaacatatcccaagcttcattggtaaaatcaaccaaaagtatggcatcccacgagtagccatgatcgtcaacttggtattaagcatgttgatggtctcggtgtttagatcttggtccacattggcaaccgtcatttcgacttcgaccctgatcgcttatctgactgggccggtgacagccgttgcctttcgtaaattggcccctaattttaaacgtccggttaaattgaagaacctcggttggatggcaccattgtcctttgttctggcctctctggccatctactgggcaatgtggccaacgaccgtcgaagtcatcctggtcattttggttgggctgccgttttacttctattacgaataccgggccggttatgtcgacaccaggaaagctttctactcaagcatgtggatgattatctatctgatattcatctctgttatgtcttacattggtagtgaacagttcaacggaattaattggattcactacccttgggactttgttgtcatcgccctagcctcactcgtgttctattattggggcatcaaaacggcgcacgtcttcccagacttttaccaagccaaggaactcaacgacaccgtcaaattggatgacgattaaaatcttatccatcataaaaaagccgacaactgcatgaactgcagctgccggctttttgagcatcaagtgcccctgccaaggtaattccatcataccccaaatcatatcgattggcgaaattaattcaaaaactgccaaaccgttttggcaaaaaagataactagcacaataataatgatcggtctggcaatcgcactgccatactttttgtaatatgaagctcccaggaaattacccaaaatactaaaagccccggcggtaagccctaaccaaaccaacaccttaccattcatgaaaaagactgctaaggcacaaacatttgtcgtcaggttgatcaccttggtgttaccagcagccaggttgattggcaagtgggcaatgccgaccaacgtcaaaatcaaaaaggttccggtccccggaccgtaaaaaccatcccagacaccaagggatatggaaatcagaatcgttgcgacaaactgtgaccaggtcaatggcttgaactcagccagtcgcgagttcagcgagtgtcgattcaataatagatacaacgccgttatcggcaaaacaaacaataaaatcagccgaaaataataatcagaaatatgtaaagccatgttggccccaaacgaagaacccaccatcgcagctaacacagagaagaaagccagtttgacgcggatatacccgctccgcataaattccaaggtagcgactgtcgtccccatggctgatgataacttgttggttccaaccgcaaaatgagccggaatcccaaccatcagataagctggtaatgaaatcagaccgccgccaccaccaatcgcgtccacaaagccagccagaaaaaccaacggacaaacaactaaaaattcgctgagcatcccctcatctcttttcttataatgattcccagtttactgctaaatgactgattagaaaacgccaaatccaagtaagatgctgaaagctataagcaataaattaatttaaatttacatgcttggaatgattccgattgtggtataaatatatatgagggggatacatatcatgaagaaaatgaaatggttattactggcatttgccagctgtgcatgcttgttactattgactgaaaatccacgggttgacgcggccgggtcgattccacattggtacttgggaaactggcaggccgttaacggtaaagatgtttacgtcggcattcgtcgaaatgaggtcatgctccaagtcaaaaacgacggtgtttactggaagcccgtcacttggaagaaagacacccaagaatccggcgtcgtttttggcaccggaatgggcgctaaaaattcgaagacctattttgtattagtcaaagaaaagatccaaaagaaatggtatatgattatgaccatgaaacaaagtaaaatcaaaccgagtgatctgaggaagcacccgatgatcatgaaacgttattagacacaaaagtcacccatgtgagttcttgccaggagctgaagttcatccttcaaccttggaaaccccacagaggtgactttttctatatatctcgatttttctgccaataatcattaaccgataaatatgtccgtgaatcgcccagcgactccgctacggccataatccgcggtggtagcaatcccactcgctggacaagttcgtgatcgctgaacaaatcccgtggactgccggcgaagccaaacttcccgtgctccatgacatacaccgactcaaactcggcggcgacccaatccatgtcatgggtgatggtcacaacttggtggcccgaatcagccaactgatggaaaattgcggtcaacttgcgccggctttcccagtcaagcgacatcatcggctcatcaaataaatagatcgccggatccactgccaaaactgtcgcaacgctcaacagcttgcgttcagacaacgacagatcatatggattttcagctgttttatcatccaagccaactcttttcagagcttctaaagcccgcctcgtaatcgtgtcgtggtcatccatgacctgcgcgacactccactccacctcttgttgaaccgtcgggttgaaaagctgatcgtcaggattctgaaaagtaatcccaaccttcagtaatttttcgactggtttaagatcgttaaaatcttctccatcaatcttaatcacaccggtttgtggcgtcagcaatcccgtcaataacttgaagagcgttgatttgccggcaccattttgaccgacaattgccaccatcggatcagcgaagtgttcgtcttcaacatccaagctaaaggaccgttccggataggtgaacgtcaggtgattcagttcaattgtggacatatcgggcctcctttagctcagcgtcattcaccggatatcggccatcagccaagtgccaatccattttttgagcaagctgctgaattgtcggggctggaatctgccagtcagctgccaaatgattaaacacctcacctggcctgccttgggccaccatttgaccctcgttcaatacccacacgacgtcgccgacttcgcacaggtcgtcaatttcactggtgacaatgaagacattcgtctctttgacttgggccagccattggaaaaattgccggcggccaaggggatccatctcactggtcggatcatccataatcaaaacagccggattagcagcaatcgccgtggcaatcgccaaccgctggatctgaccgccagaaaggctctcgggacgcaaattcagctgttcaatcagccccatttgcgtggcaacttctacaacccgtttttgaatcagcccttcagccatcccctgattaatcaagtcaaaggcgatttcatcggcaaccgtatctgccaacccgcttagttgaccagccggattttgcagcacaactccagtcatggcattataggcgcgccaaccgtcggacacccgccggcctaacatgtgccagtcgccttcaatctcagcagaaacaatctttgggatcacgcctgccagcacacggcacaaagtcgatttgccggagtggctgttcccaataatcccaaccacctggccggtgtgaacctccgcgttaatctgacgcagttgtggttgctccgtacccggataacgggtggtcaaattttcaattacaatccgtttatcttcgaccatatcttccacccaatcaataaaattgccaatccagtcagaccaatgtgcagcgtccgtgacaggcgatacacgcgctgggaggttctgacagtccggttgggattatcaaaacctctaagttggagagaaatcgaccgcgccatcgattgatccaaggtcttaatcaccaatggaatcagaaccggcaggactgactttagtttctgaatcaacgttttttgcggattggttccgcgaactttttgagcctgctggattttccgcatattgcgcatcatttccggcaaaatataacacaccgacatcaaaacgtagacagttttataagacaatccagacagctccaaataggctgcgttttctgaaatactcgtggtcaccatgaaaaagccactggtcaaaataatcaccagtactcgacagccgagagtggtggcgtagatcaggccttctttgtagaacgacaccccgagcacagaaaacagcaccgtttgattccgactgtaaaacaacccttggatgatcagcatggtaccaatcaaaaacaggctgaatcccagtgccttaaaggtggtcgaactcaatttggaaaataacaatagcagtgtggcgacaagaatcagtccggcctgaagcaataaattcgtactggcaaagctcagcaacgtcatgtccaagatcaacaagagcttagtaatcggatcgatcacctggtaccacttgagcttgacccgtggtgctccagaaatcaatgtttgatcagtcatcatttatcatccctaaagaagtgcaccatccgctgcggcagctgacgatatataaagaatgccaggtaagccacacagactttatccaaaatatccaagacaaactcatcggtaaacgaggccagccaaactggtgcatgattggcgaccattaccgcaaacaatgagtcaccccaggcgatcccggtctgaccaccccaaaagatgacattgagtggcgttgaaatgacagctgaaacgatggcaataataatagcagaaataaatacccgtcgtgctgacgagaaccacccattggcgtgcaggatgccgacagcaatcccaattccgatgctggtaatcgcgtacacggttgaaattggcgataaggtcagcccgtagatcacgttgttgatgaaaccactgatggcaccggcaaccggcccagccaacatgctggcaagaaaagttcccaaggaccccagccaaacgggcagctttaacccctcagccaatgctttggcaacatagttaattcccacggcagcgggaatcaaagtcatggtggcagcacttaacttaaatttccacatactggtacgatgaatcggttctgttttcataatcttctcctttgattttgattgtcataaaagtatcttctacttttaagtaaaagtaaaagatacttttaattcgacttggcacttattgtacaagtttcagctcaaatgtcaagaaagcgcctactcattttctgaccaagttgtgctcaaaccggttaagaaacctataaactatcgactgattggcccatggacatttcaatatgcccataataaaattattaacgatcatcagggggaaattatgctacatcgtcatcgcaaattattgataactattagtctgttagccgtgatcgcaattgtcggggtgatttttatcaaagccacccttagtccggataaaacgccgaccgccgtcactgctgttaaggaagaagtcttccctaatcagatttttgaatcgtacaaatatccttatgacctgcggattatccactcaaacaccaaactatactcgacgccagccggtactaaaggatcaaaatatctgggaaccgtcaaatccaatcatctgactcgcaaaattgttggtcaagaacgggctgatctgaatcaccggcgctctgaaggttacatttctttcgcccaaaatggacatacttactgggtgagcgcacaaagcgtggtgtttcgggacctcaacaaactcaaaggcgacgaccccaaaattgaggcggcgatcgatgccggactcaaacttgtcggcaaatccaaatacgattacggtggcggtcgcaatttgagtgacatcaaaaatcgcaagttcgattgttcatcatttgtccggtactgcttcagtaaggctggcgtcacccttggcaatctggatagcgtcacgacgtacaccctggtcacaatggggcgtccggttaaatttcaaaatatgaaacgtggtgatctgttcttcttcaccaattcacgtggtcaggtcaactcgcacgttgccatttaccttggagaccacttattcttacacgaccacgggcaatcagatactggtggcgtggggatttcaaccttgaacgccccgggttggcggaatgaagccaatgggaccgttcggcggattgaatgagaaattaagggcgcctggcaaaatttgattttttgctcaggcgccctttttggtttctggagattacccttgccgaatcgtgggaaaatacgcagcttccggccatataaggggggagtagccaagcatccaagacctggatattaccttgccgaatcgtggaaaaatcagcaacttccggccatataagggggatttgccaagcatccaaaacctggatgcttgactaatcccccttatattctggaagctaagcgctgatttttccacactaaaatgctttatccacttccgcaatatcccttcgcaacccattcacctggcgatctcggtcatcatagaagtaccacacggcactcagtaaaaagaccaggacaccggcaatgatcaattccagtgagaaactgaaaatcaaataagcggtgaccaacaaggcgataatcggaatcaagttgccacctcgcagtcggaatccctggggtagcttgttgtggttgcgcaatttaatcgccgcaaaaatcgttgggacatactgcacaaatgacgtaaacacgatagccgaggctaagaacaaataatttcctgaaaataacatcagtgcacaaagcccgcaggacagcaacaaggacacgattggcacaccgcgtttattctgcctgcccaacattcgcggcagcaattggtgttccgacgccagtgaactggcaatcgtcggcgtcgaaaatgagaccgacaaggcaacacccagaattgaaatcagcattccgaccaatgccaaatcatacccaactgttccggccagacggtaaaatgatgcggcaatcggcacgttgtcgttggctaagctactgcccgagaccccgattgccgtcaactggacaatcatatacaaagttgccgacgtcaacagcacactgatcagcgctttaggaagtgttttttcgggatgattcatcttggaagcggcaatcggcaaaaacgaaaaaccagtgaacatataaaagaccattccaaagccggtattaattcgaccgaataatgatgacccgtttgacatgccggcactcatattggcgtaatttgccggatgaataaagaacagccccatcccgacgaataagaccaaaacaccaatcttggcgaccgtcgagatattatcgacccaatccatcaaactgggaccaaacaagttaagaatcgtcaagactgccaaaattcccagtgccgccatcagatagttgccatgctgattgaggctgggaaacacactccgcaggctggtcacaaatgccgatatttcagtggccatggtaataacacccaacaaccaagtaaaaatgccaatttcaaatcctgcaaaccgaccgaaagcagtgtaggtgtacaaccaagcaccaccatccccaggaattttgctggccaggttggcgaaacacagcgcaatcatgagcactgagatgcctgccagcatcatcaatccggcacttaagtcaccaactttggcgtagacccggctgggcatcaaaaagatccctgagccgacaattccgtcaacacccagtaaaaagacgctcaaaaaacttagtggtttaatccttgaacgtgccatgtgacggcctccccttctaagcagactccttagcagctgccggttttctgcgcgatccgaggtaacgaaccaaaacgatcactaatgccaccgcggaaatgacggttgctgtccaaaagacgttggcaaatgcatgaataaacggcagaccgacactggccgtgactcgtttaacccctggcagctggaagaacagcaaggatgacccaaagctgatcccaattgtcatgcccaaggttcgggcaaacgaattcaatgatccggcaatcccggagagtgatttgtcaaccaatcccatcgttaaagcgttgttgggcgacaggaagatggccatgccaatcccgtttaagataattggtggaataatcttccacatatccaggttattcgggaagaatgcgtaaccgacttgagaaatcatcaaaatcaacaacccgacaacggtcattaactcccggttgatccggtcagcaagatagccggcaaatggcgtcgtgcaaagcatcgtcactgactgcagcatgataatcagcccgctgtaaaaggcgctcatgccgttataactttgaaaataaaatggcagtaaaatgtttgaaactgaattaaccagcataaccagcgccaacgctgtaatcgacgtcatgaagccacggttatgaatgacttccggcgcaatccacggcaggttggccttatcatcttgaataaacgcatacagtgcaataaccccgccaacggcgaagaagataatccccgtcaatagtttggaacggccggcttgaaagaatgaaccgctcaagaagaagataatgattccaagggtaaataaattctgcccggtccagttggcgccctgggtgacctggcggacgtgggcccaagattctttgggaatcggcaaaaacttgaacccaagccatagaatgacaatccccaaaggaacgttaatccaatagatccaccgccagctggaagctgaaataatcaggccgccaatgccgggcccggagattgaaccaaccgaaatgaacatcgaaatgacggccagagcttctgcccgccgtttatcaggaaaatactgagtgacaatccccattgagttggccataatcatcgccgatccaatcgcttgaatcacccggccaaataaaataatcggaaagttcggcgcaaagccggtaatcgccgacccgatcaagaagccaatccccccagctaaaaagaccacattttttgataagatgtcgccgatgtggccaaacatcaccaacagaatggctgtcgtaatcaaaccgatttgaacgatccacgtcgccatactactggaaatgtccatgtcaatcgcaattttagggatcgccaggttcgtactggagccggacaaggccgttagaaatgagaacatccccaacactgcaataattgaataattttttcccctacttgtcgcgttatcagccataatacccctcctctagctttcagtatcatttataacactatgcaggagaaattttggctctgacgacttttttgttgaggatgggagagttcgaaaaaattgcaaaaaatggtgctatccgttatattagttgtgggtgtaaacagaatatactttagggggaatatttatttttctgaatagtaatagtattatcaaaattgttgctaccagtgtaataacactaggcggatggttagcgctgtctcaacagccatcgtttgctaaatccaatgaaatcatcaataatgtttcgctttcttcaattgatccaaataaccgaaatgttgtgttgaccggcgatcacaaagtgtacaacaaagctgcaagtctcaaaggggccaaacagcttacctcaagttctcaattaaaaaaactggctggctccgtccgctcaaaggatacctttagagtctatcgaatggctgctaccaggaaccatcgggtttactacaaggttgtttcttttgaaggaaaatatcgtggttggatttatgggggaaaagcaaagagagattacgcgggtggccttgaacgcgttaatacaacttcagaagtgactttatcagatcagattcgtcaaactacgtatcatttaaagagttccggaacttccagtgatgaaaacgtttggaatgacattccttggactcagtacaaagcaagtctcaagactaaggattccacaccatatgccaaggatgatttgaccgtcatctcggctaaaaagatgacccgccaatactatcaaacttactactacatcgaagatgcccagcacccagaatttaacggctggattaacagcaactccttggagggcccagcaacaacggtcaccaaaacagtcagcgtcccaggcccaacacaaacggtgaccgttcctggtgcaagcactactgtaaccgtcccagccaagaattcgttgacgatcaactacgttacaaatcgttatgatccatccgcgaaaacacctgcagtgactgaaggtaatggacaggattggccagaagaacctcaaatttcaaagtccgttcaaaaggcttaccaagaaaaattcaaatctgcattagcagaaattcagaacaaatcagaaataactcaagcagacttggatgcattgggcaatggaaaagtattttggcatgaggacgatgcttggggagactgggacgtcagtattcgggtcagttacgacaagctaaagaatgttgtaacaattaatctcgtttgggaagatgttcagaccacatgggataaagccgttaattactatttgcatatcggtgacaagttcactccatgggacttaatccacgacttcgtttacgaaggatattttgtcgatacccaaaattacgccaaattctttactgtgaccgaaaacaccgtcgataccagcaaagctggcaactatgtggtcaaatactacatgaaggattatccaaataacatcatcacggttccggtcactgttcaaagtaattaataagtactgtatcaccctcacctcaccacgaccactgtgaatcagttatactgatactaacagcagtcattcggaggtgaacccatgctcacaacgattatgaccagcatcctctcatttattggaaccaacatcgacgatacctttgtcctggcagtctggttttcacaagttgatgcttctttgaggcgccgagatatcgttatcggccaattcattggatttgaaattttggtgctggtcagcgtgttggcggcatatgggctcagttttctgccaacagaacaagtcggctggctcggagtggtcccaattgttttagggatccgcaaatggcttcagtatcgacatcaattgatcgaaactcatgagacagctcacgttaaaaccaagctcaaccaagagctgaaagttgaacggcacaaatctgggttgcgaaaactattcaagccagagatattagccgtttcattaataacaatctccaacggtgccggcaacctaaccgtctatattcccctcttcacggaatatacagtggccgagttgggaatcaccgttttggtcttctcgctcatgacaggcctttggtgttatatcggctatcaaatcgccaacctgccgatcatcaaggataagttggagcgctcaaaacaaatcctcattccgattattttcgttgcgattggggtttatgtgctcatagaaagtggtgtccttgggtaaaacggatcctaagtgactaattaaaaatgggccttcatccgaatttcaaaattcaggtgaaggcccatttcttataaaatttaatgatttagctgatgtcaatcatctgcgggtaccatcaaacttcggtcccaactttcggttcagcttgataattcaaaatcacgtccataaactgctcaccgtatttttccagcttgctctcaccaacacccttaacatccagcatctgtgagtcagtcgtcggcatcacggcactcatttcatgaagcgtcttatcagagaagatgacaaatggtggtacaccctgcttctcagccaattcacggcggagttgtctcaaggattcaaataaatcatcattttcggcaacacttttagtggccttaaccgagatctttcgagtgaccttcgtctcaccttggagcacggcggcacctttggcagtcacctttaacacggggaattggccaccggacgccattaggtaacctccagctgtcaggtaatcgattaatgaaaccacatttttctgtgagtcacccttcataatgccgtatgtggagagctgattgaaatgaaaagctttcaccttttgcactttggagccagtcagtacttgagccaccaaacttttgccgaaccgttccttcatccgcagaacacacgataaaaccttctgggtgtccacggtaatatcttgggattcgcgggtatccagacagttgctgcagcgaccacagggttggccgtccttctcaccaaaataattcaaaataaactgctgcagacattgctgagtattggcatactgagtcataatctgaagctttttgtaggcttgatgcttactttgctcgtcacgttcagactgatcaatgaagaagtgctgagtctgaacgtcttttaatttgaacagtaaaatcgcttcactgggcaatccgtctcgaccagcccgaccagcttcctggtaatattcttccaaactaccaggaaccgaatcatgaattacgaaacgaacgttgcttttgtcaatccccattccaaaggcattggtagcgaccatcaccaaggcgcggtcataaagaaaatcgtcctgattttttcggcgttgctccttggtcatgccgccgtgatacatggtcaccgagaatttgtgcttggacaaaagcttcgtgacccgctcaacttcttttctggtgctggcatagatgatgccggattcagcggcgtttaatttcaaataatccagcatatatttgtcgctgtcttggttctgaatcactttaaaagccaaattatcccgggcaaaaccggtcttgacttcttcttttatatgcagacgctgcttaatgtcgtcggcaacttgcggtgttgcagtggctgtcagcgcaacgatcgtcggcttagtcggcaagtcatgaagccgttcggtcaatgccaaataacttggccgaaagtcgtgcccccattgagaaatacagtgggcttcatcaaccgctaccagatcaatcggcaggctggccaaacggttaaacgccccggaatccaagcgttcaggagaaacatacagcagcttaacctcaccgtctcgggcctgctgaaagcgctcgtcaatttcgtcaaaatccaggctactgttgatgaacgtggcgggaatgcccgtttcgttcagggcgtctacttggtccttcatcaaagcaatcagcggcgaaaccacgagggtcaggccatcttctaacattgccggaatctgataacacagcgatttcccgccgccggtcggcatgatggtcaacacgttttgatgggccaaaatatcgtcaatgacggtctgctgtccaggacgaaagctgtcatagccaaatttagtttttaatagtttttcgggcgtcaacctgttcagtcctcttttcgaattagtcacatactatagtatacgaaaaaatcagccccatgtcttcaaccatcccaggatcaaagtcgacaaccggcgacaaaatccatgagagaagcgtttgcttatgctattctaaaaaaggaatactaatagaagtgggtgatgattatgcagcaaatttccacaaaaactttaaatatgaatgtccaaaaagatttgaattttacctggtcaacgcaagcaatccttttctgtgccatcatcattgcctgtatcggcctcaacgttgattccgcgcccgtcgtcatcggagcgatgctgatctcgccattaatggcgccaattgtcgggatcggctacggcttgggaaatagtaatccaaagctattatcaaaagcggcaagactctttttgattcaggtgacaattgggatcatcggtgcaaccatttactttttcatttcgccattaaataccgccagcgcccaactacttgcccgaaccgaacccactctctgggatgtattaattgccttttttggtgggtttgccggcgtcatcagttccgcgaaaaaagatggtggcaacgtcgtccccggggttgccattgccacggccttgatgccgccgctatgtacggttgggtatgggattagtcatctcaacgcttcatttattttgggcgcgggctacttatttttgattaacgcctttttcatcgccttggcaacggcagccgggaccatcttttttcgcgtccgtagcggtgaacggctgaatgtatcattgcgccaacaagttctgatcgtcatcatttcgattatcattgtcattcccagctcaatctcagcttatacgatcgtccacaattcatttgtcgacacgcaattatcacaatttatcaacgagaagctcagcaatcaatacattgccaaacaaaatgttgacggcaaaaatattcaaatctcagtcatcggccaacgcttgtctgccagccaagtcgagcaactgcagcactcactgaagcagtatcatcttggtgactatcagttatcgttgacccagctcaccaaaggaaattacatcacacccaaagaatttcaagattatatgaagcaatcagacaccaatgacacgattcaaaccaacaccaattcagacgacaatgcctcattgaccaatgtccaaaatgacatcatcaaaaaatatcccaaacaaatcagcaatatcttcgttggccaagttcaagacaaggccaatcacacgatttccctgattgccattcagctctcggataatggcaaaggcaaagcggctgagattgagaagactgccacaaaaactgctgataataacaatgttaatgccgtcgttcgcatgatgacttcttcccaacagagtgattaaagtcacaatgtatgattctttgattatcaacttggcttgtgcataaaataataagttatcttccttgtacgcgcataaaattcgtagtattcttcgcgtatggaagggcttacacgaattgattagagacggtcgagttattttcgaaaggagtttttgttatgtcacgacaaattactggtgcggtgatcgaagagttaaatgcaccgttcaagttggaaacacttgaagtcgacgatcagccaaaagcacatgaagtattggtgcatattgttgcaagtgggatttgtcactctgatgaagcggttcgtaatgggtctgccggcgactacgcataccctggggttgtgggtcatgaaggtgccggaattgtcgaaaaagttggttcgtcagttaccaccgttaaagaaggcgaccacgtcattctctcatacgattacgatgggacttgtcgtcactgcttaaccggtcacccatcttcatgtattaactgggggaagctgaattttgcgggcgttcgtcccgatggatcagtcgcctttacccgtgaagatggttcaccaattcataatttctttaaccaatcctcatttaccaccgagacattggttcaggaacgaaacattacggtgatcgacaaagatattgacttacgtaaagtcggccctctcggctgcggctttgtaaccggatccgggacagtatttaacggcttaaaccctaaagaaggcacaacaattgcgattgtcggaaccggtgctgtgggttcagctgctttgatggctgccaagattaagggctgctcaaagatcatctgtgtcgatatccacgattcacgtttggaaatggctaaagaacttggcgctaccgatacaatcaacagtctgaacgaagactgggttgataaagtgcatgaaatcaccaatggtgaaggtgttgactttgcaattgataccactggaatttcagctattatgcaccaagccatcaccgctttggcatccggcggtcatctggctccaatcgccgttactgccaagacattggaattcatgccatggaatgaaatcactgcgctgcaaaaacacgttgatggtgttttgatgggcgatgccattccacaaatcgggatccagactttaattgacttctggcaggcaggcgaattcccatttgataagctggaaaaattctacacctttgatcaggtcaatgaagctaacaaagcttcaaatgacggctcggttatcaaaccagtcatggtgattgatcaggactacgtaccgggtgaataaattgatttgtattattaacgacattttgacatccaaatgagaaaggcggttctcaacagctaacttgctgtgggaatcgcctttattgattcgtttggttgaatttttgagcttatgatagataaatttgcaaattccaactaatccatttagtaggctgacaacaattagtgtcgctttagcctaccaaccgtcaccaccagtctgaggtagtcctggtaactggcgggcaactgtctccaaaaggattcgaagttgctggtccatagccttattcagtaaccgtttctttagcaaatcccttgatctcagcctgctgatgctgattaatattgcccatcttcggcatcaagccgtgaaggtacaaatgatccttggcaactttaatgtgcttttgatccaaaatcttggtcaattgcttgcccaccgtgaatagactgccggatgtgccaaacaaaaagacttctttgacttgcttgggatccagattgcgggcaaattgtttcaagcgttcatcgacgttcaggttataaattcccccacctaaatacagtcggtcaaccgttccggtcagcggtgtatcaatcgatttcgcctcgatcttcaattgattgcctaacatgttcgcaagtttttcagtattccccgttcgtgaataatatctaattgcatccatattgtgcatctccttacattttcgattatagttctgtatccgctttctttcaaataagaatcgcgttctatccgcatttattatctaaaatgaaataattataaagttcaatttaaagcgtttacatttgattaaggacgcactatactcgagtaagtgaggaaaaaatatgaatcaaaattttttaagggggttatttatttatggttgaaacaattagtggttcagatgctgttcttaaggtgctcgaacaatggggtgttaagaacatctacggcctgccaggtggctcatttgactcgaccatgaatgcgattcacaaccaaaagaaacagattaactatgttcaggttcgtcacgaggaagccggcgcaatcgctgctgccgcaacggccaagttgaccggcaaagtcggcgtttgtttcggatcagccggcccaggcgctgttcacctgctcaatggcctgtatgacgctaaaagcgacggcgttcccgttgttgctttagttgcgcaagtcccaaccggcagcatgaacatggacttcttccaggcaatggatgaagagccgatttttgatgatgttgctgtttggaaccgcactgctatgacggcagatgcattgccgcgaatgactgacgaagccatccgtcaagcctacatgaaacacggtgttgcagtcttaacgattccaaaggatcttggctgggctcaaattaacgacacgtatcagccaaacgtcaagtcgcatcaaacacctgtctatccaagtcctcgtccagaagacgttgaagaagccgttaaattaatcaaagaagctaaatcaccaatgatttacttcgggattggtgccaaggatgctgccgacgaattgaaggaagcttcagagaaattcaagatgccattggtttcatcattcttagccaaaggaattctcccagacgactatccagcctatcttggatcaaccggccgggttgcaccaaagccaggttcagaagccggtttcagcaccgacctaattctgtgggtcggcaacaacgtgccattcagcatcttcttgttcaacaaacacgctaaagtcattcaaattgatattcaaagcgaaaaactcggtgagcgtcggcacaacgatgtttcaatgttggctgattcaaaggttgctttggatgccattctcgaagccggcgaaactcgtcagccttcagcattctatcaggcttgccttgccaacaaagaaaactggaacagctggttggacagcttcaaagattcggatcaaatgccggtccgtccagaaccaatcttcgatgtcttgaatcgaactgcctccaacaaagcagtcttcgccgttgatgtcggcaacgttgacatcaacttcgaccgactgatcaacatgcatgacgaccagaaatgggcaacctcaggcatttacgcaaccatgggctttgccctgccagcatcaatcgctgccaagcttgagtatccagaccgcgacgtatacagtctcagcggtgatggcggctttgcaatgctaatggaagaagtcatgactcaagtcaaatatggcctgcacatcgtcaacatcatcttcaccaacgaaacgcttggctttatcgaagcggagcagactgacgatactcatcagccattatccggtgttgatttgcctgacaccaactgggctgaagtcaccaagggaatgggcgccgtcagttacaccgttcacaccaaggaagatatgcaaaaagccctcaaagatgctgaaaacactgataaaccagtggtcattgacgttaaattaacccacgagatgccattgacgactcagcacatgttcctggacacttcatggcaggataaggacaaagttgccgaatacgtcaagaagtatcaggcacaagatttgaaaccattgagctacttcttgaaagaagccgagaaccatcagcttcaaaccaactgataatcgttgtgaaagaagatcaaaggccggaaacaagcgcttttgtttccggcctttgcagtacatagaaaagtaggtagtaaggagtgccagcgatgaaagtcgtttacttgaatcaacattctcaatcaaatatggcgagttcccccaccccaattgtcttggcactgggcttctttgacggcgttcacaaaggtcaccagaaagtcatcgcaactgcccgaaagattgccagccaaaagggttatcaactagcggtcatgaccttcaatcgacatgcctccagagtgtttaatcatagtcaaagcgccagttttcggtatctaaccaccctgaaacagaaaattgaattggtgcgggcaactcacgcagatattctgtatgtcatcgactttaccaaacagtttgccgccttaccaccaaagcactttgtagaccagtacgtgattgggttaaatgccaaagtcgttgtggccggtttcgactacacatttggccggggtggaacaacaaccatcgattcactggccaaaatcagtggcggtaaggtcaaaacggtcacggtcaacgaattggccagtgaccaactaaaaatcagttcgacgcgaattcgccatttggtccgcgacggcaatattcaagaggcgacacgcttactgggtcatccctacgaaaccactgggaaattgattcatgcccaaaccaatgggttgtcgatcgttaatccatccagccgtttgcagcagctgccggaaagcgggcggtatttgtgtgaggttcgggtggcggaccacctcactaaaatgccgatcaaggtggttcatgcccgagacaacagccacggtattatttacattgaccgtcggaaatttaatcatttaccacatgtgaattcactgccggtgaagattcagtggttaaagtgaatgatccccacccaaataatcgttaatgccagccgtcaaagcagtcaataactttggcggttttccattccaaaagatgttgggagtccatgaatccgatggcacgaattccacgaaaaaattttgaatttttcaatgcaccattagatataagagttataatctaattgttaactatttcgtaatttggggggatttgaaatgagtcaattggattcatcaagtcattatttacgcaattttttgttattactctttgggatgttatcattcctggttgtcggtaacgaatttgtttctgcaaataataccggtgccgtagccgataatagttctcctaccggaaccaaagtcacaattaccaaagacaactatacccaatttttcaaaaacactggtttgaccagttatgatccatctactggaaaagtcacttttccactatcaacagtccaaggaaatcctgcttcaggatcggtaaccattgcaggtaaatcatatcccgcttctctgggatctgacggcagttactatgccgacgtcaatggccaaaaaagttttatttactacaacggtggtggatatccattcaattgggcacgtgtcagcggccagtcgtatatggcaagcaacatcgaccttcaccgaagttttgaattcaaaggaatgtacaatctaacacccggcccaaggagtatgtatggcaatatgggtgacggcgtatctttcatgttcaaaacgggtgatccttctctgcttggcattggtggagcaggatttggtgttggtggtctccaaggtgcctttggcttcgtaatcgatggatctccatacggtgatccggcagcgtccacaggccatacgccaaccatccaaatgttcgaaacgaccggtgacaattcccaaatcaataccggccaatatgacggcccctacgatgttgactttctcgggacgccagatacaagcgtctcttcggatgaatacatgggagctgacaaagagttaccaattgacattacttgggatgctcaaactaagacattacactataaactgtttaaaaatggttccaactccgacgttctctcagaaggaagtcaggacttttcgtcatatcttcaaaaatatggttactacgcaagctttgctgtttcctcatcaaatgggggtattcaatcttcggttcaattaaccatcaactcaattgaatactcagtaatcggcattgtcaacgttgactatcttctcaacaatcagaacagtgacaagattattccaacccaacaggagagaggatctctaacagataaagcgatcatcaaagcttaccctttaggtgtcagcagtgatacctatcgtttagtaaaggttaaggctcctgagggatataaactcagtggggatttgttaactctgccatttgggaatggccaagcacttttcccattttccgatgtcttacaaaacttgaagctgtactatgacaaaaacagtaaccctcaagaaaaaatgtctgccacgatcaagcatgtcgatcaaaataacaaaccaatcggtactgatcaacatattactggtgtgtttgggcaagcagtcaatattccacaagaatctatttccggttacacaccggataaaaccaatccaaagcaatttaaattcgggacattggacgaaaatggtgatgtggcaaaagttattacgttaaaatacaccaaaaatcaatcccctgttccgcctacaccaaatccaaaacccaacccaaacccgatcccagaaccaagtccggttccaactccgagcccagttccgacacgtcagcccaatccacaaccaaccctgccaaattacgcggcgaccaagggtgaagcagtttatgcattgcagaaaatctacatgtacaaggatgcaaactttcataaaagccttcgtgaagtcaaatatattcaaaaacccagggtttaccgtcccatgtttgtagttacagggtatagtcgttccgacgctggtgccttaagatataaggttcgcgatgttaaccatttaagcaagacccatggtaagcgtggcttcattacggcaaattggcactttgtgcgtcccgtgtattacgagagcaaacatcgtacactgactgtcatcaacccacaaggtattaacgcttacaaacggtcaaatctgaccggaatgattaagcattacaaacaaggaacgattctacatctaaccaaactggttcatcacaatttaaccacgcgttatattctaagtaatggaaattacattacaggtaacagaaagcttgtcaatgctggtaagcataagcaagttcagcttgtaatcgtcaaaaagccaattaatcgttataatacagtgaacttgcgtggcgaaaatcgacgcattaaggtcggtaccaagctaagagtcaaaaattatgattactcgcatgcacacaatatgacgatctctggagctttgagatatcacattgccggcggttatatcaccggaagtagcagatacgtaaaaatcgtcaaataaaatggtaaaaggagtcgctcgaaaaatcgggcgactccttttgattgtctaattgtcgaacactttttgatgactgttaaaacgctatttgtcgcgatcaaagaagtctgatattctaatgaaattttcaggattcacgaaagattaccaagtgttctcatcacttcagattgcatccctaaaataaatcatctatgattcaaactatatctgtgaccctcacttaacaaatccactaactcaaggagaaattatgcaaccaactcaactagccgtcaacttaatcaaacaaatgccggaactgcccaccggctgcgaaattaccgcagtcacgatgatgctccaatatgctggccaacccgtcgacaaagtgaccctggctcacgaaatgccctacgatgacagcgattggaataagggcttcgtcggtgacccatttaccgagaacggtgacagcatttatccaccggcattagtcggtctggtcaccaaatacgccggtcatgcggtggatctcagcggcaaatcaatcacccaattaaaacaatttctggccgaaaagcaacatccaatcgttgtctgggtcggccaattcgatggctttgccactcatgcgctggtgatgaccggctttgacgaccaacagatttactacaatgactgctggactggtgagcggactttcatgtcgacagaaggttttgagcaaatccgcttaaagaaaatgaagctggcaattagttattagaagtcttcgcaagccttccctgaacgaacacctgcttcacgtccgcctttgaagcgtggtacatgattttttcaaatatttgatccaggctttcatcttcgaaagacttcaacggtgacttgaccacttgcaagtcagccaaataacgggccttaatttgcccggttttgaggtgcaaactcttggccccaccgacagttgccaagtagaacccatttttagcagaaatcggtgggtaattggttccccgctgtgccggtgccagttcagaattcactccatcatttaacatccgcgaagacatcactgcttggcggatattttgatagatgcttggcgagtaaccaccggaaatgtcggttcctaagccaattttaacctgttgttgcaggagcttgctgacgggcagcacagcgttaccaaaatacacgttggagattggacagtgggcgaccgccacgccacgggctttgaaggtatccaagtcggcttgagtgagcagcgtgccatgagccatcaccgatttgtcagtcaatagaccatactcgtccaagacttcggcatcccgtttatggtagtgttccagtgcataaccgttctcccaatcactctcgctgcagtgggactggaccggcaaatcatatttcttcgccaattcccccaagcctttcaatgattcaggcgtgcaactggggacaaaccttggcgtaatgaccgccgtttgcttgatgggggaagtctggttgaggcggtcaatttgttgaataaaacgttctgtgtcatcgactgcactttgagcagaggcatcccgatagttctcaggcgtctggtcaggattatccatcgccaccttgccaataaagccccgctggttgtgattgacgcaagctttcgccaattccaggttggcggggttatctacactgccaaaataaagaacggttgtcgtcccatttgcgagcaattcaccgaccagatcgtcataaacccgcttggcgaacccgacgtccttgtacttggcctccatcggaaatgtatatgtatcaagccattcattcagcggccgatccagtgccaccccggcgttaggccactggggtgcgtggacgtggaggtcgatgaagccgggcaataggtattcatttgacttcaacgtgagcaaccgatcattttgctcggcgtcgcgcttgaccgctgaaaaatcgtcatctgattcattgatcacgcgctctatataaccggaatcgtcaatgcagaccaactggcgctgctggcagtcgacctcatcaggtgttgcagcagtcatggtcgggccttcgattacttttgtgattgtgataatagccacctcagttttcattatttttaaaactaactattcaaattccctatacaaagtgattatatactgccaaatgtcccgactcaatgcatgccatttcaccaatacgaaatggcatggacttttcgacaagaaatgccggataaatttgtaggaagtgccaaacatttccacccctcacgatttatactgcggacaaagtggtgttcagcagtcaagttaatcgttattgagggggttaaaatgatgactcaaagaggtttattcagcaattattcattagttcggcggttttattagggctattggtgggcacaaccggctcggtgaaggccgcaagcaccccccaccatctcagagctcaccagtttcatctggcatcgtgcagcctttagcggccgtaccccatcagaccggcgaaattgggacagtgacgtaccaaattagtgatggcattctaggtctgagtggtgggccatctcaagccaccccgaagagacctatccatggaattttaatgaaacgatcaccaaagttgagatcaatggaccaattattctggagggaaatgcggccagcagtttctttatggcattaccaaatgtgacggcaatcgagggcatcgaaaaattggataccacccaagcgactgatatgagccacatgttcgctgatgataccaacttactcgagctcgatttatcgacgttcaatacagataatgttaccgacatgaatagcatgttctctggtgacgcatcattggaacatttgaatgtttacactgaaaatgtcactggaatggaagcgatgttcgcaagagacacccacctaacaactctggacgtttctcattttaaaacaaccagcacttacgatatggccagtatgtttcaagacgatgtacggctacaggaattatctgtcaacaactttaatactgaaaaagtagatgatatgtctgctatgttttccggagaccttgctttaacaaatctggatctctcacatttcaacacggaaaatgttgttagatttgcttatatgtttgcgggagaccaatctttaaccactgtgaatgtttccaagtttgatacatctaaagcagaattaatgacgggcatgttttccggcgaaacttctttaaccagcttagatttatccaactttgatactcaccagacgttgattcacggagcatgggggctgtcaaatatgctggcatccctgaccagcttgaccaatctcaaactaggtccaaacgtggtgtttggccctgctgagagtatcggcgatccacacttaattgccccggctggcgcagacaactggcaggcagtcagtagtggtaccccagaagatcctgaaggcccagtatactcacctgatggcatccgcgggttatatgaacctaccaatcctgaacacccaactgaagtggaaactttcgtaccggaaaagccgtttgttgatcaatcggccatctcggttcaaccaacatacagtatgacaactggaaccaagtttgatgccagcaaggtcttcaactcaattaccacaccagaaggcaatgtcggctacattaccgccaatgccaaatttgtcactaatctctactattaatcattgcctaagaataaagagattacggtcattgctgcaagaggcgttcaagcctacaagaataagaatttgacccgaaagacaaaggcttacaagcaaggcacccatcttcgagttaaagcgatcgttaagcataatctcacgacacgctaccagttgagtaacggttactttgtatccgccaataagaagttagtcattcagggaaaagcttaactgaaagcagttcatatttttagccaccagtatcgtgctggtggcttttttaggatgctggtgagaatccccggcacaagaaaaaactattgtggactttctcacaacaatgcccctgcaatctttgtacaaaccaacaaacaaatctccccatcttctctctatactgaaggcgaattgaacctggttcaggttttgacagtttgtaaacgtcgagggggcgttttctatgaaacaaagaaaaattgtgatcaaagttgttgtcgctatggccgcggccatggggttgctgttagggacggctgccagcacgaatgttttgactgaagcagccgaaacaaataccgctgttcaagatgagaccgccagtgggcattttggtggcccagatggtccagactggacccgtgacggcaataatttcaatttaacgggtggtgtcctgacggagagaatcgacaatcaattgacttcaaatataagaacggcaaccgtgattaacattacgggtaagctttatcttgagggcgaggcctcgcgtgagttgttttcctccctcaataatgtgaccacgattaatggcatggagaatgtggatacggcaaaagcaacgaatatggagttgatgtttgcggaagatcaagcactcacctccatcgatgtgtcgtcctttgacactaggaaagttaccgatatggcagcgatgtttgctaatgacagttcaatgaaaagcatcaatgttgccaactttaatactgataatgtgacgattatgcccaacatgttcgccgatatgcacgaggttgaaagcatcaacggtaccaatttcaatacccaaaaggtcacagaaatgacggcaatgttttggaatgatcctaacttaaagacggttgatgtgtcgtcttttcaaacaccaaacgtcaccagtttcagggcaatgtttgcggatgattcaagtttaaccagcctcgatttgtcagggtttgacacccaaaagctcttaggatattctaacggaaccctcggactcatgctccggggaacatccagcctcacccaattgacactaggaccaaatattcaatttgataaaaataagaccattaacggcgcgtctgcagggctcccaacactcggcgcccctgccggctctgaacgatggcaggcggtcgctgccgataaaggcggtaccgtcgacaatcccaaaggagcgactgccttcctccccgatgaattgacttccctgtatgatcagtcgaatgccaatcatccaaccaaggtcgagacttgggttccctatttcaaagacacgttggatgttaaatcgccaatcaacctgacagtcggccaatcatttgatcccaaagcggggtttgtctccgcagcggatggcaatggtgaaccggtcacttatgaccaagccgtcgccgaaggaaagcctggcgggttggcagttgacaccagcggactcgacacctccaagccgggaacctataacgtcacctacagctaccatatgcgaaaggccgttgtgaaggttatcgtgtcggcagcccctggggtgaccccaaatccgaccccgacaccaaacaccaatggcaataattccggtagcagcaatcctgcctggaacccgactaatccaaagaatccaaacggcaccggtctgcccaactatgcagatgttcggaacgatgcggtctacgcaaccaagaaaatttacctctaccaaaatccaacttttaaaaagtcacagcgaatagccgcttatcccaaaactaagcgaatcaaccgaccaatgtttgtcgtcattgattttgccaaatcaaatggcggtgccctccgaatcaaagttcgtgacgtcaaccacggcaaaaagactgctggcaaggttgggtacatcaccgctaatccaaagtatgtaaccaacgtctactaccagaccatgccaaaatccaatcaggtcaaggtgatcgccaccaagggtgtttacgcctaccagaatgctaatttgtccggcaaggccaagcactacaggaaaggggctcgtctgaccgttaagaaattggttaaacacaatctgacgacccgttatcaattaagcaatgggcattttatcaccggcaataagaagctggtcattcatagccgttaagggcatcaattgtttcagaaagtctgcgcactctcaccatcaactgttacaatcaaagtaatgggcgtgatcgttgtgtgcgcatccgacaatttggcttcacccttcccgcccagaaaatcactcaaggaggaatttctatggcggtattttcagaagaacaacggctgcaaattttcaaagatctcatcgcgattcaatcggtgaacactgatgaagaaaaggtcagcgtttatttaaaaaatctttttgagaaacatggcatttcggccacaattatcccagtcgatgagaatcgaactgatctaaaagcagaaattgggacaggcaatccagtcctcggagtctccgggcacatggatgtcgtttcaccgggagatacctcgaagtggaccagtgacccatttacattaaccgagcgcgacggcaagctatacggtcgtggtgcggcagatatgaaatccgggttggctgcaatggtcattgccatgattgagattcatgatcagggcttgctgaaaaagggtcggattcggctcatggcaaccatgggcgaagaagttggcgaattaggttcacgaaccttcgctgacgatggctcaatggacgacgttgatgcactgatcatcggtgaaccatccggctaccgaatcgcctatgcccacaaagggtcaatggatattcgcctaacttcaactggtaaagctgcccatagttcaatgccggagcatggctacaatgcgctggatccactgattgatctcctgcacgacgccaatcatcaatttagagcaaccgataaaaagagcgcaatgttggggaatctggcatttgacacgactatcttcaagggcggggatcaagtcaactcaattccagccaaagctgttgccgatatcaacgttcgcaccatcccagagttcgacaatgacgttgtcgacaaacagctggatcaactcgttaaacagcaaaatgccaacggcgccaaaatcgtcaaggaaacttacatgtctcagccatcagttgaaacgaccggcgacaaaaagttgatcggcttggcacaggaaatcggcaaacaatatgccgaaaaagacatcccaagtggtgccatcccagctgtcaccgacgcatcgaacatgctgcgggataagccgaaggaattcccatttatcatctttggtccaggaagtaacagtgtccaccaagttgatgagtttgtcgacaaacagatgtaccttaactttgtggagatttatcagaagttgtttacgcagtatttgaactaaagacgaatccaatcaaatagcagccgtcaaaccacttgcttgtgatttgacgactgctattttgttctgatagatactaccaagccaactcataataagtgaaaaatgccataccgacccccacccacacgagcaccataatcacaatcatgagactcttaacggccgtattaaaaattgtataatcagcgaaccgctggtcaatccacttgggtgcagaaatcagtcccagcacgattaacgtaacaggtaagataaaaatcgtgattttgctgcctggactgtctgcgacgccaaagccaaaatgagtcggaacgatttgaggtaatcgtggataaaagacgatggccgccattgcggtaattatggtcacacaccagtggacggcaaggattttagagtaaactttggaaatcagaattgagaaattcatgtgggtcgcttccttagtggctatgtactttttgttaatgctgtggtaatcatatcacggttaactggtaacacaatccttattttgaatgaattgcaaatgaacggaagtcagaagatagccaattaatgacaatacttttgggagaatacttctgtgctataataactgacaaatcgttatgaatcctgcaatacaagaagggctatctatggaaattggtactattttaaaacaaactagaaaacgacagggtttatcacaaaaagaattatctgatggaatctgtgcgcaatcaatgctctcggccgtcgaaaacaatcaatacaccccaaatgcgcaattgctgatcaaattatgtcaacgactttctgtatcccttgaccaattcagtttggctgataatttcgatattagcccacgtaacactttcaaccagacagttgagaagctttgtaataatcacaattatttaaaacttaaatctttcttgtcagaaaactcaacacttgaacaaattgaaacaccccagcaaacccaggcatattactactatttgggagtatcccagtttcatactgataaaaaactggatgacgctcaaaacaatttagaaatgtcggttaacattgctgaagaaaagaatagtttatcagttctaacacgcttaggactgatcaccttagcaattttgaagagtaaaaatcacctccaaagtagtgccacaaagcttattcaacgtgcaatgcaaaacatcggcaacatcaagtatgaagaaaatatcaatgttattttttatctggcagcattcattgactatcaatcaggtaacaatgccatggcggtcaaacaagtcgaaagtgcaatcactttcatcacaaatcataattcacactacatgctcgctaactgttactatttgattgcacagattgctaagaattcaggagacaaagaccaaatgctcgaatccctgcaacggcaaaagtttctaactgaactatttcatgaaaaagtttatgataaattctaaatatcagtattctgatttttcaacaagtctaatatttagtaaattaagaccattcaattaaggaggtctttgtttatggaaactaaattgttttcgaatgttgtaatggtaaatgcagatatggaagatgtaaagggtattttgtctaatcctcaacaactgcttcagtgggtaccggacatttccactgtagatcaatctgagaacggttttctcatcaaacgatccggagcggcattaaatcagtctgaacgcattcggatcgagactaatgggtcaaagattacttacatcagtactcagggacgacttgaatacaaactgattttttcggtacatgcacaaaatcaccaagctgtcgttcaagaggatctatacattctcaaagatgcgaccaatcagctacccgttaagttattagccccaattgccaagcatgctttttattctaacctaattcgcttgggatcctttgcagagctaatagcggcaaataaccaatagatattttttggatattgaggatgcccaaattaagtcagttgaattgcaactgacttttttgtgcatcctcaatatccaaacgcctaacaactagcacaaagtccccgttgatgatacgataaaaccaaaattatctctatcaaacaagcataattattgcatcagtcaatcaggggaggaattattatgcagtctgtggatgaccagttaaaacagttatcaccagaggaactcattaaattaacatctggcgccaatttttgggaatcggtggcactgccagaccaccagattcccagctttcgaatgagtgatggtcccaatggccttcgctaccaggcgggtgaaggcgatgcgctggggataaatgacagcgctatcagcacctgttttccaacagccagcgcagttgcctgcacttgggatccggatttggtcgctcaaatgggccacgccatcggcttggaagcccgcagcttaaaggtggatatggtgttgggaccggggatcaacatcaagcgaaatccgctttgcggccggaactttgaatatttcagcgaagatccttatttagccggcatgatcggcgccggttggattaaaggcctgcagtctgaaggtgccgcggcctgcttgaaacactttgccggcaacaatcaagaaaccgatcggctgttatcaaattccatgattgatccaactgccctgcacgaattgtatctggaagccttccgaattgccgttgaatctgcgcagcccgaaggcgtgatgtgttcatacaatcaggtcaacggcacttattccagcgacaacgcctatttgctgagcaaagttttgcgtcagcaatggggattcaaaggcgccgtcgtaactgattggggcgcgctcaatgacaaagtcgccagcttgaatgccggcggcgacctggaaatgccatccagtcacaacatgttcgacccgcaggcgctcgaggctttgaatgccggccgactcaaacgaccagctcttgaccgagcagcgggaaacgtcgttcgaattgctgaaaagcagcggccggaattcactggcgatcgcaaggacctactgacaaaaaatggccaactcgcccagaagattgccgaaaacgccgcggtcttattaaaaaatgatgatcacatcctgccgattgatccatccactaagctcttggtaatcggccagatggcagctgaaacccgttatcaaggtgccggatcttcccacattaatcccccatcgcagacctctattttgcagggattaaccaatgccgggattgcctacgattatgcgcagggctaccaatttaccggtgaaaacaaccgtgaattggcgactgctgccactgatgctgccaagaatactcaaactgtcgtagtggttgctggactgccagaaagtgccgaatcagagggctttgaccgtcctaacatgaagctgcctaataatcagaatgagctgattgaacaactggcggcggtgaacccgaacgtgattgtgttactggttgccggagcgccggtagaattgccgtggcgaactaaagttaaggggttgatcaacctctatttaggcggccagtttgtcggcaacgccgcggctaatttgttatccggtaaagtcaatccatccgggaagcttgccgaaagttacccgattacctatcaggacgttccgtcggctgagctatatgaccacaatccacgttcggctgcttacgccgagagcgtctatgtcggctaccggtactatgaaaaggccaaccaaccagtcgccttcccgtttggcttcggtctgagctataccagctttgaaatgagtcgtctacagttaaatcagcaccaaattgaagccggccaatcgattaacgtcaccgttgacgttgccaataccggcagccgcgatggcgccgaagtcgttgaagtttacgttggcaattcgtctgaccgcgccttgaaaccattgaaggaactgaaggcctttcaaaaagtctttttaaaggccggtgagcaacagacagttaccgtcaccctgcctgctcaagcctttagcgagtgggatgagcaacagcaagcctggcagctgccagcagtctcgaagaccatcatcgtcaaaatcggatcgcgtcttgaggaactcaccgcaccagttgaagtaatcggccaagccatcaccccaactgattccatcccgagttggtacacccatccagttggcaaaccgacgatcgctgatttcaccgaactgactgggatgaccgttgcgccaccagcaactccgcaaccggggcaatataccccattgaacacgccgcgggaactgagtacccactcggcaattattcgtaaaatcgtttcagttttaaaagccaacatgaccaagggcatttcagatccaaatagttccgaagccaaattcatggatgccatcgtcatggacacgccactgattcggcttgctcaacagtccagtggaaaactctcacttagtttggtccacaaactagtcgcacttgccaatcggcattatattcaggcaatctttaaaaattaatcgttgtatgtaagggggaagtattatgacacgaggggcaagatggcggttggcatccgcacttttatcgatttcaattctcttaaccagcgccaatgcggtcgccggaaccattccgatcatggcggaacggttcccatcgattccactgagccaaattgaaagtctgaccaccattcccagtttgagcgtcttgatttttgtggtcttgagtaatccgatcgccaaaagattaggcaacaaagcaaccgtgttaattggggtcttcatcgtcctgattgccggactgattccgactgtcgccaattcattctggctgattttggcgtcgcgattcctactgggtgccgggataggtttattcaacgcgatggcctacagtctaatcagctattattacgagggaacgcaacgccagaccatgatgggctatgaaggctcggtgaactcactgggcaacattttaatgtttgtgttttcctcaattctaatcgggtttggctggcgccaagtctatttatactatctgattgccatcccagtcttcatcctgttttggtggggtgcgccaaatgaccgccaagaaaagcaaccgcaagccgatcaagaggcggccacaccatcagtcggtttgggggaactattgaagggccggttaatgatttatgcattattagtcttgttcagtatgatgattgcccagacggtgatcgttaaaatttccggcctaattttaactggcggctacggcaaaattgccgatggcagcattgctctggccttcctgggggtcgccaacatgattggcgggactctttacggccaaatattcaaactcattcatcaattgattttaccggttggcttgttgattgccgcagtagccctgtttgccctggcacgatcccaatcactggcgcttacctacaccctgacggtagttgccgggttaagtacgtcgctggttggaccctacttgtttgccagttcagccgaaattgccggcaaaggcaacgaaaccttggcctcttcaattctgattgtgggaattaatatcggcgtattcttaacgccttacgccttgtcgggattgagccatctgatcggcagtgatcagccggcaccgattttaatcgccgttagcgttgtcttggcggtaattggtgcgttaaccttcttcatgaaagaacccgatcaacagtctcaatgatcacgccatttctaggccatcttaatcagtccaacgccgatgagcatcagcaccatgcccaatgcctgagcaggcaccatctgttgcttgatggaccgccaccaaccgaattgctgaatcagaatcgagccgatgatttggccgatcaaacccatcataatcgttaggccagcgccaatttgtggaacggccaccacggtcacaaataaaaatgagccaccaagaatgccacccagccagttccaaggttgggtggtttttagttccctggtggtagggacacgtttgtcaatcatcagggcaacggccgcaatcaacagcgtgccgatgaaaaacgaaatgaaggccgcttgactggtcgaatgcagtaatgttcccaaatgaccattaattgcctgctgcatcgcggccaacaccccaacaatcaccgcccaaatttgccagccaatcacgcgtgtcggcccgtcttgtcgagcaacgttggcgtcaaaccggcggatatcgcgattggtgaggctgggtaaggcaactgccaccagaacgccgacaatcaaaatcagaatgccaaccagccgccaagcagtcatggcaactttatcggagccgaaccaccccaaccaatcggtcacggtgcccatcgtgatctgccccataatcggtagaattgtcgtttgaatggcgccaattttgggaaacaataggatatttgatgttagataaatcgaacccagcagaccacccaaccaaatccaggctggctgcgcttgaataaagttgccatttggaaacaaccgcccggtcattgacatagccaggatcgctaaaaacaaggtgccgataatgaacgaaatcgtcccggcaataaacggcgatttcactagccggcttaaatcagcattaatggggctttgattggacaataggaacccggcaactaatgaaatggtcataaaaatcagcattgttttccaccttcaaatcatgaaatcagactatttgatacacgacatatagtcgaaagaaaagcagtcaactatttcaggttaactgcttgtgtgaatgattggtcacgtaagtaaagatcaccagtttggatgactgtattatacaccgcccatctttgaaatctgaagatgaaccgaaccactttcctgaatgcagcttaaacaacgtgcgcaacgcaatctccataaatgtgattcatttaataaatgtaatcgctttcaagactccaactaaggtgctatcgttaaccacgaatcgtgttcctcatggatttaaggaggtcatcaacatggcagagttggacggaaaagttgccatcatcactggtggtgccaatggaattggtctggaaacaacgaagctctttctccaggaaggcgcaaaagttgttttcacggatgttaatgcggatgcgggtaagcaggtggaagatgaactgaataaccagaacgccctgtttatccaacaggacgtcggtgacgaagcagaatgggaaaaagttgtgaagaccacgcttgatcaatttgggacaatcgacattcttttcaataatgcaggaatttacattattggtaaaattgctgatttaacagtcgatacttggaataagttaatgcgaatcaacgtcttgggaacttttctgggattgaagcacgtcctcccagtgatggcagagaacaatcacgggtcggtcatcaacgcatcatcaattgccggaattgccggttcagccggtcatattctctatggtgccagcaagggtgccgttagaacgatgaccaaggacgccgccgcggagtatgccagcaagaatgtcagagtcaactcgatccatccaggctatattaaaactggaatggccgactacgcctcagcatcccttgggataccagagaatcaacttggcaagattttcccgctgggtcgtttgggtgaacgaatcgaagtggcccaaactgttgtctttctggcatcggataaagcatcatttatcactggggttgagttaccgattgatggtgggttcttggcacagtaatgagaagaccattcatatgcggttgtggttattatgagtcagtctgattatgacaatttgatggagaaactgaatagctaagtgatgcacattcagagtatattcctaagcaaaaaatggttttgcttggcatcagggcgaatcattatttttcaatcaagaaaccgttattatcctgggtattaaaacagctctcgacgcaatatgtcgggggctattttgatgactcaggctttagttttatccagacataattttccgcctggaaagtaccaattacaaatttcactttacaccttaccgatcaacgtttttagaagcgcaactatactcaacaacgagcttgatgaattagtttctagataagccacgccataatcaagtatcactggataatccagtgggataacagtaacattcgattcagtcgaatcaaccgtaaaagacggtaaaactgccaatccaatcccccccttcaccatattgattgcagtattaagagtgtcagccgtttgatagtgaaaatcctctggtgcttgaataaaagtattctgaagagttgcactttcagggggtgcttgcaacggattgaaaaagattaactgtgattttttcaagtccgaaaaggttaacttagatttctcactcaaccgattcccaatcggtagaaccacattgaagtgaccttgaaacatcggtacaaacttgacacggggattatcaccaatagtgtccttggttgcaagtattaaatcaaaaacaccgctttgaagattactcaaaccagtgcttaagtcaaaacttcgtaaagataaacggagattagggagctggtgatgtgcgctcctcaacagtttaggaagtagcttattttcaatcattgcattggtgtaacctatcgtgagtgattgctgatccttttcactaatttcacggctatcaagaatagcttgctcagtcaatatcaagacgtttgacatttgcttggaaaattcttgtcccgccaccgtcagtgacacgccatgctgatttcttcgaaacaactcaaatgcaagctctgtctcaagctgcttgatgttcttagaaactgcaggttgagatagatgaagacgggtggcagctgtcgaaaaattaagtgtttgagaaactgttacaaagcattgtagttgttggaaattcaaatttatcattccattctttcatgatctataaataagcgtgataatcgattggccttccatgtgataatctgaacttgtaaacgagaaaggaagattattatgcgatatattattacaggcgctgatggcaagctcgctggtcgagtggcagagttaatgctcaaagaagtaagtggtgagcaattaaccttcacttgctacaaaatagaccgggttccaaaggataagttaaagcactggaaagatgccggtgttagagttgttgaagctgactacaacgacaaatcctcaatgttgaaggcttttgaaggtggggaccgactgtatttgatttctggccttgacgttggcaagcgtgttcaacaacatcgtgatgcaattgatgcggcgattgaagacggtgttaaacacatttcctatacatcatttgttggcgcaacagaaccagcttaccaacatatttttgttactccagatcacactgcaactgaaaactatttggaaagcacaggtattgactacacggcactgcgaaacaacctatacatggaaacattcatgacaatgagagctatgttagcattcatgtccaacaaccgttgggtcacaacagctggtgagggcaaagccacattagtttacaaggacgactgtgccaaagccggagttgcctctctacttggtaagggaacccgaaaggtctacaacattgtaggttcggaatcaatttccgttcgccaaattgctgatatgatcagtaaacgatcaggacaacaacttgaatatgtcccagcttcgcgagaagaatattatgactacttggccgccttgaacatcccccatgacatgtcaggtgacttttcaaaatctccagcaccgtttagtgcaaatgacgttgtagataatgataaatcaattgcggatggactgctagatgttaagtccgatgatattgaagaactaactggcgccaagcctaagacccctgaagaagtgattggggagtttgattatatttggaaagatcatatcaccaactggcgccagatgaaataaccaacaagcttaaggaaactgtattgtacatgtattcatctcaaaatgtaagtgtgagctgtatttgtaaaactaaagcttcggctttaactttgcagatatagcccacacttttgcgattatttgtcttaattttattgtttacaaaaattctcccatgttattaaaatcaatgctttcaaagtctgccatattataacattaagttttttcagcaatggccccgtctttcaaggcccgaatcagtttaattaagaaattaaatgaataaaatccctggatatagtagctgccgtcaataatgatcctctctgtccaatttaagttttgatttttagtggtttcaatttgtttggcatatccatatgctgtcagttgatcggcatatagccagtcaacatttccatcattaattacaactccacagattctgatgctgaaccatttcgcatcagagatgatcccaggtattttcaaggcagcatcttctcgttgatcaagcattttgtccaacacttgagaagttaatgaattgatgggttctagccccaatgcaccatcttctgaaggaatcgtctgattaaaccagttcggtacaatgagcatctgttcaaagaaaattcgtgtttctaacagcggcgttattctattcgttggatagccaaactgctgcatcggtttatgtctgtgactataactcataataaagttatcacctgtatttacgatgaattgtatttggtgaaatttgtaattgccccattctccacttgtccgtttatcgttagctctcctgacggaaatgtaaataagataataaatttcagatgggtggaattgggcggaccaacgcttcagcgcatctgaaacacattctcgttcagcatcgtttctcacttcgaagtggaggcgtgctaattcaaaataaaacagtcgtttcaattcattcaagacaagatgtctgtgtaagttggtcgtttcagcttcacccattatcatccctttgttggggtttgtaagcgtctgtaggaggatgtcatcagatagcaaatcactttgaacccaaacgtcccatgccacatcagttaggttaaatttggctgtttgtttgtcgaatgaaacatcagtgaagacatcaaaatcactcaacggagaaagcaccagtacgccgctcgtgtacaacttttcaattaaatttgatgaatcggttccaaaattgtcctctaacctttcatcaatgaggtgtcgactatatggtccaacatttgttagctttgttgcatgtagtttttgtaatatgacagctagatataaacgactttctacatccaaattttcaaattcatatttggtgcgcatttcattattctgttgaatcatttgcgcaaacttctcccgctcctcttcttttttcttcaagcatccatcgcaatgacattctcggggagggtaatgccgagcagtcgaaaaaatagtatgaccacatttaggacaaatagaattttccgaagaacctgcttgactggtccgagatggcatctttctaagtaaatgatttccatcatatggacagacagccacatcttgtacctttggaagattcttagcaacgtcctgaattttgatatttagctgatatttttcaagcagctctttaactgataattcagcggagtaatacaatttcaaaaactgcttcagatcatcctttgttaacatactgaaaatgttatcttggggaataatcaatttttcaatttcataatctgtaaattccatgtgtgcacgactccattcagacaagtttgattgcgttaattggaataatatcataaatcatttgttattttcaattggcatctaaattaattttccaatatcatcgacattcttgtaccttaaaagcacaaaaaagccctggcgaccaaaccagggctacatatcactcaacgtattcaaattgtgttttctaaacaggctgagaaacattattaaaatagtcaaccaaaaattgtgaaccgttccacgtcactttagtaatgctgccattgatggttggcacgtagacgggcagattactccaatgcgcaactaagtttcgaatggcggttccatgagttgcaaccaaaatctgatcatggtcagtggcctgagaaataatttcttgaataccgcttgagaagcgttcccagaattcagcgctggtttccgcatcctgataaggatccgcagaggcaacgcggtcctcagcctcttcaattgagtgttttaaaatcatttgctcaaacgaatcaacgccttcttctccgcctaattcatgccacaactgattttcatcgctgccttcaaaatatccgtagttcaattcacgtaatgcttgcattggcttcaattgcagttttggagagacttcctgattttcctgtaatatcagcttgccggtattaattgtccgcattgtatcgctggtataggcttgggtaaaatgaattcggctcagccgactgccggctctttttgctgcggcaattccctgctgagttagcggagagtcacaatttccttgaatccgattatatttattcaagaacgtttgtccatgtctcacaaaatataaagtaattgacatcaattgtgcctcccttcaatgactcaacttctcagtaacgctgactggcctctttggacccgccaggttaatcctgattagcaattactgaatgtcaataaacggtagttgaaataacgttgccaaatccttaatttgttgttctgaagcagtaaatgtcaaaacggtatggtgaccgccgccattttgaatccactcagttgcaccatgtttcagacccatctttggtgtccaatattgtttggcaattggcagataaggtgtcttcttagttggtttgtgggcagtcacaccataaccgatcattctaaattcggttccaaagtcggaaatggttacatccattgcatcgccatctattccatcgaacacgaggcgggctggatcgtccttaccaccaatgccaagtgggtgaacttcaacccgtggcttatcactggcaatcgttggatcaacttccagcatgtgcgagcccaaaatagcttcgttgcctttggtcaattccaaggtgtaatcttccataaagacagtccgatcattatgggtcataatcttaagtaaacgatcaagtgcagcggtcttccaatctccttcgccggcaaatccgtatccttctgccattaacaactgcacagccagacctgggagctgttccatcccgaacaagtcttcaaagttggttgagaatgctgtatagccacccttgtcaagaagatgcttgatgccaaagtattcccggatctggtagcgaacggagtgctcatatttggcagcatcattatcaccctgaacgaaggtatacttttgttggagttcttggtacttattgtcgatatcagtgtcagaaacctgattgatttcttcaaccaaattgccaactggctagtaatcaacagtccagccgaattgaatttgaccctgaatcttgtcaccttctgtaacggcaacgtttcgcatggtgtcaccaaaacgggccactttgatgttgaaactttcattgtaagcaactgcaacatcttcccaatcggcaatttcttgttgaatttcgggatcagcccagtgaccgtaaatgaccttattgtgcttctgaagtcttgcattaatgtagccatactcacgatcgccatgggcactttggttcaagttcatgtaatcaaagttgatggtgtcgtatggaatatgatccaaatattgggtagcaagatgcagcaatggcttttgcagcaacttggttccgtgaatccagtttttggctggggaataagtgtgcatccaagtaatcacaccagcgaccttatctgtataattggcttccttcatgactgctgtaatttcatcagcggtggtagcgacagctttaaatttaattggatagggaagcttgccggaagcattcaatttgttgataatatcttccgtatcagagcggacctcacctagtatttcttcgccatagaggtgttggctgccaacaacgaaccaaaattcataatcagggaccttaagcattgatatttctccttccgcaactttcaaaatggggcgtttgaagttgacatttaatgaaaaatcattaaatttgattgtattattgaacgttgtttcgcctgtctgttctaatttccagaacttggttcataaacgtttcaacacagtcatgataagggaacactgactcgataaatgcacgatattgcatgaaaaaatatgcatatttgatagtaaatgatcactatttcaatcttgaaaggaatctattatgagaatcgcatttagcaacctgaatgacaccatgccgatttcttgcgaatcaattggctatcactggcggcagtatccaatataccgacccaacggctaccgcttttttcactggttacaaaccgaaagcagctcaggaaccattaaaattgatggccagcaaatccatctactgccaaactccggcatcctcattcgccccaccgttccgcattcttatagtgctgactcagatgccaaagaatgggatactgcctacatcaccttttacggtccgctcgccaattacctggtgaactatctggaagtcgaggactatcgggtgtttgaagatttacctgaaaacattaccaatttcatccaaagtaactaccgggcatttatcaacaatacaattgccgaccaagccaaccaatcagtgctgatctatcgctacttgctgctgcttcaccaaatggatatcgtccatggtcaacaaagcaaatctgatccaatcgttaaccgaatcaccagttttttggaaagtaattatcaatttaacattaccaatcaaagcatcagtaacatcaccggcctgtcgattccttaccagacgaatattttccggcaaaaatacggcgtgaccccacttcaatatttgtttgactatcggatccgtcaagctgcctatctactcgtcaccaggagggatctccaagtccaagaagtgtctgaacaggttggcttttccgacacgtccagattcattaatgcctttaggaatttttatggggtgacgcctaagcagtatagtaggacggcctaccaaggtaataattgatgacgaaggctcaattaaaaagcaagaagtgacttacaacggaatgccggctacttaacgatttgcaaaacaaaaagtgaaccgaaccccttgaattagatttctccaattcaaggggttcagttcacttaatcacaagatcagcttcacaaaaggatagtcgctacaaaaagattttgttaacgaaacacgccaaccgctatgcaactcggattgatcaattttatcagcaaaataacaaagaattaaggcatgttctcggtgacaagaatacagatactcttgtagaaaatttgcatcaaattcaaaaatattttgatgataagctgaattgacagacattatgatgatctctcaaagactgatatattgattgttagagcctaccccgacaattttctacgccctgaacaaacatcagcagccctgaacagctgatgtttgttcagggctattttgtagtgttccgattatcacgtggcctaaaagtatttattaacgggagcgttaaagatgagcgaaccagacttccgtgaagttaatcgctcctgcttttggactgataaattggcaataaaacatcatcaactaacaattccaatttgcgctccgttaacggctgattagtaaaaagttgaaatctgagccaatcgaatggtaacaatgcaatctcctcaggcaaatctgtttttacgatttcgcctcttttttttgcccgtgtaagaatgtgatcaagagcgttaagatcgatcgcgtttccatcgctcattaattgttgaatcgtcgtattttcttctttagttgcttcccccagcagttctgtaatacggaagtccttaaatgtttgcatactaataatgaatcgttgaagcagctgcaataaatcctcgcgtaacgaatgaccagtcaaagtgaaatcatccgttcggccgtgattttctgacgttatcttgtcctgaattgcggcaattgccagagagaatggcgtctgccatcgacgataaataacagatttactggtgttagccaaatcggccacatcagcgaaattgaaacttaaaaatcccttagttttcagaagctgtaaagctgcctgataaatcgcttgttccagttcggcaccccgacgacgtttttgaaccataatgatgactctcctttttgtaagatacttaaagtatcttattgcattttttatcttcatagtgtattatatcaattatcgttttaagatactaatagtttcttattcaggaggaaaagtgtaatgaataaacaaatcccaaaatccacaatcatcatcgcttgggttgtcgtctttggtgcaatggccccattacttgattcaacaatgatcaatattgcgattaataagttggttaatagttttaatagttctgtcacaacacttcaatggaccattacctgctatgtattggcaactggaattgctgttccgttttcaagttggttattaaataaatttgatggtaagcatgtctttatgctcagtgaaatcttattcggcatcggttccattttagccgcagtttcaccaaacatccaatttctaattggagcgcgcctggttcaaggctttgctggtggcttaattatgccgttgctaaccacccttttagttcaaactgctggtgccgccgttatggggcaaatgatggcaacggtcggtttacccatgatcttgggtcctctgatcgggcctgtcatcggcgggattatttttaattttttgtcttggcaatggattttttggattaacgttcctgtaaccttgacgtcactcggtttaattatttggaaaatgcctaattaccctgcacaaaataaatccgcaaaattagatctcatcggaacactgcttctgattggatccagcaccagtatcatttatgggatggttaaagctgcccacaaggccaattttagcaacccgtcaacactcacctttttggcaacgggggtttcgctgctaattgtctacgttatctggggcgccattcgcggcgaaaaagcagttatcccgcttaatttgtttaaacatgggtccttcaatggatcaattataggcttgtttattgctggaactgttcttaatggtgccatgttattgttgccgctgtttttccagaacgtgcgtcacatgagtgtcttgatggcctcactggcgttgatcccccaaggattggggatgttgatttcccgcccactcaccggccgattgaccgattcaattggtgcaaagtatgtcgttcttgtcagtgtgtttattgcttttgttggtacgattcctttttactggatcactcaaagcacaccgtactggatcattgccgtcgttctgctggttcgtggaattggggccggtggtattttgacgccattgatggctgactcttattccggaatgaggaccgaccaaatttcgagcgccacaatcggttcacggatcttgcaaaacatcggcagtgcctttggttcagcattagttacaactgtcgtaactgctttttcagcttcgcacgttaaaagttttcagcatcaattaaaaacgggtagcctcaaaccggcatcagggcaattggctgcttttatccaccaacatttagttgctattcgacttgacgcatttcaacaaggatttttaatgatttccctggcggcactgttaatcattctgccgaccctgctactttctaacaaaatgaaatcaaaagaataagcagatgcaggttaccaaactacgtgaagtattcaagagccttgcctgaaggaaggttgattcgatcatgaaaaacgatatcttaacaatcatgcatgggtggtacattgcccttggcgttgtcctgtggcttacactcgttacaatttttgtttcgaaacgatacctcagcagctccccggttaattgggctaaattatatttaactcctatactatttattgtatttggtattgagaaaatcgtccgctttcgacatttggccgccactttaacaattttcttagtgattattgtgttagccagtttctttggtgctcacttggcctacaaataccaatcttttttctggcgagaaaatcaaatcaaaatgattggcggcaaatacgcgattagtttaatgattatgaatgtcatcgtgatgatgctgattaatttccatggttgggtaaaccctgaaagttatgagacttggtcatatacattaacctatgcaatcacttcggcaattgttaaggggttgttaattggccaatcggttaatatgtggtggcatttgaaggtattgcctaagaagctgtaaccgttagttgatcataattaacacaaaaatgagctgtgtcctcgaagataacagaaagaattcgaggacacaactcattttttgtttgataggcttcggatttggagacctatcctgttaaaagtctgcaatctcaagagatcaaagaaagtcagtcgacccaaatatcatccaagcgttcgagtaccaatcgcaaataccgaaattactgatttccaagcggtaaaacgcaacacaatattttgttaccttgaagcaattttcaagaactcatcgggattgttaaaacacatgagatttagctaagttattcagttaaattgggaacctcattgaactgagagatacttcttgaaaaacattttatctttataaccgtccgttttacttttttgacagatatatttgactattttgtaagtgaatttttcgacgtcggattttataagatccattcgattgtattgaccactcagtaatgtatataaagacaacaaaaagtcgccaatctttcagcgactttccttactaaactcgattcaattcatttatgcgtcccccgagagtcgaactcggatcatgaggaccgaaatctcatgtgctatccattacactaaggacgccttacatcatttaattatagcgttttctgaatattaatacaacctgaatgttcatgaaaatttgcgggcgactttatcggcttgatcttccaggtaccacatcaactgattgccgtccttttcaaaatcagcttgaaacgactcaccgattggcttaatcgttgtcagcaacttttcgccaatcccaatgacctgaatctcttttccaaccaatttgccagtatcatagtggccttcctcggcctcatccaagtagccttgaaaagcgtcttcaatcacttgcttcattagtccgtccctggtggtttccgggtgacgggctttttcgatggcaaatttatcttcaaattcatgcatgttttctggataatctagggacatgattctacctccacattttctcttacaaccattataaagcaccaaaagcagaaaaaacacggatcttgtttatagaaatccccaaccggcacattctacttgcaattgatgcgtcaatagtcgaacatataaggtgtgaagtgcttacatcatcctaatgggaggtaatataatgacacaagcgatcacggttgaagaatcacgtgaattagatgataaaacgattaacaaaattggcatcccttccctcgtcttgatggaacgggctggcctcaaaatttatgaaaatatgctcgataacaaagatctcgacttaagcaacgttttgattcttgccggaaccggcaacaatggcggcgacggcttggttgttgcccggctgttggccactcatggctatcaagtttccatcttaacggttggtaatccggatcacgccagcgaggatcatctggctcaggcgcggatctgtaactactatcagattcccaaggtcttcatgaacgctgatttcaacaaattcaccaccttggttgatgccctgtttggcagcggtctatcccgcaacgttggcggtgacttcgccacggttatcgataaggctaacgcttcaacagccaaaattcacgccatcgatattccgtccggcttgaacggtgacaccggcgaagtgatgggaaccgccatcaaagcaacctcaacgtcaacggtggcttatcccaaggtcggcatgctcaaagatcaagctaaaccttacactggcaagatctatgtcgatgatatcggcatttatcgtggtaatgcatttgaaaatgaataaatattaatataatattaacttaactagaatcttctcagaatacgtggaggtgccgagatggctgataagaaaacacaaggctatatcaatgttcacgatgttgatccagacatcattgttgacctgaagtacgcaaccagtgataattttactcaccaagtggtttatgactttgaccaggcaatttctcgaattgatacggtcaagaagctcggtgaagccagcaaggatcttaagtcacaaggataccgaatcaagatttgggatgcttatcgcccaacatacgcccagaaacgtctgtttgaggtctatccggaccccatttgggtagccgagccggatcctaacttcagccaccaaaagggcgtgacatttgacttaactttaaccgatgcaaacggtaacgacattgagatgcccaccggctttgacgattttgacgggctggccaagcgcagcatgaaatcatcatggacaccggctgcccaaaagaactacgatatccttaatgaagcgatggagaaagccggctttgagggatacgaaaatgagtggtgggacttccgcgattcggacaaggatcaatttggcccacttgaggtcgatccaaaggattattaaattcaatattaggagtatgtgaaatgaaagttggaattattggggcaggtccaaggggaattttattaacctctcaattgtttaatcaatataaatatcacagtgaccagaaatcaccactatcgatcacgctatttgacccatacggtatcggtgggcgagtctggcggactgaccaatcggatgaattgatcatgaacagttcagctgatcaaatcaccttgtttacggatgcttctgtaacgatgtccagcaaggtctatgacggcccttctttgtttgaatgggccaagagtgttgaggccaaccgttatttggatagcaacggttattcatcagacgtgattgccgcggccgctcaattacagatcaacggctatgcacctcgcgttttatttggtgcctatatcaaatggttctaccaagatttgattaaacaacagcctaccgaagtttcaacatcattaatgaagtcacaggtcatggatctcacttatgataccgatcatcacccggtgatcaagaccaacgatggcacctttacattcgataaggtcatcatgagtctcggccagcaagacaactacctcagcgatgaggaacaaaaattggccagctatgcccaacaaaacgccctgacttatattgcccccactcaccccggtgacgctgatctcagtgacattccagctggtgaacccgccattatccgcggcttggggctgagttttatcgattacatttctgaattgaccctggggcgtggcggccactacatgcaaaatgaagacggcagcctgttctaccaaccatccggcagagaaccgcgaatcattgccggctccggccgtggaattccatactaccccaagccgatcaacgaaaagggttacggcgagtgtgacgtacctaagtttttaaccaaggaaaatatccaaaagaattcaactgatggtaagatttccttcgataagttcatggaacttttactgttagatttaaagctggtcttctacaagttgaccatcaatgataaatacccatacaagagtgcctcggagtttgaaaccgaatttttagccaacgacgataaacaagccgttctcaaacaatttggtttcgccgaagaagacgcctttgattgggattacatcatcaacccgttcaaggatgtccaagcagttgggaccgaagactatcagtcagtcctgattaactggctaaacggcgaaattgacgactccctgaaaggctcaaagactggtccgctggccgctgccagagacttactacgagacttcagacccgcctttcgccaaatgctcgtcgatcactgcttcagtaatcaagacttggttgagaaattctggagtcaactcgactcaacgattaacttcttaatcatgggacccccagtggttcgcagtaaggaattgtcggctctcatccgcagtggcgtggtcacgattttggcacccggcatgcaggttaaaggacaagacggttggtttgtgactgcggcaccgaagcgcaacaccgataccttccgttcagctaccttaattgaggcccgggttcctaaagccgacctcgatatcaccgccaacccagtgctggaaagcctagttgacgccaagctggcaagaacccaccaggttaagattaatgatcaatctgtcggcctcaatgcggtcgacgtggatccaagtaccgaccagttgttggacgctaatggtgccggacaacccgacatttacgtttggggcgtgccgttggatggcttacgctatgtcaccaacgctgcgccacgaccaggcgtcaatgacaccaatttacaaactgctgatcgcttggcagccgaagtactcggactgccggcagctggaaatgttgaaatggcttagttaaaataaatgagatcgtaaaacggacgccgtcagtggcgtccgtttttgtttaacgattaaaaagtctaatcccaaataaccgagcagtatcaccggcagcactgcgaaagaccagtttaatatcaggttgctggttaatcaaggtgactgaaatcggtatcctaacgtgataaaagccttttgaatccgttggctgattctgatcaacggtgaggacttgatcgaatttatgatcgtcgttaaagccaaccacaatggaatgccctgcgtcttcaacattcaaagtaagttccaaggacaagcccggttgagctttgactaaagagaattggtagctgaaccaaccgtcttggtgggcaactctgaagcgtcgacctttggcattgctagcctcagaatgatactgttctagatgcttatcaaattcaaaattgttctgatcaaaattatccagttgaccgactgtttttcgccgatattcgcttaacgcttgcaattgttcttcgcgacgctgagcctctttggagcccgcctgctgccactggaagtaaaccccatatcgagtttcaaaggtttgataataaggcacaaaagtgattgtttcacttgtatttggtaacttcaacttgaatagtgtattcgtcgtctcggtatcgacaacggcttgattgttcaatgactgctgccagtcgtgccaatccataccggtggtcaatgttgatggagatgcgtgatcatgggtactgattcgcaccaacacaccatttgggcgatcatcattgatactatgcttccccagctggcccgcaagaacatatggaccgtacttgaaagctaaataatgcgggttatcctttgtctgcaccatttccaaactcatcggcatctccaagtcaacggtcgttcctgggccggcgttatcaatctcccaaaaatcagcgttttgatccatctgctgcgaaatgccatcgactgccaatttggctgactgaaccaaccaggcagggtttctcaatttcaaattgattgtcccagcgctatcttgtgaccgtattttaacaaccgttaagtgcaccttaccggctttccgatcaacctgttcagtcatctggaggttccttgaatcgagccgtaaaacatttgagaagtacaaactcaaatacaattgatctcctgacctaaagtaataactgtcgcccagcttagtgaagctttcgatgccggtacccgtacagcaccaaaattcatcgaatggccggttatacactttggtgtagccggctgccatcggctgaaaataagtcatcatcccggtgtttggattctgtgagcccaagatggcattggtataggtctgctcataataatctaaatattttttatcaccggtgactcgaaataactcccggctcaatttcagcatgttataagtattgcaggtttcacacgttgttgccccgtcctccaatactgcatcatgaaacagctggccgggttcgtggaaatgctcactttggctattcccgccagtcacataggtatgatcatcaatcacgatttgccagaaattaaccgctgctttcagatacatattgagtgaccctttttcttcagggcttaaatattggtcggcccgtttcacgtcatgaagggattcatagcggtgtaaagcgccaatcaacttgggaatcgtcgtgttggcgtgtttcccagccaggacatcgtcacccttagccagctgtttaaacaacgtcgtttcgtcaaaataagtcgctgccgtcagcatgcgtttatcatcagtcaggtcaaacaattcatacagggcatcgttcatcccaccgtactcaatcttgagcatttgagtggggtcagccagttgattgattcgcttaaagacataaagaccaaattgatgggcacttttcagggccttctcagacagaagtggatcgatattttgaaggttgacgttgaccgccaacagccctgccaagactttatgcaggttgtaccatggcaccaacacattctctttctcatcttttgggacttccctgccctctacctcatccagggcaacttctctgaacgccgaaacgtagccggcactctcaggatgcttttttgcataggcggcttgggcagactggagaccatttacccccaggcgaagcttgtcaagcaattgctgccgaatggcgttatcttctgtagcgagaatcgcttgggaaagtgccgacagataatggccgaaaaaatggccacgaaaattcaaaccatcggtgcgctcccaaccttggtaaccagttacgccacctgagtcgataccggcaacttgatcaaaagttaccaaaaatctttttggatctaacgctaataaatacttaaccgtcatctgctgggcacgggcaatttctggatcacttattgtgacgaatctctgatcaatgttttgttgcatatcccacgccccccttagcgtcttaattgttcagttaatagaacatcatgactgccaattgtgacagttgaccccactaactgactgttatgccacacatcacgggcgtcattttcaattccaatttgtttcaactgcgcttggctaaccataatcggcttggacgatatgttgaaaataccatagtaaacatgatgatcactacgcgcgtaccaaacaatcatttgatcggttctggttaattcaaatttttcagaaattgaattgtccattttcaaaagggttgaatttgtcagtaaactctttgtccaatcatccagatccgttaattcgccacccataatgagtggtgactgcattaatgaccaaagactcatcatcgtccgctgttcggcgtgagtgaagcgggtttgacgattaccgcctggtccatccactgaacggatgccaatatgtcccaaaggcagcatatcgcaatctggccaattgccaggacgggaaattggcgcccactcttccgcacggtcaaacatattatataaaagcggccattcatcccaaaaatcatttgtaattcgccacatattggcgttccgctggaagaacgaaccgtttttaattggtgccggtccgggcgataacgaaagaacaatttggcgtcccgtctgagcaatggcttttcttaaggcgaccacttcatttttgtgcgttttatcatagagctgtgagttggcaatatcatcgcatttgacaaagtcaactccccaggaggcatataaatccatcaatgagttgtaataaatttgaccctcggggatatccatgttgactccatacatatcagaattccaggggcaaatattattcctggcgatctccctggccgacttgtcggaccccttgatggcggttgcttgatggaccgcttgacgtggaatgccccgcataatatgaatgccgaattttaatccaagactgtgcacgtaatcggccagcggtttgaatcctcgaccgcccgatacagatggaaaccggccaggatcaggcaataatctggaataattgtccatgaccaaaggataaaaatcatgatagcgagacgaattggcggtcggttcataccactgaatgtcgacgacgatatactcccaaccaaattgcttcaggtgtttactcatatactcagcattttttctgacctcttcttctctaaccgaggccccgtaaccatcccaactattccagccttttggtgggacaggcgcgaatgtacgatgatgattaattaacatggtgttgtttcctttctactagcgggttccaaattgcttggcgctcactaaggcactgacggaataaggcggcaaaatgagttgatgaccagagaatggtacatttcgccgttcaatttggttgttagcgcccaagtgattttcagcatccggtcggccagacaattgatagaccgagccgttggcaaatcgttcagaatctaccgtgatttcttttggctgcccagtcacattgacagccttaaagtaatactgattggtgtttcggttgtaagtcatattcgtgtacattggttcgatgacggttggagtgatgacgacatcattgatcaactgaccatcgataaatgtctgaacgtgacgatcgtcaaccactaatttgcagtgataagtccggccctttgccattgaccaagtcgtttgggtccaatcagaatctgccttcccatgatgaacacgaaccatcgaatccgtatttgcccaaccaccgagaatccagacaaaccatttgtcactttcctgctgaccaaagcagaagtgggttcccttggaatcctgatcggtcttggtcacgtcaaatgtgatcgtgtagttcgtcgcgtcagttgaccccaattcaactttttcctcatggtcaacgatttgtgaggcaaatttctgcttttgctgaccgtcatccaagacaatgttttcaaactttgcccgggctttatctccttgaacaaagaacttaccgacaattggttgatcatcgacgaccttggcctttggcaaatctttgagttgataggcaacattgtcagttccctgatatttcatgaataactgctgaacaaagtaattcacggttggggaaacttctttttggtcgaaataaatcaaatcagttccccaattttcatagtccacgttgcaaaatagtggtgcgtagcatgccagaccaactttatcagcattgcgctccagaccaatcatgtagctggcttcaaccacagcgttgtaccactgatttgcctttgaggcgtattcgcccaaaaatgccttggggcccttcggatcatatgaatcatatcgatgctgattagccaagaaccactcgggatccatataataatgctcatcaacgagatctgaatgattctctcgcgcggactgccagccacggtcgaattcctttccggcagcaaacggtcctgcggtattaattaatttgatatcgggatacttcgccttaatcgctttgtggaagtatggatagcggtcaaagaaggcctggccaacctcttcgttaccaattgccaggtactccaagtgaaatggttttggatggccgaggtttgcccggatcttcccccatttggtatcagtggagccgttggcaaattcaatcagatcaagggcatcatcgatccactcacccaattgatcgattggtgcttcgcgatcatgatggggatcatagccgccaggaagaaccggcagcggcttggcgccaatatcttcactgagttcaaagtactcaaaatatcccagtccaagagtctggttatacccccagttgttccgacgagctgggcgctgctcaactgctccaattgaattcttccaacgatacattgccccgcggtcatctggatcaagctgtccgtcgtgaacgaggcagccaccaggaaaccgcaaaaatttcgggtgaagggctttgagtgcttctccaagatcttttctaacatagttctgtcgatggttaaacgtgtcgtcggggaacagtgagatcatatcaatcaagagatgggtcccctgttcgaacttcaaagtgagtcggccttcagtggtcgtgcgatcgccaacgaaagtcagggtatacttgagccattgatgactttcgacaggaatcaccgttgggacggcaacgtcatctcccgctttgtcagtcaagtggacgttgacgtctttttgcccattcagtgttttggcaaagaatgaaaagtgatactttttcccagcttcaagatacatcccctggttaaagccaaggttggtcagctcaacgtcttgtcgggcgttgacttccaagtagtgtcgattcttggtgttcaagggatctttgtcgtcaactttcagactggtcggatcgcttaactgccaagcggtcgttggctggtaagcgtcattatcgatcggggcaaattcaaacgagcggttttgaaccatctcggcgtaaagaccgccgtccgcggcatgattaatatcttcaaaaaagattccaaataaatcattgagagctgccccgaatttggttccagggacaagttgtgaactattcaatatcattacctctttctaatgaactgtggatgcaacaaaaggatgaacacacagcgcatattcatccttttatcagcaaaactatttaacagatttaattctaaagattaagaacgcaccaatcaattcaatcacgaatgaagccgggaagattgctttgtatccaccaagataggtcacaatcagcgaagcaaccacggttcctgaaatttgtgagaacgtattggccaggttaatgaaccccatatccttaccagaagtttcagcatttggcaaaactgccaggttcaaggcaccatcaacggcgttataaacaccattaccaatggcagccaaaacggcgtaagttaagatggtccaaggcttattatcgaagaatgggaagaattgtgcaatcccgatcagtaacgttgataatgcaactggcgccttcaaacgaccaattctatcagcaactggtcctgaaattgcggtgaagataaccccgaataccaggttgatcattgaaatttctgacaaggtcttcccagcggactgctgacctaaatgcatatagtcggttaaaatatagagcatgtatgcagtggcaattgtaccacccataaccatcattaattttccggcaacggcgtaccagtaatctcgcgcgccaaccgttggcagtgaaaagtgaagccacaaagctctccatgagaatttttcacggggttcatccaagttgctgccttcatgggcgaatagaacgtgcaaaatacccattacaaagccactacctgccatgacgtacattcccattttaggattacccaggaattgagcggcaatcatggtcatcacttgaatggcggtataaccaattccatacagagtggaaatggttccccgccattttggtgcaattcggtcagcctcttgagcaaccatggcagccgcaacggcattttcggccgcagcaacgaagccccaaataacaacaattgcccaaagatcatgcaagttggcaactacacaaattaagccggattcaacaatggttccgccaagaatccagggctttcgtttaccccaacgggtccgggtaatatctgataaaccaccaaataaaatgttggcaatcgccgcaacaatggatgatactgacgccataatcgcgatagcggcaaccttaccacttggatcaatttgactgaagtactgtggcagtaatgtgtttctgacgttaccagccggtgccagccatacgaacggtccaagcagcattgccagtccgaaaagcttcgggaactttggctgttctgcattggttaccttggcgttggttggttcaggcactgattcaccggcctttaaatctttttcatctttctttgacatctttaaaccccctatgggaatcaatttatttagaaatcgttttcatttatgctgataaacgggatcgagcgaccctatttcaaagtgacactgacgacacttttggctggtaatgccaagtgaagcgttccatgcttcaattcagcaccgacaaagtctttttcaactaccgcgtctggattgtcgaatgtattgtgagcatccaacttatcagccgtcagaatcttgccggatttcactttcttgaaatcagcgaggccgctgaagtccacattctgggcttcatgggcatcgtagttacaaattgaaatcgtcagcttgtcatctttttgtgaagccgtataggtgacgttctcaggaactgaaccgacaccctccactaattcaccattcatgtgcttttgatacatatcgaagacataataggttggcgtcttcagcatctgatcacccttggttaaaatcatggcttgtaacacattgaccatctgagcgatatttgccatataaacccgatccgcgtgcttttgaaaaatatttaaattaattgctgcaaccattgcgtcgcgaatcgtgttttgctgatgcagaaatcctgggttagtgcccttttcaacattgaaccaagtgccccactcgtcaacgattaaattaacccgtttatcaggatcataccggtccataattgtggaatgcttggtgatcaattcatccatgtgtttggcacgggtcatcgtcgaatcccattcagattctgggaagccggtggcgtcacctttgctttgaccccaggttccctttggcaaagtgtaataatgaagactgatgccatccaaatattgaccggcatacttcatcaccgtatccgtccagttgtaatcatcttcatttggaccgcaggcaaccttgtaaattggatgatctttgtcatactgaggcaaaaacgtttggtactgacgataaacgtctgaataatattcaggacgcatattaccgccgccaccccacgattcgttaccaattccgaagaatttaactttccaaggatcctcttgaccattttgtcggcggaggttggccatcggtgattcacccggcatggtcatatactcaacccactcagccatttcttgaaccgtcccgctgccaatattggcattgatataggcatcagcacctaattggttcagcagttcaaaatactcatgagtcccaaagtgattattctcggtgacatcaccccagttggtgttgacgatctttttacgatcatcctttggtccaataccgtccatccagtgataggtgtcagcaaacaacccgcctggccatctcaatacaggaacgtgaattttcttgagggcatccacaacgtcagtccgcatgccgttgacgtttgcaatatcagaatttttgccaacatagagactgccgtagatcccatttcctaaatgctcagaaaattgaccataaatgtatttactgatttgtggtccttttttctgaggtaaaagttcaattgtcattttcttcaacctttcatggtttactgtttcttattaacatatatgttaatattcaaacgatgcaaattgttaatgtttaccggtaaaagttttaacgcttttaatatagcgcttacaaatcccaatgtaaacaagtttttactaaaatgttgaatattttttcctatttagtataatgattaaggacgagttgctaaggagcttcattgagcttaagatagtaatataaatgttaacaagaattagaggtaatcatatggaccttgatatttcaaataagtcgctgcccatttttgctgctttggacagtcaggtcagaatcaaaatcatccgtttactttcagaaaaaaagatgaacgtctcacaaatttctaaggcaattcgcttgagcagcccaattaccctcatgcacttgaagaagctggaagacgcccacatcatcaagacacaaaagaagggcaaccaacggatttgcagtctccagatcgatacaatcaacgtcagctttccgcaacaactctatattccttatgagaattgggatattgagctgccaattgggcaattcaccaattttgatgttcagccctcttgtggcttggcgggtcaaaagggcttcatcggcaaagtcgataaccccagttatttcatggaccccaaacgttatgaagctgggatgctctggtttgccaagggatatgttgaataccaggtgccaaactacttgaagcctgaccaggaactggaaatgatcgagttgtcgatggagttaagctctgaatttccattttcaaacaaccgctggccgtctgatattaccattagtctggatggcaaagagattggtacctggacgagtcccggtgacttctctgatatccgtgggcgctacacaccggattgggtgtataacgacatgaatcaatatggcatgctcaaatctctgcgtgtttccaaacacggctcgtttatcgacggccagcattctgcggatacgacgattaatgaattagacaccaccaagaattcgtggacgctgcggattggggttaaagataacgccaagcatgccggcggttgtaccatttttggcaatcaatttggtaatcatgatcaggggattaagggtcggttttattttagtgaaaattgacatacaaaaagctgtgacggcgataatcgctaccacagctttggttgtccctgctattttgaggacggcgactaagccccagatccctccgcttaaaaaagtagtcgggtgtaatgcgcaagaaacgcgcatcacacccgactacttccttaatgctcgggatctcccgggggtgctgttattttctttggttgtccctgctattttgaggacggcgactgacccccagatccctccgcttaaaaaagtagtcgggtgtaatgcgcaagaaacgcgcatcacacccgactacttccttaatgctcaggatctcccggggcttagtcgcccactacatgcataaacgacttatccggaatccgaattaaactaaatcgatcggcctgccggcctgcatggagtccaattccattgaaaaagttcttcttatacgtcgttgtcaccgttgccacccaggcgtgctggtaacgcgtatcaaggtgatccaggtattccttattccacttgtaggtttctgcttggacattcagattactcttgccatacaccaccgtggcattcatgctgttcaccaagtatttaccgccattgacataatacgtatagttttgaatcggctttcgaccattgccatttctaaccgtcacgtagtccgattgatcggagcgataacggataatcagtggtttgtaagcataactggtggttgttcgattcgtgtccaattttttgacatcttggaaaaaggtcgtgtacgacatcccccacaaaaacagcaggaaaattgccacttcactacacgaaatccaaaagttacgccacgtgaaactctttttttcagtcacgatcaagcgaagccgacgcgcccgcatatcgtgaataatataagcaaagtaacagatgagaagcagccaaagggccatcccaactaaattccaggcggatttcataatcattcccctttttcttcttaattaatttaagtttacactagtttattggtgagtgcgagtatgagcaaagataagttgaataccattctattgcccagccagcgatgctttgtcataatttccattcaaaatcgtgttatatttaacttgtatgcgattccatcaaaactaatcaatgaggtgacaaatcatgtgcaccagcttaaccctagaaacacttaatcaacatgtcctcctggcacggaccatggacttcccggtcaaagcggcttggaaaccggtcctgattaaccagccaaattatgtaaccgctttatcaggcacccggctgatcaaatatccttacattggcggcggccgcaccgaagaaaatgacaacatcctagtggcagacggcgtcaacacccaaggcctgagctgcgccgagttgatgtttcccctgaaagcccattacttagacaatgaagtcgatgacaagctcaatttgacccctcaggatttcttaccctgggtgctgggagaacacgcttcactcaaagaagtcaaagccgacctcgacaacatcgccctgattggcaaatactggatggccggcaaagaagtcttttcatttcactggattctgactgacaaatcaggtcaaacactgatcctggagccaacggttgacggtttggaagtcattgaggactcaattggcgtcatgaccaactcgcccacttatccggaacatatggcccgactggaaaagaagctgaaagtgaccaatcaacaggccctggccgcaaaagcgcaacaaatcatcatgagccaagacctgcccaaagcaaccaataccccaaccaccagatttttggtggccgcggttaacaaactcggcaccctgcccagtcggacccagtacgaagccagaaatcgcctgttcaacgttttggatgaagtggcaattccctacaagccgtcaatggacgaccatccaaactttaactatacccattatatttctgtgttggattcaaccgaccagacctattattttaggtatcacgattccagacagctgttgtccttctcgttaactgatctggtcgaagaataccccaacaccagccgcttcttagcttaagtagtcagcgatttttcgttggacgccctgctcattattggaataagccgtcacctgctcaactttttgaagcaaatcagcagcagaattcttcatggcgtatccctcaccggctgcgttgaccatttcaaaatcattgccgttatcgccaaatgcggcaacatcggccagagtcaggccccaactttgcaggagcatttgaattccggtcagtttgtcggtaccgtcaaccatgacgtccaagccgttcatcccagaagaaatggcgttcaactgaccgctgaatttgtgattgaattcatcctggcgcttgagcacaccgccttcttcccaggtaatgtcgagcttataaatcgagtcaaagaccaaccgcaaatcagccatcgactgcatgttttcgtagaaatatttggaagcctggaagcgatcggaattctccggtagattgcagtacgtgccgtttcgaccgactaggatcacttcagcgccggcaaaactgggttcgcttaaaatccaatccagggctttcttcaagactaaatggtcaatgatctcttcgtggatgatcacccctcgttcgtcgatgactaatgcgccgttgttacaaacgtatgagatcgggccgtgaacatttttgaacagacccaacagatgctggtattgattactgctggcggagatgaagtgcatccccttatcgcctaattgatccaattgctgttggaactgttgctcatcaaaagttccctgatcattcaaaaatgttccgtccatgtcgcttgcaatcactttcaccacaatgactcctccattcaaatttcgataattggttatactctcattttaagggattagtttggtttgtaaattaattttatatcttgtatactgaatttgatcatacaactatctggggtgccttattggctgagaaaaacccatcgaacctgatctggacaattccagcgaagggagcatgctccgttgtatttagatggataaattgcaattagatgaatttctgaggccagggcaaaacgaccagttttgtgcctggcctctttgtgtgctcagcaattggactttcagtgacttatttgatcaaaatcatatttggaggtcttgttatggataacaagagtcaagcaaccggcggcaaaaagcaaagccaatggacgcttagaaacattattttaattgccttaattgctatttttactggtattattttttggggagccggctttttatacaccggattgactgttgccctgaccccatttggaatggccccatttgccaacgacctgttgatgggcctgtggtgcatggcgggtccattaaccggattcattattcgcacgttcggttcggccttcctgggtgaattcctgggggcttcggttgaagtcttccttggcggtcaatggggcgcaggcgcctttatttccggcttggtccagggaattgcttctgaactcggtttcacgctgaccggctacaaacgctatgactggttcggattgaatgcctcaatcttcacaacggttgttttgacatttgcctgggacatgattcgaaatggttatgacaaattcagtctgccactgctcttgggactattcgtcacccgttatatttcaacctttatcttcgccggtgtcttgaccaagatgattgttaaattattggatcgtagtaaagcaattaacttgtaattataggggatttgatcatgactgatgtttcaattaaccatttcacttttcactatccacaaagcgacgtcaaggtcttaaacgacattaatctgaccttcaagagtcatcatttctcactgctgtccggaccatccggcagcggcaagtccaccttactgtactttattgccggcctgtacccgcattttatcgggattgatgcagtcggtgagatcaaatttggcgataccaacatcaaggatatcccccgggaaaaaatcagccagtcagtggcgatgatgttccaaaatcccaatcagcaattcgcgatggacactgtcgttcacgaaatgacgtttgtcttggagaacttgcggattgcgccggataaaatggacgacatcatcaacgacgccctggaattctgtggcatcaaacggctgcgttcgcgggtgatcaacactttgtccggtggtgaaaagcagcgggtggctttggcctgcatcgttgccatggatcctcaggtgatcgtgttggatgaaccgtttgccagcattgacccggggtcgcgggaagatttgattaacaaattaaaattactccaacaagaacacggcaaaaccattattttagcggaccatgatttgaccagttatcggggattggtggatgaattctactatttggatccggatacccatcaaatcagccttttggatgaccaacaagctgaacatttcttcaaaaacttcgaatcaactcaacaaatgcacaagcgagttgagattcccactggcgatgaccatgcgattatcaagctcagcgattttaaattggagccgcacgcctctctgctattgaccctgaatcactttgatttttacaaagaaaaaaccactttgatcaccggtgccaatggcattggcaagtcaaccctgtttaacgcgttgaccaacctgctgccctataaagggaccatcgtctttgacggcaaggatatccaaaaaattcggccactgccgtatgcgaagaaagtgacattgttgttccaagatgctgagaaccaatttttgaacatcacggtcaaagaagagctcgatttatcactcgccaaccggacgaataccgactacacgcaagcagacgttgatgacatgctcagcaagcttgatatggccggcaaagacgaacgaatcgtgtattcgttaagtgaaggacagaagaagaagctgcaaatcattgaaatgttgatcatgaatccgccagtattattaatggacgaaccattcaaaggcttggactatcattccctggaagtcgtggttggtttcttgaatcgggccaaaaccgatttccatcaaacccagattatcatttcgcatcagctgtccggattggataccctgattgattatcacgccgcctttgaagaccaaaatctgacttaccaggaggttatcaaatgaatcctggaatgaaattattattggtgatgctgattgcgttggaaatctcatttacccaaagcttaatcgtcaacatcatcctgatcaccatcagctttttatatattctcacccaacacgtcagtatgaaggccttgtttgggattatcttctggccactatttcctgccgttggtctattcgtttctcaatggctgtacggaagtgccggcatccattttgcctggattctgtttacccggatctatgcctatgtattcctgggggcaaccttcacgttgaccagcagcatcaccgacctgtcgttgaccttggagcaggattttcatctgccctccaaatttgcctatggcgttttggccgcatttaacttaatgcctaaaattgctgaagaagtccgcattatcaagacttcggcattgatgcgcggcgaggcactgcatttctggtcaccgaagctgtactttaaatcaattctctcgtcaatccaatggtcacagaacttggcagaagccatgacctctcatgggtttgtcgaggattatgaacggacccactacaaggtcattcgcatcacggcaattgattgggcactgtttgttgtcctgctggccgccgttcaagttttgctattctttatcaaatactaaacgccaatattccaacatttccttttttgacttataattatgtaagagaaagatatattggaagaaggcgttttttatgcgggcaaatcaattcgcatttgcgtttggaatttttgcgttaatcgttggaattattgttgatatttatgggttagtcacccaatttggctcgctggacagcgcccaggtggtattgatcgggtcaatcattttggcaatcggcctggcattcttgtccctgccgaaccgctgggaacgatatgccggccagttggtcgttggccttggtttactgtactatttttacattcaaaccaacaaatggtgggtggcagtcatcatcgccattatcgccatggccttaatggaatatggactgaaacatcgttaaaatgtgtcaaaatttcaattattggtataatagatttatagagcaagttggatcacgaattttgatggaggagaatgacgatggcagaaaaatttagtaccttagcggaagaaattattaattatcaaaagaagaacgatatgcccgacacagcgttagcatttaacctgcacatatcagttgaacgcctccacaatatcaaatcaatggaatcggaccccacaccggacgagaagagaacgattgagcagtttgtgcgttagagcgcgacgagacccggttagggccctgaacataagtgagaaaaatcaatgatgaacggtctttgttcatcgttgattttttttgcttatgtggctgggtcctgggtcgtcggagcgtattttaaaagctgaaggatcctcaaaataacataaccacaccatggcgcgacgagcaacgggtgaggcggtttctaagggtactttgattgaagtccctgggtttgggactttaattaaagtgcacttagaagttaccctcagttgcgtcggagcgtattttgaaagctgaaggatcctcagaataacataagcgcaccagagcgcgacgagacccggttagggccctccaattaggctaggccgttttcatccggccgtcggaacataagcgaaaaatttcaacgatgaacgttttttgttcatcgttgaaattttttgtttatgtggccgggtcctgggtcgtcggagcgtattttctacctatagtcaagttataccggcaatttaagaccattctttttctgtcgggcatggctgtgccgtaaattaattgtttttctggttaggtaaagtggctttgagggtaaactaaataagccttaacaatttaatattttttacaaggctggtatgattatcgtaatcagatttatgactcagcttttggtcgagttttgagataatcgtatttctggttatttaggatcaagtggtaaatagtccggttaagacgactaattgcacccatggcaatcttcttgaaatcagcctttccagaagattgctttttcctttcccggcaataatcattgatgtgggatggctttgtgcgagcacttaccatcatattgagaattgttcgatacagaattttgcgggcatatggattaccacgcttactaatatgatcgacggcgatatattcgccagactcaaagtgtctaaggtcaatgccgacaaacgcgttcagtttgttggcactcgtaaaccgacggatatctcccagttctccaatcaggcggactgctgtattaacggaaatacctggaatactttccaaaatggccaattctggcaagtcttgagctaatcgagccattttttgaatgatgtcatttttcaagtcatctaatctaagtaactcggttgccaaataacggacctgcataaccactccagagtcttccccaacacaaggataggactccgaggctaattgacgtagccgagcggctaaagcttggctatttgggacagataactggcagaactttctgatatgctgacttagttccattgaactactttgtcgcaccatgctcgcaatcgggaacgcttgtaaaaggtgccaatataagtgccctgttggactgttaagaacgcccccagcttcgggaaatgtacactgaagggctttatgaagtcggttcttatttgcgactgagtcacaagtaatctcatcataaaagcgactccaatcaagtaactgctggtatattggatcttgctgataagttaaagcacgcctgatctcaaactgagtttcagctaagtgtaaggcatcatttttgtcagtcttattaggacggagtcgatcaagctgcttctttgaggctaatgggttcaattgagtgtagcggtaaccataatcatctaggaacactcttaatctccttgaatataacccagttgcttcaaaaacaatctcagggttttgaaagtcattcaaacttttttggagtttattaaatcccggctgattatttgtaattttaaaatggctaaccgcttgcccattaacgactatggcaatttccgaagttgctttactgacatcaattccaaacgttactcgcataaaatatcaccttacctttaaagttgttgcttcaagtcttatataatctaattttcaatacacgacgttaaacgccaacagacttagagcagatttgtataagaacagtgaagttagccagttttagagacggcgtccagcgccaaatatgctcacggcattactaacttcacaatcactttataccaaaaagtgatgaactaaagccccgtcgggttttaattcatcacaagcttagtctgttttaaaggccggagggagctcagaaaaacataataaccgtgcatttaaacgacgagacccgagtgacgctaccaaataggctaggctgttttcatccggtcgtctaagtgtattttacaagaggaagagagacccaaaaatcccgacaaccgttcccccgagaaacaaaagaaaccacaaacgaaaaggaccgaagcagactcgcttcgatcctatttttgatgcttctcattcttctcggcccgataccggctcatcccttctttataaggattgccaaacaaccgactcaatcccgtccaccaggaattggtacttgacggttgagcatcatcgactggcaacttcttgccacagttcagacagacaacgtcatccggcttcaacttcgccccacaatacggacaaaatgaaaatttttgctttgccatcttgcttacctcgattgctgttggcctttgttgcgattggcattgcgctgacgccgtttttcggcttcagcttgttccttggcagccccagcttggcgaatttgttcttcacgttgctttttagctttatcttcggcaataatttggttgtgcattacattcatccggtgcgacagaaagttccagccgccgattaaaaacagagcgccgaccactgagtacggaaatgtccaccatggaaaataactgccttttttgaaaaccattgggccaagaaaattatagagtgccatcaatattgcgaccatcaaagtcacctgcagggtattgaccagccacttgggcatcttaaatccttttttctttgccaccatgcatccccccctaatcaatttcattttcagtcagaaaggccttgaaataatcaaaggccatctcgcgaatattctcgatgccaatttgtcgggttggcaaatcaccatcgtcatcaacgtctagcaattccacattcaaaactcccgtttgcagatcgattgaggttggatacccagcaaaattgtcctcatcggcagtttcaaagcgaatcactttttggtactgaatcgattgggtgatgatatgaatcaagatgttgtccgcgttatcaaatgcccgatccgaattcagaaccggcaacgcaaaatgcttgttgtgtttattctcaatcacaaatttatcgatcacccgtaaataatccgagtccgtaataattctaccaatatcatcgtaacgaatccagacgtaaccgccaaatcggccgttcatatcgacaaccatcatgacaaattctttttcgttgctggaaataatcttgccaacgtaaaaatacttccggttatcattggtgtcaatcacgacccaatccccgctgttacgcagttgttcaatctgatcacgaaagacacttggatcaacaatgatctcattttccacatgattttcaggcttgaccatatctaagacgttttgcagcagttgtagttcagtcccaccaaactcaataccacgaatatcatcaaatcgaatgttgaacaccgactgctttgagaaatcaaacttattaatgttagtaaagaccattccgtcgtcttgaaggtccgaaatgagcccttcgttgtatttcagcttgccggcctgtgcggtaatcaccagaccaactttttgatcatcctgcaatgtctgaatgacccggtcgaacaacgagtcgctcatcttgattggtaaatcaaaagagggctgggaattgaggtggtgcttctcgtcaaactcaattcgatcctgcatgtttgccaagtcgtaactgtcggtatcaatggatttaactgaagaaatcttcaaataaacttcaccatcctgaatgccgtaatcgttgtaggtcaacatgatgaaatctttatcgcttaaaaactgaatgacaccggtgtaaacgatatcggagtcattttgaaaagcgttaatcagctgctcgtcgatttgggcggtacgcagcttgtcgtatagggttttcatggtgtcacttctttcttgggtgggttagttgtttgtggtcttgtttgtggcgcttgcttgtggtcgatttgggtttttaaggtttaattttctctagtggaaatgtgctccctggggcagtaacctgcatctaaggaacttcgaacgaaaatcaaactcgagttccgttcgaagcaccttagactccggttactaaccgccccagtccgcactctagtgaaaatacgctccgacgaccctggtctctactgcgtaagtcaaaaatttcaacgatgaacaaagaccgttcatcattaaaatttttgacttacactccgggaccacccaggtctcgttgcgctctctacgaaattgcattccccataaattccctaagttcatcacccgacatattatcactcaatccaactaaaagcttgattcttgctttctggccgttcaatccttgacagagaatcgttcccatcttcattaattggatgcccccaccctcatagtcgtagatatcctgggcgacgccgttataacatcttgagaccaagacgattgggatatgattatccaataatcgttggatcgccggtaaggtctgcggtggaacatttcccgctcccaatccttccagcaccaatcccttggtattgtcgttgttgatggcatcaaacaacgtgccgtccattcccgcatacgccttaatcaaatagacgccttcgaccacctggttgatgtcacacacttcggtttgaattaattcctggaagtattttgccttgttttgcgttacaatgccaattggtccgaaagttggcgttctaaacgtcgccacattggtagtatgcgtcttggtcacgtatctggccgtgtggatctcatcattcatcaccaccacgacccctttgccgtaggactcatcagttgcggcgaccaggatggcatttctaaaattgtacaggccatccgagccaatttcattagatgatcgcatggcacccgtcacgacaaccggaattgtgttgggcagcgtcagatccaagaagtaggcggtttcttccaacgtatcggtaccgtgggtaatcaccacgccgtcgacaccgtcatcaatcgccttcataatacgctgcttaatttttaacatcacctcaggagtcacgtgaggagacggcaggttaaacatttcatcagtaattaagttaatctgaccctttaagatcacttgttcttcggcaatcgggttctcatcattggggacaacttcgcccttttcgttttgggacatcgaaattgtgccgccagtatgaatcgcaagaattgttttcatcaatttcatcctccatcaacctgttaatctataccattgtaccgtaaaatggaacatgaataactatcaatcaagaaagaagtctcagatatgccaaattccgaccgctactatacgccgcaaaattcaaaagatgcgatgcgccagatcgaaaaactatttaataagtataaggacgccccactcacccaagaactcgtcgactaccatcagaatttggtgaaccgcttaaagactgacattctggcagctgccaagcaggaaaacgttcccgccagaattgagtcaatcaacacgatgatcgccgccatggagcgttggttaaaggtccgcttggccggcaatccctataacggcaagatgaagaactttaaatttgtcagtgatgaatcactgcctaagttcaagcgccacgtccacaagatgaatggcggatcgacccaccgttcttcaagacattaagactttctctttgtaatctagactattacattgcagaaacgtaggaaataaagcagtttccggccatataagcaagaaagctaaatatcccggcccgggatatccgactttcttgcttatattctgggaactaaccgcttcatttcccactctcaatcgttataattaatttatcaatcatattagggggaagaccgttgagcaaaaccattgttgaattaaagaacgtctacaaaaagtacgacgacggctttacagctctcaaaaatattagtttcaaattacaggaaggcgaattctacacccttcttggcccctccggctgtgggaagacaaccatcctccaatcaatcgccggctttacagaagtcacatccgggcaagtgctgtttgacggcaaagagattaacgatattcctgccaacaaacgccagctcaataccgtttttcaagactacgccctttttccaaacatgaatgtgtttgacaatgttgctttcggcttagtcgttcataacgccaaaaaagacgaaattcagacccgggtgcacgatgcactcaaaatggttcagctcgaacagtacgccactcgggaaatcagcgaattatcaggcggccagcaacagcgaattgcgattgccagagcgattgttaatcggccaaaggtattgttactcgatgagccgttatcggccttagacgccaaattacgcaaggatatgcagtatgaattgcgtgagcttcagcaaaatcttggcattacctttttatttgtcacccacgaccaggaagaagccttggcaatgagtgatgaaatctttgtcatgaacaagggcgaaatcctccagaaaggttcaccggtcgatatttacgatgaaccgatcaaccactttgtcgctgactttatcggcgaaagcaatatcattcccggtaaaatggtggccgattaccaagtcgcctttttaggacatcaatttgaatgtgccgacgccggcatgcggcccaacgaaccggttgaagtcgtgatccgaccggaagacctggtcatcactacgccggaaaaaggcaaactgcaggtcaaggtcgacactcagttattccgtggtgactactacgaaattcttgcctatgatgaggccggcaacgaatggctgatccattccaccaatgccagcacggatgatgcgattatcggcttgacgtttgggccggacgatatgcatatcatgcgttataacgaaactgaagccaagttcaatcaccggcttgaaagttatgaagagtagggggggcggaacatgaagcgaaattatcgggggctttttttcacgccttatattttgtggctgacaatgtttgtcatcgcgccagttgccctaatcatctattattccttttttaatattcacaaccattttacttttgccaactaccaggaattcttctcgtccggaacgtatttgacgatgacggccaattcggtcctctatgcctttttgatcaccctgttcgcaattttgatcagttatcccatggcgctggtgatcagcaaattaaagcaccgcgacttgtggatcttgttggtgattttgccgacgtggattaatttattactgaaggcctatgcatttatcggcctgctcagccacgatggcttagtgaatgatttgttccaattctttggcatccctgcccagcacatgctgttcactgacgccagcttcattctggtcgccgcttatattcaaattccgtttatgatcctgccaatctataactcattgactgacatcagcgattcctacatccgcgccagccgcgatttgggcgccaccaaatggcagacactgaccaaagttatcattcctatgaccatgccgggaattaagtccggtatccaaattgttttcattccatcgctatcactcttcatgctgtcgcggctgattggtggtaacaaggtcatcaccttaggaacggcggttgaggaacactttttgacgacgatgaactggggaatgggttccacgatcggcgtggtcctcattatctcaatggtcatcgtgatgctgttgaccaacaccaagcgtaaaaggaggcggacatcgtgaacgataaggcttccagaaccggtaaaatttatatcaccattatctttttgctattgtatattccaatcgtctatttaattctgtactcattcagtaagggcactaccatgaccaatttccaaggcttttcgctgaaacactacggtgaattgtttaacgacaaacggatgctggcaatcttcttgaacactatcctgattgctctgctgtcttcggtctgctcgacgattatcggcaccatgggggcactggccgtccataatgccaaacgccgccacgaacgagaagccctcctgtcgctgaacagtatcctgttggtctcacctgacgttatcattggtgccagcttcttgatcttctttaccgccctcaagctgccgctgggattttggtcagtgctgttaagccacattgcctttgaaattccaattgtcctgctgctggtattgccaagattggacgaaatgagcccgtcgatgaccaatgccgcgatggatcttggcgccagcccggcccagattttaagtaaaatcgtcctgccttacattcaaccggggattattgccggcttcttcatggcaatcacctattcgttggatgacttcgcggtcaccttcttcgtaacgggaaatggcttcaccaccctgtctgtggaaatctattcaagagcccgccaaggtatcagtttggaaatcaacgcattggctggtatcatgttcatcttctcgctcatcctagttggcgtgtactattggattgagaccagaaacactgcctcgactggtaagaaaccaattgtggaggtgactgaccgatgaaaaaatttctcgcagcattgattgctattctggcgttgtgtgccggcttggcttatggcagtaatcagctcaccaaatccaccggcgataccggcaataaggtccttaacctctataattggggcgattacatcgatcccagtcttttgaccaaatttcaaaaggaaaccggctaccacgtcaacgtcgaaaccttcgacagcaacgaagcgatgtacaccaaaatcaagcaaggtgggaccagctatgatctcaccgttccaagtgagtatatggttgaaaaaatgaaggccgatcacatgctgattccactggacaaatcacgtctggttggcatgaatcattatggccgctcatttctcaacaaatcctttgacccgcgtaacaaatactccatcccctacttttggggaacgctggggatcatttataacgatcaatatgtcaaaccgggatccttggagcattggaaccagctttggagcaagaaataccgcaatgatattatgctgatcgattcggcacgggatattctgggcttttccctcatctcaatgggccagtcggtcaatacaaccaattcagctgaactgatcaaagctaaggataaactcaatcgtttgtcacccaacgtcaaagcggtggtggccgatgaaattaaaatgtatatggcagagggtgaggcaccgatcgccgttgactggtccggtgaagcatcggaaatgatgtcccagaattcgcatctgcactatgtcgtccccaccgaagggagtaacatgtggttcgacaatttggtgattccaaagactgctaagcattttaaggcaatttacgccttcctgaattttatgaacaagccggaaaatgccgcccaaaacgccgagtatattggttattcaacaccaaacatgtcggcttttaaactgctgccaaaggccacccgcgacgataaacagttctacccaacccaaaatgtaattgaccgactgcaggtttacagtaacttgagtccgcagaaagtccaagaatataacgatttgtatttggaattcaagatgcaccattaacccggattaaattcttaattggtctttgaccgccaaatgcattaaactgataacgaggtgaaaataataatggcaaagaaaaacatgcgacaagaaatcatcattgatatggacgaatttatcgtcacatacgcagcaaccctcttggatccgaaccagaacctttccgagttggtgtataacacagcaaaagaagatattacaaagtgggacgacttgttccacgaccaaggatttggtcgcaaaaataaatttatcaacatcggccgaggctacttaagagatgcccaaaacttggacgctgaagaggcggaaaagcaaggcgaccagttagcccaagaagccatcgattacttgggaaagcacacagacttttttgagaagtggagaacagactagagcgcgagaagacccggttagggcccagaacataagcgagaaattccaatgatgaacggtccttgttcatcgttggaatttcttgtttatgtggccgggccctgggtcgtcggagcgtatttcagaagccgaagggagcgcaaaatgacctaacaaacgcgccccacgtttcctaacataaagagtaagaaatccattgcaccccaaaagaacgcccacaagctttttccaccaaaattccccaactttgcgtcataatagacctaatcaaaatatgagaattctggggggaagggctcaaaatgaatcacacacctgcacaatcaacgacacaaaaaaatggttggtggattttggtttccatcggcatgtttgcattcatgtcgaacctggattccagcatcgtcaacattgccatgcccatcatggccaaacagctgcatgtcccgatgaatcaaattgaatgggtggtttcgtcatacctgatcgtcttaactgcactcttgctgtttttcggtaaactcggcgatatctatggcaaaatcaaagtctttcgaatcggaacagttgtcttcttgcttgggtcatttttgtctggcctgcaaattaattttccgttcctgctggtcggtcgatttattcagggaaccggagcagcgatgaccttatccaacacttacggcatcaccacctccacctttggtattaaggaacgtggccgggcaatgggctttgttgggaccttcgtggctttgggggcaatcgccgggcccggacttggtggcctgattctttcaaggctatcttggggctacattttctgggttaacctccccattggcattatcgccgtcattctgggcgccattgtaatgcccaaggcttatcaaacggtgccgggaaccatcgattggctaggtttcatcaatttctcactgatgattatcggcttgttcctcggtgtcttcatcggccaagaacttggctatgggtcgccaattgcgctggcattatttgcgttagggctcatcaccatgtggggctttttccacgccgaaaaacgggccaagaatccattgatgccgctgtctttgtttaaaatcaagccattcacttatggcctcggggccgctgttttgatctttctttccaacttcttcaccgtgatcattgtgccgttttacctggaagatgctcggcacttgtcagctggtgaagccggcgcattgctgatcattttcccggtcgtcatggtgtttgccggcccgtttggcggttggttggctgatcacttctcgccagccgcaactgccactggtggtctgttgatcgtcgctgtcgcccaagccatgtatttcttcttaaccctaaccagcccaatgtgggtctacgtggtcatcacgatcattatggcttttggcaccggcttgtttcagtcgcctaacagcgatatcgtcatgtcagtggttcccaaggattcattgggaagtgccgggagtttgaacgccctggcacggaatgttggcatgatctctggtactgccttatcgaccagtgccctatttatcgcaatgagtgtcaaagccggattccatgtcaccaactatttaccaaaccagccggaagtctttattttcggcatgcacgttgcctttgcggtttcactggtaattatccttggcgcctgggtactgtcaatcatgcagggtcgaaccgtcaaacctggtgatttgaaataaccaattgatcagttaaaagatccctaaattttaccgataacgaagcgctttgattatcatcaatctttgtaaatagtccttaaataaaaagtgagacccggcgataagccggatctcacttttttgcttacttaattttagttgcttgtcccttacgcttccgatactcaattcttcccagcttgataatttcggtcacaaccagcacgataaaccctgcgatggttggtacaacccagccatagaagaagtcgatgctgccagtgtggaagacgtcttgcataaacggaatgtagaacatagctgcttgaagcgccagcagaattccgatgatgataaacgccatcttgttctcgaagaaatgcttggaaataattggataggagttacgaatattgaacagatagaaaatcttaccgaagataatgatgttgaccgccatggtactacccagaacagccgtcaagacaccagaatcaacaaatcgatcgaaggtgaagatgcccagggcggaaattaaaatcgatacgtaggtgatttcgaaaacgtccatttttcctaaaatccctttggcaacatttcttgggccacggatcatgattgactcctcagccggttcaaagataaacgcgaattgaatggtcaatgctgaaaccgtgttaatccacagcagttgcgttgggaacaacggcaactcttgtcccataatcatactgatcaggacaaccagaccttcagcaaaactggttggcagcaggaatcggattgtcttttgaatgttatcaaagacgtgccggccttcagcaaccgcatcaacgatggttgtgaaactatcgttaaccagcaccatatcggcagcttccttggcaacagcagttcctttaatccccatggcaattccaatgttggcctgcttcagagcggcagcatcgttgaccccgtcaccggtcatggcaacgattttgctgttggcctgttgggccttgacaattcgcagtttgttggctggcgtggttcgggcaaaaacattgtaacggccgatgttcttaattaaatcttcgtcggacatttcatcaatctccggcccggtgatggcatgaatactttcatccaagtccaatttgcgggcaatcgctgatgcggtatccgggtggtctccggtaatcatattaaccttgacgccggcacggcgaaggctttgaatcgaaggaatcacttcttcacgaggtggatcaataatcccgacgaccccgcttaattgaatgccgtccgcaatcttgtcctggtcaatctcgtccacatctgtgggaacgtttttgtatcccagggcaaccactcgcaaaccttgctcagttaatttggcaacccgttcataccaagtctggtcatcaaagttggggtcactttgtttgaccatgtcgaaaatggttccgggtgcgcctttaaccattaactcgtgatgatcattttccttgatcaaacgggcactgtatcggtacgccgaatcaaatggcagtgtatccacttcatcgacttccggctcacggccgattaatttgtgaaatagggtcgttaacgcaccatcagtcggctcaccgtttaattgccattcgccatcggtttgcaccaactcggcatcggtagttgtcccggcaatgtcgaccaagtcgcggaattgctggtcttgtttccaatcatatttttgaccatccaataaaacatccccatcaacacctttatcaccggcaataaatccaaccccggtaacttgatagtgatgttcgtcggtaatcacatcggtaactgtcatttcgttcttggtcaacgttccagtcttatcagtgtcaacaatatccacggcacctaaagtttcaacggcgggcagcgttttaacaatcgccccttttttggtcatcacctgaacgccccgcgccaaaacaacggacgtcgaagctggcaatccttcaggaatcgaaccaaccaccattgtgataatcgctatggtcaaggttggcagactgtaaatcttggtgtaaagaccgaggacaaacagcaaaatggcaatcgccacaataaagagtgacaggttaatccctaatttgttcaaattccgcatcaacggtgtcacctgagtcttcacttcggcaacactttgttgaatctgaccaatttgggtatccttaccagttgcaatcacaattccgaccccggatccctgagtcaccgctgttgaagcaaacgccatgttggagcgttctgccaacggaaccgaatccttgttaatcggatcttcggtcttttcaacggaattactttcaccggtcaaagtcgattcttgggcccgcatattgtctgcagaaatcaggcgtaaatcagccggaaccgcgtccccagcctcaaggttaaccagatctcccacaaccagttcccgggccggcacttcaatcttgtggccgtcacgaatcacatagttctggctcactaagagttccttgattttgcttaacgcattgtcagcctgcatttcttggaagaatccaataaacgcgttggcaataataacgatcccaataaccgctgagtctgaatagtgatgcatgaacagcgtaatcacagccgcagcgatcaaaatgtagatgatgctgttgttaaattgcagtaagaactgcagcagcttgcttttcttcttagcggttaattcattgtaaccatctcgagccaggcgtttggcggcctcttgctcgctaataccgtcctcttcgttggtctgatactgttttaccaactcatcggtacttctctgccacaacttttcatcgggaggaacctcgttcatattgtctgccattaaatgtatcacctttccttttacaaaaataagattgttgttaagagtattataatatattactcactacttttggtatataaaaatcttaaaaatcgaccacaaatcatgtgatcgatttcaaatccctattcgacaactttggtccactcatcaatcgtcttgccgttttcatccttcaaaaccagccaactgttggtgccggcaaaatagaggaagaggcccacttcattgaccgattttaaaacgatatctttggtggtcacaaaattgtggaaactatcggcattctcagatctcagtttctgagcaaacttggctgaaaatcccagcgacccatcctgattcaaatcgggttcggctttcatcaccgcacctgccttaaccaacatttcgttacgcttctgccagtagacgattgctttagcgccatcatgatcaacgtaaaacggaatttcactcacctgtttggtgaatttgtggcgtggcttgcccttgaatttcttcttgggaacaaataccgatcggaacccaagaccattcaggacggttaaaaccaaatttcgaaaggcttcaacagtttttcgctgattgctgggaatcttgaccatttccaacagatctttcttaagaattccccgttcaacggcatactcggaaaaacttttggccaaagaaccagcctccaagtcccaggctggttcgatctgaatcacaccgtcggccttgtcagttggttcagtttggacgctgatcagctttccgtctttaaggtacaggttaacgtcggcattggcctgatcgactgtccttgtgaccacaattgtcccttggccgtccggtaaggtcatcctggtcgaatcatcattgatttcaactgccaatttcatgctgcattccccatttcatttgttcttctcatttatcataccattgaataacaaaaaagaagcccacaaccctttagtggtaaaggatcatgagcttacttttaatcgaagaagaagtttgtgatgcacagattattctgtggtcagtttgttggttaaattaccggaccatttccagttttgaacctctggaatatccgtgccgtattgacgaatgtaatcgtggtgcttttggagcatttggtccatcttagcttcaaaatcgtctgccgaagcggcgaacttggtccgagaaatggcatccttagccaagtggtaacgatccaattcattcaggacccgcatatcaaatggcgttgtgatatccccattctcacggtaaccatggaaactgatattgtgattatgacggttgtataccaggccacggaaggtattctcaaagccatggaaggcaaagataaccggtgtgtcagtggtaaagtacttgtcaaattcagcttgggttaggccacggctatcctgatcttcgttgcttggacgcagtctcaaaatgtcaatgacgttgatgaagcgaaccttcaattgagggaaagcctcgtgcagcatatcaatggccgccaaactctccatggtggcttcggtaccggcagtcgcgaagatcacatccggatcgccttcatcatttgaagcccatggaataatccccaaaccatcgttaaccagcttcgtggcttcatccattgagaaccattgtggccgcgggtgtttggaagccacaatcaaattgatcttctcgcgagtctgcaaggcagtattcataacggccagcagtgagttggcgtctgctggaacatattcgttaaccaactcatgacccttttcagccagatgtcccaacatgccgggatcttgatgagtataaccattgtgatcctgctggaaagcgtgggaaacgttcatgatgttcagtgacggataatcatgacgccacgattgttcagaggcctttctgagccacttgtagtgctgagtgagcattgaatcaatgacgcgggtaaatgcttcatatgaggcaaagaatccgtgacggccgcttaagacgtatccttcaagccaaccttctgcttggtgttctgaaagctgtgaatcaataacgcggccttcaggagccatgttttcatcattcggggtcttgattggttcctcccattgacgcttaccataatccagcattgagaagaacttattggatttggtttcatctgggccaaatgctctaaatgacttgccgtttcgcttcatgatctcggtgtagaagttggataatacttcagtatcctgagcttctttgtcacctggtttgtcaatcttcaaagcgtaatcggctgggttaggcatgtccaacttcttggggttgataccaccgttgacgattggattcatcgccatccgctggtcaccgtccggtgtggttgccttaatttcagctttcacagaaccgttgttgttaaataacttttctggttcatatgattttagccaattgatcaacaaatctttatgatccatctgaccggcactgacaggaattggcacttggtgggcacggaatgatccggcgattggattgccgtccaagtcgaatttaggacctgtccagccctttggtgaacgcagaaccagcattggccagtgtggcaaagtatcatcattattgtcacgggcgtgcttttgaatggccttgatttcagtaatgattgcatccatcgttttggccatcgtctggtgaacccgggtatagtcttcggggtcacctttcgtttcaacgaagtatggcttccagcccatgccttcaaagtacttggttaagtcagcgtcactcatccgggaaagaatggttggattagaaatcttgaatccgttcaggttcagcattggcaagatggcaccgtcatggattgggttgatgaatttgttggagaaccatgatgcggctaatgggccggtttctgcttccccatcaccaatttcaactgcggcaatgacgtcggggttgtccaaaattgccccggtaccgtgagcaatggaataacccaactcgccgccttcatgcattgaacctggtgtttcaggggcagcatgggaagcgactccgcctgggaaggagaattgtttgaataatcgttgcaggccagtttcattttgggcaatctttggataaatttcgctatagctgccgtcaaggtaggaattggaaaccatcacctgaccaccatgaccggaaccttcaatatagaacatattcaaattatatttcttgattacccggttcaagtgggcatacataaagttctgtgaggcaattgtgccccaatgaccaattggcttaatcttaacgtcgtcagcgactagatctcgtttgagtaacggattgtctcttagaaacagttggccgactgataaataattagcagccttccagtacagattgactttttgcaggtattcatcggaatcgaaattcgtcatattagtaacctcctgaatttaacagtaacgttattaccaattcgattattggaccggtccaaatcaaattacaagtttattgtatgcctcaggggttgatatttcaatggtttaagcattggaataatttattttgatatagacgaaatttatactaaattcatttagtataaggattagcgcagatttcatgaaatatattcagacaaccaggattagaaacactttccccaaataaggctgggacactttttacaaatgtcccagccgatttaattgctctttgatccagatagatcctgtcagacctactcatcagcctgcttgcgactaatagtgacgctgtcgatgaatgtgcaagtacttggctaagaaatacgccaaatcacaataccaggtttcaatttgtttcatgattcgtcctccaatacaaacatgacccgttttaattcacccagcgcatcccctggattctgccattgaaaatcatatcccagggaaagatttcgataccgaatcccattttctatgacggaattgggcatgtgggaatgaccgctcaatgacaagctgacatgattgtgttcaaacaactgtcgataccggtcgctgcccaactgatacatgaagcgatcataaaagggaatcggcagctggcgagccaactttttcgtcggcagcatgtggctggccaccaagatttttttgccgctgacagccaatcgattgatttgatgctgccaagcaagaatctgctcgactacccatttacgatctcgccgataactgatttgattgccgttaatgtacaattgatcgggccagacatgtttggcaacaaagttattggcgtatcggggaccggctgcttcggaaaaatgattggcaaaggtgtagtcgtaccagccattaattccggtgatcagccagtgcctggtctcaaatggatgccgggttaaagacgttggcagccggtccaggtcacgataagccgttcgggaagccgtctgaatctgctgaactgatttttgccggggatggtccacgtagagatcgtggttgccaatcaaggtgtgaaacggaactggcaaggcttctgccaattgttgatagaaccgcaagttgcgttgaagtccattcgccgagtcccccatgatcaccagctggtcaagattttcatcactgatcaattggcccaatacggacacaaaatcatactggcggttaaaatcaatgtgtaaatctgacacaaaaccaatccgcatggttatctctccaatctggttgttttctatattgtagcgcacgaaaaacagagcaaattaaaaaatgagaatctttacaagttcgtaagtaaaagaaagctgctgacaagcaattagtgacttgattggcatcaaacgacactttgataccagaaaataataaaagatccgcatcatcccaagcatcgggacggtgcggatcttttttaaggtaaaggattatcaaagccttccagcttcgttctagccgagataaggattctcgggaacccgtaccaaatcatcggcaaccaagcgttcagcaatctgaaccgcattccaggcagcccctttcaagaggttgtcggaaacgacccacatgttaaatgctccttcattttcaaagtcaggacgaacccggccgacaaatgtttcgcgcttgccttcagcttcgattgactgcggataaatttgatgggcagtgtcatcttgtaagacaacgccatcggcaccatccaatgcagctttgatttgatcagcagtcgcattcttatcagcaacttcaaagtaaactgactcaccatgggcaattcggatcggaactcgaacacaggttgcagtcaccttgatgtctttagcgtccatgtcgtccaacataatcttcttggtttcgtgaatcatcttccactcttcatgagtgtagtagccgtctgattcgaaaacatcaatctgtggcaataaattaaatgccatctgataatgcttcttgtcccccttggtaggcaaaatctttggctcagttggttcgccgttcaatacctgttgggattcttccattaactcattcagtgcagattggccggcaccggaaaccgcttgataagttgagacgataacttgcttcaaaccatactttttgtaaatcggttcaaggcaaaccaccatttgaatcgttgaacagttggggttggcaataatgccgcggtgattataaagagccttttcgttaacttcagggatgaccaacggaacttctttttccattcggaaggcactggtgttgtccacacagactgcgccacgcttaaccgcttccggcaggaattttttggatgttgagccgccggcagatgacaataccagatcaattccgttaaatgagtctggggtggtttcttcaaccgtgatatcttgaccacggaattgaagaaccttcccggcagaacgtgacgaggccaatagtttgacactcttaaccggaatggttgactgctctaattgttggatcatgcgggtaccgacagcgcccgtagcacctaaaattgcaacgttaaactctttcatcctaatgaatccccttttctctattttgttaactcaagtaaataactgttcatgcgatccattgccaatgtgatgtcttcatcagacgccgcatatgacatgcgaatccagccttcgccgccggggccaaatgcagaacccggggtcacgccaactttggcgtcctttgccaaatgagtggcaaattcaaccgaggtttcgtctattgtatcaggaatcttggcaaaaatgtaaaatgcgccttggggcatgacaatctgcatccccattttttcgagccgatcagcgatatagtcacgccgtttgtgataggcagcccgcattggaatcggatcatcaaggccgttggtcaatgcttcggcggctgcgtattgcgcaggattggaaggagcggtgaccacgaaggcatgcattttggacgcgttggtcacaaagtcctttggtgcagcaatgtagccgattcgatatcccgtcatggcatgggatttggacaaaccgttaatcaaaatggtttgacctggaatcatggccgcgattgagtgatgcttgacgccataggtcagctcactatagatctcgtcagccagcacatacatcttgtgttgggaaataatatcagccaacgcctttaattgagcctctgtgtattcaactccagttgggttggatggataatttaaaataattgctttaacactatccccattttcatcaaggactttttgcagcttttcaggagttaagacaaacccatcatcagaagtgtcaatggtaatcagttcagctccggcaacttgaataattgggaaatacaaggcaaatgccggtgtgggcacgataaccttgtcacccgggttcaagatggtggtcaacgctgaatagatcgcttcggtagcgccaacggttaccacgatttcagtggccggatcatagtaaacacccgtccggtccttgagataattgctgataccgtcgcgcagttcaggaattcccttttgtgctgagtagtgggatttattttcctcaatactcttaatagcggcctgtttggcatgttccggaacatcgaagtccggttcgccaatcgtcaatttgacgatgccgggaattgaagaaatctcttggtcaaattcacgaattcctgaaggtccaactgcgtttacattttgattaacgacttctgaaagtttgctgtctaactgtggcatgttttcctcctgatttaattacataatattttctaagccgacgattagcttggtcgctttggcggctgccggcactgccagttcaaccccgctcatgaaagaggcgcggtcaaacgagtcttggcggatcgtcaaggcttcacctttgctgccgaaaagaacttgttcatgagcaacgtaaccgggcaggcgaacggaatggatcttaatcccatcgtaatcgccgccacgaacaccctttaaggtttcctcagttgccggtgaatcgtgttttccgcgaacttcagcaatcatcttggcggtcgccaaggcagtgcctgatggagcgtccagtttgtcgtcatggtgcatctcaatgatttcaacgcccggcatgtatttggcggcttctttggcaaacttcattaaaagaaccgcggagatgccaaagttgggtgccaggattccgccgacgttggtttgttgagccaactttttgagctgatcaacttgctcatcgctcatcccggaagtcccaataactggatggatgccgtgttcaatggcaaatttggcattatcaaatgcagccgcaggaacggtgaagtcgatccaaacatcggcgtcggtgtcgatttcatccaaactggcaaacagcttaaccttatcgtccattcccatgcctttgagatgaacggtgtcgattccaggattgtaggcccccaccaattcaaagtcatcatttttattgaccatttgaaccgtcttttgacccattgagcccatgaaaccagcgactaaaactttaatcattgaaaaaactcccttgtttatctgtgtttgataatttccaaatcaaccgcttaactgcgcgccatttcagtgccgtcaaccggaatatcttccaagcggctgacacctaatttacttgccagggttgctttttcttcatcgttcaatgaaagaatcggcaagcggcaatcaccggccccaaagccttgaacattcaaaatggctttgacacatgacggtgatgggtacatgaataaggcttgcacttttggcgtcaagaaacgcatcatgtcgccggcagtctcaacatcccctgattcaagggcgtcgtacatcttccgcatctcccggccgtaaatatggctggtaactgaaatgacaccgttggcaccaactgctttagcagacaaggcctgggcatcttcaccggtgtagacattgaaatcatccggggtattttgaaccagatattccaagtcttccaatgaggtacactgcttaacgccggcgatgttggcgttatgtgataattcgaccaccgtatcgttagccatcgtgacgccggttcgaccaggaatgttgtaaatgatcaatggcactggtgactgttcagcaactgccgtaaagtgggcgatcatgccacgttgatttggtttgttatagtatggcacaaccacaagggcgtaatcaatcccggggatgttacccacttcagctgttaaacgcacggtctcggcggtattgttactaccggtcccggcaataatcgtcccacgcccgttcacaatttgagcaaagcgggtatacaattcaatcttttcgtcatggctcaaagttggtgtctcgccagtggtgccaccgattacaaatccgcggctcccagtatccagtaagtgattggttaatttttccaaaccgtcaaagttgatgctgccgtcttcgccaaacggggtcacaattgctgtcataatatctgcactaatcatcataaatccctactttcttttattgggttaattattcattctgtattcaagaaatctggtaattgatttaattccctttggaatcgatgattctttggggttcagggtagctgaatgaagctgtgaatcatcatcgacgcccaaccaaaacatggtaccgggaatcttagataataggtaaccaaaatcttcgccggtcatcgccggttgagtttcaacaaagtcggtttccggatcctgcttggcaaattcaatcaatcgtcgagtcagttcgtcgttattttccaccggcaaatagccaccctgattaaagtgaatcttgacttctgcgccatagctggttgccactccattggcgaccatttttagccggtcaacaatgtgttcaatcatcttctgggttaagccacgaatggtaccttcaattctggcttgccccgcgataacatttcgaatggtgccggcgtccagtttaccaaaagtaattacaccgccctcgatgggattgacacttcttgatacaatcgtctgaacctggccgatgaattcggctgcggcaaccaccatgtcgttggcgttctgcggataggcggcatgaccacttttaccaatcagatcgacgttgacctcagtcgttccggcaaacaaggttcccattcgacagccaatcgcgccagccggtaaatccgggttgtcgtgcagtccataaaattcatcgggccgccactttccttcaaagacgcctaattcataagcaaccttgccgccgttttcgctttcttcagccggttggaagaagaaaaccatgttgtcagccggctgatgctcggaaaaccagttgaggactcccagtgcgacggtcatatgaatgtcatgaccgcaagcgtgcatcacaccaggattcttggatgaaaatggtaagccggtcttctcgctaaccggcagggcatcgatatcggtgcggtaaccaatcgtccgtttagggtttgatccgttcacgtacaccagcagagccgtcggtaatttggggatttctcttatttcaatgtattgttgattgaaagattgaatggttttcaacaggtaatcatgagtggctctttcgtgcatcgccagctcaggatattcatgcaaatgtctgcgaattccaattaaatcttccttcgttagttgactcattggatcacaactttcttaaatcatcttccagaccagtttccgaggttgtcttttcatcaacgtctttgacctttcgcgctgggacgccggcaaccacagtgtgtggggcaacgtctttggtgacaatggatccggccgcaaccacggcgccttcaccgacatgaacgccttcgataaccacggcattcgcgccaactaagacgttatcgtcaatttggaccggtttggcagatgccggttcaacgacgcctgccaaaacggctcccgcaccaatgtgggaatgcttgccgacaattgctcggccccccatgacaacgcccatgtcaatcattgtgtcatcaccgatttcggcaccaatgttgatgatggcgcccatcatgataactgcgttgtttcctattgtaacgtgatcacgaatgatggctcccggttcaatccgggcattgatctccttgatatctaataatggaactgcagaatttctggagtctgcttcaacctggtaatcatcgatggccgatttgtttttcttaaggaaccgtttgacgtcagtccaatcgccaaacaaagttgcggtgtgcttttcggcaaatgccttgattgattttggaaacttgatgtccttaatcgatcccttgagatagatcttgaccggggtcttcttcttggcattgccaataaaatcgatgatttctcgtgcgcttagttgttccattgtgattctccttaatgtcgttattttgtatgaacttttaatgtaatttttatcgggaactggaaacgtctcaaccagcctgcggctaaaaacacgtttgttagattcttttgaggtagcttaagctttgaaaatacgctccgggagccagatgctaacttctaagacaatcatgattcaagcccaaaatcagggcttcaatcatgattgtcttagaaaccgcatctcctggctccctccgcgctctactctagttgaactcctcatccaacgccaccaaatcctcaaacgtttctcgtctgatggcaacctgcgacttgccgttttccacgaataccactgccgggcggggattacggttatagttggaggccattgcatatccataagctccggtatccagcatcgccaggacatctcccggttgggtggccggtaaatcctgcttttgaatcaagatatcaccagattcacaatacttgccggcaatccggaccgtttctttaatcggtgcacttggattcttggcaagaaccgcctcgtatttggcttgatacagcgcgggacggatattgtcacccattccaccgtcaaccgtgacgtacgagcggattcccggtacatctttgcggctgccgactgtgtataaattgtagccggcaggaccggcaattgaccggcccggttcaatccaaacagcgggcattggcaggttaacttcttccgtgcgtttcttgatggccttaacgattgcatcgacaaacatttccggagcaatcgggtcatcatcttccgtgtacttgatgccaaaaccaccaccgacgttgaccactttggcaacataaccaatttctttattccagtctgccaaagtatcaatcaacttaacggctgccatttcaaagcctttcacttcaaagatttgcgaaccaatgtggcagtgaatcccaagcatgttcatccgctgatcttcaaggacaaggcccagtgctttacgggcctgaccgctttgaatatcgaagccaaacttgctgtcgacttgaccggtctgatcatattcgtgggtgtgggcggaaacccccggtgttacccgcagcatcacgttgatgtgtgattgtttatcttccaaaacttcttttaacaggtcaatttcatggaagttgtccaaaatgatgaccccaatttggtgttcaactgccatttccagttcttcgcgagatttgtcgttgccgtggaaactgacccgttccattggaaagcccgctttaatggccgtgtataattcgccgccggaaaccacgtcgatatgggccttttcctggttaatcagctgaaacattgcaatgcaggcaaaggctttgctggcataactgaccgcaaaatcgacgccgttatcttggaacaccttttgaaaatggtggatctggtcacggatggatttcacatcgtagactaccaagggggttttatattgcttaaccagatccaatgaatctactcccccgatttccaagtgtcccgcttgattggttgataactggtcgatttgattgctcatgttttctcctccaaaatatctttttgtgaatgatggtgtggtgaggtgttggtggctcggtagaagctgtgtctgttgggggggttaaaagcacgcttgttaggggcttttgaaatcccttcggccttgaaaatacgctccgacagccgggtgaaaccctgcctagcctaccagccctcatcgcgcaggaagcacgtttgttatgattctttgagctccctgcagcttccaaaatacgctccgacgggccagatgctaacgtgtaaggccgggatgatttaaatccaagttcgggattttaatcatcccggccttacacaccgcatctaccagccctcgtcgcgctcttaataaaaaaatctcctcattcggcgttcgccaaacaaagagattcagaattttagttcaatatcattccgtatcatttgtcgttagcgccccgcagccgacttatccgccgcgacagtccatagcctcttaagctaagtcccagcgcgccaagtgctacctcacatggtgcttcggcaaccgcccctttcattaacttcaaagttcaggtaggaactccactaattactgatgttggttgcaacctctaatgatttaattgacataattctataatgattctcataaagtgtcaaccacttttatgagtccggatgcaaattcatgcaaaccaatcacgataaactgatgactcttgcaaattaattcaaaactgctaaaattcgttttaacaatctctaaccgaattgttaattaatgggaatatccagggagtgaatgaaagttatgaaagtcgttaagtttgggggcagttcgttagccgacgccgcccacgttcaaaaggtgattcgaatcgtccaaagcgatccggaacgaaaggtggtcgtgacttcggcgccgggcaaaagattcgccgatgacatcaaagtcactgatctcttgatcaaatatgccaacgcaatcatcaatggaacggatgccaaatccattgttgcaaccatttttgaccgttaccaggaaattggcaatggcttccatgtttcaaaaagcgtccttgatgatcttaaggccaaattaactgcccttcccgatcaatcatatccaaacgacgactacctaatggccgcctttaaagctcatggtgagcgattgaacgctgaattatttgccgcctgcctgacagaggccgggacccaagcacggttcgttgatcccagtgaagccggcatcttattgagtgacaatcccaatggcgccaccgttcttgaacaaacctacgacaatctcgccaatttgacatatggtgaggaaaccttggtcttccctgggttctttggatttaccaaagaaggcaacattgccactttcgcccggggcggatccgatattaccggctccattttagctcgcggcctaaaggcggatctctacgaaaacttcaccgatgtcgacgcaatcttcgctgccaacccgaaaattgtgccggatgcccgacccattcacaaaatgactttcagagaaatgcgtgaactttcatacgccggcttttcagttttcaacgatgaagcaatcattccagctattcaaggtcaagttccaattaacgttaagaacaccaacaatcccgatctcccagggactttgattgtccccgaaaaagattttacttcaaaaaaaccggtgaccggcattgccgcatccaaccgattctcagctctttatctccacagatacctgctgaacaaggaggttggctttaccctcaaaattctccaaatcctgtataaatatgacgtttcctatgaacacatgccatcaggaattgacgacttgacgatcatatttgaccgcagtcagctggacagtgatacaattaaaaaaatgtgtcatgacatccaggttgaactgaatccagacacgttggattggatcgatgattacgccatcatcatggtggtcggcgaaggcatgcgggcaagagtcggcacgattgaaaatatcatccggccattggctgagcacgacatccctgtccatatgattaatcaaggggcgtctcgaatttcaattatgctgggcactcgtcaatcagacgccgacgcagcagttaaatatatttaccaacatttttttaaagaagatccttccgttaaccaacttgaataccaggcggaagtgtagaggaggcgcgttatggttcaattactcaaagttcatggatcacaaaataagttctttatcttagatcaaacagctttacaaactaaattaagtcagcccgaattggtggccttggctaaacacattaccgaacctgaaacggggctcctcgatggtgcagacggcctgttggtcattgacgattccgaccatccagacactttgggcagcatgcaggtcatcaacaccgatggcagcattgcgtcaatgtgtggtaacgggctgcgcaccgtttcccgttatctgtcagacaaatttggcgaagatcaattcaaggtcgaaacgatggatagtgatctgcatgttcatcgtgaagcagacttggccgacaacgtcccaaccttcagcgttgaaatttctccggtcacttttgctaaggaaaccctgccttttgataatttaggcaccgatacacttatcaacaaggccgttcccgagtttgcgcccgaccttaaattcaccgcaattagtgttcccaatccccacttaatcagttttgtcgacgaggaaaccatgcactcaaagactttggggcaactgggcaagatgctcaacgaccccaatccttatttcccagatggggttaacgtcagcttcgcccagattctcgatcacaacacactgttcgttcgaacttatgaacgtggtgtcggcttcaccaatgcatgtggaaccggtatgtcggcaaccagcttggcattttgtctcaaccatccggaaatggccgactttgacgaactgatctcggtttataatcctggtggcatggttaagaccagagttcacagccgcgatgataccttctcaattgacttgatcggtaacgcgactttcactcacaagattgaaattccggaagccgatctccatgccaatgatttagagcatgcacagatcacagaaaccgatgaacaaccggcatatctgagatttgtggaaagtcttaagaaccaactgattaaatagacaagagtcgaacacaaggcatcttgatttcagaatttaagtaaaaaaacgagttattcctgttttggaatgactcgttttttttgcttgaatggccgggatcagccgctggttccacgtttaagctagctatagcggcccagacatgatcaacaaatagtctgccttagcctcattttttagtgtgctcattaacccacacctcatggattaattgattggccaacaccttgcaaatcatctcaatcagctgatcctgcatgaaagtcgtcgcgtcaaagtctgccggctgcccattaacggcggtaatccgcatcccatcagtttgaatttcaacgttatatttggcaaaggtatcaacaatcgcctgtaatttttgcgcatttaacatttactgacctcccagccgcagctttagtcgccattcgtcttggcggacttggttcggcttgatgcgtaaatccagatagggcgccaccaacagcaagaaatctttgacgtcttcataatgtgatttgcttgagaagtaatgattggctttgcgttgggacaacttgtcaattttaatctgcagcttgtttaaatagtcttccaccagctgaatggtattttcccgaatactggcaatctgggcaatcttttcgtcgtcaggatcctcaatctccaactcttcaaccaactggtaatggtttaattcctggtcaccaggattaatcagttccaagtcaccatcgccaactgcggcagcaaaggattcgccatccgttcgcgccaaataactgggcaattcttccccggtcattttaaccagcagaacggcttttcgagcaatcccctggccaaatttgatgtgaatgacaaaattctttttgccgatataattgacgttgtctaaaattaattgtgggttatgggtaaccacttcaccaatcgcgaaataagtcgcccgttttgttcgataaatctcaccaaattgtggtgtcaattctacacgtcctttcgttgttgctcataagcatcatcatacgttacttgaagattttttcaaagtcaggattttccaaacatatgttcaataattttgtataatgggtattggataattcaaaacgaaatggaggggtcgtcatggccgtacaccaagtcggtattcgagaactagtggaatttttactgcggaccggtgacttaagccccgttatcagcagtgagaatacggcacaagaaggcagtcggattcaccgcaaaattcaacgaagccgaccagcttcttatcaatcggaggtggcacttaaaacctcgatccagtatttggatgacgaatacgtcatcagcggacgagcagacgggatcgatgaccgcgacggcaaaccgttgatcgaagaaattaagacctccgacttggaattcagctcggtgccggactccacccttcaactttattggggccaagtcaaagtctatgcttacatcgtcatgcatcaagcagatattcgatcagttgatctgcagttgacctacgttcagacacctgatgaaaaaatcaccaccaagacccagacgattaccaaaaccgactcggaactcttcttcaccgccttggtcaccgaatttgagcaatggatcaaactccgtcatgaactggacgaaaaccgaatcagttcagcgaaaaaactccaatttccattttccgactaccgacccggccagcacaagttagcaactaatgtctacaagaccattcttttggaaaagcacttgtttgttgaagcgccaactggaaccggcaagacgatttctaccctttttccggcaattaaatcaatgggtgaacagctgatcaaccgcattttttattttacggccaagcagagtacccgtcacgtggcggaaaataccatttcgattatggctgaacaagggctgaaattaaaaagcatcaccctcaccgccaaggacaagattacgttcccaactgaaaaagaactgccacctgagaacaacccctacatggtcggctactatgaccgcgtccggccggcaattaaagatattattcaacacgagaatcaaatcaccaaagccaccattcaagaatacgcagagaagcacaaagttgaccccttcgaattttcactcgacgtcagcctgttttgtgatatcatcatttgcgactataactatttgtttgatccccaggttcacctgcaacgtttcttctcatttcccgatcccaccaactgctttttggtcgacgaagtccataacctagtccagcgatcacgggagatgtactcggcaacgttggaatcatcaccgattgatcctcttttagagcggttggtgaagaaaaaggcaggcaaccaaaaagtcattaaacggcttaaatccttgaagcgctcatttaaacgttatagcaagccagcctcagaagtggttgataagcagatcgctcaactggcgccactggataatttcaataacactttggagaatctaatcgaaacgattcaccagtggctggcaacccaaaccccgagtgataccgttgacgcggtagtcgactattatctgcaatgccgccgttattacctgatcagcaccttttatgacgaaacctaccgcacacggatcatcattggcgatcacaccatcatttttcgccagttctgcatggatcccagcaagcagctcaaagcctgcttgaaccttggccgggctgcaatcctattttcggctactttaagcccgatgtcatattaccgacaagtcttgggcaacgaagaagacagtttaggaatgatttcacattcatcatttccaccccaaaattgccaggtgattatcgccaacaacatcaatacactatacgccaaccgggaaaatagtctgcagccgatctgtgagaacatttacaccatgatcactcaaaaggttggccattacatgatgttcttcccttcaatggcctacctgaacgccacattgagtaaatttgtcgagctgcatccagatattgacgttatcaaccagcagccggaaatggacaatgcggcccggaccgcctttttggatgcctttcgcacggaagatcatcaaaccaaggttggctttgctttactgggtggcattttttcggaaggcatcgatctgaaaaatgatcagctgattggcgtcggcattatcagtgtcggccttcccggcatgaacaaagaatccgacctcatcagagactactttgactcattgaacggccaaggattctcatttgcctatcagctgccaggctttaataacgtcagccaggccgccggacgggtaattcgcactgacgaagacaaaggtgtgatcgttttgatggatcaacgcttcaaccaaacccgttaccggcaaattttcccccagaattggaccaacattaaggtcaccaataatcccaatcagctaagaaatgccctgcaaaacttttggcagcacggcaatcagtaagtgttctcgtgccaaaaaaagcgaatgggtgtatactaataacgctgttcgttaatcgaattaaagccaggaggggtaatcttgaaattagcaatgtatgatcatcagccaacatttgtggcgctccaaaacggtcagttctggggcgttccaattattggttacgactcaatcgacgatattttaaacgattggcagaactttttggctaacgtactcattaatattaacgacgataaaatcatcgacaatgacaatgccactcaacttgatccacaacattttgagcagcctgttcaacatccccgtcagctgcctgctgttggcttcaactatctcgatcacatgaaagaaatggacattgtcaaaccaaagcggcccaacatcttcaataagtttgtcagctctttagccggccctcacaactcgattcatttgagtagcgacaccgtcgactgggaatccgagctcgtcgttgtgattggccgtggtggccgcaacattagccgtgaagacgctgaagacgccattgccggctacatggtcggccaggatatttccgatcgaaccgttcaatcaatcgatggtcccagtacgcagtttgaccttggaaaatcctacaagaattattcgccggttggcccttacataaccaccatcgctgacgttgacgatattgtctccaagaccgttaccaccaaggttaacggcgaaatcatgcagcaggcgacaattgataagatgatttttgatattcaaacgctggtctcttacatttcgaacgtcattgaactgtaccccggcgacctaatctttaccggaactcctagtggaaccggcgttggccgtgatccgcaagtcttcttaaagtccggggacctgtttaccagtgaaattgatggtctgggaaccatcgagacaaaggtcaactaatcaagtcagttatttttaaagaatttccaattaaaaaagctggagctaaatcgttgtgatttggctccagctttgttagtttaagttttaattgcaaattgattctgactcatactcgtcaatcttacttcttgcgtaaaattgaaacgccttcgggtaccgtgaaatccttttgaatcatggttaatttgccagactcggggtcacgcgtgtacaatgtagcgttgtcagaattttggttcaaagcgatcacaaaggattgatcatcgcttaaattaaagtcgcgaggaaaatcgccttccgttgaaatccgctgaatcaatgacaaattaccggattcatctgaactgaagaccgcaatcgaattgttcccacggttggagacatacacgaagcgcccatctttggaaactctgatggcagcggccccattatgttcggtccagtcatcgggaatagtcgagtgaatgtcccttaacgacaggacccctttgtcggcatcatagtccaatacggcaacattgctgcttaattcgccgaccaaataagcgaccttcttcttggcatcaaagtaaatatgccgtggaccataaccgtcttgcatctgcagttcgctaaccggcactaatttaccgttggcttccaaatcatagataaagactttgtcgacgcccaaatcaacggccacaactctaccttccggtgtcaaattgatatagtggggatgaggaccgtcctgttgctcttttcgaaagccgagggttcccttatccataatccggtcggcctttgaaattgaaccgtcatcggcaatccggtaggtgttaaccgttccggcatgataattggcggtgaagactaaccgcttatcttcgtcaaccgcaatgtaagccggtgaagtttcctgatcatgaaccgaggcaattggtttcagtggaaaatcatcgctggtaccatcccattcaacgaagccaccggtcacgtctcccttgtcatctttgactttggtgatcgcgtaaatccgcttttgattggattccgcaacgtaggttgggtcaatggcgctgccaacaaacgttaaattttgtaatttttgattttcagtatctaattctaactgataaacacctttactaattcttctggtataggttcctagcaagtatttttctatcaaaattttccctccaataaaagtttatgtcttcattatgccacagataaaacctaaccaaaacacatttgaaagctttttcacgaaaggaacacattttatgacatcttttgaaaaatttcatcccgtcctcaccgcccacttaacccttgattggctgacccaaacaccggtaaaatccattgacgatctgttttccaagccggcagttacaaccgccaaggccgagaaaatgcccagccaaatcctcgatactgttaaagagatcaatcacataatgcgccgggtaatgaacgacaaggaattgacctggggaattaccgactccaactcagacgcgtttgtgggcatcatcagcctgcgcggctttgaagcagctgccccatcgggatcaattgaattcatcattgaccaggatcaccgtgagtatctggcagaagttgttgaaagagctgtccgattttcccaggatcattttgaattcaatcagctttcaatcacgtttaatgatgtatcttcacaaaccgcaaaagaactgagtggaattggttttgtaggcgacggcgaacagcggtttaccatccaactttaaactaatttcaaagtaacaaaattattaacgacaatccaattcagaatcgttgcatatccagaccaagcatattagaattgttctaaagtaacgattggattataataacagtaaagaataacagaacgctcctcatggaggtgccaataatgacaaacacaactttaaaacgttccctgggtcaacttaaaaaacagggcgtccggattactcctcaacgagaagtgatcttggattatttgattacccaccataatcacccggatgtcgaaaccattcgcgacggtatcgaagacaagttgcccaacctcagcgtggcaacaatttataacaccctcaagatgctggtcgacaatggcttggtcattgaactgccaaataacgatggcagcatccgctatgactattttggcgttccccattaccatgcaatctgtgaaaattgcggcaaaatcatcgacatttttgatgatgactatcccgaattagtcaaacacgttcaacaaaccaccagagaaaaaaccgactttttggtgaccggtacccaattagaggtcaccgggatttgcccggattgccagcgtaaactccacctggccaagcttgccaataaatgattattacagcgttaaactgttgatatatcagtcattagctcgataatttaagaattttgtcaagaactcttaatatgattgacaattagtaccgcaaagcccacgggtacgcgttaaatcgctatccgtgggctttttgtccggttgaattgtatcatgcaaatcgtatatattaatgaccgtagctaattaccactatgtaaaaataaaataaacatttaaaacgaaacttaaaaaaatctgcaataaacacttctgaagggaataattaatttgaaaaaaagagcgattgtaacagccctttgctcgctgacactggcggcaatcggcatgtttggactaagcagcactgcgggggctagcagtgtcaacgattatattgccaataacaatatcggccatgccagtgttacatcatcggtgtggagcggttttccaaagaacgcctaccgaaacggaaccggtaagcctgaaggggtcgtcgttcatgaaactgccaaccccaactcaacgatttataacgaaattgcgtacatgaagaagaattataataacgcatttgtccattctttcgttgatgccagtcgaatcatcaacatcgccaacaccaactacttggcttggggtgccggctatccggccaatgcccgctttgtccagtttgaacaggtcgaagtccacagcaagtcagcgtttgcccacgaaattgccaacgcagcttactacaccgcctacattttggataagtatggcttaaagcctaatgatgcagcgtatgacggcaagggaactgtttggtctcacgggggtgtctccaaatatctgggcggtactaatcacaccgatccagccggctactatgcatcagcaggtaagaaatatttcggtgccagctatacgtttgcccaattttatcaattggttaagacaacctacaataatttggcagacgatggcgcagcccatgggtcattaaccgcttcatcagcaaaaacagcgtatgacaaggtcacatacgccaaagcagatacaaaggcgtcattaggagacaactacaagtcatacagattatataatcacgttaagaattcacgatccggggtcaaatcatattcgtggtcctcagttgacgcttccgttggtaagaaggtctatattgatgacatcgggactaaatcaaacggtcacgactggtatcggattaccttctccaccgacagtggtgcgcaaaaatattgggtctacgaaaaagcccttgacctaatcaattgacatcatttatgaattaatatatgattatgacaatttagaagaccaagtagtgtgcgtacagagaaagtgccgtcggctgaaaggcatttaagaacacgaatcctatcttcaagacgattgccctaatcaggcacggatttttccgttataaaacaaaaagtgtgaagcctggctttgaatgagaatggtaccgcccgttgtgggtgtctcaatttcaaagcaggctttttttatacaaaaatatggggtgagcagatggacaaacggattattaacgcaaatcgaatcgtggtcaaggttggtaccagcagcctgatccacccaaacggtgcggtcaacttgaagacttttgatgagttggcgtacactttgagcgcgctgaataaccagggcaagcaacttgtcctggtttcctccggggcaattggggttggcttgaacaaaatgcacctcaagaaacggccaaccgaaattggtgcccagcaggccttggctgccattggtcagtcagagttgatgacgctgtttacgcaacgattcgaccactatctgacagatattgcccaagtgcttttgacccatgatatctttgattatcccaagagcaaccagttcgttatgaacaccttcaattgtctactgcgggacaatgtgatcccgattgtcaacgagaatgacaccgttgccactgacgagttggaccacaagaccacctttggcgataacgaccaactttcagcaatcgtcgccagccacgtggatgcggatttactgatcgtcttgtcagatgtcgacgggttctatgatcaaaatcctaataaagtcgctgatgccaaccttatcagaaccgtgagtcacgtggatgaaaatgaatttggtgttgccggcggaaccggcagccgttttggaaccggcggcatgcaaaccaagctgctggccgccaaacgaatgcttgatgaagaccggatcatggttttggccaacggtgccgatccacgcattatttttaaaattttagccggcaaagatgtgggaacgatctttcaaaaggagagtgtagctcatgaatgacaaattaatcgaaattggcaaaaatgccaaagctgctgcttataaattgaacctgctggataccgtgaccaagaaccgaatcttaaacgaatttgcgatcgccttggggcaaaacactgagctgattcttagcgctaatcaaaaagacttggctaacgccaccgacatgcccagcaaatttaccgaccgattaaagctgacttcccaacggattactgacatggccgagggcctccgccaagtggccggactggccgatcccatcggtgatatcgacaagggctgggagaatgacgccggcttaaacattgaaaaaaaacgggttccattaggcgtcatcgccatgatttttgaagcccggcccaacgttactgtcgacgcctccgctttgacatttaagagtggcaacgccgtcatcttgcgtggtggcaaggaagccatcaacaccaatttggcgctggctgaggttctccggcaagttctaaaagcgaaccagttagacgaaaatgccattcagattctgcatgataccagccatgatacggccaatgacctgatgcatttgaatcaatacgttgacgttttgattccacgaggcggggccggcttaatcaatgccgtcgtgaaaaactcgacggtccctgtcattgagacgggtgccggcaactgtcacgtttacgttgacaaggatgccgagttacaaatggccattgacatcgtcgttaatgccaaagtccaacgcccatctgtctgcaacgccgctgagaagctgttgatccaccgggatgtagctgaaagcatgctgccggcaatcgctcaggcgctggaggaccacggcgttgagcttcgtggtgatgaagccagccggcaaattgtctcctcaattaccccggcgactcaagacgactggtcaaccgaatacaacgatttgattatggctgttaaagtcgttgacgacgagcaggccgcaatcgaacacatcaatcaatactccaccggccactctgaagtgatcatttccgataactatcaaagcggtcaggaattcttgaataaaatcgactccgcctgcgtttacgtaaatgcctccacccgatttaccgatggcttcgagtttggcttcggtgcagaaattggcattagcacccaaaagctccacgccagaggacccatgggcttgaacgaattgactaccaccaaatatgtcattcggggcaatgggcaggttagaaaataacgagtttaataagcatattgatgagaccgggagactgggacaaaatgaaagattctgttccagcctctatttgcgtccgaatgttatctggcagaactgtgcgccaataagcagcttccggccgtataaggggattacccaaacatccaagccctggatatttgggtaatccccttatcctctggaagcaaaccgcttattggcccacgctgccgttttttattgaaaatacgttgtctttcacttcccttttgtgaccagatgacgtatactgtatttagttagccggctaactaaataaagaaaggggaccaatcgtgagttattacaactttgtcgatcgacccagcaagcagcggattcaagagatggccgatcaattacacttggcagtatcacctgatgcggtgcatttattcttggattttcaactagcctatcgggaggtcgaaaagaactatgaaagtctggtggcgagttttgacctaagcgaatccaggttcatcatcctgatgttcttgtattatgcagatgacaaacagcttctgccctctgagattgcacacaaattgggagttaccaagccaacgatcagtaagttgttgcgggggatggaacaacaaggtcttgtcagcagtcaccagtcttcaactgacaagcgggttcgggatattcagttaacacctgcaggtgaaaaactgctacgaacttttttgccctataactatcggtccagttccctactatttgaagattttactgacgaagaaaaacaacaattcgcgcatttactacgaaaactactcaaatccaaagacaagatccaacaactggaggaagactatcatgaacacagaaaaaattaatttactagaaacctatttaagcctgtacattaaccccatggacgttttaaaagccggtcaaaccggtcagtcgccctatgtgattttagacgttcgaaatgcccctgcccagattaaaaaagaccagatcaaaggcgcagttgccatgccagccaaagacttggcagctcatctgagtgaactggacaaagctaaaacctacgtggtttacgactggaatggcggcacaatcttgggtaaacaagctgttttgatcctactcaaagccggatttgacgcattcgaacttgccggttccctggaaggctggaaaggcatgaacctgccactggaaaccattcaataattttggacgcatttcatttgaacaacagacaccaagaaggccgaaacattagagaaatcctgatgtttcggcctttagtctgtctatttgaatttacttcagtaaatggtgctgttgcagatattgcttagccacagccgcggccgaacgatgtttaacggtcacttggtaattcatctcctgcatgtcacgggttgtgattttgcctgctaatcgactgagggcgcgaaccacttgtggatgcgtcttggcaaactggtcggtcatcaatggcgcgccttgatatggtgggaagaattgtttggaatccttgagcaccaccaaatgatactccctgatttgcggatcggtggtgtaagcgtcggtgacgtcgacccggccatctgccaaggcgacataccgtagagagggctccattgtccgaactgattttaattggaaatgataggcttttcgcaatcctgggtaaccgtcggactgctggtaaaagtcgggatcaaaggcgccggttaattggctgccaacccgttgcaaatccgcaattgtgcgtaaatgatactttttagcggtcgactgacggacggtaatcgcatagccgttttggtaggccattggtttcagataccgcatatggaatttttgactcaaggcatttttagcatccctgtaggccaattgaggctcgctattcacctttttgggggaatgaaccagtgattggagaaccgtgccggtaaattcaggataaacgtcaatttggtcactctgcagtgctttgaagagaaaactggttccgccgaagttgggtttaagttggacttttgtctgtaggctctcttgtttgaccaagtctttatacatattgatcaaaatttccggctcaccgcccattttcccagcaatcgtaatcgtttgggacggcttgttgaacaaggaccaccctaatcccgcgccaccgaggatcagtactactaagacgccgattcccagctttttgaaagaaaattgagataagactttgattaaccaactggcaaccagggccaagatggctgataaaactgcgccaacgattaaggcggcattgttgttagtctgaatgcctaacaggatatatgttccaaggccgccaccgccaattaaagcggccagggtggccgtcccaatcaccaggacagtcgcaattcggattcccgaaagaatcatcggcatcgctaatggcaattcaatccggaacaatttgaaccgtttggtcacgcccaaagcgtcggcagcttccaacaacactggatcaatgtgggtcaggccggcataggtattttggaagattggcataattgcgtacagcaccaaggcaataattgccggtaccgtgccaatcccaacaaacgggatcagaattcccaaaactgccaggctggggatcgtctgaatcacgccggcaatttgtgaaatgatttcgccgatttttggccggttcaccaaaccaatcgctaaaggaatcgcaatcacgatggtaatcaagatcgcaatcaatgagatttcgatatgctgccaaagggcttgcatgatggcagcggcatttttatcaacatatgccacgacttcgtcaatcatttgtcggctcctttcccaaatcggcgacataagaaatcaagtcactttgcgtcagaatggcaccgtccaccaaaatcagctggctgggatttttttccaacaggccggcccattcatagactgtctggctgttctgcagcgtaatcgcctggtcatctttaccaactggacgccccaggccggcattaagcacttgttttaaaagtctggtgccggaattgtcgacgtcaaagaaccgtttgacaaactcatcggcgggattggccatcaaataatccggctcaccttcctgtaaaagaaccccattatgaataaccgccaatctatcagcgagtaaaaacgcttcgtgcatatcgtgagtcacgaatacaatcgtggtgtcaatttgttgatggaggttcaaaataatcttctgcagttgcctacgggataccgggtcaagggcgctgaagggttcatccatcaacaccaacttggggcgggcagccagggcccggacaatgccgactcgctgagcttccccacccgataattcgtcaggcatccggttcaaaaattgatcagggtccaaattaactttgctcatcaattcaaccacccggtcatgctttttttgagccggccatcccaagttatcaagttgaatggtggcattttgttcaacggtcatattgggaaacagcgccccggtttgtagaacgtagccaatgtgtcgccgcaatttttgtaagtgactgtcggcgacgtcctcgccgtcaattttgaccgtaccgctggttggtaccactaaacggttaattgtctttagaagggtcgttttcccacttccggaagggccgaccaacacaaaaagctcaccatcatcaatggtgaggttcaaatctttcaatgcaaattggccgtcaaacttttttgtgacattcgtaaactcaatcaatgtcgatcacctcgtaaaatccatggtgttttaaatatactcattttgacgatcgaacacaactcaatgctttaactgggctttgtggagccgcttcaacttgaaactcatcagccaagtcgtaacgggaatcgtcgtaacgaccccgattaaggaaaccacaatcgcgatcaattccgcagcaaacaccttgtcgttaagaatatcgccgaaggaataattcaagccatagaaccaaatgaataacgccaacgaactgccaaagaagccaaagaacagagtattaacggccgttcctatgatttgtttgccaatcacggtgccatccaagaagagctgttcacttttaatggcttgatgttgagttataatttcatccaagccagaggcaatcgcaattgcggcttccgcgaccgctcccaatgaactcagaatggcggttgcaatcgcaattttcgtgaaatcaatgccgacatacgttgagaggccttcaagttcctcgctgtcttccaaaccaaaaccgccaacctgggcccaatattcaatcggaataataatgactacaatcaatatcaaaacaatcaccgaagcctgaaaggccgtggtcgaggcgttgtcactggcactgctccaaaaaatggtgatggacagtaaaatcacgctggcgacaatcgtgacgataattggcggcagatgaaaggcaatcagcacaatcgtgaaaaagagaatgccaaaattaaccaccaggctgagaaatgaggtgatgccctgtttgccgccaacaatgatcatcaagaccagtagaacaatccccaaggctgtaatagctcccattagcgttcatcccctttaatccagagtccggcaaaggcactcgataaaatcaccgtcaggacgatcccaatgccgctaatcaggctggaagtcatccccaatgacatgttcatcgaaaacgaatagtgccaggtgttgccattttttaagtaaagtaaggtcatcgccagggtttcggccatgaagatgaagaacaaaacgttaatcaggggccccataatcgatttgccaatttgtctgcctgatttaaaaatcgccattcgagacagttccgggcgctcctgcttcaacgtcgccaaagaagcgacaatatcggtggcctcatccatgacggctcccagcaccccaatcaggacttcggcgataaacaatggcttgggcagctgagtaacgtactgcatcgactcataatagataccccgctcgttggtgaggccgaagacgatcaacgtaatcaagatcgttgccgccgtcgcgcacagaaccgccgacaacgtcaccagcattttcttgctccagcccataaccagcagtaaggtcacaaagcagaaaataacggccaaaacgctaaaaatccagataaccgcagccccgttattattgtggtcaagcttaacagctatccagaacagaatcgtgttgatcaggatgctggaaatcaccgtcacaccgcgcaatttaagaatgacaaataacaggctgatggcaatcgcaaatagaaaggcaatcggcgcatcccgcttaatatctttaactgtggcgtgtagtttgggctgagtatgtaacgtaataaagagcttttgtcccttggtatattgatggtccattgcatgcgaatctgagtaggcattcttaatgcttaatttttgaccagcatacttcccgttggtaatcgtgccgaaaagctgctgattgtggtaatgatcgacattttgaaactcatcggtcatcttgattgctttgccgttttgcacccggtccacccgataaatggtctgctggtacaggccatcattgtgctggcaaaaaaaggccgctaaaaaacaaaaggcgacgaccaggacaatctgaagccacgtcattttactcgttaatttagagttcatattgcacatcttttcagattaattttagaattattgtaacatctgtagaaaaagaagcgtggatttatttggaatcgttaggaaagtgaaagattcaccggattaaaaaagccggtgacaaggataactccttgatcaccagctattcatcaggttttacaaacccggttactcattattttttataatcgacaaccatcacattaactgttgaatgccggacaacgtaagctgttgtggaacccagaatcgctctggatatcccgttgaccccggactttccaatgacgatcaacgaagcgtcatacttttcgggtaattctttggcaatttgaatctttgggactccaacaacgaagtgggtttcgactttagcgcccttcttctcggcaatttctcgggcatcgtccaaaatttcttctgcccgctcacggaacgactccatcacgtcctggcccagcgtcacgccgtactgaacataacgttgatcactggcgaccgaaacaatctgcagggtggcatcaaatgacttggccaaatcagcagcttcttccaccgccctcattgcattgtcactaccatcaactggaaccaaaattgtgtcatacatctccaacacctccgaatctgactatctaagttaatcataccattgtgtgatggaataaacataaatcaagtccggataaatctactcaaagctcagatgcgaaataattgttttgttatctgccaactcggcatgccgttcttttaaccggtcgtcataggtagcaagcagatatttttcttcggcagactcaccgaccaactcagggaaatggatctcactgatttcattggtgacgatcagcgtgcaaaaagccataaaggcaacctgaacgtctttggtcttggtatcggtggtcaaaaatttggtaaagacctccaccgcacgcttactgctgccagtgacataggagatgcacgttaaaatctcattgggccgggcaggtgataggaactggacatggtcatagcccgcggtcacaaaggacaaatttcccgggagaaatttcaccccggccaaaccggcattggcatccaaaattcgtaaggtttcgccgccaaattgaattcgattgttattcaactgggctggaaacacatagctttcatgaatcgccctggtgtctgagcacttgatcgtttcgatgataatcgcctccaaattcaacggattttcaatcacttgctaataaaatctacacatacaatgataaccttttcatgcctataatagcaagctttttaagtgttatatgaaaggattgtgaacgaaatattaaattattcagctgcttattgtaagcgatttcacataggtgtaaacttaggttgttgatggtaagaagtttttcattctaggaggtcataattatgaaagcagtacgtatttatggtgaaaaggatatcagagttgaagacgttgagattccagaaccaaaggatgatcaagttcaaattaaagttaaatattgtggaatttgtggaagtgatttgcacgcctatctcgaaggctggggcctgccaaccgttccttatccgttaaccggtaaaaccgtgccaattacgctggggcacgaattctcaggtgaaattgttaaagtcggtaaagacgttgacgacttacaagttggtgaccacgttgccgttgaaccacttttagcttgcggcaaatgtgaaaactgtcgggcaggaaactataacttctgtaaccgtgccgtttcaactgatggcgccggcaacttcctgggcttctcagaagatggtgggatggctgaatttgccaacgttcaaggggtctttgcccacaagatgccaaaagacatggactttgaattaggtgctttggcagaaccaaccgccgttgtttacgaagctatcaagaagagtcatttgcgtgaaggccaaaacgttgctgtcatgggagccggcccaattggcttgctggaagctgttttagctaagatcgcaggtgccaaccacgtatacatcgttgatgtttccaaagttcgtttggacaaagccaaggaattaggcattgaacatgtccttgacccaagccaagacgacgttgaaaagatcatcaaacaagacttaccaaatggtgtggacattaccttcgaatgtgccggcgttcaagcaaccttcgattcagcattgaaagttacgaagcgaaccggaattattcaagtagttgccctctatgcaaaaccagttaccatgaacatgactgatgacctgattatgcaaggtaaagacgttatcacaaccctctgctacaacaactcattcccgaatgtgttaggcattattgataatcacaaggatctgttcaagaaagtggtcactaagaaaattagcttggataatgcattggaagacggcattaaagctctctcaaccgataaatcacaagttaagattatgatcgatccatcactgtaatcatctagtaagttaacgagaaagtaggaagaccggcaacgatgaacaaaaaatgttcatcgttgccggtcttttctttgttagagaagttgctcattgggcttaaagaataaccaacagatattcaatccatcggcaaaaacatatgttataatcttcatatgaaaggaatgacatatatgactgatgaccccgtttcaatcaactcaatcgttctcattgataaccgacatttgtcagaatcggaacggatttttaaattacttagtaatcccaaccggctgcagatgctaaaagtccttgcgcagcaggaactgaacgtcagtgagctgggaaatctgcttggtttggagcagtcctacgtttcccaccaattagcattattaaggaaacatcagctggtgtcatcccaccgcgacggcaaagccaactattatcaactggatgatccccacatcctctacgtcatcaatgagatgctcaagcatgctgatcacgttatcaggggtaaaaagcatggagagtaacactgattcacaaacactagttgtccgcagcctccacactgaatacttttcaacggcctggatggctttcgaattcatggttgggttttattcaggtctcaaagccggctcaattctgttaatcgcatttgggctggatagttttttagagattatttctggaagcacgctcatttggcgactacgaaaggaaaatactggtgccggccctgaagcaatcgaacgggcagaaaagcgctcctcattaattgttgggatcgttttactgttgctggctgtttatgtcaccgccgtgtcactgtttaacctattcactcacgcaacggcagacaccagttattctggtatcgccattgggattgcctcggttttattaatgcccattttgatggtccggaaacagtcattgggcaaagcgctccactcagatgccctcgttgaagatggcatgtgcaacatcacctgtgcctacatggctgcgacagtcttaatcggcgcactgttaaccgcgctgctcaactggtggtgggctgactcagtcgcagctttgattttagtgtattttattgccagtgaaggatgggagtcgtttcaggaagggcatgccaaatagagtggggcacgaggcgttttgatcccggccatttaacgcaagtatggccaaagcatctccaattctattctcatttttatcattttgaatattacattgtggaaacgtgggaattaaagcagtttccggccatataagccagcaatccaaatatccaaacgcgggatattcggattgctggcttatattctggaaactaaccgctttaattcccactctggcttacattcccataaccagccgaattacaccaagcgaaataacccccactaccacaatcacgagcagatttttggaaatgactgctgccagcactgtcggcagtgaagcgaggaaattttcccagtcaatcgatggtaagtgaccgacgtgttgaacaaataaattctcaaaccatagcgctgacataatcgcaattggaacaaaactcaagaattccacgacgcctttagacagctgaaattttttcagcacgacaaacggggtaattcgagacagccaagtgacgatgcccgtgccaatgattgtcagcagcacaaaattaaaagaaggcatgtttcatcaccaccccaaagctgcaggccacaagggtcaccagcaaaattaataaactgcttgggatgaagatcaagcccaagtaaattgcaaccaacacaaacccgaccacgatcagttgcaagttgaatttgattgatttgtcgctaatcaattgcagatacagtaaaccaatgaacatcgctaccagagcaaaatccaagccaaatttttcaggattgctgatgaaattccctagaaccgcaccaaccaacgaagaaagaatccaagtcatgtaagaaatgacgttggcggtattgaaccaagcgaagttcagatggttatcagaataattcagcttgttcatccctaaagcaaaactttcatccgtcagcaatgtcccaaccaaaatatttttaaacatgctgtcatacttaaaataagaggccaaagtcgtgctcatcagaatcatccgcgagttgaccaaaaaaacggaaaaaataattgaaaaaatggggctgtgggtcaccagcatactgacaataacgaactgtgccgacccagcatatgtaataatggacatcaacgttaccaacagtgggcttaatccagcggctttgccgacaatgccgaaagccacaccaattcctatgtatccaaataccgttggcaatgtatcctttgaagcggcagaaacagttaaatcaccattcatttaacacactccttctttgtgacatgagaatgtaacttattagtattagtaaaattttaatggtgttctaatttaaagtcaatgatatttagataagaaaatcctgaagttcagtcattatactgaatttcaggattttgttagttagccagtgctctttggtaggcatcatacgtcccgggatcaaaacacaccatcgtcacatcaagcggtgcgtcaaacgttcgaatggcgtcaatggcaatcttagcagccttatcaagtggaaaatcatagacccctgtactaatcgagggaaaagcgaccgtctggcaatgattttccactgcccgtttgaggctattcacatacgaatttcgcagtaattgcggttcattgttatgtccgccacgccaaatcggcccgggagtgtgaatcacaaatttcgccggcaatctaaacccgggtgtaactttggcttctccggtcggacaaccattgagcttccggcaggcctcgtcgagctctggaccagctgcgcgatgaattgccccatcaacaccgccaccaccgctcaaggcggtattagcggcattcacgatcgcgtcaacctgcattgtggtgatatctcctttgatcaacttaaattgtgccatggtttcacatcactttctatgggctttctcccatgctttgatttgttccaaacgttttttgaagcggacttcattgccttgctcggtcggttcataatacgtgtggccaaccagagaatccggcattgtctgcatattagtcaacttatctttggcttcgtgagcatattgatagcccttgccataacccagcttggacatcaacgaggttggcgcattgcgcaactgcagcggcaccggctcgttaattgagtgcttgacgtcggtttcagcacccagggttgccttatacacggcattggacttgggggccaaggacaagtaaatcgcgcactccgtcaaatggacgttacattccggcatccccaaaaattggcaggcctgaaatacattaattgccacgttcaaggcgttagtatcagccaaaccaatgtcctcactggcaaaccggaccattcggcgggcgatatacaagggatcttcgccgccgctcagcatccgggtcagccagtacacggcagcgtccgggtcactatttcgcattgatttatggagcgcagaaataatgttgtaatgttcctcgccatgcttatcgtacagaaatgacttggtattcatcaactggtggagattgtcggtcgacactgtcaccttgccatcctgcttgggactgttgttaaccgccatttccaaggtgtttaaggcaaccctggcatcgccattggcaaattcggcaacttctttaaccgcttgatcgtcaatcgaaatggtttcttttggaaaagctgctggatttttcagcgtctgatgaatcagctgaacgatgtcatcggtctccaaaggttgaagcacgaatactttgcaccgtgataacaaggctgaattgatctcaaacgatggattttccgtcgttgccccgatcagagtaatgctgccccgctccacgaatggcaaaaaggcatcctgctgggctttattgaatcggtgaatttcatcgacgaaaacaattgtcttgccgcccatctcccggttcgcctcggcgtctttcataatctctctgatttctttgatgccgctggtgacggcactgaaagtgacaaacttggcctgcgtttttttggcaatgatctccgccaaagttgtcttcccaacaccaggcggtccccagaaaataattgagggcaactggtcactttcaataatttctctcagcactttgcctttgccaaccagctgatgctgaccgacaaattggtccagtgtctttggccggacccggctggctaagggctgattgccgtcctggttgccggcaaataatgattcctgtttcatgaagacacctcctgacaaatgaaactgctatgtatatgcccattatacgaacgcatgttctaaacgtcaactctacctttattttagcgcactcagctttcattgaccgaatttcgcaacttatggcctggctgattgtcttcctctcaggcaatgtcaaagtgacccgaattaataagactctcaagcaacgcaatcaatcccagaataaatcgtgatttgatgggtgataatttcccctcaacaataacaaacaggttataattaagctgaatttatgggctgtctgtttgttttttgagggagatggcaaaatgtcatataacaataacttctatcgggagccggcattttggctgagcatctgtgcggctgccgtgggcttgatgtccctatttcttggtaatgcggtccagtacagcatcatctggtggctgcaattgctgatcgtcgtcattgcactgattgggattttttatttcttttcgaaatattcaaaggatcaggaaaataagaataaacatttatagcactagaatcatcaaaggcgccccgtttctaaccagaaacgaagcgcctttaatgctttaactatgacaaattaatccgttttcgatacttccgaaccagtccgaggcctaacaaccccagccagccaacaatcgacaaagcggtgaacaagccattgaatttaactccacggctttgaatgctgattttggcttgcttgacggtctgtggaatggtgagcttaaaggtcccccgattcgaagttgccggcttttggatggttttgccattgaatttgaccgtgtaattcatcccggcatagtggacaaatggcaaatccaatgtggttccctttttcatcggcacggccagctggtaagaaagcgaattgttgcctggatgcaaactggccgtggcaatttcaaatcgctgtccgtttaaaatggtcaccttgttggccagatcatcaatgtgcttgccggcagtcattggtaagtaatcggtccgcccggaaccgttatcggttgggaactgattctgataatcctggttgttcaccttgtaattttgcaggttcaggttggaacgtggaatttgatgcgttggggttgctttgtaggttaactcaggctgactggtgcggttgaactgattatcatacgggttctgatcggtagctacgttcattgaatacatcgctgaataatcaaatgaattaatcagacaaagacttgcaacaatcaccagtgcactgacgccgatcgttctgcgactgaactgggttgccaacagataactgccaaaagcggcaatgaacattactaaaaccggaataatgcggtgcccactttgaatggcctcgattccattaagcaatggaatgtgatgaattaaattccatgggaacaagttggataacacaaacaacgttacaaaactactaaagtaggcatatcgaccaattggcggcacccgtttgatgaagaagcccccaaagatcaacagcagcaataaaatcaggccgattcctttgttggccagactctggttcagccaggtgaacaaactttgcggatctgcatacagtgtttgcggattcggtcgcatcaatttttggctcatcgccaacaccgcgatcggtccccaaacgatcagactcaaaattaaactataaacggcggcgatgccaatcttcatcaatcgagccgcccgttctttaaccggctgcttggtgaaaaaggccaggtaaaacaccaataaggcgatgaccacaatcaacgtcgtcggtgcgtgcgcgtacatgatcccggtaaccccaatggtgagcaggtaccagcgattagtatcttcgaacatcacctcgtaaagaccggcaaaggccagtgggatgaatgggtaggccagaaattcaccaaactgagtggtgatgatttccatcaccaaataagtagtcagtccatataagatggcaaaataaaatgaaattcggctggacttggaaaccaatttcatactgtaataagcaatcaccagtgtggcgaacacaaccaggacgtaggcaaaataaatcgcgctaatcggtgaaagcacgaaccgcagcccggcaaatatgtacagccaaatccatgggtagcaggccaccaccgcatccccaatttgattaaatgtccgggtggcaatgtggctgaatggcgctccgttttggagattggccagcatttcctcaatccggctcaaatgaaactgtaagtccgggccggaatagacgtgcatcgtcagccaaaacggcaaaactgcaagcaaagatagacaaaaaaagccgaggttgatgaccagcccctgatgctggcgaaacttggaaagtaattgttgagacataaaaaatggacctcctaataaaaattagcggtcccccctgtcgctgttgtattttatgatacgagatatccggtcaaaattcaaatcttattctgacattagtggatggtgcaaaaaacaactcttccaattatgaaagagttgtcttaatggggaaaataacacgtgtaaaaagattaaacttaacggtcaatcgtatccgcagtcatgtggaatacgtcagaaagtgaagtcgtcttgtcagcaaacttcttgttcaaaatcaactgacgaaaatcttcgactgagatattttcagtatctttaattgggaatgcctgaccggtgtatgaaccggttattaacgtgatcaccaaaccattcttgctgtccaaatgaacttggtaattctcaaagtagatcccatcatcataactaccggacaaaaacttgtgagttgcaaaatagtccgaaataaaatcattgaacttctcttttgaactcagtgcttctttaaattgtgtttgagttgcgactgtcatcgtaagactccctttctctcaaaattgtgtctaatcaaataacaacgcacatctatttttgtaaatggtctttatgagtcatctactaattttcattttagtccgtcagtcgcattgtgcaagtgaaaagctaatgaaaacgttgtcagaacgcaatttgtaacatttgcattctggcaacgtttccaattttatttattctttttcgacttctctggaactttttccaattcagccagcgctttttccaattcggccttctctgattctggcaggtcggggtacttaagcggtaattctttcattcggcgatcaatgatgtcagaaacacaaagtctggagtaccatttatcgtctgaagggatgatgtaccaaggattggtcttgttggctgtgtgctcaatcgcatcctcataggctttctggtaatcgttgaagtaacggcgttccttaatgtcagctgaggcaaatttccagttgtgatccggcagttcaattcgccgcttgaaccgatcccgctgctcatcggcagacatgtggaggaagaacttcaagaccatgaagccgtttcgggtcaaatagtcctcaaagaaattgatatccttgaatcggccatcgaagaatttgttatccacttgatcaagtttggtgatcgaaccaatcttagcgttgacaatcatttccgggtgaacccgactgatcagcacatcttcgtagtacgaacggttaaaaataccgataatcccatgttccgggatgtgtcgatgaatccgccacaggtaatcatggcttaattcaattgaggttggtgacttaaagcttgtgacctcaattccctgaggattaaccccgctcaaaatgtgtctgatcatactgtccttgccagacccatccatgccttgaaagattaccaagacaccaaaatggttttgggcatataatttcccctgcaaatcttgaagcgtcgcaatgttgttttcaattcgtgctttgatgtcatccttgttcaaatcttcaacggtggcggaagtcggaatcttggcaatctttagatcccgatccccgttgtatcgaaaagatttctcacggtcaaaaattttcttttcgtccatagtgttgccccctaaggaatcatttgtaacaactttataatagcttatcccttggaaaaataactaagagaatgtttattctccacatttatttctcatattgagtatactagattacatagaattagtttcatataacgctgttttagtgtcgcttgaaacatctatcaactctctttgaaggaggacttaatttgaatatcttaaaagcaaactcaacaactggtggccaacccgaccaaccagccgaagattcaatcgacaagtcgttattaaaggacgacctttacaaagccgttaacggccgttgggaaaagaccgccaagattccggctgaccattcgtcaacgggtggcttcatggatctcaatgacaacatcgacaaacaattaatgagtgacctcgatgacatcatcaaggaaaatcagccacacgaggagccgttctccgaattcttgaagttgtacgaactggcccgcaactataagaagcgggatgcagatggtggcgaaccactgaaaccgtatttggaaaaaatcgaaaacatcactaattttgatgatttgaacgaacttttgccggagctggttaaggaaggttacccactgccatttggcttttgggttgaacctgacatgaagaatacacaggtcaacgctttattcgctgcggttcccggcctgtttctccccgaccgaacctattatgaaaataataatcccgcttacaagcaattgatgccggtcttcaccaagatggccagccaattactggtattagcagactacagcagtaatgaagcggatgaaattgtcgaatcggccaaacgatttgatgccaaaattgcaccaaacgtcaagtccgctgaggaatcggccgattacagcaagatgtacaatcctcagaagtttgcctacttctcagaatcaagttctcatcttgattttgtcaatctggccgacgcgttgtttggcaaggcaccggagcagatcatcgtgaccgaaccgaagttttacgagcgctttgacggtctggttaacagtgacaccttcaaagacatgaagaactggatgctggtcaatatggtccgtttagcatccggctatctatcagaagaattccgtcagaccggttctgtcttcagccgtgcgctatccggtaagaaggaagcaacgccacagaagaaatcagccttctatctggcagaaggaacattcggccaaacaattggtgactattacgccaagaaatactttggcccgaaagccaaagctgacgttgaacacatggttaaaaacatgatcaacgtctacaagaaccgcttaagcaataacacttggctgggcaaagacacccgcgagaaggccattttgaaactggacaaactcgaactccaagtcggttatcctgaccacatagatgaattggaatacaaattcaaagtgacccctgaaaatgaaggtggcaccctatttgacaacatgtccaagtttggtgcgattaccgttcaagacacctttgaaaaattgggtaagccggtcgaccgaacaaaatgggaaatgagcgccgcaaccgtcaacgcttactacgaaccatttaagaacatcatcgtctttccagccgcaatcctccaagcaccgttctacagcttgaagcagacttccagccagaactatggtggaattggtgcggttatcgcgcatgaaatttcccacgcgtttgataacaatggttctctgttcgatgaattaggtaatttgaataattggtggactaaagaagatcatgaatacttctccaagctggccgacaagatgatcaaggaattcgatggcattccatttgcgggtggtaaggtaaatgggaagctgacggtttccgaaaacattgccgatgccggtggtctgagctgtgccaatgaagcggcaaagaatgaagccgactataacttgtatgacttcttcatcaactgggctaaggtatggcggatgaaggccacggaacagtataagcagctgctgttaaatatcgacgtacatgccccagctgaattgcgggccaatgttcaggtgaagaatttggatgatttttattcgacgtttgatgttaaagacggcgatggaatgtatcttgaacctgataagagagtgaaaatttggtaggaagcagacctattggaacgctttttatccaaataataatcgaataaagacaaaatggcacctaacctcaaaaaggtttagtgccattttttattcttaccatttgttattagaagccatttgttattagaagtgatcaataaccagccaaaagtagcctttgccggcccttgggcaaaaaacacgcttcttaggttcttaagcgctcccttcggcctctcaaatgtgttccgacggccgggtgaaaccctgcctagcttacttggcgacggcgcggaggctaacttctaagcgcacctgaactaacggggcttcgtatctctctgctcctcaaggagaaaagcacgtttgttaggccgttaagtgctctcttcggcctttaaaacagactaagcttgtgatgaattaaaacccgacggggctttagttcatcactttttggtataaagtgattgtgaagttagtaatgccgtgagcatatttggcgctggacgccgtctctaaaactggctaacttcactgttcttatacaaatctgctctaagtctgttggcgtttaacgtcgtgtattgaaaattagattatataagacttgaagcaacaactttaaaggtaaggtgatattttatgcgagtaacgtttggaattgatgtcagtaaagcaacttcggaaattgccatagtcgttaatgggcaagcggttagccattttaaaattacaaataatcagccgggatttaataaactccaaaaaagtttgaatgactttcaaaaccctgagattgtttttgaagcaactgggttatattcaaggagattaagagtgttcctagatgattatggttaccgctacactcaattgaacccattagcctcaaagaagcagcttgatcgactccgtcctaataagactgacaaaaatgatgccttacacttagctgaaactcagtttgagatcaggcgtgctttaacttatcagcaagatccaatataccagcagttacttgattggagtcgcttttatgatgagattacttgtgactcagtcgcaaataagaaccgacttcataaagcccttcagtgtacatttcccgaagctgattgcgttcttaacagtccaacagggcacttatattggcaccttttacaagcgttcccgattgcgagcatggtgcgacaaagtagttcaatggaactaagtcagcatatcagaaagttctgccagttatctgtcccaaatagccaagctttagccgctcggctacgtcaattagcctcggagtcctatccttgtgttggggaagactctggagtggttatgcaggtccgttatttggcaaccgagttacttagattagatgacttgaaaaatgacatcattcaaaaaatggctcgattagctcaagacttgccagaattggccattttggaaagtattccaggtatttccgttaatacagcagtccgcctgattggagaactgggagatatccgtcggtttacgagtgccaacaaactgaacgcgtttgtcggcattgaccttagacactttgagtctggcgaatatatcgccgtcgatcatattagtaagcgtggtaatccatatgcccgcaaaattctgtatcgaacaattctcaatatgatggtaagtgctcgcacaaagccatcccacatcaatgattattgccgggaaaggaaaaagcaatcttctggaaaggctgatttcaagaagattgccatgggtgcaattagtcgtcttaaccggactatttaccacttgatcctaaataaccagaaatacgattatctcaaaactcgaccaaaagctgagtcataaatctgattacgataatcataccagccttgtaaaaaatattaaattgttaaggcttatttagtttaccctcaaagccactttacctaaccagaaaaacaattaatttacggcacagccatgcccgacagaaaaagaatggtcttaaattgccggtataacttgactataggtagaaaatacgctccgacgcaactgaggcttgtatattaaagatgtcagcaaggtaacattaatttgtactaaactgatattaagcgctgtggattagtccatctgaggtacggatcctaacggatactggttacgttagactctaaccacagtcttttgttgtactgttgattagtttgataacacatatcccaagatatgatgtttcatttaatgcaagaatacagggcaagagatttgtggagcacagcgttaattacatacgtgaggagcggtaatgatgatttatgctggaattgatgttgcaaaatatgagcatcatctatcaattattgatgaccagggaacggtactattagctgatctggaatttctaaataatcgtgagggttttttgacggctcaagcgacacttgacaatgcgcggacggctgatggtcaagtccaagtgggattagagaataccggccattatggttataacttgatcagctatttgcgacagcacaagtttcaagtgtttgcttacaacccattactaatcaaaaagtatatccaggccaataccttgcgtcacacaaaaacagatccacaagatgcgttggagattgccaaaaagctaaggtcagataccactaaggttagctttgaagcagacgccgatatcattgaattgaagagtgatacccgctatctggaaggacttaagcgtaaacgagtaaaaaccaagctcgcatttacaaatgtcctcgaccaagaatttcctgagttggcgccaaatctagggccagtatccgcaaagtacagtcagtggttgttggcacttttgaagagatacccgtcaacagataagttggctcatggacgaatcaacacgatgacaaacatcattaccaaatactccatgaagcagcatggcgaggaaatggcaattaaagttcgtgaactggccagagaaacgattggtcaagcatctgatagtctttcatttcaactcctgcagttgatcgatgcgctacaatttgagacccagcagatcaaggaagctgatcaaaagatccacaaaattatgaatcggattaagacgccgctcctatcgattccaggagttggagaaacactagccgccattattttagccgaaattagaaatgtgaactactttcaatcaccaaaccagattctggcatttgccggtgctgagccctcaatcattcgctctggtgaaatgcaaggtaactacggtcacatggttaagcacggttcaacgcagctacgctgggcgctctttcaagcagccagactgtgcgcaatgtattcgccaaccatgcgagcgtattatcagaaaaagaggtctgagggcaaaccatatttggtggcattaagccatgtagtcaagaagctagttcgaattatttaccacattctaaaatacaatgacccatggtctgagacggtgattagagattaaccaagcctaaaaaccatgtaattatcaaattcaaaaaataactatttttgaagcttatttcttatacgctcaaaaatggggtaataaacttcaataaagtcattatttttccttgacgtaatatagtttgtctaacttctaagtgcactttaattaaagttccaaacccaggaacttcaatcaaagtgcacttagaaaccgcctctcccggcccttgtcacgctctgactttttgccccgcatacaccgccgcaccgaccattcctgcttcatcgcccagctgcgccgtctccagcttgcaggcttcacgggcaaccggcagggaatgatgcgccaaggtttcgcgggtatatttgaacaacggctctccggcagccgagacgccgccacccaggattaacgtttccggattaaacaaattaatcacgttgcccaacccaaatcccagcaactcgccagtttctttaaagacttcaacagcggttggatctccttttgctaccgctttcgagatcaatttggtggtcagttcctgcccttgtgacatccattcacccactaagctggtttggccgtcagccagtttttcctgcatggttttgacaatcccgcgagcggaaacataccgtcccaaacagccggtactcccacaagcgcacggccgaccgtggcggtacatgttcatgtggccgatctcaccgacactattggaagcaccatataacacttggccgttaatcagaacagctgcgccaagtccggtaccaatggtgaccaagacaacgtttcgatgacctcttccggccccaaacgccatttcaccgtacaaattaacccggacatcgttgtcgatgaagaccggttggcccagcttatcctgcagccacttggcgaccgggacatccttccaatcggtaaaattcggtgaaaaaattgaaatccccttttccacatccatttgcccgggaatgccaaaaccggcagccaaaatatcatctgaggtaatcttttcctgagccattaattgctggcagcacgcccagatccgattcagtacttcagtaggaccggcctcttcatgagtcggcttatgtaatttttggaccgtttgaaaatcctcatcgaacagtccggccttaatgttggtcccgccaagatcaacacccaaataatattttgtcatatcgtccacctcacaacagcgatcaattcaatcaaaaacgcttacttactatgataataaccgattagactgcataaagcttccaaaaacattccaatcaccatcagatacatgacgaccatattcatgcccagataaagcagaatgcccatcaccaaatacaacagtacaaagaaccaacgtaaccaaatattattaaccatttcgatcccctccaaatccattttaactcttacattagaatctttacaatctgtgaacaaataatttgtaaaaacgcggttttaatgtaaactaatgattattaggatataatatatgtaaagagtaattggagaggtgataccatgaacttaacagaatatcttcattcgcagctcaagtttttaaatgaccagatgagttccgctaagaaagataaagacgaaacgatgcaatatctggtagattcaaagattacagaagtcaaattaatcttggaagccctccaaaagggaatcatcgatggaataagttaaaatgtggccgattggccattttttatgttttaatagactagtgcgtaataaagtttgattaaaaaaggaagtagaatattgattacattaaaatcaccacgagagattgagaagatggctgaatcaggtgctgttctggctggcgttcataaggaacttcgcaagatgattaagcccggtttggacacatgggacatcgagttgtttgcccgccgctatatcaaagatcacgacgcctacccttcagaaatgggctttgacggctacaaatttgcgacatgtatttcaattaacgatgaagtcgctcatggaattccccgtaaaggcttgaagttaaagaacggcgacatcctcaaagttgatatgtgtgtcaacaaggatggcttcgaaagtgattcttgctggacttatgctgtcggtgacgtcagcgatgaaatcaaaaaattaatggaagttacccgcaaaggcttgtaccttggcattgaccaagctgttattggtaaccgtcttggtgacattggaaatgccattcaaacttacgttgaagatcaaaaccacatgggcgatgtccgtgaactgattgggcacggcattcagccttccattcatgaagaacccaacgttcccgcatatggtgtcccaggccaaggccttcgtttgaaggaaggtatgacgatcaccatcgaaccgatggttaacaccggtacttgggaaattgccgaccgttacgacaagaaggatgactggacatactacgtttcagccgatggtactccttcagctcaatacgagcataccttggccattaccaaagatggtccaaagattttaacctcccaggatccagacattgacgcaaaatatctgctttaatttaaatcatcaacaaacggccgggacatttgttccggtcgtttgtttagattaaaatagatgtgtagaaccaattagtaagaaaatcaccacattatttgtatggggaggaatgattgcatgaacaataagaactttaaatttcctgacactgctgcctacgaatttgttattcaagcgctcaaagaccgcggggtgacctatgaagacatcgccgagatggcctataatcttcaaaagaaatttgtccccaacattcaaatggatgaagtcaaaaaagacaccatcgacgtgctccacaaacgagaggttctcaataacgccatggtcggcctggagctggatcgattggcaactgaaggcaaaatcaaagaaccccttgaaagcatcatcatgaatgattccggcgtttttggcgttgacgaaggtattgccttaaacattgccaacatctacggcacgattggaattaccaattatggctttgttgaccgggaaaaaactggcgtcacaaaaaaattggatgaagccaaagacggcacatccaatacgtttattgatgatattgtcggtgcgattgccagtgcggtctcagcgaagatcgcccaccggaacaactaacgccaaccgtgtgatttttgatcataatcccgctttttaataccggaaacatagggattgcccttaacaaaataccgcagcggcttggtcgcccaagtcccttgattcgcaaccccgattcgattagattcttcaatctgaatggggatttttttgtcgtcttgatgaatatttaacttgctgtcaccaaagatttccatattcatgtctttatcggcaatcccaaaggcttccatcaattttcccggaccattggtgagctcaacgccatggcgggtgcggttctgttccataacggctaacccaattgttggctcaattgcccggattagaatcccctgggggacgtcttttgcttgagccgcaacatccaagaggtatcgcccatgaatggaatagatgtacactgttcctggaggcccgtaaagcggttcgttggaagctgtccgccggcccttaaaagcatgggcagccgaatctttttgccccatataggcttcagtttcaacaattcggccacccaccagacctttgggggaatcataggttaaaagcatccccaacaatttcttggagatttcgtcggtggtgccgttagaataaaatgggtcttggtccaaatcaaccatccctttcaacaaatggaggttatcacatgcaattaaaattagaacgaatttacgataagccgcaggatctttccggctaccgagtcctcgtcgaccgcctatggcctcgagggatttccaaagtcaatgccaagctggatgaatgggaaaaagaaatcgccccatccaaagagctgcgaacctggttctcacatgacccagaaaaatttcccgattttaaggaaaaatacgtcgctgaacttgatgccaacccacagaccaaagatttcgtcaaactaattggtgatcagctcaagaatggcaatgtgatcctgctttatggtgccaaagatcgtgagcataatcaagcagtcgtcttgaaacagtacttaaccgatcacttaggccagctttgacgaatattggccagggtcaattctttagttgattcaaagttaatatcggccattgttagaacttccggatcaccaacaccaattgagaccacgttagcagcgttaatcgactcgacgccgacaatcccgtcatcgatgccaatacattgatcaacgttcaggtggagcatctcagcggcctttaaatacacatcgggtgccggcttgttatgcttgatgtcggccaaattcacaatcaatggaaagtaatcttccaattcaagtttgtggatctctttaggcgcattagccgaggccgaagcaataatcatctggtagtggttcaaccggagctcggctagaaagtcgcgaatccccggtaaaatatcatctggattcatgatctcaagcatttgctgataaatggcgtttttcttgtcagcaagtgcttctttttgctggtcagaatatttgccaaccaacccgccgactcgtaaaatctcgtttaacgaatcgatccggtcacggcccttgatcgcctcttccaggtcttgattccactgcacaccaatcccttcggcaatctgacgccaagattggctatggtaccgccaggaatcggtaatgatgccgttaagatcaaacaacacccctttgatattagcaaaatcagtcatttcaaacaccctttcttacaaaaaaagactgaaaacaagattgtgttttcagccccagcggcagcttgaattatttaacagcgttaaagatccaagtgatgccatacttgtcaacaatctggccgtatttgttgccagaagttttcttttcaaaagttacgattactttgacttcttctgattccaccactcgctcgtacaaatcctgcaacgaggaaagggcatcggaatcatgcagatcaacttcaaacatcagcgaaatcatcgaggaaatcaccggcttacctaaaaaactgtccgcacaaaaaatctgcttgcctaaaatgttgaaactggcttgcatcgtaaggtcgtcgagattgacatcgtcattaagcgacatgtcttgcgcctgcttttcagttggggattcacgttgaacatccgtggcaccaaaaacagtttgataataatccaaagcttctttggtgttttcgaacgtcaaatatggaattaaattaatattactcattaggtcagcaacccttacattttaatattattcaaagtttagaatacctttaaatacaatagttgtcaacgtcaaccgtctgccaatgcctattctgataggaaatggcgtcctttttggtaataatttttggaaaagtgatagacttaaattaaacggatcgggaggaactatttaatgaaacttgcaatcacaatttttgtattaaacgcgttatacatttcgattaataccttcagaacaatgctggttgtgaaaggccaccaatttttagcccccatcgtggccgtcggcgaagagtttgtctacgtgatggccttggcgatcgctttgcagcatattgacagtccgttaaacatcgccgcatatgcggttggattcggtgttggtatctacattggaattgtcatcgaagataagatcgccttggggtacgtcaactttgaggtaaccgtccagattgacccgacgaatccgattcatgcccacaatgaagagttggccgaaaagttgcggaatctcggttacggtgttacggtcagccgtgctgaaggccgctcaggagcccgtctggttctcagcattctggctcccagaaaagccgaccgccgtttgatggaacaaatcaaggaaatttcacctgacgctttcgtcatggttcaagaaccggttcaattatccggtggcttctggagtaaagaagttgaccgtcgttatcattcaaccaatcatatgcactaatcgtcatcttcatcgaataagccgagctgtttgagactattttcaatatcttgaactgaagttggcgtcgttggtgccgtttttcgatgaatgggctttggctgccttggagttggctgttgtttgatcggttgaggtttaggaattggctgtggaccctgcttatccggagtaacggcagggctggcctgcggatccggctgacccatttgatccatggtttggtttaacaggtggtcgacaaaaacatttccctcatcgcctgcgtgtcccttggtccaataataccgaatgatcgggaaatctctcagattggcatcaactgcttgccaaagctgcttgttatgcagcttcgagccgtcactcttgttccagccgcggcgtcgccaaccagccagccagcctttttgaatcgcatccagaacatactgggaatccatgaccacaccaatccgctcattttgcagaccttggcgtttcaaatacttcagggcttccaagaaggccattatttccattcgattattcgtagcaccaaattcgccaccggattcgaaatatttttgactaccagtttgaactaaaaatgcccaggctgctttatcgctggcttttacgtggccgccacgatggttcccgtggttgcgcgacccgccgtcggtgtagacgatgatatcaccatccggttggactgagcggcggcccgttgaagcctttttgtgagatttgtggtgtgtcttagtgggcgacgttgtttttttcgccccgttgagataggcattggcttcggcttcggtcttaaaacttttatattgggcaccggaaaatcctttaactttcttttcggcctcgtcccaactagtaaagataccggtctttcgaccttttttaactgcgtaatatttcatgaaaatcatggctcctcagtgtaaaaatttcagaaaaaatgttaattattaattataatgtttctatctactttgcaattagataaatctatgcgaaaatgttaataaaagggggcaaatttaatatgacccaaactaaagccacattgatctcggtcattgaagccaaagcacttctaaaagaccagtcagatcaaataaacgagcgttttccccgattaaaaaaacaaggtaagtatattctacctgattatcggttaacaagaaaacgtgaagctttcaagattcgaaagcatacatttttacagcatcacgcacgttcctacgttgcatttgattccgagaacggacagacgctttggatgcacaactttccaagcctgaccgaagccttgttttggttggataccggtcttaaacctaccgataccgacactaacacatcgtataagtcatggaaagatctgcacgaagatgacattaacgccctcaaagacattttgaaggaacgttctcgtaaacgcaaggaagcggcggctgccaaaaaagctgcctcggttcccaaaaagaaaccggcggctgtcaaaaaatcgacagttgttaagaaaaagaaagctaactaattcgttattcgaacctaaaaaaggtatgactgtgaatgaaagatcattttgttcacggtcatgcctttttattgtccatttagttattgataatgaccagcaatgtcgtctggactaaaatctgtggtgaattgacgatcataagccttttcataggcagcaactttttgttggtaatcaatttggcgcatcttttcagcagcttcgcgctgtgatgtggtcgacttttcgaccgcatccggataaatcggcggtaacacatggaccgtataattgatgccatgcggatccgatttggtcggggcgtcaaccatcgaaacaaagcaggacacgattggcacattcaatctaacggcgtagtagtacgctccccgttcaagcggccgcggtttgcgatagttgaaccacatttcccgttccggataaattagaattgattgtttgcgtgccaagctactttgcaaaagggcaataaaccccttgcccatgtaattgacgctgtcgctgacaggaatcgtatcagcgtatgtcatcaaaaatcccagcatcccgggcattttaagattggtgagctcaacgacaatcgacaaatcaggttgattcagggctgatcgaaccagcaggctgtcaatcgggctaaagtggttacaggtaatgattgccggccattctaaagcctttaaattgtcagttccctcaacttttaaattgggattcatcatcctcgcagccatattcatgaccgaccgggcttcagctgcccgccaatggtaacgtttagtttggtgaagcttcaagaagtggtccaacacctcatgctgctcggtgagtgtcagtactggatcatgtagttcgactttttgattaaattttccctgacggacgttttcagcaatgttttgaatcactttgtcacgctcgccaagctttaccggtgtaaaagtcatagggcaatttttactccttgcttggcccttgcgtaaaatgtcgttggggtcttaataatatcaacggctaattgaatcaaatcggactgattcttctgatcacgggcaacttctttaggattcatatctgcgagctgctgtttaagcatagtctcgtaatcagtttgtttggcataggtccaaaaatagctttgtcgaggggcatcatcataacgccacggcttggcaaataagttatagtgaatcaaccagggttcaacatcctgtggcgtagtgatttggatattccatgacgggttcaaataataaattcgatttctcgcgatggcattcatgtagtcctgatccggcgccaaactcttgaaatggtacttgttcaaaagctgcaaaaagtgttcagcgaattttgaacggcgcatttcggcgaggttcatcaacaacacgccggaattaacgtatttctgtgaatcaatcccaacggcttgttcagcatagtcaatcgtttccggagtgtggccgatgaagtgatccggcactgcgccaaccaggttatcacccagctgagtatcaaataactcacccacatcctttaaaaccaccgtgtctgcatccagatagagtgccttatccaatttggggaacaattcagcaataaacagccggaaataaattgtaaaggtaaagtaatcgctgcgaagtttgttattcttatcagtaatttcttgcttcaagcggtcattaattgaaacaaactgaattttgagattgtctgtttcaaaggctttgagccgcccttgattgtcggtattgagatcatcacacaacacaatcacctggtaatgcctgtccggtgatgtatgcgcgaccagtgaagacagtgaaactgccaaataaggtgcataattgtcatcgacagcgtaaaaaattggcacggtttgattttccataatgaatcccccttaaatcaatgtgattgatgctggtaggtcataaatgacacgttgctttggtgactgcgggtcaccatttgggcatgaatctgatcatggagcttttgttggcgttgcttgcgcggaagtgacttgtccggcataaacggaccgtcaaagtataccacctgcttgggtcggctcaacagtcggcctttttgatatgtaatcgtcatgctgtaactgggcagatcggcagcgaccggataatggaaagcgccgactggaaacggacgaatcttggtgtaatacggccaaacatgggcttcagggtagatgaacactcgttgatgctggtccaatcgagcattcattgcccgctgaaattgaatcatttgtgataatttggcaggtaagatcaacgccccacccatcgttaaaagacggccgacgatgggaataccaaggttggcgggttccgcgatcggatacgcccgcctgggtactgccaccagcatcggcaaaagcgcatccccaagcggctgggtgtgattggcataaatgaaggcgccccgtttgccttgggtgcgcagacatcgcttattccgaaaagacgtccgcaaatacaggcgacaataaacgaagctgacaacaaccgccacccagtagacgaccgtcgccgttacgcggtaaaaccaattttgatgcagccaaatgtagccctcaggaatggtggcattttgattcttggtaaagaccacgtcatcatcaaaatcatgatacgtaaacacttttgatgcccgtttagtcattaccaatgtcaccctttcttccgacaagttaaaatcatgaacagaaccattctaccccaaatatgacattattttatcatacaggacgtttaaaaatggcaattcgctaaaaatcgtcctttaaatgattaaattggtgtaaaattaaggcttgctatgctaggatatttgggataacaatggatgtatacacatcattagaaggatttaggggataattttgatgcaagctcagtccaagaacaatacaaagtttaactttaaaacatttatgggcctaatcaaccgaattcacccccgttactggcaactgctgcttggtttttttctaggagttgtcgcaacggcgatgcaattgatggttcccggcatcgccaaggggatcatcaactcaatcggtcattcaatggatgtcggcctaattgttgccgtcattttactattcgttttcagtaccattatcggagccttttccggcagtattttaggcttcttcggcgaagacgtcgtctataagctgcgaacaacactttgggataagatcttaaccctgccggtgggttattttgaccaaaccaaatctggcgaaataacctccaggttggttaatgattccacacaggtcaaggaactgctggccaattcggttcccaaaaccgcaacttcgattctgcaattggttggcgcattggttttaatgctcatcatggactggcggatgacactcattatgtttatcgccgttccactcgtcttgatctgcctgctgccaattgtccgccaatcccacaaagttgccagagcgagacaggacgcactggcagatctcaatggtaaagctggtgaaatgctgggcgaagtccgtctggttaaatcgtctacggcggaaaacttagaacgaacagccggcgacaaacggatgtatcgcctttatcgtatcgggttaaaagaagcgatctatgattcgattgccggacctgtcatgggcatggtcatgatggccatggtcctgggaattctgggctatggtgcgatccgggttcgggaaggtgccattgatattgggaccttattttcatttctgatgtacctggttcaaatgattagtccatttgcggttcttggccaattcatgtctgatgttgccaaggcaagtggctcaaccactcgaatccaggcattattgcaaactcatgaagaagatcatctgactggaacggatttggatattggcgatcaaacacttcaaatgaaccacgtcagtttttcttatgatcagcatcaccccgttttgtctgacgtgtcgtttacggcagaacccaattcggtcattgcctttgccggtccatccggcggtggcaaatcaaccattttcagcttaattgaacgcttttatgaacctaacgagggcagcatcacgatcggcaataccaatattactgatattcaacttgccgattggcgccagcaaatcggcctggtcggccaagacgctgcgatcatgtctggaacgattcgttacaatttaacctatggtttgccgggacatttttccgatgagcagctttggcatgtcttggaaatggcttacgcaacgcaatttgtccaaaagatgccccagggcttggacacggaagtcggtgagcgtggagtcaaggtatcgggtggccaacgtcaacgattggcgatcgcccgggccttcctgcgtaatccaaaaatcttaatgttggatgaagcaacggcgagcctggattccgagtctgaaatgatggtccaaaaagcgctggaccaattgatggctaatcgaacaacattggtgatcgcccacaggctaagcacaattaccaacgccgacgaaatttatttcatagaaaacggcagggtaacgggccagggaacccaccagcagttggtgaaaacgactcctttgtatagggagtatgtgaaaaatcagagcgcgacaagacccggttagggaccggagtacaaagagaatcaggccatgatgaacgtttcttgttcatcgtggtctgattctttttgtacagtaggtccctgggtcgtcggagcgtattttaaaagccgaaggatcctcaaaataacataaccacatcactgcgcgacaagcaacgggtgaggcggtttctaagtgcactttgattgaagttcctgggtttggaactttaattaaagtgcacttagaagttagacaaactatattacgtcaaggaaaaataatgactttattgaagtttattaccccatttttgagcgtataagaaataagcttcaaaaatagttattttttgaatttgataattacatggtttttaggcttggttaatctctaatcaccgtctcagaccatgggtcattgtattttagaatgtggtaaataattcgaactagcttcttgactacatggcttaatgccaccaaatatggtttgccctcagacctctttttctgataatacgctcgcatggttggcgaatacattgcgcacagtctggctgcttgaaagagcgcccagcgtagctgcgttgaaccgtgcttaaccatgtgaccgtagttaccttgcatttcaccagagcgaatgattgagggctcagcaccggcaaatgccagaatctggtttggtgattgaaagtagttcacatttctaatttcggctaaaataatggcggctagtgtttctccaactcctggaatcgataggagcggcgtcttaatccgattcataattttgtggatcttttgatcagcttccttgatctgctgggtctcaaattgtagcgcatcgatcaactgcaggagttgaaatgaaagactatcagatgcttgaccaatcgtttctctggccagttcacgaactttaattgccatttcctcgccatgctgcttcatggagtatttggtaatgatgtttgtcatcgtgttgattcgtccatgagccaacttatctgttgacgggtatctcttcaaaagtgccaacaaccactgactgtactttgcggatactggccctagatttggcgccaactcaggaaattcttggtcgaggacatttgtaaatgcgagcttggtttttactcgtttacgcttaagtccttccagatagcgggtatcactcttcaattcaatgatatcggcgtctgcttcaaagctaaccttagtggtatctgaccttagctttttggcaatctccaacgcatcttgtggatctgtttttgtgtgacgcaaggtattggcctggatatactttttgattagtaatgggttgtaagcaaacacttgaaacttgtgctgtcgcaaatagctgatcaagttataaccataatggccggtattctctaatcccacttggacttgaccatcagccgtccgcgcattgtcaagtgtcgcttgagccgtcaaaaaaccctcacgattatttagaaattccagatcagctaatagtaccgttccctggtcatcaataattgatagatgatgctcatattttgcaacatcaattccagcataaatcatcattaccgctcctcacgtatgtaattaacgctgtgctccacaaatctcttgccctgtattcttgcattaaatgaaacatcatatcttgggatatgtgttatcaaactaatcaacagtacaacaaaagactgtggttagagtctaacgtaaccagtatccgttaggatccgtacctcagatggactaatccacagcgcttaatatcagtttagtacaaattaatgttaccttgctgacatctttaatatacaagcctcagttgcgtcggagcgtattttctacctatagtcaagttataccggcaatttaagaccattctttttctgtcgggcatggctgtgccgtaaattaattgtttttctggttaggtaaagtggctttgagggtaaactaaataagccttaacaatttaatattttttacaaggctggtatgattatcgtaatcagatttatgactcagcttttggtcgagttttgagataatcgtatttctggttatttaggatcaagtggtaaatagtccggttaagacgactaattgcacccatggcaatcttcttgaaatcagcctttccagaagattgctttttcctttcccggcaataatcattgatgtgggatggctttgtgcgagcacttaccatcatattgagaattgttcgatacagaattttgcgggcatatggattaccacgcttactaatatgatcgacggcgatatattcgccagactcaaagtgtctaaggtcaatgccgacaaacgcgttcagtttgttggcactcgtaaaccgacggatatctcccagttctccaatcaggcggactgctgtattaacggaaatacctggaatactttccaaaatggccaattctggcaagtcttgagctaatcgagccattttttgaatgatgtcatttttcaagtcatctaatctaagtaactcggttgccaaataacggacctgcataaccactccagagtcttccccaacacaaggataggactccgaggctaattgacgtagccgagcggctaaagcttggctatttgggacagataactggcagaactttctgatatgctgacttagttccattgaactactttgtcgcaccatgctcgcaatcgggaacgcttgtaaaaggtgccaatataagtgccctgttggactgttaagaacgccttcagcttcgggaaatgtacactgaagggctttatgaagtcggttcttatttgcgactgagtcacaagtaatctcatcataaaagcgactccaatcaagtaactgctggtatattggatcttgctgataagttaaagcacgcctgatctcaaactgagtttcagctaagtgtaaggcatcatttttgtcagtcttattaggacggagtcgatcaagctgcttctttgaggctaatgggttcaattgagtgtagcggtaaccataatcatctaggaacactcttaatctccttgaatataacccagttgcttcaaaaacaatctcagggttttgaaagtcattcaaacttttttggagtttattaaatcccggctgattatttgtaattttaaaatggctaaccgcttgcccattaacgactatggcaatttccgaagttgctttactgacatcaattccaaacgttactcgcataaaatatcaccttacctttaaagttgttgcttcaagtcttatataatctaattttcaatacacgacgttaaacgccaacagacttagagcagatttgtataagaacagtgaagttagccagttttagagacggcgtccagcgccaaatatgctcacggcattactaacttcacaatcactttataccaaaaagtgatgaactaaagccccgtcgggttttaattcatcacaagcttagtctgttttaaaggccggaggagctcaaaagagcataaccgcaccaaccaattgataatctttccgcccctgcgcaccaatccaatcaagacaaaatataaaaagagccaatcattccaaaaacaggaataatcagctcgttcattaaaattctaagggcaacacatctcgcatcgcaccctcactcagttttcaattccccttcagcatccaattcagccataatctcttgatactccgctaaaatatcatcatattcatgcaaatgaagttgctgatgaactttatcaacttcccaaggcttgaccgaaaccgtgtggacgatcggccataatttccaccgggtggagaaatgttgaaaaacggtgtcagattgaacatcctgctgctcattgtatttttcaggggcaaaagccttgtgcttagccagcttattcattgcggactggtccggcataatcatcggccattttcgacagtactcccggcagcgggccagcaatttgtcttggcggatcatgtccagattcatcaggagcatccccgagttaatgtaatcaaatgctctaagttgatgatggaagaaccaacggccgtaatgatccaagacgccaacaaaatcagttcctgccagtgattgatgataaaaatcttcaaacggccggcgacacacaacgtcagcgtccaaatacagaattcggtctgaaaattgcggcaccaaatcactatacagccgcaacatactatagggcgtgaataacgtgttgatgttcgccttgggcaaatccgcctcaaactgagtggtaatgtcaattttggtaacgccactatcgacattttcccgcttgaccagttgattcaaaaaggctgcgtgatcgtcagtcagcgcttgaaattgctgatgtcgattatacaattgcccagttaaaatgtagatgttgagtggttcttgcgcgtgttttgtcagtgagaggattgaaataatcaatcctgaaaacatgtggtcatctccacaatataaaatatccaaaccgcattcatcccccaattcgtgtctcatcaatcaaagtgtgtcatacttcctgataaatggcaactaatgaccttggaaatccccccacaattcaaaaaggcacccagccgacgcagcaatgtgtgtcaaaaggctgagtgcttttaaattaatcttcgaaatagtttttgacctgtttgggctcagtttgaaccagaatcttaccattgtgaatggagtagagaatttctgagcgttcatttaacgcgttatagaaattatcattattcataatgatacaattagccggtttaccgacctggatcccgtagtggccagtgatatgcatcgccttggcaccgttagtcgtaataaactggtaggaattcataatatcgtcgtaccccatcaaatggccaacgtgaatccccatctcaaccgggtcgagcatgttaccattgcccattggataccaaggatccttgatgtcatcttcaccaaaggcaacgttgatgccatcctcggataactctttaacccgagtcatcccccgccgctttgggtaggtatcgaagcggccgccaaggttggtattcactaacggattggcaatgaaattgatgtgagacattttcaggaggcggaacaacttgtaagtataggcgtcgttatacgatcccatggcagtggtgtgactggcggtaaccttgtcgcccatgccgctttcaagtgccaaggtggccaaaacttccaagtttcgtgaagctggatcatcaatttcgtcacagtgaacgtcgaccagtttgcccttgctttcggcaactttcatcaagaatttgagtgactcaacgccgtagtcgcgggtaaattcaaagtggggaatcccgccaatcacgtcggctcccatgtcggcagcggcaatcatcaattccttgccatttggataggataaaatgccttcttggggaaaggccaccagctggagttccacttgatcggcaacctcgtcacggacctcaattaaagcctttaaagccgtcaaatcgggatcggtcacgtcaacatggctgcggacaaattgaatcccgttggcaacctgaatcttaagagccttttttgcccgcgtcttgacatcatcaatcgtcagctttttctttcgctcactccaaattcgaatgccatcaaataaggtcccggattgattccattcaggatcaccggccgtttgggtcgcatccaaatgaacatggggatccacaaacggcggcaacagtagtttatcggtggcgtcaatcacctgttcaccgtcgccaggttgaattgaggcggcaattttgacgaacttgccatcctcaattttgacgtccctggtttcttcagcgttttcaatatggacattttttatcagcatcagattatccctcacaatcaagtatttaataacattatagtctattttaatgccggagttgggcgcaatcggtggaatgtgcgataatacagatgacatcattattagaaattggcatttctgccaagtgaaaggtactgattctttgaacttaaaaacccggttggcactcccgcagattttaacattgggatttctcatcatcattctggtgggaacttttctgctgtcactgccaattgccagcaaatccggtcacatgaccggctacattaacgccttctttacggcaacttcggccacctgcgtcactgggatgaccgtcgtcaataccgcgcttcattggagcgttttcggcaaaattgtcatcttgatgctcgtggaaatcggtggtctgggattcatgacctttgcggttctcctgtttgttttcatgcgccgaaaagttgatctgacaacccggttgttgactcagcaatcgctaaacctgcagtcatttgccaataccagttcggttgtgtttttggtggtccggatttctttggcgattcaagtgttgggaacggcactgatttttatcgatttttatccccggtacgggtttgccaaaggcttgggctacagcatttttcattcaatcagcgccttttgtaacgccgggtttgacttgtacgataacagtttggaacaatttcagaccgatccatacctgctctttgtcttgacgattttaattatttcaggctcacttggctttctggtctggaaagatattcttttctacaaggaagatcaccatttaagcctgcacaccaaattagcattgacgacttatctggggctgattggcctcagctttgtggtgtatatgctgactgaaggcaacttcggccaggaaagtcatttaaccatgttccagcggatcatgaacacctggtttttggcggtcactcctcgaacggccggcttttacaccctgccggtcacccatatcacaatgggcggcatgttcttcaccatgattttgatgctgattggcggaactcccggatcgactgccggtggtatcaaaacaaccacagtcggcatcctgctgatcagagtgtggtcaacattgcgcggcaagcgggacgcaaccttttggggccggcggttcagtaacgataacgttacccgttcattgtcactggtcttcttggtggcagtggtcttgtcgatagcaacgatgattctaacgtttacggaaacgatccccaaaaaccagggattggaatacatcacatttgacgtcatctcggcattcggtaccaccggctttagcctgggcctggtggcgcacctgagtgtcgtcggtaaattaatttttgcggcgctgatgttcatgggcagagtgggtatctttacggtgatgtactcactgctcaactcaaagcgcccggaagatgctttccggtatccggaggagaatgtgatgattgggtaagagtgcggactagggcggttagcaaccgtagtctaaggtgcttccaacggaaatcgagtttgattttcgttggaagtatcttaggcgcaggttgctgccctagggagcacgcctccactaggtaaaataaaagcactaacacctctaagtgcaatgagtgttatgaatcatattttcaagctaaacactattaaaaattaacccaacaaccaaaaggagcaaaacaatgaaacaaaactacgcagtcatcggcctcggcctcttcggttccagtatcgtcaacaccctgctggaacacgatcaggaagttctggtcatcgacaaaagcgaagctcgggtcaacgaatttcgtgaccgggcaaccgaagcaatcgtagccgatacgcaaaatgagttagccttaaaccaactgggcatcgggaactttgacaacgtctttgttgccattggaaccgatctggaagccagtatcatgaccaccatgatttgtgaagaattaggtgtcaaaaacctgatctgtaaggccgaaaatgcccgccatgcaaaagtcctggaaaaattaggtgccgatgaagttatccagccggaacgagatatgggtcagcggattgccctgcacgtgatggagcctaagattctcaatgatttgaagctaaagggtgaattgtcggtgattgaatttgaactgaccaatccaaaactctttaacaagacgctcaaggaactcaacttaaccaatcgctacaagatttctgtcatcgccctctcccacgcggacgagaacggtgcgattatcccgaatcagtcaacgattactaaacctggtgacattgtgacgattatcggcactgagaaagatgttgaggcatttgaagcagtggccacggcataaaaatagagtcagacagcttggttagctgactgactcctatttagtgtgaatcatgatgttaaacaaattcaaaaaaattacttagcaggcttttgcttcaagaaatgttgcaagtctgataattctttgtttcgcttaatatcttttttacggttaactggacgacgtccttgtacgccgtgtggatgacaaattcgcataattagactctccttattttgtattatgatttcataattccaatagactaaattattataatacaagtttaggttggaacgcaaatcaatctgcggtttctctatgatttctaatgaaatgtggtattcttaataattaaatgaacagttgaggtgattaatttgacagaacaatatccacaggcactgacaattgcgggctctgacagcgatggcagcgccggcatgcaggctgatttacatacattttttagacggcacatctacggaacggctgttatgaccgccgcggtggcaggaaatagttacgggattcatgattcggtaaccctgccgacatcttttattgaccaggaatttaaagatttggccgacgattatcatgttcgggcaagcaaaaccgggatgctggccgacacagagttgattcgcaccgtcatcaagaactatcaaaaatacgatttcggcccattagtggttgatccggtgattaccaccaagcatggtaacatgcttttggaacaaagcgcctaccagacgcttcgcgatgagctgatcccgctggcaaccgtcatcactcccaacttctttgaagcccaaaaattggctgaaatggacattaacactcaggatgacatggttaccgcagcccagaaactaaaggatctgggtgccgccaacatcatgatcaaaggcagccaccacaaacccggccaaaaagaagtgtccgattatgtcctcctcgaatccgggaaaagtttctggctgactggtgacttcttcgatactgaccgtaaaaacgggaccggcgacagtttgtccgcatgtatcgctgccgaattagcccgtggtaacgacatcgaaaccgctgttcgcattgctaaaaagtttgttgacgtggcaattgaaaatgagatccaagttggccacaaatttgggccgattaaccactgggcaccgggatatcccgatcctgaacaatcaaacaattcctaatggccacctccatcatcggataggtcgcatcataaccaaatcggcagaaaggcctgggcaaaactaacgattttgctcagacctttttgctatcttagtattacctcgccgaatagtgggaaaacaagcagcttccggccgtctaaggaggattagccaaacatccacaaccaggatatttggctaatcccccttagactctggaagctaagtgcttgttttaccacactgttccgttacccaatatgtctttcaaactttttgaatccaaataacttgtcgattcggccaaagtattcttctgggatttccaaatcaacagccttcaaattattttcaagttggctgggcttgctggcaccagtaatcaagctgctgattcgtgggtcacgcattgtccaagctaaagcgaaggtcgccaaatcagtgtccaactcatttgccatcttaatcagttcttcaaccttatctaagttgtcgtccgttaacagcgcttggatttgatcttgataagttgctcgtgagccggctggaatcttgtgacccttacgatacttgccagtcagtaagccttgggaaagcggcgaaaatgggacgatccccaggccaagtttttcgcagacatccatcagttcatgctcaatgtagcgatcaaacatgttatattgcggctgaaccacagacatcgggtgtaagcccaacttttgaatcactaattgtgcttccaaaatttgcactgggcgccactcactgacaccgtaataaagaaccttgccttggtcgacgagatcactcaaagcagttaaagtttctgccaacggtgtgttgggatcaaatcggtgacaaaagtacagatccaggtaatcagtctggagattcgtcaatgactgatcaatcgattccataatatgtttgcgcgaaagcccacggtcgttgactccaggacctgtcggaaagtaaaccttacttgaaagaacgatttcttttcgtggaaattctttgagtgccttgcctaaaaaccgttcggctgccccaccactgtaagcgtcagcgcaatcaaagaagttgatgcctttgctataagccagtttcaaactctgatctgccaaatcctgcttggctgaatcactcacgtcggtcatccagctgcctaaagccaattcactgactttaaggccttgtttacctaaattacggtatttcattttgtttcctctcctcattttgatttgttagttgataacttgagtttagcgcttcgagtgtacttgaagtaaaggacatttagtaaaaattgtttgggcgctgttactttgctgagttgtgctacccaggcaggcctggtcctgtaacttcgggggttgtttgactgttatccttagggattttcactgttactttgttgaattgtgctacgcaggccagactcctccgcttagataaataggaccctttgatgcaagaccagcctaatcctgtaactctagaggttgtttgactgttatttcggggtatttttgctgctactttgctgaattgtgctacccaggccagactcctccgcttagataaataggaccctttgatgcaagaccagcatcaaagggtcctattcacctaatgctcggagtctaaccggcctggttcgcacactgttttttgcaccgcgatcaacccgagtcttgtcgcacactaatccctgaacaactccatattctgcaaataagtcatctcatcagtcgaaatccgcgtttgcagcttttctgccaaagcggcatcgatttttccggtcgtcaaagagttttgaatcagctcatactcgctatgaaacgcccgcatgaacatctggtagacaatgtccatatcaacatcctggccattaattcgccgatgcctggttcgatagaatcgcttgaccatgttggtctcgacaccattttcaccctgcttagtcttcaaaaagtccatgaccgcgttaaatccggcttcctcaattgggaggatgttttctccatgcttttcaaattgctcgcgccaatagacttcttccaaagccaccggggcggtcaaaaacgcctcttgagcgcggttcaaatccttatataatctaccaacatgcagactaaacctaattctcaataagacatttttccaaatcttttcatccgcggaaaaattattcaagttcaaaaattttgtatagtacgtcagctcatcctgagaaattttaccgtcatcaaacatcttctgaacggtcttcagctccacttggtggctctcactcatcagctgcctacgcaaatggaaattcggcgtgctgtccaaaaccaactgctgctgaagcgaatcaatgaccacctgggcctcggcttgatgctccttttctttcagcaggtcactaattgcggcttgaatcatccgtttaacccaacgataccgcggctgctgccgatcttgactcggtaaaatgattggaacaaaaatcgtcggcataatgagactggtcaagataaccaccgctgcgacaaaaatcatgatgcctcggaactcaaatggctggccattaaccgtgttaggcatcgagaaagccagtgagagggtaattgtcccgttcgctccgctaagtgccatgacgaggctatcacgccactcatggttcgatttaacacggcgcttgagcatatatctgctccaaaccagtctcaaggttccttttaccgcataaacgccaatcccaatcagaattaacttcaaaatattcagatcaggatttggagattggtgaagtgcctgaataacttccggcaacgacaggcccagcagcacgaacacaatcccggataatgctccggaaacgacttcccagacgttgctggtaaccagctgcatccgcgatgaagttaaccgtaatttgtcacgttcagatccctgaaccagcccggcggcgacaaccgccaagatgcctgacaatgctaatttttctgccagcaaatacactaaaaatggagacatcaattggatcaacaccatgataatcggcgtatcgtcgttataacgaatcaaaaacagccgggcactgacaatcgcaactccgatcaggctcccaaataacaagccgcctaaaaattcccagagaaacatcgcaacggccagttttaacgaaaaggtccccgagacaaaggcagtcagcgacaagtcaaacagcacaatgccggccgcatcgttaaacagcgactcgtgctgcaagatccctgcctgctcttcagcaatcggattggcctcaaaaatcgaattaaccgctgaagcatcagttggcgtgacaatcgccagcaatgcaaagcatagcgtcagcggcaggatggtcatgacggcgtgtaggcctgaaccaaccaccaaaacggtgaccagtaccagcccaactgccagcgacaaaatgttggtgatcgaccgaccaatccaaaaccgcgaactgttttgagcctcattaaacagcatcggcgcgataattgccaaggcaaacgtcgatgggtccaaatggaaattgcggtataccggtagaaccgccagtagaatccccagcaaaatcaggaaaaatggcagcggaataaacgagacgtgtcgcgcgagaatattcgcaaatacgaccgcagccaaaatgatggtcagtagtagtaccatgtccattacattcacccctccgcttcaatatcgattctagtttatcactgattggacaaaaaaagccgtgtcgacacttggacacggcttacagatgaaaggcagatatatttctatttaacctaccacttatccgggctccaaatccgcccgtccaactcatcttgggattgctgcgctcgcttttcctgctccttagccaacgcaatagctgcttgataaatcgatttattaacaaatgattggtcagcttcctttagttgggtcagctgttgaaccaaccaatccgttgtatcactcatccctattcctcctgatcgcgaatcattttcacgtcttgttttaaactttcaacattattctgttgatcttcaatggagttgatcaccaaatcaatggcctgttgaaggtccgctgacttatctgctttggtatcctgcagccgagcaaccagccattgctcgcggttggccaaactcaagggcatctcggcactcaagtattccagatagtcgaccagtaacttctctttttgggccggatccaaataaccaaattgattaacaacaaatggcttcagataagtcatacctgctttattagcgaatgcctgaaacggacgcagcaactcggaaatggtaaactgctccgggccgccggcttggaagtcggcctcagcgtcccccaaagacacgacaatacccaattccttggtttttaaggatcgtttggcaacgatatagtttctggtgaaaacatcgtccatgaatcgttttaagctcgccggcgatgagtaccagtacattggaaattgaaaaacaatccggtcaaaatcccgcagtgcattttgttccttctcgatgtcgattgtcccggttgctgtatataattcatcaattacctggtatttcacatcatccagggaataaaagctggttttaagaaattgttgcgttcccgaatcctcaaattgaggatgggaaattaagatcaatgttttcattgttatcctacgcctttcataagcctttttcatttcgtttccacttaaaatcatctatattaagattgtaaaccaaatcataatcaaaggagagttaaactatggcaatttataacgttcatactaccttaagagacattggcgctcaaacaattaacactgcgggggtccatcagtttgtggctgacgaacccacgagatttcgcggcaccgatgccggccccaacccggttcaatacttgctgggcgcagtcggtgcctgtctgggtgccagcgccgcatcattggttcaccgccccggttccaatattaaagtggaagaatttgaagtcgaagttaccggcgaaacagaacgttttgccgacaagtcttcacgggtcaaaagtattcatgtgaaattgacctgccacaccaacttggataaggaaggcaacgatcgattcatcgaggataccattcatctgtgcaccgtccacaatactttgaaagattctgtggaatttacctttgagattacggattaatttcgatttaatcgaagaataacattactggtaccgttagcacttcatattatggagtgctaattttattttctacaatttagcaaattgtcttgcgaacgttggtgtacaagcgtttatggcaattaaatctttgtgttaattgtttgacctcattaccaatatatgatactatatagttgttcgaaaggggaatggatgttcgccctcgaacattttcaacaaatataggaaatcatttagaatatgggggtattgcctatgaataacgatatttttggaactaacggttttgacgatattttcaacgacccgttctttaggaatgcaatgtcagattccaacggccgtcaacagtcacgtcaacaacccattcaagttcaagaacgcagacctcaacagaagaaaactttgttagatgaatatggaacagatttaaccaaaatggccaaagatggcaagttggatccagtcatcggccgtgataaagaaattgaacaaatggaagaagttctcagccgtcgtaccaagaacaatccagttctgatcggagatgccggggttggtaagacagccgttgtcgaaggtttggcacaaaagattgtcgctggcgatgtgtctgagaagctcctcaacaagaagatcatctcgattgatgttgtctcacttgttcaaggaactggaatccgtggccaatttgaggaacggatgaagaagttaatcgatgacgtttcaaaggataagaatgtaattctgtttatcgatgaaatccatcaaattattggagccggctcaactggtgaaggtgacaagatggatgccggaaacattttgaagccgaagttggcacgtggcgacttccagttaattggtgccacaaccagtaatgagtaccgggacattgaaaaagaccaggcccttgctcgtcgattccagccaatcatggtgaacgaaccaagtgaacaagatacgttaaccattatcaaaggcttggcaccgaaatatgagaagttccaccacgttcaatacactgctgatgctttgaaggccgctgtcagcttgagtaaccgctacattcaagaccgaatgaatcctgacaaggccatcgacttaattgaccaagccggagccaaagttgccatgggctcatcactcacgaaagacaagtccactctgcagcaagaagcagaacagcttgaaaaggataaaaacgcagcttccaagaaagaagatttcgagcaggctgccaagttgcgtgacaagctggacaaggttcaagatcaaatcaagaacatcgacagcggtaccaaagtcacgacaccaaaggtcacccctgaagtgattcaatcagttgttgaacggatcactggagtcccggtaaccgacgtcaacaagaatgaagtcaaccagttgaacaatttggataaagacctgaagaaagaagtcatcggccaagataaagccctagatgcaatttccgctgccattcgtcgtagccgggttggctttactgaaggtaaccgaccaattggcagtttcttgtttgtcggccctaccggagttggtaagactcaaaccgctaaggctctggccaaagaattgtttggcacgacaaaagccatgttcagatatgatatgtcagaatacatggacaaaatcagtgccagcaagttaatcggttcagcacctggttatgttggctatgaagaaggcggccgtctgaccgagcaagttcgtcgtcatccatacagcctgattttgatggatgaaatcgaaaaggcacacccagacgtcttgaatctattgttgcaaattttggacgatggtcgtttgtcggatgctcaaggtcgaacagttgacttcagcaacaccgtgattatcatgaccagtaatgccggtcaaggtgaagccgataacaaacaaaatgtcatcgaccgattgaagccatacttcaagcttgagttcttgaaccgaattgatgatattattcaattcaactcattaaccaagcctgatctgttgaagattctcgatttgatgctcaacgatttgaaccaattagtcgacaagtcacgtgggatccacttcagcgtcactgccgacgccaagaacaagttggtcgacatgggttacagtaaagaacttggtgctcgtccaatgcacagagtgattaccaaagaaattacagataaattaaccaatagttatctgcagaatccagatgtcaaagacttcaaagtcgttgttgacaaggatgccatcaaggttgaaccagttgctgccaagcaagcaattgcttcataatcccgaaatgatcgtaaactaatttgacattgacctggtatgttggtatattatagtcaatgtgtttaagggttcgattttcaaaggtatttgttttatagtattatgaaataactccttggaatcactgcaacttgatacattaaaatataattatgcgctaaaagcgcaaggaggtttcatatattatgaaacaaggtactgttaaatggttcaacgctgataaaggttatggcttcattactactgacgatggtgacgtatttgttcacttctcagctatcaacaaagacggcttcaagtcattagacgaaggccaaaaagttacccttgacgttgaagacagcgaccgtggaccacaagctgctaacgttacaccaattgaagactaattcattagtttaaaatttgaaagaaccagcgatttcgatcgctggttctttttttatgctcaacttcatccaactgcctatatacatataaggtgctgaattatataatagaatggttctgaaaatattaagaaaggagaattcacacatgaacatttcaaagcatttcaatcactcgatgaagttaacggcttgcttgggtgtttgtttgggagttttgctgcttgccaaccctacatatgcggatacatcgcaagctcaaaccagcagtgagccaactgcgacagcaaccgctagttcatcaacgatagattcacctgtgccatcaagtgatagtgactcacaaacgactacggttgatcaaccaaatgaaaatgccaagtcgcaaactgttgaatcaagtaatgaacaaccgaccgccccagagactgatgacagttctagcgagcaacccgttcctgcagatcattcaaccgccgagacgacaaccaccagttcatcaactgacaatcgatcagatgcagatactgccaccagcaccactgacagcccagctgatagttcaggtgatacgccagatgtccagccgaatgacagtcaagccacgccagctgacggtgctcagaccacaactgatcagtcatcaactactggtccatctgacaaggatcaaatcaccattgacggcattaatcagtcaactgatcccgccatcaagcaatccagcaacaatccattgatcaatttcttgaccagcatcaccagtggcattgccgcctcggtgatttatccattagtagctagtcgtcaaggggcacaattcatttcgcattttcgaacattgttgtccccaaaccgctgggatgtcagtcaaaattgggcggatttggatcagaaatataatccggattacgtcaaaacatactataccgacgctcaggactggtacgacaaccgtgtccaaaagcaaacttgggaggttccttttgcggacgggactggtactgccagggcaacttaccttaaaaatggtgactcgaagaagaccatcatttacggtcaaggctggacaaccgagccggagggcatggggcgaatttccaagatgttttatgacatgggctacaacgttttgatgccctacactcgcggccaaaactccagtgacggtgaatggttaaccttcggggataaagacaaacaggattgggtcaattgggttaacaagattgaccaaaccaatggccaagacagccagattgttctctacggtcaatcacttggcgccgacactgcactacaatatgccggccaaggcaatttgccttcttccgtcaaagcaaccattgcggattgtggtttttcgaccatcccatctttgatctaccatttgtacactggtgcagctaacagtctcaatagcatcacttctaaaattggctggaacctcaacggctcaattccactggttccatttgatcagctcttaacggcgatgaacgggattaacaagcttgttcaaggctttagcctggatgacgtctccggcatcacagcagttaagaattcgaaattgccaactttattcatttcaactgaagatgacactttcatccctgatactgaaactgaaaccatgtacaacctgagtgcctcaactgataaaaaactgtgggtgcttgacggccacgttggcggtcatgcttcagcaagcaacgccgttcaggattacatgaagaacattgaagattttctggcttccgcaatgaatcaaagcagttcgtcttctgatgatcaactgaatgttccggcaaccaacaaagttgctgcatagcacttcaatatcaaccttggaaaaggctcagcgataactagtcgctgggcttttcttgatcaacaatcaagtttggggcagcttggctaacaaaggatttattaaaattgacccagatcaattttttaccatccaaaacgtgctaaagttaaaatgtaaaatgtttcgatgatatgtattgacatcagttttgccaatctgtattatgttaattattaactaataaaaagtaagtacactactggaggaattttaacccatgaaagaacaattattagatcttgccaagaagcgccgctctatttacgcattaggccgtaacatcaaccagagcgaagacgagattgctgacttaatcaagaagaatatcaagtgggccccaaccccatttaacaaccaaaccactcgcgctgtgatcttgtttggtgccaaccacgagaagctgtgggacatcgttggcaaacgcctgaagtcagaagttcctactgaagaagcttaccaaaagactttggaaaagatcaacgccttcaagtcagcatttggtactgtcatgtactacactgacatggacgttgttcaccgctttgagaacgactttgcactgtacgccgacaactttgccgactgggcagaacaagctcagggtaacgctcaatttgccgtttggacatcccttgccgaaaacggcatcggtgccaacctgcaacattacaacccactgatcgatgaccaagttaaaaaagcatttggcatccctgacagctggaaattacgtgctcaaatggactttggttcaattgaagccccagctggcgaaaaagaattcatgaatgacgaagaccgcttcaaggttttgaagtaatttaattgcatgccaaaatggttcccaaccagatcacatctgattgagaaccatttttttgatacgcttacttcttcaattgaaccttcacaagttcatcgccatgactgacgacatcttcttgcgtgtaatcactttgagtaaccttgtcaccctgcgtcaacaagaccagcacggtatctttataaccggcctgttgaatcttgtctcggttaaattccagcagcaagtcacccttcttgaatgactggccggaatcaacgtggttaatgaagccttcaccgcgcatattcacggtgccaaggccgacatgaatcaggatttccaacccgtcgtcggaacgtaagccaatgacatgcttcgtggtaaacaacagaaccacttggccatcaaacggcgcataaatctttccttcggtcggttgaatcccaataccgtttccgggcaatcctttatggtcatgctcgtcaaccacatctgccaagttgactctcacaccactaactggggccgcaacttcaacgtttgcttcttcagagttggtggcagctttttcagaggtggtagtttccgtatccgagttatcactaatcccttcaacagctaacttgtgctggagttcatcgacgatctcagcatgtttcttttcagaaatcttaaccttgaagacatagatgaataatgccaaaacatgcaagataagtgcggcccagaatgcgaccagtttgaataatgaaatgccgcctggagtcattgaagccgcggtggcggttccagtcatcccagctgcaacggcaacccagccaacaatcgcatttgaaatggcaccggacatcttatccaacatcggccgaattgccaaggtaacggcttcattccgcgtgccatttttcaactgaccatattcaatcgtatcggttaaggtcaaaataaccgccataaaaatgaatccttgtggcacataatacagaatcatcgctgtgacaaccatcactaaattatccgtggaaacaatcagtaggatgtatgccaagatcatgctgcacatgctgacggcataaatcgtcttccgggtcacccacttattaataattggataaagcggcgaggtaaagaacccggcaatcgttggaatcagtccggtaatccagaataatcccggcttatccatgacatacttgaataaatagaacatcaaaccggcagtagccgcattcccaaaaccataaatcaggtatggaaaggcagtccacaacatctggtcattatgtgccaaagcccagaacatttctttcaaactggtctttttcttagtaactgcccgcaaagcattttgcttctcgtgggttccaagagcaaccaccaaggagcaaataatgcccacaacggcaatcaaaattccaaaggcagtccagcctggttggccttcattgtgtttgccggtaaagaagaaggtcacgtaagtaaccaccggcacgataatgatcgtgacaatattttgaccaaagccggcaaagttggcagccgcagtgaacagtgaccgctcgtgactatcttcagtcagtgcaggcaccatgccccaataggacacatctctgaatgagtagaaaatatcaaaggtgatgaagatcgggataaagagaatggtgaaccaggttgcactcacccgagacaagccgaagattccggaaaacagcagtgccagcagcaaactcgaaatcgttccggcaccgattaaccacggcttaaatttaccccagcgtgtattggtgttatcaacaatgttcccaataatcggatcaataaagatttcgaccaaccgaataatgaaaattaacccggtaatcatggcaattaacttgttggcctgagccttgggaactcctgtgaacattgcggaagtgacatagaccatgaagtaagttccaaaggtcatgtagaccgcagatccacctatgttagcaaacgcaaagttgaaaatcgaccagaaatttttccgccgatctttcttttgtacagcatccaatttataaaacgcctcccagcgtgccgattcgccattacaaatgggcggttcggtatgaaaatttcgtagaaaatatttccttacgaatcgagtatataatgtaagggttttcatcaatgctatatttttaccgtaaaatacccaaatttaacccaattatagtaaaatatactaaaagggagtgcgaagatgcgaattgcgtttaataaacctgcagaaacaatgccgctgtattgtgacagtgtcggctatgattggaatcagccgccaattcaccgactaaacggctattacgcctaccattggctgcagaccgaaagtggcgccggtgtgattaacattgaccaccagtcgatttccctgcaggccaaccagggaattctcctccgtcccagagtcgcccatgaatatcatccaaccggaaaagaaccttggaaagtatcgtttttaaccttcaatgggacactctgcgattcgctgtctgattttctgaaactggctgatttcctggtgatcgacacggtttcaccagaactaacatcgtttattcccgaagtcttgaatgaatttaacaacaatcatccaatcgcactgcttgatcaatccgttcaaatctataaatttatcatgctgctgaagcaaaatcatttactgaacaatcaccgttatcaagatgccacaattaccacgccaattcttcaatacattgcggcccactatgccgaaccgattacgaatgacaaattgtcgaaagccaccagttattcagttacctaccaaaaccgggtttttaagcggctatatgatatgaccccgctggaatacctgaccgattatcggatgcgaaaggcgaaggaattgttgttaaccaacccaactctggaaattggcgagatcgcaccaaaagtcggctttcataatccgtcgcatttcattgaccagttcaagaaatactacaaagcaacgccgtctcatttccggaaattcatttagaaaatcttacagattcaaaacggtaccatttgtgaaatcagctttaattagtggtaaactttgcctacaacaataattgaggagtgatcttatcgaatcaactgttaagcgtggttggggcatcaccaacttcgacatcaaagtacttggaattattctgatgttcatcgaccacgtgcatgaaatgtttaacggtatcggtgtgcccaactgggtggactggtttggccggccggtagcaacgatctttttcttcctgagcgttgaaggcttcattcatacccataatcaaaaacgctacttgtccaggctgctggttggcttttgggtcatgcagattgggaacctgattatccaacatttcttcaaactcggcagtttcggcttgattaacaacatcttcggcgacttgttcattggggttttgacaatgtatggcctgcagaccatttctcaggggcatcagaatcatcaggcagccaaaatctgggaaggtattctcattattgccctaccattgatctttgccggcctgaccttgctgacaatgggccaaggcggcaacagcattgcctttcgaattgtgaccctactgccaagtccactgattgctgaaaacggctttatcctttacctgggaccgttgatgtatctgctaaggaagaaccgcaactggcagatgctggccgtcgtggcagtagccattttgtccaccggctttaatttcagcagtatgttcacgactaacttccagtggttgatgtttcttgccattatcccaatgtacctttacaacggtcagcttggccgcagcatgaaaggcttcttctacgccttttacccactgcacatttggctgctgtacattctggcttggttcatgggcgtgcgctattaatttagacaaacaaaaaatgagatgctggtttccattgagttggaaatcacatctcattttttaatttaagcattattttgtgataaatacatacaaggtactggttgagtaccccaagctaaacaatagcccattggaatggaacttcggtgccgttgtcgagctggacttcttggccttggccgccttctggaatttgttcaaaacgtgcttggcgttagcgccgacactgtttgtcaaaatcgagaacgacatgatgaacggcttgaggtcctttttgtgcttcaagttgttaaccggcaccatcattgcgatgcctaagactttatccccggacttattgacccgcaatgtcatcttgttggtatcaatcaaattgtggatgccatctttggggttggctggcagaagctgatctttgacactagccttggctttcttcattgccggggccagtttagcttgcgtttgcttcaattcagctgcctgcttttgcagagctgtcgccttttgcgccttggcctgcatggctgccatactggtagccttgccggctttcaactcggcagcttccttcttcagttgggcaccctgcttagccattgattgggccagctgttggtccttctttggcaatgcggcgccggttaagccttggttataagtcgtccgcatcttctggtagctgccaatcacgttggctttggcgaccgtgacggtttggtgcttgccatccgtgcttaatttgacagtttgttgataattcttggttggcacactaattacaaatgcaccgctgtttgttttaactgtttgcttcgtaccgccattcacggtgtaatcgacctgcttttgattactcttgcctttcagcgtcactgccaaagcattcgcgctcaaatggtgattagagaccgtcaacgttggtttgccacaaccgctcagaatgaccatcagagaagcggcagcgattactaaactcattaattttttcatcgtaagctcctccttaatcaaatgaaacgtcgtctgagaattgactgttgtaaagatcggcatagaagccgtttttagccagcaactcattatgggttccggtttcaaccacggcaccatggttcatcacaataatgttgtcggcgttttgaatcgtggacagtctgtgggcaaccacaaagctggtccggttttccaacaactgactcatcgcgtgctgaatctgaacttcggtccgggtatcgactgaactggtagcttcatccaaaatcagaatttccggatccgccacaaaggctcgggcaatcgtaattaattgacgctgaccttgagaaatattggaagccgattcattcaagacagtatcgtaaccctttggcagtttgcggacaaattcgtccacatgggcagccttggcagcctcgataatgtcatccttgctggcatcttctcggccatacttgatattgtcatagatcgaaccggtgaacagccaagtatcctggagaaccattgcaaagtgtgaacgcagatcttcacggtccagatcacgggtgtcgacccccttgaggcgaatgctgccgcccttaacgtcgtagaagcgctccaacaagttgatgatggtggttttaccagcaccggttggcccgacgatagcgacctgctgaccgcgtttaacggccaggttgtaatccttcatcaacaattcgtcatcggtgtagccaaattgaacgtgttccaattcaaccaggttatccgtgtcggtttccactggtcggttggctttggtattcttcatttcttcttcgtcaatcacttcaaacacccgctcagctgacgcaatcgtcgactggatggtgttcatcaagttggcaagttgagaaatcggctgcgagaattggttggtatattgcaggaaggcctgaacgtttcccaaagttaccgttccgttggcaacctgaatcccaccaacaaccgccacgaaaacatagccgatattgttcaggaaaatcatcaatggcatgataatcccggaaataaactgcgctttccaagcagcttggtagtatttcttattttgaacttcgaactggtcgatcgtatcttgttccttgttaaaactcttcagaacaatttgaccggcatagttttcttcaacctggttgtttaacaaccccaggctcttctgttgagccgcaaaatatttctgcgatcgaggagcaacgatgccaacgattaccaaactcaatggaatggttaccagagcaatcaaagtcaacttccagctaatcgtaaacatcatccagagagttccgacaaaggtcacgaaactggttacggcctgggtcaaactttgctgaagggtgctggcgatgttatccatatcgttcacggctcggctcatgatatccccattactatgagaatcataatacttaatcggaaccagccgcatcttgcccttcatctgccgccgtaatttgtagacggtgttttgagaaatccgggtcatgatgtactgctggaagaaactgaaaacagccgatgccaggtacatcacgataacgataagaatgatttgaacgattttttcataattgattggcagcgaagccacgctaaaaccggctttctgctgggcatttcccttcatcaatcctttaaaaatttcagtggttgcttcacccaaaatcttgggtgtccggatttggaagataacactgatgatcgcaaaggcgaacaccaaaatcaggccaatcagtcgatcctgcatgtaattcagcagccgcctggtggtgccccaaaagttatggggcttttcaacgacaccttggaagccgccacggccaccatggccacgattggaggtaggttgtggtgccttatctttatcagccattatttgtcatcctcctctcgtaattgtgagtgaataatttcttggtaaaccttgttgttagcccgcaactcgtcatgagtgcctttgccaaccagtttgccgttatcaaggaccaggatcagatcagcatcagcaactgtcgcaattcgttgggccacaatcacagtaatactctgctggatgtgttgatcggcccgcaaagcagctcgtaaatcggcatcggtcttgaaatccagtgctgagaatgaatcatcaaagacgtaaacggcggcttgcttgactaatgatcgcgcaattgccaatcgttgcttttgaccaccggagaagttgtccccaccttgttcaacttggagatcaagtccggcgggatcttcttcgacgaagtccttggcccgggcgatttccagggcgtgccaaatctgatcatcagtcgcatctgggttcccgtatttcatattgtcacggatagttccggtgaacagagtggccttttgtgggacaaacgaaacttggtctctgaggtctttcatcgagaaatcattaatgttatgcccatccagctcaatctcacccttatcaacatcatagaatcgagggatcaaggaaaccaaagtcgtctttcctgaaccggtcccaccaataatggcaaccgtttggccactatgggcctcgaagtcaatatcacttaacgccggcaattcagcttggcgataacggtattcaacatgatcgaatttcaagtcgtgctgggtagctttaggatcaaggaccaccggatgctccggctgtttcatggttgatttcaaagccaacacagtctgaattcgcttggctgaggcctgtgcacgaggaatgaacacgaacaccattgagagcatcataaagctcatcagaatctgcatggcgtaactcatgaacgcaatcagattaccaacctgcattgactgggcaccaattagcttggcaccaaaccaaacaatcgccacgttagttccactcatgatcaaggtcatgactgggaaggccaaagcgacaatcgtgttgaccttgatggcattatcggtataatcccggttggcatcttcaaagcggtcttgttcaaattggtcctgccgaaatgcccggataacccggacacctgtcaggccttcacggaaaattcggttaattttatccgtcttagtctgcattgctctaaacaatgggactgagaaatagagtaggaggccaacaaagataatcatgatcggcaataccaccaagaagatggtggttaactgatggtccttggtgtaggccaaaaaactggcaccaatcagcataatcggcgccatcagcatcatccgcagcatgataattgctacgttttgaatttgaaccacatcgttagtggtccgcgtgatcagtgatgacgtctcgatttgatcatattcatctttggagaagttgatgactttacggtaaacgtcactccgcaaattttgccccaacttttgtgaggtccgggcagccagaaagacgttgcagaccgccgccagaatactaatgagtgaaaagccggccatttccagacccactttccaaatatagccaatgtctcctttggcaaccccgttattaacaatgtccgaggtcaggctggggaggttcaaggtcgcaatcacttgaatcgtcatgaacagcactgccccgagaactgccacgtacgagatccggtttttggcaattttcagcattttcctactccttccaggttcgttttaagattgttgtgcgcttaattaggtaccgaactatattactgctagtacatttaaaatacaagtataagttggtaaataactaggtaaacagatacatcatattatgaacttttctgcggtgagtttcattaatgttaactaaaattttgctttcgatgttgcacgggttagataaccgcaaaaaatgacaccgggaccatcttgtctgatgatttcggtgtcattctttctatattattatcgtgtgaaaatgagtggacttgaatttttaacaggcaatccaaattttctcacaccacttcgctcaatccatccaaagtgaatttaagcttgcgcaacatgttcttcaggcgtcttaaccgcattctgcttatctcgttcaaggactgacttcatgtagctgtcaacgtcaaaggtcccggcaaattcggccaagtgaaccaggtttctcaagaagtcgtgggtcttggcttcgtaatgatactttaagccaaggtcgtagatgtagccgttgatgtagtccacttcggtttggcgattcttggagatatcttgatacattgacgggaagtgaagtgggttggaaacggtgctgacgtacttaacggtttcccactcttcctgacgggtattcaataacgtgatcccggcgcgttcgcaaacatcgaaggcttcatcgattaattgaacgcccaacttctcggcaactggtgattggatatactcacccatccggatcttaaacatcgtgcacaaggtgttgataacggagttaaagacgactttggccatcaaagtaccaaggaagttcgtggtcaaattaggattgagccccgctttttggaattcagcgacaatcttgtgagtcatctcatcaggtttctcggtttcattcgcaatgttcattgaaccggcacccttgggaccgatgaagtcgacgtcgccggctttgttcaacacagttccgatcagagcggttccgccgagtaaacgttcctttgggaagtactggttaagtttttcaacgtgacccatcccattcatgcaagtgacaacgtattgtttgtcgttgaagaatcgtgaacagcgttttaagaaatcagcgagttgatattgcttggtaaagacaatcaaaacatccggatcacccttatattcttctggatagtacacgttgaccggcaccagatgtttattttgaccgtcacgggaaacgtaaacgccaccctgttgacggaccgtttcaacttgtggttcccacgtatcgacaaagtcgacatcgaacccggcctcctgcaaaagaaccccatatctcaaacccattgcgcctgcacctaatactgtatatttcataaatataacttcctctccactataaagtatgtaatcaacaatctttatcaatcccactaaagcaacccgcgatacaaaaaaatcgtccttctgtcactaagacaaaaggacgacaattggccgcggtaccaccttcatagacacttttcgtatccactcgttgcttgctttaacggacaagtccgaaaccggctaacttacgctcaccgatttatgggtaaagcatgaaagtcacagtctacaatttcactaccatctctcagccgccgaatggattttctgttagcgaagcttgtagaaaacttctttcaaattgatagttcgtattatgatagttagattagaatatgtcaacactttttgagaaaataatgtgagcagctaacatcctaacatcacaaaaaggcgactagagcaatgtctagccaccttttaattgattatttaattatggttattttttgattgattcctcatttctcttgtttgcgtttggtgtagtaaatcgttgctgttcccagtaagccaaccagcatgaacattccaatcaccatgagcagtgtgttgttgtcttcgccggtttgcggtaaggcggacttgccggtatagccggatgacgggattcccattgggctgtcgagggtgcctgacttgccggaggttccggtggtgtcattgccatcgagcgtacctgaggatgcatcgtcgccgtcttcttcgcctggcaatggtaactccccttcatcgtcttccaaatcgttgtggtaaacgatgctgtcatcttctttagtcgccgttccggtaaccgttggactgttcacaaccgctgttcgcttggtaacagttgttacatagccatcagctgagtagtccttttcagagacttcatattttgcaccaagtggtatgaagaacttgatggactggccatgagttaatgtgaagctgccgttaccaccattgaactgaatggaaccttcaacaacttggccattggttgtgacctgggtcttaaacgtcccgtttagtgggttattagctccatcggttgcttcaatgtggaattcaaacttgcgagctctgtcgcccagttcgttcacaaatttgcttacagagaggattcccagttccatttccccattcttggtgttggtaaattcgaccgtccctttttgatcttcaactaacttgaaggtttgagtggtcatcccctcttgaaccttggcgccgttgacctgataggttggtgcaaagccatcaacatattcttcgcccaccgcataagtgtaatcaatcggcaagccggtaactgtcaatgattcgctgtccttcaaggtaagcacgtcggattgaccgtcggcgaatttcacagtgatttcgtgtgagtctccgtgctggtcaaccttggtggccttgaattcgccagttacaccagagtagatgcggaagttgaagtcacggtcatggtcgctagttgtcaaaccatcgccggcaatttccttgttaatctttaagctggcaactttctcggtgtccttgctgttggtgaagtccacgttgacgcgatccttatcaaccagcttaaattctttggttttaacgccgtcttccatccgggttccgttgagttggtactgcgtgtggaaaccggaaccatttgtttcagtaaccgtgtaagtgttgtgttcacttggcaagccataaatcagaatattttcgtcagccttcaagttgacagtggctttgccgtcggtgaatatcactttcactttgtcatgaccgtttacgagtgcgtcgtattcgccgtcaacacttgcgttagcttcaatcacgaactggaaggtcttgttcttgtcagcgtcgatgatgccgccgccagctaggtgcttgctgatcttcagctcggccgtttcggcttcaaatttggtgttggtgaaaatcacggtccccaatttaccttcctcagtcacaaattctgaggcgacattgcctgatttctcggtgttttcgttgaccttgtaacttggatcgtagccttcactactttccttggtttcagttacttggatgttggcaccaattggtaggccaaggagttgagctttttggtcgtgcttgaggttgaaggcaatgatgttgttagcattaaacgaaacgggggtgtcggtgtacttcccacttacttcgtatttacgcagggtgaattccccgtctaatttgccgccgttttcattggttccttcaactctaaatctaaactgcttgttgaagtcttcatccccagcagtttcgcccttgactgtctttttgacttcaatgccagtcttctgagaatcgttgttgaagacaagttgtggcatatccttttcagttgtcacatcatgagtatcgccatcttcttggtgtttaccaaattcgtgactaactttgtaatcatgggctttggtttccgttacttgaatcttcaacccttttggaataaacattctaattgactgtcctgccttaagagttaattcataattaaattctcccgttttaggatccttgacaaatttcaaagactcttcgtcattggagtcactcttgatataagcaaacgggtcagattcttcaccccacgatgtaggtggattcttaactgtcaacttaaattcaaaattcaagtcttcatccacaggtggaatcagtccgctcacagtcttcttgatcccaaattcaaccaagtcaggcgcaatattttcaaaggtgattgaatttgccccatcaggtcgattcaaagtaatttctgcactgttgccttcgttcttactttccccatctacccgagtgtaagttgtaaactcaccagtagtagtttcggtgactttaaacttagtcgccttattcggcaggccaagaatcaccaatttttcattatcttgcaacgtgatctcttcaggtggtaacgtaccatacttaatcttggttacctgaccattttcgtcaaaggtcactttaccagtattcttagtcttgccggttgttgcgtttctaatgtcggcagtataattttccttcttaacagcatttcgagttgcgtcatcgttggctgcgacttcgaaattaaaactatcgattccgccaggcatgtcacctgcaacaaacttttcaaattccaactggttcacaacttggctgttaatgaacttcagcatcgtattcgtagcattaatggaaccagttgctttccagccgtcttcatccgaatcgccggcttcattttcatccccatcgccaactttgtaatgaacttcggtatactgagtatcttgtttttcatataccctcacttttacattggctggcaattgaatgttccgataactttcgccagttttcagcttaatcggtaccgtgctaccatctgtgtagatgatttctttggcaacaccaccgacaaatttaaacttgactggaatgtctccacctgagtgtttaattccttcaatcgtgccgttaaagctcttatccggctgattgtcggcatccaataccttcagcatgaaatcaaattccttgtctttgtcagcattcgcatttggaccttgaattgttttggagaatccaaaatgcgtcgtctgaacatcattggtaaactgcacgattccggctggagcattcttaccgatcatcatttggaaagtatttgtttcattaccgccattgccatcaggttcaaccgtcgttaagttgtcaagtgagtgggttgtgcggtatgaaccattggctgattcgatcacccggtacgttttgtcctgtggtaatccgtgaatggtgatcacctgaccgtctttgatctcttgaagattagttgaaaccccttctttgaagttcacaacactttcgtcaccatcaatatcgtaggtgaaatcgtcattgaagtcggtatcgacgtcaccctcgtcgttgatcacatataccttaaattcaaatttgtcgtctttattggtattcagtgaattggtaaccgtctttttaatcttcaaagcattagttcggtggttcttagcagtgacgcaataagtgttttcattgccatcttcagtctcttcttgggcatctttaatggtaaattctttcgagacccatctgtcatcataattctccagcccctgagtttcgataatccggtatgtcggtttatcgtacagaccgtcgaatgatgcgaaaccgtctttgtcggttgctttaggttcaccaacatttttccaaatactatccagatctttcatttgaagttggaatttgacgccttcaagtggagcaccagtcgtggcatcaactttcttaacgttggcagcgaaagttgtgtactgcccggcaacttctgcacttgattggatttcttctttgtcttcaaaatctttagaagcaattgtcaacttgatctcattactataggttgtcccaaccgtcttggaagtaacggtatgatactcaaccaatagcggtgttttaaccttgtatgagttgttcacattaatcgtcatcgtattcaaagtatcagagtaaaccacatcgtaatcgtggccttcaattaaggctttatcagatatcttagtgtaatgaacttccttattgaccaaggatcgttttgcttcatagattttcagcttgtagcgatcatcgttggtcttcaagtggtagtgcccaccactaagcgtatcggttagtttaactggcgatctaagctcgtagccattcccgttaattgccaaattccatttaacggctccaacggaccgggtctgcccgtcaccctcgtctaattcaaggttgtgttcaagcaacttccctgacttgtcgagtaaatgaccgccgtctgcgtaagatacactcgcctttgcttcaagggtatgacgagtctcatcgtcagcattcagtttccatccggcagtgactttgttattaaatgtccaagctttgagatgttcataggtcgcttcttcatcggccttaaagttcaagacttttgattgatatttcaactcgaacacttttttaccgagtaccctttcgccatcgccattctcatggtccagatagatattgttgtaagcatcttcggataactttaagttaaaagttactttatgattttcatcaacatcaacccgaacttcatattgatcatcaactaacctttgactgtcagatacgccgcgaccatcagagttaatcctagccagggagatctgtagggtatcttgtaaacgttgctgaatatcttgaagattacgtttagtaagctttccagtagcgtctttgatcacatccggtccaacttcatcagtgatatcaatcccatcagtgaccaaggcggcgtgctcatttgaacccaggtattgccggtagttgaaacgcgtcgtccaattaatgaggccattgttcaggaaatccttatccaattgcccatcctttgaaatgttgtttcggatgaggcctccctgattgacgcaagtctttacacttgcgtcatcagaacctgagtattctaacccagcatagttacaaattttttcaagttcggcataattggcatttaagattttttctttgtccaatggaacatcctttagataaagattaaatgatttttcaccagccggtaaattctcaacggtgatgataatctggttgccggaaagtttgacactgaatgctttgttgtccttgttcttgccccagtatgcttctccatcgatgatcgtgtaatcccatgtttgatcattttcatgcttggaaaatgaaattcgtttcttaacttcttcagtcaaaccacctgtatctgtaaaactgttataaaacttcttataatccaagaagttgagcgtctccccttcgattggttccgtgatcttgaatgaaccatcaatttgtcgattgatttggttgacgtggatgctccatgagctcatcatcttttgccaatccaagctcacgttgttcttactgttgatttgggggccaaagtgattacccttcttttggccgttcacctcaaccgtattgctgatactctggtaatctttgtcagtcacgtctgctgttggcttaatgatgtaactaaacttatatacctttgacccttcgttttcgctgggaacaattacatcagcaaactcaaccgtcaacgtctgaccgtcaattttgggatcacctttcatccaaccggtaacggatggtattaatgtgtaatcatcaatattctcactaaacgtaaatctcttggaattcaaagtatccttcaacacaatatttgtttgaccaggatcgacggtgaattcaacggtatatttgatgctgccgtctttatccatctttgcagtcttcttcacctgaccattttcacgggtgatcgtcgctgtgacatccagcgttttggcagggtccttcacaccaacaatttcgacatccgtcgcacgaattgtatttttgaaatctcgattgttgaaattagttacgggggttatcattttcactttaatttcaattattccccgttcaagcccaagtcctttagcgttaaattggaaatttggaccggtggctaccaatttatcataatcgtcatgatccttagtgatggacactgtctgcccgtcagcacctttcacttcaaactcatagctgactttatcattggcggttgcatagccgccaccgaacttatctcgaagggtaaccttatttgcttctttaccgtcctgcaccttaaaggtagatgtccattcaagcatgtcaagatcggttaccccattagatgtgtgtaacacaccatctttttgaatagataccagatcttcttcgactttaattggatattcacctttagtactttcaccaaaactaatttcctcggcgttcgcattgatttccgtcttgatttttgctttgtaatcaatatttgtcacaccttccaagtctccaggaaggaaaataatcttagcatgttgcgtgtcacggtcctctgcatcacgggtcatgataaaccgaccaattgtccggcccccataggtgatgtattcgtcaaaggaacctgatggaccgtattcatacttcaatcccttaagatcaaattggtagtagtcgccatctttaatgtcaatcccggtattttctttgatgctatcaatatcccaaagataagtaatctcaatatttttatgctctcgaagaatagccggtagttgaagctcttgttcaagtacagatggtactttctgattttgagagttaccatccttatcaatatagctaaaattgattgaggtgaagaattgagggtttgaggcagcgtggatagcatcggtaatatcagtctttccttcatcaccgaacacaccattgcccggtaattgccgagttaattcgttactcgtcggctcctcaccatctgaggcatcgctcgcaactgcttcttttgcgcccttcagatcagaaacatctggtgtttgtggtgtctgagattccttgctctcaccattatctttgactgctctcggatcattttgtgtcccaacagctgcttgttcttctgctttacgattctcttcaatcgcctgacggctcttttcctcagccttcttctgatcagcttcacgcttctccttcagcaaagtttcagccttctcactgttagattgctttggctgctgaatgtcatcagcttgagaggagttctcgtcaatttcggtttctttctttggttctgcttgttcttcggtcttaacttcagcttcctttttagcctcagcctgcttagcttcttccgcctcgcgggcagcttgggcttcatcggatgccttttcgtcagccagcgcttgcttcaagatgtcgtcatcttgcaggttgccgtctggctgatcggttgtctctccttgtttaactttttcgtcttcatcaagcaccgtcaaagttggtagcttaatctttttatcgtccaccacaaagtccaactcgcggtcattgacagtccggttgaatttcaccggcaaaatcacctcgaggtcggtcttatcaatggcgttggtccatgaaatggttgactcttcgccatcaatgtcgacgacgactttagtgtcaccatttgaaaatttgaattgtttcttcttcactttgaaataatcagcattatagtcaaagtgcacagtgccggcctgcgatagcccacccactgtcatatcaaatgccaagttggcggagtcgccaacttttgatttcgttactaatgcgcgtttatcatcaatcaatttcgcgttatcgacgacaacttccttagtcgaaatcacatcggctaaagcggttccggcagtaaaaaaattccccagaaccagcgtcaacacgccaattgcttgtatccaaaagcttgtccttttcttcattgttgtcttcctccatatgattgattacatccctctcttatcaacatcataaggatacctgaataatatgcgtaattttggaagaaattatgaagattccgtatcttttgtatcaggtggcaggcgtggattttgggagattgttgcaaaacggcatggcgttaagctttccggagaatgacattgttttccccttgagtattcaataatccgaatagaatgattaccgatcaaatcttagtcataaaaagttctaaagctaaagttttcgctttaactttggaacttttatgtcgacaagtggttagccatttttgttgtcgtagtaattactaggtgttactatatatttaataaaaaaggaggggattagtttgaaagcacgtaagcagggaaacactttggttttaagtattcccaagcagttcaaagtcgctgaaggaactgaatttatgagtatgcaggccgctgatggcagcctcatctatacgccaaaagccccaaatatttaccaagatcccaaatatgctacgactgatcttagatttatccccaaggatactaacgaccaaccagtcggtcgggaggaaatctgatgtcaaatcacccaattacccattatgattatcatggttacactcctaagcaaggggatctggtttacattaattttgatccaagtattggtcgcgaaattaagaaacgtcgtccagccattgtagttagcagtgacgcttttaatttgcggactggttttataaccatctgtccaattaccagtactattagagacttaccatttttcatcaatttacacggtaacaagttacacggtcaaatcaatgcagcacagctgcgaacaattgatttcatggccaaggaacgccatattgaatttgtagaacgagccgccagcacagactttatgcaaactgccaaaatcattatggatgggcttggctttgagagcatcattaataatctttgacacattctatttcaattcgagcagctcagataacttcaaaacgggcttttaagggaggaattccaatgtgtggacgttacatgtttgagccaaagcgtaaccgtgaaattgcgcggatctatgagctggcaacccaagctggctatcagccaacaacgggtgaagtcttcccatcgaatcaaacggcgttggtcattgcccagcagcagaaaattcaagttgtggcgatgaagtggggcttccctggctttcataagggccaactcattatcaatgctcgatcagagtcggtcactgaaaagaaaatgtttgccaagtccttccaggcccgccgatgcgtttatccaaccagtggcttttttgaatggacacctgacaagcaaaagtattggttcaactacaacgaccaacccgaacccttatacattggcggtttctacaacatctttgaaggcacaccgcaaagtattctgatgaccacggcgcccaacgattccgtcagtatcattcataatcgaatgccgttgattttgaagaagtcggagattaggacttggttgatggatgatgaatttgccaatcactttttgacccgacagatgccgatgttgatgcgacagaaggttacttcggaataaacagcttcatttttttgaaattggcctcgtgtattgactgcaagcaattcagctatgctataaaaaggtcctgccaattttattagcaagacctacttaacattattattgtgcggtataaccgccatctaccaggaattcgctgccagtagaataagatgattcatcagaggctaaatatagaatcaaatttgcaacttctacagtttcaccaaagcgccccaatggaagcattggcaaatgctcgctaactaacttctgctctttaggatcattatctttttcaggcttatggattggccccggatgaactgaattcacacgaatattgtacttttgctgagcacaatataatgccgctgatttcgtcatcaaccggaccccaccttttgctgcagtgaaggcaaataaattcggatagccaattaagccttcaatagaggacatattaataatcgaaccaccattagttttcatattttgaatggcatgcttgattccaaatgcaactccgtctaaatcaacggccataatctgatgccattgctcagcagtgaaatgttccgcatcccccattgccgcaattccggcattattaaacaaaatatcaacttttccaaacacatcaataaccttttcaaataccatggcccaatcagcttccttagaaacatcttgttggataaagatcgccccattgccaattttcttcagggctgtttcccgattggtatcgttaacatcagtaataacaacttttgccccttctgtagcaaaccgagtggctgtggctagcccaattccgttcgcgcctccagtgataactgcaactttattacttaaacgtcccataatgataatctcctttcagaacatgattaatgacctagaaatgttgctaaatcgtaagatataatgactgtgaattaaatcggaaagtatggtgaatccgcgatgaacttaaccagtttgcgatattttatcgaatcagctaaatacttgaattttacaaaagcagcggaacatctttatgtgacacaacccacactcagcagacaaataatggatcttgaagcagagcttggcgtccagttgtttgttcgtggaagacacacgctaactctgactagcgaaggcgatgcgttactggaacaagccattgatattgtgacgaaatttgataatatcaagaaaaccattcagccacatactaatgaattaaccggcaagctcacgatcggatatcaaagtttctttgatactacgctcatgtacgatgtcttaaagtcagtaactaagaaatatccaagagtcaccctgtcactttttcgtggtacgccacttcagttaagacgccagttaatcaataatcagtatgatgctatctttggcttaaatacttacatagatagcattccaaatatcaagacaattgaacttcaaaaaaacaagttgcaaattgcggtacccagtacacatccactagccaacatgaaatctgttgacattaagcgattggcaaatgatgatttcattatgctcaatcgcaagatctcaccattcattgttgactatgcgatcagtctttgcatgaaaaatggtttctcacctcacgcgttgtattacgtaaatgatgctgagcaggcattgcttcatgtgggttctggacaaggggttaccttcctacactcaatgaataaggtgaacaacccagttgaaagttacggcgtcaacctgcttgatattaatggtctggataatgatctgaacttcgttttaggttacaaagaaactaataccaatccaattacggaaatttttgtcagagaattaatgaaagttcaccagcaaaaagatggcagcaattaacagaaaagcttaaggacgagaggtctttaagcttttttgcatcaatcacttcgcttcaacgtcttcaagttcaaaaccaactgatttgaatccaccgtttaactgaataaggtgcactttagcctttaatggcaatttagcgattaaatcatctttattttcttcagtgacaccatatagggctgcatggaattgatgagaaccatttggccaatgtccgactgatacacaatagggatccttttcagtgaaaaattcatcggcttttctaaatgtgtaatcgccacccacactagagtcctcaaagcgaatttcatcgattatggcttcatcgcccatctcgatccagtccaggttatagctgccacaatcttggcaagttgggagcggaggccagacgactttgccacaatcctggcacttcatccctaacaccttgccgtcttcgagactgtcataataggtttttaaaattggacgtaatggatacatattactcactcctcaattttgatcttccaaaataataccaactgttgtatggccgccacccatacctcgtacaaggcacttattaacaggcttgggaacttgcgatccaccagcttcaccgcgcatctgtaaaattgcttctccgagcatacatactccagcacacccaaaaccatgcccaaagctaatatcgcctccatgagggttaattggtttctcagcatcaaatcgcgtcttaccttccaactcatacttgtagccttcaccctcaggtagatacccgaacacttcggcactatccagttgttcaccagaggtcataacagtggtaatcatcaaatcaaagtcgctccctttaattccagggtgcttcttgtaaagattgtctctgacatcaacgttcatttgatggaaattaaaaggatacctagtcgtgttggagacagttgcatcgtcaatcacttgaattgggtgatctgaatatttcttagcaatatcagcagaacacacaacaatcgctccggcttccatgttatggagaacactgccgctcttgcgaatatattgagtgattttaggattatgttctgatctcatatattccaatggatcgtcgtaaccggccttcttagccatgtcctcatatctttcatgcatcaaggcgcgaggattgtgtgaggcattatatcgaagattcattgccattgagttataagtgtcatccagttcaccctccgtaattccatagtgtttaatgtaatgtttgccttgttcttcagtaagcaaattatcactgacaccatcaaaacgcgtgtaggcagtatcaaacaatacccgacctggtgaccaccaaccattgtcatactctttaataggttttaatttatatgctggttgatttcgagaattgaaatgtttaggattctctaatccggcaactaaaacaatgtcatattgtcccgatgcaacactatttacagcttcagtaaaggcaatatatccgccagcacaggcctgctcgatatgcgtgattggtttacctgccaaccctgcccactcctctaagctgcctaccggagccatcacaccacccatggtgatgaagttggcaaactgggaataaacaactttgtcaatatcttttggtttaacatgcgcatcatccattgcttgatgacaagcatctgcccatagttcataaggcgaaagaccagccattttaggatcgtcaaaacttcgttgaggaagactacttgtcccgataactgataccggtcgtgcaaattgttgtttcatcatgatttcctcttttctttaaatatgtggtgatagttaaaatgtttgcgcttacatttttagatggaaatatcattcaaagttttttagtaccatgtccctttgacacttaaatcatatcttgaatgcaaactcctgtacaattggacttttacgaattaacgtagacccatgttaaggtattcacaaaacgcataccattattctgtcatccttctttataattcattggattgaagtcaatatttgagacagcttttaagggaattggacccaattcaaccctataagaagccataataaaagccctgtgaattgaattacaacgcttcaattcacagggttagcttatttataatgatgttctgacttccgttaagatcaacagccaactagaccagatgctgtgatcaaaacattgaatgtccactcacaagaacctattcactcttatcaaaactactcatcaaaaagtcagtcaatcgctcctcatcaaccgtctcaatcccagccttcttaaccgcacgcttaacattccaccgactaggcttcttcccactcaaggcggcttcaatggcattcagatcgccatcaatcttgaagaagggattgaacttcagatgggaaagcttgccgtcatcaatggtccagttgattcccagcttgccctggtcaaattcagtatcggcgtaatcgtaatagccaggattatggccgaagttccaggcgtctgtcccataggtttctgccaggcgtttgtcagcaacttcccagtcctgatcagtcatatggtaggtttcaatgtcatccagcgatttgacttcaaagatttctttgagcaggtattcacggaaatcagccatcgtcatcccatccggaagaaagtccttcaggttaacaattgggctacgtttggagcggactcccaagcccttttggatttccatctggtcttcagtgaggacttttctggcattttcaatgttcaaattatacataatcgttccgccggccgccaagccttggccgctcttaaacatggtcatgccagaccatttcttaccgtccaaaatgaggtcactggaattctccctcattttgacgtcgatgtttaatttacgaagcgctttcaaaactggttctgcaaaatgcccataatcgccaaagtcgtcggcgttatccgtcaaaatgttttcaaagatgaagttccccatatcgtgatagacagccccgccgccagacgttcgccggaccaactcaatgtcgtgctcgtgcagatagtcgatatcgacttcagcccacacgttttgatttcggccaataatcaccgatggcttgttaatatagaacataaatccgtgtccaggaagtttgagatcattcacaaaataattatccaatgattggttcacccgcgcgtcatagctgggcttgccattcctggaaatatcgattaggtacatctgacattccccctttgttcaaattctcgtacatctctaattatacggtataattgaggtaaataatatcgaggcggtgtcgttatggcaaaaatttcaatttggcaaaaaatcattaatttcttcacaggcaaaaagcagtctgctcaggctccggcccaggttaaagacggaatctggtaccggaaggaagccgacggtaactatctattgggcatcgacaaatctgtctatgatttgatgggcaagattacgttcgctgattttcccaaccagttagatacgattgaagtcgatgacgatctgttggacatcgaaggggacaaatcggtggaaactttgaaatcaccaatttcgggtcggattgtggctcgaaacaaagaaatcggcaaagatattgaaaccctcaacaagcccgacccacaggtaaattggattgtaaaagttcagccggcagcttaatcattcaaataaatcgaacaaattttgagccactttctcaaaaagaactataatgaagttagatcaaatagaaggaggtaattatttatggctgaagaaccaggtgcagaatctccattattgaacaaaatgatgtctgaagcattcgactggagcgatcaaaaattaccagtccgtgatgctatttgggactattacatggagaaaaacgaccacgacactctcaagactgaaaaagatgttgaaccttacatgaacatgtcaactgatgatcttaagagcaaagctgaagcattactcaagaagtaatttttcagtggttaaacaaatacccgcactagtttcgtgctaggcattcaaatgatcttcaagcttttggcttggaggtcattttttgtatggaatcaaaaagaagctgaatcatcagctcccaattatcaattatcttagtaagtacccgccatcgaccggtaacatcaccccagtaacgtaatctgatgcctgacttgccaaaaacacgacaggacccatcaactcttccggcacaccccactcacctgatggaatgtggcccttgatctccggccccctgattggatcttcctgcaaaggtttggtcatatccgtcttgatatagccaggtgcaaggccattaacttgaatgttataaggggccagtgcgtcggcataggccttcgtcaaccccataaccgcatgcttgctggcagtgtacgggaagatgaacttaccagcgcgatacgactgcattgaaccaatattgatgatctttccactcttttgcttgaccatcaccttggcagcctcgtgtgataagtaatacaaagcgttcaagttgaggtcgatcaccttttgccaatcggcatctttaaagtcaagcacgtcattgcggatttgcatccccgcattattcaccaagatatccaagtggccaaatcggtccaaaactgcttgaatgacctcactcgctgcaccatcggctgtaatatccttctgcagaaaaccgacgtgttggccgtttgcctcaacggcctttttggcatcatcccagcccttttgtgatcgactcacaataaacacatctgcgccatacatcgataaagcaattgaataattaagccctaatccagatgcgccgccggtaatcaatgccacttttcctgcgatggaaaaactgtctttagtaaatgtcgtcatttggaagtcctcctatattgaatgtgtgggtagattatttttactatacattatatttcccaaattggtgtgaaaaagataatggctaaaatgaatcatctatggagccttacggattagtaccaattacagtatcggtaccacctgtttggcataatgaaacaccaaaacccgcttaaccgcaaattcgttcaccatgtatgacccatcgtcagagaggtaggcttgcttgtatggaatcagataatgaggatcccgatagcctttttccaactttggattacacttaactgccaatgccgggtgcccggcattggcaattctaactcgcactgattccttgggagacagtgaaatgagcgcaatcagcacgacaacgccgacaataaagatgccaatatatttcaagattcgtttcagataaatcatattctccccccaattagtgccgccaacactatttttcgagtttctttttccccgcattcaaaacctcatcagacacatattcactggtaaaccgttgcagtggtgtgtattgatgccgatctttaaaggcaaccgggatcgccttgataattccgaccatcaaattattctcggtgataaaaatctggccgacctgcttgaactttcccttggtgtgtttgccggtccgccagctatgtagcttaaagtccccggattcatcgcgcttgatgcgatactgcccggagtcatcggtttccagtgggacgccgatgaattggttcacttcgtacttgcctttcatgaatttccgccctttcatgactaatttgtgaataaagttagaattaaaatctaatctttttcaaaacacaacaattatagttattcatgctatacaataatagtataataatttttcgaggaatggggtgaaatgatgaatcaaattaaacttgtgaccgactctgcggctcacctatcaaaagctgaccttcaagcatacggaatttcggtcctgaatccgccaattatcatggatggcaagctccttggttatgtcaacaaaattagcagcgagaagttcctgcaattatttgatcaatgttccaataagccgatcattggtgacgtttctgtcggtgaaatcactcgactatacaatgagttgggcgctgacggcagccagattctctcgattcatttaagtgataagctgtctaatacctatgccaatgccaagaccgctgccagcaagtcgaccagccaagtcaccgtcgtcaacagccaggtgaccgccgccggactatcctatcaggtcttggaagctgccaaactcattgcggcaggtaaatcgattccggacattttgccccaactcactaaaatccgtaaccgtacccggatcttcttttcggtccgcaacaaccagcagatcgtcaacaatcgcatcatcggcaagcttcgcggcttcttgggcaaacacgccaatacggcctacatgattcaattcggcgataacgatttcgacctggttgcccatggctccaaagacgagtcgctcaacgaattctggcagacccaaatgcaggcgatgcacgacgaatgcattgttaaactgaccattctgcattccggcaccaacgcccgagcccagttcttgcgggaaatgctcaacgatgagttcccatttgtaccaatttccatcgtgccaaccaacccggagatgaccacctttattggtcgggagtcgaccggcgtcacctatttactcggataatcggctgttcaaaaaatgttatgtaaccaataatgaccgctaacgcaaattcaacgttagcggtcattttagatgttaatttacaagttaatctgcctcatgaattggctttcccttgcggacactctcccgttcaaccaatcgagtagccacaacgactttttccggcgtgtgctcatcgttgtccagattattatccagcaggcctaacaaacgaacagcgacggcgcccatcttaccagtattaaccttaactgccgtcagtgacgggatcacatacttggcaaccgcagtgtcgttgaaactgaccaaactgacatcgtccggcaccttcaccccattttcatggagcgccttcaaagcaccaactgccatggcatcgttggaaacaaacagcgcgttggggaacgattctttcgaccgtttcagtgcttcgtcaacggtgtcatagctggactggagggtgtaatcaccgacaaatacgttggctgggtcgtacagggaacgcttttcgaggtagtttttgaaaacatcgaagcggtgatcggtaatcttcaactcatgatcactactgtattcaacaccggagatcatcccaatgcgcttcaagccattctcaatgaagtatttcagtacagacttagtggagctgtcaaagtcggtgaccacacaatcatgccccttggccaaagtgtcaaagtcaacaaagaccaggttgtcactgacttcctgcatctcctcaatctgggcatcactgaacttgccaatcgccacgatgccgcttacgtcgtcaatcgcagtcagcggatcgccggcaaaataacgtttgatcttataatgatcgcgttcggcctgcttttccacgcccatccgaatcgacaaatagtacaaatcatcgagttcctgctgctcggtgtaccattcaacaatcgcgatcgtatctcgagtcgagctcgaccgcttctttttcgtgtaatccagcgcttcagccgcctcaaaaatcttcttgcgagtcaggtcactgacagataatgatttgtcataattcagcactcgcgaaacagtggtgatagaaacccctgctttgtgcgcgatatctttaattgttgccatgatctcacccctccatcaaatactgcgaatttatgtatcgaatccttttagttaatttactaaaataaatatatgttctttaccttgatatgtcaaggatattccgttatattggcgtttttggctagtaaacttgttgacgtgtgcttggtaaatttctataattaggttgattttaaatataaggagggtcatgtcgtggacgacaaaattgaagacgcttaccaacaatggaccaatcaacctaatttaccagaaaatcttgtacttgatttaaataaaatgaaaaataattcagaccaaaagaaggatgcattcggaacggttctctcatttggaactgccggaatgcgtggggtgctgggtgccggcactaatcggatgaacatctacaccgttcgccaagctgctgaaggcctggcttcatttatggatactttggatgaagccacccgcaaacgtggcgttgccatcagctttgactcccgttactattcaaaggaatttgcccatgaatctgccaaagtcttaggttatcaccatatcccaagttttgtattcgacgacattcgccctacccccgagttgtcattcgctgttcgccatttgaacacctatgccgggatcatgattaccgcatcccacaacccgaagcaatacaacggctttaagatttacggccaagacggcggccagatgccaccgaaggaatcggatctgattacttcctacatccgcaagaacagcgacttgttcgctatcaatgttacgccagaacaagagctgcgtgaagctaaaatcatgaacctgatcggcgaagcagtcgatcaagcctacttggaaaaagtgcaaactgtcaacatcgaccacgacctgatcaaaaacgtcggggccaacatgaaattcgtctactcaccgcttcacggaactggtaaaattatcgctcgccgggccttggaagccgctggtttcaagaattacgttgtcgtgccggaacagaccatcgccgaccccgaattcccaaccaccccatttccaaacccagagttcccgcaagcctttgatttggcgcgcgaactcggtaagaaagtttctgccgacgtgctgattgcatctgatcctgacgccgaccgcttaggctgcgccgttcgtcaacctgatggcgattacaccctgttaagtggaaatcaaattgccagtgtcctcttgaactacattttggccgccaaaaagaaggccggcgacttaccagccgatgggaccatcgttaaatcaatcgtttcgactgatttggcacccaagattgccgcttcgtacggcgttgccaccaacaacgtgctgaccggcttcaaatttatcgccgaagccattcaccactacgaaaccgaacacgaccacaccttcctgtttggctttgaagagagctttggttacctgatcaagccattcgttcgtgacaaggatgccattcagaccgtgctattgctcgctgaagttgctgcttactataagagtcaaggcaagactctgtacgacggcgttcaagaaatgttccagaagtacggttactatgctgagaagaccatcgccaaggaatttgacggcctggacggtaaggacaagatggcccacatcatgtcagaactccgtgacaatccactgactgaatttaacggccacaaagtcttgagtcacgccgattaccagtcatctgaattgacggatcaggatggcaagcggacgatcattgacttaccgaaatccaacgtcttaaaatactggctggacgatgagacctggctggctgttcggccttccggaactgaacctaaagtgaagttctacttggaagtcgatgacaagagccaaggcgcagctgatcagaaactcgctggctacgtggatgccgttgacaagatgattgacaaattgatgaataactaaatttttaacctgaagctgcctgatctgaaaggattaggcagcttttttgccgtctaaaatgctacaataattttataggtcgtatcaaaaggaccatccaagggggaatctacattgaaaccaaccactcagctgattgcgggggcgttattcatgctcggggcaacatttatccagactcagccggcccacgccaccgtggtcaaaaacagctttttgaaaacccagcgcagcatcagtacatacaatagcaacaagcacgccaaactcactttgcccaaaggaacggtggttcaagtcgccggcaccaagcatctgcatggcaataagtatgtcgacgtctatgtcgaccggttaagctataacatcagaaagccgctgctctcggtgaaaaaaccgaccgtttacagtcactggatccgcgccaaaggctacaactttaagcaaatccacaagcccacttatctgagctactacgctgcccagtccgacggcaaaaagtcccaggggaaagtcagaaccgaaaccggcgacctctggaaaggaacccgtttgccggttgactacgccacttcggctgccgctcgactgcgagtgacgaccgacggctacctggaatacgatgccagttcgccatttgtcttcaaagtctcacccaaacccactgccagcctgaaagtcgaaaaggccagccacccaatggccagcggcgagacgattttgaccaccaaatcacgagtgaagcagcttccctttgtcaaaaaatccaaggaccactaccaattgaccatcaccaatgccgaggccggcactatcaccgtagtgccgaatacctccaaggtcaaaaagatcctcaccaattggattttcaaagttggtaaagaatcctggtatgaaaataacagcgtgaccacgtttaaataaggggggaaagcaccatgacaaaattcagattacaattcggactgtttgcgttgggggttctcttaacgatcggggcaacaattccggtagatgccagcacttatctatcacatttttccaaagatcaatacctgatgaccaaaaagacgatccacaccaccaacagtcactataaaaacatcaaaatcaccattccaaagggcacggtctttaagtccagcagcctgaccaggagccgcaaaaccaagcatccatacttaaccatcaatttgaaccgcctgcactggtcactgcgaaagggcgtcgtccagtcataccacaacgtgacgaccactagcggcatctgggccaagtccagcaccttcaaaaaagtccacgcaccggcttaccaaagttacttcaagcagccgtataccggcacgatcggcggtctgatctggcagggcaccaaagccttccccctacgccagcagtacaaaattgaaaactgcctgcgggtgaccgatgacggctacctggaatatttcaccggctacgactactgggtcaaaaagatgccagagccgcattcagccgccaaagtggaacagttggtgaagaagggtaacgcctattacttctacaccaagtcaaaaatcagcggtctgaccatgaagcacgtcgccaaaaaaggcaatcaccgctaccgtttgaagatcaccaagaccgaccagcacatggctaccgttaatcccgcccaagacaagaagtatgatgaaagtgtcaccatttcgatccgctattacgttggcggtaagaagttctacgtcaatagtcaggtcattgaaccgtaatcggccgtcaagatacttgcatacctgccatagattgtgaataataaaaatatgtcagaatgcttatttaacttttagggggaatgattagattggaaaattcagtgactcgtcgttattggcaggccgccattcttgaagtgctggtatttggtttgttgatcgcgatttattcaattgagctggcacttgggatgggcgaaatctcacagattgctgttcaggaaattttgttattagtgatcttttttgcgttaaattattattggatcaagcaacccgtcagattggcagccactgtcaactttggcaaaacgctattaatttcggtaccatttattctggttcttttgtatttgctattaatttcactggccccgcacagcactcacactatcgtgatggcggccgtttccggaatcggtgccggcgtttttgaagagtatttattccgtggattgattttaggcatcctcttgaaatctttccctcatttttcaaaagccaaaacgatttggtacgcggtgaccatctccagcatcttatttgggatcgcccacggcagtaattttatgtctcaatccgtttcatcaactttggttcaaattttcggcgccatcagtatcggcttcttgttaagtgccctttatctgcggtcaggatcaattatcgttccaatgctgtttcacgcggcttgggacgctactatcgtcttggtttcgggcagcaccttcgccaacgtcggctcgtcaaccttctcaccgctggcaaccgttggtgagttagtattgttcgtactgatcgcgatgttctattttcgaaagtccaaactcagtgagattgatttgaagcattttgaataatggtctgtaaaatctggggtaattcaaatgaaacaacgatcaaaagtgctgatgttatcaattggattaggtctcgcgctctctgcgtgttcagcagggactcccgcttctaaaaaggattcggtcacggtctacgacgcgcataaccgccagatcttaactaccaccagccaggcaaaaatcaagcgcgtcaccaacttaaccagtcaaagtgaccgcagcacggtcaatggccaattaccagctggcctgcgggtcaaataccgctacttgctacaccagcgggcgcacgacgttaacatcaatctgtacgtctatgccaactcacgaaatgtcaaaatgactcagatcccaattctgcatacgatcgtttatcagttgtccaagcaggattatgagaagttaagtcaaccggagacgtatttaaagtaaatttgctggcgggcaatgataaaagatgacaaaaactcacaacttccgactggcagttgtgagtttttgatttggtcctttttctaatgaatggttaatgtatcgagggacaaattacggtataatttttacttgtagggttgtcaaagcggtagtagtcgttttttgaatcgaggtgttgcgcatgcaacaaaaatctatccaagaaaggattgctctaagtcttaatgctatgtgcagcgatgatttttgcgatcgctgcatgtctaaaagcagttgcctggataattttcgcagttgcggatcttatccgggcaatcaaaaagaaccgctcataaactttgacgggtctagcggttctccgtaactactaagctatcgctctacaactttaccacgactctattatatcatgggtcgtggtaattttgtatccagttctactggacaatgatccgagccgaacacatcagtcaaaatcttcgagtcctcaatctcatccgccaaccggttgctggccacaaagtagtcaatccgccagccggcattccgatcgcgggaatggaaccgataactccaccaggaatagatgtccgtctggtcgggataaaagtgcctgaaggtatccatgaagccggcttttaacaggttggtgaaatcttggcgttcctcatctgtaaagccagcgttgtggtggttggattgcgggttcttcaaatcgatttctttgtgggccacattcagatcgccacagagaatgaccggctttttggcatccaattcagttaagtattggtagaaagccttgttccagcccatacgaaaatcgagtcgtttcagcccagccccagagttgggaacgtagctggtcaccagataaaagtcgggatattcaagggtgatcgcccgcccttcgtgattgaactcgtcgctgttaatgccataggtcacatccaatggcgcgtgcttggtaaaaatggccgtgccggagtaacccttccgttcagcataattgaagtattgctggtagccaggcaagtccaactccaactgcccttcctgcatcttagtttcttgaatgcagaagaaatcagcatccaacttcttaaatgtctcggcaaagtcatgcttcacggcggcacgaagcccgttcacgttccaagaaatgaatttcatgtgatcccgtccttttttgttgttgggttaattataacgtaaaattgtattatctttcactatagtaaataagtgatgagctttacatacaaactatttataaaagataaaccgcacggactagcctctatttaatagctaacgtaattatgctaaaatagttatgtgagctgaatttacaacccattaatataatatactttttgagggggtattcttttgatacgaaataaattttgtacactgtctacaaagttagcacaacttattcttacgacagttacaattggtattgcattcttaattttaggagggatcacttcgtttgctgcgactgcaagcgataacggcgctactatccagcgtacaatgtggttaactggtgaaccagcgaatggtggttcaccagtaaccctgtcttcggtggtttcaagcgacagtccgacaaactataaggcccctggtgatgttactaccccacaaaacggaagaactgttaacctggacaaatataaaaacttattgattcactattcagttgagaatatttcatcacaggcagaaaaagttgaagcagttttatttttcccaaactatgctcctgttttttcatacgattcgtcgagagccaatcagatatcattcaattctgagcaaacggatcctaaatttaccgatggatatagctacgtgggaggatcttacactgctacacccatttccgaccagactccgattgctatttacatgggaggacccatagacccagctgacggcgctccatcagctcaaagtctaagcccaacgaagaaacttacaatggtggcccctgttaaacccaactcacacttcgattttaataatccaattgatgatagcttctacaatgacacatatgttttcgggttcgtttctgacgacacagatactcaattaggcgaccaagacttatatgccaaaccattcaaaaatatcgtcctggcaaacgaagagtcattgccggccaccaactatgacaactataacgatttagtaaaagccgccgttgccaatgtgaccgcattattcaacgacgatgccacgaaggatacgactactgatccagcatcaatcgtcaaagtcaccccaggaacaacagcaggaagttggaatatcgactataactatagtggtgtatcaaagcatataactggtataaaaaccaccgatgcttcttacattgacggaaaagacttcaaagtaaattacggcagtaactgggattcacagaaattcaacggtttaactaaacatctcgaccaaaatggacaagctgtgaccaaattatccgatggcgttaacgtcaccattcagttaaatggcaaaaccgtcaatgcagtagatacaaataatgcaggtgcggtttacgacgtcacttacactaccggtaataatgctgcttcaaagaccgtcaaagtaactgttggccagcgtggcaatatcccaagcaacaacaactcaaacaataacaattcaaccactaacaacaacggcaactccggcaacagtgcctggaacccatcaaacccaagcaacccaaacggaaccggcctaccaaactacgccgccgttaaaggttcagcggtttacgcaaccaagggtatctacatgtatcgcagtgccaatttcaagaagtcacaacgcatggctacctatccaaaggctaagcgggttaaccgcccaatgtttgttgtcttaggctatgacaagtccaatggtggcgcccttcgttacaaggttcgtgacgttaaccacggcaagaagaccgctggcaaggttggctacattaccgccaacccgaagtacgttgtcaacgtttactacaagacaatgcctaagagccacaagattaccgttattaacaagaaaggcattcacgcatacaagaacgtgaacttaactggtcgcgctaagaccttcaagaaaggcactcatgtaaccgttaagagttttgaaaagcacaacctgaccacccgttacaagttaagcaatggcacttacattactgctaacaagaaactggttattcaaggtaactactaatatgtaggaattaggaagtctcgaccttcgtcgaggcttcttttttgtggacttcctttgttttgaatcaaaataagggttaaaatacaattacaaccccgaaaagaggataatcgaaatgaaaacagccgtaattaccgacagtgccagctacctcgatccagtggtcgctgcccaatataacatcaccgttctgccgattaccatcatcttcggcacccaggaataccacgatggcgttgacatcacctcgcaagaattcctgaagaaattggcagagactgacaaattgccgacaactgcgcaagtcaccatggcccaaatgcaggaagcctttgatactttggctgccaaaggatatgatgaagccatctgtgtcaacctctcatccgggatcaccagcttctatgagaatttagtggcctacagccaccaagtcaccaacatcaaggtctacccgtttgactcgaaaatcgccagcgccggcgaagctgacttatgcttgttagcgggtaagatggccgaaaatggtgagaatgccgatgtgattatccccaagcttgaacagttgcgcgactcgattcacgtttctctggtcgtggacagcttggatcatctgcgcagaaccggccgaatttccaacacctccgcattttttgggaacatgctgaaaatcaagccaattctgacgtttgacgacgccggcaagatcgttccagaggccaaggagaggaccatgaaacaagcgctccagcacatcatcaattccatcgaccagacgactttcgattcgccaatgcggatttcagtggtcgacgccaacaacccagacttaagcaaagcctgggtgacagcctttcatgaacatttcccgaaggccagcgtcagcacctaccaaatcagcccggcgattgccgtccataccggcgaaaaagccatgggcgtcgtctgggatctggattggaatcaaatttaaagccaccagcaagtaacttgaaccggagtgagtgaattgccactcgcttttttcttgccctggaatttgtctgagaagttttgagcatctgccattatttcaaaagtcaacattcaaagtatcaagaagaattcaaattaaatcccattttcaactattgaatcagaaagagatgaaatcatgtccaacactaacgaaaaaatcagccggcaaacctatcttgccctgctggctgccgcactgctctcatttaccggaatcctgaccgaaacgtcaatgaacgtcacctttcccgaattaaccaaagtcttcaacgtcaccctggacaccgtccagtggattaccaccggctacctgttgatggtgacgattgtcatggcaacaaccgcctttctacttaagaaattcaaatcgcaaagcatccacttactggccgccattgcctttgtggtcggcgacatcatgtgtgccacttcaccaagctttcccatcttaatgagcggacgattgatccaggcgattgcgaccggattgtcgacgccgttgatgttccacattatctttaacaaaattcccgcaggtcgaatcggttcgatgaccggtctggctgggatggtcatttctttggcgcctgcgcttgggccgacctatggcggaaccgtgtcatcgaccatgtcctggcggatgattttctggttaatcctgccaatcatcgtcatcagctggtacctcggatcgcggtatattcgcattgatccagtcggcactggcggctttgacgtcatcagcttgatcttcctggctgccaccctgttctcatttgtcttcggtgtcagcaaggccggcaaatattcactgttgagtgggcaagtcttgatcccgtttgtcattggcttcattagtctggcaatcttcatttactccgatactcacggtaaaacccagctgctggacatccgaattttgaaatggctgtcgtcttcactgtcggcgttcacctacttcgtcctgcaattcgtcaacatcggcgtgtcattcctgatccccgtctattgccaatacgtcctccacagttcgccatttatcgcgggactggtcctgctgccgggatcactagttggtgcggcgatttcaccatatgccggccacctcgctgacagtaagggatacgccttgccaattattctggggctcagttcaatgacgttgggcggcctgattttcttcggcatccaagccgtcttgaccgcctggattgtcctgttgaactacaccttcctgcgttttggcttcaatatgggcttctccaacaccatttccaacgccatgttaaacgtgccgcggaagtataccgccgacgtcaactcactgttcagtatgatccagcaatttgccggctcgattggagtcgggattatggcggcggtgatggccatcagtcagaacaacggtacaggaagcttggctgctcgttcgtttgtcggcgggaaatatgacttcctgttggcaaccttactgagtgcagccgcattgattgccgctgtgattaactttagactgcagaagcgaatgaaattgaatattgaagaatctgattaggtccttctaagctgaggccgttgtgcaagtcgctttacttgcatggcggccttttttgaccgccattcatagttcaagttgccaagtcgctttgattgaatttccccctcaatccgcttaaacttactttgatgattacaacaggttgtacacaaagtaattatcatgtcgactgtcgatcagaattgtaagggggatttcacttatggtaaagataggaattaatggtttcggtagaatcggtcggttaattttacgccgaatcttggaaatcaacgatcctgatttggaagttgttgcgattaacgatttgaccagtccatccatgctggcttatctcttcaaatatgactcaactcacggtaccctgccatatgagatttcgtcaaccgatgactcactggtcgttgatggaaagaactaccgtgtttatgcagaaaaagacgcaagtaacatcccttgggtaaaggaaaatggcgttgatttagtccttgaatgtacaggtttctacacttccaaggaaaaatcccaagcccatttggacgccggggttaagaaagtcttgatctcagctcctgccggcccaatgaagaccatcgtgtttaacgttaacgacgatactttggatgccgacgatcaaatcatctcagcaggttcttgcaccaccaacgctttggcaccaatggcttacttcctgaacaaggaattcggcctcgaagttgggaccatgaccgcgattcacgcatttaccagttcacagatgattcttgatggccctaaaggtaagaagttccgtcctaaccgtaccgcttcggccaacacgattcctcattcaaccggtgccgctaaagcaatcggcctggtaatcccagaacttgaaggccatttacaaggccatgctcaacgggttgccgtggttgacggttcagtttgcgaattggtttcagttctcaacaccaaagttaccgctgaccaagttaacgatgccatcaaaccgcacaccgttgataacccggcatttggctggaacgaagatgagattgtctcatctgacattatcggcgacacccacggggcagtctacgacccaactttgactgaagtaacctctaacggtgacttccaagttgttaagaccgctacctggttcgataacgaatatggcttcgtttccaacatggttcggactgccaagaaattcgctgaagtctccggcttgaactaatttaactaagcaatcaaaaaaatcgtcacaccatttattgagaaataaatagcgtgacgatttttagtgtgcccgagttaagctgacagtcaaaacattatctttcgtggtgctgtagctggccaagatgccgttgacgacgtcggcggccttgccatgactaagagttgagcgatggtaagtgttaatccaagtccccagtgcttccatgccaaattcgaagccttcaaacacccgcatgtactccagtgactgcggttttggtgtcacaatcgtgatcttttgtactctctggtcggcaatgaccatcgacaatttgatcacgtctgtgtcgaagaaaacctgagtcccatcagctacgctggtcggcagtttgtaatccggcagctgaatgttttcgttgtacacccgtgaaacgtactcgtatgtccccaaatcagtggtgcctaattcttgtgtcacagaaaatcccccctagaagtgttacgtgacttattggtacttacaatgattatatattggtttgggtatttattggcaaaattagcttgcaaaagcggaccgttatggagggataatcgtgaaaaatccgggaccaaaagccagcaacttccttgctgacggcaaataaaaacaccattgagattgatttctccaatggtgttattcgaactatttgatcactttgacatacttctgattagcagtcacataaccgcccttgacggcatagcgcatcgtgccggacttgatcagtgaagcttcatgactgaaggtataacgcttaatcacgagtttggtgcctttcttgaagtgcccatttcgcttagccaaatttggatcggcatatcggttgatgaagtgggtggcttttaattgctgaggctgcttgattttacccatcttaactaacttccggttaccggtaatgtagtggccattgctcaggacgtaccgggtggtcaaattgtgtttgacgaagccggttacgtggagaaccgttccctgcttgatattcttcactttgcccgtcaaatttttgttgaggtattcattgacaccgcggggattgatcaccgtcagtgtttgatgactgctgtgataatagactggtcgaacatagtcaaagttggtggtaatgtagccagtccagccgtcggtcttgctcaaatggttgacgtcacggactttataacgcaaccagccagcattggacttagcgtaatcagtgaccacaaacatcggtcggaagacccgtggcttcttgacatagccaaattgacgatcggccttcttgaaggttttatctttgtagagataaatcttcttcaaggaataaaccacttcgcccttcttagcaatcttaccggactgattgtcagtagtcgttcctggggtcggttgtgggctcggcgtcggcgttgggttgaccggcgttaccgggttaaccggattaattggtggattgactggagtcactggggtttgtttttgcttgtagtagtagttcacatcaggcgtcttatcactgtatatcccagtaatattattcggcagtctgtcagtatccaaagtgtaagtctgcccattaacagtgagggtttgcggttgataggaaccgtcggcccggtaggaatcgttaattttaccgtagatctttttggattgaatcaaagcaccagtttcttcattgatgtagttgacagtgactgtcgccgagttatcggttggggataccggagtggcatcctttttgtagtaatagttgactgcaggtgcattttcggtaaacttcccgttaatattatcaggcagcttagccttatccaaagtgtagctgtcgccgttgacggtcagcttgtctggttgataagggccatcagcttggtaggtgtcaccatttttgccatagattttcttggattgaatcaaatcgttattgtcttcattgatatagttgacggtcactgcggtagagttattggttggcgttaccggggtggcatctttcttgtagtaatagttcactgcgggcgtttgatcggaaaattgacctttgatatttgccggcagtttgtctttatccaaagtatagctgtcaccgttgacggtcagcttatctggttgataagggccatcagcttgatagtcgccaccgattttaccgtagatctttttggattgaatcaagtcgccggttgcttcgttgatgtagttcacattaactgcggcagaatcattggttggggtcggcggtacgtcctttggagtgtagtagacattgatggtatcgtctttgcccaagacacctttgacgaccggctgatcagctgtgtaaccggctatttccggagaatcgatttcgtaggttcccgcaccactggctttgtatggatcagccagcactttgttggtgcctttttccaggtagttgatggtcagatggtattcggtgattggttcgtagacaaacgttagtgggttgccgacgggtaacggcattgaggccgtcgcataagtccgaatcatgccataactgaaatcggcagcaataaagccacccggcgtcgccttaacagtcacagtcttactttgagctttgccagtaaaactaaaatcgggaatcttcgagtaatcaaatatcatgtacatctgttgagtattttggtcgtcaatcacttttctggcaattgtcacataccgattagattgttcaaattgccaatcacctggtgtcgtggccgtaatgttattgattaaaaattgatgggcgttattcatgtagggaactctcacaagtcgatacccaggaatggtggggtaattaacatcgacaaaagttcctgaatagccggagatgttctgggttggcgccaactcgttgcctttggcatcaacaaattttgccggcacattatttaaataattaagaggattggcggaacttgacgcatacagatcattattctgtaaatccaactcaatatgaccattttgccaggaaaattgaacattaccggcattataggtccagttgggattgaaatcactcgccgttggccctggaacctcaatcgtattcgtcaattttccatcgctatcgacgttatgcagataaaatttcgagttgtccttggcccagccgatcatccaggcattagagccggtgtaataagcatagttgatcgtttcatctggattgggtgcttgaatataatcattagagttgatggttccctgtgtatcggaaattgtctgggagcccactttcgcattggtgcccattgggttggccaattttccggaaacgtagatgggtgcttgatgaaaaacacttcctttgtaaaaattggtcactggaatatccgagtgttccttaggatcaatcgttgggttgtcagtcttatcagcgggatcgggtgccttcaccactttcatcggtgtcacaatcgtcccgtccggtaccgcatcatcagcaacttgcgtggtcgcggcatgggccacatcatttgaagtcatcgtcgaatctgcgttggcaaacgtcaggattccccctgtgctaatcacgagaagtgacattagcaagtatttattgactttcatattcgtattcccctttggttattgttgctattagttatcttatatattcaaacccattataacgaacatatcccagaaatgacattaacttgcttgccgcaaaagacaaaaaaacgcccactttgagaagtctcaaagtgggcgttaaatcggcatttcaatcgtataaatcacttaattttttctgaacgtctgggtgattaatgaactcatcgtaggttgtatccgccttatcgatcagaccgttgttggatacttcgattatgtggttggcgatcgtttgaatgaactcgtgatcatgagatgtaaagatgatcgacccggggaagttcaccaaggcttcgttcaaagccgtgattgattccaaatccaagtgattggttggatcgtccatcagcaaggtgttgcctttttggagcatcattttcgacaacacgcagcgaactttttcgcctccggaaaggacgttgacttccttgttgacatcatccccagagaacaacattctccccaggaatccacgcaggaaagcatcatcatcgctgcccttttcagcaaattgccgcagccagtcaatgatccgttgatcgttatctttgaactctgaagcaaaatccttcatcagagcagacatctcaaccgtttggccccatttgatctcaccactatcaggcgtgagttcaccagccaaaatctgcatcaaagttgtcgttgccaaatcattacggctgaccaaagcagtcttctcacctggacgcagagtgaaggtcacgttatcaaggatcttgacaccgtcaattgacttggagagcttgtcgactctcagcaagtcattccccaatggccggttctcctcgaacttgatgaaaggatactttctcgaagacggcttgatgtcttccaaggagatcttatccaattgcttcttccgcgaagtcgcctgcttggatttggaagcattggcactgaaccgggcgacaaaggcttgcagttccttgatcttgtcttccttcttggcattggaatcggcccgcatcttggcagccaattgactggattgcagccaaaagtcgtagttgccgacatacatcttgatctcaccaaaatcaacgtcacacatcatcgtacaagtctggttcaagaagtgacggtcatgagacacgatgattgtaatcttggggtagtcagccaagaagttctccagccattcgattgagtagacatccagtccattggtcggctcatcgagcaacaggatatccggttcgccaaataaggctcgggccagcaataccttaaccttttggccttcagtcaactcgctcatcaattgttggtgcagatcttcaggaatttccagtgactgcagcaattgtgaagcatctgattcagcgttccagccgtccatttcagcgaattcggcttctaaattggcggccttgatgccatcttcgtcggaaaaatcagctttggcatataaagcatccttttccgccatgacgtcggccaaatgttggtagccttgaatcaccgtctgcatgacggtctggtcttcaaagccataatggtcctgacttaagctggaaatccgctcgttcttatccatgtggatttcaccgctgcttggggtcaattccccccgcaacagttttagaaaagttgatttgccggcaccgttcgcgccaatcacaccgtaacagttgcccggtgtgaattttaagttaacatcttcataaagttttttacctgagaattgtaatcccatgttttgaatcgtaatcattgatttacctcgttcaatagcctgcgcgcagtcgtgttcaaaaatacaccgacagcccacgtttcccataatcaaaaacaatggccagggcttgattcgtcctgaccaatacatgtcttacaaatatatcatattaatagaagagaaacaactagacctcgccgagattgttgaagtactcgacgtcaatgtcatcatcagtgatgatcaacttggtgacactgccgttcttagtagcgacacccagatccagttttggtgcgtaacgatcgacaattgagcggatcgtcatcccgtgggagacaatcaggatatcctcgccgtcatgggtgttttggcgaattttatcaaagccgtggtcgagccgctcccaaaacatggcgttattttcagcattgttgtacaagtcggcccggtggatcaagtcccgtgcccgttccaagccaaaattggtcaacacttctttttcggtggtttcttgaacttgggcgccgacgaactgccacatttgattaaggtcgttaccttcgaaataaccgtgaaattgttctcgtaattcgggatattggtaactaacaatattcatgttatgcggattagctttcaaaataatttttccggtgtcgattgcccgaccggagtcactggtaaaggaagcggcaaaattaatctttgcgagtcgtttcccagcacttttagcatcttgaattcccttttcagtcagcggagaatcaatccaaccttgaaccttgttgtacatgttcaagtatgtttgtccgtgacggaccatgtaagcagtaaccttcgtcaaaaaatcatcccatttctcaaaaatttgcttttacataccctaagtatagcggacttatcatggtttagcattaaaagtcactttgaatctgagaaatgtgaaactgccgccagactggctttcactgccagcttcttgttatacttatggtaggaactgaactttacttataaagcgaggtcgttatggacactttaatgaattttgctccctggcagcaggcactgttcgccacattattcacgtgggcagtcacggcattggggtccgcattggtatttgctttcaaaaccatccgcagtcacgctttggccttgatgtatgggttcgcagccggtgtgatgattgcggcatctttttggtcgctgttggatccagccatcaacttggctgagcagcaggaccggatcccctggctggtcgttggcattggttttgccgccggcggattctttttgtatctggctgataaaatcattcccggaatttatttaaaacgcgctcgaaccgagggtagttcccgagcggccgtcaaacgcgcgattctactggtcttttcaataaccctgcataatattcctgaaggtctggcagtcggggtggcctttggggctatcggcgctgccggtaatggcgaacaggcggcaatgctgctggcagccacgacggttgccattgggattgggctgcagaacttcccggaaggtgcggcggtttcgattcccctgcgccaaggcggcatgagtcgattccgagcctttatgtatggtcaggctagtggtgcggttgagccgatcgccggggtgttaggcgccctgttggttgcttcggtcaactcgctgctgccatacgccctgtcgtttgcagctggtgcgatgatctacgtcgcctgcaaggaactcatcccggaagcccacgccaggactaaggaagaatctcactgggcgatctttgggattatggctgggtttacgttgatgatggtgctggatgtggcgcttggatgatcattagaataaaagagtgtaaaaataagcaatcacttccagagtctaagggggttagccgcgtatccagattttggacgtttggctaacccccttatatgaccgaaagtgcttatctttccactattcaaatcggtaaaatcgagaaataccaaagaatttcgataatcaccgactgtgagctataccccccataaaatatgagagattttttgtgatctcaatcgcttaattatcctttcatcccagcaatctgcgattcgaccgtcaacacttgcatgagtccgctggcacactcggatcccttgttgccagctttgccacccgcccgagcgagcgcctgctcagtgttgtcagtagtcaacaccccaaacatgactggtacgggaccgtttagcgtgagcgacgacaatccggttgtagctgcttgacacacataatcaaaatgagccgtctcaccacgaatcactgcgcccagggcaataatgccgtcaacctgattggaatctcccaacaatttgacctctcgaggaatctcgatggctccaggaacgtggacgatcgtgatggcggcatcaggaattccaagcagcgctaactgcgaaaggcagccttccaagagccgactggtcaccaattcgttaaattgggcaacgacaatcccaattcgcttgtgctgactgattaactttcctgtaaaattattcattagtttccgacctcactcaataaatgatttagttttgttttcttcgtcaataagtagttcttattttctggggtaaggcccacctccagtgacacccgctcagtggtttgaataccatattctgctaactggtgaatcttatccggattatttgtcatcagccgaaccttggaaacacccttgcgcttcaaaatggcagcggcaatttcataattacgattatcaatgggaagccccaagtgttgattcgcctgaacagtatcaagcccttgctcttgaagagcgtaggcctttaacttgttagccaggccaattccccgaccctcctgacgcagatataggacggcaccacggccgttgcgttgaatcctgcgtagcgcttcttggagctgaggcccacaatcacaacgcttcgatccaagaatgtcgccggttaagcactcgctgtgcagccgtgtcaataacggctcatcccccgctaagtgacctttggaaattaatagtgtcggctcactatcatccccagtatcaaaggcttccagagtaaaatccccgtagcgggtcggcaagctaacagtcgtgatactttgaatcggttgtgcgtcccgataacggcggtaggcaataatttcgtcaatcgtcagtagcgtcaggtggttgccttccgcgatggctttcaaatcctttcgccgggccattttgccgttctttttcaaaatttcacagatataggccaccggggaagccccggccaacctggccaaatccaccgctgcttcggtgtgcccctgccgttcatagatgccgttctttcgggctatcaacggaaagatgtggccggggtgatagaagtcatcccaggtgctggtgccatttgccaactgatgaatggtatctgctcggtcgaaggctgaaatgccggtggaggttgttttggcatccaaagtagtcgtgaatgccgtcccaaaggcatcactggaatccggaatcatcagccccaggtttaagcgtttggcaacctcggcccccatcggcacgcagagcagcccgcgggctttggtaaccatctgattaacatttttagcgctcaccttttctgccagcccgatcacgtcgccctcagcttcccgatcaaccgaatcggcaacaataattaacttgccggcttttaattcagccaatgccctttcaactcttttaattatctgctcattcataatttgccaatcctttctgtgccagattcaccacgtatttgcccaaaatgtcggtttccacgttcacctgatcgccaatggcaacctgccccaacgacgtgtggatcattgtataaggaatcaaagctacctcaaaggttgtcagagtggtggtaacgacggttaaactaatgccgttaaggcaaactgaacccttctcaacgatgtagggctgatacttctgatcaatcaaaaatgtcaatctctgagaatcatcgtccggtttacgggccagtagagtggcggtcgtatccacgtgcccgaggacaaagtgtccatccagacgatcagaggctgccagcgctggttcgagatttaccgaatctccaaccattaaatccttaaaattcgttcgcagcatcgtctccggcatgacatcggcaacaaagccatcgggctcaaatgctgaaatggtcaagcagacaccgtttacggcaacgctgtctcccaaggaaaacgcggactgacgtattaatttagtttgaatcgcgagtttagcttggtgattggccctttggatgcgggcaacccgcccctgatcctgaacaattcctgtaaacattagtcatccctcctggccgttagtttaatatcatcgccaagtctctgaatagtcggcgatgtaaaacgaagcatatgagcattaccaaggccagtcactgccgacagccccgtgccaccaatcattaatggtgtaatgtaggccactagcttgtccactaagcccgccgcaacaaaggccgcttgaacatggctgccaccttccaccaataatgattggatcccctggtcacttagcagcttaacaaccgctgccggtgaccaatcaggtgcctcgaacgccttcacaaattcaggtagtgcaaacgttggctggtgactggtcaaaatccacacgggttcagaactttgaaataatttagcgtttaaatcaagatgtcgagcatcccgaatcaagataattcgcagcggctgggtctcatctctcgccgatctgattgtcaatcggggatcgtcaacgcgataggtccgctctcccactagaattgcctggttcagttgacgcagtcgctgactatcttgccatgcctcgtcgcccgacaaccgtgtccggttattgcccgcctgattaattttgccgtcaagggacatcgcgtacttcaatgtcaccattggccgtttgcgacggtaataaaagttgtacgcttcgttaaccatttcggtgtcatccaagttatcaacgaccacgccatgcttggttagtcggtcaatccccttgccaccaacaattggattaggatctgcctgcccaataaccacccgggaaaaccccaaggctaccaatcggtcggcgcatggcggtgtcttcccatagtggctgcaaggctccaacgtcacgtaaatcgtggcgcccttggcatctgtcaggctattcaaatgggatatggcatcaatttcggcatgcggttcaccaaatcgatgatggtatccacgtgccaaaattcggccatccttcacgatgacggcaccaacccggggattggtccaagtcgctcccagccccttccaggcttcagtaactgctagctgcatataatcttgatcattcaatcttactcaccccacgaaaaaagccccgcaacaattgcgaggcattaattagataagctaaataagatttcatacgagtcttggagaactgactgattggtaacgaagaagacaacctaaaaaggcgacttccaattgctcaccaaaccatctcagttctcaccgatgttttgaaatgcttactttttcttctcccatccagactttactgtcggtcccagactcacactgggtcaaccgcttaacgcgggtcacggacttcgatttaaaaatcgtcaccgtcggtcgggaattgcaccctgccccgaagaaatctattcagttttcagaattatcatacatcattggtgaactggtgacaatcattaatcagcgatcaaattgaatccatttacggagtaatgtcgataacccttggcggaacaagggttatcgacattgggaaagtcattaaaatttgggaactaaatgacattccacccagaccaatgacggtgatgacggtaaatgttaaaaccaattttgtaaaaaagcgacatcctcgtcttgttttaatcatctttacacctacatttggattgaacggatatttataaaccagtattgccgtacctctgttggtaatcggcattactggttggctcccgttttacaagctaagtgcgactctaaacagtgcttaaaagctatctcaattattgactgagattctcaaaagaactataccttttatgaatgggtctaaagtgttcaacttaattaataatctgaggggaattgatactaatgagattcaagaaaccgtttaataacatttttaaggagatcagcgactatcaggtgaccgcggatcgtatcagtagttgggcttttgacatttttcttgttctgttttttagtattgctgtcaataccaccctttcattgcttgagtattggatcggccttatgttcacatttgtattaatatggctgtttcgccctaaatcccgaattaataaagagattttgaagctctttaataggcataacaactaccaagcgaagtgaaccctgctgtctggagatcgtaatacgtacatatgtttaataaaaagttggtgtaactgattaccacgcaaagcgagaactgcagacaaagtcaacaagagcttatttatatccttgtaaaaatctttcttcgaatttttttggcgatagtgtttacataatttttagcgagcctttttggtgtatcccctttgatcatttgtttcgatcccacaaaccaactgccccgattgcaatcgctaaaaccatcagcacaactataatcggaaataaaaaataatttcctgagatcacctgctgaataccggggatcaaattgacaacgaatagcactgccgcaagaattattaacacggaatggcgatgtgtaaacaagcagacaattccaccaactacgttcattccaccggcaaatatcagccaataaacagcggccatgctcttggatattggtaacggccccagcgaaaagatgctgagaaagatcgcaataccgccaattagaatgaacaataagccaatcaaaatctgtgatatcttcctgctactcgtttccatgttattctcccccaacagataaatgtgttaccagaactgcatctaactcataattcagttatatcgctaatccgtcaaaaaacaagctcgaagaatggaacatcacttttgaacttcaggtctctttctacaattccaatcaaaaagactttgttactgaacgctaatcagttcagtaacaaagcctttttaaatgtcatcattaatgatgcggatactgatgcccaatctcataaaccatctcaggctcctggctgatccgggtgttccggttcaacccatccacctgtttcatttcaataaggaccattgaataccgtaaatgccgcattctgtttaatccgttttaatgagctatcttgaagataactgccccacttaaaagccttttccgttcaagtcgataaatattagatcatctcaaaagtatcggtaagtagctgtagccgtatggaatatcaagatagtatgaacttcaaatagtaccacatgtttcattccaagccggttatatgcatacttatcttgaattgtatagatatttgcatccattgccttacttagtcctgtatcatggactggattacatttaatagcataactgggatgcccagataaaaacattgtcatcctaaccgtatttgcaggagaaatagataaaagaatcatagaagttaggacagtgaaaacgataattgaagtaatcatttttattctcttcttcaatgttttaaaacttaatctcatcatttaaatccccattcttataactcgatatttactaatcctagcactggcccctgccttaactaaaggcttaaacaatacattcctatcatgagaagtataataaaccatatgctttgttacttttgaaattgtgacagtgtggaaccacgagttatgtttttcgctagttcgtcccaaaaattgaacaacatccccgactcttacgtgagccataactcttctcaaggagtgtgtaacaaaatgtggacgcttcttaacgtgagtaaagtaatgccaaaatccaccaactgtcgtccaacttgttgaatacgccttatgctttattagctgtcccctttttcgataaactccagcataccattttttaggattcttgcaccgatatccgtgaacaatatgataagtttctttgccgcgtgatgtcttattatatccaccaacatgcgctagctgagaactccaattagtacaatctccaccgcctgcataatggaagtctggatactgagcgctgtaatatttataataagctttcatatacccaacctcacgacgctgacccttatcaagtctttgacctttcttccacgtcgttttataaggtcttgctttcttacgattttcaggactaaattggccgggctgcgttaccttagtcgatctaactgattcaacctggctatgttcatctggcttaactgctgccccactcttttgcgatgtgggggtacttgactgagacgactggcctgctttgtcattatttggacttggttgttcaaccgagttctgactaccttgcttcgtcatatttgtgctggaactggtagttgcattaggagccttagaagcaggcgagttcgaattattgggatttatggcaaccgtagctgacgcgccaccatttccactcttggccccagctgtggcaccaccggcagatattcctccatcgccattattattgacgctacccccactggtgtttccaccaggaatgtagcctccgccgccatgattgttattattgttgttatcgtcattaccgttgtcattgtcgttgttgccatcatcattggtttgattctgactgttagtgacattattgaattgactctggtcatgagcggacgcaccagttgtcccaatcaacaacaccgacattaccgaaatacccactaaacttaaagctctatacaaatatttgtacttgataggcttcatcatcattatccccctctagatcaacttaaagcaagtttctgatggttgagataatctcacagattgaattaacaattgcggtcccctgccccacaatattcgaaaaagcacccgtgatatcatagattgcttggcctttatttgcagagatttgcgattgggtcagctgtggttgcaattgaatattttgattttgtgcatcctgattggcttgggcctctgccggcgtgatcgttggctgagcctgagtggtattttgttgtgcggtagtattattggcattcactggggaagtggtatcggcttgcgttgaattggtgctgtcatcctgattgctggtatttgacttgttagcggactgattagctgactttccctttttcgtattattaacaacctgtttgcgaatcacctgttgtttaaccgtcttagtgccccgtctggtcttcttaactttggtattggtcttagtttctctgtactccgttgaacgggaaactgtctttttggctttaggtgttgctgtttggctaactgcctccgcctttagactggcggtatcattgctcgatgacacattggcagttgagttagcactttgagaaccattggatgcctgggcatcatcattgacagccgtctgactttcggcaggcttctgaaccgaagtttgagcaagcggttgattatctgtgttgaccgtcgccgcatgaacccccaaccgatccccctaataatgttccagctaccgaaagtgcgattaacatgttacgtgcaaccatattcatggttaattcccccaaattattaattttgttaccaggtaacatttgttgtacccatttctggttatagcactttacaaatatattacaatgactttgtgtaatatataacgacatgttggattctgtcagattttttcttctatatatgcgacaggacagccaaactaaataaatattttaaatgtttttattcacaattttgtccaaaaaataattgacaagttaaataattagaactaatctcactttaggtactaaaaagttaccaacagggggaattgttatgaatcgatttacaaaattgcttatatctttgctttcagtcatgcttatgaccatctgcttgggggaatcaacgattgcaagtgccaactcaaaagttcaggatggtgtacctcccgtattgcagggaaaatactgggccgttactatcaggggtagtaagaatgttcagcccacccatgaatacttttatacgactaaagacggctttgtcgcaaaacatacaaaggatggcaactttactgctaaatggatgatttaccgccaaatggaagataacgattacatattgaacggctcggataccaaggatctttcaatggcctattggatattcattgagcccaataaaaattggacaaagattaagattggttatacccatcttccgattaatcaaagcctcaaacattacccttcttactactgtcgcagcacagccaccagagtctcaaaggtcactgcaatcttacattaaattccaaattaaactaaaaagtgccaagccgacgaactcaattaacccgagttcgtcagtttggcgctttattcattctaagatattaatgatgcggatactgatgtccaatctcataaaccatctcaggctcctggctaatccgagtgttccggttcaacctatccacctgtttcatttcatcttcgctcagctcaaaatcatagatgtcagcgttctgcttgatccgttcaggatgaactgacttgggaatgaatgaatctcctcgttggaaatgccagcgcaaaatgacctgggcagctgatttaccgtgctggttggcaattctgacaatcactggatcatcaaaaatccggccgcgacccaacggtgcccatgcttgagtgacaatgtgattttcacggtcaaaatcaatcatagcctgctgtgagaggtatggatgaacttccaattggttgacgactggcatttcattagctttggttgccaaatactgcagatgcagcatgccatagttgctagtgccaatcgacttgaccaacccctgctctttaaggctttcaaatgcccgccaggtttcaaagaagtgggtgtgaatcggccagtgaaccagtagtaggtccacgtaatccaactgcagtttcttcaatgattcttcgactgaagcaatggtctgatcatatccttgattctcttcagcaaccttggttgtgacaaaaatgtcatcccgggcaacatccaagtctttgatggctttgccaaccgcagcttcgttgccgtacatttgagcggtatcaaacaaccggtaaccatcatcatatgcggatttaaccgacttaattaattcatcttcatcagtcatccgataaacacccagtccttcttggggcatcgtatgaccgtctgctaatttgattctactgccaatattctctttactcatcaaaatcctccagtattaattaagatgttttaagattctggctggattgccgccaatcaggacgttgtcaccaaacgattttgtaaccaccgctccggctgccaccacaacgttatctcctaatgtgactcctggaacgattgtcgtgttgccgccaacccagagattatctcctattgtaacattcccaggatattcataattggcgatccgttccttggctccaagcggatgattgacagaataaatcgaagtgttcggtcccagcatggcgttcttaccaattgtaatcttaccaacgtcgataaacgtacaaccgtaattggcaaaaaagttctccccgactgaaacagtgtaaccataatcacattgaaagggggattgaatatccaccttttcaccagtttgatgaaaaatttgcttaatcaattggctcccttgctcaggatcttggcgggcaacccggttaaatttatctaccagcaatcggttacggtgccggtccgccgccaattcgtcatccgtattcaggtaccgttctccagctagcattttctctttttcactgcgcatcatcaatttcctcctatatataaccgctatgtacaaaacgaggtcgaggcaaacgcaaatttgtctcaacctcattttagttttatgaagtcccgtccgaagcctctcggaggctttgttggtggactttatgttgagtaatctctcggggttactcgggtggtagtagttttaggctacctagtcgaaacgtgttccctggggcaacaacccacacctaagccaactttgggagaaatcaagatttcccccaaagccgacttaggcaccggttgttaaccgccccagctcacactctgctgaaatgtgttccgtgagccagatgctaacttctaagtgcactttaattaaagtcccaaacccagggacttcaatcaaagtacccttcgaaaacgcctcacccgttgctcttcacactctattacttaatatcctcaaatggtaaaccaaacatttgggcaagatcttgaatttgtgtttcacttgctgagaatgtcaaaaccgtgtggtgtccgccaccatcatggatccattgggtagcaccggcctttaagccgacctttggagtccacatttgcttagcaactggcagatgtggtgtttccttaggtgctttgttaccttcaacggcataaccaatcatgcggtattcattaccaaagtctgaaatcgtgatgtccattgcgtcaccggcacggcctgagaataccaaacgtgcaggatctgctttaccaccaatgtccaatggatgaacttcaacacgaggcttgtcactggcaataccagggtcaacttcgagcatatgtgatccaaggatagcttcttgacccttttgtaattcaagagtgtagtcttccatgaatgcagtagcctgattatgagtcatgattttaactaagcggtcaagggcagatgtcttccagtcaccttcagcaccgaagccatagccatcagccatgagcaattgagctgccaggccaggtaattgttccaaaccataaaggtcttcgaagttggttgtgaatgctgaatagttacctttgtccaagaagttcttgattccgaagtattcacggatttggtaacgaactgagtgctcgtacttgtccttgtcattgtcgccttgaacaaattcgtacttgtcttgtaattccttgtacttagcatcaatatcactttcagaaacagcgttaactgattctaccaagtcgccaagtgcgtagtaatcaacggtccagccaaattggatttgggcttcaactttgtcaccttcagtaacagcaacattacgcatgttatcaccgaagcgggcaactttgatcttgaagctttcgtcataagcgacagcaacattttcccagtcagcaatttcgtcttgaacttctggatcaccccagtagccgtaaacgatcttgttgttcttacgaagacgagcattgataaagccgtattcacggtcaccatgagcactttggttaaggttcatgtagtcaaaatcaatggtgtcatatggaatgtgatccaagtattgagttgccaagtggagtaatggcttttgaagtaacttagtaccacggatccagttcttagctggtgagaatgtgtgcatccaagtgataattccggctactttatcattgtagttaacatctttcattaattgagtgatgctgtctgcagtggttgcaaccatcttgaacacgattgggtaaggtaatttgccagaagcatttaacttatcaaccatgtctcgtgcatctttttcaacggatttcagttgttcttctccgtaaagatgttgactaccagtaacaaaccaaaattcataatcaggtacttgtaacatagttttctctcctcttgatgatttattatttttagacaaaatgtctaaaattggttaactattttgtaacgtttgacgcaacgtcttctccggcagccttatgaaggtcaagttcgatctcttcaagtgacttaccacgagtttcaaggaacttgctgtggcatacccaaatggcaattccacagataactgcgtagaacaggaaggcattgtccaagccccatgagctaagcatcattgggaaggtcaatgaaacgaccatatcagctgcccagttggttgctgaacaaagtgatgttcccaacccacgaatgttcaatgggaagacttcaccaatcagaacccaggtaactggtgcccaagttgttgcataaaaggcaatgtaaacggtcagtgccaaggcactcacaatagcggcaacgtgtgatccattatcaaacttgaggacagcatacataacgaccagtgaaaggcccattcctgcagcaccaaactcaagcatcttcttacgatcaactttatccatcagtaacatagcaacaacagttacgataacgttaacaacaccgattccgatatgggcaagtaatgcggcgataactccccagccaacatcagtaaagatggttggcgcatagaagataacactgttactaccaataacctgctggaagatggcaacgccaagtccagtaatcaatgcaggacgaacacccttaccaaataattctttccagccgccaactggtgctttggcagtttcttcaatttcagtaagagcaacatcaacggctttggcatcatgcttgttggtgtccatcaggacttcgcgagcttcgtcagtcttaccaatcttaactaagaatcgaggactttccggaaggaaaagggctccgaagaaaagaatgaaggcaggcaatgcagcgaatcctaacatccaacgccagccggtatacagatgagcaaatgagtagttcaagatgtatgccaacaagataccaatcataatcatcagctggaacattgtagcaaccgcaccatgcatgctctttggtgccaattcatgcaagtaagctggaatcaatgctgatgtaataccaacaccaatacctaataccacacgggtagaaacaagtacccagaagtcaggcgcaaatcctgatgttaaagctccaatgaagaagataactgaagcccagatcaataatttacgacgtccataagtatccaagaacttacttgttgccaaagcaccgataatcgcaccgattaatacggaactaacaacccaaccttgttgccatggtcctaagtgaagttgcttttcaataaacagaatcgcaccagaaactgacgcaatatcgtaaccgaagagcaaaccacctaaggctccaaacgtatatataaagccattatttgtgacctttttcaaaacgagcaccccattcgtattttattaaaccaattattgcaaaaactttgtgcgcacctgtaaacggtttctgacatcgcttacaaaaagagtataaaatatttatacgcataaatcaagatatattttatttgttagcacaaaatttttctggaaaataaaacacggacgggaaatccgccgtgcatcacctcctttcaagcgaagtgatcttggaatttattttctaaaagccggattaaatgcttttagtggaggctcgaacaatcagatccgagtctaaaatttttgaactgccatccttgccatccaacatatctaataatagttgggcagccgtgtggcccatttttcgtttgggatgatccatcgtggtcagcgttggatcaatatactgagaaatttgataatcatcaaatcccgctaccgagatttgatctggaacttgaataccctctttgcttaacatcccaatgacttcaattgccaattggtcgttatagcagacaatcgccgtcggcagggcattcatctcaacctggacccgggtcttgatcttatccaagacgtcatgaatgtcatcgctggaacgatacatcatgatatcgcctgaagttgagacgttgggatgggtctggtaggacttgatgaagccgttcattcgatggacgccttggagatcatcaacttgaaagacccccaaaacccgttcatgaccatgatccaacaaatagtcgaccaaagtcttttcggcatccgtatcgttggtttcaacgtatgggaaattcagttgtggataatgagcgttaatgaacaccgccggcttgccggaatcgacaatcatctggtagacatcgaggttcgggttgtccagggtacttctggttggttcaataatgaagccaaccacatcattgtccagcatattcaataagttatggcgttctttttcatattcatcatgggtattcccaatgagaatcgacaagccttcatcagagatcacctggtcgatgccgctgatgatgcttgggaaaatataattggcaatgtgggttgtgaccacgccgacgttttgattggatcggtcagaagagaccttattgttgatccagtcgttcacgtacatcccgccgccttgaacccgataaatatatccttcatgttccaaatcaccgacagcacggcggaccgtgtagcggctgaccttatacattgccatcaactcggactcggtagggattttatcgttaatcttgtatttcccgttaatgatgtgtgatttaatgttcttcttgaccatgacgtactttgtttccatgatgagatccccccgcgttcaaattgataagtgttctacgttaacattaacaagccaaaagtaatgaagacacaaacgattgcccagataccaaaatggtgattgggcttcgtctgatcttttctggcgaattcatacattgccataaagataaaagcaataattaataaatcggtaatccccgataaaacatacaaaattgtcgtcataatataacctctcgaatttaaataaaatactccagtaataaaagtatcatactttgagtaaaatttatatagaattatacggataaattaaaaaattggtattgcatcaccgtacaaaaacatattataatacagataaaagcggtttcacgaccgtaatttattttcgtaaggagaaagatgctatgaataccaagaaagaattgttcgataagttagatggtcaagacattgaaaagttcaccattaccaacgatcacaacgtttctgtttcagcaattacctttggggcaaccttggaagaattcaacgttcccggacccgacggcaaaccaaccaatattttggtcagcgtgcccagcagtgaagaattgatgaagaatcaatacttctgccaggcaatcggtcgaactgccggccgaatcaccaacggtactttcaagatcaagggtcaggaataccacgttgattcaaacgaaggcaccacgactttgcatggtggcccccacgggttcaacacccaaatctgggacggatcatttgatggtgacaccatcgtcttcaccaagcatatcgactcttctgaggattcattccccggcaacatcgacgtcaagattactttctcactcaataacgataatgaattaaccgctacttacagtgccaagagtgacgccgacactttgttcaacccaacccagcatatgtacttcaacttgagtgaaggtgacagcattaacggccaatcacttcaaatcaacgccgacaagtaccttgaattgaacaaggacaagacaccaaccggtaagaaagtcgccgtggatgacaccccatacgacttccgcgataaccaaaacctcaaggtcggtatcgccgacatgaaggccgaagttggtcacagttatgatgaagtctttgaaatcaatgaccatcaagacgacgaaccggtcgcaaccttatccgatcccgaaagcggccgcagcgtttcgatcagttccaagcgaaatgcattggttgtcttcacaccggatgatctaaccggcaccaactatctccgcggaaaaggcggcccatacatggcaattgctttggaagcccaaaacttgccagacacccctaaccacgcagacttcggtgatgtcatattgccagctggtgaggaaaagacctacagcattaagtacaaggttgaattctagacccatcattaatcaaacatttctcaaacaactcaaagagctccaggtaagaacgaaactgtccttatctggagctctttattgatggaaaaattcacttgttatccaattgtacttagcgactgttgcttctcatattcacgatcaaattttacgagataaatcacactagcgaccagaatgacgccaaagacgccgataatcaccaaccagttcgttgcatcaggtactgcacccgaggcaatatcaggttgccaatcaatcaagaagtgcagggcaatcggccagatcaaagtattggtcgtcacgcgaatcacaaccaacaagaggcctagcacgactgtgtaaacgacttgctgaaccacgccttcgatgttgtcctgactcatattcatcatgtgcaggccgccaaacaccagtgaggaatagatggcagctttggtgaatttcagggaacgccggtggttcttggcgttttgtaggaaggcagaaaacaccaatcctcggaccagactttcttcaaagaatccggctgtcagagcaatcagagtgttaaccacaacgtgtcgggtcgtcaaagtggtgacgacggtcgctggcaactcttccagtaacagcatcccgatcaccgtggcggcaaaaattgcgaaccacaccttcaaattagtggttaatttcaaccgggtggttgttaccttatacgttcccacctccaggtacacgaaggcaaaaacaatcaaaccatataccagttggatcgttgaaaagacaattggtgcggtatgttgaaatgccagcatctcaatgacgtagacaatcaggaagaaaatcgccatcacgatttgttcaatccatgagcggcggcttttgataatcaataaaatcactactttctcaaaaaatgttgactacctgccaaaatgtttaaaggtatcagcaggcagcccggtgtaacagaatctgccaccgttgcgcatgctgagttccccctcgccttgcatgccataattagtaattacgcaattttctttcgtgatttttatttttattcaaaaacccaaaaaatctccccaagctaaaggacttcctttaacttgaagagaatttcattgcaatgtttgaaacaatcaactgaactatgagccttaaagcgctgcagccacatcccggaccattgccaactcttcattagctggaatcaagagaattctggctgatgaatctttggtgcctaagtcgccgggcttttgctgctcgttgaggtcgccgtccaatttgatgccaaaaatttccagcttcttaacaacctgttcacgaacccatttgtcatgctcaccaatcccaccagagaagacgatggcatcgacaccaccgagttcagtaatgtagctggcagcatacttaaccgttcggttgacaaacatatccaacgctaatttggcacggtcatcatcggagtcttccaaatcacgcatgtcagaggaaactccggagacgcccagtaggccagagcgtttgttaaacatgtcgatgacttcttcagcactagcccccattttcttcataaagaaaggtaccaaggctgggtcgacatcccccgaacgagttcccatcacaaggccattcatcggtgtgaaccccattgaagtatcgtaacacttgccatctttttcagcagcgacagaggcccctgagcccaaatgaagggtcactaatttagcgtggtcattgcccaacgccttctcagcttcttgtgtaatgaagccatggttaatcccatgttcaccgtagcgacgaatggtaaatttctgggtcagttcatagggaatcccgtaaatcgaattgacttccggaacatctttaaagaaggcactgtcaaaaattgcgtactgatcagtgtccggcaaaattctgcggataatttcaatgtattcagcttcgactggattatgaatcggcgcaatatcgcccaactcaacaatttgtgacaaactatcatcgtcgattttgacgactttatcaaagatgtcacttccagccacaactcggttaccgattgcgtcaatatcccgtaaatgatcgatgacgccaagatctttaagattgttcaacataatccccgccgaacgctcgtaatcaatcttatcttcttcggctttatagacttcaccgtcgccatacttgattttgactttggagccgggcatgttcaaccgctcaacctcaccgtcagcgagcaccttttcttggggcatttcaaacaatttgaattttaatgatgaacttcctgcgttgacaatcagaactttggacataatcagtacctccgttgtttttattggatatttccattcgaaatgaaaacgtaaccacaactaaaagtatactatttgttaggagtttgtgacaatattagctattttaattttccaaaatcattaccaaactgggtgaatcatcgcgcaaccaaaaaagcgccaatccatttcaccgcaaccggcaggaacgaattggcgcttcaattcaattattcatcagtatctgaaaattcacgttgatactcggcgattccttcatattctttagaaagatcgcgactgagccgcagataaatcggcattagagtccgataacgtttaaagacgtcctcgtttggttcatacacggtttccttgcccatatacttcttaatgtcttcaaggttgtcttccaatcccaaagccattttggcgagaaacatcgctgccaaactaccactctcgtaagattcaggaatgacaatattgtgctcgaagatatcggccatcatctgggtccaaagagttgaccgcgcgaatccgccggcagccaaaactgccttgggttcgccggtaacttctttcagtgccaaggtaactgagtacagattgtacataatgccttccataacggcacgaatcatgtgggcgcgggtatgtttgcggttaaggccgaagaacgacccgcgggcattggcatcccataatggggcacgttcaccgccaaggtatggatggaaaattaagccatcagagccagctggcaccgtggcagcaatctttgaaagcatgtcgtaagagtcgatgtgcagcagttttgctgcttcaacttcaccgccaaacagtgaatcatgggcccagttgagaacaatgccgccattgttgatcggcccgccaactagatatttacccttcatgactggatagcagtacaaacgggctttgggatccactcgcggtttatcgacgaaggtccgaacggcagccgaagttccgatgttgattgccaggacgccggtttgaatcgcgccgacaccaatcgttgataatgcgccatcagtagcgcccatgacaaagtagacatccttgtcaatgccaatcactttggcatactctgacttaattccttggaatttatcggtcgtatccaccaactcaggcagttgtctttcagtgaggccggtttctttgagtgcttcctcgtcccattgggcagaattcatgttcaataggccggttgcggcagccattgagacttcttctttgagcaccccggtatacttccagatgatatattctttgatgcccacccaataggcggcctggtcaaagatttccggtcgttcatttttaaaataaagcaatttgtagaagggtcccatcgggtggattggcaaaccggttcgtttgtacatttccatcccgcggccattctgcttgtattccgccgcatacttctgggaacggttgtcagcccacgtcaacgacctggtcagcggcttaaagtccttatccaaggcaattagactgtgctgttgggcagaccaggaaatggcaatcactttgccatccgttatgttggcttttgccaccacttcctgcatggcagaaaccgtcgcgttgaaaatctcatccggatcttcttcggccatatcaggggtgtcttgataaagcggatagcccttattggccttgccataaatattgccgtcggtatcataaatcagcgctttggtgctggtcgtcccaacgtcaattccaataatataatccatcatcacattctccgtttcaggttctcgggttgtcatttatataaccggaacgcgttaatcgtccaagttatgagtcaactcacgtcccggacgtttgccggcaacaattgccttaacatcgctgacacatttttcgcccatgccgtgaagacattcataagtataagcagaagtatgtggcgtaaccaggatccggtcgttcttcaagaatggatggtctgccttaacgggctcaacttccattgcatcggcagcgtagccggagagctgacccgacttgatggcggcgctgatggcgtcttcttcaaccagggcaccacgggcattgttacagatgtaagcacccttcttgaggctcttgatggtcttggagttaatcatatgaaggctggtgtcatccaaagaagcattcaatgaaatataatcacagcggctaagcaaagtttcaaggtcaacgcgttcaacgttgttgttggtaaaccattccggttcagttgccggatgtggatcgttgaccaagactggtccgccaaaaatactgaacaattcagcaactcggctgccgatgttaccacagccaatcacaccaaatgtcttaccactgaattcgttacccatgaattgggcacggtcttcataacggccggcacgttcgcgttctgatgaaggaacaacttggcgaaccaaggccatcaaattggcaagctcgttttcagcaacggagtttcgttcaaccttttgtgggacgatggcaacttgggtgccatgttctttggcagcgtgtaaatccacgttgttaaagccgattccgtgacgggaaattaacaaaagttcatctttgttatcgaagaattctttgttaaagaacggggtcacactggcaataatgacgttaaagccgtgaagcttttcagctaataatttaccatcaatgtcggttggcagcatgaaccgcttaacagtcccaatgccttccaattctttccaatgctctgtgaagacctgaccgaaactatttgaattaacaactgcgatattgtattccatgatgttctctccttaattttaaatcataattgttggtgcactaacatactagttctgcgatttggttaatcttgatcaaagaaatggaactgatcgtgggcattattatatgaaatatcttctacaatcttgcccaagtaatcttcatcatcaggtgcttggccacgttcagcccactcaccaatgacattacataagacgcggcggaagtactcgtgacgtggatatgacaggaaactccgggaatcggtcagcatgccgacgaagttaggcagaagactttcttcagccatgattgtcaactgtttcttcatcccgctgaaggtgtcgttaaaccaccaggcagctcccaactgcagcttttgaacgccgtcctgttggaaatcacccattccggttgctaattccatccagtcatttggattcaatgagtaaatgatcatcttagggatttggtcctcttcctgcgcatccatcaagagtttcatgaattcctgggccaaatcaggctgggttcccatggaatcaaagcccccatcagtcccaaagctcttcagcattggcttgttagcgtttcggatgacattcatgtggaactgcatcgtccagttgaattccttgttcagatgcatcagggcttcaaccaacatggtttgatactggtcaatttcagtcttggtgagttgcttattattgcgggctttgtcgatgatctcgttcatttcatcgtctgaagcctttacaaagtggaagaagttgagtccgtggtctgacaatcggccgcccaggctttcaaagtactggaaccgttgccgaagggcgccaaccaggctcttaaatgacgtaatctttttgccggaaacttttgcaagttgatccagatagtcgccgtaaccgtcgtcagtcaagttgaatgccttgtccggacgcattgccggcaatactttgaagccattttggtcctcttcttttttgagcaacttgtggtacttcaaatcagaagcggggtcatcggtggtgcaaacaacttgaacgtttgagcgtttaatcaaattgcgtggtttaaaatcatcggtggctaacagctggttggccttttcccaaatagcaggcgctgtcttggtattaaagacatcattaatcccaaagaaacggcgcagttcgagatgagtccactcgaacagtggattgccgagggctttttcaatcgtgccggcccaggcaaggaacttctggtaatcatcaccgtcaccggtaatcaaatcttctggcacaccatttgcgcgcattaaccgccacttataatggtcgccgaagttgccttcgttaatccaaattcgactgatgttcttgtaattcttgttttcatagatttcctttggatccaaatgacaatggaaatcgatgatcggcattttttcagcatgatcatggaacagctttttggccattggcgtggtcaataagaaatcatcattcaataatgacatggtttgtctccttagttaatttgtttagcgtactttgataacgtgtcttcaagcgtcttgcgaacagcaccaaccccgctgatttgtgaagtgaagtagccttccacaacgtcgcccaggccaatttcgtacaagtcatgaccgaaaatcttctgattggataagatatctttcaggtgggcatgaacgtcggtcttttcgccgagcttaatgtcttggacctttggttgaagttctgacaagagtggatcgcggcttggttcaaatggtttaccttggtcgtcaatggccatcaggtaacgacaccaggttgcgagaactaacggaatgaagtggaggtctttgggatcacgtttgggatcatcaatgtaatgctggatggtgacaccataacggattgacagcttctgtgacgtgtcggcggcgattcgctgcggcatatccggaatgtatgggttaggcagccgcttgttgaccaactggtcgataaaggtcttggggttgataaccttaggatccttaacaaccggcagcccctcaacgtaaccaatttgtttgatcaggttcagcatgtctggatcgctgacttctttggcaattgagtcaaagccaagtaggctgccgttcacagccaacgcggtgtgcaatggattcaaacaggtggtaactttcatttcatcggcatcattgacggtgtcacgatcagtcagggtgacaccagcgactttgtccaaggctggccggccatttggaaagtcgtcttcaatcaccagataatgaacttcttcagtgttggtgaaggcagcgatattggtgtggccaggggtatggaaaatttgatagtcttcaaagccgtcagccttgagcttttctgaaacggcttctgaaggattaggcgtaattcggtcgatcattgacaatgggaagctaaccttgtgatcgtcttttaaataatcaacgaaggcttcaggcaccaacccgttttcctcccagccttcagcgatagtcaaaacacttttttcaagcttttcaccattttgagagaagttatcagtgctcagtaaggccattgggtatttgccggctttaaagcgggcaaacatcaatgcagtcagggaagccatgttattcttgggggcctctggaccgttcttgatatcatcttcgatggctggcaataagttacccttgctgtcccacaagttgtaccctttttcagtaattgagaaagtcgccaattgaagagcaggattttcaaaaatcttgaatagtttgttccagccatcgggattgctttggtcaaagaacaacgcatcggcaactgaagcaaataattctttttcaaagttcccatcctcgtgggtgatcacccggagaattttatcgttaaattttttataggcgtcttggacaacgtctttgtcatgcgtttcagcaacgaccacgccggcatccaaatcaccggattcaagcagtcgatcggcaatagcagcgtggaaagctcggaacaagttaccgccaccgaagtgaacccattttgtggcgcccgttttttgtttaatatcataagttggaaccttaattccagcgtcagcaaactcttgttgattgttcaggtaatcgtcagtaatttttaccattaattaaacctcctgtattgcgttgcgtgagccaaacatgaacgtatgccagctggcttaaaataaactagtacaccagtccgttgaatacgctttcggttttattatattctgatatatcagattgtcaataccccagttttttcaaggatcttcgttaactttttcaccaaaatatgctaatatgatgatatctaaaggagacttattatgttggataatatgcgcagtgacgcttacaatgaaattaaatatcgcatcatccacttcgactacgtaccgggacagaagatttccgaaaagctgatctcccaagagttaaatcttggccgaaccccagtcagggaagccatcatccgtattgaacgtgaaggtttgatcgaagtgatacctcagagtggcacctacatcactaaaattgatatggcagatgccaaaaatgcccgctttgttcgtagctgcattgagcccaagattatggtggacgccgctgtcaatatttctgatgaggccatcgccactattcagaaaaatttagatcagcaacagcagaccgccctcaagaatgagccggataacttctttgatctggaccaggaatttcatcacgcgttctataaagtagttgataaggatacggtttggaactggctgcagattaataacacccagctcaaccgattccgccgactacggttgaaggaaactgaattggattgggatacgttaaccaaccaacataccgcaatttttaatgccgttaagaataaggatatcgacgatttgagcttcctggttacccagcatttgcatttgatgctgctggagaagcaaaaggttgtcgatgcgtatccggattatttcaaaaattagtgtgcgacgagacccggttagggaccggagtacaaagagaatcagaccatgatgaacgttctttgttcatcgtggtctgattctttttgtacagtaggtccctgggtcgtcggagcatagctcaaaagcagaagggacttgtaattgtcatgacacctccatacatatgacaggatgtccgttgtggaaaatgcggtatagcacgttggaaatcaaagaaagactgttatgaaacaaacttattagtgtgcgacgagcaacgggtgatgcggtttctaagagggctttgattaaaacccctgtttctggggatttaatcaaagccctcttagaagttagcatcagttgcgtcggagcatagctcgaaagccgaagggacctgtcaattccataacccctccctacctatgacaggatattccttggaaaaagatcgacataaacatgattgaaaccaaagagaatcagaccgtgatgaacgttttattcatcgtggtctgattcttttgtacagtaggtccctaggtcgtcggagaatagctcaaaaacagaaagcccagtaacttccaccccaaaacagcctcccaccaggtgaaattattaaaagtcgatggcattgcgccaactgcaaagaacatccgcaatgggaaatatcccctcatcgcccatttctacgccatttcacgtgaccaaccatccaaaaattctcaacggctaatcagctggttgagaactgatgatggccaaactttaatcaatcgaaccggatatgtgggcctcaagtgagtgatacgctataatcaataattgaagggggattatcatgcacaagaaattcacgctggccatcctggctgccgggctgctgactgggtcaattgtttcaattcagtccgcaccgaccgccagtgccaagaccaaaattaccactaacaaaacatttaaaaagacatcatttttgaccaacactccaaaatctgtctatgtctggaatgggagttacaccaagaagctcgccaatctgaagaactacccgcacaccaatctttattcgacaaagcgggtcacaattcgcacgagtagctattacggtagttattactatgtcaaaagtgccaaccataagatcaaaggttacgtttggcatgggagcttagttcccggctcctacattaaaggtggcggctatcgctatccaaccaaacatgttttaatgtcgagtaccccatacaataagaaagactggtccacttccagcgacattggtcaaactggacggatatttggcgtcatgaatgcgacttcgatgaaaccatacctcaaggtgccaaccaccagtcaacaaaagcaggtcatcaatttccttaaaaagaagaatcaaaacgttcccaagatgattgaaaaccgcgtttccagaggtgtccgcatctcaatgatgaaactatatattagcggccaagctgttgaactgccgatgattgaaacgtatccttatcattattggatggacgttaattcattctatccagttctccaactctccaaactgccaaatcgagcaaagccgatcaagacctacagcgatgccaagacggtcacaacggtctttggttctcggacctacgactttgaagatccaaccgcccaatccacctcgaatatggaggaaggccctatcactaaggtatatggcaacggctatggcccgaaccatgatctttccctggtggattgtcgggatcgcctacgttatgtcacaaccaaaaatatcatcagtatttccaacaaccagccaactttacgcgatggcatctggtacgtagcaccatcctaccaattcgtcagcattggcggtcatgagcagaaattacgaaatttgattgatacgtcaaagtcgactgattatcggtatgtgactccgaacggtttcacccaatacaagtacgagaacaacagttggaatcctaaatttggtctcagcttcgattttcaaaagaacggtgatgtgaaagtcaccatccatcagctatctggaacacttaaccatccaaaaaccgttggtgatccacaaacgatagccacgttaactggggcgaatgccgatgctgaaatgatgacttatttgaatcattcagctgggtggtatgaccagtacttacaatagaatccgatccaaaaacaagcgctcagaatttaatctgggcgcttgtttgctttcaattataaaaatgagttacttggcagcagctgtgttatctgcttctttagcagcggcagctttgctagcttcgtcaccattaatcatgttgtatttcttttcataatggatcattgtaaatccagcaagaccgaagattgcaacgataccaacgaatccccacattgtcatcttgatagtacttgggaggaccaacaatggtgtgaacattgctaaaattccacaaaggaaacgtgaaaccccattgataaatccttggatacttgcacgaatttcttcagggaatgattcctgtgtccaaactttgtaaatagcttcaccggagagcatacttccaacaccccaaacgagcatgaaggcaacgatcaaggcaatcgaagtggctccaaagattgccagaccacccattgcgatcagtgcaaagataacgccaagggtgaaccaagtatttcgttttgcggaaccagcaatcgttacgtagaagcctaagataaacagcgcagcgatgtgcagtcccaaaccaataccagtcgataatgtctgtgaggcaccggctttaacgaacatgaaggttgtgaattgaccgaacgtgttggcaacaaagttccagaaaatgtagtagatagcaattgcagcaaataatcggatgtaaatcttgcttcgtgaacttctaaagagtacctgaataactgaagctttttcggttggcttttcgtccagttgtgcttctttggcagctaatcgttctgcagcttctttgtggagaacacgaattcctttggtgaatgtccgccatacccaaagaatcaaagcagtgatggcgaagaagccaaacacaattcgtccaccagtaacactcatcgtagaaacaacgaaggcagcaccagttgaaacaaattgaccaacttgccagaaaatttgagttgaagcaaccatttcagaagccatcttctggttaggtgcatccctggaaatcaccgtcaacgatacgggcaggtcagttccagaagcaaccccacaaatcacaactcccgcaagcagcatgagatacccgtttgcgaagacacaaataccggcaccaattgcataaaggaaattcacccaatcaaagattgccacaatcccgactttatcggcaaatcgactcccaaaaattgatccaaaagcaatggcaaaggttaacgcaccggaaataatcccgacttgaccattggttaaattcagtcccatctgccagacggtaatcgtacttgccaaaccaacaataattcctgaaccaagcatcgaccccagaccagccgagacactcaagttccaatatcttcctagatttttcataatcctgttctccttatcgtccattccaaggacgcatcaaaatatttaacttacaacaatattagttggtacgatatgagatttgataattgccggatcctaaaacaatctgaccagccttcgtaagcatcccctccaaatcagttccattacgatcttgaatcgtcattaaatgactaccatcaggcaacatcactgttccctttgcattcattggaacgtggacagtgacaatctgttcatcggttcccactgttagagtggccttaataatcccttttgctgatggcgtttcaacgctcacacggtggaggctgcccggccgaattttgacactaaagttttcgaatcccggcttggttgggttgattcccataatcccttgcacgatcgtcaatcctggggtcgctccccacggatgagacatcgtcatattaggtttatagtgattgctccaagcttcaggggcaatcgtcgccttcaaagtattcaagatggccgcaaacgtcttttgatctttacggtcgtctgggttagttaggagacgcaccgcctcatcggcatgaccgctgtcgattaaacctttgagcataaagtaaatgaagtagatgctgccaacaaatttgccatcattagcgacaaatcggctcatcttatcggccatctgctgatcggcataaacgccatagcacagtgcataagctgttgcgtgatgagatgtatgcttattaatcgaaaggtctttattcatcgagtcgtagaaacgaccagtttcggggtcatacattcgattaattaattcctttttaatgcgagcagcccgacttcggtaatggtcggcatctgtgtgatgcccaacaacgtcggcaattttactcatgctcagataagcgccatagaaaattgcgttgaatggtgtattgtactcaccttcgacaaaaccatcgcgttcaggaatcggccaatcaatcaacccatcgttggtaacaaggccaacttcttcgtcaaagttgtcaacgcctttggtatttttcaaagatcctttaaagtcttgtgaagccccgtcaaaactttcctcgtttttgccgcgattaagcttgtaagtcaaatcagtatatcgattcttcaagaactcatcattaccggtgtagagataatcttgccaagccatttcaatactgtagagcttgtaatcttcgggccacgttggattatcaattaagtaatccatactatggcgattgagcgagtatttagatgaaacaacgaaactggtattgccgttgactaacagatcaccttcgtacggccgtcgctcacgggcttgggaatcaacgtaaacatcctggttagttgctttgatcgtatacttggacatctcatattcgcggttgagtaggtcattatcactgtcaaaggcggattcttgagattcaaatggttgctcaatcgcccatccattaatatcattttcatttaggttgccttggaagccaaccaattcaatatagcgaaagtttttaacctgaagagtagtgaattgattctgtcccttcacaaacgtccagttttcgacataatcgggaccggccgctagatgatgacgaacatgtccatcatcttgaagctgctcacccatcaaaatcgtgacccgttgattaagtggactttgaagattaaccttaagacttccaataatttcttttcccaagtcaaccaggtaatcctgatcacctaacttgatcacctttttacttggctcatgggtttcaaatcgccgggtattttcactacggtaaggaataaaaacttcctcatcggaaaccatcgattgtggattaacccatgctgccggccagttgtcatcgttatattcgacctccgaccagccttgtgggtagtagcacaaatcaacattttcagacaccatgccgaaatacaagctgcggattttgacaccataatcgccaaaggccgtgctaccgtctaaaacgtgccaatttttgtcggtcacgattatcttcttcttagtcccatctgttaggtagacttcgagtttgcaccagaaggcttttcgattcgacttggcagttgccatgacagaaatgacgttttcaccattgatcaattcttcagtgacatcgtatttgttatagtaaatcccagtcttgtcagttccttgataatggacttgacggtgagccgatccaacaccaacgttggtaccgttcaccagcaagtcaaacccttggataaacagtggctcattacccctggaaaatgcggtgataaccgccgtatcaacatctaccaggttaagatcaaagcgtggactacgaataaaaacaacgtttcctaacttgggcagttcattatccgacttaggcccacgatctgcccaaatcccatggatcggctctacttgaggcttatcagtactgatgaatttttcgggttgggaaaaatcactgatattgttgaaattatccttgatccgaacttgccaataatacagctccccagcatccaagacccgctcaatttgaggaattgcaacacccgtattttcggaggattgtacccagcccgtatcaaagatatattcttgattggccaattgatgaaggcgtttggaaatcaccacctgataggccgtttgttggctatttgaaatattgctgtgatcccaccagctgaatcttggggacttatcgacgttgtagggaaaccgtaataagttcacgttcaggtgagtaggaattaataattcttgttgattgttagtcatcaattattttcctctctaaaacttcatttatcgtcgggccaaaccttgtcataaggaacaccggttagatcagtaacagtctgagcaacctttggctcaacatctgcctttttaccaccatttcgaagcctggtaatctcttcaaggacaatttgatgtgtctgtttgttaagtttgaaggtcaaagcttccaacaatgccaggataatcagtccgccagtcccaaagagcaggatcgctgcaatggcgtgctgagcttgaggcgactggctggcggcattcttggcaaagccgttactgtccaaaataaatccaactgcaatcgttgcgactgcgacagttgatttacgagtgaagctcatgacagcggcaaagacaccggcacgtcgacgtttagtgacaatttcatccaagtcgggaatgaatggaaagacgttccacggtgtgaattccaaggttgcccgcccaatttgatagaacagtgaaatgaagaataaaatcaagatcacatggttggtgacgtgcagctggaatatcagatagtaacccacaagcatcaacagcattaacccgtaaccgacttcatacaagaacttcggtccgtatttgaccattccaaatccggcaacgattgtaacgaccaacccaattaatgacagtgatagcatgttggctgcaaccgttgctgagagtcccaaacaataaatgcagaagtaagcaaacacagtgttgaaggtatcttttccagtaaacgagaataaatagatcaacagatgctttctgaagctcttaattcgaagcgttgacccatagtcacacaggagtccccagaagcgatgaagcaatgagccttcattgactgaatctttctcaagctctgcgcgcatttgaggggtaactggcttttcccaagtaaccgcgtaacaaacgtaaacgccaatcgcaaaaataatcgcaaataacgttccgtttactaagaacgggatggggctatgctgacccatgatggcaaacaattgtcccggaataaaggttgccaagaaagttgctccagccgagatgaacattctagcagatgataatttggttcgctgattataatcatccgtcatttcatttggtaatgtttcataaggaatcatcatcgcactggaaatgacttcaaaaatcatataagtggcgaagtaataccaataattcatccctgcgatccacagcgtaatatagagcaacataagtggcgaaccgattagtaagaagaagtgccggcgaccaaatcgttgccccaacttcgtcttataaaaattatcggtcagactccccatcaataaactacagattgcgtcagctacccgggcggcaccaataattgaggccccttgaacggcagttaaattacaatacgatgtatagaaaaatagcatccacgcgccgatgatggtcatcgaaccaccaccgacaaaatcaacaatcccataaccaatcccacgccagacggtgatctttcgtggggtataaactttactttgttttgccattgcttaaatctcctattctgaattcgttaactaaacgaacctcgtaacctcctttgcaaaaatagttatctggtatatcaatctgatatatcaactgtattaaggttatcttgtgaacccagatcggtcaataaagcgtttacaatctctataataaaaatttggtatatcgggggtaagccttgatatgtagggaattattcgggatttgagaaattattcagttagcaacagatatgtacatttgatacataaactaggcagaaagcgatacgacttcacaatcttttttgactcttggacaatccgatctattttctgggtaaatgaaaagacggctgcttaacaccgttatttatttactaaaaaactagtaaatattggtaaatcaacggttaaacagacgtcttaattcgtaaaactatttagtttgaattttctttccgactggatccaggtgccattttgtagtaactgatatatttcttatagaaaaaggtccggtttttaatccctacctccttgataatcttggaaactggtagagtagttgacttaattaggatattagcgttgatcagccgctgctttgtgagaacatttgagaatgtatcacccacctctttcttaaacaggttactcaagtagtttcggttgtagtcgtacttcgcagataatttttcaagagaggtatccttataattaccgttaatttctttgagcatttggacagcaatctcctgagattttgacattggcttattcatatctactttgtagttgcgtaccagctgagcaatcagaatcgaaagataggagctgatgatggtatcggcaaagtcccgctgtaaatagtattcctcgatgatccgatccaaggtctcttgaacctcgctctcatcttcgtgcccaaagaccaagtaatgaatcggactgtcatcgccgattcgccgattcaataaaaattcgtacaaaacgcttttactacttcgcaggtcgcttaacaaatccaggttgatttccttgtcgcggaacaagacattaattaatagatcattggttcctagataaccaactgaatgtttgcaaccaacatcaaggagtaaaacatccccctgctccaagtgaatctgttgtccctcaacaacctcatcacaagaacctcggagcatatagttaatttccaaaaaagtatgggcatgagttgggtacggcgcataccgattatgcttactcacgtaaatgctcttgtttttgaacaaagcatcgctgatgatcggcgttttttcctgttcagataaggttgtatcatagacgtctattggcagatcattatgaaattccaggcttttcagctgttctttttccagctttgtcggcttcatgagtgtatttagaatggtatcaagcatattattcgttccccttcaggtgatattgctatcctatgataacgcattcaaaagaattaacatattgatattgtcgacgaacctctttcttatgtaaggagaaaatcgacatttattatataagtatcatatatacagcccggtctattaattatctgttttgaaaaggcaattgcaaaacgtgtcactttaattatgtatcatttgtacatctgtatttgaaaacaacattttttaatataatctattaaaaataacaaatgtttctcttgtctacatattggatgtgctattcaagccagctttttccgcttaaccaaataacgggtagtaatgtgcacaacccgcacattactacccgttattccgttcatgctttaatactgaattacctcagcctttgaggacagctcctacagccctgacccctaccgtgtaacacaaaaaagccaacgatggacaaagaacgtccatcattggcttttccgcgttacactccggggtcaacccgggcttagtcgctcacttattttttcatatccatcgcatggccaccgaatccgtgacgcaatgctgatacgactttacctgtgaatgtatcttgttccattgaacggttacgggcgaacaatgcgtccgtgataactggaactgggatgccttgtttgagggcttcttgaacagtccacttaccttcacctgatgagaacatcttgccgctgatttggtccaagttagcatcgttagcgaatgcttcttgtgccaattccatgagccagccacggataactgatccgttaacccaaactttggcaacggcttcgttgtcatagtcatatgggctgtggtccaagacgtcgtatccttcaccgatggcttccatcataccgtattcgataccgttatgaaccatcttcaagtagtgacctgaacctggcttgccagtgtaaaggtagccgtctttttgtgaaataccgtcaaataatggtttgatgtgctcgaaggcttcggcactggtaccaccgatcatgaagttaccaccgttgagggcaccgttcttaccgcctgaagtaccacagtcgaagaagttaatgtctttgtcttcggcaatcttaccgtgacgaattgaatcttgatagaatgagttaccaccatcgatcaggtagtcgccctttgaaagaaggccaaccagttcagtaacagttgagtcagttggcttgcctgctggaaccatgatccaaacagtgcgtggtgcgtccaacttgctgacaaggtcagcgttgcttgatgcaggagttgcgcctgcttcttgagctaatttgatgtttgcttcgtccaaatcaaatgcaacaacttcgttaccgttacggatcatgttcttaaccaggttaagacccatttttccgagaccaatcataccaatttgcataagtattgtacctctttcgtcttatatattagttagttacttgtctacgatgcttattatatattttgaaaagaattttcgcaagcattattgataattattttcaaaaagtgcgatattctttggaaatatcatgaaagccctttctaaacgccgacatattggggttcatcatgaaaatcatttttaacccggatgcccgttaaataacttcattgttgaaaatgttttacatatttgatttcaaccgccgccagatggcagtcccagtcagccccagcagtccgacaatcgtcagcaatgctccggctagtagtcctctgatgtgatagttaaaggcaatttggtgcttgccaggcgtcacacggacacccaccaagccgccagcaacctttttaatcggccgctggtgcccatcaactttggcctgccaacctttatcaaatggaatggttaacaccagtgtttgagctcgtttgccaaccgttacatgccccttaaaatgtgctccatgttcgttgagcaggcttgggttttgcaatttaaatttatggttgtcctgatagttttcaacctgcctaagcttggcgagatcgattccgccaaggtcgccggcaacgtggtgcagttccttggttgaatgaatcgtcagggttgaaatttgccccttttgcatgtaccccatcggaatcatttccgtccccaagccactatacaacttggaaagtttttggccgttgatatagaacgacacgtttatcaatctgacccgtggaatgtataagtagtgcggtccggttgtattggcccagaacttgactttatattcaaaatagtcgcgatgaacgaacttggcgctgctaatgatcgtcggcgcgtacacatactgacgttggtttcccgccgttgcttgaacaaaatcattcaagttgtcaaaggcttggccccgtttcaacttgaggtcttctatctgtcggttggccataaatcccagcccagacgtgcgttttctaaccgttaaatgattcccataacgccccaggacatcataatacttcagaccaaagaaatagttggtaatcgccgttccgcccaacatatcgatccggcgaatgttgcgggtcgaaaatcccaagtcgcctaaaacatggtgggtgtgggcattcaaagtggaactatacgaactgatgccatgatttcggtataggaatgaatcgttatacccgctatagggcaccttgaacaaatctcggaacggtttatcaataatcaagaaacgatagaagccatcatctgattgatatcgcttttcaacgctcccgattaatctggtggattgcgcgtaagtccgttcaaaagccttttggttgccaagcggcgcaccatcagtggcaatcataaagttcaagctcaactcaaatgccaagacgacacccaaaaagattcgactggtcccccgttgtctgccgacgccaatcatggcaatcgtcgtcagaaaaatcagtccgaccacaaaagcaaagatgatattacggacagacagttggggaatatcaaaacggaattccattaatttttgcccttcaatattggcaaaaatatacccaatcaaaatcgctgctccaaggccgaccgccgaacgaatcaacaacttctcttcggcaaacatcccctgcaggtaaccctcataagtcaccatgatgatcgcaaagctgaacagaaagaccattctaaacggaaaaccggccggctgctgcatcatatgccaaatggtatttaacggtaaaaaccacatgccaacaaagataccgccaatcaaaatgccggcagcctgcttatcgcgctgactaaccaacttggagaagaagtagacaatcgctccaatgataaacaacgacccggtgaagaaactgggattatgtaccagccggccggcaaaatcattgccaccgacgccgagattgaccggaaaactaaggccaaacgttcctttgaccagaaagttcgcggccagcaagtccttcttcccagtagccatcatcgcgatggcagtggggatcagaatcacggcaacactcatcccagctaacaatgaataccaaataaaccaactaatcttttgccaattggccttcaagttttggaaaaatggcaatgaatacggttggttctttttaagtaagtaggccatatacagaacattgaagatgcagatgatgtatcccatgtaaaagttggtgaaaataatcatgatcaaactaacaacatatagcgcaggcttcccatggtaatagagcttttccaatccatagaccatcaccggcagccagatcaaggcatccagccacatcagatcataaaagtacatggccacaaaaccgcacaagccgtatgccaggccgccatagacagccatcaagtcatagttttgatattttttagccaagaaaacactcatggaaatggaacacagaatcaatttaacccaaataatcaaatcaatggcgatcggcagctgagctgttccaaacagcatgatgattaaattaagtgggctcaacaaatagtaggcatagattggtaccaggctgtcaccaatcgacattaaaaaggaatacccagagaagctgaagtgggccagctggtgctttaattcagcgaagaactgcaggtattgcgtcgacaggtcactgaccagtagattgtggctgccaaacggggcaattccaatcaccacaaataaggcactgaccaacaaaattggaatcagcaccgccaaaatataaaacgatcgttttgtctgacgaccacgttgtgacagcatatccgtccacctcaaatttgattttcgatgcgccgaaaatcgatttcgaacttgaattcatttccaattataactgtttgcttggataaatctttcattagagggattgattttaggaactattaaaaaacgtcaatcttttgttacacttgacccccttaacctgtaacaaagcagccgattgcactgaatttgttctgtaatgcgggcaaattgacaaatatatccaataaattagccgcttttttcaaattagattaccgtaaccattgccgtcaccacgcgactcacacaaatacgaagaaagtgtgaaatttttcttaacatttatgaaacaatcctgatactggttggtagcattcatttcatataattgttcttgtaagtttttagaggaggactattcatgacattgaaatttaaaaaaatagccggcctattaatgggtgccctggcagcatttacttttgcgacaaacgcatcggctgccaagacaaagattgctgatgtttctcagtatcaaggaagcatcaattggagcaaagcctccaagcaattaaaatttgcgatcatccgggtccaacatggtgacaccggcgatgcagatttcagaatcgatactcaaaaagatatcaacgctaacggcgcatataaatataaagtaccatttggtcaatatggttacgcagagttcagcagcgtggccgatgccaaaaaagaagccaaggacttttacaagcgatcaagttccaaagcacgtttctacgttttggacaacgaacatcgaaaaggtaagggttcggaacaatcctacgtcaacgcttggctggcacagatgagaaagttaaccaataagcctttggtttactactcatatcaaaactacgtcaacgttcacaaaatcaactattccaagtttgatggatcatggattgcaaattattccgctaagccaaacgtttcaaccgacctttggcaatacacttcaaagggaagcttaagcggaatcagcggcaatgttgatttgagcaaggtcgtcgacagttcaactgttaattcctggctcaagacttcatcagcggatgcggctaagccaacctacttcacatcactgccaagtgataaagaagtcacagcttccaaaaacatctatcaatatcacgatgttaatttcaaaactcgggtttcaaagattactgctggcaagaagctttcagttaaatcaatcactcgttcaaacggcggcgcttatcgcttccaactcactaatggaaattacatcacagctaataaagcatacgtaactgactaatttaactaaacgacgaaatataaaggagtactcatcttgtcacacagtattattaaatcagctttaaaaccattattgttgctcgcagccttgttcgcattcgctgtatctgcttatacttcagctaatacagccagtgcaagctcttcagaccaatcatattcaaaggtcttgaaggttgccaagaaacatctcggtgccagctatgtttacggtgcagttggtcctactcactttgattgctcaggtttcaccaagtatgtttataagcactcaattcagaagtcaattccaagaactgcccaagcacaatacaatggtaccaagaaagtttcaaagagcaacattaaaaaaggtgatttagtatacttcggcggcagcaagcacagcatctcacacgttggtatgtacattggtaacggtaagatgatcgattcacaaaaccgcggtgtgattactgaaaaagtttactcaccatggtggcatgtggttggattttcacgcccagctactttgagttatgatgactagagtggaacaccaggcgttttgatcccagaatttaagcaaagaagcgagttattcctgtttttggaatggctcgcttctttgcttaaatggccgggatcagccgatcgttccacgttttggctagataacagtggaactcaataagggccgaggcacagctgacaaatagctatgtcttggcccatttttgttgtggtgtttggttgtgattgatgcttgaaagtaatttacttttctatagtgaaaacgtgctcccagagccagctttctccgcttagtccgataacggcagtcaacgcaaaaccagcgttgactgccgttatcacactaatgctcaaaagctaaccggctcttgtcgcactcttagaagctgaatttatcaaccacttcaaaagtaacattctcattagccttaagtaatttagcaactgggcaggtatccaatgcttcgtcgaccatttgttgtgcctgttcgttatctaattcatggaacagaatttgacagcgtaccacaaatttataaccggtggtatccttcaggttatcgactgcagtatgaataactgtatccggtttgagattatgtccccgctccactaaaccgatggttgcgttaaagcaggtactcaacgcaaagccgataaattgctcagggttggttcctggactgttaatcaatgaactgcttacgccaagagctaatccttcgttgccccggacgaaactttcaccaactaatccatgttcattaacaacttcagtatgataaagtgatccgtcaacagccatatataattcctcctatttaacaaatccaatccttcatccaacaacttaatgatatgtgatttaaatcggtaagtccatcaaacagcacttacaattgttaacgcttactatagtaattatttccccattcaggtcacttttttgatacactggacgttggcgcaaaaattcgaatgaaagaaggtcaactacatgcccgcaaaagaaatgaatttaaaatggctaatcatcggggccatgttcagtagtgtcgggatgagctttgtctggccgttaaccagtgtgtacctgcacgatcggctcggggtttcacttaccctgatcggtgttgtcctgttgtttaattcccttgccagtgtgcttggcagttaccttggcgggtacctatatgaccgcaagaacccctatcacctactgattggtggcgttgccgcaaccacgctgactttgattctgctggtctttttccatggttggccggcatttggaatcatcctatttttcaacgggatttccggtggctggaacgtggccgtggtcaactccattggaaccagtattcaatctcaagacagccgctatgtttttaacatgctatacttcgcccagaatttgggaatcgttatcgggacctctttggtcggcttcatctacagcatcagtgtaactttgatgttcgtcgtcgccacggccttgttcgtcgtcttcctgctcatcgttctgctcaaattcaaaccagctgccaacaaatcacgtaaaaaagtttccgacaccgaaaagaccacttggagctccaagaatttgccaaagcccaatgccattatgctgtttgcttttttcctgtcattattcattatttggatcatgtaccagcaatgggtttccaacctgtccgtctatatgaccggtatcggcatcccactgcgcaactacagcttcctgtggacgatcaacggtggcgtgattgtcatcagtcaaatcatcatcaattggatttcccgctaccatgaaaacatgatttttgaagtctttctcggcgttttcttgatgtcgatgtcgtttgtcgtgctgatttttgccaaaacctaccccttcttcgtgctggcaatggtcactttgacaattggcgaagccactgccctgccgactattccagcgttggttaacacgctgaccccggttgaggccaaaggacgttaccagggactgattcaatcctgggcctccgcaggccgggcattggggccgctgtttggtggtttgataattgagatgtcttcgtacaccgccctgtttatcatcgccaccagcgccgttttattagttctgatggggttaattgtcttgtggaacaccctgcacaaaaatctggtcatgtatcgatgagttttgaccaataatctggatgtataaaaaagagcttgctgacaatatcttgtcgcaagctctttttgatgcaaatttttaattatttttaccaagttgactatgacggattccataactgaagtaaagaaccagtccaaaggcgaaccagatgccagaagcaatccacgtctcagcctgcagttgtgacagcatcagcatgcacaacagaccggaaacgattggcaatactgggtaccatggcacttggtagccatgatggttttgaatttctttgttgcgtcgtaatggaataatcccaaatgaaacgaacagaaaggcaatcaacgtcccaatgttaaccaggttggtcagttgctccaacggcacgaagccgcccatgaaagcaatggtgattgtaatggtgatcatgctatttctgggactgccctttttatcaagcttgcccaggaattttggcaggagaccatctcgaccgatggaataaattaaccgtgatgaactatagatcatcgtgaccatcatggtgaacattccagccagggcaccaagggaaataatcccggcgacccagttcaaatggacaaattgcaatgcaaaggcaaccggatcagaaacgtttaacttggtgtaagaaaccatccctgtcagaacgattgacaccccgacataaaggatcgtggcaacaatcaatgtcccaataattccaatcggcatgttcttcttagggttcttcacttcagctgcggaactggaaaccgcgtcaaaaccaaggtaggcaaagaagacggcggctgctccaccaagcacaccaccgtgggcactatgccagccaaacggtaaaaatgggtgccaatttgatggcttaatgtagaataggccaaccacgatgaataacaggataatgccaattttaacaaccacgatgatgttgttgagccgaaccgatgaacgcatcccttggttcaacatccacgaaatcagcaccacaataatgatggcaatcagattcccatatgtcccctgacttgggacgaacggccccgagatcgcttttggaaagccgatgtgaaagcctgccaaaaacgactggaagtaggcaccccaagcactggaaaccgcagctacggctaagacatactccagaattaacgcccagccgaggatccagccaatgatttcaccaaagaccaggttcccataagaataggcacttccggcaaccggcagggccgaagcaaattctgcgtaacacatggcggcagttgaacagacaattgcagcaacgatgaatgaaataataataccaggaccggctttggttgcggcaaccgtcccgggaagaataaaaataccggtaccaatcacggcaccaatccccagggcaatcagatcaaaggctgacatggtcttaatgaatttcttgtcagtctcaagataacggtccaattgctctcggcgaaaaatacgagctaataatgacataaacgtgcctccacagttaaatgaattctcgattaaaatacttattctattttaacttttcaacctgcataaagtcaatttcattcccttgatgtaaccggtttatcgaaaaataattacatatttaatcgaaatcgccaaagaaccattcactgcgaaattattgtatccttgtactaaagagacttcgaggggggacgaatttgaaaaagaatcggctggaagcattcactgacgccattgtaccgattattatgaccgttctggttctggaattgaatccgccagaaaagctcagctggcatggattctggggaattcgcgaagaattgatgtcctatgccatttcattcttcttgctggcaatcgtctgggggaaccatcatcacatgttcttactggtcaaatcaattgacggatttgtgatttggtcaaacaccgttttattattcttcttatcctttgtgccgtttacgactgcaatcgttgacaatgatcccaacagcctgtttggctcccaactttacacgctgttattcatctgtattaacctttcgtggaacctattgcgggtcagtctggtgcgggccaacaagtcagtcaagccgctggtcgcatcgcttaaacgagatccaaaaagtatttacacgctggtcgcattcattgcggtctttctcatctcattttactggcacgaatttgggatgatcggaacgttcatcgtcatgttgctttgggtgatgccttatcggaagattgaggatgccgctaagcggatttgaacttgaatgtgctcgggtgactatttaaaacacagaaagagccaaggtaacgctgcttgttagcgataccttggcccttttttccacctcatggctacctatccgaatcgtggaataacaagcagcttccggccgtataaggggctcagccaaacatccaaaccctgggtatttggctgagccccttatactctggaagctaagcgcttattattccacactctgctttgtcagatccttcaattcaatattactatccataattccactctcaccactcaaaacaacttggttgttcttgtagtcgagtttcatatcttcatcgaggtaaatcttgctgtaacccttgaagtaccagtcgccggaattggctgacaatttggtgtcataatccggcaccttggcgtccttgtcaacggcaatcacgtcataactggtgtccaacgagcaaacgccaacttttgaaaatggaccaacgccatcgtcaaagctgagcaacagcttgctattggcaggaaagactttcttgagttgtgctaatgctgcatctgtaattgttaatttcattttctcacctctcctatcatcctaaactcctgagacaaaatgtcaattagattgtacacaatccttttaatttttcatcaacttcattacctgttatgatattgtcgaggtgattaaatgacaaatcaaatgaacgccgtcgtgattaacgattacggcgatcgagatcaactaactgaaactcaaatgccaattcctaacattaaagatgatcaactcttagtaaaagttgttagtatcggggtcaatccgattgactggaaaactcgtaaaggcctgaggaaagcacgctacccatttgattttccaattattttgggacaagaaatggctggtgtcgtctcaaaaatcggtgccaaggtgacgggtttcaaagtcggtgatgccgtgatcggttacggtacgcccagcaaccgcggaacctatgctgaattttatgcgattgacgcagatcaagccgcccacaaaccaattacggtctcctttcaagaagctgctgggctgggacttgccggcacaacggcttggcaggccttatttgatgccgggcacctcaaagttggccaaactgtcttaatactggccggctcaggcggtgtcggttccatggcaatccaactcgccaaacacatcggcgctcatgtcattacaaccacaagcgccgctaacgacaactatgtcagaggtctgggtgctgataaagtcattgattacaaaacacaggatttcgccaaagtctcgccagaagttgatttagtctttgacacattaggcggtcaaaaccaactggatgctttcaaagtcgtcaagcctggtgggcgcatcatttccattgttgaaaccactgatcaggcagaagaactcagtcaaaaatatggtgtgtcattcgaaaagatcaacgcccatcccgataaggacgtgatcaccactctaagcaataagctcggcgccggtaaactcaaagtatcgattgccacccagctcaagttcaatgccgaaaacgtccgcgaaatgcataagctcagtgaaactgggcatatagttggaaaattaatcttgaatgtttagtcccaatcagtgcgaagtcaaaacgatcaagccatcagtataaacaattgatgttttgccgatttgttcataaaaattagcaaaaaaagaaggtcaaccggatttctccagttgaccttctttattacggcacctaccaaagtagatggacttcttggattccacaatccgctaaagtcaaacaccagcaaatctgtgccttaaattgtgtcccgctcgaattcacattaatcgcttgcgcgacagcataaatgctgtgtgatttctcgactcatcgcatacaagtattatgccacgtttccatgaaaacatcaaggtatcttttatccgcctatttttcttcaggctgcttttcaaggttttctttgaccatatccaaatgctcagccacccagttgttcatctgatccaagtagttggcgacgttgcccacgtagtcatcggcactggcgacctcatcaatccgcaaactggatttattgacccatggtgaactgatcaccaggtacacattcaccggtaatgtctcttgatcctgcatcattttactgataactttggcatcttggaatggtaaattgatcaagttggtttccaaacgaatcgcaacatcttcatcggacgccttgacctcgccatatgcaagcttgcctaagttcagttgtccctcaacgtagtcatacaccggctgcatcactttggccggatctttcatgatgtcgtcgagcttcttggtgaaagatttgccttcaatcttttcattaaccaaatcatccacgaaacttgctgcatctttttccaaattagtcacctatcttcttaatcctttttgcttgttaatccgccgttgaaatgtatcgtgttgaagcgctgctctcaatctgaacgctaaaatataccaatagacgttgacgacaatcccaaatgcggcaaccgccgatacaaacagcttaaccagaatcgtcgcgtcactgttcaggaacatcgtcgaaatcatccccacgaagccgactgaataaatggcgatcaccactgccagcagataatagctgattttaacccgcagtgccgccaaaatcaacgtggccgcgtaaaaggcgatcgcaatccaagtcacctgcaatgcttctccagtggtggccggtgctttcagtgccatgaaaggcaatgtcatcaaccaagtcactgccaggaaaaccaccaacgagatgattgcccagaaaatggtctgcttttcttcttttttcatttaacgttttaccctccagaattccaacaaaaaaagataaattcgatgatggaatttatctttttattaccagttttagtgtaccttattaaagcggtttagaaaagcatatcaaagaaatcgtcacgagaaattccggtgaagtactggttcaaatcaacgtctttcaaggcatcttcgaagtctttacgttcgaaacgaacaccctttaatttgtcggcaacttcagttgaatcttgtgggccaaagtaatccccaaagaatttaacgttggataccttgccgtcatcaacttgcagacgggcatcaatggttccgttagtgaagtgttgacgcttcttaacggtgaattctggtgaattgccatatacccaatcccagttgttgtagtaatcatcaaaaatcttatcgatgcccttttgatcgtcatcggttaaatgatattccttgtccttgatctggtcgaggtcatccacgtggaacaactctttcagtaaacgatcacggaattcaggagtggttaagtcttgatacttcggtgacaagtatggtttcaagttggtaacccgtgagctgactgacttgattccctttgacttgatcttgtcttcaggaacgtccaaagcctttggaatgactgacaaatcaacatccagcatcaatgtaccatgggagaacgtcttgccgcccttggtgtacattgcattgccagagaatttcttgccgtcaaccaaaatgtcgttacgaccactaacttcaacggacttagcgcccatgtcgtgaagagcatcaacgattggttgaacgaatgacttgaagtcaccaaactcttcactgtcactgtcaaccacgaagctgaagcaaaggttgcctaaatcttggtagacagccccaccgccggaaagacgacgggtaacaacaattccgtgttcatcaacatattttttattaatttcttcaagagtgttttgattacggccaacgatgatacatggtccttcaatgtagaataaaagtaacggttcatcaaatttgatctcgttcatcaaatactgttcagtagccaaattgcgcctgatatcattggatttcatgacataatagtacataaaataacagcctcttttcatttagttgatcaacttgaatattagcacgttaggaaagcgattacaatcacaagcaaaaagttgaaaattttaattgattacaagcatcgaagagaatggtatagtttaggtaaggacaatacgaatacggggtgattgacatgcaacagcaaaaatatgaaaatgtcttggtaccggtagatggctcaaaagcaaccgaaaaagtgctgaatcgagcaattgaggtagctcgggacaacgatgcccatttggatatcttaaacattttggaagtaaaccaatttaaccaaacttatggaagtgctgtaagtggggacgttgttttcaagttaactgaaaatacggacgatcagctaaagaaatatcaaaagaaggctgaggacgccggcgtcaaaagcgtcgacatccacatccgatttggcaacccgaaaccaatcattgcacgtgaatttcctaaagaccacaataacgatgttatcgtgatcggctccaccggtctaagcgccgttgagcggttgattatcggctcggttaccagttatgtgacccgaaccgctaaatgcgatgttttgatcgttcgaccaaaagacaaagtaacaccaaacaaataacaagaacagcgtgtgggcggcggcaattatgtcgacgcctttttgctatcaacgattaaggacaatgaagatgaaagatattcagtggcgcttcaacgagaccgtaccggaagccatgaacggtcgccccttaaaggcgcttttaagtaattattggcagctgcccaagcatctagtttacagcatccgtcatgccgaacgggtgctggtagacggccattatcagccggttaattttcccgttaaagctggcagtcaggtccagctgacgtttgtgccggccgattttgccagaccatttccaaatgtcgcggctgattcagcggccacggttgcgattctctatgaggaccaaaatttaatcgtcatggataagcggcgtggcgataagacccatcccaaccaacctggtgaagttggggcgacgattaaccatttagcggcttatttggcaaccgaaaagaccgttccctacatgattcaccgattagatcaggagaccagtggggcgattattttcggcaaaaatccggtggttgtgccaattttggtggccaacatcgccaacaaacaaatcaaacggacttatttggcctgggttgagggaaccgacatacctgacgaaggcacaatcaatctgccaatcggccgtgacccagatgataaacgtaagcgaaaaatcaatgggcctcacgcggctcctgccttaactcgttatcgcgtactgcgcaaacagtccgggtacgcactcgtccagatttccctggaaaccgggagaactcatcagatccgggttcattttgccgcacttggtcaccctttagttggggatccgctgtataattcaagtaatggtagccctttcttgatgctgcattcttggaaggttgatttattaatgccattcactaaacaacgaaaattaattgaggcacccattccgagtcattttatcaagtttgagcaagaattatcccgtcgttaaccgtgccttagagaggagtcgaatatgacagaaacacatttatccagttactcggcaactgaattatcagaattaattcgccaagggaagttggaccgggtggcactggtccaagaactaatcgataccgtggagcagaacaatccaaagctcaacgcggtcactaccttatggggcgatcgcgctaaaaagatggccagtcaatttaatgataccggtcaaccatttgcaggggtgcccattttattaaagggccttggccaatcattcaagggcgaacctgataccggcagctcaatgctgctcaaggattacaaggcaaacattaccaacaacttcgttcaagctttcttgaaggccggcctcatcccagtcggtgaaaccaatgcgccagaatttgggttcaagaacgtcaccgactcaagattatatggtgatgctcacaacccgtggaataccgattatcaacccggcggctcctcaggtggttcggcagctgcagtcggcgctgattggctgccaatcgctggtggaaatgatggcggcggttcaattcgaatcccatcgtcattctccggcaccattggcctaaagccaacccgtggccgggtaccaaccggcccaggcgagtggcggggttggcaaggcgcatcaatcaactttgcgattacccgggatatgaatgacaccgcccgcttactggatgccatatcaacggtccaaatggccgccccattccaagttccacttccagcagcctctttcactgagaccttgaacagcctgcccaaaaccttgacaattgcttattccacagaatcgccagttgggacgccagtttccgacgaggccaaacaagcagttatggatgccgttcagtttttgacagatgaaggatacgatttgattccggcagacgcgcccatcgacggtgtcgggttaatgaaaagctactatttgatgaacgctggtgaaacagcaacgatgtttgccaacatgcatctcaaagatgacgtcattaaggaaaacgttgaaccgttaacctgggcgctcggttatgccgggcgagcagtgacggccgttcagtacagtcaagcactgactttttgggataatatcgtcagtgatatggatgccttccagcaggaatttgacctttacctgacgccaacgactgcccatcaagcaccccgaatcgatcaaccattagtctcagctgagaatttaactaaaatgaagcacattgaagaattaaatccagaagaacaaatgcagttgatttgggaccaatggctacctgccctgaccttgtcgccgttcactcaactggcgaacatcagcggccaaccagccatcagcctgccaacctatgtcggagaaaatggtctaccactgggaattcaattcatggccagaaaaggccgtgaagatctactcctgcagatgggcaaattcttcgaggataatcaacaatttcatttacttaaggactaaccagtttcacaacatttgaggaggagatcgcatgattaatattcgcaaactaatcggcttactgacaattaccgggacactcggtgttgtttcaatcacatcctcaaatccagtcctcgccaaacaaaatccaaaaaccaccgcagttaaaaaagcaaccacccagccggccaaccaaaacgccttagccaagggaaatgttcccaagctttggtcgcaaggttatcaaggccagggaatggtggttgcggtcatcgatagtggcgtgcagaataatcaggaatttcaattatctagtaacaccgcagccaaaatttccaaatcccaggcccaaaagtttatcgctcaaaggggttacggcaaatacatcagcccgaagatccccttcgcctacgattacgtcaacaataataacgatgacagttccgcagacagtgtttccggtttccatggtctaatggtcgccggcgttgccgcagcaaatggtgtcgcacgaaggaacaaagccaaatttgtccagggagtggctccggaagcccagattctcaatctgaaagtctacggtggtttctctgatgaatcaccaaacgacgttgcccgggcgatttatgacgcggttgatctcggggcagatgtgattaatatgtccctggggatcggcgtcggtaatgaatcactcgacgatcaggaacaagcggccgtaaaatatgcgaccgatcacggtgtctttgtggctgtcgccggcagcaactatgggcatgcgggcagtatcaccaccgattataatgagcaatccaattcaacgattacgacttatgaaccggctaactctggcaccatcagtgatcctgccatttcaccatttgccaccacggttggcgatgaaaacaccaagcagggtgacaaaagcgagatggattctttctcggcttggggaccgacaccggattttaagttaaaaccggacgtcagtgcacctgggcagcaaatcgccgttttagatcagaacaatcactttacgaccaacaccgggacctcatttgcctcgccatacattgccggttcggcagctctactcatgcagaaatttaaaaaatatcagccaacgttaaccggtgccaagctggttaaggccgtcaaagtggctctgatgaatgccgcccaaccaatggccaacgacaaattcaaaggggaactgatttcaccccggcttcaaggtgccggtcaggtgaatgtcaacaacgccgctaatctaaaggcatccgccaccgatccaagtggtaaccaaggatcaatttcactgaaaacagttggccaaacgaccaagttcaacgttgccctgaccaatcaaatttcagagccgttgacctaccatatcaacacgacaaatgggccgtttacagaaagccgaaaaaccaacaatcataatgttgggccggttcatgacactgcgatccctggggccacactgcaatccgccaatgataccgtcaccgttgaccccggcaaaacgcagctggttccttttaccctcgatttgggcagccaagctaatttgaacagcgtcgctgaaggttatctaacttttgaaaatgctgattcaaatcaaaatttgacagttccctatttcggctactatggcgatccaactgatgagcaggttgtcgataaacccgccaatcaggccgacagtattttcaacggcggctacctgatggacactcaggatatgccactgggattgagcgaccggacgtcgttggccagttggttgaacaccttgaaggatccggacgaactgcgagacgatatgccggaaaaaatccaatctgacaaagtggccttctcgccaaatggtgatggtcattcagatgccatcagtccctacgtgttcaccacccagaacctccaaaacgtcactgctgagattaccgatgccagtggcaaggtcatcagaaccgtcgacaatgaaaccaacacccagaaatcaattgaagaaggcggttccggctacattgacgatttaaccctttcaccttcgatgcgcttgaaccccaaagcattgaattggaatgggatgacttatgatcagtcaaccggtaagatggcggtggttccagatggtcagtaccactacgtcttacaaaccaccaatttcaacaatggcgccaagcagcagcaacaatacagtcttccggtcaaagtcgatacggtggcgccaaagattaccaaggcaacttatcgggacggccgactggcggtgaactactccgacgttggggttggcttcacttcaatatcaacacttgccgtccaaattggtcatcagtccgccggcgttagcctgaacaattctggtcaatcaaataccggcagcctggtctacaaactgtcggcgtccaagcaacacgccctcaagcaggccaaaggaaaactgaagatgacgttggccgacgttgccggtaaccaaaccaagtgttcgatcaaagtcagtccaaagacgtataaccacgttcaaacgtcatcaacccctggttccaagcttgtctggacattgaaaactgacgatctggaatcaacgatgagtcacgataagtatgcggtgaccacccgtttttcaccaactaagggcattacatttaaagggttaaaggacaatgacttcaccttaatcaacgcagccagcaaagtgtatgatccgcagacccatcaactagcgattgccgggaaagtggctaacccgaagtcgaggttaaccattttacgaagccccaaccaaaatgcgaaaattaaccaagtgaaaatttcaaaaactgggtccttcaaatttgagatgccaattaatccaacgacccagcaagggatcggctacatcctaaaagtacccaagaagcatcagtggacgacagccaaagggactcttgtggttattaccgacacaaccgcccctacgctgaatttatcgatgcctgacaatgtttccgaaacctcacagaaccactatcaattgacaacttcgaatgatcaattcaccatcagtgggactgtgaatgataacgttgatggttatcgcctcttgatcaatggcaacaatcttttccatgagcaaaataacgcgggttgggtgaatcaccaagatttaggtgccaatcccaatccccacggtcctcatcaattcactcagacctttaacctgaatcagggaacaaatatcttccaggtttctgccgttgatgaaaccggtaatcaaatcacaaaaacaattaccgtcacccgcgagtaattctcaaatatatatatgtatcaaaaaaggagcccgaaatcatttctgatttcgagctcctttaaggttttagtaggcattaagtcgtaatgaaattacttcttaaggccttcccacttccagtcaacaacttctggaagatcagtaccttcttgacggatgtaagcattgtgcttatcaaccatgtcgttcatacgttggatgaagtaaccacccttaacagtgtaagctggaatatcttgaacagcttcctttgcaaggtcgaaacgatccaattggttcaagacacgcatgtcgaatggtgtagtgatatcaccattttcacggtagccatgaacgtgaaggttatggttgtgacgatcgaagaagatatccttgataaggtcttcgaagccatggaatgcgaagataactggcttgtcagtagtgaacaagttgtcaaattcttcatcactcaaaccacgagggtcaaccttaggtgaacgaagcttcaagagatcaacaacgttgatgaaacgaatcttcatttctgggaattccttgttcaagattgagatagcagccaatgcttccaagttaggttctgagcctgcggcagcaaagacaacatctggttcttgaccttggtcagttgatgcccaatcgatgtagccaagaccattcttaacgaggttttgagcttcatccattgtgtaccattgacgacgtgggtgctttgaagtaacgattaagttaatcttctcgtaagttctgaatgcaacatcaccaacagctaacaattcgttagcatcagctgggagatactcacggatgaattcaggcttcttctcagctaagtgagttaacatacctggatcttggtgggtataaccattgtgatcttgctggaatactgttgaagtatcaacaaagttcaatgaaggatattgctttctccagtattgttctgaagctttacgtaaccacttgaagtgttgagtcaacattgagtcaactactcgtccgaatgattcgtaagtagcaaagaatccatgacgaccagtcaatacataaccttcaagccaaccttctgcttggtgttctgaaagttgtgaatcgataacacggccgtggtttgaaagatcttcatcaaatggttcgtgaatgtcttccatccattgacgcttagagtcatcaagcaagctgtaaagacggtttgacttagtttcgtcaggaccgaatccacggaagctggtagggttaagttctgcaaccttttccaaccagtttgaccattcaatcatatcttgcttctgagttacaccacgatcgaatttaacttcgaagtcgcgaacatcagggagcttcaatggttctggcttgataccaccgttagtgattgggttaactgacatccgcttgtcgcccttaggtgcaacggcacggatttctggtttaacagtaccattttcatcaaataattcttcaggcttgtatgacttcaaccagtcaatcagcaagtctttatgttccattgaacctgcggcaacaggaattggaacttggtgagcacggaatgaaccttcgatagggttaccatcgagatccttcttaggaccagtccagcctttaggtgaacggaagataatcattggccagttaggtaacttaacgttatctggtgtttcgttttcacgagcattcttttgaattgacttaatctcttcaataacatggtcaagggtcttggcaaattcttcttcaaccttggcatggtctgtatcagcagttgcttcaacaaagtatggatcccagcccattcctttaaagtaactagttaagtcttcgtcactcatacgtgaaaggatagtagggtttgaaatcttgaaaccgttcatgttaatgataggaagaacagcaccatcggtaattgggttgatgaacttgtcagagaaccatgaagcagccaatgggccggtttctgattcaccatcaccaatttcaacagcagcgattacatctgggttgtctaagatagcaccggtaccatgtgaaagtgagtaaccaagttctccaccttcatggattgaacctggtgtctctggtgcggcatgagaagcaactccacctgggaatgagaattgcttgaataatttagccatacctttttcatcttggctgatgtttggatagatatctgagtagctaccgtcaagatatgagttggaaaccataacttggccaccatgacctgatccttcgatgtagaacatgttcaaatcgtatttgttgataacacggttcaattctgcatagataaggttttgtgatacgatagttccccagtgaccaataggcttaactttaacgtctttggcttcaagaggtcgcttaagtaatgggttgtcgcgcaagaacaactgacctactgaaaggtagttagcggcacgccagtacttgtcaacaagttccaaatattctttggaatcgtaatctactgtcattaattaacactccttcttcgatttagcaacaaacttctgtatagaatgtccgtaaaattcaccaactgtttcttgatcaatttacatcactaatactaaacgatattttcaaaaagtcaaccttttagaaaattgatacggtccaatatttagtgggcgaaaatcctatacttatgtgccattatggacgctaacaaatatttagtccactattattaatattttgtaacaaaattttcgaacattttactcaggcatttttccgtttgaaattaacgacaatttggacgataaacaatagaacaaaaatcgccgttgtgatccaaaatgtgaatcgcattccaaaaatgaatgttcctggttgggcaaccggataatcattggttgagtggccgagattcatactgataccagtaaatagtagaatgtttgcgaaaatcgctccaactgtcatcccagtattccgcgagaaccccagcagtccactggcaacgcccagctgatcttttgacaccgagttcataaccagcacgttggttggtgcttgaaacaggccgttgcccaagccaacaaaaccaagccagagacataagatcaatagaggtgttgtatggttaacgctcgccaaccccgcctgacttatgatgagcatcgccaaggaaatcgccgcaatccggtgtgatccgaatcggtcgctgagccacccggcaaacggtgagacgataatttgaatgatgggaaaactgatcaaaatcaagccggccaggtcggtggtgatgaatcgattttgctccaaatagattggttcgatgatgttgacgacaaaattaattccataaactaaaatcgtcgctaacaggctcagcgaaaagtcaatattgctgaataaatgaaaattcatgaccggatcggctgcccgtttttccagattaataaacatgatcagtaaaatgattgtcgcaatcatcaagctgagaaaaatcaaactcataaacccagcttgttgacctaagatgagtcccataaataaactgccggccataaaaatcaaaaccagcatcccccaagtgtcaattctaccggcagctgttgcttctgctttgggcagcacaatttggccaaggataattgccacaatccccaccggcacattgacccaaaagatgtagttccagggaagacaagtcagaatgagaccacccaaacccggaccggcgatactcccaagggcgaccaccgaaccaaagctgccaagtgccaagccccgctgttctttagaaaaggtctcggtgataatcccggcgttggtgctcaacgtcatgctggcacccaaagcttgaattgcccgcatgatcaagatccagacaaaccccagattgatgccgcagaatagggaagcgatagtaaaaatcacggtgccaatcttaaaaacccgggctttgcccaacacgtcacccaacttgccaaatggcaataagaacatgcacgtcacaattaggtaacttgaggccacccacgtcacttgggcagtcggcaccgccattgctcgggacatgaccggcaatgcaatgttgacgatgctgctggtgagtgtcgacatgaatgacaataagacgacggcggtgaaaatccaccattgattttgctgattgacttgcctagccatgctgcgtgcctcctccagaagattcaaagctttcatctataggataggctttttcagtggcgtggttggaaaatttgctcacaaaaatactgcaggaatcactgtgtgactcactgcagtagaataaaaatttaatgaaacatatgtgacataacttcggtgcccattggcgtggcaacaatcgccgcaaagatcagcagtaagatgccgatgaccatgaacacgccttttaccgagccgaaatgggctccgacgggccagatgctaacttctaagcgagctttggttcaaacccaagcccagggtttcaaccaaagctggcttagaaaccgcatctcccagcccttgtcgccctctactacttgtcctcatccaaattcacaaaggtattataattcaaatacttataatgaatgcgcatattggaaacttcaaacggcgtgccatcatccaagaagaaaataccttccatcacgccaactggttcgacgggcttcaagcccaacaactgctggtcttctttggtcgatggatccgctgtaatagtcataaatgacttggtgaccgagttgccggttgcgtcttcaaaatagttgaagattgagccctccactcgttcgctgttgagttccggcgccactcgaattgggatgtagccgagttcaatcatgaagggtttgtcgtcaaaggatcgcagccgcttaatttcgtacacaaattcacccggatttaaaaacaattcggtttgaagctcttcgcttgcgggaacgaccttaaaatccaacaacttaattttaggcgtctgaccgtcactcttaaagctgtcagtaacccccaggttggatccctcgtattgaaaaatcgtctgattcttctgatatagcgggttaataaaggttccagaaccccgctttttaaaaataatgccttggtttgccaaaacattcaacgcgcgtttaattgaactgcggctaacaccataggattcgctgaggcttcgttcatccggcagcttctttgaggcaaattcattggcctgaatgcgctccttcaaatccttcatgatattgcgatatactaaatcagccatttgtgctccttattaaatcgttaaattgatctattatcaataaagtataacagattatcatcttttgttcagacagaatcgttttgccgattgtgctaaaatatccctgaggtgttatcaaatgtcaaaaaagaagaaaaataaagttcataaaacattagtcgaacaaattctcgataagcacaaaattccctttgaacagatggaatttcccacccacaaagaaggcgacgtcgaacaaatcagcgtcgaccacgtggatactgacgagcaccagatttttaaaaccctggtcttctccggcaaaaccaccggcccagttgtcggtgtggttccagtcgacgaacacttggacgaaaaaaagctcgccaaagtttccggcaacaagaaagttaatttggtacctttaaaggacctgctgaagacgaccggctaccagcacggcgccaacacgccaatcgggatttgggaaaagttccactaccccatttatgtcgatcaagaagccaaagagatgggggaaatcatcgtctcatctgggcaaatcggccggtcggttaaggttgattcccagcagatggtcgacctgatcggcggcaaattcgccgacataaaggaatgattgaatgctcaaagatattctaacaaatattggtttggtactcggattaatgatcggagtaccatttctttttatctatctattgtcatccatcaaccacggcaccaagcaacggattgccaatcaatttggtattggcggacaaattggctttggctttctggggattattattcatgaagccagccacttattggtggcgttaatcttcggccatcatatcgaccagtttcgcctgttgcgagtgccgtcggcagacaacgacaccctgggatacgtccaccacacctggaacaaacgcaatctctaccaaaatatgggtaacctattcatcggcgtcgcgcccatctttggctgctgtttatctgtcctgctgctggcaaaatactttgtccccgaagtctaccaatcattgatgacaactgccgaacagccgctgagtcaactagtcgtggtactgccaacttttaactggctttcgatgggtctatttctaataattgctgccaacatctgtattggtggttttgatttaagccccgccgactttgaaaattccaagcagggattctggcaggcggtcatctgcttaaccttgttagccatcatcatctcgctcaccccgctacaagcgacgcttttcagcttactaatccgtttgacggtgattatcgtggtgatttcgctatttaatttactgatttcagtcgtgatgaacctgatttttcggtttatttagtgccattccattcgtcgacaaattcgcccacaaagtcttgcatgacctgttggcggtgttcggcgatttttttggcggttggcgtgttcatctgatctttgagtttgaataatttctcgtaaaaatggttaatgaccgtcccgcgcttacggtattcagccttatccattcccgtccgcggcataatccgtggattatacataatttcaccgaagtggccgccaaaataaaaggtccgggcaatcccaatcgcgccaattgcgtcaagacggtcggcatcctgaacgatctgcccttcaatcgacaagtggtggtgggtcttcagattggcactgtatgacatgttatcaatgatttcgaatacttgcttaacaaacgcctcatcataaccaacgccaatcaattcatcagcaattgccttgcgtttggcagccggattggtggtgactttatcatcgctaacatcatgcaggtaagccgcaatgattaccaatgactcatcagcatcctcaccttttaaaatcaacttggccaaactgaccacccgctcaatgtgcgtgtaatcgtggccagtggtttcgtacccgagctccttttgaacaaacccgcggatttgtcttagtccaataatcattcgaaaactccttttaaatatttatcaagatgctaaaaatcactcgaagaatcaaaatcccccagaataactgccaatagcgcagatatgtatgagtcaatgaggcgaaccaggtggcaaaaaatgtccaccagtggacccgactgcgattttggccataaaagtcgctaatttctgcaatcatcacgaaaagcaacaagtgcagcatcatcaacagaagtaagtcaatgacgtaggctgtcgccaaataccatcgaacaccgcttgaagcaatctgaaatgatgaagtaaccagggaacccagtccggcaacgtttagcgccccagccaaacttaaccaaacagatgagagaatgtaggtcggaatcagtgatagcaaaagcagcggcaggatcagccgggtatcactgaccagctcttgggcagttattgagggaatcgcaccgattaatgactgaatagatggcataacctgaatttcactagcaccaaattgaaaccgcgtacccaaaaagaagacgactgccgcaactgcccagacaatcacaaaaaaattcttccggtaggccgtcgcgatcgagaacagctgtgttttaagattggaacgagtattccccaatttgaaatccccctactttattcaaacaactattagtatacccttgcaccgtcaaagctgaaatagccgtgctagaaacggttattctctgctcaaccacaaaaagccgtcaatccgagaacgctcatggattgacggcttcattaagcatgtcactttattgaattgaatagactgactggcccttcaaggccgccttataagctgcaactgccaagttgacctggccgacgccatacaactgactagtggcatttttaatcgagccggttttgttcacatacgtcaacatagcatacaacggagttgccttttggccagcgtgcatagctgtgctgttaacatattttttcgtgcttgacccattcgccaaggcaatgatcgcctcagccgttgaattggcattgggggtggtcttgccgttaaatgtgtatccaaaagcaccattactttgtgccagactgtacaagaactgctggcctttcttgatgcttgattcaaccgagccggttgctgatttgcctcgtgatagtccagtcaaaaccatgctcgtcgtatcggcatccttggctccttgcgcgttgttgtaagtccagccattattgttcagttgaaccttaaccaaccgggaactcaagctggccttgctaaatttggcattgctgggacgtttgaaatgattgctcatcgatacggcaatcaaggtttcggcctgagaactggccgtctgcttggcaacgctgcttcgatacagtcgtgacaccaagtttatgcccgttttatggccatacggcttgtagttctgcgcgttcatccccatggcttggacggccatcacggcattggccaaagttgcggcggtgctattgctcttaataaccaaatttttccgcaggagattcttttcgcctgtggtaaattgataatgatttccctttaaccccagtaaaaagtcagaatacccagatgaggctccggtttctgagtacagtttccggctgaaaatcgagctggtcttaccagacaaccccgtcttgttttctttaagcatcttctttgcgtaagtgtatgtcagtgcagtccggcggtgaatcgttgatgtgctggccttatgaatagaggccgcaccggcgttggctgtcaaggtaacggtcatgaccactgcactaatcgaagctaaaatatttttcgttaattgattcattttgaatacctcttttatttattgtagttcagagaaatccggtcaccattggccaccacataggcaccaatcgatgtattgggctggttgccattaatcgagtaaagccagccggtcatcgtacctgcagggccggcgttatagccgttgatccctttcacatatgccgtgatgccggagccgaccgttgtgatcgacatgctgtgctgagaagccaacgcattcaaagcatccagcgcagtggcgcctttggaaagggtaatgctgccactggccagcactgatccgttggcattgacacttaccgtgaccgtttctgtgttggtattggtatccggatttgaattgtcgttagtggtcccggaagtgttggtcgacgaagagctagcattgttggacccagttggcgtcgtggttggcacacttggagtcggagtagtagttgtggtcgacgacgagctggatgttgaagtcgtcggtgatggcgtcgtggcaaccggcgttccagctgcatcggtattctggccgctggtcttggcaatcttggttgccagaaccaaccgtttattggctgacacgtaccgaccactggtgagttgcaatcgggacgtgtgcccatagtcgaccactttttcaacgtttaacgaccgattctttttaacgtgtttctttcgcccgcttagttgtcgattactgtattcattgatgccccttggattaagaaccttaatccgggtgactttggctgagtagtaggcgccggtcaaatatttcgaagccgaaagcatgtagccgatcttgcggctcttcagatctttaacccgataaatggcatgaccctgtttgttagtcgtctgcttgaggaccaaaaacattggtcgattaatgcgggcctgcttcttgtagattttagtcagctgacgcttattaaaatcggtactcttgtaaagcttaacggtcgttaaagcataaacaaccgatcccttggcactcttggccttcttggttgtggtcggtttagtgaccggtaccgcagatgatgaactggaagctactgaagaacttgatgaacttggtgcgctgttaataattgtcgtgtagttgttggtaatcgtcgtgccactgctggacgaagctgcacttgaatcaacgactttgacattgttaatttccgcaacaccaactgcccgatcggcaatcgctgcttcatcagttgtatcagcattaatcttggtaatgtagttctcaagcgtttggttaatcgtgctgatcgcagttgctttgtcggtagctgacgattgtgaatcattattgactgcttgccgtttagtcgttgcagccgcattaagttttgccagttcccgcgctctaaaggttggattttgggcaaaattaaagatccacccctggccgccgtctttggtaaatttcgcctgctccaacgtgtaagttgcctgctggagcagcatggagttactgtcagcactaatatctttctggtccaataaccgttgaaccggtgcttgataatcagatttgccgtttaatgacgtgtagacgtcaacgccggcaacagccagagcattgaccattgtgacgttattgtactgatcttccttattgctctgattcccaaagccgccattttgttgataatagtcattttcaatcacactaaccgctttttgaatggcggctgggacaccgggctgatccatattcatggaaagggactgaatcgcccgggcggtcaaatcaacgtttccccatgaagccgtccagatgccggatgctgaatcgcggtcttccaagatctgtttggtcaaagttgcccgcgccgtttcgctggctttaccataactgcaggtactcaatgcttcaagatcgttaaccaaggtgtacaaactcggtttggcaattttggccaatggatcattgataacttgacccacaaggtccttcttttcaacattagctgggtcgttgcccagtgctcttaagccaatgaccccggcaacatctgagacaccgctcggatcttgcacagttccgcttaagaatccattagtggtgatgatatcctgataagcattttgggcctgagcatcagtgatgccattatcactcgtcgccaaaatcatggcatcccaagcatccaaggtgtccttttgagcggtcagcttaacaccggtcgtaatcgccgaatcaacatcagcggcggtatcagcttgggcgaagttttcgccaccaacaaataccaggaacatcccgactaccagtgatacccaataaataaactgtttcttcttcatacctgtgcgctcctccaaatcatgaaatagtgatggtaccctcaacaaaaaaatgaacacaacaaaaaagcccggctagttagactagccagggccgtttctcaatcactaataacctaaattcagatattgaatcagagcacacaaaaatatccgagaaatacgctattaattgacaaagccgaccctaagaagctttgcaatcggcataacaaacgtatcctgacttgatctcgtcctacaactgtcctctttccagggtgtcccagtgagttgtgacagcttcgtcaatcttacagtagcgaaggggctgtaaaggattttcacctttttccgttttattatgcttcttaacatgaaaattatagcatggaatttgggtggatttagggtaattgagaaatttattgataatggtgctaattgtttcctggtttgggaaggtgacgctcctctttttttgctggagagatattggtttctgcgaggactgggttatttttgtggacagctacgcaaaccagcggaatctaaataagagaagagccccagccacgcgagtaatcgcgcaactggggttgttttccacggttaccaagttgagaatgctatttaattgtttgtttatttaaggattctcccagtttgagtctgcttttgaggacagctgcgcaaatcagcgatacctaaataagaaaagattcccagccacgcgagtaatcgcgcaactgggagtgttttccacgactgcaaagttaatgaggctacgtctctgcttgtcaatttaaggatttctccaggttcagtctgcctttgaggacagctccacaaaccagcagtatctaaataagaacaataccccagccacgcgagcaatcgcgcaactggggttgttttccacgactgcaaagttaatgaggctacgtctctgcttgtcaatttaaggatttctccaggttcagtctgcttttgaggacagctacgcaaaccagcagaatctaaataagcgaagagccccagccacgcgagtaatcgcgcaactggggttgttttccacgactgcaaagttaatgaggctacgtctctgcttgtcaatttaaggatttctccaggttcagtctgcctttgaggacagctccacaaaccagcagtatctaaataagaacaataccccagccacgcgagcaatcgcgcaactggggtattgttcttatttagatactgctaaacggtttgtttcgctcactacttctccacattagtcccctcataatcatcaatcatcaactgtttcaaatcggcaatcaaaggttccttagggttcgcagtcgtgcattggtcttcgtatgctaatactgcaagacggtcaactgctgcatcgaatttggccttgtcaacgccccaagccttcaagcttaaggtaacgccaacttcatgagccaacttgataattctttgaactaatccttcgattaactcatcgtcgttcttaccttggatcccaacgtatctggcaatttctgcgtagtccttgttggcacggaagtactcgtacttaggccatacggcaatcttttccggtaatttggcattgtatctgataacgtgtggcatcgtgattgcaatggcaattccgtgggttaagccgaattccccacccagtttgtgggcgattgaatggttaattcccaggaacgcgttaccaaatgccattccggctaaggttgcggcattatgcatttcttctttggcgtgcatgttgccattgtatgagtctgccaagttgtcaaataccagcttgatggcttgcagtgacaatggacgggtgtaatcagaagccatggttgaaacgaatgattcgattccgtggcataaagtatccaatccggaagccgcaatgttaccctttggaacagtttccacaaattgtgggtcaacaatcgctacatcaggtgtcaaagcatagtcagccaatgggtacttaacgtgggtctttgagtcagtgataacagcgaatggggttacttctgaaccagtaccggaagtcgttgggatagcgatcatttgtgccttcttaggcttgttgaaacggtatgcccgctttctgatatcgatgaacttctgcttggcgccgaagaaactcgtcttaggatcctcgtagaataaccacatgttcttggcagcatccaatggtgaaccaccacccaaggcgataattgtgtcaggcttgaatgcgttcatttgacgaacacccttttcaactgtgtcagtggttggatctggctcaacgcctgagaacagtgagtattcgattgggtttggacggcgtttcaattcatcaagcaccttgtcaacgtaaccgaattcaaccatttctggactggtaacgatgaataccttgttaatgccaggcatgtccatgaggtaacgaactgaagtcttttcaaagtaaacccgaggtaacttaatccattgcatattatttcgtctctttgcgatagttttgatgttcaaaaggtcatagtcggtaacgttatgagaaattgagttggcaccccatgagccagttcccaatgtcaatgatggggtcatttcgttataaaggttaccaattccaccgaagccgcctggtgtgttaaccagaacccgggctgctttcatctgcttaccaaattccaaggccaagtcgtcgtccagagtttggatgccggcagtatgccccattccaccgaagtgaagtaattcgtcacagagcttgaaaccttcttcatggttcttagctttgtaaatactgatcactgggctgagtttttcagctgaaagtgggtacttaggaccaacgccagtaatttcagcagccagaactttggtgttgtcaggaactttgattccagccagtttagcaatccctttagctgatttgccggcgattggacccttaacactgccagtcttagggttaaacattgcttcggctaatttgtcatggtccttcttatcaacaaagaagacaccgttcttaactaattccttcttaacttcagcgtagatatcagaatcgataaccgcactgttttcagtggcacagatcataccattatcaaaggtctttgagagcaccaagtcgttaacggcacgcaggatgttggcagtcttttcgatgtaaaccggaccgttaccaggaccaacacccaacgccggcttaccagttgagtaggcagctttaaccatgcctgggccaccagttgccaaggtacttgcgacaccagggtggttgattaatttcgttgtggcttcgatacttggttcttcaatccattgaatgcagccttcgggtgcgccggcagcaatcgcagcgtcgcgaacaatcttagcggctgcaattgatgacttcaatgcttgtgggtggaaactgaagatgattgggtttcgagtcttcattgaaataattgatttgaataaggtggttgaagttgggttggtaactggtgtaattccggccaggacacccaaaggttcagcgacggtgatcaattgacgttctttatcgtctttaatgacaccgaccgtcttgtggtcgcgaatgctgtgccaaacttcttcagtggcgtacatattcttgatggccttgtcttcagcaaccccacggccggtttcttcataagccatgagtgccaggtccatatgtttgtcttggccggccattaccatttggtgagtaatgtggtcaactttttcttggtcaaatgaatccataatttcgagtgctttttgcgcttttgataccaagccgttgatgacagtgtcaacatcagttgtgttcgtcttagctgctttggtttcttttactttattatcaatcattgattttcctccaatgaaaagtttataggttgtttgtgctttgttatctttttcacaatattaataatatcacggatttttgaaatgtaaacagttttgttcaaaaaatcacaatttattttttgtaagtgcttgcacactgatataacaatatccaaaacaaaaaggacttgttcagcaagtcctttttctatgaaagcggttccattatttatatgtgaatgatttcacgactttggctatttggtcacttttgtgagtggcttttgaataatcgccaaaagtttctcggattggattcggtcaataatgacattgacggccacctgcattaatttatcattcaaattcttttcttccaatgcccgactattccggctatccatgttcttgaatgagaacaagagccgtttgataaaggtgtcgtaagcctgctgcggataaatgttggccgtcacctgatcgatcccgtgacgaatcgtttccagggaaaaggctggcttcaataaactgatcaaaatcagatcggcaacctgcatggtctgatacttccgcttgaccggtgccatgatcgccttgttcttgacgtaattgttgatcattgccggagtgactttatcaattccgattggccccagcgtctcgttcaccagtgccacgagttgatccatgtacaattcaaatttgggtaaatctgcccacagcggcagttccacctgcttgagtttttgttcccactgctcgtattgttcttcattgtatgccatgttatcactccttcgagtttattataccacgttagctagtgtggggcactagataatctaacttggagtggagtaagaggcgctttgatctcagaatttaagccggcaaattaattattccagggtttggaataattggtttgccggcttaaatggcgggatcagccgattgctgcacgtttcagctagataacagtggtgctctacttaccctccgcttgtttgcgcagtcgtctcttctcccgcttatccaagacagtggcaataaccccctgcatgaacatgtagagcggataggccgttgcgataagtggaatggcatacagccaaatgtctttattaaagaaggagaccaacgagaaaatattattaaagaagatgatgatcgtcaaaaatgccaccagtaccaagatgtccatcccaatcttcagccggttcagtggccgtgataccatcactaatgccaaccaacagattgccccggtcaacaggacacacagcgttgaggtgaactcgtattggagtccaaaaagctggccgatgatttcaattaacatcacgtagccgacaatacaaattgctgccggagtagaaataatcagcacctgcttcatgaactgattggtaatcttgttgaagttaggctccaaagccaagaagaatgatgggattcccaccattaatgaagtgattggagtcagctgaatcggttcaaagggataccccgtggcaaagaaaacaaagataaatgacaacgcaacggagtacatcgtcttaatcagatacatggaagcaacccgctcgatgttattaataacccggcggccttctttcaagacatcaatcatggcgtcaaaattagaattaatcagtacaaagtcagcaatactcttggtgctttcacttccggaagccatggcgatcccacagtcggcctgtcttaaagcaagtaaatcgttaaccccgtcgccagtcatggcaacggtatgttttttggactggagaccggcaatcagccgcttcttttggtcaggggttacccggccaaaaacggtattgttggcagcaatttccccaaagtcgtcctcatccttaaccgttgtcatatcaacgctgttggcagcatcctgaatgccggcctgttgagcaattgtggaaacggtggtcgggtcatccccggaaatcaccttaatattgacatcttgattgcggaaatattcgaaagtgttggcagcattgggccggatgacatcagaaatcaataccaggccaatcaactttggtgcgtcaagtggctttcgtggatccaaatcatccacttgggcaaccgccaggactcggtaccctttccgggcattttgagtaatcacggcttgaacctgttcatccaagtgttcaaaaataaactgcggtgccccaaacacatagtcgtggccatcactcaaaccaacgccactccactttcgatccgaggagaatgggatgatcttttcggtctttagctcaggatcatcaacggcatctttgatcgcgttggccgtttcattcgcatccccggtaccatacgtaatcccggcaaccactttttcaacttccgcggcagaaacattcttcatcatgggaattgcttcaacaaattttaaatcgccgctggtaatcgtcccggttttgtccaaacaaatcacgtcaactcgggccaaggtttcaatggctggcaggtcccgcaccagcgttttcttacgggccaaatgcatcgccgaaaccgccagtgtcattgaggttaacagcaccaagccttccggaatcatgccaatcatcgctgcggcagcacccagaattgcccgattgatgccggtgccgccatataatttggcaacaaataaaataattcccaatggaatgatgacgtacgtcaaaactttgataatccgattaatcgtatttaacagaatgctggaggcgtcctcgccctgcttggcttcgttggataaatggttaacaaaggtgtccgcgccaacagttgtcacctgcattttgccggaaccgccgaccaaatacgtaccggaggttaatggatccccaatatttttggaaatggttaccgactcaccggtaatcggggattcatcgacttcaatcccccgtgatcggacgacgatgccgtcaaccgggatctggtcgcctcgtcccaactggataatatcgcccaggacaatatcgttggagtggacctgcagatcctcaccgtttctaatcacgttaatttttccttccgccaataagaccattttgtcgacttggcgtttggaacggatttcttggataatcccaatcgcggtgttaaagatggcaatccccagaaaaagcagatttttgtagctgccggtgtagaaaaccagtgcccccaaaatcacgttaatcaagttaaaaagcgtgaacgtattgtcgcgcaaaatatccgaaacacttcgggtaagtgattcctcgccagtatttttgtggccgtctttaatgagttgctcaacttgagcgtcactcaatccaacttcggggtcgacctgttgactatttccgtctgccatcgcttaacacctcgctttaccataattgtacaaaattacggccgaaaatcacatttatttggacgcaacaaattaagtttatcggatttttatgattttcaggccaaaacgttgccaaacatcgactggcgggtatgctaaaatgaatctaactaactcgcaagggggaaatgaaatgtttcaaccagataaaagtacctatcaattagccgacggccatcaaatgccaaagcttggtttcggcacttataaaatcgataatcccgaattaatggatcaaacgattgcgaccgcctatgacagcggctaccgaatgtttgataccgcgcaactctaccgcaacgaaaaacagctcggcgacgccatcaaaaaagttgccagaagagaagatgttttcattatcgataaggtcatggaaatgaaccagggccatgatttgaccattaacagcaccgatttttcactccagcagctgggcaccgactacgttgatctcctattaattcactggccggtcgcagaacacttctttgaaacttggcaggcaatggaggaattgaagaagcagggcaaggccaaatcaatcggtgtcagcaatttcacacgttcccaattggaattactgaagacccaggccaacgaaatgccggtggtcaaccagattgaaacccacccatatctaactcagcagcctttgatcgatttcgacaagaagatgtcgatcgtgacccaggcgtggagtccgttgggaagaggcattgtcttggataatccgatgctcaataagatggccaagcatcatggcaaaacgccggcccaaattattttaagatgggacctccaacgcggaatctccatcatccccaagtcaaagacgccggcgagagtcaaagaaaatacccaattggactttgaactcagcccggacgagatgagcatgattgacgtcatgaataagaaccagcgaactggcaatgagcctgaattggtctatgaactgggccaccaatactaatttgggctcgcaaaaaggaggcttttaccatgtccacagaagaacaacggatgctgtccggtaaactctataacgtttacggtaaggacttggccaagaagtacgcccaaaaagatcatttgcttcatcagattaattttgccgaagaagggaccgacgttcaaaagctcttcagacaactgctgggtcgaaccggtaacaacgtctattttgaaccgccgtttttctgcgactttggcggaaacattaccgtgggcgatgatgtctactgcaataccaacggcgtcttcttggactccggcaagattaccatcggcagtcgcgtcctgattgggccacgggtcaacttatttgctgccggccacccaattgatgccggtgttcgcaatcaatggctcgggttcgccaagccaattacaatcggcgatgatgtctggatcggcggcaacgccaccctgaatcccggtgtgaccatcggcagtaatgtggtcatcggttccggatcggtggtcactcacgatatccctgccaattctgtggcggcgggaaatccctgccgggtcattcgaccaatcactgctgctgataaagctgaatgggaaaatcaggaaactgaataccgggaatctttaaaataatatttcaaatcttaataaggaagtgatggcatggcccttggacaactgacgaatcaaattgtgttgatgtttgtattgatgttaatcggtgtcctcatcaacaaagtcgggttcatgcatacccagacttccaacgatctcactaacattctgctgtatatcgtttcgccctgcctgatcattggggcatttgaacaaacctattctgcagctcgcatgaagcaattgatgctggtatgtgtcggcatctgcttcttttacataattgaaatcctcatcgccaaattttcctttggccgcatcagcaacatcaacctgcagcgaattaccaaatatggcagcatttactccaacgccgggttcatgggcattcccctgacctccgcattatttggcaacacaggggtcttctttgccgtcgcgtcactggctggtttcaacatttttagctggacccacggtgtttcactatttaagacgaccaagaagcatcccgaccactggcagaattttcgtgaaatcatcatcaatcccaacatcattgcgatctttgttggcttggttattttcctactatcatttcagctgccgacaccggtcgaccgcgtcattcactacgtcagctcgattaacacaccattgtcaatgatcgtcattgggaacagcttgggaaatattcgcatcagccgtcaactgattgactggcacctatggctggcaatcttctttcgcaacctgttattcccaatcgtggcgatgttcattctccaagcactgaccgtttccggtgttgccttggatacgactgtattgatggctgcctgcccaaccgctggcctggtggttttgttcaccttacaggcatacggagatgccagcccggcagttgcgttgatgagtttatcgaccattttgagtttggcgaccattccgttagtgtttgctttaatgatggcattttaaatttgataagcgtgcgcaagaagagggggaaacaaagcattgcgcttgtgtttcctcctcttttggcatccaatattattcaaaaaaggattgaccctcatccccacttccggggaatcggcatcaatccttttagctttagtgaaattcgcaatcgtaactggattgttaaattcactaagcaactcaattaaaaattaacgaacgatcttttgacccattacgtcagctaatttcttcaacgcatcgtcacgagtcttaatcacatccatattccaaatgattgtgtcgatttcacctccggcatagtcaaacttttcataatagatgtaaggatccttgtcgctgtctttaaatacattatcgatcttgtcggcaaatccctttgaccagtcatcgtcatccatttctggaatatccttcttggtcacgtaaccttgctcgttaatcagatcaactgcttttttaatttgttcgtcggtgtatttgaggtctttatcattatctcgttcttcggcatcggctttcttttcggcagcactttcctttaccttttcagccatgataacatcccctttattttgatctatcttaatgctagcactgattgaagacaatagttaagaaaaacgaccatttccatcaataatatttcaaacactttaaaaaataccttgtgggggcgtataattagatgtaatctgtaggttacagattgatctaatttgaatatatcatttttgaaatgaggaattgaattttggacgatagccagatactgactaatctaattattgtgatagtaacgtttttgttcgctgctttcttcgtggcaagtgaatttgccctggttcaaacacggacaagtgcgctggaagaacgcaagaaaaatctagaagaagccaaaggcaataaagccaaggggttaaagaagctcgaccgtgagattcacatggtcaccaacctgaatgaatatctttcgaccacccaagttggtgtcagcttggccggaattatcctaggttatctgggtgaatcatttgtggtcacaattttggttgatgtgatggaaatccacaactcgccaatcgatccaaccgctgctcacgctgtgggcgctgtactggggatcatcatcttaacttatttggaagttgtgttaactgaaattgttcccaaaaacattagtattgatatgccaatgcaggtgctgtcctttatcagcacgccgctgcattatttccatgtcatcttttatccgtttgtctggttgctcaatatttcagccaacggaatcgttaagatgctgggcttaaaagttgccaacgaaaacgacgagtcgttctcgcaggcagaaatcttgaacctgtcgagaaatgccgttaagagcggtgcccttgaacagaacgattatctgtacatgcagcgggccttccagttaaatgataaggttgccaaagacattatgattgaccggacccaattggtcgtcatcgacattacaaccacggttaaagaagccgttcaagtctatctgcagcagaagttcagccgaattcctgtggttgccaatggcgataaggataagattctgggctatgtctacaactatgacctgattcgtcaatctcaagttgaccccaccatcaagatcgaccgcctgctcagagatatttcaaccacgccggaaatgacgccgatcactgatgttctccaccaaatgattcagaagcggaccccaattgtcgtcgttgttgacgaatacggtggaacttccggaatcattactgacaaggacatttacgaagagttgtttggaactgttcgggatgaaattgatccatcaattaccgactatatcttcaaacagccaaacggcacctatcaggtgaacggaaaattaaccactcatgactttgagcgatactttgatgctgatttcccagagtttaccaattcagacgccgttaccctggccggatacttcttggataactacccggatatcaaggccggcgatgtgatctcatttgagaacttcgatttcaaaattgttgactacgaaaactcatttatcaattggtttgaggtaaccaagcacaaggttgtgccaaagcctgacgatgatgacgatcaccatgacaactaatggttaaaatttcaataagactgtgacaagacaattgttttgcgagcagtctttttacatattagagacgatttagacatcataacgtttaagggggatctaacaagtgaaaaagctatggcaaaaaacaccaacgtggatcacatacacggtgctgtttaccgcgctgatctgtgttttagtcggttgcttgttcttaacaggtcgatcaatgatttgggagctggacggaatggcccagcactatcccattttagtgcagctcaggcacatgatactgtcatttctgcataatccaagtggtggctttacccattgggcttggaacatcagcttagggtccgatcagctgaccaatcttgcttattatgtgattggcgacccgttcaattacctaatcgcactgtttccaaagagtcagatcgaaaatgtctttgccttgctggtctttctccgaatgtatttttccggtctgagctttatgttgtgggcttcattgtatcaatttaagaagtccagccggatcatcgggtcgatcgcttatgcatttaacggttacgccttggcaactgccttgcaccacccattctttattctgcctttgattttcttcccactgctttgctacggcatcgatcgcgttttacataacaagtcgtggctgccattgatctttgccgtcttcctggtctttttaagtaatttctactttgcctggattcttgggtttggttcaattgcttatgtcattctgagaatgctgagcctgagaaaatggcctgattttacgcccctcaagtcctttggtaaattggtcctttcagcagtgattggccttgggatggctgctatcgtctttttgccaacgattattttggcgacgggctccacccgactcaatgacaactttgccaatggcatgactttctttccgctccagtattacttagatattcctggggcaattctaccgactggtcgggcgatgaacttttggctggtcatcgggatttccgggttgtcatatctcggcctggtgtacatgctgaggcactttaaacgctatttatggcaaaatgtcgccctgattaccatgttcatcgggatcctattgccggctgtcggcgccattatgaacgcgatttcgacgccttccaaccgctgggtcttcctggtaaacatcctgtttgggtttgcaacaatggtctttattgaacatatcagcgattttacgaagcaggatatcgcctggttcggttgggcttcgattggcctgattgtcttagtctgggcatttggcggcttcttaatgaatctccagccccacgatttcatcgtctatggcttcttactgctgacggtgattgtggtgatgggctgtgtcgtctttgattggaaacgatcgactaaagtcatcctggtctcgaccgtcttcatgctgaacttatccgccaacatcatcggcatttacagtccgcactccagcaaattagcgctgcagcagctgaaccgcggtctcgcaacccggtttagcaacgattactttagtggcgcacagaaatacctcaaaaagatgcccggcttcttcagagtttccatgaatccgcggtatcactacaatacccacattcaaaatttagccaactattcgaataccaataccgacttcccgatcaatagcgggctcaacgacacgtcagtctatctgaccctgcagaatggttatctgggtaaattctcacaatcagtcggcaacagccaattttcaatgaacaccccgattgctcaaggtgattatcgaaccgcctttaacaacctgctgggcgtcaagtacatgtttgccaaagccaacaccaagaatccaccggttgtcccttatggctacaaaccggttcgtgacaagaatggtcaaatcaaggtcttccctgccaaggcgcggacagatgccgtccaggcaatcgaaaatatgtatgggacgacaatttataaatccaataacgcactgccgctggtttatacgcagtacaacaccgtttctcccagtgcttatgacaaaatgagtgctgtcgatcgggagcgggtcatgactcaaggggcggtggtgaataaatcaaagtataatacccatccccttaattaccagtcacccaagaaaaacattgattataccgtcaaaatggatacctccaagattgtctataacggccgtcaactcaccaagtatcgacttggcattatcaataaagccaactcggaccagctggtcgatcaaccccacgaacaggtcagcctgggtgccaacctgcaaaagaccaaggacctcttggcaaccaaccgctcgatcatcgagactaaccactacaagaacattaatggcctaaaagagatgacctcagacgttgttggtaatccaatcgactataccttgaaggttaagaaccccaaggccaccaagaacactgaattgttcctggttctctccgggattaagcaaacggatggtacccctgccgaacacagacagtggatggctaaccagttcctgttggataataaactctactcgcggatgggcaagatggacgagtatcgtcacagcattttgaagccaacctttggcggttacattttcaatgccttcgctaaagatcatcaaaatgggtataaccaatatgacaacaataatctatccaattaccgtcagatcagtaatatcgtccttaatctgggttactcaactcaccaacgcaagaacattgacctcaacttcaatcaggtcaaaaacatcaagttcaagtcggccaagctggttgccatgccgttcaataagacttatgacactcaaatgcagaaactcaagcagactaagcctgccaatttgaaagtcaacggcaatcacgtcagcggcacgaccaacaaccaacgctccggcacgatggttacctcgattccatactccaccggctggaaattaaccattgatggcaaaccgacgaagaccttcgttgttaataagggctttgtcggtgccaacctgcctgctggccagcaccagatcaagcttgactatacgacgccaggcattaaagtcggcaagttggtttcaggtattagctggttggcatttatcatcctactgggatttgcgatcatcggtaaattcttaccggaacgaaccggtcaacagcacaagccaaaacatggcaagagccagtcaaattgaggttgccaactggtcgcccaatcgttaaagttaggataacaaacaaatttttcaaaaatcatttccatctaatctgaggaggtccattgtgagcccaataaaaattctattcatttcaattgagggaaatacgcgttcattcgttaaaaacttgaccagttatgcgactggcatgcacgaccaagaccctgccaatccattggtggtctcaaaggaaatcagtgaacagacagattttgctgacgaaacggaaccattctttgcttttgtcccgacgtatttggacggcggcaacggcattgacaacggcgttaaagaactgatgaccaatgccttgggggaatacattgcctacgatgacaatgccaaattgtgtcacggaattgtcggcagcgggaataaaaatttcaacgagcagtattgtctgaccgccaagcgttacgcctcacagtttaataaaccttttcttgccgactacgagctccgcggaaccggccgggatgttgagcggatttataaactattggcgcaaagctaaacgggttccacaattaaattaacaggaatcaaatgattctgaattaatataaagcaactggttacctcaccctgagaataatcagttgcttttttatatcatcgtcaaaaaaatccagttagcagctaaactaagccaattgctaactggattgatttctacattatttcgtttcaacgagccgttgccgagtccttcgtcgattcatcgcccataaaatgaccacaaaaataatgatcaagccggcggccagcgagaacagctctttataggacgcaaagtccagcacaatgccgccaatcaacggcccaactgcccggccgcacgacatgaacaggttatacaagccttggaactttccccgttgttgaggcgtcgataagctgtcaatccacgctggaatcccaggaaagccaatcatctccccaattgtcgtcacgatcatcaccaaaacaaaggcagtataatcgcgggcaaagattaaccacacaaacgatgccgcaaagattgccactccaacatacgtctgagtgctcagcttgaagtgagtcccgattcggttcacaaatggctgaccgatgacaatcatcaacccgtttaacgtccacagtaaactgtaattttcaaaaggaatgtgcaggctggtcatgtgcaccggcaggacactttcccataaggcatacgccagatagactgacaggaccacgccacaaattgccagaatcatcccgccaactttggcttcaactggtgccccaggcttaactggtttcccaggtgcccgccgatcaacgtgaacattgaattccaaaatcgtgatgaggaccagtgccgcataaaatgctgccgtaacggtaaacaccagggtgaccccatgctttaacaggaagccaaccattaaagtcccaatcacaatcccgacgttttggccaatgtacaagatgttaaagatatcccgtgtcgaacgggttttgatactggcggcatatgaattcagcagcgtcaaacaagcaccgtcaccaaagccaacgaacagcagcataatcccaaacatcggccagccatggaagaagaccaacgtgacaatggccgtcgttgaaatcagcgaaccgataatcgttgccttgtagggagaccagcgatcaaataaatagccgccaagataattccccagcatcatacaacacgacatcgccagcaggaccattccggctagcgtcaacgacttatgtaggtagttatgcagatacaccgtcaccagcggccacatgaaagccgccccggcgtttaaaatcagtgaatacacaatgaccgaattaaatctaatttcactccgttgttttatcaattgctcagtcccctcttacactcatttttaaccacaaaatcttctacgtccattttcgcatattaacaacagaaactgtatttattactgaagattatttaaaataattcctttttcagcctaatatcgtcctggtcggtaatctttcggagcacacgacaaggattgcccaccgcaagggaatcggctgggatatctctggtgaccacactaccggcgccaatcactgacccgttgccgatcgtcactccgccgatcacggttacgttactggccaaccagcagttatcctcaattgtgattggcttgctgtactcttttccgggtaaatcattattggcggcaaagtttcggtcttggtagcgcagtggatgcatcggtgtgaccaagctgatgttcggcccaaataaaacgttgtcgccgatggtaatcatgccggtatccaaaaaagtaatgttagtgttaccgtagaaatgatcgccaatcttgatatgagtaccataatccacaaagatcggtccctgcagataaatccgttcagatgaattgggcagcagttgcttcaataaatcagcccgcttctcgcgttcatcgtcaaaggtgtcgttatattgtttgaccagccgatgggccaatcgctgacgcgccaataattcagggtcgcggggattgctcaatttgccggcaagcattcgttgatcttcattcatcattaaggcctccaaacctttgggttacagttatcatagcataggcagagtggacacgaggcgttttgatcccagaatttaaggcacaaatcgagttattcctgtccttggaatgactcgatttgtgccttaaatggccgggatcagccgatcgttccacgtttaatcaaggataacagtagaactcaaaagggactggaacataactgacaagcagttaagtcccagccccgaatcaaatagctggttaaaattatttaactaaagcaaatttgtagtagtgaagcggcgtgttgccatattgaaccttgatggcgtggttggctttgttgacaatgatgaaatgcgtattgtcagtaaatctcaagtagaacttgtgataagtcttgctgccgcgttcacggtaagtaattccccagaaggtctttgagtaagtcgtgactttgtagttggcgaagttgatcagcttcttttgatacttgccattcttatacaggccttggttcaaaccacccttttggctgaagttggtgacaacgctgtaaccattgttgttgcctgattgccaacgaccagttggttctgaaatgttgatcttactgctggttgatttggtgcttgaaccagtcgtggtcgttgccgtggcagtcttaggtgtcttaacggtcataattcgatagaagtatgaggttgatgacttccgtgcgtatacataaagcttctggttggctttaacactggtgtgcagctcggcgctgaacttgccagttgaactgtcagccgtggtgctggcaatggtggttttgttggtgtttcgaacaataatggcaacacctttggtggcagttccagtcactgcctttgaggtcgtataaatgttattgactttaagtgacggagaacttgcagaagcgttgacactgaacccaatcaaaaatgatgcgaggacagcaaagaacgcgataaacttaaatttcttcatttgatattgctccctaatctttattttgcatgactcattataaaggatatgggcaaaaaaagccgtcaagtcggccttcatttatccttttcttaagaaaaccgtcactgtttaggcatcgcttttaggcggctaattatgaaaagaacatgcctgtaaattttattcatttacattggcaattcgcttttgttggggtctcatgtgttatataatgttggggaactggtatagacatataccaaattacttagttaatattctgataggagtgaacattttgccaactgaaagacgttctttgattatgctcttcggagcaactggtgaccttgccactcgtaaactttatcccgcaatgttaaagcttttcgagaagggaaacattcgcgatcactttgctgtgattggaacttcccgttacaagttcgatgatgaaaaataccgtgaaatggtcatcaagtctgtttctaaagaatctactaataaaaaacaaattgctgatttcgccagccatttctactttgtgacccacaatgtgactgaccttgaacactattctgtactgaaaaacaaagctaacgaactcgacaagaagtatgaattgaacgggaaccgcgtgttctacatttcaatggcacccaacttcttcggaaccgttgctaaaaacttgaaggctcaacaccttctctccgaaggaaacggctttaaccgcttagtcattgaaaagccatttggccgtgatttcgaatcagccaaacaattaaacgacgacttaagcaatgcctttgaagaagaccaaatcttccgaattgaccattacttaggtaaggaaatgatccaaaacatcgaagctattcgtttcggtaacaccattttcgaagccctctggaacaaccgttacatcgacaacattcaagtcacccttgctgaaaagctgggtgttgaagagcgtgccggctactacgacaactccggtgcccttcgtgacatggttcaaaaccacattatgcagattgtcagtttgcttgcgatggaacaaccggttgcgttcaaagataccgatatccgtgctgaaaaagttaaggctttgcgtagcctgcgggtttacaacgttgccgaagcatcaagcaactttgtccgtggtcaatacgctgccgttggtaacgataaagaataccgagaagaagacggtgttccaaaggattccaacactgaaacctttgttgccggcaagttgttattcgataactaccgttggtcaggcacaccgttctacattagaaccggtaagaaactcgctgacaagttcacccgagttgatgttgtcttcaagaagccattagttgacatcttcgccttcccacaaagcggcagtgcaccattgagtgccaacgttttgaccatcttcatcgaaccaaaccaaggcttctcattgatggttaacgccaagaactccgaacaaggattccacactgaacccgttcagttgcaataccttgaagattcaaagcggacccgcgaaaccccacaaccttacgaacgtttaatccacgacgttttgaagggcgacggtaccaacttcgccagctggccagaagttgccagtgcatggaagtttgttgatcaaatccgtcgagtttgggatattcaacaaccaatgttccctaactacattccaggatcaatgggcccagtttcagctgatgaattgcttgcccgcgatcaccgtgaatgggtatacaaattgaataagtaacatctaaccaatttagctgaccgaaaaccaattcgtttccggtcagctttttgtttgggttaatatttgaaataaattgaaaatttttaccattttgctgaaagtccatggatccagatttacatttttcaagcaacaaaatcccttaatgattgaaaatcggtcattttgaattatgtaagcgctccccacgaaacggcttttcattttcacaatctctcatctaacaaattcggcatactgttccaacgcgtttttgtttcactttccacttgtgagatggtacactaattgtgtagtaattcttatatagaaaaggatggttttgaaatggctgatcaaaaagcaaacattggtgttgttggtatggctgttatgggtaagaacttagcccttaacatcgaaagccgcggttacactgttggtattttcaacagaaccggctccaagactgaagcagttatgaaggatcatggagacaagaaactagttccaagttacaagattgaagactttgttaaatcacttgaaacgcctcgtcgaattattttaatggttaaggctggtaaaccaaccgatgctgttattgatgaattactgccactcctcgataaaggcgatgtcttgatcgatggtggtaacacaaacttccacgatacgatggctcgaaatgcccgtctcgataaatcaggaatcaactttatcggcatgggtgtctcaggtggtgaacttggtgccttacaaggaccatcactgatgccaggcggccaaaaagaagcttatgatttggtagaaccaattctcaagcaaatcgctgccaaagcacctgctgacggcgaaccatgtgttacttacattggaccaaatggtgccggacactacgttaagatggtgcacaacggtatcgaatatggtgatgaagagttaattgatgaaagttacaacattttaagaaaccttgccggctactcagttgatgaattagctgacatctttaaagattggaacaaaggtgaactcgacagctacttaatcgaaattaccgccgacattttgactcataaggatgatattggtgatgacaagaccaagccaatcgttgacatgattcttgaccgtggtgccaacaaaggaactggtaagtggagctcacaagatgcccttgaagtcggtgttgaccaatcagtgatcaccgaagccgtctacgctcgttacatttcaatgattaagaacgaacgtgtcgcagcatccaaagttcttcctaagccagaaggcaaagttgattttgataagaaagaaatcgttgaaaaagttcgtgaagccctctacttcggtaaagttatgagttacgcccaaggctttgctcaattaaaggctgcttcagaacaatacaagtgggatatcaagttaggcgaaatggctaagatttggagagccggctgcattattcgggcccgcttccttcaaaatattaccgacgcatatgacaagaacccagatctgcaaaacctgctgctggatccatacttcacggatattgccaagaagtaccaggaatcagcacgtgacgtcgtcgcattggcaaccaaggccggcgtcccagtaccatcattggcagccgctgtctcatactacgactcatatcgttcagaagttgtcccagcaaacttgctccaagcacaacgtgactacttcggtgcccacacgtacgagcgtgtcgaccgtccagggagtttccattatacttggtatgaagaacagtagtgcgcgacgaaacccgggttgaccccggaacataagacagaaaaatcatggatgaacgcttcttgttcatccatgatttttttggcttatgtggtaggggtcagggttgtcggagctgtcctcaaaggcagccaaatctgaaaaataaccataaatgccaatcatcttttgagcattagtttaataaggaccgttaacgctgcttttacgttgacggtccttattagactaagcgggaattccgactttttacaaaaagagctggcactaacacaccagctcttggtatttcacttaattggcagccacaatgtcgaccgccaaggcacataagcgtttacgaagtttatcaggaacttgaccaatgatcgcgccgttacgggcaacataatcataattgggtgtttgccaagtcacaatatagccattggtacgactacttgggtcaagaatcggttcgaatcccttttgaatttgaccagtgccgtgcatgataggcatcacgacaacaaatcctgtcaaccgattatattgggcgttcgataccaccactgctggtcgtcgcgggtggccagtcgtatgtccgcccatttcatgcccactgtggggttcgaaatctaaaacgataatatcgccttgttcaggaaaggatgtactcataattcccgacctttccttgactcgtttccaacattgaaaccaatctcgtcaatctggctacgaaaatcaacattgttatatgcgcccgatatccacgggtttttatggctgtgggcgcgccggataatcaaagtatcttcatccactttttcgattaccaccggctcgttgctcgaaaatcctgtgcttttaggcaaggttacgctgaccgaattgccagttttatgcgtttttgtgtttgcaatttttaagttattcatgatcaattcctccctaaaatttgagctaagtatatcgtaattacaatgttattacaagtacttaccttggtaaatactcatcctttaagatgagctgatcttgatatttgagcatcaaatttgttcactcaagcactcagataacatacccactcaaccactgtcaaattaacgccaaatcccctcacaggattcaaattcaaaatcccattaataaaaattgctcgcaatcatattaaaatactatatttattgttataataattatagataggaaaacagttatagagtgagggctcttgaattgactgtttccaagtagacatgatggccaacttggctcacaccattgacaaggatgccttcagcaaagcacttcagcgtgctcaaatcaattttgaaaacagattgtttcaatgcttcgacataatattcatgcctatattgttatatataaccaacaggggggggtgatgataacgcactattttttgacgtcgcagattgatgagaacacatctgcgatcgaaattgcggagattcaacgattacatttattttcgaaactcaaggttcctgccacgattgtgacccgcaaccgcaatcgtggtagtaatcgggtgttacagcagctaatcgacaatcatcaagtcattaacctctaccaatactttactgagcttcccaaccaagccgagccgattcccaaagctgaagatgtgttgcacgatttcactaacattccgattgaaaatgatctgggatataaggatggcaagctccgggttcgagtcaatgaacagaatggctggatcaataacatcgattatttggaccagttcggcttcaccgaccgtcgcgacctgtacgatttcaatcagcgcgtgtcttcagagtattttgacgatcatgccaaattgatcacgcgggtattctatcaaaaagatgggcacatcgtcatgactgaatactatcgaggtggccctggcaaccaaccggtgctgacgctgattcacttacggcataacggccggctctggcagttcgataatcaggacgcattaatgggctactttcttgactgcctggcagcagacgattcgaacgccacgttttatagtgaccgcgaggacgttgccatccccgcatttaaattgatgaccaagcccgccaaacgctatctcattttgcattctatttttacgcaaaatgccaagcgcgatggtgagctatttccatatttccagcaagcgattgacctgaaggacaagttatccggcatcatcgtttccactcagcaggaagccagtgacattcagtcacggttcccgatggttcaaacgaccgttattccggtcagttaccttgacgaccagctgattcatcagtcggaatcatttagcgaccggattcccggaaaagtgattgctgtcgcgcggatcacaccgttaaaacagctgagccacattattcaagccattatcttagttcatcaacacctgcccttcgttactctggatatttatgggtacgaaaatgtcaatgacttccaggaaggcaacaaactgcgccaactcgtcaaaacatctggggctgagagctatatcaccttcaaaggctacgttcacgatttggcgtcagtctatcagcacgctgacttgttaaccctgaccagttcatacgaagggtttgcaatggcgatcttagaagcccttggttacggatgtccggttcttagctacgatatcaattacgggccggcagaaatgattcaagacaagcataacggggaactgatcactgcaggcgatgaacgtgaactttatcgccgactgctgcacctactgacacaccgagagatccttcaacggtacgggcaaaatgcgccggcatctgttgagaagtattccgcaagccatgtgcagcagatgtggcacaattttattcaaaatcaatgaatgacaaactaattgaacaactcaattaagttcatttttacaaaatacattattcgaggggaaataataccatgacaaaattaaatagaaccaattcaaaggttcattacaaaatgtataaggccgggaaacattggctgtacgcttcactactcaccgttggcttgatggccggcggcgcgtttggcgctagctcagtcgaagccgatgccaacgataatcaggcaccggcaacaactacgaccgctgcgactactcaaccgagtaccgatacgcaagccgctgctcaaaccagttcagctgacaactcgacagccacaacggataatagccagacgccagcccagtctcagaacaccggagcgacaaccacttctgacgctagtcaaacaagtggtgcaaccaccacgactcctgatgccagtcaaacaagtggcacaaccactacaacaacgacagccgacgatcagggaactgatcaaacaccgaccgcggatcctacaacaacagggacgaacgactcgacccaaacgactgggactgatcaagacaataatcaacccgcaacgactacgactaatgatccgtctgcaactggcactgacaatgatgccaccacgactgacccatcgaatcagacaagcgaccaacctgatcaaaatgcggctgacgaccagaacaaagcctctgacccaaccacaaccgatgatccgaacacggccactactgaaaacactgatgcaaccgctgattccgcaaagacagccactaccacggatccaaccgattcatcgacaacagccgatcaaaccgcttcgttagctcagacgcctattgatacccaatcactggcggacccaaattccagtgatttttgggaacaggtctttcaactagcaactattattccccaagctattgccggcgcggccatttcggcacctgcaattcttggcggtgggacaatatcactgtacccaattaactcatcatcagaaccaatcgtgattcctggacgagttcttcagtttttaactggtggactgtggtcttccccttgggatatttggaatgccttgaaggatgggttggggattaacagcggatccaccgctaccagcgcacctataactaattctaatcaaagtgaaatgacaaacttagcggccgcaagtgtttccggtcaatctatcgtgggtgatattggccagctctttcattccgtagtaaccaccattcttggtgaactgcagtacccaatactttctgacgtccctggaatcattctgtgggttactccatccacacctaatcagccaactggacctaaccagccaactgaacctaaccaaccaactcagccaaaccagccgacgcaacctaaccaaccaactcagcctaaccaaccaactcagcctaaccaaccaactcagcctaaccagccaacgcaacctaaccaaccaacgcaacctaatcaaccaacgcaacctaatcaaccaacgcaacctaatcagccaaataaaccaaataaaccaaatcggcctaatcagccgaataagccaaataaaccaaatcgaccgaatcagccgaataagccaaataaaccaaataaaccgacacaatctaatcgaccaaatacgccgaataaaccaagtcggccaaatcagcctaaccagccaaccaagtcgactcactccaattggccgactaagccaaatcactcaacgggaaccactactaaccgcacatcgcggaattcccgagatataactggcaagacaccgattgaaaaagcatccgtcttaccacaaacaggtgataagcagcaaaattggctcagtattctgggtgacgtttcattggccgtcattgtcatttccggcgccatgattttcaaacggcgtaagcgtgattaattaattttgaataaatcacgtaagttcaacatttcataaatcttcagatgcttaaaatggcccatggccaaattccgatcatgattgttctcacaaacatcatgttaccgggatttgaccatgggccattttttgtataaatttttatttcactggtcaacagttagctaaacgctagccctgctcgccagccttaatcttcttgccaaaggcagtttcatcaaaatgatcaatcacgttttgaagatccgccttggtcaaactagcaccaaacagctcgctgccgggctccgtcatgatgccgtcagcaatgttgtaatgaaccacagtgtcaaagcccatgctgtcgacaaactcggccacttgatcaacggcggcttggttatcgccggtcacaaacaacgctttgcgattgtctgctccagctggtttggcctcttcctgcaggttgtgatagcccatgtggttaaatgttttcaccacggtactcttattgaaatactgctgaacctgttcactggaagtcgacgatgggtccagcacttcttctcgaatcccgtcagtttcccaccaatagttcatggcatcgatcaccaatttgccctttaagagcttggatttgatgttcttgtagcggctcagtggaattgctaagataatcaggtcacttttggcaacaaccccttgattggtcgccggaactgcccccggtaccaaagtctcgatggtcatggcaatcttttcgaccgacccggatccggaaattcgcacgtggtagccagcctttaacgctagctgagctaacacgattcccaccttgccggcacccaggatgcccacatttttaatttcagccatgcttagccctcctcagacaaaatttctttgacacgaggaatcaccgtggtcgcgtaaagctcaatcatgcgttcacgctgggcagccgtctggttgccggcaccgtagaccaagtcaaatcgacccaggttcatcagattaatggtgcgggccattcgctgggcgacgtgttccggattgccaacgtaaaatgagccgaccttggtttcaccatcaaattgttcccgactcatcggggcccagccacgggtcaaaccgatgcggtcgaagttggccttgatattcttccaagcaacttcaacggcctgatcctcatcgtccgcaataaagccgtgagaatggacggcaacgggttgaaccggcatattgtatttttcagcagccttcttgtacaaattcaaatacggcacaaagcgatccgcctggccgccgataattgccaagatgaccttgtaaccataccgggcggtccgaataattgattcgggtgagccgccgataccgatgtaagtttcaatgccattataatcggtctttggatagacatcctgatccttcaaggattgggtgaacttgccatcccaagtaatcggcttttccttaatcagttggctgtacatctctaatttttcattgaataaatcatcatagtcggttaaatcatagccaaagagtggaaatgattccgtgaaggatccccggccaagcatcacttgagcgcggccttgggataagccttcaagcgtagcaaaccgttcatagactctgaccggatcgtcggagcttaacacagtcaccgcggtcgccagcttgatgcggtcagtcaccgaggcgagtgcgcccaggacaatttcagggcttgagacactgtaatcgggccggtgatgttcgccgatcccaaagacatcgacgcccagcttgtcagccagctcgccttccttcacgatttggcgaatggattggccagccgtcaacagctcgccgtcttctccccgaacgatatcgccaaacgtttcaaggccaaattgtaatttgtctacatcaaccatgctcatgctttttcctcctgctgcttactttttgtaagtatgataatagattatagtaatttgggggaaattgcaactaaaatagctggggaattggcttcaaaagtctaaaggcagaaattaggactcgcacaataacaggcaaggctgaaagttagttcaaatcatattcaaactgttggaaaaaggattgaagccgccattgaataaattaattcatacgtaaagtccccctaaaaccccagaaaatgggcacatttacagttaaagacagttggggttcacgactttcaaataacgtgttaacagcgatcaattttttgacccactaaatcgaatttatcccattttaagtagccaactgccgatctttaagataaaataatatgaagatccagagataaccacaattttaactgaaagaaccgagaggcagaataagacagagggacatcaaatgactataaagccttggaaaagccgatatgagcttgccaaaacactgattgatgaacgacacctacaaaatactaatgttgaagagattgaatccacattaaaaaagatgaattattttcaactgatcaatggattagaaaatgatctcttatctcaaaaggtcccgaaacgttttcgtaccgaaacttttgatgactttaaacgtttatacaaattcaataagcaacttgaaagtgcaatatttagcctgattgaagattttgaagatcagttaaaaacatcccttgcacataatttcagcgcaaatcattgccgaactctgaatgatacaatgcaatacaccaataagaacaattattacaacatcaagaatgactatcagtatccctttactcgttatcaatacaaatatacgtatgaaaatttcgacaagtttgaactatttaagccaaacttcattgataaattaatccgaaacaatgactttatagatcccaaattttatcaagatccaaactatgtgcaaccaccaggagttaccccctatcataagaataaccaagttgccgtccctctatgggttacagtgcaaacactcgatttcggcacattaataaaaatgactcactatttaaaaccggctgatatgaccggtattctaagtgattttaacttcaaaccgagctcgagatttgcgtttctaagtgcactcgacgtaatcaaggagcttcgaaataagtgtgcacatggcttccttattgaaagattttcaacaccagaatatattaagctcaaccgtaatttagtggctaaattatcactcgatccctatcacaaaggcggtaatagcgtctttccgtctaggctaaaattgttcgattctttaaaagtcctaggaatgtttgttgatttaaggcctttgggaaagattttcaagagtttgatataccaaaacaataaaaacttctcgaaaaatagttatgatttaaattccagaatactgcaggatattggcgccccatcatataaagcgttaaaagccgcctgcgttgacagtgttagtaatagatggtaaattaaatgtacagagaaataaatagggccttaaggccacaaggcggcagttcccttggtgccttcgataaaacagctactcattacgagtagctgtttttggtttcttaagctggaattttaattctaaatgaggccaattgtagctgtcacttatgatcctgcaagaaatacatttcaagtcaacaatgaatcaaaagagtttttgagacttcttctacagtgctggctgcattagatatccccatcatcaatttacttgtaaacctctgccaacttggcaaaatcagtcgtccccaacccgcttgcctggttatataccgtaccaggttgtcccgtatagaataagttcgagttgtcagttgtatcattcaatggatgaaatggtgaatctgattgctgagctaaacgatagatttccgcattccaaaatcccattcgtggtcgcccttgctcgctattaatcagtgcggtcatgccggcatactgcggtgcaacaatacttgtcccggcgccgccagtccaagggctctcacctttttccttttgatacatcaaatatccattcaatccacctgcattagcagagacatctggataatttcggcctgtatcagttccatgcattagcggtgtgtcgaaaacgggttgcgcaagattggatatatattctcgggcattgaaggtattaacccctggcactccctgctggtatgaaggtgttgcttccaaatggctaaagcccccgccactacccccaaagccatgaattgactttagaaccgtcgtggtgtttccgtcttgactcttaagtgagttccaagcccagtcggatccccaagcgcgttcctttggaattgttactttgcctaagttaagaggtgttttgatggtatgagttgaagcagggatagttcccccgcacgacgtaatccatggacttgaactaatagggtctgaatcagttgttgctcgatcgagtaatccctgatttccagatacaccacgcaatgtattaataagtgcgccggtatcccctgacgccgtgaaattagaaataccttgaagtgcgccttgcgccaatacaaggttaagcacttgaagatatttgggagtcaagacccgccgttttactaacatttgtgaaattgaattgggcccgatcccccaactattagaaaccgagccaactttgttttcgttgaagacagttgaataagcattaattgtatttgtgaaggtcgctaatgggctgttctccaaataaacttttacatttgcctgaggtgcaacagcaccagcatactccgcatccatagttgtttctgattcgtctttactgacaaagccatttttaaaaacgcttgtaggaacagactcaacggagagtcgatttttattggtgctggctccttgagatttccagaaatgaaacacattagacttaacgacattgccaaaggcaattatcccaacggtttggcctttacccgttagtccttgctgatatagtggctttgcattataatcttttgcaaacgattgaagatcgtacatattatttggaactctttttgttttatcaatcatctggacatctgcgtctggaatgacaaacttacgattgtggtcgcccatgcctaataccgtatagacagatttttgtagttgagccggaaatcgtggtgctgacttcccaaactggagtggattagaatgatacgttgcatggttcatatcaactttaaataatttatctatgtatttagctttgccagatacgcttaaaattatcccgttatcatagacaaacgtgcttaagtggtgtttgcttaaataagctttccaactattagtcacacttttggattgcccatatgcattacgaatcccacttggggttagataatttctaaactgtgaatcacctggagtattcacggccatggcttgcttatataattcttgagtattcgttggctttaaaacaatatcaattgttgttgatgaacttgacttaacaggactaggtttcagcagcggagccgaagtaacagcaccatacactttgctaatcacttgcgttccttttgcatgagcagaacgtccacctatcccaacggcagatacactcatacataaaacggcaaattgtacccaacttttcatgattgatcttcccttcatggagatgattataaaatcagacatatcataatcctaaatgtcgaagcagacaatatgaatattggtataattagttggttattaacaatctgtatgattagggggacacaaaacatggtacctaatattcaattaattcaagttccaataaccgataccgaaacaatcttagttatgtacaaggctgcattcaagcaactctttatgaaatatcatgatgtcaatacgagcccctatctagaacagaaaagcaacctcgtcaagaagatgagggatccacgttcaacttattactatatcaaaactagcaaacacgttgttggactcgtccgggtgattgtttctgatagtggccaagaagcaagaatttcaccgttatcaattctgccagaatttcaaggaaatggctttggcagcagcacattattacaattagaggggctctattcacgcgtaaaaatttggtcggtagatacaattgtccaagagcagcatttactagccttctatacgcattgtggatatcagacaacccatgaatctgtatatcacatccaaccaggaatggatttggttcaactggtcaaaaaagcttagcaattgctgggcattttccagacaattgccaagacagaaagaggcacttcattatgaacaaatcagctttaatcgtcattgatctccaaaatggtctcaataaggtattcaacttccctgaactggtggcaaaaattaatcggaaaattgatgcctatcatcaagcaaatttgccggttgttttcatgcaacacgttgatgatgaacttgtctatggcactgacagctggcagatcgtcagtggaactcaccggttagaaaccgatcgcgtctttttaaaatatcacagtgattcgttttatgagactggtttagaatcatacttacgacatcaaacggtcaatacccttgatgtctgcggacttcagacagaatattgtatcgacactgccatccgtgtgggacacgatcgtggattcaggatgatcaccacctcaggccttaattcaacattcgatacggacgatttgactgcccaacaaattattaaacatcatgaagggatttgggatgggtcgtttgcggaagtacaggcacccatctaatcagcttaattggttgatctcatattatttaaggagacatgcatgaagaaaattttgctttcttcaagcgcgttcataaatcaaagaattactgacacttttttaagcatgttagacaaaatggtattggcagcaccatcctttaagtttaaaattagcaaacaaaaagggcaaaatcgtgctttttggaatggctggttggaatccgcgggcgactgatttgttgactgttatgggaaatgttagaccatcgccacgggtattttatgggactaacttatgagttttgatgagcgccgaaacgccgcaaacgattattcagctattttcttgatgggaaagtctatttatgccagctgaccgttctccgcttatctgaaggtcggcagcccaacagctttttggaatctggtgaaaactctgggaagatattgccgattctaggtccgaaacgacttggtgttttcattcttcacattttcccctccaaaacaaaaacctcagcctgtgaaaacacagcaactggggttttgttagtccagaacctattcctcgggccctctgaacttgatcgataaatgaatcgtattagagattacagtgcgtgtcaatgatcctgccacgctgaacgtacgttgcttctagaacacgattcgtggcccgatataatttacccaatggcttcctcaaccgcatcccgcaactcccgggtagcactggccggatcggcagccttcataatcgcagaaaccacagccactccatcaacgtgcgcaccatcaattgcctcgacattatcagctttcaagccgccaattgcatacacgggaatatccaccaatcgtttgatcttaccaagggtttctaccgtcgtatgaacggtcttaacgtgtgtcgtggttgggaaaatggctccggttcccaggtaatcagcacccatctcttcagctgctttagcctgcttcaatgtcttggccgttgcaccgataatctttttgggtcctaagattcggcgagcaatgtccacaggcaaatcactttggccaagatgaacaccggccgcatcaactgcctgggcaatatccaatcggtcatcaataatcaggggaatcttgtaccgatcggtaatggcctttacctttagagcaagttcaaaaatttcgcggctactgccctctttttgtctgagttggaccaagccaaccccattttgcacacccgcttcaatcgcgccaaagaattgttcatcagtcaatccggtgtggtccgtcaccaaatagagtggtcgatttgttagtttcacaatcatttcctccaatattttgtcatttgccatcagtgtaaatgaaccttggcaaaaagtatagaagtatttctcacttgactttcagattgtaagcggttataaatagattatgagcttgagcaaagtttcaagcctaattgaatatttcgtctggggtgcctgaaacggctgagattacacccatcgaacctgatgtagtttgtactgccgaaggaagagcgaatttaatgttgaatttattttgaccttaaaccttctttttgcggaaaagaaggtttttcttttctgtgaatcgaccttaatgttgaaaagacatccaccgacctctttcttcggaatctgaagaaaggggtctttttgtatggtgatggttaacggtgaacaagaatccggcatggttggtcaaacaatcaccgagttcttgaaacaaagagaagcaccaattgaaaacatcgtcgtcgaacagaacggcaagatcgtccaccgctctgaatttgacacaactaaaattgccgacaacgacaaactggagttaatctcgtttgttggtggcggctagaatggtggttccaagtggaagtctgcgggtaaccgtaaccgcttggatccgctcactgattaggacagctcctccaagcagaaatctccgtgtaagcacctcagagaaaaattccaaacccgggaatttctctctgaggagacttacactccgatttctaaccgcttggatccgctcactgatataaaaggagtcgattgacaacatgcaagaaccagaaattcaaggaatgagttacgatgacgtttatctcggcatgaaagaacgcaatgtcaaggggtcaactgacaaattagctgccgctcacatcaccattgccggggccggtggcttaggttccaacattgccattgcgctgacccgcattggtgtcggccacttgacgttgattgactttgacaccgttgagctcagtaacctcaaccgtcagcaatttaaactcagccaggtggacatgccaaaagttgtggccttaaagcaaaacctgcaggaatttaacccgtttgtggaaattaacattcaccaaaccaaagtgacccatgacaacgtcaaagaattatttcaagacgctgacatcatcactgaagcgttcgataaccctgctgccaaggcgatgctgctggatgccgcatccgagttctatcccgacaagccaattgtgatgggcaccgggatggccggcattcacagttctaacacgattaccaccaagcatccccgcaagaatttatacatcgccggtgacggtgaatccatgggggctgagggcttaatggcaccgcgggtcatgattgcagccggccacgaagccaatatgattacccggctaattttaggagatacagaaatctgaggaggatttattcatggcaaacgaaaaagatgagttaatgattggcggacacgccttcacatctcgatttattttaggttcaggaaaatattcatacgatttgattgattcagccatcaataatgccaaggcccaaatcatcaccatggccctgcgccgcaacaagaccggcaaggaaaacatcttaaactacattcctgaagggatcaccattttgcctaacacgtcaggctcgaccaacgctgaagaagccattcggacagcgcgaattgcccgcgaactaagcggcagcaatttcatcaaattggaagtcgttcccgataagaaatacttgatgccggacaactacgaaaccctcaaggcaaccgaagttttggccaatgaaggcttcatcgtcatgccttacatgctgccggacttgaatgtcgctcaccaattggtcgatgccggagctgccaccgtcatgcctttgggcgcaccaatcggtaccaacaaaggattgtccaccaaagacttgatccaaattttgattgacgaaattgacctgccaattatcgttgacgccggcattggtcgaccaagtcaagctgccgaagccatggaaatgggtgccgcagctgtcatggccaacacctcaatggcgaccgccggcaacattccgctaatggccgaagccttcaagctggccgttgaagctggccgcaaagcatatttggcaaaaccaggccgggtcatcgaacacggtgcggttgcctcatcgccacttactggtgtcagcgcggtgaaataggggcggtcatatgacaacaacccaattaaccgaactcgcacatcgattagcaacaattaaccaatttaagaccaatgaagccggtcaaaaccggctggtctattcaccaacctgggttgaggctcaaagacaagtcattaaatgggggcttgagcttggctttcaggtaaacgttgatgactttgggaccgcctatctggacatgcctggaaccaccgaaccggaagcggtcattgcgaccggctcacacattgataccgttgcgcaaggcggtcaatatgacggcttgtacggggttcttggcggccttcaggcaattgaaaatctggtaacagaattcggccgtccgcagaaaacgcttcgactgatttcattcagcgaagaagagggcagccgctttccggatacctttaccggctcgaagcactataccggccaacaggtggatttgacgatgaaggatcctgccggcattcaatttgatgatgctcgacaacaggcggttaccaaattgatgctcgctggggttcaccaccaactgccggatttaccggatacctttaccgaactgcacatcgaacagggaccgcgattaattgaccatggcctacaaattggcttggtcacaggcattgtcggccaacgccgttacaccgtcaccgttaagggaatcgccaatcacgccggcaccacgccgatgaatgaccgagcggatgccctgcagcacgctgtggatctcatcgtcaccctgcgagaacaggctcgtcgattgaatccggatttaactttcacggttggggaaatgcacatttcgcccaatacgtctaacgttatccccggcctggtcacgtttacggttgactgccggaatagtgatgaagccgttttggatcaatttgaacgactccttcagcaaaccgttacggctcctggcaacccgcagattaccagttcggccgatcgctgggcgaaaagcgacgtgaccctactagatcgccagttgctcgagaataatcaggcaattgccaatcaactggggttcaaatccattcagctggcctccggtgccggtcatgacagtcaaatcatggccaagcacactcggacgacaatgatttttgttccaagcatcaacggcatcagccatgcaccagcggaaaacaccagccaagaagatttacttcgcggcgttgagctgttagccgccagcctccaccaacaagcctattaagtttgggggaaccattttgaaacacattagtataactgcacaaattggaatcggcatgattggcggggcgcttcttggattggcatttggtccaaaaatcgccggcatccaattactgggaaatattttccttcgcctgattcaaatggcggtcgtcctgctcattttcggggcggtcatcgaagcactgggcagcttgaaatccgatcaactgggaagattgggtggcaaaactgccatgtggttcttgatcacaaccttaattgcagcagtcctcggcttagccattggctacgcagtcaatccgggcagcggcatcaagctggcttcggtcagcacgtcggcaacggtcgccaaggcaggaactagttttagccaaacggtcttggacttctttccgacgaacatttttgacgccctcgccaaaggtaatgtgattcaggtgattattttcgcgattctgtttgggattgttttgaaccgtgccaatactgacggcaaattcaatcaagtattgagtttcgtcaaacagatgaaccagctaactgtcaagctggtcatgctggtgatgaagctcgctccaatcggaattgccgccttgatggcctgggtcaccgctaccagcgggattaaagtcatcctgcccctgctcaagttcctaaccgcatttgggctgggctcgatcgctttcttgattgtcctgttcagcttcatcagctggtacgccaaagtaccgctgagaggattggtccgcggcttttcaagaattattttagttgcgtttacaacgacttcttcagcaatttcacttccaattgaaatggaagatgctgaaaaccggttgggggtcgaaaaatcgatcagccaactggtattaccgctgggaatggcgttgaacagcaatggtttggcaatgtatttgtcgctgtcatgcttgacgctcacccaactctacggaatgtccgtttcaccaatgtcgatggttaaaattgtcctgctgtcagtgatcgcctgcctgggaacggttgtcgttcccggcggcggcctggttgcattgacaatcgttgtcccaactttggggctgccattgcaaagcattgccattttagccggcattgactggttctcaggaatgtttcgaacggtcctcaacgtggttggagatacgacaaccgcgattgcagtggcctctgacgaaaaattgctcaaccgggatctttacaaactacatgtcgacaaaatggcaccaaaaaacaacttgtgagatcacttcttcgatttaagtaccatagattcatgcaggaaaacctgcaacacttttctaccacaaaaaaagaccagcacctgagattactagacgtctcagcgtgctggtcttttgtgaaatgcgttacccgacgtccatcagtcccagcctactcgaccaggtaatgaacgcccgctgttttattcgtggtgactaatgccacctaatcgttcaatcgtttcttgcttgaggtagtaaggggtaatcccgtcatcaatggccttggttaacaacccctgggcttccttttgtgcaagaatcgtcggtaccttcaaagacatgactgatttgttgataaccatttgatggacatcaacgtcagtcttatattgcaatttcttggaactttgctttttctttgatttttcggtctttcctttagccatgaaaatccctccccactactctgtatagctcaataatagcaaattcacaattgaatgtatattcaaaagcctagtcgcgatcaggaactttttcaaactttgcctggtaccattgatcccaagaacctgccttcaggctcccgttctcatcatactctgggttgatcactgaaatcacgtgtttaaggtcgtttccgcgttgttccaataaatcttttctcatctgttctggcgtgaaggacttgttttcgaaaatgtaatggttaatgtcagccaagtaatagtcaatcttgtactcagccaaaatttccaaatcatttttcttgaaccatcgaaggtaaaaatcgataaagtcttccactgcttgattggttgctgtctcatctaacttatcgaaagatactacatctgccacagtgccacctcctcttgtatttccattatgccacaaatcctgtattggcgtctaatttagtagtattattaaattgaatccaatataaacaaaggatgcggataaaatgtcagaacgaaaagtttacacagattatttttttgacgaaccagcttacaatacccatgacggcggctttgttccccttgaggaacctaagacaccgcaacagccgctgaagattccggaattgctcaagccggataaagagaccgatactgacatgtactacacggtcatcgcccaaaccggtgaagcacagctgatgcctggtaagaagaccaagacatggggctataatactgatttacttggtaaaaccattttgttcaaaaagggcaaaatgattcatattactttaaaaaatgaattacctgaactcacgactttccattggcacggtttaaatgttcccggtcccattacggatggtggctgccacgcaccggtttatccaggtgaaagcacccaaattgattttaaatgcgaccaagttgcggcaaccttgtggcttcacgctcacccatgcccagcaacggccgaacatgtttggaagggattagctacggctgtcgttgtcaaagatgacgttgaggccgcactaccatttccaagaaattatggggttgacgacattcccgtcattttgcaggatcgccgcttccacgaagacaatcagtgggattacatggccgactatgaccctgacggcgtccaggggccgactgcgatgatcaatgggaccattaatccatactttgatgtaacgacccagcggctcagattacgcttcctggatggtgctaaccgccgtgaatggcggctacattttagtgataatttgaaatttacccaaatcgcttcagacggtggtattctccctgaaccagttgattttacccatctgatgctcacttgtgctgagcgggcagaagtcatcgtcgactttggccaatacaagcccggcgatgaggtcaccttgttctgtgacgacgtgccaatcatgcgctttagaatccatgaatttgcgccggacaacaccaccttgcctgatcatctggtggacattcctgatcccgatgtcaccccaggtgcaccagtccacaaggttgttatgtctggaatggatgaagaagtcatgatgaacgggaagaaatttgatatgcagcggatcgacgacaaacaaaagctcggcaacgttgaatattgggacatcagcaacaccaacgatatgagtaacgggatggtccacccctaccacatgcacgggacacagttcagggtggtttccagaaacggccatgcgccttatccaaatgaaaatggattgaaagatacggtcggcgtcaaccctggcgaaaccgttcggctgaaagtttggttcaatcatctaggcgtcttcatgaaccattgccacattatcgagcatgaagatggtggtatgatggcgcaatttgaggtttatgatccggatcatccaaagcaatacaagctaatggatatggatactttgatgaatgcctttgctaaagagcggggcgtcaaggttgaagatctgaatattcctggaatggatatgtaagcctaattgttgcgcataattggttgacgtgatattataaattgtggaatgaaaaatgaataaagctgttaggtgaggctcctatgtggaaaatgctactgctcagaaacgtcgaaaaacgccaatgagtcagctgtccaagtcaaagtaaggcttggactaacgtagctgttaatttttaactacatcacatagtgctaaagctcaacgactggcgagaagtatttttgatgtgtccagtcgttgaacggctggacacttttcattaccaaataaaactttgaagaggtgagagttatgacagcagaatttatagacccaggagcgacgaagcatcagtctaccaagggaagcccggttgtgataactctctcacgacttaatcgttaacgagaaattgttgtaaccgatcttcccgaattgaataattgtttgacgactctaaacgttttgtttcttgcttactagctttacagctaaacgcatcacaagaaatttcccgacttcgtttgtttagatgagtcaacttttgggaattcggttaatgcaatttctcggtggtctcgaacacgttggtactggcgtacttgtgtccggtcgactactcatagtcgaaaaacgcttcaccttttaggaaactaattggggagaaatcaattaatcgtgttaaattgccacacataaagcgataataatagtaattatgaggaccatacctccaagaatccggtggaaactgattcttgaaagatgactgctatcttatcgaccaataacattataaagccgtcaacgtaaattcgttgacggcttttaatttgtcgttactttacaaaaaggccggagcaaaacattcagttttgtcccggccattatcttagcaacctatccagcttcttcgacaggttttttctttttaaatgatgcaatatatttcttggatttctcttcgtcaaactctttttcagatttaccaatgacaaccgtagcgagtgagttccccaccacgttcacggcagtccgacccatgtcgacaattcggtcaattccggcaataaaagtgagtccggtaactggtaccccgatggtcgaaatagttgccagcaaaaccacaaatgaggcccctggaacgccggccattcctttagaagtaatcatcagcaccaccagcaaagtgatctgttggccgatcgagaggttaatatgataagcctgagcgaggaacaaggcagcaatcgattgatagattgccgacccatccaggttaaaagtatagcctgtgggaatgacaaacgagacgattccttgactactcccaaatttgtccattttctcaatcatcttaggcaaaacggcttcagaactagccgttgaaaatgccaaaacaatttcatccttaatgaccagcaagagatcaaaaatactaaagccaaagatcttggcaacaattcccataatgatgagaatgaaggctaccatcgtggcgtaggcaatcgccacaaagtagccaagtgggattaatgcaccaatccccatttcagccaaggcaactccaatcaaagcacagactccaatgggtgcggcatgcatgacccagttagtcactttaaacatgacttcggcaactgcattcaaaccgtcaattagaatctgtcccttttcaccaatggcggcaattcctaaaccaaagaaaactgagaagaaaatgactggcatcatatccccatttgctagggacttgaagatgttggtgggaataattcccagcagtgtcccccagatacctgtatgctgagcagtcttggcggtcgccatatattggctgatatcagatccgtgcagcgagtgaatatcaatcagtgtcccaggatgaaggacgtttgcgacaaccattccaagggcgatggcgatggtcgtcatcaactcaaaatagataatcgtcttgagaccaactcggccgagcttcttaatatctcccatactagcaattccaactgttaaacatgaaacgacaatcggtaaaacaatcatttgaatcaagttgataaacatggttccaatattctgcatggccgttatcgcggtattgtttttgtagaagatcacaccaaaaaagacaccaagtaatagaccaataagaatctgccagccgaggctcagccggtaagctctgtatcgtttcataatttcacccattttcccaaaaatatgtactatttcaatataaaacaaaagccttcaatagtaaataccattgaagactttctaaattgcgtggcaacgtcctaccctcgcagggggcgatcccccaactactcttggcgtgcagaagcttaacttctgtgttcggcatgggaacaggtgtatccttctggctatcgccaccacactatttttccttgaaagaacttcgttctctcaaaactagctaatattaattttctgcccttgaacaccatttctacttggttaagtcctcgaccgattagtattggtccgctccgtacatcactgcacttccacttccaacctatctacctgatcatctctcaggggtcttacttccatataggaatgggaaatctcatcttgaggtgagtttcacacttagatgctttcagcgtttatctcatccatacgtagctacccagcggtgcgcctggcggcgcaactggtacaccagcggtatgtccatcccggtcctctcgtactaaggacagctcctctcaaatttcctacgcccgcgacggatagggaccgaactgtctcacgacgttctgaacccagctcgcgtaccgctttaatgggcgaacagcccaacccttgggaccgactacagccccaggatgcgatgagccgacatcgaggtgccaaacctccccgtcgatgtggactcttgggggagataagcctgttatccccagggtagcttttatccgttgagcgatggcccttccatacggtaccaccggatcactaagcccgactttcgtccctgctcgacctgtctgtctcgcagtcaagctcccttctgccttttacactcgttgaatgatttccaaccattctgagggaacctttgggcgcctcccttactgttcgggaggcgaccgcccaagtcaaactgcctacctgacactgtctcccgccacgctgagtggcgcgggttagagtgttcacacagcgagggtagtatcccaccaacgcctctgccgaaactagcgttccggcttcaatggctcctacctatcctgtacaagctgtgtcaacacccaatatcaagctacagtaaagctccatggggtctttccgtcctgtcgcgggtaacctgcttcttcacaggtatcttaatttcaccgagtctctcgttgagacagtgcccagatcgttacgcctttcgtgcgggtcggaacttacccgacaaggaatttcgctaccttaggaccgttatagttacggccgccgtttactggggcttcatttctgggcttcgccgaagctaactcatccacttaaccttccagcaccgggcaggcgtcagcccctatacgtcatcttacgattttgcagaaacctgtgtttttgataaacagtcgcctgggccttttcactgcggctgtgcttgcgcacagcaccccttctcccgaagttacggggtcattttgccgagttccttaacgagagttcactcgctcacctgaggattctctcctcgactacctgtgtcggtttgcggtacgggtagttgatgactcactagaagcttttctcggcagtgtgacgttggttgcttccctacttaaatttcggtcctcatcaccacttgtcaacccgccaaaaagcatttgactctttgactgactcgtggcttgaacatccctttccaactggatgcacaacttagcctcctgcgtccctccatcgctcaaacatcatcaactagtacaggaatctcaacctgttatccatcgcctacgccttgcggcctcggcttaggtcccgactaaccctgggaggacgagccttccccaggaaaccttagtcattcggtggatcagattctcactgatctttcgctactcataccggcattctcacttctaagcgctccaccagtccttacggtctagcttcattgcccttagaacgctctcctatcacttgaccgaaggtcaagtccacagtctcggtaatatgcttagccccggtaaattttcggcgcggaatcactcgactagtgagctattacgcactctttaaatggtggctgcttctgagccaacatcctagttgtctatgcaactccacatccttttccacttagcatatatttagggaccttaactggtggtctgggctgttccccttttgacgatggatcttatcactcaccgtctgactcccggataaaaatcaatggtattcggagtttatctgaacttagtaacccatgacgggcccctcatccaaacagtggctctacctccatgattctacgtccgaggctagccctaaagctatttcggagagaaccagctatctccaagttcgtttggaatttcaccgctacccacacctcatcccagcacttttcaacgtacacgggttcgggcctccagtgcgttttaccgcaccttcaccctggacatgggtagatcacctggtttcgggtctacagcaacatactaaaacgcccatttcagactcgctttcgctgcggctccggcttttaaaccttaacctggcatgttaccgtaactcgccggttcattctacaagaggcacgctatcacccattaacgggctctaactgcttgtaggcacatggtttcaggaactatttcactccccttccggggtgcttttcacctttccctcacggtactggttcactatcggtcactagagagtatttagccttgggagatggtcctcccggattccgacgacgtttcacgtgtgtcgccgtactcaggatcctgaactgagggtcattgatttcacctacggggctatcaccctgtttcgccaaccttcccagattgttcgattatcaacaactttggtaactcaaatgttcagtcctacaaccccaatgagcaagctcattggtttgggctgttccccgttcgctcgccgctactgagggaatcgaaaatttctttctgctcctgtgggtactgagatgtttcagttccccacgtctacctctatacagctatgaattcactatatagtaacagtcgattaaaactgctgggtttccccattcggaaatctccggatcaaagcttacgtacagctccccgaagcatatcggtgttagtcccgtccttcatcggcttctagtgccaaggcatccaccatgcgccctttttaacttaacctgtacatcacgacgtgatgcaaagttaattgagtatttgcgattttttctagttaacaaactcaaaataacgcggtgttctcggttgaaattatataaaatacaatttcaaaaaattattacagaaaattaatattatctagttttcaaagaacgaattgagagtagacctctcaaaactaaacaaaactttcgacaatgtgcaggattccgtttttccttagaaaggaggtgatccagccgcaggttctcctacggctaccttgttacgacttcaccctaatcatctgtcccaccttagacggctggtccccgaaggttacctcaccggctttgggtgttacaaactctcatggtgtgacgggcggtgtgtacaaggcccgggaacgtattcaccgtggcatgctgatccacgattactagcgattccaacttcatgtaggcgagttgcagcctacaatccgaactgagaacggctttaagagattagcttgacctcgcggtttcgcgactcgttgtaccgtccattgtagcacgtgtgtagcccaggtcataaggggcatgatgatttgacgtcatccccaccttcctccggtttgtcaccggcagtcttgctagagtgcccaactgaatgctggcaactaacaataagggttgcgctcgttgcgggacttaacccaacatctcacgacacgagctgacgacaaccatgcaccacctgtcattctgtccccgaagggaacgcctaatctcttaggttggcagaagatgtcaagacctggtaaggttcttcgcgtagcatcgaattaaaccacatgctccaccgcttgtgcgggcccccgtcaattcctttgagtttcaaccttgcggtcgtactccccaggcggagtgcttaatgcgttagctgcagcactgaagggcggaaaccctccaacacttagcactcatcgtttacggcatggactaccagggtatctaatcctgttcgctacccatgctttcgagcctcagcgtcagttacagaccagacagccgccttcgccactggtgttcttccatatatgtacgcatttcaccgctacacatggagttccactgtcctcttctgcactcaagtctcccggtttccgatgcacttctccggttaagccgaaggctttcacatcagacctaaaaaaccgcctgcgctcgctttacgcccaataaatccggacaacgcttgccacctacgtattaccgcggctgctggcacgtagttagccgtggctttctggttggataccgtcaagatgtcaacagttactctgacacctgttcttctccaacaacagagttttacgagccgaaacccttcatcactcacgcggcgttgctccatcagactttcgtccattgtggaagattccctactgctgcctcccgtaggagtttgggccgtgtctcagtcccaatgtggccgattaccctctcaggtcggctacgtatcatcgccttggtaagccgttaccttaccaacaagctaatacgccgcgggtccatcctaaagtgacagccgaagccgtcttttaaaccaaaaccaggtggttttggttgttatacggtattagcacctgtttccaagtgttatcccctacttcaagggcaggttacccacgtgttactcaccagttcgccactcgtctcaatgttaaatctttcaagtgcaagcacctaaaatcattaacggagacgcgttcgacttgcatgtattaggcacgccgccagcgttcgtcctgagccaggatcaaactctcatcttaaattgtttaaaatgataagcctgtgatagctcatgatttaaatttattatttgttttacgaattgacttcgcaaatgtttggttccaattccgaagaattgaaacgccctgcacatttgtttgtcgaaaattttgttcagttttcaaaggtctacatcagaacacaaacatttttggcgaataaattaaaatcgttcgtttattcaaatccttgtgccccttgcctctaacagcaagaataattatataacagccaatctttcaagtcaacaaaaactttttaattagcaattggtatatgtgttcatgtcattgaagcaacgagtaatatactatcagctatttcggccgaggtcaacaggtaatttcaaattaattcaataaatcgttgctgacaaagcttaaagattgttaataccgggaacaaatcctccccgcaaacaccatttagcctgtatactggcaattgaaatcttcgcgaaaggaactgtcatcatttgaagaaaattgtaattatcgatgccaaacgatcagccatcggcaaattaaacggctcattatcttcattaactgccgaacaacttggttcaaaagtcacgcgtgctttattaaaagatgctggtctttccggcagccaagttgatcaagttatctttggcaacgccatccaggccggaaatggccaaaacattgcccgacaaatcgaattgaacagtcagattccagaaagtaaaacagctttcacagtcaaccaagtctgtggatcaggactacaggcaatccatcaagcacaatccgccttgcttctcggagaagcggaaacggtcattgccggcggaaccgaaagcatgtccaacgttccttacttgaacatgtcacaacgaaagacaaccaagtttgggccggtcacattatatgatggactgcaacgagacggcctaaatgattcagcgacggatgaaccaatgggaatgaccgctgagaacgttgccgatcaataccatgtctcacgtgaagaacaggatgcttttgcattgcgatcacatcaactggctgcgcaagctactgaacagcattattttgatgatgaaattattcccattgaactcaaccaacccaaatcacacgctccccacatcgtagcgcaagatgaatcgatccgggtcgacacaaatttggaaaaactggccgcccttcgtcccgcttttaaaccgaacggatccgtcactgccggcaacagtgcaccactaaacgacggggctgctgctctgatcatgatgactgaagaccgggcaaaccagttgggactatctccaatggcagaggtgctgggttacgccgagcacgggatcaacccggaagtcatggggtatgcgccctacttagccattaatcaattggtatcccagctcaacatgtcagtcaacgacattgacctctatgaaatcaacgaggcctttgcttcccaatcagtagcagttgttcgtgatttaggtatttcacttgataaagtgaacattaacggcggtgcaatcgcactgggtcatcctctcggagattctggtgcccgcatcgtgacgacgttattgcataatctgcgccggaccaaccaagaatttggcgttgcctctctttgtatgggcggcggcatgggatcggcgctggcaatcaaacttctttaatcacaaaaaataggaccgtaggctaaacgctgacaacgtttgacccacgatcctattttattttaattaagttttatctgttcatcttcaggtaagtggtctttaaacgaagattgatacagccaataataaacccgcttggtggcttttgacatctcagcatacgccgggttgatcgatttaacttccggatagacgcgcattaaatgactgaaggcactgaagcttccagcagcagacatcccgtcgtcgtccttcttccctcgttgaaccaggccaattaattgatcaacctggaatctggccagggcgtccacataatcaaagagggttccggcagcttggaaactcggctcaatcacctgccgtgacgttgtgtactgtccggaggcaatttgggtcaacaactgatttctgctcatcgtatattgcaccatcaatggcgttaaaaaaacattctgtagaatctgatgagtggtttcaaaaatcccataggctaccttgaccgtttcaccgcgatcattcacctgtggccggtcattttccagcacccgactgtaccgcaattgatagttctgatgtttggcattcctggcactgccggcgttacttaaattcaatacagccaacttttctgccagatcagcacctgattgaggtaagttcaaatatttcccaattgcctcaactgcggctttggtcttggcaagaaccgttgcctgatcagtggcactggtgaccggtgcaccgactaaatcgggattattttgagtgaattttgcgtaaaccaacggatataaaccgattgatcccagggaattgaccattcctgccaacgtgttgttgacaaatagattaatatcttctgtcagcgaaactttgccgattgcatcggtcatcatcttgggtaaatcgtgctcgtcgctaaaatcgtcttcattataggaataatttccgagcagcggctgttcatcattgccgactggctggttgcttaaaaagccatcgctaatttccttggcaacgccggtggcgatcgtctcatcggcggccgatggcttggtcgtttggttattgatcgctttaaatggtgaagcaccgttcatatagccgttgacgtggtcaaaccactgattaaccagggtccgctgttgattgagatccaggttctgcaaggcagagttaattcggaaaacaacgccaccggcgccggcaatcgcccggacaaattgaatcaccgctgtcttataaccaacaacgtacttttcgggagcctggctctggcttaagtactcagaaaattggttcccggctgcccggttgacgactgaactgtcgtcatctccggtcgcccacagtgacatatagttaaattgatcaatgctgacatgttttaaatccttggcggctgccaaataccccatctgcattggtttggacattttaaactctgccaacgaaacacttggctgcagcggaccgggcaaaaacgaccgcaagccccgggtaattcgttcagaatagattgagcttttagcgtaagtattttctcccagcacttttgaagtcattaaccccagcatgctgagaattttttgttgtttcgaacgggtgtcggaatcatttaccgacgaactggccttattcatgtcgaaaccaccccctagtattatgactataatatcataaactatggcgaatcattgccaacaaatggggaattaaccattctgaaacaattttcaaatctgaggcgttatttttgtgattcattcaaaaagtttgtatgcttatggtagagataaggaaagggtgtgaaactaatgggaaatctgaaaaacaagtccgatgaagtcatcggcaaagtcaaagaaaccgttggcgacgtaaccggaaacgacaagttgaagctgaagggcaaggctcaaaagacatctgggaaagccaaagataaggttgaagatgccaaggaaaaggcgtccaagaaagtgaatgatgctttggacgacaagaagtaaaatcaagctgttaaataagaaacccgatacctgcgaatcgcatggtatcgggtttctttcccaaaaaatgagaaagtaaaactttttacatgttttgtattgcatgccaaataatattgttctataattcactctcgtgttattttgatctaatcaattgaattagaaatatgaacggggatgtgaatcgaaatgtcagcaacttatttgcgtcaagcaaccaatgcagaccttccagaaatcaaaaaaattattgaagaagcaaaagcctaccttaaaaagcaaggcatcgaccaatggcaggatggctatccggccaccgaagacttggagtttgatgtcaacaacgggatcacctacgtgttaattattgacggccagatcgccggaaccgcagctctccaccaaggattggatgtcaactacctcaacattcacgatggcgaatgggtcaacggcgtccacggccgctataccgccattcatcggatcgccatgtcgtcgaatttccgcggccagcacctttcccaaaagatgatcagcggcttaatcaccatttccggtgttctgggttacaaagatatccgaattgacacgcatcccgacaacttgggaatgcagcacgtgatcaccacaaatggatttaccaaacgcggcacgatttacatggctgaaaaagaccgcgaagcatcccctcgttacgcctaccaactggttattgggtaagcgaacaagttggagtacaatatggttaatgaggtgataatatggcacaagatgatgctgccgtaaagaccgcactaatcattatgtacgttatcggcgtggtttgtctgggaatcacattcttcctactcgataaagtcaacggaaaatggtttaccaagttctcagtcggccttgtcggggtgattttagtaatgggaattatcttagtcaatgtgattaatctaaattaaagagtgggaccaaggcgttttgatcccagaatttaagcaaataatccggttattcctgtctttggaatagccggattatttgcttaaatggccgggatcagccgattgtcgcgcgtttaaacgagataacagaggaataaaaacaaacgggtgagacaacacaaattgtctcacccgtttgttttatttaaactaaatttgttggaatgcctgatccaaatcagcaatcaagtcgtcagcgtcttccaggccgacggacaaacggatcaattcatccttaatgcccattttcaggcgctctggcttgggaatctcgaagtgtgacatgaatgccggcacttcgaccaaactttcagcagcgcccaaactaacggccagaatgatgagctgaaggctgttgacaaacttggcagcgtccaatccgggttggacttcaaaggagagcaccccaccggcacctttggcttcatcactgatgatttggtaatcctgactggctttgtcaacagttgggtaataaatcttggcaactttgggattactttgcaaataagcaatgattttctcagcgttttgaatgtgccgatccatccggatgtttagggtctgaataccacggcgaagcaaattggcttcttgaggtgccaaaaccgcaccaatggtattttgaatcgcataaatttgatcgctcaaatccttggttttggtgacaatcatccccgccgtaaagtcagaatgaccacccaagtatttagttgccgagtgcagcaccacatcggcgcccaagtctaatggacgttggagatagggtgtcaaaaatgtattgtcgacaaccaccaaggcattgtgctggtgagcgatttgagaaatctgcttgacgcttgaaaccttgagtaacgggttagtcaccggctcgaagtagacgcctttggtattcggtttgaaagccgctgccaccgcatcagcatcttgggtatcaacttcggtgaattccaacccacgcggcttcaaaaaatcattcaccagtcggaaagtcccaccgtaaatgttatcgccgataatcagatgatcgccaggtttaaagagcgccaatgccgcatgaatcgccgccatcccgcttgaaaaagcaaagcctcggtcaccgttttccaatttggcacacacgtcttcaacggcatctcgagttgggttgccggaacgttcatagtcccatttaacatccgcccccagcttggggtagcgaaaagttgatgagttgtagattggcacgttcacagctccggtggagttgtcattgggacggccgccgcgaaccagtaatgtattaaatttaaccattaaaaaatctcctatctctccaaagtggtggtgctacttaacaggaaccaattgatctgatgataacagatacagatatttctttgtaaccggcctgccaaggatttgatccaaagcagtcgcgtacaggcggatctggccgtcataacgttcatgaatcgtatcaacggtggtcttcggagtcagtcggtcagtcttataatcaaacaacacgacacccgcctccgactcaacatagccgtcaataattccgtggatcaagatcggttgatcatcatcttggtcaaaatccttgaaggcgtttttagccttcatcaatagagaaaacgggacttcgcggtaagtcgtctctgggttagccaaaacaaccgcgcccagagatgacgcataaaatctcagaatcccgtcaacgttaatttctccggcaacattctcttccagaataccttccttcaccaggttggcaatcagctcaacgatagtggcctttgtcggctgttggtgtaaatcaacctgctgcagtaccaagtgggtcgctgttccgacctcagtaggtgccggtttatgggtaccgttttccgaaataaatttcggtgttgccaggctgggttgggtgtagcggccgggtttaatcagctgatcgctgtcaattagcgaataattgcccagctggacgttatcgggatcatcgaacagccgcttaatttcggaaacggattggtaggctgtcgtgcgagttgctgcctggtgtgggtaacggaaattcatgatggccttaatttgtcggcgattaacgtctgaatcggattcgaccggctgctgctgatcgatccagctacgaggatcaactgctgcacggccagcctgcttctttccttcagccaccttggcattgtcataaaatttcaggctcaaccggctggggtcatcggcaagcaggttgacaattcggctgtcgccataatctttaatcacatccggatgacgggaaattgccggaccaatccagtccaaatagcttttggcgctgttgcgctctgccattggcaataagatggccgattcttcagtctgtgactgccagctttcaacgatcgcctgcaaatccaacgttggtttgcgagacccgccttttcctggatcgactttaccgaccagaaagagccgctgttcagcccgggttaaggccacgtagagcttccgcatttcttcagacaaaccggcattcttggtcacatccaagacggcctggcgctgcaaaggttcttgaatctcccgggtttgggtatccaaataagaaataccaattcccagatgatcattcaacaccgcacgtcccgtagtgtcctgctggttgaattgtttaccaatatcattcaaaaagacaatcgggaactggaggcctttactgccgtgaatcgtcatcacgtgaaccatgttgtcagatgtattcggcaccgccgtggctaagtcgtcatccctagcctgcattcgctcgataaacagcacaaatctgaacaaacccttaaaaccattcttctcgtagtcaaaggcccgctcatacaaagcatgcaggttcgtctggcgctgataaccgcctggcatcccgccaacataatccaaatagccggtttgcttataaatttcccaaatcagagcaaccaagccgtcttgtttggcaacgtttttaaaatgatccagctgcttgaacaaggtgtcgattaacggatagatcgtctgagcatatttgttgggttcagcgttgggatagtcccggtaaaatttcaacaccgactcatagtaattccctgtcttttgattaattcgcaaataggccagctgattttcatccaaaccgacgatcggcgaccgcagcacggctaccaaggggatatcttggtaaggattgtcgataatcgacagtaatgacagcattacctgaatttccgtggttttcagataactcttggcaccggtaatttcagccggaatcccgtaatctttgaaaattgaagacatggtaatctggctgccccgggttggcgaaatgacagcaaagtcaccgtagtcaaccggtcgatcgccatcgccatccgcaatccgttcgtggtcatcgaccatctggcgaatcttttgggcaatgatttcaacctgtccttcatcggtgtccataacttgctcggcaggaaggtcttcaccctctgatagcggctttttagggctgtacagcagcaccgaaacgtcagcatttacgtcttttggataatacttggcgccaaactgcagcttggcatctgagtagtcaatttcgccaacttggcggtccatgatctgctcaaaaatcaggttaacgaaatgatcgacgttctcagttgaccggaagttatcggccaaggtgattaattcgttgtcattatcagccagcgaataggtatgctgcttactaataaacatttggggatcggccagccggaagcgataaattgactgtttggaatcccccaccatgaaccggtttccgccgccttctttagccagtttattcaaaatggcgtcctgaagccggttattatcctgatattcgtcggtcataatttcataatactgatcccggagctttgcttgaacttggcgggcctgtgggctgtcgtcattcaaaatccggtaagcagcctgctcaatatcgatgaattccatcaaatggcgctgatgcttggttgcctcgtaagcggttcgaaaggctttgaccgctgaaatcagtttggcaacccgctgcttggcggctgccatcaggtcaacgttggcctgttcgtcgataccgaaatatttattgcaaaaggcattgaagtcttttttggtttgttgattaattgcgctaatttggccatgaaactgtttttgttcaccctgcggtttggttagccttggcaaatcggcaaattcgaaaccagtcagtgacttgcggacatcgtcaaatgatgtgcaatttaaaaccactttttgaagggtctcaatggctgccagctggtcagtgaaagctttttcgtccttatccaaggcaccgctttgggccaatttaatcatgtattgatgattgattttgagcttggtaaatgcttcagcaatctttggggcaacgttttgttgatagaaatcactgtcatacaatggtttgccaccgagatcataaaaatcggtgacagcattcagccaaccatccggatcgtcggtaacgtttgcgaactcgtctaatcgataaatgagatccgctaagccgtcgtcactgcggtcgttggaaaagttctccgtcaaccgcgcaaatgagccatcttcatcgttgccatataggtcttctcgaacggctccccaaacttgatccttgagcaactgtttttcagtatcgtcggccaaaatgcgaaagttgggatcgattcccaagagatagtagtatctgccgactaatttctgacaataagcgtccatcgtcgtaatgtcggccaccgcgactttttggatttgggtgagcagccggcccttttcggcttcagctgcctgattaaattcttctcggagggctgcctgtagtcgttggcgcatttctttggcagcggcgttggtaaacgtcaccactaacagttggtcgatgtcgacatgctgatttttgaccatgtcaataattcgatcgaccaacacccgggtcttcccggatcccgcagaggcggaaaccaggacattgcctgccgggcggtctttaattgcctttagttgatcaggcgtgtattcaaatgccatcggacttttcctcccctaattttttcttaatatcgtcaatcgaatcactgttaaccggccggtactggttacccggcaaaattgggtcaaagttcatgattgatttgtacggggtaaactgcatcccggtggtttgaccctgcttaaacggccacagtcgaacgtcaccggcaaaaatcttttctgccgcatcgacaataagtttctcagtgtgggtgagaaacgcatccaattgcaatggattaatcaatgattttttaccagtgtagcctttggcggtctttctaattgggtaaatcggtgagtagccgctatccagctcctcatccaaatgatcaatcaagccggactcgtcaaccaaaatgccgttatagcgatgcttctttaacaaggcatcgtcaaaggtcaccttttgaaggtcctcgggtttgaagacggcattataaatgtgcaagtacaacgcgccggccaaagcgacttccttatcgtcgggattaagtcgttccagattgtgttttaaaacatccagatacgtcaacagctgcattgacgtcccgtcgtaagctgcattgaaatcaaatttgcggtcagaggacttgtagtcaacgatcccgaagtagcgtttgtccttggtggtcatcgaatcaattcggtcaattctgccccgaactttaacctgatgatcatcagccaaatcaaagctcagaccattgagggcctgcttttgattgggctggccaaaaatcagttcggtattttgcggccgcattggcgtcagtttctgttggtcacgcaaggctcggatcatctgctggatggtcgcggctaattgcatggaaatataatgcatccgattggaactggtcagcacaacgtagtcaaagttttggggatcattgatgattcggtcgacggtttctttgacgaggtcgctcacatcttgatcggataagctggccaaatcaatgttttgggcatgaatctgcttaataatccggtccatggcgtcatgataaaaggtcccagtcgatgccgtcgacagctcaaacttcggtcgttcctggagttttaacccatatttgaggaaatattcataggggttcttatagaaggtttccagttgagaaatcgaaatatttagttctgacccgtatagatctgtaatgatttcaggagccaatgactgcggcacatttgtgtaattaatgctcttaagcagcttggccgtctgccggttgacttccggatcccgctgcaggtactgcaaaatcactgcccagccggcactcaagtcctgatgaatatcaaagtgattttgaatgacttgaatcaaatggtgaagtgtcccgcgcttggtgcccacgtatggcatcacgtcgtgctcatcatcggggatcgccgggttgttgacgattttgaggttaaagaaatgctgaatccgtgaaacataaggtgaaagtttcacagcggattcgtcgtttaatttgttggtgtaggtaaaaatgagtttatccgaagcggtcatgaaggccaaatagttcaagtatggttcaaaagccatttggacttccgcgggatcatttaaatactgatcgtcactgagattgctttggagttggttgatgtcgtcatcgccaaagagattttcattaactaggcgatccggcatgttgtcatcgttggcgccgatcatgaacgtgactcgataatcattcatctgaaccatgccgctttcagagacgctcacttgatccagcgtggacggaatttgtgaatagtccgctccttcaaagccggcatagatgagtgaccaaaaatcgccgggcacaaacggtttgtcccccagaatttggacgcattcgtccagtagagaacaaaatgtccgccaaacctgttcgatttggttggaacgattgatatcgccctcgtctgttgccgcatcccgccagtcctggagccggtcaacaacgccggcatccactagaaactggtagagaatttgagcagcttcctggttggttttagctttgaaaaattgtttataaaaactgggtaataagtctcgcaccaggtggcgaatgatattgattttgcgggaaatttcccgatcttggtcagtgatctttgtggtcgtctgttcttcgtcgctgtccggcagccaaacgtactgccaatcagccttttgtgtccagcgggtgtcggcgtaatcgtttttcagcaccaaattatcggtcaaagacaccgcttgacgataatcatcgattgccatcggcttgccgtcaatcatcggtaggactaattcagattttaaaaaccgcatcacgtcatcgtaacggtaattgcgggctcgatttggatcgtagatatcaaataacgctgctaataattccaccagcggatggtcagccattgactgctgaatatccttgaaataggggatctgctgggtggtaaacaccggctctaaaatattttgatatgcgtctaaatggcgggtcaaaatgagaaaatccgagtaccgatatttaccggtggcaaccatttgatgaatcttcgtggcaacttggtccagttcagagtaaaggttgtcagcttgataaatttgaaccgactccggggaaatttggtcaggcagttgatgagtcccgaggctgctggacgtgatccagtacgcctctaatttttgcatatcttcatcaacccgcggctggtcagccatgacggcctttaaataaggcacccggttgtcagcggcaaatcgatagagctgatggaacaatttagccggctgaaagaaaatattcggctgttccggcagttcagttgggtatggccggtccaacgtcaatgacaccgtcaccgaagcggattgattgatcaaggtttgcaccaagccgcattcctgggcagtaaattttgaaaaaccgtcaatatagaagtgatagccactcaaatcaatgtcctgcagtttgctgctcagcaggttcaagacggtgtggctgtcaaaatagttctctgaaatgcgtttgacatattgggaataaataattgaaaaatcgtggagtttatcgcgcagatcattggtaatcgtgctgtcaggccgctgcagcatttccaaaagatcttcaggcaagacatttccggcctgcatctcggcaatctgggtagcaatctgatcaataaacccaggattatgaatttcgtggtcaaagagcaccaattgatcggcgttatcaacaataatttggtacagcagcatactgataccggcactgctgatccgctgcttttgatattccggtgtgttgcgcagaaagaaccacgctaatcgggtgaaggataacacctgaacatcactttgagcagtggtcatttgattggcgtcgccaagttgttttaaaatactgacttctgattcaaacttaatgtggtttggaaccaaatagaaaaattggtcgtgtggattgtctgatttttgctggcgcagaatatcgatcattttcgattgatgatcgacacctgcttgacctaagacaaactgaagggtcactgctctcacctctttaaaattactttaattttaccatagtatattcctcatgtttgatgaagattgacgtggatttcttcagcgaagcaaaccgccaatcgcacgcccagcaagggattagttgggtatcaaaatgatttgtgaatttccggaacattatcattgaacattaacaaaaagggtctattatgagggttggatgtatcttacatccatctatttgacctaaatgaaagctttatgcttgcattgatcttgttagagagcctaccagtgcattccacgattaagtatcggaagcaagaatttacgatctacccccaatatatctttcaagttcaaatactgataggccctactcctaataacgcccggtgaaaactgggtgtacataaagaacagagtgcggaacagaccggttagactccgagcattagcagaataatgagttttaatgctgaaagcgttgaaactcattattgggctaagcggaggagtctggcttgtgtagcacatttccactatataagagtaaagcttcaaactttgatgcgctttttgcatcaagactcattgttggataaagcggaagaagctggtctgtgtagcacctttcaacagagtgcggaacaagccggttagcttcggagcattaatttgataaccagttttgatgcgtatttcgcatcgaaactggttatcggattaagcggacgaagctggcttgtgtagcacctttccactaaataagagtaaagctccaaattttaatgcgctctttacatcaaaactcattgttaattaaagcggacgaatctggtccgtcggaacacatctttgccaactaacagtcacacaccacaaaccaaaatacattaaaggaggcagccaacacggttgcctcctttaataaaggtatcgatgcaaagaacctaagcccgcaccttattttcttccatcaccttattggtataaaactccaaatcatcgactgcctgatcatcctgatccccctgagcagtcacagcgtggagattctgctgggcaaccgcccaataaaccaggttggtggtaatcggcagaatgtcccgaatgacgtgaaagtcgaaattatcgccatttgtggatttcatattcaaaaagttattccagtcggtcaccatattgacaccactgtgttctttcttcgagaccgcagaaatgatgacgaagtgggaattgcgatttgcttcttccaactgattttttagctgttcaatttgttctgcttccagtttaattgccattctatcactctcccatcggtgtttgatcaataattccaattgaatgattcattaatttttgctcgatcagcatttcataagccagcttggcaaccgcttttggagataccgttttagccggcatcggcgttccttcattaaacagttcatagtcgctggcctgctggtcctttaattgacccattctaattatagaatacgcaatttcggattcatcgacaatcttgatggcatatctttgctgttttataaattcttgggggtctttcacgccagcataagtgactgactcattcagctcgtcatcaacgccggcgtatgagagcatcacaatatcactgattggcggctgaacctcatcgaccgcctcaaagagcgcttccacatagaggtcggcgtcgttgggaccaacggcgatgaaaagtaggttggtatccggcaaggcttgagcatagtcatttgctgattccaaattacccgaatagacctcgacagaaatgtcggagcgttgcttaagtaacgcgtttaacggtgacaccacggggctattttgattaatgattaataattttttcaaatcggtggcttcctaatctaaatgtttttcaaattgtgcgtaatggaccataattaatgtgtaccataataacaatggaaaatcaaaggaggacgtaaaaatgtcccaaaaagttaaaattggtcaatcagacgttgtcagcaccccgttaggctttggaaccaacgctgtcggcggtcacaacctgtttcctaatttggacgaagaggccggcatgaattccgttcgggcggcattggatagtggcatcaccatgctggataccgcatttgcctatggcttcggtcgctctgaagaattaatcggcaaggtgctcaaagactatgaccgctcaaaagtcgttgtggctaccaaaggcgcccaaattgtgaacggcgatcaggtcaccatcagtaaccgaccagccgatctcgagaaatttgtgaaggacagcctcaaccggttggataccgattatctcgacatcttttacattcacttccccgatgatcaaacacctaaggcggaagccatcgccaagctggccgagctgaaaaagcaaggactcatcaaagcgattggcgtttccaacttctccttggaccaactcaaagaagctaaccagaatcacgatgttgatattgtggaagaccagtatagcctggtccatcgcgatgctgaaaaagagctgttcccttatctggagcaagaacagatttcctttgtgcccttcttcccactggcatccggtctgctaactggtaaatacgatggtagtccagttaattttcctgaagatgaccttcgaagcggcgaccccaacttttctggcagccgtttccacgccatcacgcagtcagtcaagaacctgcagccaattgcagacaaccacgatgccacaattgcccaagttgtcttagcttggtacatcaagaatcctgacatcacggttgtcatccccggtgccaaaacgccagagcaagtccgcagcaatgccaaagcaatgaacgttgccttatcggatcaggaatacaatacgattgataacgcatttagattctaatccacatctaaacagacatctaggccaccaatgtttagcgcaaatttctttgccaaccgcttcaatggtcaggccttgatatagaaatttttttaaatgcatttgtgacccccgcttaacggcacatggtatactcaagttggatcggagagcgcttacaattaagttatggggggcctcctttatgaaccgtttagatggtaaagttgcaattattactggtggtgttagtggctttggtttggcagctgccaaattattcgtccaagaaggtgccaaggtaaccattaccgatgtcaatgattccaaggctgagcaagctttaaatgaaattggcaaagacaaggcgatttttgttcaacaagatgtttccaaagaagccgactgggatccggttttccaaaagacgattgaccagtttggcccagtgaatgttctgttgaacaacgcaggcatcttaatttttgacgatgctgaaaccgtcgacatggatcaatggcacaagattttatcagttgacctggatggtgtcatgctgggagttaaatatggcatcaagtatatgaaggaaaaaggcggatcgatcatcaacctggcatcaattgccagcctgatcgggatcagcaacctttattcctacaatgcagccaaaggtggcgttcgactcatcacgaagtcggctgcgctatacgctgctgagaaggattatccaatccgggttaactcaattcatccagggtatgcccacacaccaatggttgattcttaccctgaactcagacaaaagctcgagagccttcacccgatgaaacgactggcagatccaaaggaaattgccaacatggccttgtatctggcttcggatgaatcatcattctcgactggttccgagttcgtcgttgacggtggttatacagcacaataattcatcgtggtttgaaaattcctgacgaccgtccaagtgattggatatgccgatcaatctaactcacaatatgaattctctattaactgcttgcgacaatcatcgtaagcagtttttttgctgagaaatttatgtaaccagttgcataaatgcttcgacataacggtaaacgttttgttactttttgttaatttaattcgtttattgaacccttttaatgataatgctaaaataaatatgtaattttttattcatacacgaacgatagaaggagctattatatgttaaattcaattgccaagtatttcgagtttgatgagcgaaatacgaatttccgtaaagaaattatcgccggaattacgacgtttgtttcaatggtttacatcttgttcgttaaccctaacgttcttggagtcagcgggatggacaaaggggccgtctttaccgcgactgcccttgcttccgcatttggctgtttcatgatgggcttcattgccaactacccaattgcgatttctgccagtctggggatcaatgccttctttgcctattcagttgtgattggcatgaaggtttcatggcagactgctttagccggggtcttcgttgcgtcagttatttttatgattttgaccgctttgaagcttcgtgaaaaaatcatcgattccattccagctgacttgaaagctgccatcggtggcgggattggtttattcattgcctttatcggcttgagtgacggtggcttggtcactgccaacaaagacaccttggtgagcctaggatcgttacacgtcgggacaacttggctgacgatcttcggtctgttaatcaccgttgttttgatgagcatgcggattccaggtgccatctttattgggatggtcctcaatgctattcttggaatggtgaccgggttgattccattaccccatcaatgggtttcttcgattcccagcttaaaaccaacttttggtgttgccttgtcacacattggtgatatcaactcggttcagttagtcgtggtcgtcttaacgttcctgctggtaaccttctttgataccgccggtacgttggttggtttggctgaacaagccggatttattaagaataacaaaattcctcgaatcggtcacgcattaattgctgattcttcaaccatgttagttggatctgttctgggaacttccccaatgggcgccttcgttgagtcttcagccggaatcgccgttggtggtcgaactggatttactgccgtcatcgtcggaattctgttcattttaggtactttcttctcaccattattgaccgttatcaccagccaagtaacggcaccagccttgattatcgttggtattttgatggctcaagcactgaagagtgttcactgggaacaatttgaaattgccgccccagcattcatcacacttgtcggcatgccattaacctacagtatcgccgatgggattgcccttggatttattacctacccaatcacgatgatcgccgctcgtcgtggcaaagaagtcagtgccatgatgtatggattggcggttgtgtttgtgattttcctttggatactcaacaattagagcgcgacaagggctgaaagaaacacttaaagaatctgacaaacatgttctcttgcaccaaattcaacccttcagaccaaaactattttgacctcgcaccccaaaagcggtaaggtataaaggttgtttaacaactgaatatttaacaaggaaggaatttgttatgaattctaagactaatttgtttggcatcagcaacgttcgtgacctcacgaaagccgctgttgtatctgcactctacatcgtgatcacgatggtctttgcagccttgagttttggcccaattcaattccgcttttcagaaggtttgaataaccttgctgtcttcaataagcgttacgttgtggcgatcacgctgggatgcttcatttcgaatatgatgtcgtcactcggaccactggacatggttgtcggaactggtgaaacgctgattgcgctgttgaccatcaacatcgtgacccggttcatcaagtcactgccattgaagctggttgcatccgttttgatcggaaccttttacatgttcatcgtggctgcagaaattgcttatctcggaaacaccgccttttggccgaccttctggggtgcatatctgaccactgccatcggtgagtttgtgaccatgacgattggtgctgtgttggtttacatcatcagtttgagatatgatttgaataagtaaatatgaaaaccgcaatcagaaattctggttgcggttttttagataaccgaatcgtttacctcctgtccaaaatatcttaaaatatagttgtgaatataatcacaatttttatttaggaggttccatcatgacagaattatttgcaagtcccaacacctatatccaaggtcccggcgagctgttcaagagcgctggatatattgaaaagtatggcaaaaaagttctcttgctgtctgatccgacagtgctaaaaattgttgggaacgactttaacgattatcttcaaaataatggcttcgacgtcacccttgcccagtttgagggtgaggcttccgaatccgaaattaatcgggtgactgagattggtaaatccaaccaagaccagatcatcattggtttaggcggtgggaagactgccgactcagccaaggcaattgccgacaacctcgacattgctgcgatgatcgctccgaccatcgcgtccaccgatgctccctgctcacgattgtcagtcatctacaccgatgacggggcattcgatcactaccgcttttacaagaagaatcccgaaattgtcctcctcgacaccaaggtcatcgctggcggtccggttcacctattgatatccggaatcgccgatgcgttggccacaaacgttgaagccaccgacgttcgtgctgccaatgccgataacatgctgggcgctaagcaaaccatcgttgccggcgcgattggccaagcctgtgaggataatttgtttgaatatgccgacctagcgattgccgctaacaaggcccacgtcgccacccctgctttggaccacgtcgttgaggccaacacccttctcagtggtttgggcttcgaaagcggcggcctggcagctgctcacgccattcacaacggcttcaccgctttgaccggcgacatccatcacctcactcatggtgagaaggtggcgtatggcacgttggtcgaattgattttagacggcagcgatcacgcccgtttcgaaaaattcttgaaatttgatctcaaacttggcttgccaaccactctggccgatctgcatttaagttcagcttcagatgaggacctgatgaaagtggctacccaagcttgcgatgagaacgacacgatgaaatgcatgccaaccgacattacgccggaagacgtcttcgcggccatcaaggcagtcgacgagtatagtaaagactttcagaatcaataaccagttggttcaacccgatttttgaacttataatgtacgcaaagacagcggctattccgagaatgggatagccgctgtctttgtctaaatggcccagatgagccaatattaagatcgatttattttgtctcagtcgtcacgataatacggccgtcatgctttttgctcaataactcgtgtccttggatgacaccggcgacggtaaatggcagttgatagccaattcgaattgagagcttgtcctctgccatcaatttcaacagtgcggtcaaagcttcggcatccgaaattacctttgtcggcataatcggtttgaactggaactgcttattggataatggctcatcgccgccaaccgtcgtgatgatgccattttccttcacaatccgggcatcgctgtcactatcggcaccattcaaggcagaattgatgaccacatccgcccggttggccagaaccaacgccgggtcctgcttgttatatgagacgtactcgtcgactcccagcgatttgacgtaggcttcattcttactggcaccgatgccgatgacagttgcgcccaaattaagcgctaactgcgccgccagcgaaccgacgccaccagaagcaccgcgaaccaccaccgtttggccggccttaacttcaccaaagtaataaacagctttgtaggcggtaatccctggggtaacaatcccggcagcttccgcaaatgaaaccccatcgggaatcttgacggttcgagcagcggtggcataagcatattcggcgtaagccccatggccatgggcaactactcgatcaccaacttggaagccatccacattggcaccaagcttggcaaccgttccggcaacatcccgaccaggaatgacctgatgggtggtcgccttatattccccagcccgcatcgatttttcaaaattattcaggttaaaggccttggtctgaatcaaaatctgatcgtcggaaatttccggggtcggcacctcgtattcttcaaagacgtccgcagccccgttatgatcgtatccaaatgctttcattgctagcactcctatccttatatccgatattgtttaataaaattgtaagggttatcaatttggttatcaaacaaaaggctcttctgcgatcaaaacgcctcgtgcctcacactcaaaaataggacccaaccaccctctaggtgatcggatcctatctgaaacatgttgtctgaaaggcatttgaaccaatcattgaccaattcatggtcggtattcgtatcatttaaatatcttctgcagggtggaacggcagactactcggatctaagctcgctgacttagcacctacattattttcggaaatccctcgtctgtcttgcaggtgattagttcattcacctttcaccattattatataatttataagttagcggtacaaccaatccgtcttcaaaattattcctgcaaatcgcggaagatttcctgcattttgctttcaatgtcgaataattcactggcatattccttgagattaccggtgtgctgttcaactttttcttccgggacatccgtcttataacgtaacttgtgttccaagctggcccacatatccatcccgatcgttcttaactgaacctcgattggaacatcaaacacaccgttggattgaaagaccggcaccgacaccaccaaatgcaggctgcgatagccactgggtttgggatccttgatgtagtccttgcgtttgatcaaggttacatcggattgctgagtcagggcgtcttcaacccgataaacgtcgtcgatgtagttggtaatcacccgaatgccaccaacgtctaaaattttatgatgaatcgtgtccatgttgagtgggtagccttttcgctgaattttacccaccaaactgcggacacttttcatccgttcttccatatgatgaatcgggttatggtcataattcattgaatactcttcgtccaggttctccagcttagttccaatctcgttaacccccgagtgccgcaattggtagatttgggctaattctttgagatcgccaatctcgcttttcatgggcaatttatccaattctttcataatctgcttaacatccatgaagttacttcgttctagtatcatatttgattccaccttacactttcaaaatgttacaaaatcggtgacagcagcctgctaaacgtctgcttaaacttcagccacagcgactgctcttcgaacttttccggggtctgtaattcgctgacatcaatatcgtttaagaagatgtcacgcaaatcggccgagaacttctgatcataaataaacgcgttgatctcaaagtttaacttaaaactgcgataatccaggttcgctgaaccgaccgaagaaatcttgtcgtcaatcaccatcgttttggcatgaatgaagccatcgccataatagtaaattttaacgccttcctcagccagttggcgggcataatactgagtcgcccggtagacaaatggatgatcgggcatgcttggcaccatgatccgcacgtcgacaccagacatggcagcaatccgtaaggcatccatcatactatcgtctggaatcaggtagggagattgaatccaacagtaatctttggccatggtaatcagcttaatgtaacccattttgatctgttgtaaatccgagtccggtccgctggagacaatctgcatgttgacattgcccttagtagtcgtaaccgggaagtatttcggttcaacttgatcctcatcgatttgatcccggggactggtggcgttccagtccaaaatgaaccgggcttgcagtccaaagacccccgacccaatgatgcgaatgtgggtatcccgccagttgccaaactttttcttgcggcccaagtactggtcaccaatgttgaagccaccagtatagccaatagttccatcaatgacaataatctttctgtgatcacggaagttaatccggaaatccaagagaactgagcgggtgttcaagaatggaaaggccttgccgccggcatcaaccagtggttggaagaacttccgggtcgtgcccatcgatccccatgagtcataaatcactcggacctcaacgccttcacgggcttttttaaccaacaggtttaaaatttcatttccgatctgatcattgtaaaaagtatagaattcaatatgaatactctttttggcagcttcaatgtcaccgatgactttatgaaataagctgttgccgtcagtaaaaatatgaactttattttgacgagacaaaaaagcctgatcggttgtcatgaacatatcaacagcggtcttagcctcggtaacgacttcatcggccggtgtcttttcatcatggcccaattgttttcgctgttcgttaagtcgttcatccagctgcatctgcacgtgtttatgtaatttgaataaccgattcttaggtaattttcgacccagaaaggcataagcaataaagccgaccagcggtaaaaagaccagcactaacagccaagcccaaatcgcggcaatatcgcgcttctccctaaataccgtgaagatcgccaaaattgcgttaatgacgacaattacattaaataccatcgaccaatcaatagtcattttttcctccccgcagccacttttaggctaaaataataatgcatactgtaagtatactagaaagaagcggaaaaattatggatttattcaattttcttattgcgggcctccatggggtccactcaattcgttttattcacttcatcttcaatgaacaaccgctccttggcatcgggctgatcgtggccttggtgctgtatatgatttatcgttatatgaaccgataatacccatttggaaatccgattaagcaattgccttttagagaacggatttcctagttcacttatgaaacacaaataggcctaagccacgaaggcttgggcctatttggtgcatacctgcttcaccacttgggggtgtaaggtgaacgctggcatacagtgacttaatgcaataagggcgtaacaaaatactaagtgatcatgataacttttcaaattattttgaaagcggtaccatatctttaatataaacttctgggtaagcaaccacactgttaaaaccaatttggttttaatgacctacccctttttgccgatattcggccggcgtcactccaaaaattttcttgaagttcttgtaaaaatgactcacatcggtgtagccaaccttatcaataatttcttcaatactcatcttagttgaaatcagtaactttgctgcctcacgcattttaatatctctgagaagctgagagaaggaatacccagtttcccgtttgataaatcgactgatatagccttcactcaaattaaaatgttgagcgagactttccaagttcacatctttgcggttgacacgaatatactgaataatgtttgaaaccggctgctcgtcaatgttgccttcaagaattgtggcatcgtcagcgtgattgcgaataatctgaccgaacaacaacaggacgtaactgttcaggataatttgagatccatgcatggatgcttgagactccatgtacaagccaaaaatgatgtgttcaatctccttgtcattatcacaatgaactaacaccaactgagagaactcccgacgatacagcattctcaaaaagaagttggaaatatcattttgctccattagcagaggagaaaatgcatcctcgaacgatgatcgccgcataataatgttaaccacaatatcgtcgtcagcattacagaaaaacgcctgtttgaggtttgggggaacaatgaccaggtctccctgttccaaatcataggttttaccgttcagaaaaaacttgcaatgcccattgaggacataggagatttttacgaactccaaggtatgttccataatcggcagataacgcaaatgcttaaaaacaacaatttcagaatttaaatggggtgggtagatcagcttggaattggaattgccattttgctccggatgagtcacaggctgtgaaaagaattcactctcgaagaaccgcggacgaatgtcagaaagtggttgatctggaaatttcacaggattcttcatctttgctcgatactgatccgcaaaagcctgccaagttgaaaccggcttaaaattgtcgtatggattggcgacatacaacttcttatactcaatttcagcagtttcaagcttcattaatgaatttaaacttggagagttcaatattttcacttccttgactagacaaacaatgaccggtgacaacagtccgtcgtcccagtcgatcgtttgcaactatttaagatgcttggtaatcaaaactattttcatagtgtccatccctgagttcaactgtgtcatagcctggaatatcgacctttgcagtggcgccataaggaacgtcaacagaaaccgaaagcttgccgtcagtgtagttccattcaaccttggctgttccaaatggcgtttcgtgtgaagtcttggcagacgttaagttaccacccggacgaggggcaacttcgaactggtgccaagccggggcagtcggcttaagaccaccgaccgttgcatgaatccagtccgcaactgagccaagtgaatagtggttaaacgatgtcattacaccagggttgaccgagccatcgggcaacatcgagtcccaacgttcccaagtagtggtgccacccattttgacttgatacatccagcttgggcattcttcagacaggaacaattgataagcctcatccatatgacctgtctcagtcaatgcaggcaggatgtaaggggttccagcaaagcctgtgccaattttaccatgagcgcgacgaacaagtaatgccaacctgtgaccggcaaattctttaatctctggatcgtcatccaccaacccaaaggcaattgccagtgcataggcacattgcgtgtctgaagtcatgatacccttgtcgttaaagaatcgcttcttaaatccaaggtgaacatgattggctaatttggtatattcatcggcctcatcatccttaccaagttcgtgacccattttaacaaacatgtcacaactattggcataaaatgcggttgcgactagattcttttccgtcatggcctttactggatcatccgccggcgccgtgggatccagccagtcaccaagttgtcccagtgagtatgccggcttacggtcccaaacaccatcttctgaaaggtaacctttgacctcatcgatccaacctttagcagtttcgtactgcttggcaagcatctctttgtcaccacttgccatataaattgcccaaggaactcgaactgcagaatcaccccaaatggcaataccttgcggttcagtccattcagcaaatggaataaatgggacataaaacggtactgttcccaatcgcttttgttcatgtgaaacatcttgaagccagctgctcaagaaaccttcaacgtcgtagaaatatgcggctgtggggctgaacagtgagatatcgccagtccaacctaaacgctcatcacgttgcgggcagtcagtcggcaaggaaacaaagtttgatcgcattgaccaaagcgcattgtcatcaagccggttcacattctcattagaggattcaaaagtcccggtttgcaacatgtctgaaaaatagactttacactgcatatcatcggcagtcagttcaccgcgccaaccacggatttcagcatatctaaatccatgggtggcaaagcgggcttcaaagtgagcatccgacccatttgaaatgtattgatcaatttgttgaccccgacggagtggccgagtggaaagcgacccgtcactttccaatacttcggcgtgctgaagttcaatcacatcgccatcctgtgcgttggtaatatgcagatcaatccgttgagtacagttttgaccaaagtcgacttgccaatcagccttgccatcatactcgcgaatttttttgattgaaatcggctggttaaccatgttggcacggactggtggcaggattggaaactccatcttccgtcgatcaaacggaatttgggcaactggcagccaatcggcatcatcatatcctggttggtcaaaaccgtccttctcaagatgcgaatcataagtctcaccttcacacaagtcagactgggtgattggccccttggtcactttccataatccatcatgtgaattagagaaaatctgctcgctggtaccgtcaggataagtcacttccagctgcgcgaagacaccaattttgtctccatagacgttcgccttaccgcctttgaaaccaatccggccgcgataccagccatcccccaagtaaaagccaaacgcattttgaccggctttcaagtcgcccaccaagtcgtaagtccagcattccaaacgatcatcgtaggctgtccaacctggcgttaagatgtctttgccaattgctttgccattcacgtgaccttcaaccagaccaagtgcagaaaggtaaagtcgtgcatatactggtgtgtctttaagcgtaaactcattgcgaaccagtggtaaatgacgatggtcagtttctgcttccggccagctcggaccaacaaagcttgattggagttcccagtattcaagaattccttcatcaaatttaagggtttgtgaccagtcccctttggtatcaccatcaaccagacgggcctttacttcaacctgttctctagaaaccaatggatccaatggccaggcaaacaaaacgttgttaaccggttcggtaacaattgattcaactgtcccagcttggcctggcatatgccgggtaatttggagttcgacctcatctgaatcagccacatggccatcatacttccatgaaatccgcggagtagcggttctaatggctaatacatcgccgtgatagtgttcaacttgtaaatcatatggtgcttttgcattaacgatcacagacattctaaaaatccttctctcttatcagattctgttttgacattaactaactcaattatttttcaattccatacttgcgctgcagacgaatcataattgcaccagcaatgaagctgacaacaacgactccggcaaagcaccacatcgtaattttgatgacccctggtaaaacgagggctggggtaacgaaagcaaatagtgcacaaacaacccgtgatgttccgttgataattccttgaattgaagaacgaacctcaaccgggaatgactcttgcgtccaaactttatacaaagcttcaccagccattggactaccaatgttgtagaaaccgatcgcaacaatgattgcgattaagctaccgccacccattgtcattccaaccatggcaaggaacataataacggcaccaattacaaaccccgtattacgatatttacttccggcaatggatgagaaaacagcactgacaactaacgcaatcacgtttagaacgattccggcaccggttgccaaactttgtgaggcattggccttgaccatcatgaaggtctggaattgaccccaggtatttgcaagcaggttccaaccaatgtagaagatcaaaattgcaatgaagaagtacaagaactttttgttttcgccaaacaatatcttagtaactgatttagtcgcaacctctttactgttcttgcgattttcttcgtaacgagctgttccttcgtcatgcagttctttgaatttgcttgacatcgtccgccacagccaagtgatgattgcgaaaataaccaacagtccaaagacgattcgagccccggtggcaccggtcattttggaaacggcgaaggcaccaatatatgaaataaagatgccggcctgccaaaagatttgcgttgatgacaccaattttgctgaagttttggcatcaggcgaatctcttgaaactactgtcaaagaaatcggcaagtcggttcctgaggcaatccctgtaatgatgaccccaattaataacgtgatgtaattcggggcaaacacagcaattccagcaccgattgcatagaataaattaatccagttaaagactttaatcaggccaattgattcagcaatccggccgccaaacaatgatccaaaagcgatggcaaatgtcaacgccccggaaatgatcccgacttgaccattcgtcaatcccaatcctgattgccacaccgaaatggtagcggccaaccccacaataatgcctgaaccaagcatcgaaccaatcccggcggcatacgccaggggacggtaatatgaaatgtcttttgtttccatagttaatgagtctccttatttgctgctaaattttgattgtactttggatccagtttgcgagaactgtatactggatcgggaatatcatgatgagcaataaagcgcataacgagttctgcagataaccagcaaatccctagtgacccaaccaatagccaaattaataatgttggtgaataggccatgatggcgggtgtgacgaacgaaaagactgctgtaactgcccgaacaattgaatagctaataccggttacgcttgcacgaacatgtactggatataatgactgactccagattttgaataagggttcaccatgaagcatgttggcacagcagtaaacaaaatatgaaatggtgaaaatccaccaaacaccaccgaacactgctgagagaacaaatgataagatacacagaattaaaccgaccctagtcataatgtaacggtacttcgtgtcagcaaacttcatgtagatgccatagaggacaaatgcccccaagatgttggcaaagaatgcacacaaagtggaaaattgctggctgcgaccatcgacggtcaccaaaaagtagttcagaaatgatccccaggtgttagccggaatattccaaaacagataaaaaccagtcagcccaatcattggcacaaagtaccttggcatagcgatgagttttcggaaaggaattttttctgcggcaacttcttcctcagtagaagcccgtctttcaaccgggacaaccatttgagtctccagattatgaaacttcggtgaaagggcacggattccccaggttacgagcgcaaccagtgccagccaggcaaacaggattctggaactcatatagcccatgtcagctgtcaagaagcccaatccttgagaaagaacaattccgcccaaccaataaatttcggttgaagcaatcactttaccgtactgatcaggttctgttcgttccgaaataactgccaaggaagtcggtaagtcggcccctgaggcaaccccggcgataaacaaaccaaccacaatcattggcagatttggcgccaaggcgactaataatgttccaagggcaacgaataaaatatctagattgaagacggtgacccggccaaacttatcagaaagataacccccaaccgccgaccccaaggcaacagacaatgtgaccaatgtactgagtgcgccaacccaccacgcgttcaagccgaactgggttttccacattgccagcacaattccagtcgttaccaaaatacttgcgtcaagatatgaggcaatacttgcgttcatcgtcaacatccatccagatcttgatcgagacttcataaaatacctccattcttataatcaacaatatgtggaaccgctttcgtaaacgtttacaggtattagaatatgctcgggatgaccattcaacaacgtttcaatttattggttttttatgacatgcaaataaagccactcttcatccggatacagacatgtacgctggacctgcattcttgagacaaaaaacggaaccaatcaacgacaaatgtttgtcgttaattagttccgttttttaatcgatatttatttgagcgtcgccgcaatcagcagcatcatcggccgccttaattcatcacgcatctcttggctctctgccaacattttactggtgggagtcggttcaacgatttgatctaaattaaagcctcggttcagcaacgtgttcaaataggtggttaacgtccggtgatatttctcaactggataaccgagaaaatccgtggcccgttttgattcgtcaaagtagcgatctaccggccaatactttggtcggccatcatctccgaggatccattcctcgtgaccttctgcggtgaagatgggatgttcaacactgatgattaatttaccattgggaatcagtttagccttaatcaagtcaatcaatccggcataatccttgatatagtgaaccgccagcgaactgatcaccacgtcaaaactgccggcaagctgatccattgccatcatgtccaatacgtggtaatgaatttgagcttggtccgtcattgatttggctttttgaatcattttggtggatgcatcgattccaacgacttcactggcgccgtgatcagcggcgtatcggcagtgccaaccataaccacagcccaagtcgagcacgcgtttaccatgaaaatctgggaatagttttctcagttcatgccactcgccggctgcattcaggccatcctttgaccgattcatctggctgtacgcttgaaaaaatgctgcatcatcataaatatctgacatcgtcaatctcctacttatcgataaagttccggccgccgatcctcaaataccggcatgaaaccgcgagcatcgtcagtttctttggtgtcaatcgtgaatacttttaattgaggctgatcgtctaaagtcacaatttcatcccccatcggattataaatacccgaatggccgccaaacggattgtccggatcactgccgacccgattaacggcaaccacaaagctttggttttcaattgcccgagctgccagtaatcggcgccactgcgggattcgtgaagtcggccactcggcaggcacgaacagaatccgactatcgtccagactcaaagtccgcagccattccgggaaccgaatgtcgtagcagatcacactggcagcatcgatccccttgatttgaaaatgatcttcttcaaccccggatgccaaatactcatcttcatgcatcaacccaaataggtgaactttgtcgtaagttgtcagcagtttgccatcaggtccaaagatataagttgtattgtagaacgcaccatccttttcagttgagaccgaaccgccatgaatggtcatttgatacttcttggccaatttccctaataaagcctgcgtccgctggccgttcttatcggccacctgatctaaacgggtcaaatcgtacccggtattccacatttctggaaagacaacaatatccgcgctttgttcggcggcttttcgaacatttggttcgatttgagcaaagtttttgtcgggatcaccgaatgtaatatccaattgtgccaatgcaattttaatcttcatgtgaccgtcccccctgcatttttgaaaattatacaacaaaaaagcacattcaccaatcactggcaatgcgctttgacgacgttacataattgcggtgattgcggcgatcaatccaaatatgacgccgggcacatcggccacaattaaaatccaatcccgctttggcttgacccaaccgtaggcaacccacaatgccgcgttaatcgaagcacagaaaggctgaataaatgacgtcggttggccgttcaaattttgcaggatctctcctatgtatgagatatacataatcatattggcgatggttgcgatatcgccaatgactttctcctcactgaatacatggttactctcgtgtagttgatgaccaccagggtgactcaactggttttgcacactaatccctccaatttctcttggttcagtgataccatactcaccaagagaatgctagacgttgtcgagattaaattgcacaattctcgtaatcagatcttcaggcaagggttggtcgaccggcagttggatggcgccgatacttgtcttgtagccttccaactgatctttaaagacattgatggcctttgggccgggataaatcccaatatgattcttaaaatttgcgaagtgaatgatgtttttgtggtaatgaaacgtcggcatcccatacgaaatcttttcatcatagcctgccggcatttgtttttggataatttcatacagttgcaaaagcttcttttgccttgctgctggttggttatcgatatattcccgtactaatttttccattgactcaaccccctcgtgaaaaattgttttgatctttatgattaaaatctgttgacatttacattataaggctctaatatacaaagcaacaattaattcgtccataaaaccgatgaagtggagatcaagatcattgtgcacgcaaagagagttgccgatgctgagagtgcaatcgaacgcagatgattaaatggaccactgagggttcttccgaaagttcgcgagtacggagaaacgtgttggcatacgtcagttgccggagggatgttagtcccttgctaagagtgattaattggggaacttaacagatgttttttatctaccctgattaattgaactaaggtggcaccgcggaataatccgtccttaacaatcaacttttgttatggacggattatttttttatctaaattgacggaggtcacacttatgaaaatggaaattaaacgatggcaaatcatagagtgaatttcaactaattgataactcgacacttactaggacagctcctccaagcaggagtctccttgtaagcacctcgcaagcaaatccccaaaacccgggaatttacttccgaggagacttacactccgactcctaaccgcttggatccgctcacttatatcaggaggaaaccactatgataaaacaagccattgaaaaagttgttaaccacgaagatcttacatttgacgaaagccaatccgttctcgatgaaattatgaacggtgaaacatccgaaattgaaactgccagcctcttaaccgcattaacagctaagaatccgaccatcgacgaaattgccggggctgcctcatccatgcgaaatcacgctttgaagttccccgaagccggtaacgtcttggaaatcgttgggactggcggcgacaaagccaacaccttcaacatttccaccaccagcgcaattgtcgttgccgctgccggaaccaaagttgccaaacacggtaaccgcgccgcatcatccaagagcggggccgccgacgtcttcgaggcactcggcttagacattaacgaagatccggccaccagtttccaaagcctacaggacaacaacctgtgcttcttatttgcccaggaataccacaaatccatgaagtacgttgcgcccgtccgcaaacaattagggattcgcacgatcttcaacatcctcggaccgctggccaatccagcccacccaaccagccaactgttaggcgtctacgatgaagacctgcttgaaccactggccaatgttttaaagaaattaggcgtcaaaaacgccatggtgatccacggtcgggatggtctcgatgagatgaccgtcgctgatgaaacggccgtcgttgaattatgggacggcaaattaaccaagtacgttttgacacctgaacaatttggcttcaaacgcgcagcccgaaaggatttggtcggcggtactcctgaagaaaatggccaaatcaccaaagacatcttagccggtaaaaaaggtcctaagcgagacattgttttactcaacgccggatcggcactgcaccttgcccacccagaattgacgattcaagaaggcattaacctcgctgccaagaccatcgacgagggcaaagcccaagccgagcttgaccgactgatcgccttctctgacaaacgcaaggacgtggttgcatgattttagatgatttagtaaccgcaacccacaaacgtttaaaaaagcacgaagctcaaacaccactcacagaattgaaaaatgaagtcgctcaaatgcctgccagtgtgaagcctgattttctggacgttttgaatgaatctggactccacgtgatcgccgaggtgaagaaagcctccccatctaaaggaacgatcgtcactgatttcccgtatctccaaattgctaaaagttatgacgcagcgggagcagatgccatttctgttctgacagaaccggattacttcaacggccacctcaactacctgaagaaaattagccagtcagtctccgcaccaacgcttcgaaaggatttcacgattgatccttacatgatttacgaagccaaagccaacggtgcctcgatcatccttctgattgttgccatcgtcgatgaccagcaattaagagcctaccgagaattggcagagcgcctgggcatgcaggccattgtggaagcctacacggcagatgaagtcacccgggcattgaaatccggcgccaagatcatcggcatcaataaccggaatctcaaagatttccaagtggattttgaaaacagtttgaaattacgggcaatgattccagaaggcatccccgtgatcgccgaaagcggcatccagacccaagcagatgttgaagccctggccgatgccggcttcaacggcatcctgatgggtgaaaccctcatgcgggccaacaacaagcaacaactgattaaagaattcaaagcagctaccgtcaaataaccttcaggaggtgtgtccatggttaaagtcaaaatttgcggtttgatggaaccggcagatattcaggccgtcaatgaagcgcaggctgacttcgcgggctttgtctttgcgaaaagccgccacgtcgtttccttagcaactgcgctggcactgcagacccatttaaatccaaacatccaaaaagtcggcgtcttcgttaatgaatcaatcgccgacatcttggccatttaccaagctggcgccatcgacatcgcccagctccacggcaaaagcacccctgaagagattgccgaattgcagcgcgccggactcaaagtcattcaagtcttcgaacgccaagccattgatccaaagtccaccgccgactatttgatggtcgatagcggtaaaggatccggccaatccttgaattggcaggcagtcccccacgttgatcgaacaatgatcctggctggcggattgacgcctgacaacatcagccaagccattcaaattgttcagccggatattgtcgacgtctcatcgggtgtcgaatccgacggcaaaaaagatcccaacaaaatcatgaattttatcaaaaatgcgaaagaggaatatgtcctatgaaaaatttaactgaagctcaaataaccaaacgaccaggaattttcgccgatacatacggcggccaatacatccctgaaaccttaatgactgaattggaaaaagtcgataaagcctttcacactttgaaagacgatcccgacttccaagccgaattacacgatttattaattaactatgccaaccggccatcactgctctattatgccaagaacatgaccgaagacctcggcggcgccaaaatctacctcaagcgtgaggacctcaaccataccggtgcccataagatcaacaacgttatcggccaagcattactcgccaaacatttgggcaagaagcgtctgatcgctgaaaccggtgccggccaacatggggttgccaccgcaaccatcgctgctttgttcgggatggactgtgaaattttcatgggtaaagaagatactgaccgccaaaaattaaacgtctaccgaatggagttgcttggtgcgaaggttcacccggtcaccactggctcgatggtcctcaaagatgccatcaacgccacactccaggaatgggctagtcgttccgaagacaccttttacgtcatgggatcggctgttggcccctacccatttccagaaatggttaaatatttccaaagcgtcatcagtaaagaatccaagcagcaacttaaagccaaagaaaacaccttgccagacatggttgtcgcttgtgttggcggcggcagtaacgctatcggcagtttcgccgattatatcgacgacccaagcgtcaaattagtcggcgtggaagctgccggtaaaggggttaacagtgatcagaccgcagccaccattgaacgcggctccgtcggcatcttccacggcatgaagtcattattcctgcaaaacgaagacggccagatcaacccagtgtattcaatttctgccggtttggattatcctggtgtcggtccggaacacgctgccctggctaaagaaggccgagcgcaatatgtcggcatcaccgatgatgaagctgtccaggcgtttgaatacatcgcccgacaagaaggcatcgttgccgcaattgaaagctgtcacgcagttgcttacgtcgaaaagattgccccaaccatgtctaaagatcagattatcgtctgcaccctgtcaggacgcggcgacaaagacgttgccagcattgccaaatacaaaggagtcgatattgatgagtaatttatccgccattttcaaaaatcataaagcatttattccgtttgtcgtggctgacgacccggattttgataccacagttgccaatatcgtcgctttggccgaaggcggtgccgacatcgttgaagtcggaattcccttctccgacccaatcgctgacggcggcgtgattcaggcggccgacctgcgggcatttgacgccggcgtccgtaccaagacggtctttgaaatcgttgaggctgcccgtaaacaaaccgatgtgccgattgtttttctcacttatttaaacatcgtcttcaagtatggttacgatgcattctgtaaaaagtgtcaggccctcggcgtttctggcttggtcattcccgacatgccctatgaaagccgcgatgacatcgttccaaccgctgataaatatggcatcgacatcatcccgctgattgcgccgacttccggccaccgagttgaaaagattgccaaggcagcgtctggattcatctacgtggtttcctcactgggcattaccggtgaacgaaatgaattcttcaatggtttgaaggatctggttgccgaaatcaaatcgtatactgacgttcctacggcaatcggctttggcgtccacacgccggagcaggccaagacgatggcggaaatcgcggacggcgtgattatcggtagtgcgattgttgacatcgttgccaagcagaaacaaaatgcccctgaagcagtaaaagaatttactcattcgattcgttcggctgttgatcaagctgaaactaaagaagccagcgtctaaaaaaagtccccggtgcgaagaagcactcggggacttttttaaaatttacaaacaagctgacgtgattgttaccaaataaatccggtatctttaccattggactaatcaccttagttgtagagttaatcaaaaattggccaaaaaaataaccgcccataactttagccagtttgcggttatttaataactaaaaatgcgctgccgtcttaaacggttccacaataggaagtcctgttgaatcaggacttcctttttgtgatttcattttaacatggatacgagattatcgacaaaacaaatctcctgggacgaggtagccttttacggatttctgcgggacattaaaacaatattttgcccttcttgtgtaaattaagtctataatttattctttcgtagaagatctacaactcacttcccacatgctatactaaaataaatgaacaagtggaggctgatatcttgataaaaatcgctgtaatcttaggatctatccgcagtaaacttggtgaatccattttcaaatatttacaggccaactttcccgactctgatcaagtgacctacgattggatccggctggaagacttcccgctggaaccgtatcaccatgatgaaacgccattatccaatccgattaccggcttaaaggacaacgaacaaaagtggctcaaccgattgaaagccgatgatggcttcgtaatcatgacgcccgaatatgatcacgcaattcccggcgttttaaaaaatgccttggactatgtcggcccggaggtagatcacaaaccggtccagattgtctcgtattcctactatagtgacggtggtatgctggcagcggaatccttcgtggaaattttgcaaatgctcaaaatgatggtcctgccgacgccggttctgttgtggaatgccaatgataatttcacccaagcaggcgagctgatcaaagatgccgataacagtgaccattttgaagcccgactgaaagaagcttttcacgagattgccttttacacccaattactgcacgagcacccatttaaataaatcagaggtcagtcatgcgagccattttacccaacaaaactgaattcatcccccacgcccctcaaaatgagcacgagatcttcatggcgatgcgcacctatcccgacaacgtcaaagtctaccatccccacggcagtatcgacgccacttcggtcttttggcataacaagctacacccaaatgccttgaacttcgctgtgtatgtcgatcccaaggccaccgaacaggatgtcttgtttcaacgtgtctatgacgatattgaaaaattagcttggaaattcgatgacgaccgcatgatcacgcgtgactatgcccctcagcatcccttcaatcagtggttaacgacgaagcacttccagttggtgcaaactgccttgactgcaacagtggatttgggaaccctatcgctaaacacgccgattgcgtcagggacgctcaagacgttcgctgaagtatcatcgcagaattcactctaccaatccgtgctggaacgtagcatgcgcaaatacgcaggcaagccaacttttaatccggcgatcacgatgccattaccagattggtcagcactcatctcacaccgacaaatttcaacggccccatttgcgttaattcaagacgatcagctggtcgccttcagtttcctatatggccttggcgatcacttggttgaacttggccaaatgaatgcgactaatgctcaggcgctaaatgagttattgaaccgacagcttcagtggcttcaagacaactaccagaccctgactggtgaatttggaatgaccaaccggctggacatgaaaatttttcaaagtttgccgtttaaagatgttaacaagtacgaaacttatatgcgtttaacgtaaaacagactaaccctcgtagtgaaccccaatcccgtcggatctgaattcaccacaaaggttagtctgttttataatgctttaacaatgtatgaacggccaaacacggtcattgccttctgcaggagatttaaactgacttttaagctgccattttcaattttggcaagctggctttgttcaatgccaatctttctggccagctcaacttgagtcatccctgcttgacggcgttggtatttaatcgtgtaggcggcgtcagcttcagcaggaagctgaagaacttcattcaaaggcttattagcttgagctgctaaaattaagtcggcaagttctgaattcgtcaagcttcggccaattgcctgactgataaatgatagttctcggatgccaatcgtgccattgaccagttcagaaagcctcgaagcagcctgctaatagcagcggagtcagcccggtaattttcaataactgtgttcaaatgatccaaagtattgatcagttctgtcttggtcatgtcagacacctctccacggatagtacttttcaacgactaatttgctggcttgggtattgaaatcacgttttgtgaaagccaaaaataacttttttcatttaaaattataacagaatattccaaatttgaatattaaccagtcttattctgccttctcctcaccctttagatacgaagaaaagcaaaccactctctattgaaaatgcttataccgaaaatatttataaccaagcttatgatcaaacatcgtctccgataggcccgttcgattggccataaaaatataaatcccaagggctaccaggccaaagacgacgcagtacaggaatgccggaatcaaacggcttggcacgatcaattgatgagttccccaagtcagtgccatcacaatcacaaagaacagcaggttaaccaagacactgaccttcaatcgtccaaatgggacatggaactcatacataatttcgccataacttaacagacaaatgaagccaaaaccgatggcggtggaaatgattgccccaaatccttgaagcaaaatgaccaatggaatttggaacagcaatttggcaaccagtccgacaaccagataatacatggccttcttactgtagtgcagggcttgaagcagggttaagccgttaatggccagccccaacatcaaactttgcagaatgttggcagcaaggtacttcccgccaagcaaactgaacgagaagaaaatgccattggtttcgtaagacagcccacacagaatggtcacgatcggcagcaggacaaacatcagcatgttcacattttgaaagatcaaatctccgacgtcacctttcttggaggcctgactgtttgccaacagcggcagagtcgtctcggccaccgccagtgccagtgaaacgaccaccgtggtaatcttggttggattggcagaaaacagcgtgtagatgtactgggtatattcggccgaaaaatgctggacgccctgcataacctgtttgaagaataactgatcaatcaactgactgagggtaatcccggagccgacaatgacaaagggaatcgattcataggcaatcatcgtgaaaatcttcttgatactagtcaagtcaaacggcgcgctcttcttggccatttcagcgtagtgcgccgattgtttacgataatacagtcccaggtaaaggtaactagccaaagcgccgacaaaggccgccatgacacttaaatacaccgcctcgatataactgcggtgaaaaacgtcaatgaccagatacgttgataccagaataaagacaatccgcacgaactgttcccaaagctgagacacgccgtacggtttgaggtcttgattaccttggaaccagccacggacactgctcattgacggcaaaatcacaattgccggcaccagcacgcgaatcgaagtcaccgcactttgggtggaaaccacaggactattcttggcgattagcggcgcaatcacccaaaggactgccccacaaacaactccggagagaagcatgacaaaagagccaactttggcaagttgacgtgaattcaaaaatttattttgaccgttataaatcgcaacccgccgggcaattgcggagggaaatccggctgttcccagtgcgataaagaggccgtatggattataagaggcgttaaataaagccatggcaacgttcttgtgctcgggcgacccaatcatatacaaccacggaatcaggtagaggatccccagaacccgggaaaagatactgccaaatgaaagccagaaggatcctgacataatttttttgttcatggcgacatgcacactttctatatttcaatcataaccaacattataatatctttcgggaaagtttgctatcaaatcagaaacttggtttgcgatttttgagaacttgttgggatacagaaaaacagcggtctcgaaacaaaagttgattgcttttgttttggccgctgttggttttggtttgtttggttgcgaaatgtgctacccagcccagccctaatgtataaggcgaaaggcgaatcttcgttggtcaatctgtccttttttttatacattaggggcttcagaaacacgtttgttaggttcttatgtgctcccttcggcctttaaaatacgcttcgacgggccagaggctaacttctaaggggactttaattaaagttccaaacccaggaacttcaatcaaattccccttagaaaccgcctctaccggccctcgtcgcgctctctagtcttccgacacctgcgcgttcttttggatgtctggtgacagatcgtacatctttgctgcttctgttaacattgcgtgatatgaataggcgccatccttatatggttcgatgacaacctcgtcagcaatctttgaaaatggcttcttgccgtcttttacctgtgctgaatccagatctgcgacaattttcttctccacgtcggaataactgcccacaatctgcttagtctctaaactgccttgtatcgaaattttactcattagcaattcctcacaatcatcagttatatttagtgtcatcataccgccaaaagagaagcgatatctctaggtacatcataccaatttattgacccctatttcaccaaaaatcgtaaagaaagtcaaatttaatttttaatatcaacaaatgcttcccagcaaaaaaagcgcccaacaccagttaatcacttgtgtcaaacgcctgaatacaatttattgatgatagaagtagctggtctgggccttatgcgtatcacttgatttgtaatacatcttcaaagccgtcttgccgttatgcttcacgtgcttcaagtacacgggctgattctgtgacaacaaggtcaacttccagtaaccgtgactgttcgctttattggcaaccttgaacaagtaagacttgctcttagtttgtcgatattttttgatgttaacgtaataggttctggcgtctgctttttcagatgccttcgatgatccctgacggaatgaatatttggtcagccggtacttaaccggaacgttgccaaacaggtcatcgtgatacttgccgaaccaagtcccctgcagcgtcgtcggaacggcgtgggtcgtggtcttggcagcggccggctgcgcttcgatggcaatgatgccaactccaagcgtaacggcgaggaatgatagagttttgctaaatttcatcgaactgtcctttcatttgcaaaaaagcaattggaagtagtctaacagataattcaatttcatgcaaaattccaaactaggatacgacctattttgattatcctactaaattggcagttaccaaggaatacaaaaagtcagctgaaattgatcatcgtcaattccaactgacccacttttccatttggtccaacatcttcaactccttaaccgatattcaaaccatagtcgatcctcgtatggcttgagggctttttccagctggttgcggacgatattcacccgaagatccgcagccaaaatcagcccacaaatcaccagaatcgaaatctcaatggccactaagccccaattctgtttggcataaatcaccaaggcttgctgaagcgctagaatcgccaacatcgtcccggtcttattggccaaaaaataccaacgattaatcactcggaccttcttttcggtcaaagcccgtgcttcggctgataaattaggtgcgtttgccaatgccaatttgagcccttgggcgtccttcttcagcagctcagaaatatatgtcgaggtcttcccaacattttgcttcgcaaagaaatccccaaaccataaactaatcagaaaaaaacacaagaaaaaatctgctaacttcaacgtgtccgtcatcgtaatccctccgttctggcagtgactgcggttaacccccttgacaagttcaacgatggataggtaacttatcgttcaattactaatttacttatcctggtacgagcagtatataacgattagctgggctttggtaataatctgcttgtgagattcgggtcgtgtgtaaggcagccgaatgcaaataaatagacgacactctttgctggtttcacaaagaatatcgtctattggcttggcaggaagccaaaatattggcaatttcatttttcttcatctgacagccacttctccaactcgtctttgttagtaattcgtttacggggaagatctttgatagcctcagccaaattcttgtcagcttgaacgtctgccagtttcttttcgttggtcgtcacggtatcactcctagctcgtttactactaatattatagtatcatgtgaacaaaacacgaagccataaccttggtttagcggttgtttcctgcaacacataatcctcaagcttccacaaagtcccgacccatcttccgatcacagaccatcgcggcaacggccagtccaaatgagcagatgccaaagatcagccagctggcaaacacaccttggctccccaagttggcaatggttaagaaaaagccactgccaattggtgcgccaatcaagagcaccatgttaatgaaccccattgatgcccccaatcggtcatcgggaatcagtttgatgaacatggcagagacccgcggattgattttgcctaagaggtagccggtaatcaccgagaccaccgcaatcaagacgatggatattcccgttaggaatgtggctgccaaaaacaccagcatccaactgatgtaggctgccaatctgacaacggttgtgtttgccaaaaagtcatgctgaatgacggcgccaagaatcattcccaaggacatgctgatgctgaccagggcaacactgttcccgtagttgcccagccatagcgcctggttgtgcagcaacgacacattaatcaacccggtcatcccactggcgatcgtgttcatcacaaatgcgaaagccaaaataaccacgaccacctttttggacatcatgaaatgaccagtcacgatcaaacttttcagcaaggattgtttgggcgtggctgattttggctgattaacgctgagcttcggatcaattcccttaaaaattgaccgccgagtccaaatcacgattgccgcgattaggaaagtcgccgcattgatggcaccaaacagcccgtagttatggttcagccagacaatcgcaacggccccaacgccttgaaaaaccatctgcaaagtcgtttctgtcgccatttcaaatcccattgcatcgttcatttcttcattggggattaaaaaccggaagtacggtaattcaagactaccggaaaacgttcccagacaatcgctgatcacgttaatcgccaacacccccccaaagaccagcgtcgatcccggaaggccaatcatcagggctaacccaataaacaaggtaaactggttgactcgggcaaggaccatccactcgtacttatgatgggtattatcggcataatagccaaggaccacgttaatcatctctggtatgtaggttataaatgaagcaatactgacggcggccgttttgaatgacaagctgccagcataaatgataaacacaatattgaacaggctattgccaatcccgttgaaaatggcagcgttcatcaatgcccggtagcctttacttctaaaatatgagtgcatgtgatcccttctttctcaatacttgcttatacattatctgagaattacacttagagtattaaaattccactatatgagaattaatttggggtgatcagatgcaagaaccgggaagtttatatcgtcagttacgaaaagaacgccatttaacacttcagcaggtagctgacagtgaaaatagcgtttcatttattagtaaatttgaaaagggtagctcacagattagctttaatcgaatgatgcatctgctgggcaaaattaatttttcagtcgaggagttcctctatcttcaaggacgcgacaccatccagccaatcaagtcgaccttcatgtcacaccatccaatttatctgacagcgccgttcatgacgccgatggtcacgttactcaacagtctgacgggcgattcagcgacttcagcgacgttgccccggtcgatcgaacaatacgacgctaaaatccaccagcttgaagatgccggtaacctgaattggcaacactacttggcgattctctaccaaattcagaaagtcttaattcagaacgacgcctcacctgcgggggatccgaagaccgcctttaccaagctgcgccaactgagcaggcccatcgtgacttacctctataacattgacaattggagtacgtttgagatcttgctctttagtatcagccactttgccatgccgcttcaaaccgtccatcggttgagtaaaatcgccatcaagcgaaccaccagtacagaaaccttcccgatgatgccgcaaatgagattcgaactgctctttggcctattttcaacctacattaatttccgcgaaatgacttgggcaaaggaaaccctggactcaattgtcaaattacttgagaaggacactgatagcaactttgcgatcatgctgcggttttaccggggctggtacgattacatcgactcaaacggcagtgtcggtgaggaaatgatgaccgatgtcgctgtcatgttcaagctattaaatctgcgccaacccgccgacctgattagcaagatcattccacagattaagcgtaatcagcgggatccggaaaagtcgatgatctttctgttttgattcaaaatcaatcctcccatttactcaaatccggtcccccaggaatgacccgatcaaacgaagtcaccggatcatcgctcacttgaaagaagtgctgcttaatagcggtgaaatcagtattttgcttaaatgccggaatctggtagcactccttcgcgtaccgccaaagattggggaaatcgactaaccgttttttattcagcttgctcttgaaataaaacaccacatcaaagcgaattaaactgaccaccagccaaaagtccggcagggtaatgtggtcacccattaagaagcgcttgtcagcgagtcgccggtccaattgcgccaatcgatcaaaatactgattgaacaacatgtcgtattcggcttgggagtcaacgtcgctaatcttgcccggaatcgacgtgatgtcggtaataatgcgcgtgttcatggcgtcaaattcaggcttcaaatcatctggataaacgtccggcacattttgatcgaaatatgccttccaagatccgcccaattcaaacataatgtctcgtgaagaatcattgaccacaccaccagtcgttaaatcaatcaatgccggaaccgttggccttgccgagaaattcgggacggcctttttgtaattctgcgacaaccgcgtggtatggagcactggatcttcatcgttggcgttcttgccaaagaaccagtcgtcatcaatgccggggtgtcgcaatggatcggtcgcaaatttcgaaatcaccttattcaaaccagtgtaatcgatcatcatcgctgccggggtggcccagggacagaatttcgcccagacatagtgataacggttaggttcaaccggcagttcaccagtggaaaatttcttagtaaaacccgcgtcattcttttgtgtcggcaatgcacaagcatccccgcgattcacattttgactcattaacatcgctccaatctctcatatttgcctctactgtacacggatcggccttaaatgtcagtaagtaaaaacggaattactcgcaatgagcaattccgtttttgattaattattgataactatcataaagcttctcaaagttcacagtaccaagcccggttgcctggttatacaatttgccaggttggccgacatagtacaggttcgagttgttcgaatcactatccagcaccgtaaatggtgtcttctccggatcttgtgccagtgcgtaaatttgtggattccagaagcccattcgagttcccttaccactgttaataaccgcagtcacaccgttaaattggggtgcaacggcactggtaccacccaccgtatgccaaccagttgccttggtgtaaatctggtaaccagtgaagacgtcggcatcagctgaaacatcaggatagttccggccatattgcgtgccgctgaccagaaccgggttgggactcggctgcatcaaattcgaaaggtattgacgcgcgttaaaggtattaacgccggaaacaccctgctggtaagctggggtatcatacagcttactgatgccaccgccgccagcgctatataacatttgcagtgcactcaaattggtttggaataactttcggtgcttagcgtatgccttgtacatataatcggcaccccaagcccgttccttgtcgacggaaatcttcacaccaccgccaagattcttggtaaatggcaacgtggtaccgccagtcgaagtaacccatggattatctgatggaaaatcagcgtaagtactgtagttagggatgttaattgggccaaacgtgccgccaacccccatcccgtaagctccggtatcaccagaagcaacgaaggttgaaatgccttggagggccccctgagccatcaataagctcattgcctgaccatataccggtgtcagcagtttcttctgattcaaatagtgggtcacgtattcatttaagccccaactcattgaaagtgagctggccttattctcgtcgaatgccgttgcgtaggcattggtcaatccgacatcactccagttggcctggtaaacgcggacgttggcttgtggtgcaatcgcacccgattgttcaacatccaaggtggtttcaagctgaccagtaggaccagttgagctgtagacgggtgaagcaatcttcttgacgctcaagcgatttggtttcacgtcaagcccctcacccttccagaaggtttcagcgtcactcttcttaaagccggcaaaagtaatgatcccaacggtttgaccttgaccttgatagcccttgtcatacagtggctttagattgtagtgattgacaaatttacttggagcatccttcgggttcatcttacccttgggtgtcttactcttggccttgctggaaaccaggccgctgccgccctgattgaaggtggtaacccccaagaccgtcagcaccttgtcggccaagttggcaggcatcactggctttttggacgagaattgaaccggattggagtggtaggttgccgtcttcaggttagttgagaacgccttgttgacatccttggccttaccagtgaccttgatgatcagcccatttgaaaaggtgcttgatttgaggtgatatttactcaaaaacggcttaaattgaccggtcacactagctggctgaccaaattggtcacggaagtgctgcggcgtatagaaattcttgaagtcaggattacccggtgtgttaacggcgtatatctgattggtaatctgatcttcattctggggcttcaaaacaatgtccaactggacttgtttgttaggagacatggtcttcttagccatgagtttcttaaggatcttctgaatcccataaggatctttcccagcagctttcttctgtgaagctgcttgagtcattggtgctgcggacacaaataatgctaaactggccaaaccgaccagccaatgattgattgtcttcattcttcccaacctctttctaactttcaatatgatagtggtcgaagtacaccggttctgaataatcccccaatcatcaggactgcataatatatgtaaaaaggcgcaatctgcgaggcgccgaaaaacatctccaactattgcgagagtacacgtttcaagcaaatatgtcaagaatgttacagaatcattcggattgggtatttatacttatacacaaaaaagcatcctgaaagtcaatgagctttcaggatgcttctatagaactatagaatttaaattattttggatttgcagcagttaatgaaaggttgctccagaattcgttattgtcggcagcagcactataacccttaacacgcttattgacaggtgaccaattcaacgtgaagttatcaggggcataagcggcttcggtattcatatacttctgccatttcttatactgctttgtacgatagcttgaattccaagcttgattgttgttcaaactattcagcaactcagtattcttcttagttgcaaagtgacccatgttaaacggtgcatcaacaccatacatttgcgttggtgttggttcagaggaagttgaccatgcagcatcaaaaatatcaatcttattctgcttaggtttctgcaacgtcgaatagaaactattcatttccataggcttgcctccggtcattttcacattcagaccgagtttatgccattgttgcaaatcgttctggtaaatagattcggttgcagcggaactttgcataaccccgaagtaaatagttaacttcttaccattagggtctgtgcgccacttcccatgcttcttataacctgctttatcaagtaatgacttagctttcttcatattatattggaagccaggattcttagcatcataaacatccttaaatgcaggcggaatcaaagtgttggcacgccatgaaaccccattaccaaacttcttataaacttgatcctggtttaaagcatacatcattgcctgacgaagattcttattgcccatcttagaattcttgtccatgacattcagtcccgtcttggcattcatatgcccgacattaaagccaaagtatccatatgaaagagcggggcttccagcaatgccataatccttcagagccttaatcttagtatattgactggatggatgagcactgtttgcagcaatgaaatcaaatttttttgacttgaacgcagcaacaaagttattgctcgaaacaacttgaatcgtaatatgtttaatttgtggctttttgccataatagtacttgttaggtgaccaactggttgattcaccttgcactactttatccaacttgtaaggaccagtgaaaataggattcttccgtaccttgcttgatgccgcaagctttgaaattggaatgcctttaaagtattcatagggttcaacagtcgtccagacgaaggagtttcctgcatatttcatcgatggggacattctagaaaaatggataactgttgttcggccattttgaccgtctgggaaagtaatcccagagattgtctttgccttgccagcgtggtaagcggccatacctttaattgcagcaaaatctgacgagtattgttgtgatgtagtatctttgttcccaataatttcatatgggtattcaacatcttttgctgtaactttagcaccgtttgaccattttgcatctttacgaagagtaattgtaacggttttagcttttcgatcaatcttttgattagctaatccaccgtcaacaattttccaattctttccaacattccaaaggccatcaactgttccttgcgcattacctccaggattaaaggcatcagtgtcttcggcgttacttgccaaagtgggtgaagagatacccgtaaatggtgcatcattaacttcagcaaccttcaaagtactattatttcctgctgtagtcgccttaccagggccactatatgtagctgacattgaaacatgcttgccggcgcctgattcactgctcttaccattagagcaagcagcgagtgtcataactgacagcatcgcaattccggctgtgagccatttctttttgctcatgaaacatccctccaaatctatatttgagctacactaccaactaaatctcacctcaatatgcaaaaaccgcatcatctcctttaatgcccaatttttacttttgatcctgaccacgccgttgagcagcgttggtggttcgacgcatgacttggccaatataactgattgacagacacaaaacgataatctcaattgcggcaggcaaccaagtccaccaatactgagtgatattttcagggtcgttggcattggcaattaaggttcctagtgatggcgttcccattggcaggccaaagcccaagaatgacagcccagtttcaacaccaatattttcagcgaacgacaaagtcgtatcaacaatgatcaatgacgaaatgtttggcatgatttctctaaaaatgatcttaaaattactggtcccggaagtcttggaagcagcgacgtaatccttttgcgattcagctaacgttcgcgaacggatgagtcgtgaagttcccatccaatagaagatcgacaggatcaacgtcaacgtgatggcattgtaatgcggaataatcgtcacaatcacaataatcgtcatcagcattggaatgatcatcatgaagtcatagacacgctgcatggccaaatcaaccaggccgccgtaatacccggaaaccaggccccagcaaataccaaaagttgatgagatgatcgtcaaaccaatcgcgattgaaattgagttccgtgagccaacgattaattctttggcaatggatcggccaccggcatcggcacccagccagtaatccggggtgaagggcttattgtagtagcccatgatgttggtttccatcattttgggaacatcaatgaattctgaagcgataatcacaaacagaataaagaatactaataagaagagggaaaccatcgccggtttatcagccttgaactcaccccacatgattttaagccgtgacggggtggcttcttcattggcttccttggttaatttagcgaggtcctctttggaaatggtcgttgcgtcttcaatatctcgtttcatcttcagcaccccctactcaacccgaactcgtgggtcaacgatgctcaagacaatgtctgaaagcaaagttcccaacaagtttaggaagccatatagcagcaccaacgcggtaatgacggtgtaatcccggaagttgatggcgttcaagaataagaggcccataccaggataagagaagaccatttcagtaaagatcgacccacccagcaggccagtgatcgagtaaccggcaaaagcggcgattggcaatagtgagttacggaagatgtggtgacggtaaatgtccttcatcggcacccctttggaacgggcggtgcggacgtaatcggagtgcttggcatcaatgacttctgaacgcaggtactgaacgatgttgacagttccaaacaacgcccctaaaagcccgggcaaaatgatgtggtcgagccgggacaacaccgtcccgccaagtccgcttgcctgagcggaaaccgatccactggttgggaaccagttcaatgcgtaaccaaaaatccaaattccgataactaaaacaacgaagaatggaatcgacattgtgacatatgtatatacacgtaccaaagtgtcttgcagtttgccttcatgatgggcagcgtacatcccaagcggcagaccgatcccgtaagtcaaaaccattgtgaataatgcaagccataaagtattggcaccacgctgttgaatcaaatcaacaactggttcctggtactcataactcatccccagatcaccgtggaacaaatggacaacccagttccagtattgctggtaccaagggtcatacaatccgtggatttccattaagtggtgaatctgagcaggatcagctcgggggttaattgacccggtaaatggatcaccaggcattgccttggccagcaagaaaaccaaaatactcaaaataatcagttccggaatcataattaagacccggcgtaaaattgttttccacatcagacgtttacccccttgttctcagactgctgttcaaattccttagctaactcaggcggtaacgccaccgagtgagttggtgagactttgacgagtggaaacgccatgccgtcttgatcgtaataagttttctgctgctcttggtaaattttctcaatttctaaacgatgcttgcggtgctcctctcgatgattcacattggtttcgggaatcgcagccagcaagcgtttggtataaatgtgcattggattattgtagatatcatcccgggtcccaacctcaacgattcgcccccgtgtcatgatggcgatgttcttgcacatgtggcgaacaactcctaaatcatgggagatgaagagataggaaatcccaaactgacgttgaattttcttcatgaagttcagcacctgggcctgaacggaaaggtccagggcagacaccggttcgtctgcgataatcaactttggatgagtggcaactgctcttgcaacaccaattcgttgtcgctggccacctgaaaattggtggggatatttgtatagggcatcagcgtccaagccgacaatatccaacaattgaagaacccggagcttttcttcttccttatcaagatgttcaaaattgcgcagtggttccgcgatgacatcttcgattcgtttacggggatttagactcgaaagtgaatcttggaaaatcatttgcacgtcgcggttataatcgagtttgcgacgattttcacccttagtgacgtcttttcctttgtacataacggttccggcagttgccttttccaggccgatgatggctttggcggtcgttgatttaccggatccggattcgccaaccaggccataggtttcgccagcttcaatatcgaaggtgaccccgtcaaccgctttgacgttatcgacaacgcggttccagaagccgccgcggatcggataatgaacctttaggccgttaatttcaattagactcatgaccggcgccctcctttacttggtctgggaaataaaagtctttgtagcaggtgcagcggactaagtgattgtcgccaatgtcgtgcatggctggatgggcttcgtgagccgaggcgggaatccaaggaatccgcggtgcaaatcgatcgccatcctttggcatccgttgaagtgacggtaccatgcctttaatcacgtagagctcatcgttttcgttatctcgctgcggcatcgatctaagcagcgagcgggtataagggtgcttgggctcattaaagatttgagcggcagttccctgttcgacaatttggccggcatacatgacagcgacccggtcggctgtttcggcgacaaccccgagatcatgggtaattagaataatgccggcgtggttttctctttgaatatctcttaaaacgtcgagaatttgggcctgaatcgtcacatccaaagcggttgtcggttcgtcagcgatgattaagtcaggcttacaagcgattgcaatcgcaataataattcgctggcgcatgccaccggaaagttgatgtggaaactggtgcgcggttcgttcaggatcttcgatgccaacttggttgagcaattcaatcacccgggcatgacgctgcttttcggtcatcttggtgtgataaaccatgacttcttgaatctgatcttcgattcgttttaatgggttcagagctgacaagggatcctggaaaatcatgccaattttggctccccgaacctggttatagcccttctcatcaagtttcaataaatcggttccctcaaaatcgatttccccggaaatttgagtttcttccggatcatgcagccccataatggtggttgccaaagtactcttcccacaaccggactcccccacgattgcgagaatttcatcatgctttacttcaaggttgacgtttgaaacggcatcatagtattgaccattaatcttgaatgcggtgctgacatttttgatgctcaagaattggtcagaatttgtatcaaccacgagaatatctccttttggcaatgtatttatgtataaacattaaaaattaatgaacggtatgattgtttaattagaaaacattatattctcattgtattctcatttcaaaccatgttaagtgttttttgtaaatatttgatatcaacatttcgttaataaaggtaaaacgccgatataacagtattaaaggtgtttattaagattgtgcgttaatcaaaagaatcgtcattcttgcatattaaaagagcaatgacatcgattatcatcgctcttatcattctcattatctcacgagcttagcatccaataagcaaccaattagaggtgccaactcgtgccgctctgtaaaatcacttatctaccgccgtaaagcgttcattatgatgagccggatgctcaatctcatcgttaatcactttggccatcgtgccggcagtaatttccgatttgccttcagcgttggtcagcagatcatttcggcccagttcgtagtccgttgcatccccaggtttaaaagtggcactaggcgaaaccgccacccaattgacattactggtattagtgagcagctgatactctttgaactgctgacggggaatctcaatgaatgattcactattaggcagtttctccaacttttccacaaatcgatgaccattgccggtttccaagctgccggcgcctaaaataaagaacagccgcggcttgtcagcacccttggcaaattcgatcagtcgagcggtcaaatcaacgtgtcggtatgcgtgactcatgtcatgagtagcgtaggcgtcaaccaagacgtccaaatcttgaacatccacccgttgaatgtcaaatgcatcttttacaaccagcttgactgcgtctggcaggaggtcctttgccttctcagcgttgcgaacaaatcccgttacctcaaacccgcggttgactgcatcttgggtaatcgcactaccggccatgccagtggcgccgatgataccaacttttaatgtcatgttaaagcctccaataattttgcttcactattttcgattgtttcaaattaattatcgaccggctgagagagacggtcaaccatttggacggtgaacatggaacataaaagaaccgggcattccagcgataggaatactcggttcattaagttaaacgatgaaatcaacacagattgatttcctgattattttgtcaattcaactgccttacctgcaacatcaatcgtaatcggctcgccatcaattaacttgaagtgggaaccatcctgatcaacgtcgacttcaattaaacgatcacggaagacttgtctaaatgagtagtgtgaccatttcttcggcaggaatggtgcataatgcaacttgccgtcgcgaacccgcatgccggcaaagccttgaacaaccgcaatccagccaccggtcatggccgtaatgtgcaggccgtcaacggtatcgttattgtagttgtccaaatccagccgggcagttcgttcgtagagctcaaccgctttgtcttcatagtgaaggtcggctgccagtacggaataaatcgcaggtgacagacttgactcatggaccgtgtattgttcatagaaatcaaagttggacttcttttgttctggtgtgaaatcatcaatgaagtcccagattccttgaagcacgtcaccctgcttgatgtaaggtgaccgcaaaatcttgtcccatgaccagttctggttcaatggtaattgatctgcgggaatttctgaaaccggcttgaggtccttgtcgaggaagccgtcgtgttgaacaaagatgttgagatccttgtcataaggcagatacatattgtcgacaatgtcttgccaatgtttcttttcatcttcactgacatttaattgtttggcttgttcgggagaaacttccttgagaatttccaaggtgtattttaacgtccactgagccagcagattggtataccagttgttgtcaacgttgttctcatactcgtcgggaccagtcacaccatgaatcatgtaattctggttacgttgactgtagtgaacccgatcggcccagaaacgagaaatctcggtcaaaacttttgagccttcgttaaggacatacgacgtatcgccggtgtagcgggtgtaattatagatggcaaaggcaatatcaccatttcgatgaatttcttcaaaggtaatttcccattcgttatgacactcgatcccatcgaaagtcaccattgggaacaaggcgcccttcaacccctgttgcttggcgttatggtacgcaccgtctaattgcttgtaacgatacatcaagaggttgcgagttactttgggatcggtaatacctaagtaaacgggcactgcgaaagcttcggtatcccagtaggttgcaccaccgtatttctcaccagtgaagcctttcgggccaatgttcaagcgtgaatcttcgccataataggttgagaacagttggaataagttgaaccgaattccttgctgggcttcggtatccccatcaatgacgatatcggatttgttccagcgatcagcccagacctgctcgtgagccgtcagcaaatcatcgtatgattggccggcaacttggtcacttaattgatgcatggcatcggttaaagcggcttgagtgtcgtaatcccgtgaggtaacaacgattacacgtttttcaagttgagcggattcgttgggcgctaaagcaccggagaattcgttgacaacttctttttcgctgggttgagctactttttcagcagtcaagtcagtgacattgcgcatttccattcccgaagtgaaccgcggcgtcccaaatggattaggggtcgtttcagctaagacgttacctgagtcagttccctgctcagttgagagaacttcccagaaacgttcgtcgtagttggcatcctcattcttaacgtcgccatcgatcgctgaatccatcacgaggtccactttatttgagccaacgttttgaacagtgacccgctgaacggacagttcctgctgggcaacactcaagaaacgttcaaatttgacagctactttggcatcacccttggttaccgtaaatgagcgggttagcaaagcctttttcatatcaaggttgagctcaaaatcgctgaactggtctttcgccaggtcaataacttcgccattaatcttaacgtgcattttaataaaattaacggcgttgacaactttgccgaagtaatcgggataaccgttcttccaccagccaacccgggtcttgtccggataccagacaccaccgaggtaaatcccgttgagggtgtcaccgctgtagtcttcttcgaagaagccacgcatccccatgtatccatttcccaagctggtcatggattcctggagtcgtttgtcttccgagtcaaagtcgtgggtcacaatattccaaggagcgacttcaaaagttcttttcataagttaacgtcctttctaagctttgtaagtttctttaatgaatccaactgaggcagcacctagggccatgatgatcccggctaacaggaacatgttaggctgtgcgttacccaataatgggaataagccgaagctggcaagtgaggcaacaatttgtggcaggcagattgaaccgttgaacagtccaagataagtccccatatgttcaccagacaaggcgttggtaaccatggttaatgggtaggtgttcatcgatgcccaagccattccaactaagataaatgacagaatcaaaatgtattgagtgtgaatgaagaatacggagataaatccaactgcaccaagggccaaactgattgagtagcccaacttgtggtgattgtttggcattttggccaagacatatgaccagataaccgcagcgattgattgaacggcagctaaaacaccgtaccagttaccggcagcttgatagcctgcagaagcggcattggtagtgttccaaacgttgctggcaatcgcaccggctgagtaggtccagagatattgaaaggcaatccagcagaagaattgaactaaggtaacggtccaaaagactttaggcgcctttttcagcaatgaccaccagttaccaccggttgagttggcttcttcagtaattccatgatatttggcgtaagtcttaggatcatattcatgaaccttgaaaatcgtcagcaaacttgtcagtaacagaattgcggcaccaacatagaaggaaatgacaactgattgtggaacgacacccttttcagccgtgttggcaacaccaaatgcggtaaagatgaatgggaaaatagctgcgatcaccgcaccaccgtttgacaagaagctttgaatcccgtatgcgtaactcttttggtcatcattgaccatatcgccgaccatcatcttgaatggctgcatggcgatgttagacgaaacatccaacagggcaacggttaccgccccaaatactaaggccgtaatcgatgcgtacccgaaaccaaaactccccgagttaggcagcagacacatgacgatgatggcaattaacgttcccagagccaggtaaggcaggcggcggccgccaagcttaggtgcccaggttcgatctgaatagtaaccaataatcggttgaacgattaaacccgcaagtggtggcaaaataaagaaccaacccaacttgttggggtctgccccaattgtttggaagatccggctcatctgtgagctctgcagggtaaaggcaatctgcacacccaagaagccaaagttaatcatccaaatggtactggcaggaagtttaggcaaaccagacttcttggttgcagctgcgctactttgttcatccatttcatattcctccaattcaaaatatcatattaataatagcgtttacattttgtattattgcacgttttaatcaatgttgcaaacggttgcatgaaattaattgagcatttttaaaatcggatcggcgaaaatagactggtaccggttactttggcgagatgtcaatcgtcataaaaatttcttgtggcattttgatacctactacttttagatttgtatttatgagagaaaaaaagttttttgacttttttcactgatatataacggctgtggtctagacctcatgtgcaatatgaaaataagacgtgtaaaactgcgctaacctttcattgcacttcaatcaaaaatgttttatattgaacaagcattcacaagtaacttgatggacacaatttcataaggtggtgagatttacatgttgttaggtagtgttgaagccggtggtacaaagtttgtatgtgctgttggtaacgaagattatcgcatcttggatcggacacaatttccaacgactacgccaaaagagaccttgcaaaagactgttgattatttcaagcagttcaaggatctcaaggcaatctcaatttcttcctttggaccaattgagctccgtaagaactcgcctaagtatgggtacattacaaataccccgaaaaaaggctgggccaatacggattttgtaggtcgaattaaagaagattttgatatcccgattagttggacaaccgatgttaacgggtccgcttatggcgaatacgtcatggcaacgctgttcaacgaaaagatcaattcgctggtctattacacgattggtaccggagttggtgctggtgcaattatcaacggtaacttcgttggcgacatcggacatcctgaaatgggacatgttcgattgaaacgtcatccagacgacctgaatttcaaggggatctgtccttaccatggcgattgtttggaaggtttggtttccggaccaactttcgaaccaagaaccggtaagaaaggccaagatgttccgctttcagaccacacatgggatatcatggcattctacgtagcccaagccgcaattcaagtcactttgatgatgcgtccggccaagattgtctttggcggtggcgttgtcagcgaaggattcttgaagaaggttcgcgagcagtttaatgagttgatgaataactacgttgacgttggcgatctcgataaatacatcgtgatgccattggtcaaggataatggttcagcaaccgtcggggattttgctttagctttgaaagaatacaacaagtaacaacttatttttttgggaagttccacaaacgtttgcggaacgaatgaattttaaaaggagattttttatattatgaaagcactcgtatttactggaaaacaacacatggaaattcaagacattgacaagccagaagtaaagcctaacgaagttcgtgttgacactgcttacgctggtgtttgtggaaccgaccacgccctttataacggccttccaggttcagccgatgctgttcctccaatcgtctttggtcatgaaaactcaggtgtcatttcagaagttggctcagatgttgacggcttcaaagttggcgatcgagtaactgttgaccctaacatctattgtggcaaatgtttctactgccacactggtcgtccagaactttgtgacaacctctcagccgttggtgtaactcgtaatggtggccttgaagaatcctttactgctcctgccacaaacgtttaccctattcctgataacgtttcattgaaagatgcagccgttatcgaacccatctcatgtgccgttcatggtatcgacttgcttaagttaacaccataccaaaaagctttagttatcggtgatggcttcatgggtcaattattcgctcaaattctccagtcttatggtgtccaccaagttgatttggccggaattatcgacgaaaaattggatttgaaccgtgaaaaattaggtgttaccaacacttacaacaccactcgtgaccagattccttcagattacgatgttgttattgaagccgttggattaccacaaactcaacaacaagctgttgaagctactcgtaagggtgctcaagtattgatgtttggtgttggtaagccagatgctcatttcgaaatgaacacttacgaaatttaccaaaagcaattaactgttcaaggttcattcatcaaccctaacgcattcgaagactcaatcgcccttctccaaagcggtgacttgaacgttgatgccatcatcagcaacgtcttcgacttggacgaagttgaaccattcttgcaaggaaagactaaaggcgtttcaaaggcagttgttaaagtaggtgactagtttgaaaaataatgaggaaaccgccagccaagttctaaatggccggacgatctcgatgtctaaatccattacgtttttcatcatttctttggtgattaactccgccggaaacgtgcttaccttggttaccagcgcccaaatccacccttcctacttgggatcggcttattggaccgccgctgaagccaacctggcagttgcgtttggctggaatctattttggacattcttaattcttggggtcgtgatcacaattttaaatgccatcctggttggacactgggattggcggcgcgcacttggaaatctgatcttcatggttcccttctcagcgttgattcaagtattcgaagacttcttccttggtaagtacccggcattgtttggtggttttccaccagccaagacgccattcatgattggattttatatcctcttgaacttcttgggtgtcgcaatgatcggaactgccatctccatttatcagcgagtcaacctggtactgcaccccgccgatgacttgatgcagattctgcgtttcaagtattttaaaggaaatgccaacacagcgatgtgggcttcatacattccaccaacactgatggcaatcttggccttcgcaatcacccgtcaattcaccaacttgggaatcggaaccatctttgcgttcttattccaaggcggaattaccgggatcgcggatactaaggccttccctcacctgaagcatcaagctttggacgtgggaaaagattagagcgcgacgatagcatctgttgcatctgaacacatctcaacacccaatcgcacgaacatttgcccaaggtgctttattaaaaatcaaccctggtttttactggaagttccttgggcttgggtttcctcgtaaatgaacgcggttacacaattaatatgaaagaggcaattaaacatggcaattaaagatgatattacaggaattcaacacgttggaattccatccgttgatttggacaaaacaatcgcattttatgaatcactgggctttgaacaagccggcttattccataacggtgagaaccgttgcgcattcatgcgtttcggcaacttaaccattgaaacttgggaaggcgatccaactgctcgtaaagctggtgcgatcaaccatatttcactcaatacaccagatgttgaaaaagctttcgctgacgccaaggctcagggattacgcatggtgaatgatgaaattcaatccattccttcattctgggataaggggattaaattcttcaacatccttggccctaacgaagaaacaatcgagttctgccaaatcctgtaggacagagtgtgacgagcaacgggtgatgcggtgtgtaagacctaaaagattgaaatcctggtcttggatttaaagctttttggtcttacacgttagcattagttgcctcagaacacgtttcagctagataacaggggttaacaaacggggctagggcaaatgctttttgtcctagccccatttgtgttttataattaaatcattgaatgattccaagaagggaagtactaataatatggctcatatttcttttgatggctcaaaattatcaaagttcgttcacgacaacgagctcggtgaaatgcaagcattggtgaatgctgcggacgatgaattacgcaaaggcactggtgccggcagcgatttccgtgactggctgactctgccaaaggattacgataaagaagaatttgcccgcatccaagcagctgctaaaaagattcagtcagactccaaagtcttggttgtcatcgggatcggtggttcatacctgggcgctaagatggccgttgacttcttgaatgacactttcttcaattatttgccagatgaccagcgcaaattcccacaagtgatgtttgccggtaattcattgagctcctcatacgtttatgatctaattaacttgatcggcgaccgtgacttctcagtgaacgtcatctctaaatcaggtacgaccactgaaccttcaattgcatttcgaatcttcaaggaacgtctcatcgccaaatatggtgaagaaggcgctaaagaacgaatttacgctacaactgacaaagctcacggtgctttacgcaaagaagctgacgccagtggctatgaaacctttatcatccccgatggtatcggtggccgttactcagtcttgagcccagttggcctgctgccaatcgctgtttccggtgctgacatcgaacagttgatgaaaggtgccgcagatgcttctgatgaatacagcgatcctgatttgaccaagaatgaggcttaccagtacgctgcctaccgaaacatcttgtaccgaaaaggcttcaccactgaattattggaaaactacgaaccaaatatgacctacttcgccgaatggtggaaacagctcatgggcgagtccgaaggtaaagaccaaaagggaatttacccatcatctgccaacttcacaactgacctgcattccctaggtcaatacatccaagaaggcttgcgaaacctcatggagacggttatcaagttggataagccaaaccacgacgttgacatccctaaagaaaaggacaacttggatggtctgggctatcttgaaggccgcacaatggactatgccaacaccgaagccttccatgcggtagtccttgcccacacagatggtaacgtgccgaacatggccgttcacatcccggacgaaacaccatacacattgggatatttgatctacttcttcgaggttgcggttgccatttccggttacttaaacggcatcaacccattcaatcaaccaggtgttgaagcatacaaacagaacatgtttgcattacttggcaaacctggatttgaagaaaaaggtaaggaacttaagaagcgcatctaacttcacttaattagaaaacaaacccgctcgctgacatcattgatgttaacgggcgggttttcatttgaacatatatttattcaaaagattgggccccgttgttatggattagcgcttcggtaagactaattctgtcatcttcattaactgcttaatgggttatttcaggaatcagcttacatgcattttatgctcttgattaatttggaacaactagaggttaaatggcggtaccctggcgcatcattggcgtcacgttggcgctcgattcggctcaaatgacgatatgctataagcgtcaaatcgatttgatacctcaaccgctgatttaatgccggagttaaattagccaacaaaaataaacttaaagaaagaagattttaattatggatggaaaatattcaggtacaggagcacatttggaatataaagtaagtctcgatcgaaagactgaggcaatgcaaacattttatgttaaagaaactaaggataccgctggcacagttactaaaagggatatctatgcactacaacgaagtggaaatgatgattatctcagtcattgtgaactaaacagtaacacgggggtctatgagcaagtggacacaatggagctagttaactttggacatggtcaattgttacaatacttccagcataacggcaatgactatttttgggtaggaacctatgctagccaagatgctacacagccatttccatggtcacaacagattggacggattcaatataaaccaggaactagcttagactacaaacaaaccacccgcttaaccgggcttagatatgctcgtaaggataagcccgcatttaaacatgcggttcgggttgaaggggctctctctagcaaaagagataaattgttaattctagtaattgatgatagctcacctcaccgcggacactttgttttgtatgataacgaagcccttaatacagttttagacggagtagagggaagtacaaacccatcaatttcttgtaatgatgggaaagtcattaaggctgcattaaaggattttgttagcgataaagtagtttcattatcctacgactcatctattgaaggagttgaactggctgataatgatgctgtgtacttttcctccagtgccgaaggtaaaaatcgaattggtattagccgatcagcctggggatcgtcatcttcaatccacaaactggttgacaattcaaattggactagtggagaaacggagggcgaagcaattcagttgcttggagacaatgttttaattggaattacacagtatcccaacggtgatggtactggcagtccaagaaataatagtatctatcgcttccccaagtcagcatttaactaacaatgacgatgtgagaactatgtaagctacaaataaaggcacagaactagcaaatatactagttctgtgcctttatttgtcaaaattcataacggcttggctaaattaatgctccaaacaaaatcttcccacgcacgattaggattaggagcataaattccaatcacataatcgctcatagcatcacgcttgttagctgggtaaccctcagaaatgagtgtctgcttaatcttggtaattcgttgctgatttgtccatttgtgaatagaaggccctaaataattagctactttttgtaaattaattcgatctgtaaaatactgcttaaaaggatcattatcgtttgcatccggatcagcagtgaactgaccaagatttgataatttaattgagagtttagtattgggaaaaaggtttaaaactgtgcgagctaaaacttgagatggtgattttttaatataatttaaataatcttgatcactagtaaagcctactgtacttagataatttaattttcgataatttcgattgtaccccttcgctaggtatccctgccagatccgtccataccgtgaagaattacccttaggcgtcacaataaaagcggcatagtattgacttcttttaccattgtgaagataggtttgtttagttaatgcagaaagccaagaattaggaaaatcctttaaattataaaggactttagtgtgcttcttgttccaaacatagacattgtggtgtttgtattgattctttacatgaagaacaccattattattataagaattaagcgtcttataggtattaacatgttgcgtgtcaattattcgataacggtcttgagcgtgggctatttgaccagtcagaccaaacaaaacaagtatcaagctacacattaacaataatagtcgtaaatgtctgttcatagatatcctccttaataccatcagtatactccgagtctgcgcccaataaaaagctaaacaattttaataatgcctggaaaacactgatgaaactgaattaattttaattggaattcgagctggttctcataatcggttatttccgatcagagcagctcgacgaagtgctaaaaagcgatgataagtagggttactttaaatcaaatagtacaaaaacagcccctagtcgttacttactagcgattaggggctgttttaataggttttccaaggggcgataactcttatcgaccctttttaaatttaaatatgcagcttgctttagtccagactaaacttagtaactcacaaaactcacaccatctcatgtccaacaatgatgtgatcaattacctgctcatcctctgctggtttatccagtaatagcttaactgccgactgccccatttcatctggatgaatatcaacagaatggaaatgctgatcggtgagttcacttggtagtgaattgttgtaaccaagaacttcgacgtttttattaggattaatcattttgaaacggtggtacatttgcagaccactgtaatcatcaatggcgacgattccatccatctgcggattgtcgcgaatgaattgatcttctaattcatcattctcttgagttgacagcacgacaggcgatttgccggcctgcttcatcgctgccaggtaacccttgcgccgatcgatttcatacggccaaccgttatgggtttggacaaaaattggattctggcactgatagtgatcaattaagtagttggtgccgtcaaatccggcctggacgttatcgttatcgacatacagccaatcttgtccggctgccggtttaccaattgtcacaaaatcaacgttttctttttgcagcatttcgataaccgggtcattttggtgggagtacagcaggataaaatgtttgatttgggcgcgggtaatcattgatttaacattctcgattacctgctcagtactgtcgccaatcgcgattgataggacgtagttgcgactgttgagctgcgcgttaatcccccgcaaaataccaacgtaaaaaatattgtcgacaacccggttattaactgggaagacgacgccgacggtattggcttcacgattggtcagattcttagcgttatagttgggctgataccccatcaaatccgccgttttcttgacgctgcggcgagtcttgagactgatgcgtttattatcattgagtgcccgtgacacagtggaaaccgataagcccagccgtctggcaatgtctcggattgtaaccatttgaattgcctcccctctactaaattttaccctttttgaagttgcgatcttgttaaacttttgtatcaattattaatattgaacgctactactagattttgacagtattatgtgataatttcaacgtatgaggtgattatggaaatgaaaaagcacagatcattagctgccatcttggcggttgttgcaagctttgcactaattttggctggctgcagcagttcttcaaataagagttccaacaacaattctaataaggccagcatgcaaaacgagactcaagataaatccgctaagcaactgttaacatcaagcgataatctttggtacatgaatggttcgattaattacaacagtaaatcaggcattgatgcttacaaattcaattcaaagaaccataccgtgaccatttacagtgtcaacaagatgcacaagacctacagtgaagctaagcaggcaaatgatctggacaaacagggaacgctgaagtacaccttcaagaatgactcggctgacaaaccggtgatttacatgaagggtaaactttcagatatcccaatgcatcagacaatttcagtgaaaaatactgtgagcggcaagaaccatcaatcaaaactggcagtgaccggctacaaggtcgttcgaaacctggataacgatccggctccccaagtttgggtaacgccaaaagactaattaattttaccagaagagacaatggcagaatcacttttgccgttgtttttttgtatcctgcataagcctcaaaaggagcgtgttaccagcccacgggccttttttcgctgttaaacagtcagttatggtaggataaaaccattcaacttgatcaaagaaggtattcgaacatgaagggcaacaagctattacgacggtcaatcagaacgttttttcagaactggggggcttacgtcagtttagtcattgtgattaatttattgttgggcatcgttgttgtgccaatcatgcagtatatgactggtctgattctcgaagtgaaccggattccctacttatcgtacacgaatgcggtctggcttttgacccaacgaccactggcggtgatggaactgttcattttgctgctggttatctttgcgatggtcttttggcagttcgcgtttctgctgtctgggattagcaacatcgccctcaagcaaaatttgagtctctggggcgtttttaaaattgccatccatgacatgcgtggattgcgactgggcagcttcctgttctttattggctattttattttagttctgccattttcagttgcctacttgaactcgccattgctttcaaaagcgaccatccccgtctttatcttggacgatttggaaaagaatccgttgattgcagccctgctcacagtcctgggcattgccgtcttttacttgggaattcgactgatccaagtcctgccgatgatgattattcaccatcaaaagggactggaagccgccaaaaacagctggcagttgaccagccacaatacctggcagtatctctggcggatcttcgtactgggaatcatcagtttcgcgtcaacgaccttggtatcgtatttgctttaccttttccagacttatctggatgcccagtcaaaaatgattggctttgttggtgccgtcaccaacatgggcctgttgaccgtctggcagcgaattgtcgcctcgtttagtgtggttgtcttcatgctgatcttgttaatggtcttggatgagtccaaatggcattcaacggcggctgtggtccgtttacctcggaagcgacggattggtcggcgggccatgggagcccttctgattggcctgtttttggtcggagacgtggcctttaatgctgtctatctccaaggagcgctgctgaccaagccaatcacgatttcccaccgtggcgtggatgacggtaacggtgttcaaaatacaattccggcactgaacaaaaccagcaaagaaaagcctgattacgttgaaatggacctccacgaaacccgcgatcaccaattcgtggtcatgcacgatgaaaatttatggaatttggctggggtgaataaagatccttatcaattgaccctctcccaaatgaccaagatgaaagttcatgagaacggccacactgcgcacattgccagctttaatcagtatttgcgggctgctgaacacgatcaccaaaagctattggttgaaattaaaactactcatcacgatagtccaaacatgctgcagctatttattaaacgttacgaaaaccgcctgctacgggatcacgatcggatccattcactggattatcatgtgatcagcggcttaaagaagcaggctcctaaattatttgtcagctatattttgccgtacaacttctcgttcccccaaaccagggccaatgcttacaccatggaagaaaccacgttgaacgaaacctttgtcaacgaggcgcatttccaccaccaacaagtgtatgcctggacggtcgatgacgaagacgacatgacccgaatgctattcttgaacgttgacgggattattactgacaacttaactgagctgaaatcaaccatcaactctacgtttgatcatccaagttatgctcagcggctgttgatttactcgaatgaattgcaggatgaagaaaattagttatccaggacatcaaaaagggaatcccagctgggattccctttttgataacctaatattcttctaaatcaatttaggcaacgtctaatttgcatcaagccattcagcttcaaccttacgccaaggagtcccaagctggcagctccactggtgcttgcttcaataaggccttttgatcatctgaaaggtattttttgtggaccacgacttcgtagacgtagtcgtccatccaatcgtcactcatggtgaagtagcccttctcaccattcttgtcaccccaggaattttcaactttccatttggtgggggtctcaccatccagatcaaccccggtaaaggtcattgcgtgcgacacttcggcttgatgatattgcagccgggctgccttgtccatctccaagtcgacatcgaacaatttcgtgtagcgatacaagtgactgtccaggtagcctttcttacggtccatttgttcgaggacatcgttgccaaaccagaccgtttcgccatccttgagctgagcaatggtagcggccttcaaaacatccatcggcagatttaaaaaggcaatctgctttccgccgacaacgttgttttgacttggcagtgaatataattggttgtaatctttttccggcgaattggctaacaccacataatcatccaaatcgacaccgaagtattgatcataaaattgttgaggggttagaccggagacccgatgatactttttgtcatcgtcgcgataggcaaaatcaacggttgccggtggttcaccgaatgaataggccgtgattcggtagacttcactcagcatttgtttgcgagcggcactgatcgcctcatcgctcttttcatccttgaccatcgaccgcagtttggcagcgtcaatccgcagttttcggttcataaccgtgtcaaaagcaccggtattctcaacgttcgccgtttccggaaaatcactgaccggcatcacaccatatttttggaccaatgccgctgccatcgcccattggccgccatcgtcgccagggaagctcaaataattttcaacttcccggtcattagccggccgactggcggtcgctaaaattcggtcatagaagatgttggcgcgctcaattttatcccagaagaataggtacttttgtgaaaggttgaagtccttcaccttatatttggcagcaaactggtgccgtaaagtattcaccaaagaaaacagccagcagcgaccgctttgcttttggttggtcaccgaaccggtctggaggtccactgaaaatactggattcaatcgtacttggacatccggatcctgagctgcttggttgatgccgttttgttcgattattttcgacagcacatcactcttaggtgcgttcttgaaatcactgtggagtgctgaaaaatcttgctccgttaaaacactattcttatcagtcattcagacatccctcctatgtaattgtgtcatattgtaaatcttttcttggttggtcgcaatgcggcatctgtcacttgctcaacataaacgcggtgtggaagattcctgtcactgagtcgcagtccgccggccctgcctgccgtagtggcttggatttcgagcctgtagtctcgaaataccaagatgctgtaatcgcgactttcagtcgcttcaacagcatggacactactgctggcaatgccggcggactgcgactcggctattttgaggatgcaatttaaccaaacaaacttggcagcttaaacactatttacccgcaacggcatcactgaattaatacaatttcggccaaaacaaaattccaattctcttttccaacaccgcttaaagctgtaaaacaaaaaagtctacaggataatctgcagacccaaatgaggattacctactgtgttagatacgcttcttaagccgtggcgtcaccaaataagcaattaaggcaccgactgctccttgaatcaagttggtgccaatcccaatatagccggcataaatgttatacagaaccgagtctgccacaaagtagccgattaccataatgacgatcccgactgaaacagcgattagtttggtccactttcgatcggtatttttaccagcgatcaagccgacaatcaagccttctgcgccgtggacaatcagtgaaaaccacatgtattggccatagccggagatcaggtccaataagaaaccactggcaccaccgacgactccgccgactctgggtcccagtaacagcgcgctgataaagattccagcgtcacacagattaatattgccatgggtcattggaattgggatgataaagaagcggctgatcgcaaccgtgacggcgataaacatcgccgttaaaaccaccttgaaaatatcactgctaaccttgccgcctacacttttacgatccattactgacttcctcccaatacataatcttctttatttgcttcagtaaaatcatacttggcccgacttccgccaatcaattttggccgtgaagaaaggcagaccacattcgccgcaccgacacggcgattggtcatgcggactggaatctgaacgtatttaacgtgcatcccaatctcggttcccccgatgtcgataccaccaaatgccgtgatgtgctccacttcaaccgggtcatccattcgttcataggcagcgacttgagtaccgccaccggcatgcattgccggaaccaccgagacaatttctaaattgttgcgctcggcaaccttccgttcaaccaagagggcccggttgatgtgctcacagccctgaatggcaacgtgaatattgcgcggaattaaaaattcttccaaagtcgacacaacggctcgaccgacgtccaatctggaattggtccccttccagtcaccagaaatttcactggtactgcagccaaccacaaaaatgccattttccgggaatgtcacccgctcaaaatattcagttaagacagccgacaaatcacgcttgattgtttgtaaatccatcttttacacttcttcccctgtttgtcctaacgtaaacttcgccacattgtacaatgacctggtcaaattcaacccaaatttccgttggtgttgcggtgtgcggctggtcaggctcactgcatcgtacaccccaataactgccttttgaaccgctgtatcaaaatccaagttaaagttcaaatacccaactagcagtgctgaaaatagatccccggtgccataaaaatgaccgccgattaaaggcgagccggcccatttaagttggtcgcccttgacatagacacagccaatcccgccgtcacggtggactccggtgacaatcaccttggctttggagtgggtcgcttcacgataatcggtaacagcttgatgaattcggtcatcactggcattaactcggaggcgttctccactgagcagccccaattcggtaatgtttggggtaataatcgtggcaattgatgcgagtcgcttaatggcatccaagtagccaggttcaaaaccggcatacattttaccctgatcacccaaaactggatcaatcagcaggtcaggcaagctaactcccgagagatagtcgtacaaaaggttagctgtactaatcttaccaacgtaaccaacgattcctgaattaaattgaagatcatccaacccattccagtgaccagttgcccgcctgataaaagaatcagtattctgagtagtaggctttccaaaaccttccgtttgagttgaaagcagttctgtcggcaaggttgccgtttgcagtccaaacgctgaaaatacagcgattgcggcagtagccgaaagcctgccgaccgcggaaaaatcttctgcaattaatacactcggcttgataatgatcatccttccaatcatgtttgttacaaatattgtaccccattgccaaactaaaagttaataccttacacattaaatgtaacattctctcatcaaaagtattttaagtataccaagaattccagaagaaacaatagacagtttgctgttaatgtcagcgactctggtatagtagagctgtaaatagtttggaatatagaaaagagtgatcaccatgaactttgccactaaaaccggcatcacaaccctggcgcaaacttttatcatgggctcaattgatgcctacacctttcaaaattttgacggttcatttgtcagtgcgcaaaccggaaacctggttattttcgcttacgaactcgccaccaagggttggagtacggcttacattcgcgtaccggtattactaggattcctactcggagcattcatctcacaagcctttaaacacattcaactggcaagcgatcgtcggttcaacgtcctcttgctgttcagtatcatcctattgggaattctggcagtggcggcagcattccacctgtcgatgctcaacatgttattcagcctcggcctcttctcgggttatgaactgaccgtcttcaacaagattggcacgaccagtgtgaacaacggcatcatgactgggaatttgaaaaattttgcaaataattcctatgaagccatctttagccacgatcgtgaagctttgctcaaagccggccgctttttgagtgggattatcatgtttattctcggcattatcttcagtgcctacctgcttcatgctgccgggccaaaagtctttggggccgcgttgatgatcaatctggttttgttgatcatcccattatttagttggcgaaatcgtcaacgggatgaaacaatgagttgacattcacttatatttgagttagattaaaaagcaattagaaaacttacgaattatcaagctatgaggagaagagtaaccactcagatcgatttcagaaagcctggcagatgagagcaggtatcgaaatgacggtgaagatgagctccaaagggcattaagccgttcacgcggattaatcggtaggaaccgttaacttcccgggtatcataggtaccgttgaggcgttgtctgcaaaggcaacgtgaataagggtggtaacacgagcattcgtcccttgattgtcaatttgacagtcaggggacgagtgctttttttcgtaagtgaaacttttacaattacaggaggattctcacatgacaaatatagcaattacaactaaatttccatatcggtacgacgttgtcggcagtttattaagaacacaggcgttaaaagacgcccacgccaaatatcatgccggccaaatcagtacagctgacctacaaaaagttcaacacgctgaaacaaaaaagattgttgacaagcaagttgagcttggcctcaaagacattaccgacggtgaatttaaccgcagctggtggcacctggactttctttggggattaaccggcgtccaaaaatacgactatcacaagagttacaagtttcacggcagtaagacccgcactgataacgctgaattgtcaggcaaagtcgccttcaaccctgatcatcccttctttgacagcttcaagtttctccaatcaattaccccggatggtgtgacccccaagcaaaccatcccgtcgccaacgatgcttttccgcgacaatcgcagtgataattggtcaaagttctatgatacctgggatcaatatttgactgatgtcgccaaggtctaccatgaaacgattttgcacttctatgaactcggtgcccgctacgttcaattagatgacaccacttgggcatttctaatcagcaagttaaacgaaactgccgatgacgcggctgcccatgcgaaatacgtcaaattagccgaagattctgtcaaagtcattaaccagctgctgactggtttgccgaacgacctgaccgtgacgactcacatttgtcgtggcaactttaagtctaccttcttattttccgggggttatgacgatgtcgccgagtatctgggccagctcaattacgacggcttgttcctggaatatgacagtgagcaggcaggtgatttttcaccacttggcaagatttggaatggcgataaaaacaaacgaattgtccttggcttgatcacttccaaatcacctgaattagaagacaaagacgcggtcatcaaccggatccatcaagcaagcggccaggtcccattggaaaacttggcactctcaacgcaatgtggctttgcctcaaccgagaaaggcaacaagctcaccgaacagcagcagtgggccaaacttaaactggtcagagatatcgcccgagaagtttgggatgtcgactagctgttagccaatcgaaaagaggcgtcgttatggataaaattagggaaaaatactcgcaagcaactaatcgccatgttacccactggttcggattggccattggcttggttggtggtctcaccatcgacgcactatttagttttcggaccgggacgtttttcacttttatcggaattgttctgggaatgagtgggttgctggattttaaacagcgttaatcgtttcaaaccgtctgccagctgccatctaactggcagatttttatgagttgcctcaggatcgaaaaacaggtacacttttattaaaagatttctcataattatgtaaaggaatgatgaccatgctcgcctggatcagcctacaacacagcatcgtagagatcaatgcacttcagtgatgaatgacacttggcacatccccaaacggacaggtttcaaataaaccgtttggctgtgcttatcttaactggagtgcaactaatgacaattaaatatcccagtactattttcaaaggctacgcgtacactttcttttcctttttcgggatcacctcactttgggtgatttacctgcagatgcaggggctcaatctagtggaaatcggtttatgtgaaagcatcttccacattgccagctttgttttcgaagtgccatcgggggtattggcggatcgcttttcctatcgtttctcacttttctggggccgaattgcctcgattgtctcggcaaccctcatgctggtagcccacagtttctggctgtttgccctgagcttcgtgctgggtgcgctgtcgtataatctccaatcagggacaatcgacgcgctcatgtatgattcattggtggcccctcaacagacccaacgattccccaatgttatcagcaatctcaacgtggtgattgaattttcgcaaacggccggtgtcgtgattgccggatttttggtccactggcatttcgaattgacctacgtcgcggcaattctgatcggcattttcggtctgataaccgttctattaatgaaggaaccgactgttcccaaatcaattgatctgccaaaacagacggtcaaatcaatcatcgtcatggcctatcggacgttgaaaactaatcgtcaactccgcggtctgatgattttccaagcggtttttgatgggatttgtaccagctattacttctatttccaatccttaatggaaacgcaccatttctctggcttcatgatctccttgttgatggtgatttctgctggaatgaacatcgtcggcatcaaattgaccccgtggattcagaaacgcttggcaaagccggcgttggtaagtggcgtaagtgcaacgttggtcgggctactgctgctcacatggattaactggatttcaacgttaacgatactgtttttgttttcccaactgctggcgtcattaattgagccgatcttcagcagctactacaatgaaatgattgcttcacagcaacgggcaactttactgagtgttgccagcgttctgttttcagcttcaatgatctttttattcccactaatgggctggctggttcagattcaaacattttcgtttggctttggcgtgattggctgcttgatgttggtattgctgttgttaagtcaaaagtattttaagtctgcaaaataaaaagaggtcggttttaaagtcccaggatgggattttgaaaccaaccttttttcattttaatgtttaaagcaatgcttcacccttatcgtgatcaactagccgttcactttctggcatcatgctaccaccggttgcccagacaatgtgggtggcattagcggtgttgaaggcgggcacttcggtaattgcccgttcgattgcggtaaagccagctgcagctgatggttcgactgtgatattctcagtatccatcagctgggcttcatatttgtaaatcgttggatcttcgaaagtaacgctgccaaataatagcgtccgcatcatcttgccggcaatgcgcgatggccggccaactgccaaaccgtcagccgcagtcttcccgtccaagccgatatcaaagaccgaaattgcattattcaactttgtcatcatccccaacgtcacggatggaacgtgagttggctcacagaagattgcgtggatgtatggcccaataatggtcttgagtccaaacgtcacgccactgggactaccgccaacaccagcaggaagatagacaatcactggatgatcgcgatcaactttgattccctgctgcttaaattggtgctgcagacgaacggccgctaccgcataaccaatgaataagtcagctgatccctcatcatcgataaaatgaatgctcggatcttctgctgctgcctgtcgagcttgtggaatgactgaggaaaaatcagtatccaactcgaccacattaaccccattggcccgaagtttggccttcttccaagctttggcatcccgtgacatataaacggtcgtcttgaagccaaaggttgaagcggcgatgcccacacttaacgctaaattcccggtggaggcaaccatcaccccgtattgggcaaataactgcttatattccggcgatcttaaaatcgcatagttatcagtttctttgagatccccttttgtcatggcgacatgttcggcgaattttaatacttcatagattccaccgcgtgacttgatcgatccggagataggtaattcactgtcggcttttaaatagagactccctgccagcgcagtggcctgggcctgattccaagccgacttcattttggtcagctcgattaatggtgattcaatcaccccatgcatccgagcagtctctgggaaagcagcttcaataaatggtgcaaagcgatcccaacgggccactgcgtcaaaaatatcagcttttgaaaatggcagttctgcaggctggccataatcaggattcttccaaaaaattggtgtttcattcatcaggtctttaacctgtgggtatttaacttccaatgattgtgtattgtccatatcgatgatcccctaaaaaatatttactgctattgtattctgaaattaaggcaacacaatgctgccacatcaacctttaccaagctttaatcatggttgcaggcagatgtcactttccgaagcgtttgtcggcgacatccccatgacagcttactcgttgacctgattggtacttggtgcattgtgcttaataacatccggtaccttaaatttcttcacttggttcacatttgaataggtactggtgacctcctcggtaatcgacttctttgatgatttatcctgatactgcatataaatatgggtattagttggtagataagtcttcttattcaatgtgtatttgtaaataaatttggtaattgtgacctttttcaagacattcttggtactctcgctgttatttgcttcagccaaaataagcttcttggcaaccatcgaccctagcttgccatggccattatatgagaggacatcggttgtctggttctttgtaagcttcagatgtttcttcagatactgcatggctttaaccgcagcgcttccggagacctgtcgacgaacacttttaatcagtgggctctttttaggcaggcgttgtttggaccagctattatcagcatgaatgtagacagtccggccatcaatgaagtaatcataatttttaaccaaaccagtggcattattcagtttggcttgaacaatcattggatcaaggtggaacttggcagtaaatttgccagtggatgtttttttattttgcgtatttttattaaccagcacaacattgccgctcttaatgccatgagcggccttctgtgcgtgattgacaatggtaacagtatcagagggtttattagtcgagtgctttgatgaacagccagccaggacgatgcccatgaccgcaactgctgcaataattacttttttcatcagatactccttattcgcatttaagtcaggttaaacattgaccacaagaccacgtaggctccggtcacaaccagcagcgacagccagtgggccttcagcactcttttgacggatttgaaccacttcgagaaatagtaaactgagcggttcttctgaaccacattgataatctgaaaggcagtcattgtggcgcaatatatcaagacgatgtaagaaattacaaataacagatccatggcaattccccgccaatttccggttaacacaaccatcaagaactgccagagatacgatccaagcataccaaaataaaagaaactgggaatgacaatggcaattctggtgggaaaaattgtgatcaccacataagcggccaacaacaaaattccccgcagcagcccttgaagtaggcggtgatcattgatggaaaagctgacggctaacggctggtatttgaaaatggcggacgccaaaaagaaggcaatcgctccccaaacaataaaaatcaggtaagtcgagcgccgcagcttcaggttttctagcaaataaccacctccttgtggattgaattaattagtcagtgacaattgtgagttggggtttccatgttttggccgttgtatcgggaacgatgtagacaccataatggccattaacggaattggtggtcaagctggtgacgtgactggcaaccacagcggcataatacttcaaggcatcggttgtccgatatttggaccaataagaataatagccggtcattgttttgggatcgacctgtttaacagtaaaattagttgttttcgcatttgtcacgccagctttggccgcggcatctctggtactgatatcctcagtggcaagcagcttggccatcgtgtctaatttggtatccgcggtactttgggttaatttggcagctacttgatccatcaccaacttttgaaattggctttgcggcaaacttgccaaagttgtcaaattatcctcaaagaattgaagtgatcgctgagctgagagcgaaataaccccctttgcggcagaagcatgacgtgagggattaacgcctttagtcagatagttgcgccaaatgaagccatcagccccattcccatagttgtaaacttcgtagtagacatggcttgaattgccatgctgcatcacaacactatttttaacgtaccaagttgtattcgggtaatttttgaggttatgcagccgtttggtgtgggtcgcattccacaaataaactgcacttttggatttagcgtgataggccacggccgtgctgcgactcaacacttttgtccatatgtaacttgaatcggtgttcgttgcggtcgaattggcagtagccgcggtggtatttcctgaaactggaaagcttgtagcggtgaagacgccaaacgtcaccagggcaagcaataataactttttcatgatgttttcctcctatgtaccagccaattaattatatcagaaaaatggggtgaaatatcgcctttagtgaatatatacgcaagagagtggggcgcgaggcgttttgatcccagaatttaagccaatcaacgagttattcccgttcttggaataactcgttgattggcttaaacggccgggatcagccgattgccgcacgtttattctggataatagtggggctggggctcaaagagtctagcattagacctgataggaactgagatacaactagcaaacagtgttgtctcaaactacttttattctaatttatttttggtatgacaatccccgccgcagacgtttccaaaaactggtgtcgtcggtctgtaaaatcaagccttcatagatttgaccaatgtaccaagtcaaaaggccgatactgatgaccagaatcgccagtgaaatgctaatttccaacccactcgcgttgtcattgataattctcatgggcatgaaatacgacgagaagaatggcacatacgacaaaatttttgaaatcagcgcgtctgaattgctttgaaacggcatcgtcaagaagaaggcaatcatactcagatagatggcaggctgagcagctttcggggcatcttctgctttggcaaccagtgcaccactaaatgccgagatgatcgtgtaaatgatcacgcctaagaagacaaatagcaggttgattcccagcatgtttttaatcacatcattgaccagtgtctggttgtccgaaatgagttgcttgatgttgtccagatgcatggcaatctggaaaaagccgtaaccaccaacaatatagacaatgatctgggtcaggataacgccaaagacaccgataatcttgccgacaaagtacttcgaggctttggtactggagaaaataatctccatgactttagtgcccttctcggaagcaatttcttgggcggtcacagaagagtaagtgatcaaaatcatatagatcatgaagactaatacccaaaatgaaatgattttggccaggttggcaccgccatggttggtttgaattttttgtttgaaagccggctgaactgccagtgatttggtttgtttggcactcaactttgcgttcgccaggttaagctgttgctgagactgggcaagaaagacgttgattttggttctcatcccgccgcctagagaatcacttgaatgatagacaccactgacttttgtcttgtccgccgataacaccaggtagccagctagattattattgccgacacttttcttagcggctgcagtggtagtgacgctggctttcacgtcatcccgattggctttgataaattgttttcggagtgccggttgatcagaaatgacggcaattcgctgttgatctgaactggaagtcgcactggtgtagccgatgcctaaagaaattgccaacaaaatgaacggggagagcaccaagacgatgaagctccaagacttaacttggcggagataggtttccatggcaacaattaaggttttattcatgagagatccccgctttcattctgaaaatttcatcaagtgttggtggctgctgactaaattcttcgatgtatttaccgtcagtgagcttctcaaagacttcaggtcccttactgggatcatccaatcgcaacaagaaccgagaaccgcgaatattttggactttaacgacatgtgggagctggttcagctgttcttcagtccaatcggtcgtgacataaatttccgatttgccaaactgatcgcgaacttcgctgatggtgccgttcaagaccacttcacctgtccgcagcatgaccagccggtcgcaaactgcctcaacatttgccatatcatggctggagaagataattgctgcgccttgatcacgggcttccagaattgcccttttcaacaaatcagcatttaccgggtccaggccgctaaagggctcatccaagataatcaactttgggtgatggatcagggtcacaatcagttgcactttctgctggtttccctttgagagatccttaatcttatcggttttcttacctttaaccgcaaactttttcagccagtcgtcaatttgtgggcgaatttcttttgcaggtttccccttcaatcgtgctaaatagacaatctgctgctcaatggttagtttgggcatcaagctgcgttcttcaggcaggtagccaatcgcatcaaaatcagcctctttgatgggctgactattccagcggatctggccatcgtacttgaggaagttcaggatgctgtgaaaggtggtcgatttgccagagccgttttggccgattaatccggtgatctggttgtcgggaacatcaaaactaatgtcgtccaatgcagtcagactgccaaattgtttgtggagatgattgatcgtgagcatgcgaatgcctcccatttcttttgagcttatcataccataatcgtctggcggattttacggaaaacatttgatgtcaatggatttgtacataaaaagcaggatcgcaaacttgcaatcctgctcagaatcattttaattatcgatactgtttcattggtttgacaaagtgccaactgcgctgatggtacgcttgatcccagaattcccattccagttcgcagctcttcaagaattcttctttgaccacatccagatgatgttgatcgtagtgttccgcttcacggtcaatcaaagcaaataactggggtaaaatgctgtcactgtcatcttccatgtcagcgtaaaaatcaatccatggtttaaaaacattgtcgtcggtattcttaccctgcttcacaaaccggtttgcgatttccaggtaagtccatggacacggggtcatggccgcaacaacatcaattaagtcgccagttcgcgcagcacgatacatgtgttcgttgtacaagtacgtgccgggagcttgcggttcgtgctgcagggtttcgtattcgacccctgccacgttgcagaagttgtgatgcggatgaatttcactattcaaaataaagtcaatttgtttggcaaagatggccatatccgctctggtttgcgatttttgaatggcatcggcgtacactttaatgaacgcattcagatagttgtagtcctgaccaacataaaaggtcagcgcctcttttggtaaatccccattgccgattccttcaacaaatggatgttgatagatctcgtgtaaaattggctgtccagctgcgactaattcttcagaaaatttcatgagtcagtgctccttaaagcaaaattttcaaacagaacgcgaccggacttggcacttttcgaactcattattccacttccctacgttggtattaaccaaatcaggttcaaagggattggcaagtcgccatctcagcacaaggcacccctagtgatcttatttgaatacccaaagtttaccatattttgaaggatattttacgattttcttcgtatatgatacgctgaaagcaacaattttctgaggattgggggaattttaatataaggagagttgtttcatgaaattcaattggaagatcgcactcatcagtttttccccatacatccctttgatcgtcatttatttgttaatccacttatacgtcgcaaatgatgttgtcgctttgctattcactttaggtgttttttcagccggatatatttttgttcattataagtatgccaagactttcttcagtaaccatcctgaacttgatctacaaaactttgaattcaacacagtcgcaaacgttgttttggcactgtggatcatcgtcatggttggcctcataattctcaggctttatccacaaagtccagaaggctatctattggcatttgatttattctactccgtcattaacggcttcaaatcctacaggagagctgcaaaatgacatttaactggaaatacgctctattcaccaatgcaccaatgttcctcacgctgatcatctacctcggaatgactgcattacgcattgatccgatctggctaattcttgtcgtcgttgtagtctggctcgcatggtatacctatgccagttgaaaagtctactctcggcatcctgaatttaattaccataactatcagcgcggtacaacttcaattgtcatcatcacaatttcgacgattggttttctgttcttactcttaaagcttcaactaatagccaacatcgcgctctttatcacttggttggccgtctcaaacttcttggtagatgggttcgccaagtataagggcctaccataatgacccgacaatttcaaaaaccggcgttgtaaatctcaaacaagatttacggcgccggctagtttatactcatcttatattaggcgttcttcacagcaaacatcggcaaagtattcaaaaatacacagtcatcccgactagttgcccgtccctcagccaaaatagaacaacgttgaacaacattggcacccactttcttcaacaagtgttctgccgaagccagtgagccgcctgtactgatcacatcatccacaatgatcacccgtttgcctcgaagctgttctgcgtcacacccatccaaaaccagctgttgatgatagtcagtggtaatcgaacgcatcccaatcgcaattggattgcgcatataggccttaacacttttgcgcaagacaaaataacgtgggtgatgggtaatcatgctcagttcttgagccaatgggatccctttactctccaaggtcaccagataatcaaacggaatgttaatccgcttggccaactcctgagcggcataacgggttaactcagcatcccccaataagacgaaggaggcaatcgccgccgtgtctgtgatcgggataatcggtaatgtccgcttcagtttgccaattgttaattcatattccttctgcatcttgatcctccagattatataagatagaaagaaagcatcaaaaacgactaatatgtgtgaaaatcgaggcttttcacagccacaactgttaacgaaatttttatttttatgttttttgttcgtctatgtatatgataatactctattttatcctttttatccacatatgatagtccagacacgaattttgcagcaaaaatgtcaaaatgtcactttcagctcacaatccgtcacctaagacgacacattatgtggtctattttgggaatcatccacaagatacccccatatatagccaaaatgggtctcaatcaatccaactatttgtcactcccaaaaccacccttagtgtgattcaaatttttttgaagctcaccaatccgcgagtccacgcgattatgcagggtacaagcaaatctgccgaatacacaatatattgattctgaaaccggttagatatactatatatagtatcagttcgagcaattcaaacgaaatgagaatataatgtacatatgggaggaatcattatgcaagcaatgaaactttcatcagtttcactatctgatgaatttataaaacaagttaaagaagaagttacgcctcactggggagaattaggctgggttacctacaagcggacttatgcccgttggctgcccgaaaagggccgtactgaaaactgggacgaaaccgttaaacgggtggttgaaggaaacatcaaccttgatcctcgtcttcatgaagacaacgttgatccccaagttgttgatgacttaaccgaagaagccaagaagctctacaagctgatctatggcctttcagctactccatcaggccgtaacctttggatctctggtaccagctatcaggatcgtaacggcgacgccttgaacaactgttggttcatcgcggttcgaccacaatcatatggtcacagccatattttgccagagtatctccaaccagacactcctgccgtttcgatgccttactcatttatgtttgaccaattgatgaagggcggcggcgttggtttttctgtcactaaagacaatattcataagattcctctagttgataagaaaatcgacttgaaagtaatcatcgacaaggatagcaagtcataccaggattctcttgatatgggagcaactgacaaggatgaatggttgaagaatcattcaatcaaagacgttcgttactatcgtctgccagatacccgcgaaggttgggtggttgccaatgcgcacttgattgatatgcacttcaatggcactaacgccgatggtaagactgacttagttctggatatgagcgacatccgtgaaaaaggtgctaagatcaagggctttggcggaactgcttcaggtccaatgccattaattgaaatgttaattgatattaacagtctgctcaattcacgcgttggccgtcatttgtcatcggttgatgccactgatattggcaacttgatcggaaagactgtcgttgccggcaatgtccgtcgttcagccgaattggctttaggctcagctgacgatgaagattttattacgatgaagcaggataaagacaagctctaccatcaccgttgggcatcaaacaacagtgtggcagttgattcagaattcgacaactacgggccggttgctgattcaatccaacacaatggcgaaccaggaattgttaacttggagctttccaagaactacggccgtaagatcgatggtctgcaaaaagacatcgacgccaatgttgaaggaaccaacccctgtggtgaaatttctttagcaaatggtgagccatgtaacttgtttgaggtcttcccttacgttgccagtcaacaaggttgggatcttgatgaagccttcactttgggaactcgtttctcaaagcgggttactttcagcaattacgactgggaagtttcccgaaacgtcattgaaaataaccgtcggatcgggatttcaatgtcaggaattcaggattggattttggctaaatttggtaaccgagttgttaccggttatgaagatgctaaagatcctgaaactggcgaagctatcaagaagccaatttacgatccacgagttgttaaagaagttgatggcttgtacaaagccgttgtccgcgctgacaaagattactctgatacacttggatgcaaaccttccatcaagcacaccactgttaagccatcaggaacggttgccaaattagccggcgtttctgaaggcatgcacttccactatgctggttacttgatccaacggattcgtttccaagattcagatccactactgccagctttgaaggcttgcggctatcacgttgaaccagatgtttacacgaagagcaccatggttgccgaattcccaatccgcgcttcccacgctgacagcgagaacttcgcttcagccggaaacgtttcgattgcagaacaattcgcaacccaagccttcctgcagacttactggtcagacaacgccgttagttgtaccgttactttccaaccagatgaaggcgaccaaattgccccattgatgagacaataccgcttcaccaccaagtcaacttcattgttgccatacgttggtaatgagttcaaacaagctcctaaggaaccaattgacgagaagacttatgaagacaaagtaatggaaatccacggcgatgtcgcaacggtctttgcaaagcaaaacgataaccatgataagaagggtatcgaactggttgaccaaaccgattgtgctggcggagcatgcccagtgaaatagagtgcgagtcgcagtgtcagttgcgtccgagcacgtttcaactaggcaactgctaaattaatgcgttcaaccttggcccctcggtcccccgccgatcggccaagccctaaaacagatcattcccacggagaggccagggcaattaacttgctgctggcctctttcattacatacatcatggaggtatcacaatgttaaaaatctacaccaaagtcggcgatcacggtaaaaccaagcaggtaaccggaaaaatggtgccgaagtacgacctgcaaatcgaggcattaggggcactggatgaactggattcatggcttggctatgtaatctcagtcctgtcccccaagagtgcttcactggcaccgaccatccaaacaatccagcgaaacctgtatgaattacaggcagatatcaccgttaaacgtcatcacaacattacctttgacgacaccaaaaagctggaagcagaaattgatgaaattatggccaaattgcctgccatcaaagccttcattctccctggcggcaatcaagccggggcgtcgctccaatatgcccgagctctggcaagacgcgctgaaagaatggtcgttgagttaaacgacaagcagcaaccgctcaatgatgaaatctttgagtatctcaaccgtttatcagattacttattcgcccttgcacgttatgccaattacctggaaggctacgacgagattaaaagtaaatattagttgggaaaaggtgaatcggaaaccagttactgaattggtttccgattcgcctttttaatttgtcattagaggttctccattacacgtggatcgtatgttccgtcgtctgaccagtaattaattttagcgtgtcatcaagggattgcttgaccatattcttaacggcaatgtcggtgtaaaaagccacatggggcgttaagaaaacattgtccatggccttcaacttggtatattccttgaggggaatgtcgccatcaaacgactgattaaaaatctccgtctcattttcaatgacatcgataccggctccggcaatctgatgattttgcagagcatcaatcagtgcgtctgtattgacgatgggaccgcgggaacagttgatgaaaaacgcggagggtttcatttgtgcaaattgggttttgtcgatcatatggtaattctcatcactcatgtaggtatgcatcgtgatgaggtcggcgtttttaaaaatgtcttccttggaagtatatgtaaccagatctcgaaatgcggcgttttcgtgaatgtcatttcccaatattcgggcaccaaagcgtttaaaaatcttggcaaccgtgctgccgatgcggccaaccccaatgatgccaatcgtcatttccgacaactcccttgagcgcaaaccttcaacaatgtagtcattcttggccattcgtgattgaaattgtgggatatgacggaccaaatttaaggcatgggtcaatgtcatttcagcgaccgcttctggtgaataggaaggaacattggtaatggtcaggccattttcttttgcccatttcagattacaagaatcaacccctgccgacctcaatgagagctgagtgatgccaaaatcacggagtttgcgatataaatccggtgtttcgctgagcatgctgcgttgacggtaatcaatgccgtcataccctttagcaagatcgacagtatcgtcgtgtaattccacgtcattgaaatcaacctgaacatctggatgctccgccgcccattcgagcacaaactctttttcgtatcctaaaatgttgtatgccaaaatctttttcatcacgccaccgtcctcattgtgttatattataaaatgattagaatttggatataatatacctcataaagccggtggtgtcaaaatcatttcaatggctggccgtcatctcacaatcccaaggcgtctctgatcatcgtcaaaatatgctgttggtcgtttccaaaaacggtcgattgtcgataggccagaccaatcttgaagactggctgggcctcatcggtcaatcttaaagcgaccacattgggattattaatcttgacggcttgggtcaacaggctgacaccaatgccgtcagcaaccatattgacgatgctttgtgcctcactggatctgaaaatcacctgcggccgaatgtgattttgttgggcaagggtgtgaaagacccgatcgtgaacaaaattatttttaaacaaaataaacgattccttctttaactggttgaaagaaacttcagtgagtttggccaaggggctgtccttggcaacgagaatcgaaaacggctgctgatcaaattcatcaacgatcagctctgaatcagtcacatcatccacgtaccccaaaaatgaaacgtccaattgaccgcttttcagatcccggagcgcagacagcgacccttcttcgacagtttgaatgtgattaagatctgataccggcagctgctttgcgaccatcggaaagtaattagtctcaataatcggcggcattccaatcaccaactgctggcggtgactattttcaatctcccggactgcgagtcggtaatgatacaaaatttcatttgcattaactaacagttgctcccccgcagtcgtcagggtaattgcctggtgtgggtttcccctgactaagagttggctgccaaatgcggcttcaagccgtttaatcgcagcagaaattgtcggctggctgaccgaatagtcttgggcaactttggaaaaattcttttcggttgatagagaaacataatactttaaatcattcatattcattttgaggtccgctttctaaaggatattcttgttaactattataaatcataatagactacgtgcacattgactatataaagttgaacagactattctaaaggaaatgatcaagaaagaggcaattagatgacacaatcaattttgaatgacccatttaaaaataagggaacggccttcacagaaactgaacgtcaacagttaggtttggtcgggatgttgccgccaatggttcaaacactggatcagcaggctgagcaagtatatcagcagtaccagtccaaatcatccgctttagagaagcgggtgttcttaatgagtattttcaatgaaaatcgcgtcctattcttcaagacattctcacaacacgtcgctgaattcatgccgatcgtttacgacccgacaattgcgactacggttgaacattacagtgaactcttcgttcaacctcaaaatgccgcatttctgtcaattgacgatccagattcaatcgaagaaagcctcaagaatgctgcaaatggtcgcgacattcggctgctttgtgtgactgacggcgaaggtatcctaggtatcggcgactggggcacccaaggtgttgatattaccgtcggcaaactgatggtctacaccgccgctgcaggaatcgaccccagtcaagttctgccggtcgttatcgatgccggtaccaataatgaggggctgctgaagaacccgctatacctgggccttaaacagcatcgggtgcggggtcaacgatacgatcagttcattgatcaattcgtatctgcagtcgaaaaccagtttccagacgtttacctgcattttgaagactttggtcgttccaatgcagccaatattttgaatcgttataaagatgaccaactcgtctttaacgatgatattcaggggactggaattattgttcttgccggcctcatcggtgccctcaatatttctaaacaaaagttaactgaccagacttatttgtgctttggtgccggaacagccggtgcagggattaccatgcgggtttataatgagatgttagcagccggcttatcaccggaagaagcgaaacagcatttctatatggttgataaacaggggctgttattcactgatacccctgatttgacgccggaacaaaaaccgtttgcccgttcgcgaagtgagtttgcgaacccggacagcctgactgatttgctttccgttgtcaaagccgtgcacccaacgattatggttggaacttcaactcaaccgggaaccttcacggaatccgttgtgaccgaaatggctgcccatacggaacgcccgatcatcttcccgatttccaacccaaccaagttgatggaggccagcgccgctgatttaatcaaatggactgatggcaaaggattgattgcgaccggaattccctctgataacgtggaatacaaaggcgttacctaccagattggtcaggcgaacaatgcgctcatctatcccggactggggcttggggcaatcgccagtgctgcatcagtgctcaacgacgcaatgatctccgctgctgcccactcacttggcggtattgtcgatccgacacagccaggggccgccgttctgcctcctgtcagcaagctcaaccagttctcagatacagtcgcaactgcggtcgcacagagcgcggttgatcagaaacttaaccagaaaccaattgaatcagttcgcgatgccattcatcaaactcagtggcagccagaatattaatattaacgggaggacatatgactgaatatcggattgaagaagataccctcggaaaagtcaaagtaccaaagaaggcactatgggggccacaaactgaacggagccgacacaattttccaaccggccctttgatgccggttgaggtgatccgggcactcatcaacattaaacttgcggcggccacagttaaccaagtgcaacagacactaacccccgaaaaagcccggttgattgaaaaggccagtcgccagttgttatcgctcaacgatagccaactcatggctgactttccacttcacgtttaccaaaccgggtcgggaacgcaaaccaatatgaatgtcaatgaggtcatcgcaaacctctgcggtcaattggactcaaaactgacgattttgcctaacgacgatgtcaatcactctcagagctcaaatgatactttcccgaccgcgatgaacattgctgctaccttggccgttctcaaactaaaaccacaggttgaacatttgattgcagttttagccaaaaagcaagaacagtattgggacgttgtgaagatcggtcgaacccatcttcaagatgcgaccccgatcacgtttggccaagaaattagcggctgggtcagcgcgttgacccacgacctccactttcttgacgaaaccagccagactttactggaggtcccgattggcggtaccgccgttggaaccggcttaaacacgacgccggactttgcttccgcaatggtagccgaactcagtactgcatatgggttgccgttcaaaacccaaaatcagttctacggtctggccaaccattcaggcatcacggcaacccacggcgccgtgcggacactggcagctgatctcctgaaaatagccaatgacatccgctttcttgccagtgggccacgggccggctacggtgagttgagcatcccggccaacgaacccggttcatccatcatgcccggcaaagtcaacccaactcaagcagaagccatgaccatggctgcgacgcgggtaatgggcaatgatacgacaattgaagttgccgccagtcagggtaactttgagatgaacgtttataaaccagtcatcatctttagtttcttggagtcagtcgagttactaaccgggattatgacgaactttaccgataaaatggtcgctggcatcaccgtcaaccaagaccgaatgaagcagttagtcgacaattcactcatgaccgtcactgccttgtcgccgcacattggttaccacaaggcagctgagattgctcaaaaggcccatcaagatggcacaaagctgaaagtcgccgctttggcacttggctatgtgaccgctgatgactttgataaatggatgaagccgattaatatgactaataatgatcgaaaataacagtgtggagcaatgagcgtttagcttccagaataaaaggggactatctaaacatccagaggttggatgtttaaatagtccccttttacggccggaagctgctcatttttccactattcggctagataatattaaaaaatgtttttttggggggcaaactattcagcgttaccccagacccataaaatgtaaggatcctcccacatttttaaatccaattctaagaaccgtgaaccatctaccgagtcaccggcccctgccaagacagcatcccgccgctaacattaatcacttgataaccagccttgcgcaaaatccgggccgctcttagacttcgtcgcccagatcgacaaatcaaataccaaggctgtggggcagatacttgggtgatattgccaggcaatccggataacggcacattctttgcagctggaatgtgaccggcttgatactcatcaacctcacgaacatcaagaattaccggcttattcggtagtagctgcttcagttcagatgggctaattgactttatctttgaaaataacaatacataacgctcctttaaaatgattgatatatcgagtataaaagaactctggcaaaagtgaaacccagtttctgattcagtagcaatactggtttgtgaaaagtcccaaaattttgtatggtaaacccaacagaaagtgagggattcattattcgaaaagcaatccacgccgcaaatgcatggctgctctttgccatcggcatcggcatcatttcagcacctttcgacttgctgctacatcatgaaagcaacttttttgacctactcaagacattttttgaaaatggcttactcggatttttaggatcggtactactagtgctggtattgggttggttaccggtatttctgatcgttggttttttcctttggctgaacaatctggtttcaaaacatgactattttaaatagttatccggaaaaaatgtttaagaacagaaatcccaaataagcgctgattaactcaatccagtattcctgaactgacattttaaccgcaccaagccatctccccagatagtggtcacttttgatatacatattattatgaaccgtccgtaatgccaccagggaaaagaagtagatgctcgcaccaaacgccaaggtatgaagtaggaaaaaacttccactccaaaattgacccttgataaacaaaaagatgaccaccaatgccccaattgcaaacatggcataataccaagcggttggaaacaggattgaccacttggtatggatcaacgaaaaaattaaaaaggttaatggcactcgccaagcaaaataggtcgtatctatgatagacgcgcgagaaacaccgaggttttcggttgctgggataagatggctaaaatgcggcaatacgatgagtagggcaatcaaccagataaaaccgccatatattaaaagcgccttaaccacagtgtgattgatccgaattttccccatagatcaacaacttcctttaatcagatttccccctcaaaatattagctactaggttatcatgaaccgaaacaaaataaaactgccatcagcaatcccgatgacagttaatgctacctaacaacttcttgaaaggtcccaatatccagtgccagggtgatcgtcaacaccagaataatttggaaaaaatcggcttcctggaaccgtcgatacacaattgacatgaatggatcaactagaaagtaagccgctactacattcaaaataacaaaaataatcgcaaacacaattcgctttgcactcatgaaaccgccccgttccgctcgccctaatgtgtcgaagttgctgtaagtgtacaaagtttgcggaggtaagtcaagcaacttgcatatggtattataaatataatctaatatataactttgatacaataaaaccccactgccaattgcgacagtggggtctcttttaacgatgcgctttattcgctttagcttcatgaataatcttcagagcccgcttacggatcttgatacttgggctcttcaagcgacgataagcactcgcgagatcttgtttttccatatcgatcactcctttgccgctgttatcttaccagctggccttgtgaacaccagggatctgacccaggtgggcatacttgcggaagttgagacgtgacatgccaaacttacgcatgtaaccgcggggacgaccgtccaattcgtcacggttccgcaatcggttagggttagagtcctttggcagcttggccaaggcctcatagttgccttcctttttcaactcacgacggatgctggcatacttttcaatcaaggcttcttgacgtttattctttgcaatcttagacttctttgccatatgagtcctccaaataagtgtatttttgatattgtgggttttaggttattttgtgtacactcaatagtaacggttactattatgccaagaaacgtcggacctgtcaagaataatcattaagaagcatgggaacgtcggtgaaatcgatacgttagctcgataatgataatcccgccccacaagccaatcggaaccgcagatgcattatctccaagctgaaaatggaagtaccagccagccaacacaatgatcgttgaaataattgccaagagacaaaatatctttctcaaattcggccatcgtaaaatggtcggtcgagcatttaactcatcctcaaaccgtttgacccgcaccatgacaagcatattcagcagtgccactaaaagtaggaacacgcctgcagctccgccgtgtcgaataaatatcatactgataataaataaaatatcgatcgtgattgtaacctgcttaatcggccggatccattccaaggcttcttttttctttaaatactctttcatcccaacatcctccttcaagaggacgtccaatgatatatggaatagatcgcttaactgaatcaaactgtcaatgtcaggataactgttttcagtctcccaactggaaatggtttgtcgggaaacattcattgtgtcagcaacctgcttttgcgtcaaacccaattcaatccgttcagtttttaatcgtgcaccaaatcgcattgtcatcctcctttcttatgagaatagtgtataacgcaaacccatcagaaacctagcaaagaatctaagcatgctattatacaggtatttagacgaacagagtgacgccggaatcccacacacaatgcaaaatcgtgctgggccagagattcttggtacgataaaacatccagccaaaaatgaggccaagtggcaacacattggcgatgttaatgagccaagcgcccagcgtcagtccttcgagatagtaaagaggaaaatgactgatctgaaataagattgcttggataatattggcggtgacaatcccgtattgcttcatcaaaaagttcatgaagaacccccgaaataagaactcttcaatcaagccggcgcccaaagtcacactcaaaaactcaccgcttttgaacggatcgtgctgaagataaaagccacggtgggcactaaacatcaaaaagaacaggtaagcaataaacattgccaacacgatccaaaacacggtcggaaagtttccgttataaagtttgcgtttgtcaatccataattgggcgttcgtccgactaatccagaacagtcccaggccaaccatgatcacggctttgatccccaaactgaccagatcgctcgccatccctgtcgtgtagtgatgctcaatgaaattgataagttcgcgaccgaaaagccagagtacaatcagaaacacgtaactcaggtaaaaggtcgtcatcgaccaggttcttctcaaaataatgccttccgtttcgtcatatttagattttgattatatcactatccgagaacaaccaaaagtgagcgacaaatcaaaaaaaggccggcgcgcaattcacaagaattgtgtgccgaccttctcaatggtcatgattaactatcagtttcaacccagtgctttaacaggtagacacttccaacagactccaacgcggtaaatccaagcaggtaaatagttgcgtaatagatacttgcaatcgtatctccattcatattaaagaagtggttcataacaccgtcgactcgattttcaatgatcgagaagacatatagaaaagctacaataacaacaacgtacagaacgaacctaaagaatttttgccgagaatcaggtaggaaagccgtcaaggcatccccggtcaaatgaatcagcgtgatcgatgcccataaaagaagggtcatggcaatcgctaataaaatcgcaccgatggtcaccagaatcatatttcgaacaaaattttgcttatcagaattcatggtgtagtgaaacatcttcttaaattgagccccaaaatctccccaaaacggaatcgcagcgatcacccacagaactacctgggtaatgccggcgtacaccatcccgatgaacgaagatagcaggttaacagagtatagcttggtgtcacttgccggaatcaaccggtaggcgtcgctcacgaaaatgtgctcactgttccgagacatcaacacaaaggcaacgatggcgacaaataccgagtacgaaagtgtgatggcaagtggcgtatcggtctccagatctccgcgataaacttgataaatcagcgttaatacaatggcaatcacatcaattaagacaatccggttcatgatccgcaacttgggccgagtcagcgatttaagtaagtcatagaagctagtcatcaatatcattcccttcataaatactttcgtaatagtgttcgattccttcagcgtactttgaacgaatctcttcggcactcttctgtgcgtaaactgttcgatctttgatgatcacgacttcatccaagatgctggcaatttcggaaacgtagtgatcggaaaccagaatcacagcgtcatcactcttccatttgatgatactctgaatgattttcttccgtgacatactatcaatcccgccaaatggctcatccaacagatagaccttggtatcacgtgacagcgtcaatccgataatcagtttctctttcatccctttggagagggccgataaccgcaaaccttcatcaatctgaagaaacccagccatttcgttatactttttggttgagaaatccgggtagacgtcctcatagaaacggataatcttatcaattcgcatgctgggattaaatccattcaactgttcactgaagctaatggctgatttcttgtctggaaccccatccgtgccggccacggtaatgctgccggaagcacccttggcaaccccggcaatcagccgcatcaatgtcgtcttaccagcaccgttttcaccgaggaggccaacgattttgcccatctcaatgtttaaattaacgtcttccaaaatgcttcgataatttctccggtaattcaaattcttgatttcaatcgtgtttgtcatgattgcacctgctttctcttattgatataatcctgcaaataatcgacaatttcctcatcgctcacattgagtttgcggaggttttcatataaatcctggagttgttctgtaatgaggagctttttgagcttttcaatcgtttcccgatcctccgtcacaaagttacccttgccacgctgaggttcaataattttctctgaaatcagctcgcctaatgctcgttggacggtattgacattgacggtaaggtcaacggccaactgccggacagccggcagcttgtcaccaggggccaacttacccacgataatttggcgatagatataattcttaatctggtagtaaattgggatcttgtcatcgaatttcattgtcccacctccctagtgttatattttactattacactataacgccattttggcaaaaggacaaggaaaaccattattattaatcatctatgcaaaaaaaccgctacacagctacgcgcaacggtcttgataaatcaatttttattaacaatcttgccaccatccatgtgaatcacttcgtcacttagatatgcaatatcttctttatcatggctagcaagaatcacggtactcccagcatcggcaatttctttgagtgtctttctcagaagccaagtgctttcttcgtccaagccattcgttggttcatctaacaaaagtaacttaggccgttcgaagatcgcttgagcaatgcttaacttctgcctcattcccaaagagtagttagcaaccttcgtgttccagtcgctctcactcagtccaattttcccaaatgcactcttaatatcctttgttgttgcaattcttttaattttcgacaacgctaccaagttttggaaaccggtaagatccttagggaatgttgtattctcaattgttacacccatactctcagggaaatcaaacttatcatggagaacttccccatccacaattacctttcctgctgttggaattagtagtccagcaattgatcgaatcaacatagtcttccccgaaccatttcgaccgactaatccataaatttttcgtctttcaaagttatacgatacattatttaaaaccaaagtatttcgaattctcttagaaacattttgtacttctactctcatttcttatcctttcaaaaaatcatagttcttaattaaatatttaaattgcaagaccaaccatgataacacaataacgccggccacaagaacgactttattgtttgataagattaccctgctatagtttataaattgtggagcaaaaatacctgtaacctctcgaagcccctttaattgaaacattgcgtgccctataaataagcatccggaataaataaccaaagtgtttaagtaggccactgcaaccgtgtatctgagtactatcatcaaaaatgttataagtaaagtagcccaacccagaaaggttattacaagtactgatatagaccaaacgatcggtacacctccaaacatataattagctaccatttgagtcacgctctggatgatcacaaacacaaacacattattggttattccccatgaaattttccgacggctatgatatcttgatataatactagtcatatgggaaagtaaatttctatctaaaacagccgtgaattctccaagtacacacacaagtaacagtatgcttattgcaaactggattgaattaaactcatatggaacgtcagctataccatgaaatccgattaattcattgaagaagccaaatgttaggtttacgattaacagacttcccgctatccttatgactttcataaaatgtcctcaaacttaattcgcaatttaacaagcatacgcatcaaaatcaatattaatgatagtctcgcaaccgaaactacaatatccatgatagttagctgattctcaaagaataacgtaaagtgatttatttccaacagggggtcccataaatggagcctgggaaaaattagactaattaatgcattggtcactataactattcccatccccaggtagtatggacgattaactgtcatcagccggtaaaactcgccaatgatactcaaaaataatcctgtagaaataatcgtttcaaaaattaatatccaaaatgaaaaatttgcaatcatcgtacctaatgcaatttgcgccaaaaatactccgacaacaatatagagagcactaaagatcagactgtcagtcgtcagagttctctggaattgtttatagcggcttactcgtgacatccgataacagtgaacgtagcttaactggttatttatcataatcagacctacaaacatattagagaatatcactccaaacattgaattggcgaaatatcccgagttagtttcaaaaagcatttgcacattctgcttgaaagtatagtgatccgataaaacagcgttgttaacccagtatgttattaaaaaaatgcccacacctgacaaatataaggcgcaatacatccacttacgtttatttgaaatagacatgcttactccttaatctgatcactacatttcctattgtaattactaccacacaaattagtaaaaaactaatcagtgaaccaatgtattcattccaatcatactcaataaatggttgtgtaaagtatgaagagctatatggcaaagcaatcatgaaaatccataagccaagagatataggatacaccaaaatggttttcctaatgctaagggcaagtacatatataactaccgaaaatagtccaaatgcaaggctcactattatcacaaacaaaatatatgctacgtatgggtgctcaatttccaaatgtaaaaggtgtgaatactttgctgaatcctccatccccataaaactcgtgcctttgtgaaatagaattatggcgacaacaaaatcacaaccaaataaaatcatataaaatgttgaaaagataaagaattgaactaactctgacctaacaaaaaacttatccagtgttcccatacgtgtactcagtagataattgctgccaccatgagttctttcaattatccgctgaagtgtaatcattataatgaaaatgggcataaaccaaatcagaataatctgtaaaaattgacctgatgaattcccggctaaaaaggcagcagtaggtgggttaatgatctccttgctggggataccatttggatataactgaaacaaaccaggaaagttactttgccatgcgagaaattctgccagcaatacaattaatacgcaaataaggatggttctcttacttcttcttgaacttataatggcactaatttcagataacaacatcgaatagacctccaaaataccaagaatgctcacaataaatgtgagcattctatgcggcagtcaacatactaatcttcaggattccaataaccgctgacctcaggttcattcgcattcaaattattattctgcgcagtcagtgcaattaaagctccatttgcgtcactattcgcactgtacttatgttctccacttccctcatggatatcgtaagatttggaaacattacgattcaataatccagtattctcaatccaataggttgccaccgagttagagcccttctcagtatcatgttgcatgttaaccatccagggtttagatgtattagacctatattcatcctctgtctgtccattgcctttaaacattcccagcttaaaatcaaacactgtatcgacatctgcactcacttctgtcataaatgatggggcaacagctgccacactcagtaaagaaagagctgcgtaggttgctaactttttcattcttgaaattcctcctaaataaatttaataaagcattaaagaatagaatcttaaaaatcctaatgcttcagaaccattatttcggaaaagtggctggtttacaagaaagcattacttgcgcaagcaacgcttgatatttgttcagcttacacaaatatttcatctttatgtcaaacgttaattcggcgaaattttgacaccaattttgataatattcataaaatatttaaagaatattcatacatttttcacatccatactgttgaatgtaattatgataatattcgataaatggaggtagaatgataaatcttggaaataacttaaaaaaaattcgtgaaagcagtgaactttcacaagaaattattgcatctaaattaggggttagtcgtcaagcaatttctcaatgggaacacggtcttacttaccccgatataaaaaatttggtaaggctaactcaaattttttgttgtgacattaacgaattgttattttaaggaacagtaatgatacatctaaactttgagatagggttataaatacacattgaatcttcaccaaaagaggtcccaggcacaacttcgcctggaacctctttgttacaagtttttaagcacttgaatttacaatttaagtgcaacactaattaaataaagaatggctcatggccaatttcctgtagaatgatgtttgcgagaacaatcatgaaaggaaactagccatgaaccactacaagcatattaccatagatgagcgagaaacaatatttttaatgcggagccatgggaactcactacgtgagattgccacgaacatccagaaaagttgttcaacggtttctcgagaattgaatcgaaattcagatggtagtaattattcaccatcaaaggctcaagctaagtaccagcaacgcaaaggtaattgtggaaggccatcgctcttaggtcagccacaagtatttgaagtcgttagggaacatttctgtgaggatctctggtcacccgaggaaatagcgaaccgcctagcggtggaaaagcacgccgtccaaattagtaccacgacgatttatcgtgggattttcaagggcttgtttgatcacttatttaagtctggtagtcccagcgcggttcgccatttgagacatcgcggaaaatcccgtcataataaagcttatcaagaaaagcgcggtaaaattccgattcccaacaagattcacgaccggccccgagaggctgataatcgtctcgaaattgggcattgggaaggcgatacggttttaggcaaaagtggccgagcctgtgtcgtgaccctagttgaccgcaagtctcgctacctattaattggtaaagctagtcaaagaactgccggtgcagttaccgacacgctaagccatttaatgaagttatggcctggccgatcattaacgattacaccggatcggggaaaagaattcgccaaggttcaatgcttcctgaaaagtttggcacgcccttttacttcccggatccccattccccttggcaacggggtaccaatgagaacaccaacggtctggttcgcgaatacttgcccaatgggaccgatattgattcaattacggacaagcaaatccaagcctatgccgaacaactaaataatcgtccccgcaaatgtcttggctggaaaacaccgtctgaagtgttctttaatgtggtgttgcatttaatttgacaattcaagcttaataaaaagaaaaccgctgcatctgtacctgcaacggtcatccaaaagccatcaaaatatggcgatctaagattagttgtcgctcaaaatcgactcaacctaattcctgactcgaactatccttactaaacacttaagtaaaaagtagaattcttaaaatgtactagtaatgaatgtcgagaacaataaatgtaatatagattgctgctaatattaatataaccaatcccaacagaagaattatttgcataattgttggctttgttcgccttttccccaataattttatgaatacggatgttacccctattatcaaaaaaactatagcaattccaattagcattagttgtctccttaactcagtttttgattaatagtttttatgagtaaattacagtttactttgactggttgaagtcagagaagcaattggaaattcatccgtaagtgtgatccgacacccaccttttgattttccattattaatcattgttttcacatccgattgtgctgatcctgatcttactgacagaatacctcctgcccctgcaccaaagattgcgccaaataatcccgccgaaattacgcccacgacggctcctccggtcaccaactcatcttgaattaaaccataatacgtacgtaattttgctaatgcactggttgatcctgcaaaatcattgactccacccttgactatcttttcatgaacactcgcaggctttgtaatcgaacgcagccctacttcattagtagcccctgcatcgttgagctgaatatctgcttcagcaccatcatatttatttaataaatcttgcatttttgcgctcaattgatcctcgggcaagttttgctgagataataacttacattccttagaaaattctttccactgctcattagaattggctaccgtaacattttgatccgaagcctgatctgtatccgaaaattttgtggtgctgtcactagccaccaaggatcgggcagaactatctgcattgacggttgatatgtcttgaaccgccacggaagataacaacaccgctgacatcatggttacacctatacgaatacttttctttctatgtttaatactaaaaacctccaaaatatgagtagatttatttatatttcaaaacccattatttcggaaaagtacacacattgcaagaaaggattgcttgcgcaagtattgcttgatattaactgagcttacaaaaagttcatccaatacttttgataatattcacaaagcttttaaacgacattcacacattattcacacgtatactgtcgaatgtatttatgatactatttgacaaatggaggtaaaatgataaatcttggaaataagttaaaagagtttcgccaatacaatgagctttcacaagaaattattgcatgcagattaggggttagtcgtcaagcaatctcccaatgggaacacaacctcacataccctgacatcgaaaatttggtaagattaacacaaatttttgattgcgatattaacgaattgctattctaaaaaggaaaaatgcagccaatcatttaaataaagctctcaaatttcactaaagaggttccacacattagatatgtcaggtgtggagcctcttttctaattgatttttctgaccagtacataaacaattattacaaagttcgccatataggtgtcagtgaacaagttgtcaattgatggttcgctatgagtagagtaacctgtttacggcattgttaattatgcaccagccccggcaactctttgccattcgcatcgattgccaagcgaaccagcacaaccttgctggaatccaccggcaggccgtcaatatagacttcccggtgctcatttccgtgcaggcgtgtgaagccctccttttgaatcgcattttccaaggccttcaatgcttcactgtccggggtcactgcaccggtattgacggtctgaatttcaatgccttcagccaaatgttcaaacttgatttctcccaaatcaaaatctgagaaatcaatctgagttaaggcagcgtcgaagtccttttcgttaatgaataacggctgtttaatccaaatcttgaagtcttcaccgtctccggtatcggtccaaaccgcttggaccgggtatgggcggtattccttgaagccctcgaccggaatgccctttcccgggccaccgctgattgtcttggcaacttctgcagccgcattggaaagccgtaagaagtcagggtcgtccgtgtgctgggtcgcatgcccttcagcagttacataacttcgtgtggtcagatcaacaaagctcggttctttatctctactgtactcatctggttcgaatgtctcccaattaaacatatgaattccccctttgatttcgcggtcaatataagctaaatcggcggggaaagcaagcaaagggctcttattcggactgtaatgattatccaaaaatgacgattaccgcaacgaagatcaggacggcgacggggaggatgacggaactattgagattcataaatccccaaaagttcatttgatcatgattacttccgatgacaatctttttctgcagccgctcgtcacccttaatcaagctgtccaaactaaccgcaaataaatcacttaactgaaccaaccgttcaatatccggatatgctgaaccaacttcccatttagagatagcttggcggctgacatgcagctcttcggccaatcgatcctgggtccagcccaacttttcacgttcttctttaatgcgttgtcccaacaccatgttaaccacttctcttcacaaatttgattgttattattatgccattattagtcgggtgatgcacgctcatcttaagggcgatggcgtgcaaccagtcgttgcggacgataataatttttaacaatgcttttgattgctttccatacccgaccacttataattaaggtgaatcacgtaaccgatttcatttattaagggggattttatcatgacaatcaaaaacgtaacggttgcaggtagtggggttttaggaagccaaattgctttccaaacagcttttaaaggattcaacgtcacagtttatgatattaacgaggatgccattaatgccgccaaggagcgaatcaaggggttgcgacacagttatcggcatgacattgcggccactgatgccgatttcgaagctggtttatcacgaatcagctatacttgggatttggcagacgcagttaaaaatgccgacctggtcattgaagccattccagagcgactagacatcaagaaaccgttctacaacaagattggtgagatggcgcctaaagaggctatctttaccagtaattcatcaacgctggttccaagtgcactgatggaagataccggccggccgagccagttcttaaacatgcactttgccaaccaagtttggctgaacaacaccgctgaaataatgggatcgccaaaaacagatccaaaaatctacgatgaaattgtcgaattcgctcgaaacattggcatgattccgattcagttaaagaaagaacaacccggctatattctgaactcactgttaattccactgttgagcgctggtgaagaactttgggtaaagggggttgctgatccagaaatgattgataagacctggatggcagccaccggtgcaccaatgggtccatttgccattctggatgtcgttggcatccggaccgcttacaacatcaccgcgacccaagccaagagtggcgaagatccaaatgctcaagttctcgctgacaaactcaaggaattgctggatgccggcaagctgggaatggaatctagcgaaggcttctaccactatccaaatccagcatataaagatccagactttttgaagatttaaggagcaacatgccaaatcaaaaacgcttcaggagaattttagttctcttgaagcgtttttgttcattggcaattaaattctgtggttaaagattgccctgattattttgtaaatgatccaaaggataccagccgtgatcgcaagactgattactccggcaataatcgaaaagttcataagaatactcccatgttgagataatttaaagtcacatctttaggttatactaaaaagatattctgggtcaagaaagcatccctttccccaaacgaggtattgttcacggaatttttcccaaccacttacatcggaaataccagaatttttatccaaaacgataattaattattgtcttgcaataattaatttccgcgttacaataatatcaaaagggagtggttaccatgattaagaaacaaccaaatacgttcatcaactttttatacgttatcagtctgctaagtgtggcttcattattaattgcaatgggaactttggcacttgtctttgtgattgctggaatcgtttatctactaatcccatctgctcgtactgggatttttcgcgatattataagtggaattggcggatcgacgaacatttgggtgatctgcttatcatttgcattattgctcattatattgggattaattacccttgtttcattttcagtcttcaagctgattgcaaatgtccgtcgaaacatctatttcaagccaattaatttaaaatacatccaaggtattctttgggggtatgggggtatcattttaaccaactactgtagcggagtcttagccgacacctataatattaactcatcgtcgatttcatccgaccaaggaggcgacggtacctcgctactcatttggtttgccctctacgtgatctatgtaatgttcaaatatggcatcgatcttcaagaagactcggacaaaattgtttaggcggtggtgtctttgatcaaagtaaatctagacagagtgttgttggataaacaaatcacttcaaagatgttggcagcagaaattaatattaccccagccaacctatcgattcttaaaacggggaaagccaaggggattcgctttgagactctggcaagaatttgtaaagttttggactgccagccaggtgacattttggaatatgttccggagtagaatactgagaagtcattcaatgattaggatttggatttaatagccccttgataatcacacggtacacacagtttttcgtgaaacataaagctgttctgcaacttccgtctgagtaacatgctgcttgcttcgctcaactttaattttttctccgaaagtcatttcagtcacctccaattttaatatacggataagtggtgcgatcgacaagataattctttgatattggacgctaagaattgtaacaattaaaaaccaatcacaaagtttgcgtttgaattcattcattgaaaggttagcctccaatttgacaatatgaaataagatcattcatccgtcacaattaccgtcatccactattcagatatcccgcaagacaaaataaaaaagttaccttagatttacgtaaggtaactacttgctgacatctatgatttttctctccaagtcacaagaattactaagacaggaataaagatcacgtttcccactgcagaccgatagtgcccaagatatgcattgaggccggccaagataagaaagcaatggtgatgaataaatttttggtcttgagtttcacggtttaaggatatcaaaaattataggttgttgcatccctacttactgctcttaaacaatctcctaaacaggaaaaagttaaccaccccaagcaacgccaacatcgcaaacgccagccggctgccaacaacaatgttttgcacataagacaaggtgtagatgtgcaccgacgtcatcatagtcgcaatgaccgtcgttccaagcgacccggccaacatattcccggtgccgtatatggcattggcatccttctgttcatcctttggcaaatgtttcaagccataggccatgctattgccaaacgccatcgaacggcccgttgcgtaaaccgtgtacagaatagtaatcaccaaaacggacatttgttgacccattaccatcataatcacaatttgaacgagaaacagcgaattccccaagtaaaggggcagtttgccgccaaatcgatccagcatccatccataaatcggctgccccaatccgttcaggacactcccgggcagcaaaatcagcccagcaataaaggcactggcgctgttcacaatttgtacatagcttggcagcatgaagttcaagccgatgtttgaatactgtagaaaaacatagggtagaaaactaaacaaaaataccggtcgtttgaagacggacagtttgaataatgctttgtgactggattttgacagccaaccgaacaagcaaaaggaagcggcactgaccaccatgtagcagatgaatttaactaaaaatccacgctggcccacaatattaaagcccatgagcagggtaatcatcgctaacgccagcacaccaaaccgcagccagtcaaactcatagtgttcggtcggcgtatactgcttgataatgaagatccccagcagcaatagaaccagggtaatcggcacggtgatccaaaaaatcatccgccaactggcaaaggacacgaccgccccaccgaacgttggccccaacgctggggcaactaagacgatcaagttggccatccccatataggttcccaatttgtgggcgggaacaacgtccaaaataatgttattcattaatggtccggtcaggccaacacatcccgcctggaccaagcgtcccaccagtagcgtccaataatttggcgccaaaccgcacatcacatccccggcaatgaacagcagtgctgctgacacaaagagctgtttgttggtgaaccgccgtttcaaaaaggctgaggtaatcgtcaatagcgccaccatcagcagataccccgtggtcacccattgaacggtgggcagggaaatgttgaactggtccatcaaagttgggaaggtaacgttcatcgatgtttcagtcagcacccccataaaggtcatgaatgccacgacggtaatcaccaggaatggatgctttttggcgttctcattttgttcattaacagtggaatccacggtgttgccccctcaaaaattcgtcatagtcgaattaactcgcaactaatatactaccatttatcggggagcgtcgacaattaaatttgtggggtatcaatgacctcaaatacttcgcagataacgggactttccagcgaaaaggacttgccacgcatcttggctttcttccggaaaagctgtttgtgcagttgccgccaatatttcagcgaccgattcccttcgccttccaaataggcgtgttcttgagacacccatttgaatgggacaacctcgacaactttaagttgaacaatgcaggccggatcgccgttccgcttgagtaacatccgatagtcgccggcctttggcaccacccggtcggcatcataaaaatcaaaccaggagctggcagcggttttctgtccacgaaccaccatttcaaccaacatatcagttgaattgggccggttggtaaacgaccacgtttcaaaattagttttctgggtacggttgcgacgcataaaatcttcccagtaatcggtcgcatccattttcaaaatatccatatgcattcctccgttcatttatgattgatggacatagtttactgtggcgagcttaaatgaagcttatgtacaaaaaagttcccgcacgcctgcaggaactcccatttcatttcatcattattttcgatttcttctatactatgtgtcaggtttcccctggaaaacatctcgacttctcactatgtcatccaaatctctgagttggtccgattatttaatccaaatgctggtatcaaccccctcaattgcttctaagttagtgctgagccacacgagtggtttgattttggtcaattgtttctttaatcgcactgcctaagcgctcgattccggtttgaatctgctcttcagacatgttggaatagtttaatctgaaggttccaggagtgaccttgtcggggtagaatggttcacctggtacaaaggcgacgttgtgcttaatgcaggtgttgaataatttaatggtatcaacatctcccggcacttcgacccaaatgaacaggccgccttgtgggtgactatagttgacgccagctgggaaatacttctcgatggctgccatcatcacattttcacgtttgcgataaactttgcgaatcttgttgacgtgctcatcaatgttatattcagccataaatttagcaacaatgtgttgggttaaattatccgaatgaacatctgcggattgtttcatcacactgtatttaggcattaagtctttgttcatcacgatccagcctaatcttaatccaggcgccaagattttcgagaaggtacttaagtaaatcacccgctcttcattatcgtagaacttgaccggctcaatgtcgtcgccggcaaaccggatggccccatagggatcgtcttccataaccataatgtcgtacttgttggcaatcccaatcatttgttcacgacgttcagccgacatggttcgaccagttggattttggaaattcgggatcgtataaataaatttggtgttgggattagcagcaacggccttttccagttgatccatccgcatgccgtcttcatccatttccacgcccacaatatgggcaccgtaactgcggaaaacgtctaaggcacagaggtatgtcggcttctcgacgatcactgtatcaccaggattgacaaacattttagccgtgatgtcgatggactgttgcgaaccggttgtaatcataatattatccgcagtggctttaatgccctgtttgttcatgcgttgggcaatttgctcacgtaaggcaggataaccaatagcagaagaatactgtaatgcttcccgaccactctcatcgaacacctcattggtgactttctttaaggcctcgatgggaaataattcaggggcgggtaacccgccagcaaaggaaatcacatctgggctgccggcaacttttaaaatatcgccaaccggatcgctatcgtttttgggaactcgttctgaaaatcggaaactcatacgcgaacacctgccttctgtgtgtcatcattttgatctgccacgttcgtttgcggttggtggtatttccgcatcatttctgccatgtgaacttcttgaaccacaaactcgtgggttcggcaaacgtagtcgtgttcacgaccaattttggcaatgtagccgttaatgtaatcaacttccgttggtcggccctttgagaaatcttgatacattgatggaaaatgatatttgtattccttgctgacactaatgactgaatcaacctgttcctgacgagtggcgataagataaattccggcccgttcacaagcgtcataggcttcatcaaataattgctgcgacatctttcgaacacccggatactcgatgaactggcccatttgcatttcaaacattgtacataatgtgttcgtcacagcgttgaaaacaactttggacatgcacatgcccatccattcgtcggcgaagaccggtcctaatttggcattggtgaagtcgtcgaagatcgcttgagtcttggtgtccggcttttcgttgttgtaacgagccatatgcatgacctcgtcaccctcagcccccatgaaatcaatatcagctgggccatccattcgagtggcaatcatcgcagtcccacagataatgttatctttagggaaatacttagcaatcttttcaaagtggcccatcccgttcatcgcagaaaagacatattgatcatcatgaaagataccggccttattatcgcgctctaattcttcagctaactgcatctgcttcttgaaaacaatccaaacatccgggtgacctttatattcttctggatagtagatgttgattggaacaatgcgtcggttttcgtggtcacgagcgacagtgacaccgccttgttcgcggatcttctcaacgtttggctcccaagtgtcgatgaaatcaacgtcgaccccggcattctcttgtaacattacgccatacctaactcccattgctcctgcgccaataataccgtacttcataatgaccactccttttattttttatttaggacagctgcgtcaggcagaaacctacgcataagcaccttgcccaaaaattccaaaaccaggaattcttgtccaaggagacttatgctccggtttctaaccgcctgactccgctcactacaaacaaatccgactaaaaaaacgccccttggttatcaaaaccaaaggacgttaagttcaacgtggtaccaccttaatttgagttgtcttcacaaacaactcctcgaagcgtacgggaaaaatccgatacgccggcacgttaatgggtgctaccattccacctcgaaaagtgaacttattttgctcgatctttcaattcatagtcttaatgccctcacaccaaccaggcactctcttggtaaggctgtaaatctaatccatcggaccaaatcaattagtcgtatttagatgttgcatgaactatagctcatgaacggagaaactgtcaacaacttttttacacttttatgagagcagtctcatgaaaattccattttatcaaggggttgagcggcttaaaaatttttgagaacttttgtaattggtggtcgatttcggtatactcgatgtatcagttagattaattggaggtgaattgaatgcgggcattaattggttttgccgggttaatttcgatggtgatgtgtatcgctgccgtgattttcttaatcatgggtaatcgaactgtcgctgttcctttggtgagtgttggattggttatcttgattgtctgttatgctgcagcaacatacatttctcattctgataacaaaaaatgagattattttaatacataagttgaaacggagggctgctgcatgctgatgattagaacaattcgtcaaagtgactattcaaacgtcagtaacttaattcgaacagcatttgccaacaccgccaatggctatcggaatgaagccgaattggttgataagattcgaaaagaccctgcttaccaaaaacgattggaagtcgtggccgaaaatgggattcacttggttggctatggcttactgagtgaaatcaaggttgtcgatggtgccaaagcatccacagggttggtattagcacctttggctgttgaacccggatcgcaaaaatccggtgttggcagtttgattatgggcgagctcgataatcgggcaatcaaccttggctatcaattcaccgttgtgaccggctggccggattactatcctcgctttggttatcagaaggccagcgattatggtatcaagtctcccacaccggttccagacgatgtcttcatggctaagccattggttgacggcggcttggatggtgttcatggaatggttcagtactcgaaagcttttaacatgtaaataaaaaacggaaaccaattgcaaacatggtttccgtttttgtatcgattcaattatttaatggtggtttcattttcagacgcagctactttgcttttcgcaactgcctgagtggcaagctttaccaggaattggccatacttgatcaccacgaagacgaccataaaggttgccagggtgatttccaggtttgcgaccatcccaatgattgagttgagaccgtttcccaagtggaaactgttattaaacagattcaatgctgtggcagagatcaccaatgggaatgtaaaggcaccaaaactgggataaaaggctaaccgaacgtacttgaagatcttcgtcagagttccccaatacaacccttgtgccaggatcaccattgctaaggcgaatccccacgatgggttagtattcatggataggtaacccgtcaggcacaatgatgccggagcagccataatagtcagtagcggcaaggttgcttcaaacataaactcccgtcgaagcaggcgaatgcagacaatcggcagcagaattgcatagagtcccaatgacaaccacagtactggtgtcccgagtgccggaatgaaattatttgcggtaaccggaatcactccgattcccacaaaagttacgaaccaacttggatagacatgatcgagctcaactgtcggacgtaataaatggcggtagataaaataacccataatgacaaattgcaaaatcactgcgaacgtccaaacggctgtgggtaatactgggagtccccatgatttcagaaaagtgctgataatcatcaaagacatcgtgaaggttggggcaacggatgcaataatcgggtcattcaagtcgttcagactcaacttaaaatgaacgccaatctttgcgatcaccagtaaaatcagaaccagggcaagaatcccccagatattgccaatcactggtaagccaattgccttaaacaggtttcccaacgaggcaatcccaagaattaatccacaaattggtaaaggtaacttcttcaaaaataacttcatacggtcgtctcctctcttagatgagcttaataatatcatttatggtagaataaataaaattgatagtatttatatttgttataaaccaaatttataaggagtgccaatatgtttaaattcctggaaaccttcatggttgtctacaaaacccgcagtttttccctggctgcccaacagctctttatcacgcaaccaacggtgtccaaccagattaagcaactggaattgcagctgcacaccgaattgtttgaacggagaagccgccgggaaattgtgcccactgaagcggccaacctgttatataaacgagcaggcaagatccttaaaaactggcaggacgttaacgatcagatcacccgcttaggcgacaaaggaaatgaaaaggtgcttttcggcatatcgcaaaccgtttcgcgaatcttgtttgctaaaattgccagtgcactgataactgccgtccccaacctcgactttgatgtgactgtctccaactccgagggcgtcttaaaccagctggaaacctacaagattgatatcgggatcatcgaaaagccactggttaccgagaacatctcccgaatttcaatcggtaaggatcaactggtcaaagccggcgtggacaatggcaattggatcactcgagaaccgggatcgggaatcggctattataccgaacagtatttccgtgaagccgatgtccagcccgccaaactaatccatgtgaacaatagtggcctcattcgtcgaatggtggcaaaaggcgttggtcaagccctgctgtctgacaaggatctacctaccgctgttccgattgaatcacttggggaacatttttcccgtgatttttatttattggtccgagaggaaagcagtcacgacaacacgctgaacaacatccaacaaatcatcaataaagcaatgtcttcccccaatcaagattagttctcgtccaaagtacgcgtccgagttgctaatgatttgaaatgatcatacgtcatctttagtaattctttgggtgcagcgtcttccaggattttaatcttatccggatttgcggccggtcggtccttgtaaatctgactgttaacatgatgggatccctccagcaaaataaaggccaggtccgtatcagtattttcaattcttcgataaataaaatcgccacttcgctcgttgggatccaaaacatcgatattaaccccaaatggttcaaatacccgtttgtagctaatctgcttgaaccatgaaaccacctcaatattcttgccggttaaaacatctttcacatcgggataatcgattgtaaaccgctcaacaaacccttttgccgataatttggcggcctttttcttaacttgatgtaattcagcggaacgatcgcgattttccgttgatgcagcgtaatgtttgttaatcacaaactgatcggtggttaaattatagttcccgcgatatacatcaccttgattgagctcaaatttatttcccttcacaaccggattcgggaaaaccgatccatctaaagcaataaactcaggttggtcatcttgaaagtggacgtagccatacatctgttgattatctttcagcaactctgatcgccgcaaatgaatcttagtattggccatccctgtcttcaaataataatcaatcgtgttaaaaagcggcagtaacgataagaattcacccactcgttcctcgtcaattctggcaaataattcgttgattaactcttgggtagttgcttgccggacgagtttgcctttgcccggcaattcatagtgccggtattgatggagctgttcttgatacttggtatttcgtttttccgagctcttcaagtgagcctttgttttttcaagttggtccttgtaatactgcttatccgctttaacctgctgagctttctggtactgtgagcttttaataaaatggcggatgccggttcgcagacttcgattgcgcctgttgagtaattggatttgctgattaagttggtcaatcgtttgtttcaactgcatttgggtatgatagtcagttgcctttagttggtcggcttcttgaagtttaatctgggcattatggactttgccctcaagttgatcatttgcttggtttaatgcaaagttttttgctttgagccgttgcattatttgctcttgggcattcttctcactttgaatagcccgaacttttttctgaagctttttattctcccgttttaacctgctcttctgtctgtcgctatcggtgtgctgcgaagcttgatttgtttgctgaccacgatttgtggtggccttttttaattgggtttgctttttctttgcctcttccaaaattctgtggaatctttccttagcctgttgtttatccttatctttgattgctttgatattcattggcttaaccattagcttacctctcacccgttccacattgtaaagttcataaattaattgtaccaaatttcacccctgatgactcgttaacataaacgaattgaacaaaaataagctgaaccacaaactcaccagatccaatgatcaaagagtctatagttcagcttatttgagtagatacattctttaaattaccatcttaagcctggtcgcacttacagcagcactccggtagattttttcgatggttttttcataatcactattggcaacgccaaagacgactttaatatcgctgccttcttggaccaccaaatgaatcttaatctgactgttatccaaaaggtcgagaatcttaccagcgattgccgggcgcttactaagttgggaggaaaccgccgcaaccatagcgatgtttttctccaacttgacactgtctaaatcgcaggctgacttcagtgagttgacaatcgccatcaatttgccgtcaacatcagtccgcttcgctaagaattgaactgaatcggttccagctggaacgtaatcaaatttgacgccaaacttttgaatcacggagaagactttggccatcacatcaagacgtttgtttaattgatacttttggattgaaatcaccacataatccttcttaccggcgattccagttaccaactggtgagcgttactgttcgcagaatcgactaccagagtcccgtcttcttcaggatggttggtatttaaaatggcaattggaatctgcttttctttggcaggttgaatcgcttcttcttggaagacgctgatgcccatataggacagttcttggagttcttcataagttaattcggtaatcttgcgggagttattgataatccgaggatcagccatcttaatgcctgacacgtcagtccagttctcatagagatcggcatccacaaagttggccaacagcgcaccggaaatgtcacttccaccgcgaggcatcaagtgagtcaaaccgtcttcatcaaccccatagaaaccgggaacgacgatgtggtcatcgtagcttaaaaagtcgcgcagacggttaatggattccccatagttgacgccgttttggtcaaataccagaaagcgggcagcgtcaatgaattggtagccaaggaaatcggccattaatttggcagttaaaaattcgcctcgtgataccaaataatcatgactgcagttaggaatctgcttggcaattttctgcaagtcggtttcaatgcccaccttcaagccaagggcatcccgaatgccgacaaatcggctttggatgtggttatacactggcatgtaatcttcaccggcatctcgaagcttctcaacttcaattaataaatcggtgactttaattgcctcactatcactcttacctgcggcactcaccacgattacttttcgatctgcatttgcttctacgattgcccggacctttttaaattggccggcatccgcaactgaacttccaccaaatttagctactatcattttgctgctcctcctttcttagttggtaaacttgccataaacgcggtttcatcgcgttgtagcactcgtctcatcttttgatgcatctcaccgactggaatgtcatgaacgaccagatagtcaccccgaagttccggggcatagtcgccaaacagctgtgagcaatcaatctctgatcggacaatgtaattattccgggtcaggttcggctggaacttaaaggtactcttaaattcccgcttcaaatgttccttaccttggaaaatatccaagatatcttgaatcacggcgttggcagttggcagttggccagctccctgacccatgaacttcaaagtcccaatcgtctcaccaatcagtgaaatcaaattatagttgtcacgggtgtgggcttcgagggtgtcgccgtagtacaaggtcggctcaaccatgtagtcaaactcatgaccccgctggtgactcttccccatcaatttgatggtcatccccaacttgtcaaagtgagtcatgtcgtcttcggtaatgttacgaatcccaaagattggcaattcttcggttggcttgataaataggtcgtatgcaatatcgacgctgatacataatttgttggcaacatcaaggccgtcgatatcggcacttggatcagcctcggcgtaacctaattgttgggcctccatcaacacttcgttgaatggtttgccggttcggtgcatctggtcgaggataaaattactggttccattgaagatgccttggatcttattcacatcgtcgactcgtaaagcccgctccaagccttgaatccagggaatcccaccgccgacactggattcaaaataaaatttcgcgtcgttttgggcagccactcgcgtgaattcatccatgtactgggcaatcaccgctttgttggcagtaatgacatgcttatggtgcttcaaggcatcgactatgtattgatgcgccggttcaatgccgccaatgacttcaaccacaacatcgacatcttgatcattcaaaatttcatcaatgctgtcagtcatttccggtaaatccggttttttattctttctgatcaaaatatgctttacatggaggttttgggcttggcgcttcgcattcttaataatcttgtaaacgccggaaccgactgttccgaatcctaatattgcaatattcacagctgaaacctccaattttttagtgttcacaaataataaacacttgtatttaacatgaaaacagattatcatataaatcatagaaatgcaaggagtaagttgatgaataaatattatacgagtaccagaaacggttcagttcaaatttcagccaagcaggccatcaagaagggcttcgctgatgacaagggtctcttcgtttatcccgacttggaaaagctccaagtaaacttcgaaaaattactaaaattaaattatcaagatattgccagagcagtgctgacgattttattgccggacttctctgccgatgaaattgacgaaagtgtccatgcggcttatcagtcgagttttgacacgcaaaaaattacgccggttgttcccgttgataatttccatatcctggaactcttccatggaccaaccagtgcttttaaagatgtcggcttgcagctattgcctcaattaatgaagcacgtattggtcgacaataataaggtaatgatcctgacggctaccagtggcgacactggcaaggctgctttggaaggctttaagggcttggataacatgggcattattgtcttctatccagacggtggtgtcagcaagattcaaaagctgcagatgatcacaaccggtgggaacaacaccaaggtcgcagcaattgaaggaaattttgatgacgctcagacaaacgttaagcgaattttcaatgaccaagctctaaagaaatcccttggtgacgatgtcagcttatcaagtgccaattcgatcaatatcggccgactgattccccaagtcgtttattattttgattcctataaacagttggtgaacgatggctcgattgaagtcggccaaaaggtcaacttcaccgttccaaccggtaactttggtgacgtcctggctgggtactacgccaaaatgctgggccttcccgtgaacaaatttgtcgtcgcatgtaatgaaaataacgtgttggccaacttctttaaccacggggtctacgatcgcaaccggccatttttccagaccgtcgccccaagtatggacatccaaatttccagcaactttgaacgcctcctctactataagagtggtcaggacaccgaatacgttaaacaattgatggatgacttggaagacagcggtaagtatgaagtttccaaggaagttctggcaaatatccagcaggatttctactgcggctatagtaccgatgacgatattgaacggtcgattgccgaagtctacgaacaaaacggctacttgatggatccccataccgcggccggctacaaagtcatgcgcgactatcaaaagctcgatcctgaaacaccgatgatcctgttaagtaccgccagtccctataaatttgttaatgcggttgccaacgctgttctgccagaaacttcagcggatgtccaacaagtgatgcgggacttacatgacgcaaccaacgcaccgattccagataacctgagaaaagtctgggatctgcccgttcgtcacgaaagtgtcatccaaaaagatcaaatgaccgattacgtcaaacaaaaagtcgaggaggtattttatgatcaagatcaaggtacccgcaactagtgccaacgtcggggttggttttgactgcctgggtttggcagtgtcctattattcaaccattacttttgacaagagctcggagcacttggtcatcaccggctccccgaaagaatttcaaaatgaagacaatttggtctaccaagcctttgtgaagggctgcagcttcttagacaagcccgttccaaatgttcaaatcgacattgaaaccaacgtccccgttgcccgtggacttggtagttcatcgatttgtgttgtggctggcctaaaagccgccagcgtctggtacgatgacgcaatttctgttgaccaactgctggtcttggccaccgaaatggaaggccatccggataacgtcaccccggccattctgggtggactgtgcgtctcctttttagatgaccaaaatcagcctcaggttatccaatatcacgtcagcgacaagctgcactttgtggccatgattccggattacgaagtcagcacccatgctgctcgaaaagtcctgccgacatcaatgagctacgcagatgcgattcatcaagtcagccactgtgcggcgatgactaaagcactggaaatcggtgatagccatatgatccatgttgcctgcgatgaccggatgcatgaaccgtaccgggctcaattaatccccgattacagtcaggccaaaaacatcatcgaacaattgggtggtacgatgtacattagcggcagtggttcaactatgatggccatcaccgcagacgaaaaggatgccgatcaaatcgctgccaacgcaaaagcggccttcccaagatggaatgtccgcaaaatggcagtcgattcaaccggcgtagtgagtgaggtaagtgaacgtggaaaagtattacatcgttgatagctcgattctcccagagtcatttgataaagtgattcaagctcgtcaactgttggagagcggcaaagtcaagcaggtcagtgaagccgtgaaagttgtcggcattagccggggaactttctataaatacaaggatttggtcttcttaccggaagaaaacatgatggacagaaaagccgttatctccctcatgctggaaaacaagcgagggatcttatccaaagtcctcacgaccatttctgaaaccagtgccagcgtgttgacgattaaccaaaacatccccatccacaatattgccagtatcgtcatctcactggacctgagtcattttaccggaaccatcgataacctattgggaaaaatccgcttggtggatggtgccagtaacgtccagttagtttcgattgagtaagtatcggaactctgcatatgtcaatcagatcatcgtttctcaatccttgatagctgctatcaaggattttttatgtattcatgatagaaactttcaaactgtaagcccttaccagcttgaaagttgtttcacagtccgcatataatacaatattgtatgcatttactgatttaaaaagtattctggaggaaatcatggcaaacagccaggaaccaaacgcacccaaaaaattccatttatcacaaaatcatcatatgacgattccttggaaatcattcacgacggacgaatctgtccccgccaaagaagccggcttgagggaacgggcttctatcgttggccgggttgggattgtcatgctttcctgtggaaccggagcctggcgggttcgtgacgcaatgaacacggtggccagagtgttggggctgacatgttcggcggatatcggcctgagctcacttcaattcacctgttttatcaacgaccacagttattcgcaggtgctggcactgcctaatactggtgtgaacaccgataaactcaattcactggaacacttcgtcagccattttgaacgggattttggcaatgcgacggtcaaacaaattcacgccaacatcagcaaaatcgaacaacgacctgtccagtacagcccgctggtttctggtttggcggccgcattggcctgcagcggttttatttttttgctgggcggcggcatccctgaaatggtttgttctttcattggcgccggtgtcggacagtatttccgggggtcaatgggtaaacaacacattaccacaattgccagcatttccattgctgtggccattgcgtgcttgacttacatgttttcattcaaaatctttgaagccaatttccaaattctggctcaacatgaggctggctatattggtgccatgctgtttgtgattcccggctttccgtttattaccagcttcctggatatttccaaactggacatgcgatccggactggaacggatggcttacgcgatcatgatcaccgctgtagcagccttagtgggctggctggtagcactattatttgatttccgaccagaaaacttcttaccattgggactatcaccactggtattgatgttattgcgaatcccggccagtttctgtggggtctatggattctcaattatgtttaacagttctcagaaaatggccatgacggccggactaatcggcgcggtggctaacaccctaagactggaaatggttgacctgacgagcgtcccacctgcagcgtcagctttcatagcggccctggttgcaggactgattgcttcactggttaaccggtataacggatacccaagaatttcactgacggtgccgtcaattgtcatcatggtcccgggattgtacatttatcgggctgtgtataacatcggcctcaaccaaattagtgtcggcgcattgtggctgaccaaggcggccctgattatcgtcttcctgccaatgggattgtttgtggcaagagcgttaatggatagggagtggagacactttgattagagtgcggagccgagcggttagtaaccggagcctaagctgactttggccaaaatcgcttttgattttggccaaagttggcttaggtgcaggttgctgctcggcggagcacatttcaatcacagtgcggagagcaacgttttgacacggagagctaaggtcgctttgattgaaatcctgggcttggatttgaatcaaagtggcttagatcgcagtgtcagttgctcgcagcacatttcaatcccagtgcggagcaagccggttagcttttgagcatttatgtaataataggtgttgatgcgcactttgcatcaatgcctctgattggataaagcggagaaagctggcttgtgcagcacacctcaacaaaaagaaccggaccccaccaaagtggcgtccggttcttttgactcaaaatgtctacttaacaataatcacgcgcccatcatgcttttcctcaagcaactgatggcctttaacaaatccatctcgattaaacggtagcttgtagccgatattaatatcgagcttgccttcacgcatcaaatcgatcactgcctgcagagcctcgcgatcgctcatcgcatcagtcggatgaatgtgggcaaatttcaatggcttatctgtcattggtgagttatgggcaacactggcaatgacgccgtttggtttcaccatcgcaacgtcatcatcagttccggcaccattcattgcggtattcaaaacgacatcgccagtgtccgccagctcagtggccggatcggtctgatcataagcaacaaacttcgttgccccaatcgattcgacgtaatcttgattgtgactggaggcaatgccaattacattagcgccaatatcagtcgcaatctgaacggcaagtgatccgacaccaccagaggcccctttgacgatcactgtctgatcaggttgaacgttggcaaaatatttcacagccttataggcggtcagaccaggggtaatcagacctgctgcccgagtcggcgtaatcccatctggaaccacaacggtggcgtctaaattaccaagcacaaactcagcgtagccccgctcagtgtgggtcatcaccagttccccctcactgagatcggaaacccgctcaccgactttcacgatttcgccaaccacatctcgtccaggaatatacggtgacggcatgctgccaaaaccgccggcacgttctgcacgctcacgattgtttaagccaacggcaattgttcgaatgagcacttggttggcagccggcgttggctctggaacttcatattcttgaaaaacttctggatccccatgtttctcatatccatatgccttcataatatcttcctcctcatttgtctaactagcgcaattgtaagcgcaatcacgagttcgagcaagtaagtcgaatcgacctcataatgtaaaaattgagtcgaaaaattgtaaacaactaggtaaatacccacttttgtaggacattttatgtcatgcttaatgcataaatttataggattggaagttggaatgatgttagatatcatcaaagcaattattttaggaatcgttgagggaatcactgaatttctgccaattagttccacggggcatttaatattagtcaacgaatttatcaaaatgagtcaaaccactcagttcactgacatgttcaacgttgttattcagctgggggcaatcatggcagtcgttgtattgtatttccacaaactcaacccactttcaccaaagaaaacccacgtcgaacaacatcagacatgggtactttggtttaaagtcatcgtagcagtgctgccctctgttgtcatcgggttattattcaacgactggatggacgcacacttgatgaattggcaagttgtctcggcaatgcttctcatatatggggtactatttatcctcatcgaaaaccgaaatgcaaaccgacaaccgctattttccgatctcaatacgctctcctatcgaactgcctttattatcgggatgttccagctgctttccctggttcccggaacctctcgctcgggtgccaccatcttgggcggcattctaattggcacttcgcgatatgttgccaccgagttctcgtttttcttggcaatcccaaccatgtttggtgcatccctgctgaaagtctacaaatatttcagccatggcggtgcttttaccggtatgcagacagccgtcctgttgactggcatgctggtttcgttcgttgtggcctacttcgccattcgcttcttactgaactacattcaacataacaacttcaaaatctttggctggtaccgcattattttaagtctgattgtgattggttacttcggctttcttgcgcattaactctccaacggctgaccatccgccagattaaccttcaatagccaagtcaacatttccggtagcattcgctgccaatacagccaatcatggccgcctgcgccagtgtgataagcgactggtagctttaaatcgttgcgcatgtactgaacgaatcggtcattggttggttttagttcatcttggtcgccaatacagtagaagaagcgaagttgcctcagctgttcagatggcgattgtttagctaacgtttccaaatagtgctctggcgcgattccatcaagaatcccctgggcatccggcatcatcgctggcaattcgctcaaatcaactaccggtgacatcggcatcacggcactgaaccactcaggatgggtgaaagccaattttagtgctccaaatccgcccattgacgtgccaccaacgaagttatcctgtcggtcactggacaacgggagtagtttccgcatttccggcatcacttgcttggttaaataatcccagtacggcaggccattgtgcaaattcatgtagaagctacgattcatttctggtgtgatgaccgctaaattcgtatatttggtcaagacttccaaattagttttgcgaataaacccactgccattatcgcctaggccgtgcagcagccaaagcacttgaagttttcggtcactttgaatctcatttggcagaatcacatgaatcgttgtctgttcctctaatcgggtccaagctcgggtcaaagttaatattgccatctgcgtctcctttgttggttattcaaacttcttgagttgatcgtcggcaatttttctcagtaactgtttatcagcatttttactcaactgatccgctaatttacgcagcctcatatagttcacatgggcatcggtgattgtgccagtgtcatcttgaatatctttggccaacttggcacttttattggccttgttgggcgcaaaatcggcaaagtaggtcgacgcataccgtaaagtttttgagcgtttccgaacatgatgaacttccgggtagtccttaaaatcgagtttctcgaatagggcaactagtttgtgatttctacgattgagctccttgacaatatattggtgccatgcagtggtttgggtgaacttaagctgggttaactgctgttggacactttccaaatccttttttaaggttgactgtgtcccctcggttaaagtttgcgccatttcatgttgccgattgtcgcgtaaaatcttcagcaagccttggtagtcggccttcttatccggatgcgagtatgcgtaggcgcccgtctcttcaatcaagacgtccagttcccgcaaatcgccaaacaaattggctgcctgactgagattcgtatcgataatggtataagttgcgggtgtcagccgtcgcttcaagaatttaattaatccccgtaaggtacgaatcatgacccgcaaatcatgcgcccgctcgggatcgaacggattattcaaataacgaacccattcaacctcaatgtcagcatatctgtgttgtaaaatcgtttgaattgacattggcttctcccccttttaaccgccagtcggcagactttccactactgagtaaattttaactttaatgtagcatattttaataatgatgagttaatgattggctgagaaaatgggacgtaaaaaagccgagagtgggactaaaggcgttttgatcccagaatttaagagcacagatcgattattcctggttttggaatgattgatctgtgctcttaaatggccgggatcagccgattgtcgcacgtttttggtaaataatatgggatcacaagaaatagaggccgaggcaaaagcgtatacttttgtctcagccccggctttctgtataatagctggtccattcggtcgataccgatatctccatgaatgatgaatcctattcaaaaaatgaattgaaaattctatctgccaaactgccaccagtgctttttcttgccggcttcttgaaatcgcgcattactcggctggtagctgtcaggaatcttatcaccttgaggctcttcttcatttactgattcgggaatggtttgcttaattgaagaagtgtttttgctttcaagctgcttaagcttattttgaacatccagctgcagccgctgtgattggtccaataattgatgcaattctgcgatttgtttgtctttggcatcaatttgtttgcgttggtcctcaagctgttcagccagcaatgcggtttgctgatcgtcgctcttaactgctaactggttagcggttttcgttgactgcttgtcagcagtttcaacctggttcttgaattggcctttgagaacttcaacaccctcatctttgatcagaatcttgtttcccttttttatcgtatatgtatctctgaacttatcgtccatatgttttctaattgcagttttcgataccgataattcgtccgccaactctttgatagtcagttccataatgtcgcccccaacataaataatatagtttgcaaacagggtgtttgcagtcacacatcatcattatagtgattaacaagccgttcggcaaatgaattctgggtattccagctaatttattataacaaacatccttttaaaatgagattttaattagattttatgttgacaatctaataaaaaatgcggtaaactactcgcatgctgaatgcgaattcgccgatttatctacatatttgttgatcgaggaaggaaaccgcgatcgttttcgtatttacaaagtgtggtttccacaggacttggtttgtcattacgcaaagttttcgtttagcgcggatatttcatagagagattaggagtgattgtatgagtagtataagcgaaaaaatgtttcgaaaagaagatccgcttgtgtatcaagataaggattctcatttaattcgaagcttaaccactaaagatttcctggcacttggcgtcgggacgattgtttcaacttccatctttaccttgcccggcgttgttgccgctcaacatgctggtccagccgttgccctttcgttcttggcagctgcgatcgttgccgggattgtcgcctttgcttacgcggaaatggccgctgcaatgccatttgccggatctgcttattcatggattaacgttgttttcggagagttctggggctggattgccggctgggcactgctagccgagtatttcatcgccgtggccttcgtggcttccgggctttccgccaatttccaggggttgatttcgccattaggattcaacctaccaaaagcactctcaactgcttcaaccggaaacaacggcggcttgatggatttagtcgccatcatcgtcattgtcttagttaccacattactctcgcgtggtgcttctcagaccgcccgagtagaaaatacgttggttattttaaaagtgattgccattttagtctttattttcgttggtgcgactgcaattaagtcggctaattacacaccatttattcctaagtaccatgtcaacgctgatggttctgcattcggtggctggcaaggaatctatgccggtgtttccgagatcttcctggcttacatcgggtttgactccatcgctgccaactcagctgaagcaaagaatccgcaaaagactatgccacgaggcattcttggttccctggttatcgccgttgtgttgttcatctccgttgctttggtccttgtcggcatgtttaaatactcagattacgcgaataacgccgaaccagttggctgggcacttcgccaaagtggtcacgcactggttgccacagtcgttcaagcgattgcggttgtcggtatgtttaccgccctcattggaatgatgcttgccggatcacgtttgatctattcatttggtcgtgacggcttgctgcctaagtggcttggcaaactggataacaatttgcctaaccgggcattgatcgttttgacgatcatcgccatcgcattgggagcgttcttcccattcactttcttggctcaactgatttcagctggaactctgattgccttcatgttcgtttcattaggtgtctattctctgcgaccacgtgaaggaaaagatattccaatgccaagtttcaagatgccgctatacccagtattaccggcactaggattcttaggcgctctgggtattttctggggcttggatattcaggcaaaaacgtacgcattgtgctggttcattttgggaatggtcatttacttcgcatatggaatgaatcactctactgcaacaattgataaaaaagctgaacacgaaaaagatttgtaaaggttggtgatttcatgggtaaattagacaaagcgtctaaattaattgatgaagaaaacaagtattatgcacgttcggcgcgcatcaattactacaatctggtaattgaccacgcacacggggcaaccttagtggatgtcgacggcaataaatacattgatttgctggcaagcgcatctgcaattaacgttggccacacccatgaaaaagtcgtcaaggcgattgccgatcaagctcaaaaattaattcattacactcccgcttattttcaccatgttcctggaatggaactttccgaaaagttagcgaaaattgcgccgggacattcaccgaaaatggttagtttcggtaactccggctcagacgcaaacgatgcaattatcaagtttgcgagagcctatactggccgtcaatacattgtttcctatatgggttcctatcatggatcaacttatggttcgcaaaccttatcgggaagtagtctcaatatgactcgtaaaattgggccaatgcttccaagcgtggtgcacgttccgtatcctgattcatatcggacgtacccaggagaaactgaacacgacgtgtcactccgttatttcaacgaattcaagaagcccttcgaatcattcttacccgctgatgaaactgcgtgtgtcttgattgaaccaattcaaggcgatggcggcatcatcaaagcgcctgaagaatatatgcagttggtttataaattctgtcatgaacacgggatcctgtttgcgattgatgaagtcaatcaaggactcggccggaccggtaagatgtgggcaatccaacaattcaaagacatcgaacctgatttaatgtctgtcggtaagtcgctggcatctggaatgcctcttagtgcagtgattggtaagaaagaggtcatgcagagtttggatgcacctgcgcacctgtttaccactgccggcaatccggtttgttccgcagcttcgctggctaccttggatgtgatcgaagatgaaggcttggttgaaaaatcggccaccgatggtgcatacgccaaacaacgtttcttagagatgcagcaacgccatcccatgattggtgatgtccgaatgtggggcctcaatggtggaatcgaattggtcaaggatcctaagaccaaggaacccgacagtgacgctgccaccaaagtgatctactatgcctttgcacacggagtcgttatcatcactttggcaggcaatatcctgcgtttccagccgccgttggtcattccaagagagcaactcgaccaagcgcttcaagtgcttgacgatgcgtttaccgcggttgaaaatggtgaggttactattcctaaggatacaggtaagattggctggtaaaatagcattattcaataaagcaaacggcacgaatcccaatttgagattcgtgccgtttttatatctattcttattgaccatgcctcataaaggctttatatgctttcaccccaaagtatactagggcgactgcgatcgcaatgacgatgataaaagtaatcacgacaaagataaaatcgccaacgtgaaaaatccccatattgattcccccaatcattaggattcaaaagtaccgttcgcactcaaattcattatgacgtcaaatctgcagcattccatgtctgcttggtcattttagttcaaagtccatgacttccggattatgatcagaatttttgaaccctaacgatttgacatgaacccgattaacctgcacgttgtctgaaacgatgaagccatcaattatcgacgtaaaggtctttccaggacgatacggtgtcccatttgcccgcactgaaggcacttttgcctgggctaatccctgcttggcaattctaaatccctttggcaattgatcagccgggaacgggtgcgtccaattcattggtttactggtcgttttaaagacggccgggctattgcccaacatatcatggttataatccccagcaacgatgacgtaattgcctgcctgctgctcagtggtcattttggcgaataacttattgatctgagcttttctcaccttggcattcttggtaaaggctgagagatgcaggttgatgactgccaactgatgcccattggccactgggatatgggtcaccgaaattgcccggtccaagtccatgaatttattaaaatcggtatcaatcggcagctggtatcgggtactatctgcaatcttagcttgagcaagggtcaacaatcccgatttggctttcccgattggccgggtgagcggataaaacaggtaggctgaattatagttttgggcatagacgctcgaatagccattcatccgatccctgagccactggacttcattcacgtgaaatgaacggtcaccgtcggtatcgacttcttggaagaacatcaaggccggatcttcttgtttgacggcttgatagatgccattgaggtcatccaagacagagaatttgctaaatgcccgcgaatatttgccgccatccataaagaaagaataattatccggataggcagcatagccaatattaaaggtcatcgccttgtacgggtgatttgtctgtaaaatttgcgagttccggttaaccggtttgagtttaacgttgtcgggcacccggtgatacgtcagataaacgtaagccacatatgcaccgacaacgagtaatagaccggaaccaatcagtaaaagtgctttccagaattttttcataagaccctccatacctaatatcatatcaaatctacagccgaacaatccaaaaatatttccaaatattggtatcgtttacaaggctttaatgataaaatttaggtatatttgttcatacttttaggaggggtcaatcatgaagaaatcacatttttggtttgcacttttatttgccggggcacttagtattggggtggggacatcttcgcaaactgtttccgccaagacagttaacatttatttgacccgtcatggtcagaccatgttcaacgtcaacggacggggacaaggctgggctgacagtccgctaacggataccggggtttccgttgcccatcaactgggttacggcctttatggcttgaagttcaaagctgcctattccgctgataacatgcggacattccggaccgcaacctatgccttgcagtcatctggtaacggcaacctgaaagttaactggactgccaatttacgtgaaggcggctatggtagtttcgagggacaaaaatacgatgacgtcaacaaaatcaccatgccgctgttgaaaccagccggtacttattcaggcccacaagactttggcaaagctcaacaagcgcttggtaaagacttctggccggcacttcaagatgcgtaccacgctgccgaaacggtcgactttggtaaatacagcgacccaactcttcctgaatcattgaaagcagaaagctcaactcaagtaatcgatcgaatgaacaccgagttgacttatatcgcccaaaaggctgaaaaaaccggcggtaacgtcttagtggttagttcaggaatgtcgattccagagtggttgtccactcaaaagaactatacggttcctggtttcgttaattggggaaatgaagcaaccatgaaggtgacttataagaatggtcaattctatttcccatcaaatgtcaccgacaagaccatcctttacaccatcaacaagggagcagctttgcagcaactgccaaagaacaccctcaaggtcaaaaagttctatttgaataagaacaaggtttccggttccacttccaccggggcgtcactggtcttgcaaaacaccaagggatcaaccttgaagaaagccaacgcaaactcaaacggaaactttgtgtttaagttaagtaaagccactttgaacaaactcaaaaagggcatgaatcttaaattgacctcaacccctaagaatgcttccaagtctctgaatatgaactctgatcaaattagtcaaactgtctttggcaacaagacagccaccattaaagtattgaagtaaaaccacttaaaacaagttcatgaaatatttaaaataggcgtccagaacaacactcttgttccgggctcctatttttttgcgaatattctgtctttgaatttttaagttacacagcaagcgtgaatgaatcttaaaccacaatcttctttctcaaaaaggtcattgataccagcaacagtacagcacacacggcacccattacgatattaatccacgcaattgcggccactggcgtcgcttcggccaaagacacaatcaccatgccaacactcccgaaaatggttccaccggcactgtacagagcagaggcggacccattatcgttttcctcttgtttcaataccaaataagttccgggtggccggaccgcactgctggccagggttgctggaaactgggttagggcaaaggcgatcggtgacatccggccgaaaaccatgactaggatgccggcaacgatcgtgaacccaaaagctgtatagacaatcgtaaaccggtcaatatacttggaaagcggaatatagaccagtggccccagcagcatgccaattgcgttaaacgagaagaacaggctaaacatccggctactgaggtggaacgtattttggaaaatataggaagatgatgaaatataggataatgacacaatcgacatgagtgaaaaagtgattagaagtgcagtaaaaccgggattaatcagcagtgcccccaagcggccaaatgatttcatcacactggtggtcccacgttctgaagcatgagtttccttaaagataattgagccatagattactgagagtcccagcaatgcttgggcgaaaaagatcccccgccaggaaataaacgtcaacagtaacgacccaatcaccggtgcaaccgcaggtgaaatgaccaccatcgactgaacgatggccaacgtcgtttcctgttttcgaccaacaaagacatctttgatgaccgccgtggcaaccgtcgtcgcaactccaccaccaatggcctgaagaatccggaagaaaatgatttcataggcattggtcgcaatcccacaaaggatactggctaacatgtacaatgtcaagccaaccaataaaatcggccgacgaccatatcgatcacttaacggcccccagaataaagtggcgatcgaataaaacacaaaaaatagaattaaagtcaggttcatcacaatttcgggaaccgcaaagaacttggtcatctccggaagcgccggcagatacaggtcggttgaaagtggcacaaaggcactgagcagagccaaaaagatgataaaaccggtatttcccattcttggttgaactttactgtctgccatctttggcacctccatcctttgtccatttcatattaaccgcaaactcatcggtaacctgatcgagttcgtggttttcttcttgaaagccttcgttaatgtaaaagtgataggcacgggaatttttttcatagactgccaacgttaattccgagcgggtttgtttggcagcactgagcagatgagaaccaatcccttgaccacggtactgcttggcgacaaacaatccggcgatgtagttcccttctattcccaagaacccctgaatttgaccgtcctctgtgtcaataaacagttcggctttggcaagttcccgtttgaccccatcataatagttggtccagtaagttggattgacaaacgaatgggcgtccagattggcatccaaccagatttgggcaatttgatttagtttttcgccttttattccttgaatatgctcaatcatcgttggtccactcccaatcaaggttcttttagtctttattgtaaaacaaaaatggcattccaaggtggaataccatttttgatttcatgttatttgacaatcttcacatatttcgtatttccggtaatgtacccaccggcaacgtgatacctcaaagcaccatgattagaaacactgtttgcatgtgagtaatcgtagttcttgatcttaatcttggtgcccttcttgaagtgcgtccgcttattacgtttactcaagttgacatcttgataacggtagattgcttttttaactttgatatagcgaggctgcgtctgcttatccatagttaccagtttccggtttgcggtaatgtattggccgtttgtcagtacaaatcgggttgtcaaattgtgcttaacaattttggtaacctgaagaaccgtgccttgtttgtagtttctggtcttggcagtcaaattcttgtacatataggcattgaccccgcgcggattaataaccgtcacggttgagtgcatcgtctgataataaactggacgaacgtatgcccactgtgcggtgatataacctgtcttgccacgattcttagttaagtggttcacatcgcgaacctggtaacgaaggcgaccatttgcggaatgaccgtatccagtgacaacaaacatcggccggtaaacgcgcggcttggaaacgtaacctgctcgacgttcatgagtactaaaggtcgtgttctggtagagataaattttctttaacccgtacacaacggtccctttgggcgctggtgtcgggcttggagttggcgtcggtgttggtgtcggcttcggcgttggtgtgggcgtcgtatctttcttcacataaacgtctacaggagaagttgtcgttccccagacaacggttggctgaactttaccattcaattcagttcccgatgctacatgatatcccgtaggcactgtcccataggtaaggatcttattgagatcccaagtatcaccagctttagtggaactggttggagtcaaagtgaagtgattattgggaaaacttgtttgaccgtcgacgtcaacaaattcagcgttcaaatttgttaactgattttcatctggggtgacttccaacttagcatacttagtttgagtatccccggcatcattactggcataaattgggatttcataggtttggccagcctgaattttgtcgtaggctagcatagattgatatttataaccattgccaaaatgcaactggttggcagaatgcggctgattatgatcagacgctgtggcaaattgttttaaaacatcctcatcactcttcaatgtctgactgtcattgttaaataacattttacgagcattacttaatgatgttttaatggttttcactgtcagtgttgggataaaccctgcgccaattgtactgttgtacatcatttgagctgttttatgaagaggcgcaccattatttgggatgtttgagatattcgatgtaacaatgaacttatcggtgactgatttagttgtaactgcgaatgggatattcaaatcgcgtccagcatctgcggcactcagattttgaatttgaataaccaccttaccatttgtgctggctgctgcatcatatttccatcgaacttccggctgatttgccattggtttatcattgtcaggactttcataaactttcagtttttccggatctgcaatgggattattctgagaatcggttgacaatgtccaagtaaatgactttggaactttatcggcatttgtcggtagtgcaacttgaacccatgcgacagttgcattttgggaataccagtagagcaatgcttcatcggcaggtgcatctgatcccattggcgtgtacgcatagaagttgccgtcccatttatcttccccgtcgctattaaacccgcttggagcagtcaaaccacctaacccgccgaaaatctcttcgttcatggtagtcgcaccaccaccggatgttcccggaacattgttaacattcagatgaagttgctgaatttcggcagttgacgtaccccttgcataagttacgtggacagggtaagtaacagtgcttttctggttaagatcgtcagttgcaggctttaaataaatcgaaactcccgctttggccaaacttgcatagtcaattccatccttggcagttagtgtaatagtagcttgatccccatttgaatcagttgacacatcaaagaagtttcctgacgaaactgcattgatctgcagcgaatctaggtcaaaacctgccgtgccactatcatccttaccaactgaaatcttaatttgatccccggccttaatgccagcagtcttctgcagcaagaaagtcatattaatggcttgattactactgtatgtactcgtgtcattaagtgtagttgaaaaactaaaagggttctccagcgccgtatcatcagctttagcattataaacaccgatgatcatccccacaaacatcgatatgacaatcatcatccaacacaaaaaatattgtttacttttcctacccttataataattattttttggtaaaccttgataactatgcattaaaatacccccgtttccatatcttcattgtaatattcctgagttctgttttcaattgccaaaagatacctctaaggttaagcagacatctggaatatccgctaaactacaggattttgcggacttttgtcccgttttcatgtacaattaacttaaaaataaggaggatttcccatgtcaacctacaaaaacaaagtctacctcgcatccccatttttcagtgatggtcaaaaagaccgcatcgcccaagtggttgccttactcaagcagaacccaaccatcgatgctgacggcatcttcattccccaagaccaccaattcgaatcagaaccctttggcagcttcaaatggcaggacgccgtcttcgcatcagatatgcgccaagtacataaagcggatgtcgtcgttgctattttggattatcaactggaagaaggcttaacggaacccgattcaggcaccatctttgaaatcggctcagcccacgaagctaacattccggtcatcatggtccaatttggtgaaaatggtcaattaaacctaatgttggcccgcagctacaccgccttctttaacggcaaagacgatattcaaactctcaaggattacgatttcaacaacctggagcaaaaatataccgagaaaaaagttctttaatgatatgtagaaagacaactcaaaaaggaagtgaaacatcaggaacatcctgatggctcacttccttattttagttaatattctttaaaatgaaaatgaatcaaatcagccaactaatgatcactcggcacaccattttctaccggcaacgacaaatcagctttgtcatccgcaggcaacagatgaattgcgtgtttcaacaggaacggtgcgatcagcgttgacaaaataatgaccagaatcaaatctgaataatacgaatccgacagtagtccagaggagaaaccaatttgagcggtaatcaaccccatctcgcctcgagaaatcatccccgaaccaatcatgtaactactgttgaggttaaagccgttgataattgcgcccagcccgcagccaaatagtttactgatacaggccagaaaggtcaagacaccgacaaataacagtgagttgccgatatttgcaaacgacatgtttaacccgatactgacaaagaacattggcacgaataccgcgtagccgatcggttccatgtgattctcaatcgtctcccgataaggggtatgagcaacggcaatgccggcaaagaaagcaccaaccgcaccgctcaggccaacggcttcagcaatgtaggccattcccaaacaaatgaccatcgaggtaattgtgacgctggaggccattagcaggcgctcgccgatctgcatcagatagggaacaatccacttgaccatcaaataagttagggcaaaaaaggcgatttgctcgataaaaatcagggcgaggttggttgatgaatcaccagttttgacaccggcagttcccatcacactgatcataattgacaggagaatgacgccaataatgtcatcagcaaccgcggcaccaagaatcgtcgctccctctttggtatccaaggacttataatcccgcaatacttcaacggagattgagacgctcgtcgcactgaagacgacgccgataaagatggcttcaagcggcgcgaacgagaatgcccaacaggccccaccaatcatgatcactgggaagataaccccaataatcgcaacgataattgccggccgtaaatacttccgcagcaatttcagattactttccagcccgccaataaacatcaagataatgacaccaatctgtgaaaatagattaatcaaattatccaaatgaatccagcccatcatagccggaccgacaacaatcccaaccaggatctggccgataaccgacggaatcccaattcgattggccaagtgcccagccagtgtcgtcaatatcagtaacagacacagggcaccgataaacgccatgtcatggcctcctttctcatgatacttatgtgtttataatctattatatgtgttttaggttctatgtgaatatgtgtcgacaaatcagtcgttttcgatctgagtcgttttagcacccatcatggcaccaatatagtgaatggctaagccaatgattaatccaatggcggctggcagcaaccagtccatcccaagcgaagcgccaggaagaaagtcatctaatttcaaaattgtgctggcaaatgcagacttggaaataattgccggagctgcggcgatcgcatccaaaatcgctgggataatggtaaagatcgtcgtccagatgtatacccgacggtcatgattgaacaatggtgaggcaattgagagaataatcagggtaatggcaagtgggtagaggaacatcagcattggtgttgaccaggcaatgattgtatcaaggccaaagttggcaattccaaatgacagtccggtggcgatgattaaccaagctcgataagaaattgatgggaatttagcatgcaaagcttctgagaatgaagtcgagagtccaacggcagttgtcaaacatgtcaaggtggccatcattgccaagagaatttcaccggtgatacccatgaaatgattggcaatctggttaaaggcaatcccaccatcaatggataacttgaaactaccaaggctggtagcgcccaaccagatcaacgcaatatagataatggcttcaagcccgatgcccaaggcaccagatttcatagtggtcattgaaatttctttggcactagtggcgcctaagctcttaatggcggtaacgatagcgattccgaagagtaacccggcgatacaatccatcgtgttataaccttgcaggaaaccgttgagaatcgaaccattttgataagcggcatccgcaattggggcctttgaagctgagctgattgggctcatgaatgcaaatgcgaaaatgatcgcaagtaatgctaagaatgccgggttcaaaatttttccaattgagttaataattccagtgggtttgcgtgatgcccagaaggtgatcccaaagaaaatcagtgagtaaatcaacagccacattggttgttgcgttggattcaaatggctggcaaaggcaatttgaaatggggttgtcgccgtccggggtgtcgcaaataagggtccaagggtcgcacaaaccaataccatgaagaaagtcgcatagcggctgccgattggtttggcgagatcataaattccgttactgtgagtaactgcaatcgcaataatagcaagtaaaggcaataatgttccagttaacagaaacccgattccagcagacatccagtgagcaccggctaattgtcccaagtgaattgggaaaatcaagttaccggcaccgaagaacatcccaaacaacattgaaccaataattagataatgtttaaatgataatttctttgtattattttccatattaagcgctcctcataatttatatacgctaaaattcccgttattttatactgattgttggtgactcggctgatgccgcctgacttgcttcgatttaacatgtttctcattttgaagacctccttaagtgcaaataaaaaacgtctcttaagatcgatacgatcttaagggacgtttgcacgtgttaccacccaaattctcgacagcttcacaactatcgactcaccatgtacggccgaaggaattcagcgatacactggcgctgtaatgggcgctcccaacaaacactcgcggactcgctcgcatttgtcgctcgaaggctactttcatcgcttaggcttttgaatcgttctcacttacccgattctccctgaaaaagttctaagagactactctccttgtcttagcaaattctaatgtttctgattgacacaaatactaatacgatttctgatcgatgtcaaccagttttatttaactaattttacgttgtgggtagtataggctaaatgccaaccttttggcaatgattgatgggcaaatttaccggataatttgttggatttaagaataaccactccagatttaaggcccttaacatctttcactaccagtttaccgcctagtttagcagtaccggatacggaaaccttgtcgccagagttgacattcaagctgcctttaccactttgcgtgtaattacctttgaccacaacattcttggcagagagggttaagttaccacccgctaaggtcaagctgccgtcacccaaggcgttatcattttcagctgccagagttccagctttgacagtagttccgcctttgtatgagttatttccaagcaagctcagggatcctgaaccttccttggtcaggctgcccttaccggaaatgttattcttccaggtgtcggctgcgttaaagccgcctttggaagcatccatgttcacggtgacgttgtccaagaaggatccaaaaccattagcagcttcaaagaggttcaaacggccccaaccttcagtatcatcagtcattgggtaacctgatggaataccagtggtatagaggacttcacgtctttgagtagcatttagatatggtaatctggtttgtaagagcacttcagcgccctttgggacaaccattggcttagtggtatcaccaattggtgagaagccataggtcaatcgataggtgtaattcttcaggttggtttggtaatcgctaaagtcgtccttggctgatttatcctgagccttggccaaatctttttgcgtgtcctggtaggcttggttgatcagctgcttgttgtcaggatcgtttaaggttgcagctgtcattgctgttccgattactcgaccacccataacagctaatggtgagtgtcgtccggcaagtactcggtcatagccgacttccgaagaacgggtaatcaattgttgataacgctctgggaacaggtaggccaaggtttcaccggtttcaaatgcggcggttgtatggccgcttgggaaatcataatcgttagcggcagccgaagccatcacattcttcaagtatgggttaactttgacttgatcgctttgacgataaggacgggtaaatttgatgtaagcctttggtgtccctgtaccagaccatgctgaatcttctgcaatatcaaccagcttaaccgcggaaccgagagttgagttttcatctgcccactgcatcgagctgtagggtgaacctgcgggaagcggggcatcgggaacggcattaaaatcagtctgaacgttggtatccttgataaatgccggagcgtagggaccaaaaccactaatcaggttatatcgcaggtcccgccggtcagttaagtatgaacggtcaatttctgcttgcgaagcaccgttggtaatttgaattgatttgtccaaattgtcttggagcactttttgattcgtttttgtaccgtcagttggattccaatagcttaaaaaggtattgttgaacaacgcgatcgccggattggtgtccggagtcgagttggtcttcacattttccttatagtgatcgacgaaatacccatatgaagctggaaccggattcaactcgtttgagacactggtatccgacttggcgtttaccttcacatcattaccttgagcacccaaaactgcagctccggtcaacgtcagcacaaaggcgcttttcagaaccgttttcaaaatcgtactgctatgtctacttcccatgcttaatcctcccaagatgaaataatttctatgaaacgattatcagaacaacaagtatcagcaaaaccacaaacgatatttcccaacccaacttgggggtatgtttgatttcgtataacattgttgacatgatcacaccatcctttagatagtccctgatagccatttctgattcaactttagtgtactgggatgacgtaaattacccgcaaaatatttgtaaaaagtgggtaaatattgatgtttcacatgaaacattccgttagattggcggcctgcgtgcatctgctctataatgtcggcaaggggtgatgactttgaacaaacatctaacacttttaatcgcaaccggatctctactgacggccgccattgtttcaatgcaaataccgaccacattggatgccaaagtaaagatcacaaccaatcagtcttacaagaaaacatcatttttgatcaattccaaccgaaacgcccatgtttggaatgctaaatacaatcgaaagttacataatttaaaaaattacccgcggacaaatttctattcaaccaagcgggtcacgattcggaccaatcattattttggcagttattactacattcatagtgccaacaataagatcaagggctatgtttggcacggctttctcatcaaaggaacctactacaagggtggcttttatcgctaccccaccttcaacgtactgctttccaaccagccgtatcgtcgtggcggcatgagtcggattggcgaatgggatgcttctggtgtgtatgcatcttcgaatcgtattcatgggactgttaatcaaaatgagctaaaaccgtttgcgataacccccgccctcaatgatcagaaacaggctttgacatatctaaagcaaaattggtcttacctacctgaaatgttgaactatggtcagcataatggcgcgcgaattgtgatgcggaaagtttactatgcaaccaatcaatggctaaaggttcctatgattgacattcttaacgggccagccatcagtggtaattgggaagaaatcaatccatttgcggcggttttggatttgtcaaagttgcccaacggcgccaagccaatcgccaattacgatgttggtcaagtaaccgtcttaccgctggggagtcgggcctttgattttcccgatccaactgctcaagtcactaattataacagcggcccgatcacgcgtatttacggcaacaacttgggccctaatcataatctctccctggttgatttgaaccgttggctgcattacgttccaaccaatgacatttttaagctttccaacactcagccaaccttgaaagacggcatctggtactttgctcccagctttgaaagtggggtcggttcaggtacccaccttcagcaaatgctcaaccaaatcaatccaactcagtcaccttactatcggacaatgaccggtgaaggcttcatccaggcacactatgaaaatggtcactggcaccaacagtttgaactctcaacaaacttaccggccttcaataaggggaacgggatcaccctcacaatttccaaaatgatcaccaaatcatcaggatccagttcatacaccactgctgacaacgctaacgccaaaaccgtcaagcattttgacagtaatgatgccgatgtttcggattacttcttcaagccggcaagctactatgaaacatttttgaataatgactaacaataagagtccgctagaaatgacgaatggtttaatatcaaacgaagcgttaggtcatttgatgaggtttccaaaatcagaaggaaagtttcacaaagtcgttgaaatcgttttctcttatttgcacgtgtttctaaacaaaaatatcaaagtttgtgaacaaaatggttgcactcagcttggataggcgttatatttttaagcatacttataaaaagtaagcattacactttagatttaggagtgattaatttatggcaaaaatgacagctggtcaagccttggccaaagtactggtaagctgggatattgaccatttgtacgggatcaccgctgactcaatcaataataccgttgatggtctctatcaggaacgtgacaaaattaaatacattcaggttcgccatgaggaagttggctccttagccgcaaccgccgacgccaaattgactggtaaagtcggtgtcagctttggctctgctggtcctggggcaacgcatctcttcaacggattatatgatgccaagatggatcacgcacccgtggttgcaatcgtaggtcaatccgcaacgccaattatgaatacctatttcttccaggaaatggatcaagatccgttgtttgttgacttaactgattttcataaacaagtcaccaatccggaacaaattccctacgtgatggatgaggctatccgctacgcctatcagaccaagggaccagcagttgtaatcattccggataatctatcgggtgaagaaattgattttgaaccttataaaactgccaaagtcttaaaaccggccaccaccatgaatgttgaccaaaaagctgtcgaccaagtttacgatttactcaagcaagcaaagcatcccgtcttatgggcaggtctcggcttgaaagatgctcgagatgaagtcgtcgccttctcagaacgattcagtgtgccagtgctcaccaccgctccggcaaccggggttatgccgaccgatcatcccaactttatgggatcgcggggacgtctgggaaccaagccgggctttgaggtaactcaggcagccgacttaattatcctggcaggaaccaattacccattcagccgtttcctacccaagggaatcaaatttgttcaaatcaacaacaatgttgaagatttagggaaacagcatgatattgacctgactgtcttagccgatgccaagccgttcctggccaaattaaatgaaaaagaaccaatagccccaaccccattcctcaaggctgctcaaaaggataagcagaactgggacgcatggttgaataaagtcgctgacgacgaccatgatggcttagcgccggaagcagttatccgcgccattaaggaaaatagtgatgacaacgcagtgtttggcctcgacgttggtaacaacttaatgtggtctatccgccaactaccatttaaccacgaccaaaagcttagtatgtcagcttggtttggaacgatgggctacgccttaccagcaagtatcgccggtaaattgagttacccagatcgccaggttttcagcatttctggtgacggtggcttctcaatggtgacgcaggatctgctgactcaagtgcagtatcagctgccaatcattaatgtcgttcttgaaaacggcgcattcggttacattcagcatgaaaaaatcactgcaagccaggaaccatatggtatccacttcattggtgccaattgggccggctttgctgacgacatgggtgcgattggcattcaagtcaccgatcggcaatcgctgaagggcgcattcgaaaaaattaaggaactccaagtaaatggcaacaccaaaccaatcttaatcgatgccaaggtcaagaaccaggatccggttgataccagcttcatgccaatcgatcccgaccaattcgatcaagcagccattgacagttacaccaagcaatcgaatttatttgatcaaccagctctttcaaccttgctgaaagaagaaagcaacagttaaagatacttgaatgcaacaaagacctattaaccataaaaagccaccaatggacgatcaatccactggtggctttaattagcgatgaatcattttcagtaattaattagcccctgctcacctttgatcccagccgagatgaaccacgaacgattatacaatcgataccccgttaaattagcaagccagggctttgagaagtgaagtaaaatcggatgttgtaatgaggctcgtttggaatttttgtataaaagtttgaattaagggggcattattctacttattatgtgatgccaactactcgctcactcattagtcagccacaactgtctcgccagcatccgtgtcatcctcacgcagcaggtcgctcacttcttgacggcgaccataaacgtaagtcaatgaaaaactaaccacaaaagcaatgaccatgctaatcaagaatgccgggatggcgttggtcgcaatactaatgaatcccaaaacactattagagcctagtgagactgccaaaacatgggtaagtcccaaataaactgaggcgacagccgaaccgatcattgaggcgatgaatgggaactttaacttaagattaatcccaaacattgccggttccgtgattcccagcaaagcggacatactagctgatgacgccagtccccgctgttgcttatccttagttaaaaagaaaaccgctagtgccgaagcaccctgagcaatatttgatactgacgcaatcgggaaaatgaaactgccaccggtttgtttcacgttagcaattagctgggtctcgattgctggaaaactctgatgcaggcctgtaatgaccaaaggtgcatagaacaagcctaagacgcctgttccaaaggcccccgaagtctggtacagccacaataaaccgttggttaagccatcactgacatcccgcataactgggccaacaatcataaaggtcaaaattccagtcaataaaatcgtaatgagtggtgcaaatgtataatcaagtgcttctggaagtcgtttatggcactgtttctcaatgactgacagcagccaggccaccgccaacattggaatgacggatccctgatagcctgcttgggcgactggcatccccaaaatgtgccaataaccaagtgaatgattggcaaccgcattgctcacatcgtagccacttacaagggagggcgacaccatcatcatccccatggcagctcctaagtatggattcccaccaaagcgcttggtggctgagaatccaattaagaccggtaaaaatgcgaacggtgcgttagccaagacattaataaacgccgcaaatcctttaaactgagggtatgcagcaactaaagaagcagtcataaataggtggggcgccactaaaacattgtgaagtgccattagcaaaccagccgccacgattgcgggaatgattggaacaaagatatcagccaataagttaatgaatccaagaaatcctttttgggtctttttaatcgttgtgataaacaaatgcatatcctcctcaaaatagtcacttcgaaccattctacgggttttcgtcacagatgcaagaagattgacagaatttcttgcctgaaagcacctctacaaacgttttcattaccatttccatggacagacaacatctatcaaaaaatctgtcttaacttgggattataaacacacactgtggttgcttgtgctatgatttgagaggaagtttcacatgaaacaatttgaccattggagggtctgcaagtgactaagtataaagttcaatcattagtattcatcctcgttgcctttatgttggggtgcaacgaattcattgttgtcgggattctgccggatttatcggcccaatttcacacgccaatctcaaccatgggttacttggtcaccatcttcgcgatggtttacgccgtcagtacaccatttgtcacaatcctaacaagtcggtacagtcgctataaaaccctgttaaccctgatgattgtctttttgattggtaacacactcagtgccctttcaattggctacctaaccatgatggcctccagaatcatcaccgcaacgacggctgggtcaatcatttcactgatcatgacttttgccagcacgattgcgccacgtgataagcgagcttcactggtttcttggatctttgccggcttcagcattgcgtcagtctttggggtgccgatcggcgttgccgtcagcacaagcttcggttggcgttataccttctggggaatttcggttatcagcattctaactttccttctattaacgcaaatcctgccaaagaaagttaagcagacaaccagcaccatcaaaaatcagctgacaattttattggatccccgaatctattacggtgtcttcctggtcttattcacggccgcaaccatgtacggctactacacatatattcgcccgctgctcaccacgtcgatgggcttcagtacccagagtttgaactggctgttgttcatcatcgggattatgagtattatcagtaaccgactttcgggaatgctggcagaaaagcccaacagcctgcaaaaagtgccgctcttttacgttgccgatatcctcttactggcagtttttccatttgcattacacagtaaaattgccggtctggccatcatattgatcctgacattgattgtgacaatcatcaattcaccggttcaaattcatttcctaaatctggcagaatcagaatacccacagtcgctggtctttgcctcatccctaagttcaattttcttcaactttggtatttctctgggatccgcgacggcttcgagtttagtgggcatcgttggcctggatagaatcagtattggatcggttgtttttgcagttctttcgcttggttcgctatttttgattaaccgggccattaaggcgcattcgtcaacgaaggcgggaaactagtttggcgccttgcattggcagtatgataaatccatcacacgcctaaacgcggttctgaatgtcccttaaaatctgtctcaaacattgacttcaatccaaagttcgttcgaatcaaaaaccactatttacaggaatggtagcaaatgtacaaattctgaagaataattaccaaactgattcatagaacccttgcataaaaagacaaacgaaaagattttgaatgattaatcccataaatacccaattttggctatttgatttccaaaatttataatttaaccaaaataataaaggtaacactgagactacagcaatatcattcacaactgatgtcacggaatatgttccttcagttattagtcttaaaacattaccaattatgagtaaaattatttcgagaattactagctgtacagtaatcttgcttgtttgattatcaacaattggcttgcatacaaaatatttcttagttaaaatacccacgcaaatataactggtaattagtatccagataaaagtagaaacagtaagccacggcatcaacttcggcttaacaaacggtaacgttcctgaattaaataattgaaaaaaggtaactccattaataacatatgcaaacaatggactaatcataaaattcagccaaaatataattgttaatcccagagatttattcattcgtgcagctcccttcattgatcattaattcctataccacagaacatgtggccaatttatatgaaacgaccctcctttccaggcagaacaattagttgaattacctttagttaatccaggtagacagtagtcaccgaatagaggttctttttacacacttattttgtctccggaaatgacaaaattagctaacttttgtttagaactgaaaagtaaaagtatgataatcagcgttgctgtccaagattttgtctggggatttccctatatcttcctagttttatgtgcaacggtgaactcactcacccaaaagtgaattagcttcagcttaatttcccaaacagaacccaagcttctaagtcccccagcctttagtttttaaactactcttaatcaggtatactgaagtagatgtgaggaggatacttatgaaaaaatggtctttgttgttacttagtctaggattagggattgttatgctgtctaatccaactactcatgccagttctggttacacggttatcaagagctcatttcctgctggggttggtaaaatgtatcatgcagctaatccaaaacagaacgcttatgtttggacgaccactaagcatactaaaaaattagcgaacattaaaaattatccaaacacttcttggcattcgaccggcacggttgtgcttcgtcataatcataagaatgctgtttactaccgagttgacgcaatttccccaaccaaaaccaagaaatcggttagtggttggatttggcggggctatctcaaaccgggctataaccctaactttaccaaagttaaaagcattagccttgataatgctacaaacgaagaatataaccagtttatcaagcaatctaaataccagcagctaacccgtgatattctggcgctgtttcccaatagtaccgtctccaagccattaagtcggtatgcgttgtttcgtgaacctaaggataaaattattaataatgtagccactttcaaggcaatggatgactttttgaatgtcaaaaaccggttaaccaaccagcagcggttagctaaaattaaggcgattttagaggctaatggttatactgctgctaatcggcaaaagaaatacgtcattggcatctacctcactaacttccagtggtccgatcaatatgataccggtgatatgcaccaaggatttgtgattggaaccaaataaggagatacttaatgacaacgccgcttcgtatgaattgttccatcgaccccaaatatgtaatttctttcaatgcgtggaatgactgttaggtgccatttcccctgatatgatatagtcaaagtcccaaaaagtcctgatagcatggacaccaaagccccaacagatacaaattgttggggacttttcttattgatgataggagaaatgaagtatgcacaagaagatactatggttgattcaatttgcgattaattgcagtttcatgatttatttggcaagcttcccgtcaaatgcagtttattctggatcaggttggtccattttaattggtctatttcttgtaatcattgcggttgttgcagcgattattttgacaaatttggttacagaaagatgaatggtctttactggatgtaagctgatcccagagacaacttttaagacagggtataatgaataaatcatctctcaaaagaaaggaatttttccatgccaacccgttacgccaacgatgcgtcgggtaaccgtcacttgaccgacatacaaaaaatgccctattaatgacactaatgaggcgctgatgaaaagaactgccgaaccagacaactctcattcaaattaattgctttcacatgcatatgaattacactgagtttgtataaatacaaacaaaggagcgattttgatgaaagcattcggttacgaaaaaaatggcggtcccgaggtgtttcaggagtatgaagtcccaacccccgaaatcaaatccaatcagatcttaatcaaaacggaagccttcaacttaaataactttgaagcattacagcgagctggtcaattcaagccagtcgaccaccgaatcatccccggaagagacgttgccggctttgttgaaaaagttggcgaagacgtcaccggctttgacattggtgatcgggttgtcgctcacggccatcattcctacgcagaatattcaattggcgaggattccaataccgtcttaattcccagcggtgttccctatctggctgcggcggggattgtgactcccggcctagccgcatataaaggtgttcacctgtttggcaaagttcaagccggccaaaccgttgtcgtgaagggggcttctggcggggttggctcacttgccgcccaaattgccatggatgttggtgccaaagtcatcggcgtcggttccagcgaaaatgaagaatacgtcaaatcattgggcgttgatcaatacgttgcttacgaccaggaagatccagcggaggttctggcagacaccgctgatgtcgtgattgatgctgcattaaacggcaacggtgccgaaagtgacgtcaaaatcgttaaagatggcggaattgtcgccagtgttgccgacaacgatgcaccaaccgataaaacggttcatttcaatcacattcacccaacccaggaaatctcggatgatgatgctttgaatgctatgttaaaactgatggcggcaggcaaactcaaaattcgcatcggttacaagctgccatttaccctcgacggggtcattaagggccatcaactgctggactccaagcacgccggccgaattgtgattgccaagtaagattgtgataaacagaaagactgaagcgcaaaaaggtcagaacatcattcaccagaatgatgccctgaccttttaaattggatctatttcatctcaacttaaatcgcttatttcgaagaatccttgcccttatctttatccttcacaattgcctcagagtatagtttatcgaccaactcgggatttgatttgccaggattcagttcaacaatctggccggcagccgaataaacaatccactccgccaggttaacgatgtgatcaccaattcgttcaagaagcttaatcaccataaagtaactggaactggccgcgattgttgcggtatccgattgcacggcctcggtaatttcatccctaattaacagatactgttcatcaactttgacgtcattatccgataactttttagcggcgtcggcatcgctcttcacataagcatccagtgcactttccaacatatcccggacttcttcggtcatcttggcaatagccttttcaaccttgggaatccgcggattacctttgacacgaatggtttcgcgagccatactaaccgcgtgatcaccaattcgctccaaatcagaactggcttttaaaatactgatgatcacccgaaagtcggtcgcaaccggctgttgtaaggcaatcaagctcaaagcctgtttttccaatttcatttcatccgaattggtttcctcgtcggcatcgatgacttcttgagcggcttttttatcatgctcaataaatgccgtagttgatttataaatttgttcactgatggtcagccccatttccacaaaccggccgtggagcttttttaactcgtcgtcaaataattctctcatcgtctctattcctcctagccaaactttccgttcaaataatcgctggtcttctcatcatcagggtgaataaacattttctcggtcttgctgaattcgaccagatcgccgttcaacagaaaggccgtcttgtctgaaattcgcgaggcctgctgcatgttatgggtgacgatgatgatggtgtattggtcgcggatatttaacaaagtatcctcaattttggcacttgaaattggatccagggcggacgttggctcgtccaacaacaccacttcaggctgaacagccagcactctggcaacacagattcgctgctgttgaccacctgaaaatgacagggcattatcgtaaaggtggtctttgacttcatcccagatcgctgcctgcttcaagctggtttcaacccgctcgtccaaaacgtgcttatccttctcaccagccagccgcagtccataagcgacattttcatagacgctgaatgggaacggattaggctgttggaacaccatgccaactcgctttcgcaggtcaacaatgtctgttccgggggcgtaaatatcttcgtcttcaagcttcatcgacccggtaattgtgacccctttaattaaatcgttcatccgattgagacaacgcagataagtcgacttcccacagccggatgggccgattaaagctgtgatatcgtgttcttcaaagtccaaactaatgccatggagcgcctctttgggtccataacttaaatggacatctttactcgtaatgatttttggcattgttcagcctcctaaccgaagttcccggagatataatcttcggttgcctttatttgtggtgtcgtaaatattttctcagtcacgtcgtattccagaacatggcccatgtggaagaatgcggtgtagtccgcgattcgtgacgcctgttgcatattatgagtcacaataataatggagtaattcttgcgaagttccattaaagtgtcttcaattttggcagtggaaattggatccagcgcactggccggttcgtctaagaggaggatatccggcttcattgcaacacatctggcgatacaaagccgctgagcctgaccgcctgatagggctaaagcacttttatcaaggtcatctttgacctcatcccaaagagcggcggccttcaggctttcctcaacgcgtttattaagctcttgcttgtccttgataccattgcgtttgagagcaaaggtgatattttcacgaatcgatttggcaaacggattgggccgctgaaacaccatactgatatgcttgcgaacttcatatacgttaatcttttttgaattaatatccatatcccgatacataatttttccttgaacggtcgcaatccggtcgttcatccggttcagacagcgtaaataggtcgatttaccggatccggaagccccaatcaaagcggtaatgcgatgtcggggaaattgtaaggtggcgtcgtgcatggcgtggttgtcaccataaaacacctgcagattttcggtggtcatcgctttttctaacggaatatcgataatgtgcgttttattatagtcatattcttgcataataatctcctacttcgttgctgtcatgcgtttgtacaaccaacgtcccaacatgcgggccaataggttgaacagtaaaatcacaacgatcaatacagctgatgccccacttgaaatcgaagctgcatcaggggtaaccccttcagtgttaactttccaaatatgcaccgctaaggtttcagctggtcgcataaaattcaggaaactggcactatccatcggattccagtcaccgtaattaaccgtcggcgcactttgtccagcggtataaatcaaggcagcggcttcaccaaatacccggccggcacttaaaatgattccggtcaaaataccaggcaaagcggctggcaggacaatcccggtgatggttttccaacgtgataaaccaagtgataacccagcctcacgctgtaattcggaaacatcctggagcgattcttcgatacttctggttaacagcggcagattaaagaatgtcagggcgatggcaccagccagaattgaaaagcccatgtggaagttaaccacaaataataggaagccaaacaatccaacaacaactgatggcaatgagctcaagacttcaacagcagttcgaatcacgccggttacccagttgtcaggggcgtattctgaaagataaatcccagaacccagggcaattggaaacgaaatgatcagcgtgaggaccaacaggtacatcgagttgaacagttgatcccgaatgccgccgccagcagcgaacgattgtgctgccgacgttaggaagtgccatgatacatggggaatcccagtaattaaaatgtagccgagcaggaagaccagaatcgccaaaacacaggcaaccagaaaataaatgacgccagtggcaatgttattactcgttttagaattcattttttcaggctccctcgctttccgattactctgactaagatgttaaagactaatgacatcaatagcagaatcaaagctagtgaccataaagcgttatttggcagggtccccatcgtggtgtttccgattccggtcgttaattgactagttaaagttgacgatggtgttaataatccatgaggcatgagaacagcgttaccaataaccatttgaacggccagggcttcaccaaatgcccgtgacatcccgaagataacggcagttaaaattcctggagtggctgatcgcagcaccactttataaatggtttgccatctggtagctcctaacgccaatgacgcagaccgataaaacatcggcacagctttaatactgtcaactgaaagtgacgtaatggttggtagcaccatgacgaacaggaccaaggttccggcaagaatcccaaaaccagtgccgccaaatgagtgacggatcaatggcacgataactgagagcccaatgaaaccatagacaaccgaaggaattcccactaacagttcaataactggttggagaattttggttccccgctccggcgcaatttcggtcatgaataaggccacccccagtgcaaatggggttgcaaccactgcagctagtaccgtgacactaaacgaagtgacaatcattgggagcgcaccgatctggggattaccgtgtttgtccagtagggccggattccagttggtgcccgataagaatttccataaactgacatggttcgttgtgaaggttgctaacccacgggtggtaatgaagtacagaattgagataaccagcaagctgacgaagccgatgcagagatacgtaatcccgcggccgaataagtcttcgtgcgtcgcttttgatgggttttgaagatcatgtttgatttcatccatgattaacctcctataatttagtcgaatgaattttaaatgagtaccttaacttgaggaaggctggaggcatttgatttgccttcagccttcgttggttttgtgtttagtttgtagagttaatggtgcgtgaagattacctagtgaaaacttggttcgagccatgagactgagttctaagtgcactttgattaaagtgtccttggaaaccgcctctccaggagcacgtttgttaggtgcttttgtgctcccttctgcctttaaaatacgctctgacgggccagaggctaacttctaagcgcactttaattaaagttccaaacccagaacttcaatcaaagtacccttagaaaccgcctctcccagcccttgtcgcgctcttacttttcagagacggcgttacttgcattcttcgttactttcatatcatgaatactgatgtaaccaagtttttgaactaagctgtcttgaaccttgcttgaatccatgtagttcaggaacttcttagttgctttgtttggttgacccttagtgtacatatgttcatatgaccagatcttccatttattggtggttacgttggcatccgttggctttacattgttaactgataatgccttgagcttgctgttaacgtatgagaaggccaagtaactgatcgttcctggtgtgcttgaaacaatcttttgaacagttccgtttgaatcttgttcttgggccttaactgctttggcaccctcaaggacggctgattcaaatgtggcacgcgtacctgaaccttgcgcacggttcacaacggtaatcttttcgttcttgccgccaacctgcttccagttagtatacttaccagtgaaaatgccttttaattgtgccatggtcaaattgctgacattgacatctttgttaacaactggtgtcattccaacaacggcaacttgatgatcaactaattcttttgctttaatcccatcttgttgttcagcgaagatatctgagttaccaatttgtaccgcgccggtttgaacttgactcaaaccagttccggaaccgccaccctgaacagaaatgttaacgcctttatttgctttttgataattgcttgctgcttgttcaactaatggctgcaaagcagttgaaccaaccgccgtgatcttgacattcgaatcagctgagcttttctttgacttagagctgctggacgaaccacaccccgcaagtaaaactccgacagctgctactgctacgatagttgaaaaaaaggatctttttttcataattcgatttcctcctaatgaaaacccaagtttttttagtactcatttaagtacattgttaatataacaacagcatgtaaatatcgagtttcgtttatgtaaaagtaacgtaaaaccggccatttttatcaaaaagtatggcataacttaagatgtaaacaatttaactaatatggaggaagaccggatgccattggaaatcttattgatcagccagaacttaaagctggcggataagcttgagaaactacttgccgcctttcaaattaataccagaatctcatttgaaccccttgatcatctgcttcaacaagtttccggagtcgtctgggacttagacacaactgaactgccggaaaacgattcggaactgcagattctccgcagtcaaattgccgggccaatcttgctgctggataaacagccacggtccgtggaaacgatttgttcctattttttggattatcatttggatgattacatttgtggtgaatcagccagtgaaatcgtcgcgaggattgttcaaaaaatttgggtctatcaaaataaagacaatctccagctgacacagcagagtcaggaatctgaaagtctggtggtcggtcacttgaagattgatttgagtaaatttgaagttaataatggtcgcaaaaagctcaatttaagtccgattgaatataaattgcttctattctttgtcagcaattccaacaccgttctcagccgaacccagattgcctcggcagtatggggtaacaccaccggggcgaccttgcgaattattgacacccatatcagtaacctgcgcaaaaagatcgaaatcgaaccaaaaaatccccagatgctaacgaccatcaggggattcgggtatttatttaagaataaaggcaaccagcaatctcaggtcccgtaaacgttgatcagacatcaaaagaggttgtgacaaatcggaaaatgttgttttagcctcgatttgcgtttaaatgttttctaacaaagctacgcaccaataagcagcttctggccgtataaggggattccccaaacatccaagttatggatatttggggaatccccttatactttggaagataacggcttagtggcccacgctcttcctatacacttttgcttgatgtttcaactcgcgctgacacagttcgacaaagtcgtcgccataggcatttctaatctcgttttcccattccccatcatttccctgctcatcaagcattggctggatccattggttggtgggtaagagtttaagcaatgaatgtttggtaaattgtgagaataagagattttcgccaaaatatgtcgctaattgatgctgaaaggctggtacatcaactggtagtaacagattattagcgttgttccggtcgcccagcaacagttggcaatcgaggaagtcgctctttaaatcaaacagcttatctttatgtgccttggcgatgtctggaaccattctgatgaaccaaattagtttatgatgctcaagagcaatcagtagatttaacacagcgatgtctttggaacttagcgtaaactttgcgttttggacggccactgggtgaagactgttggacacagcattaaataaatcaccaaatgtccccggctcttcccacaatacctcaatctggtgggcgttctgcagccaaagccgatgagtggcaatccgaagtgtcagccagaaaacttgatcatgatcgtcataccccttaatcagccagtatgaactggccgtggagcgggcatagttgctggcggccagttccaagccatcgggcagcgccgctcgaacagtctcaatcagccattcacggtaggagggtttatcagtaaattcatatgtctgttcacgtggacgtggcttagccattgagatccctccctttacatttaaaattcgtctcaatactagtttacgcttttttgaaaaagggaacaaaaagaacaccagtacttgattcgcactgatgctcagtttgaaataaatctgcatttaaattgtttcacatgaaacattatgctttaacagtcttaattgccaagaaatctttgacttggtcactcggaattgatttgataaccggtccaccaattgtgtgaatgtagatcagactcaaatggccgtcacgatttttcttatcatttttaatcttttcaaatacttggtcagaatccaataaatctgaagtaaccggcaatccaaccgcttctaaacgttcccggagttcttgagtgatgccggtcaaggccaagcccttgtcttcaaaaatctgctgcatggcaatcatgccaatgctgacggcttccccgtggcgaagaccgccgtcagaaagtgcctcaacggcatgcccaatcgtatggccgtaattaagcaattggcggaggccaccctctttttcatcacccatgacaatgtctgctttgtattgaatcgaatggatgctcaattcttcagcgttggctaaaatgtcttcaggtgagttgattgatttgactaagttccacaaatcaccatcggataaggccgccaccttgacgatttcgccgtaaccttcgactagatcgcgctttttcaaggtctttaaggtatctggatcgataattaccaaatccggttggtaaaatgagccgatgatgttcttggtggtatccaagtcaacggccgttttaccacccactgaactatcaacttgggccaacaatgacgtcggcatctgaatcagactaatgccacgcatgtaggtcgctgccagaaaaccggctaggtcaccggtcacaccgccacccaaggcaatgacaccatcatcgcggttgaaactgtcagcggccatttgccgggcaaggtcagctaaaacgtctacggattttgattcttcaccagcgggaaattggtactcgtgaacagtgaagccaacagcttctagagcctcagcgacttgggcctggtaaaggggcgcaacgttgctgtcactcaccagggcaattttgcgcttgctccaaacactggacaccaactgaccggtgcacccaaggattccgcgggcaatttcgacattgtatgaacgatctggtaaatcaactttaatgattttcataatttaacctcacttttttcttcgacaggggtcgtaatcactttccggattgcaaatgcctgctgagccatcgcacggtattcgtctggcttgagtgcttgagcgccatctgagaaagcgtgggcaggatcatcatgaatttcaacaactaaaccactggcaccaaccgcaactccggccaatgcctcgggagtcacaaattctgtgtggccggcggcatggcttgggtctacgatgactgggtagtgagtcagtttttgaagcactggaactgcgccaacgtctaaggtattacgggtgtatttgttatcaaatgtccgaatccctcgttcagtaatgatgatgttatggttgccaccggcggcgatgtactcagctgcatttaagatatcatcaatcgtagcagacattccccgttttagcattactggagtctgagtcttgccaactgccttcaaaagtgagaaattctgcatgtttcgggcgccaatttggaaaatatcggtgtattgttcaaccattgcgacgtgatcttgatccatgacttcagttaacacgtccatgtcgtaagcgtcagcggcagccctgagaaatttcaaaccatcttcgccaagaccttggaatgagtaaggagaggttcgaggtttaaaagcaccgccccgaaggattgtggccccaccactcttggcgactttagccatcttcatgacatgttcggcagactcaactgagcaagggcctgccatcatggtaaagttatcgccaccaatttgactgtgcggtgtcacaacaacggtgtcttccgggtgaaacagacggctgccttgaacagcggcgggaacgttgtcaataattaagtcaatggcattcttctcttcagcatttaagtcatcttcacttacgccttggattgccacgcggttgttatgaacaaatacctcgttggtttcggtaaagcggctcttgatctcgtcaataatgtcttcgtgcccgtttttaagtacaataatcataatattatctccatttctgtgtttgacgtgtttttgaataaaataaaactcccacagtgtgtacaacactgcgggagtcagaattttgggtaaaaaaattggtcccgcagtatatttggtaaataactgtgtgaccgaagtaagtaatcatgatgaaatactattggccgcacaagatgtgagtgagtgcccacatcctgtccggtgtgaacactaaacgaaccaatagtaataaaatcgattaatttttgaattaatttttatcatgattagaatctcctaagaaagttaaattttaattgcatagagcatataatgaattccaagatgtgtcaaccccaaagtttaaattatgaattttcttgacatcttctcataaagagcgtaattttaatggcaattaaataccgtcctaaataaaccattgaagtggagatcaagattgttgtgcacgtcaagagagtcgctattgctgagaatgcggccgaacgcaagcagttaaatggaccaccgagggttcttccgaaagtgatcgagtacgaagaaacgtgttggcatacgtcagttgtcggagggatgttagtcccttgctaagcgtagttgacggaaaagagtgactctactgaatggtggactgtctttttcgatcaattaaacaaaggtggcaccgcggaatgatccgtccttaatgtgaaaacatttggggcggattttttatttagagcgcgacgagggccgggagaggcggtttctaagggtactttgattgaagttcctgggcttggaactttaattaaagtgcacttagaagttagcctctggcccgtcgccaagtaggctaggcagggtttcacccggccgtcggagcgtattttcaaagcagagggagcacacaaaaacctaacaaatgtacttctgcacaggggacgaaacatatgccaatcaaaatatgacgcaatccggcaaataccaaaaaatggaggaacctttcatgaaaatatcaagaaaacgatggcaaatccaactttagcatttagcaaaacacactaaagcaatggaggacaccatcatgaatctagaccaacttaaacaatatacaaaggatttttcagctataccaatttcaattaatttcgcaatgccggactttgaccctattgccgtgacgcaacgattcgatcagccagacgcaccgtgtttcttactaactggaaaacccaagcaacaagaagacgggtattcatttatcggattgaacccaactctgaccattacttatcgaaacggggtcttaacccgctcagatgagcaaggcaatgtttcacatgaaacaaccgatttaaagcccgtcctggaacggattctggcagataatagaatgccaaaattaaaacacatgccgccattttcaggcgggctcgtcggttacttcagttacgactacgctcgctatgcgactaccgcagatttaccagccgtcagtgacccaatgaaactcaatgatgtcgacctgctgctcattaatcgggtcattgcttataatcacacgaccaaaatggtcacgttaattcaagtgatccctgccgatcagcttacgacgcaatatgaatcggtgatgagttccctaactgatttgaaggacgaaattatgcaggttcacaagcaacagccactcccaccatttacaatgacgccattcaaattgcagttctctttatgcgaattcgaggaaaaggtcgcagaagcaaaacatcacattgtcgatggcgacatcttccaagtccagctctccaatccgcaacattccaaaatgaccggttcgctgtttgctgccacgccaactttattcaaagaaagcccatccccgtatcaattttattttcgccataatgactttgaaaccattggtgcttcaccagaaactatgattaccaaacgggacaacacgttattcacctacccgttggctggaactaggcgaagggggaaaaatcagcttgaagacgatgcttttgccgacgaactacagcacaatcccaaagaattatcagaacataatatgctgattgatttaggaagaaatgacctggggagcatcagtcaattcgggtcggtcaaagtgaccgcttatcgaaacctgctgaagttctcgaacgtgatgcacatgggatccgtggttgaaagtaaagttgatccagacgtttcgtcaattgatatcattcattcattactacccgctggaaccctatctggtgcgcccaaaatatccgcgatgcagattattggcgaactggaaaacaacaaacacggtctttatggtggctgcctaggctatctgggttttgatggtgacctcgatatgtgtattgggattcgattagcatatcggaaaggtgatgatttagtcgtccgcagtgccgccgggattgtcgccgatagcatccccaagcatgaataccaggagtttaacaataaagccagagcaattgtgacggcactgcaggaaacggcagccaaaggaggcgtttgcgatgcattatctaatcgataactatgacagtttcacatacaacctataccaattgattggtacccagacctctgaagaaatcaaggttgtgaaaaacgatgccatcaccgttgaaaatttaatgaaagcaaatcctgaaagcatcattttctcacccggacccggccgcccagaagatgctggtaacatgccggcgatcttagacgcattcctcggcaaggtcccgatttttggcgtttgccttggacatcaagccatcgcagaagctttgggggccaaagtagtgcacgtccccaagttaatgcatgggaaaccctcaaatatccaaatttccttagacgatccactcttcgcggactgcccacgtcattttgaagcagccaggtatcattcactcatcgttgatccaacaacggttcccgatagcttggatgtcaccgcggtaactgatgacggagaaatcatggcgatcagcaatccagccaagatggtctatggcgttcaattccatccagaatcaatcatgactgatccagaagtgggaaaacagattatcaacaattttctaacaatcgtcaagatcgctaaagtatcgactacagctcgttaaaccgaaaaaagggattgcggcaaaactaatcattttgccgcaatccctttagttttcatatattctattgaacttgtctgagcacttgcgagcggctgagcatcttgaatattgctcggacacagacagcaccgaagaagaacaccgagatcagacggactgagaacaacgccaagatcattggcaggtgataatgaacataacccaaacggaacagttcatatccaaaggaaaccacggtggtcgtaactgctgaggtagttagtaccggccagccccagttcttgtatccccacagtgtgaacccaagctcacttccgattccttggacaattccagaaataagtgcactagcaccaaaggttccgccaaaaatgacctctgcagcggcacctaatacttcaccaataattgccgctcccggcacccttaccaagtaaatcgacaatggtccggccataatccaaaggccaaacagtgcctcgtttgagaatggtccaatggcaactgccaggaaattatacagataatctgtcccgacaaagatggcaccaaaaacgattgcaacaatggctaacagaatcacatcctgtaagcgaaatttctttttcatgatttttctccttttgaatgacaccaatcataaatgaatgcggccataattttggtatacgttaataattgctgaaaactaagactttcattatcactatgagcttgtttcatggttcccggtccaaaatcaaccgctggaatatggtagtagccaaaccaaccgctatctgatacagacggtgacatccccaaggttggttgtttgccggccacttcggcaaagttgctctcaagtgcctgcatccctggatggtcggggtctagctccagtgacgggaacacctcgcctttatcgactaatagcgaatcgccgccccaagtaaaggtgggcagattatcccgcagccaaggatcgacttttgctgcagcaaggacttgatcctcgatttcatgggttatatcatcaacattttcattcgggtaaaaatgcacggtgatccataatttcgtgacgctcggaatgtaagccggatgcagacccccttcaatataagccgggttaattgtatcgattcccggggcaaacccaggataacgcttggtgatcccccagtactgttccaatttctccaaagcctgaatcacgaccatcattttctcaatcatattagcggctttcaggccaccaccagtagtaatcattgctgctcggttcccatcgtggtaaatgtggggactcttgagtgtaatccagccggtcacaacgcctccctgaccttgaaaattcaagttgctggtatcgccaaccactgcaaaatcagccgtttcaccatttttcagtaaagttttggttccggcttctccagcctcttcaccaacgacagattggaaccgcaaatctccaggcaggtcaattccaagctgcttgagaagtgaaaaaatatacacaaagctggaaatgccgcccttcatgtcactgacaccccgcccgtagagtagatcaccctcgtggactaatttgaacggatcggtgtgccaactctgacgatcaacggtagccacatcaacatggccattcaacagcaaactatgatagttggctgcatcagtccccgctttctcagccgagagcagctcatcgccatcataaaaggcttctcgcttagtcttaaatccaattttggttaatttatcatcaagaaaacgttgaattgccactgtgttgcgggcaggtggtgacatcgtttcaaatgaaattagccggtccaataacactaacagttgatcttggtgcgcatcaactgcctgaagtaacgcttgcttatctgtcaacttcgactccctccaattatctgatcatctatggtttggaaacaaaaaaaaccccctttcttcaaagcctcgaagaaagagggaacagattaaaagttgaatcgactttatatctattagctcacacaaaaaagtttcgttcttccttcgacagtcctaactgcatcaggttcaatgggtatttatctcagccgtttagggcaccccagactactttattcaatttgccgcaaattacgtggctggttttatgatataacgaattgacgaaatgtcaaagttaattttttgatgttgtgaggtcaaggcccgtgagcctacttgctgatgggctgatcccggccatttaagcaaagaaacgagtcattccaaaaacaggaataactcgtttcttcacttaaactctgggatcaaaacgcctcgcgtcccactcccacaatcgtttcatttgaccaaaatgaaaactttattctcgaaaattcagttgattatgatgttgccagaccgcctgtccagtgactggcagcgctgctggtatataccttaattgagtatgttccggaaccgacccacaggctaccgctcaatgtgccagtggatgaactaatcgttttgtatagttcaccatctttgtagatactgattgaaaatggatcagcactggaggcgccactatccgttgacgttttaacattgtagtgcaaagtattaatgagattggttgccttgacggtcacattgtagccagaattgtcattagtgtactgactgcctgtctcacgaggttgttgggacagatttttaccgccgacctgcttagcggccttggcattgtcctgtttatggccttgctgttgtcgttgaggttgaactgtatcggcattggcaacaacgctgctcagaaatgttggggcaaccattgcggctgcagccccaaatgtcactaaatattttctaattttcatggatgataacttcctttcaatttaacgtttgttggtttgatctggaacctatttcagttgccctcccttcatacttgatgttgctagaatatcggggcaagcttaattgggacttaaattagttaaaattgagaaggaagccgcataatctttagaaatccttgggacttttgtaaaatttggacagcaaaaaaggtcaatcaatgaacgtaaatcgttcaccaattgaccctgccaacttcttcaatgaatctgatcaacctattcaaccttaaagttcgacttgaatataaacccgcaattagggcacctgttcaagccgtaactgatggacattggtcgatgacactttggacagttgccctgcatcggccggcgaatcttagttggtttcggttctttctcatctgcctgatcactcatattgacctccactaaaatatcattactgatcgataatctttagaaactttgccggcattgaatccaccaaccaaacgccactttcggttggataaaataacagtcctgaagccgcggcttttcttgcttcaatttcaaaaatcacaggatgaggatcacgccgtttccccacctgaatcgccatttggggatttgcggataaatggacaaaatcccgatccatcttttttaatccttcatcgacaatgaatctggcagccgcatgagtcgttccgtggtacagcttctctggaggttcaacgggtggcgtcagtggatcaacgggaatgctgtggccgtatagcgccctaatcgtgtgaccttcaatcgcataacgttgtttgtcactatctttcataatttctcgaatgattttctcactgattggcgtcccaaagtgctggttaaatttttggatgagggtttgtaagtccactcgtccatatcgatccaactggatgccaattttgtccggatggtgtctgaggacgtacgacaggcgtttgctcaacctggttaattgatgatccattttactgactccaatcgtttcaatattatctttattataatcccaattgtgggcaaaccacaaaaaacgcccggtactaaggcccgggcgttgctacaaatcatattcatattagaggggatcttacttcttgggggagacgtaagataatcaagttttatactttggaggagtaaattcacttgtaaaccaatttatctttcaaaattgattgtctttatattatggttgccaacttaactcagccttaaataagtgtgacaaaattgtgaagttgcagaaagggcggaataggggtgttgtttatcaagatttcttatataattggatacagaaaacatttgaaaggattcaacatgaaaaccatttattttgtgcgtcatggtcaaacgttactcaatcaatttcgccgaatgcagggctgggtggactcaccattgactcaaaagggcgagtcccaggcaaaagcaactggtgaaaaacttgcagatgtccattttgatttggcaatcagttccgatatgatgcgggcaattcatactttagacattattttggcaaataatcagtcctcagctggcgtttctcgagaagtgtccctggacgttcgagaaatttacttcggttcgtttgaaggaatcgacagtatccaaacctggaacatgattggcggaccgctgggacatcgtaatcaagaggacttgatcgaagaatatggcctcctcaaaatgcgtgatttcatgcatgccgctgatccatttcacgaagccgagacttctgctcatctcgagagtcgaatcaacagtgcagtcgaacatattcaatctgaattagtagacggccaaaatgccttagttgtttcacatggaacttttctgagaaacctggcgactttgtatactgatgatgcaacaagtgttaagcagccccgtaacggtagcattacccagctggatgtgaccgacacgccgcatattatttcctacaatgaataaaaaatctcaccaaaagattgcgtaattaatcttttagtgagatttttaagttatcgttaatagcctagactgttcacgttggttcgtttggtcttgttggtttcccagaagaaggtcttggcaacgccggtaatcttcttctttggaacaaagccccaataccgaccgtcatttgagacgcttcgatgatcaccaaggacgaaatactcacccttgggaaccttggtggcattggtatttttgtcccagctcttggataatgatttcaaattccaattgccggttccagtcgtccgttcgctcatgctaatgaacttctggggaacaacttttccattcacatagatattgccgttcttactggagaccgtatcaccaggtaggccgatcacccgcttaacatagtctgttttaggcttggtagccgttggatcttcaccatgggcatcaaacacgataacgctcagatgcttaatcttggcatgccgccaaacaatcaagcgctctttattaacgagattgggttccatcgaaggaccatcaacccgggcaaacgtgaagacaaactggcgaatcaatagggcaaccagcagcccaaccaagatggggatcacccagctcataatttctttaaatactttcatcttaagctcctttgtgaacaacacaattagctatgcatactatccataacggttagcttacacaatcgatattaattttatcacatttccccgccagaacaactttttcgcgcttaattaacagaaccctaatttattgctcatattgcaatcaaactgtatcataatttgtatgactccgcttgtgaaatagaggtaacaacatgaacacaaacctaaaactaggaaataaaatttggctggtctttattctgggaacgatcagtgcaaccggaccgctgtcaatcgatctgtatttaccggcccttcccgaaatgacccgtgacctatccgcccagccttcactcattcaactgagcctaagtgcctgtctcatcgggttagccctggggcagctgatttctggaccattaagtgacaaatatgggcgcaagaagccgttgatgatcgggtttttcatctttggtctggtatccttgatgatcgcctacagcagttcagtttatctgctgattggcttaaggttcattcagggtctggctggggcaagtgggcaggtgctctcccgggcaatcgcttcagatatgttctcagggcctctgctaaccaaattttactcgatgctatcagcggtcaatgggatcttcccggtcatctcaccagtcattggcggctttatgatccgctatgtcgagtggcagggaattttcatcctgttagcagtcattggatttgtcttagtcctggcactctggctgggaattaaggaaaccttacctcaagagaaacgaatttctggcagtccggggaaatcaattggtcaaatgtttaagttattgaaaaactcgcgctttgtccgcctagtgctggcaactggattggtctccggtggtttattcagctatatttctgcttcatcatttgtgttccagaacttcttccacatgtcagttcaaaacttcagcctgctctacgcgttgaatggcatcgggatcgccattggctcagtcattccaggggccttggcgggacactttagtgaagctggtcaaaccaaagttattttgacatccacctttataacttctgttctactaacattgagcgccttattcttgaacaatctcctgctggtgattatcttagtgttcttaacggttactcaatttggaatgttatttacattaaccacttcaattatcatgaacctcacattacataacaatggcggcctgtccgcgatgttgggcttgtcgcaaaatgcaattggcggggtcatgtcaccgttggtcggattgatggggactgggacctatctgccaatgtcagtggcaattatgggatgtatggggttgagtttatttcttttcagtactattcataatagtcaacgctcactcagttaataaaaacggctgggagcaaaatttgctctcagccgtttttattgtgctgttaactaaatgatcatatttaagaaccggcagccaaagtggtagagcggttcattagactttaaaactactcagccagcttactaatcttcccctgttgaatataaacgctcaaaatcgcgatatcggcagggttcacaccactaattcgtgatgcttgggcaattgtctcaggatgaattttctgcagcttctgacgggcttcggtagcgatgccatcaattgcatcgtaatcaatccggtctggaatctttttggcttccatccgcttcatcttttcaacactttgctcggctttcttgatatagccggcatatttggtctgaatttcaatttgctcgatcacgtgacgatcaggctttgtctctgcttggggaatgaaccgcatcaatgtctcgtaatcgacatatggccggcgcagaaagattgatgccagtaccccgtcttgcagcggtttgtcaccgtgttcttggacaaattggttcacctcatctgatggcttgatccgaatagtgttcaaacgatcaaattcagcttcaatggcctttttcttagctaagaacttagcgtagcgctcgtcagaaattaagccaatttcgtggcctttttctgtcagacgcatgtcggcattgtcagtccgcagcaagagacgatattctgcacggctggttaacaaacggtatggttctttagtccctttggtaaccaaatcatcaatcatgacgccgatgtatgcttcatttcgttttaagacaaatggccctttgccaagtgcgcgacgaccagcgttgatgccggcaattagcccttgaccggcagcttcttcatagcctgacgttccgttagtctgaccagctgtaaagaggtttttgacgactttagtttccaaagtcggcttcaattgatagggcgcaacgacatcatattcgattgcgtagcctggacgcatcatctgggcattttccataccaacgattgaatgaatcatcttttgctgaacctcttcgggcatcgaagttgacaagccatcgacataccattcctcagtttttctgccttcaggctccaaaaatagttggtggcggctcttgtcagcgaaccgaaccactttgtcctcaatggatgggcaataacggggaccgacaccttcaatcactccggtaaacattggtgcccgatcaagattatcgcggataatcttgtgggtcgtttcattcgtgtaggtcaaccagcaagatagttggtccttgactgccaggtagttctcatcagaagattcaaaactaaagtggtgcggtttctcatcgccaggttgttcctctgtcttggagtagtcaatcgttgtcccgtcaactcgcggtggggttccggtcttgaaacgttccaaatcaaagccgagggcttccaagttacctgaaagtttttcagccggctgtgagttgttaggtccagaagcgtacatcaactcgccaatgataatttttccacgagcagctgttccggcagcaatgacaaccgccttggcataacactcagcgccagtattggtgataacccctttacaaacaccgtcttcaacaatcaaggaatcaacaattccctgacgcaaagtcaaattgggttctttttcaatcgtatgtttcatctcggcgtgataggcatgtttgtcggcttgtgcacgcaacgcttggacagctgggcctttaccggtgttcaacatccgcatttggatgtatgtcttatcaatattcttgcccatttcgccgcccaaagcatcaacttcgcggacaactgtccctttggcagggccaccaacggatggattacatggcataaatgcgaccatatccaaattaatggtcagcagtagcgtcttgttgcccattctggcagcagccaaagccgcttcacagcctgcatgaccggcgccgacgacaatgacatcataatcttggccgcgatatttttgtttaacatcgctaactcgtaaacttttcactgtttttcctccaaatgtttcacgtgaaacaggttattttcctaaacagaattgactgaataactgatcaattaactcatcttggtaactgtcgccggtaatctcacctaagaaatcccagcagcgggtcatgtcgatttgaaccaaatcaaccggcatgccatcatccaatcctttgacaacgtcttccaaagcctgtttggcttgatttaacagaccgatgtggcgagcattggtgaccataatgtcgttttgactgctttcaattccttcatcaaagaacatcttggcaatcaattcttccagctgcgtcaacccgtctgccttaatcgctgaagtcgaaataacgttctggccgtcagctaaagacttaatttggtcttgatcaattttggttggtaaatcagtcttattgaggatgataatccgttgtttgtcttgagtggcactcaataactttttgtcctcatcggttaatggctcactggcgttaagcaccagcagcaccaaatcggcactattaatggcttttctggaacgatcaacaccgattttttcaactttgtcagtcgtatcgcgaattccggccgtatcaaccaattttaacggcacgccgcggacgttgacatattcttcaaggacatctctggtagtaccgggcacatcagtcacgattgccttgtcttcatgaagtaaattgttcaacaaactggacttaccgacgttgggccgaccaataatcgaagtggccaaaccttctcgtaagatcttgccttgtttggcagtcttcagcagttgcacaattcgcgcatggacatcggtcgccttttcccgtaacaatttactggtcatggtttcaacatcatcgtactcaggatagtcaatgttgacttctacttgggcaagcacgtcgagaatatcttggcgtaaatgtttaatcaaatgcgatagattaccatccaattgattaatcgcggctttcattgagcggtcggttttggcttcaatcagatccatgacggcttcagactgtgacaaatcaattcgcccattgagaaatgcccgtttggtaaattccccaggctcggccatcctagcaccgtgactcagtgccaactgaagaattcgattggtggcaacaatcccaccatgacagttaatttcaacaatatcctcttcagtataagtgtgaggggctctcatcacggagagcattacttcatcgacctcttcgttggtatccggatcaatgatgtggccataattaatggtgttgctggcaactttatcaaggtctttaccacgatagagcttttttgcaacatcaagtgcttcttcaccactaatgcggataatcgaaatcccgccctcaccaggtggtgttgaaatcgctgcaatcgtatcaaattctgttgttgttaaaaccatgattaagcttccctccacgaataattgaatagtgttctaatttaaccacaaaacttatctaaaagcacaaaaaaagcgccactccatgccaaaaaagatagcatggataaagcactttgactactttacctagttaagataagaatgattacctacataatattttaaagcaatgcatttgtcaattgattttgagaactattttggtgcaacgacaatgacacgatgaggttctttgccggttgaatacgtcatcacgtgatcattgtcagccaaagcattatgaatttgtttgcgttcaaatgccggcattgggttcaagtagactggcttgccgttggcaatggcattccgagcagtcttatcggccagttgaaccagcgactcgcttcttctggaacggtagtttgcagtatccaactcaacggtaacgttgttggcacccagtcgattaataaaaatctgtgacaagttttggagcgcattaatcgtgcggccatgacggccgattaagcggctctcctggtcagtatcaatgtcaatatagattgaatgccgattctttaaatccagcttcaatttgaacgagaagcccattgcttctaaaacatcgttcaaatagttggcaagtttttgggaaacttcttcaatgtcaacggcgttttcagtttcttcctcatggtgttttgattctgaaaccggctgattagttgatttattaagatttgtctgttgtttagtgttagttttactgacaagttcaacctgtgcaagtttgcgaccgaaacctaaaaatccattcttaggttgttgaataacggtaacttcaacttggtccgaagtgagtgatagtgcggttaaaccctgttctacggcgtcttggatggtttttccagagtaaattgtcataatgaactccctttatttgaattaactggttaataatagcataaaaacgcgcattattaaacggtttgttgcgaaaaacggaaactaaacgcaaactttaaatgatttgtcacatttcaaagcatcaaactaccatctcactgcaaagtcgatataatggggtgtagtagcttttttaagaaagatggtttcgtctgaatcgacatcaatctatagtgacggctgctttaggttttcgatttgggaagtgataaaatggcaaacacaaatcaatatgacgccggccgaaacattcaaatcgaccgtcagcaccggcttagcaagcttcaggaagcctcgcagatcacctgggtcaacctcagtgcctactcggccatcatggttgccgaactgatcattgggtatttggcacaaattaccgttttgattgccgatgggctgaataacctgaccggtgtttgtggggcagctattttaatcattggcctgaaaatgtccaagcgcccaccggactccaatcatgtgatgggtcattggcagtatgaaaatattgccgcacttttatctgcgacgatcatgtttgcagtcagtatccaaattttcgttgacggcgtttttgctgtccagcgattcctggctggtcacaccattcgaccgaatgactggtcactgggtgtcagcatcattgcagccataatcattggtatcttagcgcggttcaataaaaccaagggcatccaacttaaaaatcaagcactcacagcttctgggcaagaccttaaaagtgatgcctggaccagctttggaacatttctttccattggcggtgcctacctgggggctcaatggttggatggagtggcaactttgattgtcggctgcctgattctccactcatcaattagtatttttagaacaaccattatgagattgagtgaaggttttgatccaaaagatattcaacgttatagtgagaccattagtgccatccctggggtcctcggaattgaagggattgagccacggtggctcggagatcaaattgtcatgaaaatcggcatctatctggatgatgacaccgatttaaaaacggcttatgcaatcggtgaaaaagttgaacacaatttaatggaaaaatacgacattctcgatgccgacgtgatgagctatccagtcagccaaaaagacaatcctcattcggcagattaatcaaaacagtttgacaaataaaaaaatcagcgctatattcagttttaattaaatgataatttgttaaacaaaacgaatcggtgagtagtttgaggttgtctatcagagagttggcgttgatggaagccaatattcaacttaaatgaagatggccgatgattggttgttgtgagtcaataacgagcagcagacggatgagtccccgttagcagacacaccatcgactttcgatggttatcaaggtttgacgagtaatcgtcaaataaatcagaatggtaaagtgttattcgcttctgcagcattggctgcagaagcgttttttcatttaatgaataaaaaattataaatttggggtggcaatcatggcaaaattagcaattgtaactggcgcaggacaaggaatcggagagggtatcgctcatcgactggcgaaagatgggtttgcgattgcggtcgcagacatcaacggggaaacagctgataaggtaaccgcagatttggtgaatgatggttacactgccaaatcgtatcatatcgacgtggctgaccgtgaacgggtctttgaattagtgcaaaaagcggttgccgatcttggcgaacttgccgtgtacgtcaataatgccggggttgcttttatcgatgaaattgttgattccgcggaaaaagacatccggcgattattggatgtcaatttattagggacttactggggaacccaggccgcagccgaacaattcaaaaaacagggtcacggtggtcgaatcgttaacgcggcctcccttgccggagttgaggcatctgctctgcaaagcgcttattcgatttcaaagtttggcgttcgcggcattacccaagcagcttcaaaggaattggcaaaggaccaaatcaccgttaacgcttacgatccaggaattgtcagaacacctctaagagacggcatcgacaaacggaccgctgaaatcaaaggaatctctgtcgctgaacaacaaaaaaactgcctcagtgaaatctcactgggcagagaagcgacaccagaagacgttgccaaagttgtttcgtggtttgcatccccagatgccgcttatatcaccggccaatcaattcttgtggatggtggcatgaggtatcaataggataatcgaaaacgagtgtaatttaacaggacagccatgagcacaatctcatcgcgctgtctttttgtttgaactctgtccgttaagccattttaataacaatctttccaacggaccggccggctgcggagtaatccacagcagattggatatcgaaaaacggcaccacccgatcaatgaccggctgaagggtcccgtgttcgaccattttggttatcttggccaattgggtcccactaggtttcatgaataaaaactcatagccaacctgaaattggcgctgcagtcgcctaatttttgctgtagccagggaaaacgccagttgtttccacattggcaggccagcctgctgggcgaatgcccgatttggcagacccgaaattgaaaccactttgccgccgggtttcacgacttgaaacgcgttagctaattgtgaaccacccagtgtatcaaacacgtcatcgtaatcaaacaagacatcttcaaatgccgtttgatgatagtcgatgacctgatcggctcccaactgcctgaccaaacctgtattctttgcgctggtggtcgttgccacaaaagctcccaatgacttggccagctgaatcgcaactgtcccaatcccaccggaccccgcctgaatcaagactttatctccaggcttaacgtgcatcaagtcaattaacgcttggtaactggtcagcgaaaccagcggcagtgctgcggattccaccagtgataagttggccggtttcaaggcaatatcaccctgatccacagccaaataatcggcaaaagttccgatccgattcttctgcacccgaccatatacctcatcaccaaccttgaagtctttcaccaatgttcccgtctgaacaactgtcccagaaaaatcactccctaatctcaatggcatcgaatatttcaacagcattttaagtttgccatcgcgggtctttaaatcaattgggttaatacttgccgcagcaactttcactaacacgtcatgatccccaattgttggaatcggcacgtccgcgatctctaattgctgctgcccaaaatgctggatctgggcagctttcatcatttttgtcattattactagctccactttattggtttaaatttttgaacgaatagtgtccaaatcataaatcacaatttgctgggcgtcaagcaagactgtttaatgccaattcattgacggctgacaaataaaatggtttaatggtttaaaaatatgaaccgaaaggaacttacgatggctgatttacaccaaattcaaactgaattcgccaatatcagcagtttcttaactgctttaggggaccaaacacggcaagcaattatcatttctctgctaaaaaccaattcttgtgaggggctgcaagttactgagcttaccagtgtcaccggcttatcgagaccggcagtttcccaccatttgaaaattttgaaagatgcccatttagttgccgtcagaagtgaaggaaccaagaacttctactacttgtcccatgacatcaaggagattaatgaactaaaaacccttctggaccatgtcacagcaatcattcatcaaacggagaccaaatcatgaaaaaagtattgattgttttaacgaatgttacccgttatcaaggcaccaacgatcccaccggtttatggttgggggaagcaactgaatttgccgaaacaattcagaaggctgggattgacgtcgactatgtcagtccaaagggcggctttgtgccacttgatccacgcagtatgaaatacactaatgagtcgatcatgaaattctatgaaactgaggattttcaaaaacgggcgttgaccaactcactgcggccaaatgaaattaatcccgacgattatttggcaatctactacactggcggccacggagtgatgtgggattttccaaatgaccgagccctccagcaaatcgcatggtcaatttacgacaatggcggatacgtcacatccgtttgtcacggagttgcagggttgctcaatatcaaagacgatgcgggtcgctatttaattgccggcaagtcaatcacgggtttcacaactgcagaagaaattattgccggtaaaaaatcagtggtaccctttctgaataaacaagcagttgaaaagcgcggtggtaaattcaaaaagaagcgggcttacaaggagtatgccattcaagacggtcgcttgattactggccaaaatccattctcaccacgggctgtcgctcggctattacttgaaaacgtgcattaaataaatatattaaagcggggccaaggcatcagtgtattcgactgataccttgaccccgctttaagtttggacgctaaatcaaacgtccggatctcattagttgatgagctgaatcagcttcccaatccgaaaaccagtctgctcaatcaattgaggagcttggtgaatcgcttcttgaacggtcagcggacgagtcgtcgtggaaacaatcaagtcaaatccttgatcgtataaaggctggatatcagccgccaaactcccggcaacggcaattaccggaactttggctgaatcagccagtttggcaacccccatcggcaatttgccgctgagggtttgtgagtcaatccgaccctcaccggtaatgaccaaatcagcatcacaaagcatcgcctttaagtccaccaacttcatgatttcctcaattcctgacgttaacttaccctttagaaaggccaggacgccaaatcccaaaccgccggctgctccagctcctggtacctgtgaaaggtccttccccacagtagcagcagtcagtcgcgccagtcgttgcagccgggcatcaaaatccgcaatctgttcatcttgaatccctttttgtggcccaaatatccgtgtagcacccaattggccggtcagtggattctcgacatcagaaagaccgatcatttgaactacggatattcggtgatcaatctgggtcaaatcaactttggccaggtctttgagtccaccaattccacgggagatctcatgaccgtttcgatcgtaaaaatgaccacccaaagcctgagccatgccaacgccaccatcgttggttgaacttccgccaagtcccagaaggattttgctgacgccgtgatccagcgctacttcaatgagttccccaacaccataagtcgaccgaacagcaacatctgtcgtttggccttgcgtgtatccagccgctgcagccatttcgatcactgccgtttgatcatcaatcagaccccatttagcgtcgatttgactgccggtaggtccagataccctcgtcgatattaaacggcccttagtcgcgtcgacaatggccgttacggtaccttcacccccatcagccagcggtacttttttgattttaagactgggattggccactgtaagtccccgttgcaaattctccgccacttcctgtgagctggcactgcctttaaatgaatcggtcgcaattacaattgttttcatcgtcaacttcctttaactaactgttgaccttagtgtacctgaatatggatcgttcaacaaaaaagcagcgtgatcaaatgatcacgctgcttgctaattatttacgtttactcttcttggcacgtttaatggcttttttaattgcccgttgtttctcacgctcttcgcgttgtttattttcacgttcgcgacggatcttccaaggattttggataaccagggtttgacctacttggaacgcgttggtgatcacccaataaagtgacagggctgatggcaggctaatagccataatcaaaatgaagaatggcattccgaccgtcatcatcgtggtcattgaattagattcaggctgacctttcattgccagccacgaagaaatgaaggtgaacagggcagctaggatcggcaagacaaagtatggatccggatgaccaagctgcagccagaagaacgttccacttctcaaaatgtgggttcgccaaattgcttggtacaaggcgaacagaattggcatctgaacgatcaatggcaggcagccggcaagcgggttaatgcctgcttcggcatacagcttcttttgctctgcttgaagcttctgaacagtttctgcatctcttgatgaatattttttctgcaatgccttcagctgcggttggacttcttgagtcttacgcatacttctggtttggtaaatcatcaatggcagaatcacgatccggacaagaatggtgaagataatgattcccattccgtagttgtcgctaaagaatttagacagccagatgatggcccgcgagaagttcaaaacaacccagccatcccaaatgcccgtactgtgattggttattggtgcgttactacatgcggaaagtactaccgtcaaacttactaatgatagtaatactagtaatttctttattctctttttcaacttttttcctcactatcatagttgggatcgattagtttagctaacttgagcacatgaattaaacttgccttgacatcactcatcgacatctggtcagcagccggacgggcaatgacaataaagtccacgtcctgacgaagataaggctttaattccaacaaggactgacgaattcttcgcttgacccaatttctatgtaccgcattaccgatcttcttaccaacagaaataccgacgcgaaaatgtaattgattgggtttatccaaagaatagacaacaaattgacgatttgcaacagagttatgagtctcaaagacttcttgaaattcactctctttttttactcgatacgattttcgcatgatccatctccacagacttttgaaaaataaatgaaaaagaccactgaatggtcagtggtctatgcagacaatgattttctacctttttgacgtcggcgagccaacactttacgaccattgctggtactcatacgtttacgaaagccatgaacgcgagcgcgatgacgtttctttggttgataagttctcttcataatgaattcctcctttaactgtaaaagtcgcgtttaagcatttaattacaattatgttcaaatgcatttcccaaatatattaacataatttgttcattaatggaatagtcttttgaatgatcgcacatttcaaaaaatatttaaaatttgtttcatgaacaattagtgtggataaccgcagaaataatcatagctgattttagagatttgcacaaggttatccacaagctcacaccgtgttcc
